European Patent Application EP 4 570 815 A1, published June 18, 2025. Title: Bactérie du genre Corynebacterium, et ses utilisations cosmétiques. Applicant: Laboratoires M&L. Application EP. The sequence listing filed with the application follows.

SEQUENCE LISTING (26 sequences)

SEQ ID NO: 1 - DNA, 3459 bp, Corynebacterium sp.
  source 1..3459: mol_type = genomic DNA
atgaatatggctgaaatccccggggcacccgaacgctactcgttcgcgaaaattgcagagcccatcaccgtcccgggccttctcgatgtgcagcttgattccttcgcgtggctcgtcggcacgccggagtggcgcgaacgcgagcaggaactccgcggcgagaccgcgaaggtgaccagcggcctcgaggacattctcgaggagatctccccgatccaggactactcgggcaacatgagcctgagcctgtcggagccgcgcttcgaagacgtgaagtacacgatcgaagaggcgaaggacaaggacatcaactactccgcaccgctgtacgtgacggcggagttcatcaacaacgacacgcaggagatcaagtcccagaccgtcttcatcggagacttcccgctgatgacggacaagggcacgttcatcgtcaacggcaccgagcgtgtcgtcgtctcccagctggtgcgttccccgggcgtctacttcgacgagacgattgacaagtccaccgagcgtccgctgcactcggtgaaggtcatcccgtcgcgcggtgcgtggctggagttcgacgtggacaagcgcgacaccgtcggcgtgcgcatcgaccgcaagcgccgccagccggtgacggtgctgttgaaggcgctcggctggaccaccgagcagatcacggagcgcttcggcttctccgagatcatgatggccaccctggaatccgacggtgtcgccaacaccgacgaggcgctgctggagatctaccgcaagcagcgcccgggcgagcagccgacgcgcgacctcgcgcagtccttgctggagaacgccttcttcaagccgaagcgctacgacctcgcgcgcgtcggccgctacaaggtcaaccgcaagctgggcctcggcggcgaccacgagggtctgatgacgctcaccgaggaagacatcgccaccacgctcgagtacctcgtccgcctgcacgcaggcgagaacgagatgaaggcgccgaacggcgagatgatcccgattaacacggacgacatcgaccacttcggcaaccgccgcctgcgcaccgtcggcgagctggtccagaaccaggtccgcgtgggcctttcccgcatggagcgcgttgtgcgcgagcgcatgaccacccaggacgcggagtcgatcaccccgacgtcactgatcaacgtgcgcccggtttccgcggcgatccgcgagttcttcggcacctcgcagctgtcccagtttatggaccagaacaactccctgtctggcctgacccacaagcgccgcctctccgcgctcggcccgggtggtctgtcccgtgagcgcgccggtatcgaggttcgcgacgtgcacccgtcgcactacggccgcatgtgcccgatcgagacccctgagggcccgaacattggtctgattggcgcgctggcctcctacgcccgcgtcaacccgttcggcttcatcgagactccgtaccagaaggtcgtcgacggtcagcttaccgaccagatcgactacctcaccgcggacgaagaagaccgttacgccatcgcgcaggcggcgacgccgatggacaaggacaacaacctcaccggcgagcgcatcgaggtccgcctgaaggacggcgacatcggtgttgtcggccccaagggcgtcgactacctcgacatttccccgcgccagatggtgtccgtggcaacggcgatgattccgttcctcgagcacgacgacgcgaaccgcgcgctcatgggcgcgaacatgcagaagcaggctgtgccgctgctgcgtgctgaggccgcctacgtcgccaccggtatggagcagcgcgccgcgtacgacgcgggcgacaccgtgattaccagcaagggcggcgtgatcgagaacgtcaccggcgacttcatcaccgttgccgccgacgacggcacgcacgagacctacatgctgcgcaccttcgagcgcacgaaccagggcacctgctacaaccagaccccgatcgtgagccagggcgagcgtgttgaggccggccaggttatcgctgacggtccgggcacgaagaacggcgagatggcgctcggccgcaacctgctcgttgcgttcatgccgtgggaaggccacaactacgaggacgcgatcatcctcaaccagcgcgtggtggaggaggatatcctcacctccgtgcacatcgaggagcacgagatcgacgcccgcgacaccaagctgggcgccgaggagatcacccgcgagattccgaacgtctctgaggaggtgctcaaggacctcgacgagcgcggcatcatccgcatcggcgcggacgtgcgcgacggcgacatcctcgtgggcaaggtcaccccgaagggcgagaccgagctgaccccggaggagcgcctgctgcgcgccatcttcggcgagaaggcccgcgaggtgcgcgacacctccctgaaggtgccgcacggtgagaccggcaaggtcatcgcggtgcgccgcttctcccgcgaggacgacgacgatttgagcccgggcgtcaacgagatgatccgcgtttacgtcgcgcagaagcgcaagatccaggacggcgacaagatggccggccgccacggcaacaagggtgttgtgggcaagattctcccgcaggaggacatgccgttcatggcggacggcaccccggtggacatcattctgaacacccacggtgtgccgcgccgtatgaacatcggccaggtcctcgaggtgcacctgggctggctggccaaggctggctggaccgtgaacccggacgacccgaagaacgccaagctgctcgagaccctgccggagcacctctacgacgtgccggctgactcgctgacggccaccccggtgttcgacggcgcgaccaacgacgagatcgcgggccttttggctaacaccaagccgaaccgcgacggcgaagtgatggtggacgagaacggcaagacgatgctgttcgacggccgctccggcgagccgtacaagtacccgatctcggtcggttacatgtacatgctgaagctgcaccacctggtggacgagaagatccacgcccgctccactggcccgtactccatgattacgcagcagccgctgggcggtaaggcccagttcggcggccagcgtttcggcgagatggaggtgtgggcaatgcaggcgtacggcgccgcctacaccctgcaggagctgctcaccattaagtcggacgacgtggtcggccgcgtgaaggtgtacgaggccattgtgaagggcgacaacatcccggatccgggcatcccggagtcgttcaaggtgttgctcaaggagctgcagtcgctgtgcctgaacgtggaggtgctctccaccgacggcacgccgatggagctcgacggcgacgatgacgagttcgaccaggccggttcctcgctgggcattaacctgtcccgcgacgagggcgcggctgcggatacggcatag

SEQ ID NO: 2 - DNA, 20 bp, synthetic construct
  source 1..20: mol_type = other DNA
cgwatgaacatyggbcaggt

SEQ ID NO: 3 - DNA, 20 bp, synthetic construct
  source 1..20: mol_type = other DNA
tccatytcrccraarcgctg

SEQ ID NO: 4 - DNA, 343015 bp, Corynebacterium cassirii
  source 1..343015: mol_type = genomic DNA
tgatagcggcggggaaacgcccggacccattccgaacccggaagctaagcccgcccgcgccgatggtactgcacccgggagggtgtgggagagtaggttaccgccgacccaacaacaacaaaacaacaacaaaatacacacaaagcacccgatccaccggccacaaccggtagatcgggtgctttattatgcccgcacacaagcagcgtcacgccagcggcgcacaccggtaacgccaccaccggcaccaccggtaccgacagtgccacgctgaccccaaaccccacaccacacaagagtggggcggatacccgaaggcggataaacaaccgcggacgtacgcgtacgtcatcgcatatccgctatctatcatccgccccgatacaggccgcaacgctgacacacccggccaccccgggcgctgctgtagcccccaacaacaaacagccacgaaccgagcagcaaagccccagctcgcaaacaccccgaaaccccggggagctacacaccccgcacaccaacagcggataactcccaaggccccggactacgaccagcacaaacaagaagccacccccgagatacccgctatcagcaagagaagcggcgggcgacggcacccaggcgcccgccttgaacagcaggcgcccggcgccagtggcttttgaggcgtgggcgatgcgcccgcaacggcggttcatataatggtgggaacgcaaacgaaagggcatcaatgtcggaaaaggacaaccgtccgcagcacaacaaccgtggcaaccgtggcggcaacagccatggccgccgcggcggcagtggccagcagggcaatccgggccgcggccgcaggccggatcgcgatgggcgagacgagcgcagcggacgcgacaggcgagacgacgaccgggtgcgtcatgaccgctcaaacccgcgccgtcaggggtaccgcgaagaccgcatggctctccgattgtccgagccggatttgcccgacgagattgatgtgactgtgctcgacccgtccgtgctccaggatctgcgggttctgtcgaaggacaatgcggaccgcgtcgcaaagcacatgattatggcctctgatctgcttgaagacgatccgcaactggcacttagacacgcccgcgctgcgaagaaccgcgcagggcgcgtcggcgtcgtgagagagacgaatggcgtcgtcgcgtaccacgctggcgaatggaaggaagcgctgtctgagctgcgcgctgcccgccgcatgagtggcggcccgggattgcttgcagtcatggccgacgctgagcgtggcctgggcaggcctgagaaagcgctagagctcggccgcactcccgaagcggaacagctggacgaagagggcaggattgagctcgcaatcgtgctcgccggcgctcgtcacgatcttgggcaacacgagtccgcgctcgcaactctcgagcgcctgaatccgtcgttggaatctgagggctacagccagggtcggttgtcttacgcatacgctgacgcgcttttgtcgcttggccgccgcgacgaagcgaagacgtggttcgagcacgccgccaagttggatgaggatggcctgacggacgctgaagaacgtatcgacgagctggattaggggtttacaaaacgttgacgctcatcagtaaccacgacgcactcctgctcgatcttgatggcaccgtctgggaaggcggcgaagccattccccacgctgtcgaggccattaacggtgctgcggtaccggcgctctacatcaccaacaacgcctcgcgaggcgcggatgaagtcgcccgcatgctgagggggatcggcttagacgcttcggaagcagatgtggtcacttccgcccaggctgcacttgagctcgctggcgatcacctcgcgcccggcgacgcggtcctcgtgctgggtgcgccgtcgttccgcgaccttgtggcgcgagcgggctaccgcgtcgtagacaacgctgatgagcagccaaaggtcgtgttgcacggacacaaccccgaaaccggatggcgtgagctgtccgaagctgcgctggcgatccagcgcggcgcgacctacttggcgtcgaatctcgacaccacgctgccgatgcagcgcggcttgatggtgggaaacggatctatggttgcagctgtcacctccgctaccggagtgactccgcaagccgctggtaaacccgagcccgcgatgttcctgcagggcgcgtcccagatcaattcctcgcggccactcgcagtcggggaccggttagataccgacatcgccggtgccgtcgctgcgggcattcctgtcctgcacgtgtcgaccggtgtgtcgggaccgctagcgttaatcgaagcaccgaaggaacagcggcccacctatgtggctgaggatttccgcgccctccaagctgatcccgggactctgaagcccggtagccagggtggtttcggcgcccgcgtcgacggcgacgacattgtgctgagccacggtcgcgatggcgctaccagcatggaggcgctgcgtacggtgcttgaagtcgcttggatgatggatacgccgcccaacctcgtgcgtccaaactccgaggccgccgaggccgcgacgtcgacgtggtggtgatcggcgatgacagaaccgcacatccttacggcggagcaattgcgcgagcagtttgcggagctgatggctgaacccgccgatgacctcgcaaatgaggcagcgcgtctctcgaaagcacacctgctgcttcacgacgcgctgcagaacggatagcccgcgatggcaccaggaagacgccgcctcgacgcggaacttgtgcgcaggaagatcgcgcggtcccgggagcaggcgcaatcgtggatcaaggacggattggtagaagtgggtggctttgtcgccactaaaccggccaccgttgtggaaccggacgtctcgatcaaggtcaacgccaacgcggacgatgaatgggcatctcgcggagcgcataaactcctcggcgcgctcgaggtgttcgaagccgccggtttgcgtgtcgacgaccgcaaagcccttgatgcgggggcgtctacaggcggattcaccgacgtgctgctgaagcgcggggcgagcgaagtcgtggctgtggacgtcggctacgggcagttgatctggcgcctccagaacgatgaacgcgtccgtgttcttgaccgcaccaacatccgccatctcacaccggacatgatgggcggtgccgccgacgtcatggttggggatctctccttcatctcgctaaagcttgtgctcccggccattgcggagtgcatggctgacggagcggacttactgccgatggtcaagccgcagttcgaggtgggcaaggatcgcctcgggcacggcggcgttgtgcgttccgctgaacagcgtgcggaggtgaccgccgatgtggcaggcttcgcgcagacgttggggctgagcctgaaaggcgtcaccgcctcaccccttcccggcccgagcggcaacgtagaatacttcctgtggctggtcaaagacggtggaaccgccgccatcgaccaggattcgatcgccgcgatggtgggcgaggcagtgcaggaaggaccgcagaattgatggacgcgacgcaaacccgcgaagtcctgttggtgccgcatttttaccggccggacaacatctcctcggccgcgcacgccgctcggttgctcagtgacgcaggcatccgcgtgcgcctactcgatcaatcgggtgacagcgccgagcacccggcgctgcaagatccggtcttaagcacccttgagcgcgttacgccggggccggcagctgcgaaggggtgcgagcttgttctggtgatgggcggcgacgggacgtttttgcgagccgccggcgtggcccgtgagcaggacgtgccggtgctcggcatcaacctggggcatgtggggttcctcgcggagggcgaggtggacagccttgagtcggtgatcgatacagtggtgaacaagacgtacaccgtggaagaccggatgacgattgacgtgcaggtgcgcgacgccgacggcacggaaatcgggcgcgggtgggcgctgaacgagtgcagtgtggagaacatagaccgcactcaggtgctcgacgcgattttggaggtagatttccgcccggtgtcgtccttcgggtgcgacggggtgctagtttccacgccgaccgggtcgactgcctacgcgttttccgccggcggcccggtgatgtggccggccttggacgcgatcctggtcgtgccgaacaacgcgcacgcgctgttcaccaagccgatggtggtatcgccgcgctcgacagtcgctgtggagaatgaagcgacgtcgagcgccgctgtggcggtgatggacggtttccgcaaaatcgagatgccgcccggcgcccgcctcgaggtcatccgcggttcgcggcctgtcaaatgggtccgtttggaccgcaaaccgtttacggaccggttggtccggaagttccaacttcctgttgccggctggcgaggacccaggtacacgtagtgctcgcagaaatttcaatccgcaacttgggtgtcatcccggcggcgtcggctgagctggcgcccgggttgacggtgctgaccggcgaaacaggcgccggtaagacgatggtggttactgggctgcggctgctcaccggcggacgcgccgatgcgtcgcgcgttcgcagcggcgctgacgaagccgtcgtggaagggtcattttccaccgagggcctgcacacgacccagtcgcaacgtgtggcggacgtggccgaggccgcgggtgccgcaacagacgagaacggcgagtacgtggtcacgcggtcggtaaaggcctcggggcgctcgaaagctcacttgggcggccgcactgtgccggctgccacgcttgcagagctcaccgagccgcttttgactattcacggccagaacgatcagcttcgtctcatgtcgccggaccagcagttggccgcgctcgaccgattcgatccggcgatcgcgccggcgctgaaggagtaccgcgaggcgtacaccgagtggcgcaaagccgcgcgcgagctcaaggagcgcaccgagcgcaagctcgagctcgcccaggaggtcgaccgcctccggttcgcgctggaggagatcgacgcggtcgcgccccaggagggggaggacaccgagctggtcgcggcgattaaccggctgcaggatgtagacgcgttgcgggaggccgcggccgaggccctcgccgcgatcgacggtcctgaggcggccggcggcgcggccgccggcgacgagctggcggcaacggcgctcatcggccaggcggcgagcgcgctgcagcagtcgagcgacaccagcttgcaggagctgggttcacgcttgggtgaggtgagcagcgtgcttggcgacgtagcggttgaactcggaacctacctcgccgatttaccggcagaccccgacgaactggatgcgctgctgacgcgccagcaggagttgaaatcgctgacgagaaagtacgcgcccgacgcctccggggtgctcgcgtggcgtgagaaggcggcgaagcggctgggcaagattgatgtgagtgagggggccgtcgataagctgaaaaagcaagtcgcccagctcgagaaactcttgcggcaacgcgctgagacgctcagcgccgcacgcgagaacgcggcggcggcgctcggcaacgccgtgaccgaggagctgcacgggctggcgatgccgaaggccaagctcgccgtgcacgtggagcgcgcagactttagcaaagacggcgtggacgcggtggagattcgtctcgcgccgaacgcggcgctcgagccgaagcccttggccacaagcgcgtcgggcggcgagctgtcgcgcgtgatgctcgcgctcgaggtaatcctggccggatccagcggcggagcgacactggtgttcgacgaggtcgacgccggtgtcggggggcgcgccgcagtcgagatcggcaggcgcctttccaggttggcggcgaacaaccaggtcattgtggtcactcacctgccgcaggtcgccgcctacgccgacacgcaccttcacgtgtcgaagcacgttggcgatgaggcggtgacctccggtgtcggtgcgctaagcggggacgagcgcgtggaagagctcgcccgcatgatggcgggcttggacgattccgatacggggcgcgctcacgccgcggagttgctcacccgcgcacaggaggaacgcgcgcggctgcgtagctagctgcccacccctcccgcgcgccttcctaagttcaggcaggtcacggtgcacaatggccggtatgactgtctcgaccaccttcgaaggcacgctgcgcgactgcacgccgcagggcaagggcatgagccgaatgcgcgaaggcgacatcgcgttcgtggacgcgccggatatgacccgccgcctggcggagcagctcgcggccgccagacccgcggccgttgtcaacctcgcgcgcttctcatcgggtgcggtgccgaactacggcccgcacttgctgctggacgccggcatcgccctgctcgaaggcgcaggcacggaacttcgcgggttgatccgcgacggcaagaaggtcgcggtggacgctgacgggcagatcaccgtgggcaagaaactcattggccaggccgcaccggttgaccgcgcggagctcgacgccaccttcgcggacgcgcagcgctccctggtggacacgatggaagcctacttcggcaacgcaacccagttcattcagtccgaggcgccgctgcttaccgacgccatcggcgcccccgacttaggcgacgtcatggccgatcgcaaagtggtggttgtctccccgggcgcggacacccgcgagcgcctgaacgggttgaagaacttcatcagggagttcaccccggtcatcatcggcgtgggcagcgccgccgacgaggtggtgaaggcgggatacgagctcgactttattgtggctaacccgactgaggtgtcgtcagaaagcctgcgcggcgacgcgaaagttatcctgcccgcggaaacggacggctacgccccgggcctggagcggattcaggatctcggtgtgggcgcgatgacgttcccggccgccggcgagtctgccaccgacttggctatcctgctcgccgcgttccacgaggcggaaaccatcatcacggtcggcgagccggtggaactcgacacgatcttcgccgacccggcggcggccgagccggcggctctaatcacccggcttaaggccggccggaagatggtggactcgacggttatcgaaaacctctacgccgtcaacaccggaggcggcggtgtggcgtgggcctgggcaatcctgggcctgctggtcgccgcagcaacggtcgtggtcattgtgggcctcggcggcagcgacacgttcaccgacaacctggtgaacacgtgggacgccgtcgtggcgcgggtccagagctggttcaagtaggcaagtagggagggcgagagacgcatgggtcaaggagcacgcagttcgggacttgtcgccgccggtttgggttggggcgttgccgcgggcgtcgcgctgggcgcactgctagtcgcgcctgcgatggacgacgtgtccggcggccgtcccgcaaccactccggcgcagtcgagcaaggcggacgccgccgagagcaacgcgtttgcggacgaccaggtcgccgacgcgaacgatctgctcgccagcgagggcgacgccatggtggacggggtgcttgacggcgtcgcggtcacgattatccgcaccgccagcgccaccgacgaggacgccgcggctgtgcggtggaaggcgaacgcagctggggcgtcgaactcaggcggcgttcggttaacggagaagttcacggacatgtcggccgtagacgagctggcgaccatcatcacgtccaccctgcccgcgggtacgcagctgtcggaggacaaccgcgctcccggcacccacgcgggcgagtcgctcgccgcggcgctgacgacagcttccgccgacgaccgcgcgctggttttggaagctctggagcaggcgggttttgtggaactgcgcggccaaatcgtgccggcggacgtgattgtgctggtcgcggccgacgagctcgacctcagcgcggaacccaccggtgacggcgaggcgttcaccgccaaggtgctcagcgattttaccgcagcgctcggcagcggcgcgccgaccgtcgcgacgggccaggggtcgctgccgcagcttggcgaagcccgcaccgtcagcttcgccgacacggaagctggccggatccgcacagtgttgcaggcaggcgagctggccgacgtaccatcggagcatgacgcataacttcgaggtcacccaaagcacactgcttgtcgacgcacccattatcgccctgcgccgcgacaccctgaccatgccgggcggcaaggaagccgaccgggagatcgtggagcacttcggcgccgtggcggttgtcgcgatcgatagcagcggccgcgtcgccatggtggagcagtaccgccactcggtcggccgccgcttgtgggagttgcccgccggcattttggacatcgccggcgaggaggagctcgccaccgctcagcgggaactggaagaggaagccggccttgccgccggcgactgggcggtgctggtggacctggtcacgtcgccggggttcgccgaggaggcggtccgcgttttcatcgcccgcgatctgcgcgacatcgagcgcccagatgcggaggacgaggaggccgacatgggttttcagtggatcgccctcgacgaggcgcgcgcgaaagtgatgcgcggcgagatcgtgaactccatcgccgtcgccggcatcctggctgccgccgaggtcgaggcgggccgcgcgcagccgcgcgatgtgcgcgaaccgtttgcgttgcggccggagtcgctcgcgcggcgcaggcaagcagctggtgttgcgccggacatgaagaagatccagcgctaaggccggggtttttcagatgcgcccagcagatcttgcgcaccggtggcacgtccacctcgtggtggagcgggggctttcggacaacacggtgagcaactacgaccgcgacttaaagcgctacgttaattggctcgcgggcgccggaatcgaccgcatcgaggacgtcaccccgcagcacctcgaagcgtacgtcgccgacctgcgccgcggcagcgacaccgcccgcccgctcgccgcgtcctcagccgcgcgcgcgttggtagtggcgcgagggctgcacaagttcggcgtcgcagagggcgtgctgcctgccgacgccgccgctgaggtttccccgccggccgcgggggagaagctcccggataccctcaccgtcgacgaggtcgcccgactcatcgaatcgtgctcgactgaaacgccgctgggcctgcgcgatcgcgcgcttttggaaacgctctacgccaccggcgcgcgcgtctccgaggtgctcgcgctcgtggtcgacgatgcggtcgacaccgggggcgtgatcgcggtgagggggaagggcaacaaacagcgtttggtgccactcgggtcgcacgcccgcgatgcgatcggcgcttacctggtgcggtcgcgccccgtgctggcgacgggcaagtcccacgcgctgttcctcaacgcccgcggaggtgccctttcccgccagagcgcgtggaccgcgttgaagcaagccgccgaccgcgcaggaattgctaaagacatctcgccgcacacgctgcgccactcgtttgccacccacctgctcgaaggcggcgcagacgtccgcacggtccaggagctcctcggccacgcctcagtgaccacgacacagatctacactcacatcaccgccgacaacttgcgcgaagtctgggcggaggcgcacccccgggcgtaggtggggcaacgctgtacagttggcgcggtgttgatcttgcgaaaaactgccctcggtatcaccgcagcgggcgcggccgccgttatgctcactgcacccattggcccggcgcatgcgcagctgccaggtgggctcgatccgcagaccgtccgcgacatgatcccgtctccagtcagcgtgcgcgcaggggagacgaccaccgtcgatgtcggcgtcccggtcaacgtcagctacaactcgggtggttgggaggtcaacgcgaacggcacttccgtgaccgtcacagcgccggatacccctggtgcgaccgcccaggtcccggcgagcgctttcggcttcgacgcgacgatcaacttgatcgctgttggattctcggagtcgaccaccctggacgagattgaggatgcggggtctgctgcgccggttgcgccagctgcgcctgcgccgtcggaggcaccgcagcagcgggaggcagccgacgacgaagcgcctgcggcgccgcacccgccgcggtcgaaggccgagcccgccgacaccgcggcagcgaagaagttctacttcgacggggtgatagaaggcaaccgccttgtggtcactgtgccgctgtcgcgcgccgcgggtctggcgaagtacgccagcaccgaccgcgagggcgcgaagctgcgctacctcgacgtcgacggccagattatcgaaggagtcacccgggacgtggaggtcgcggcccgcaggctcaccctgatctacccggaaggcgaaacgcccgacagcccgttcatcatggaggttaaccgaaacggcaaggcggagttcatcgctgtcatcaccgccaccaacgccgagacagctgcgccggcagcaccggagaacaacccgtacgcggacgcagctgccgaaggtcaagcgcagaatagtcaaggccatgaacatgactcggggcggtctgttgtgccgctcgcgatcggcggcgtcgcgctgttgacgttgattgcgctggtgatcgcctggttgcggcgccggggcagcgcgcgggcgtagcagaggctacgcgcgaaatgccaccgttgtaagatgggggcgtcaagtgttcaggcgggatgaagtgtaaggatcggcgatggcggagacacctgcggacggcgcgttgtttaacgcccaagagaacaagacgtttttgactgggcgcccgtaccgcgaattcgccgcaccgaaggaacttgaccggcacggacccgccaaagttatttcgatggtcaaccaaaaaggtggggtgggcaaaaccacctccactattaacttgggcgcggcgctcgtggagcagaggcgcaaggtgctgctggtcgaccttgacccccaaggcgcactcagcgcgggcctcggcatcacccaagacgaagagcacgtcacggtctacgatctgctcttcgacaccaccgcgtcgatccacgcggcgatccagcactcgaaggtttccgggctggatcttgtgcccgccaacatcgatctctccgccgcggagatccagctggtcaacgaggtgggccgcgagcacacgctcgcccgtgcgctgcgcccggtgcgagacgactacgactacatcttcatcgactgcggcccgtcgctcggcttgctcacggtgaacgcgctggcggcgtcgcagggcgtgatcatcccgatggagggcgagtactactcccttcgcggcctcgcgctgctcacggacacggtggaaaaggtgcgcgaccgcatcaatttcgacctcgacatcgtcggcattttggtcaccatgttcgaccgccgcaccacccacgcgcgcgaggtgatcgagcgggtggtcgaggtgttcggcgaccgggtcttcgacaccgtcatcacccgcaccgtgcgtttcccggagacgtcggtggcgggcgagccgatcaccacgtgggcgccgagctctcagggtgcggagcagtaccgcaacctggccctcgaggtcatggaacgcatcgagcggtgatcggggagcagccggagatcaccggcttccgcctcgcgctggcgaacttcgagggcccgttcgacctgctgctgtccctgatcaacgccaagaagctggacgtgacggaagttgcgctggcagaagtcaccgacgagttcatcgcctacaccaaggcgctcggcgagacagcccagctcgacgaggtcacggagttcctcctcgttgccgccacgctgatcgacttgaaagccgcccgccttttgccgcgcggcgacgaggacgagattgaggatctcgagctgcttcagtcccgcgatctgctgttcgcccggctgctgcagtaccgcgcttaccagcaggtggcagaccagttctctcagtggcaaacgcttgctcagcgccgttacccgcgggctgtgtcgatggagccccagttcgcccaggccctgccgccggtgcgcctcgggcacacgcccgcgacattcgcgcagctcgcggcgggcgtgttccggccccgtccgccagatgaagtgcgcaccgaccacctgcacgaggttgcggtgtcggtgccggcgcaggctgggcggatgctcgacgtgctgcgcggcgccggcgcgaacgagtggctttcgtttgcgacactgacgcgcgaatgcaagcgctcgatggaggttgtcggctcttttctagcgctgctcgagctgtacaaggcccgggctgtggagacgcagcaggacgagccgctgggtccgctagatgtagcgtggacgggcgttgaggtggacccggcggttgtagccgcgggcaactgggagtaagggaggcgcatttcaatcgtggagatggtgtcgcagctgcgcagccagatcgagtcgatcatgctggtcgtggatacccccgtgcacgcagaggacatcgcgggggcgcttggggtggagcggggggacgtcgataagcaactgctttcttgggctgccgagctggaccagcggggcagcggcatcgacctgcgcgagaccgcagaagggtggcggctgtacacgcggccggagaacgccgcggcggtggaggcgtttgtgctggacggcacgcagaccaagctgagccgcgccgcgatggagacccttgctgtggtggcgtaccggcagccggtcacccgcgctcaggtcgctggagtgcgcggtgtcaacgtcgacggcgtgatgcgcacgctggcgctccgcggtctgatcgccgaggtcgagccagacgaagcaaccggtgctcaccggtacgtgacaaccgagctgtttctggaactgctcggtatcgactcgctggagcgcctgccggatctggcgccgctgctgcctgaggtcgacgcaatcgaggatgcctggtaagcgcgagaacgctggtaggctcgtgccgcaacaattgaaaggatgatttttcgatgactccacccgctcgccgcgacggcacaccggaaagggataaggacgaaacgttctacatctcctacgcgaagccggcgcgcaaacagcacgtagacgtggaaaagcgccgcgccgcaagtgccgcaaacgaagacgaccacccgttggccgacaactggtgggacgacgaagacacgaaggcccgcaagaaaaacaccgacggcgtacgcctgcagaaggtgctcgcccaggcgggcgtggcatcccgccgacacgcggaggcgatgattgaccagggccgcgttacggtcaacggcgaaaccgtcaccgtccagggcacgcgcgtcgacccgaacgtcgacgtgatccgcgtcgacggctcgcgcatcaacgtcaacgaggaactggaatacttcgcgttcaacaaaccgcgcggtgtccacaccacgatgaaggacgagatggaccgcacgtccgtcggctcctacctggcggaacgcacggcatccggccagcggctctaccacgtgggccgcctcgacgcggacaccgaggggctgctcctgctcaccaacgacggcgagctggccaaccggctgacgcacccgaaatacgagattgcgaagacctacctggccacggtgctcggtgaggcgaagcaggacctgatcaaaaagctcagggagggcattgagcttgacgacggtatcgcgaaagccgactacgcccagatcgtggacgtgcacaacggccagtctctggtccgcgtcgaactgcacgagggccgcaagcacatcgtgcgccgcatgctgaaggaagccggcttcccggtgcagcgcctcgtgcgcaccaaggtccacacagtgcagctgggcgacatgaagccgggctccatgcgcgcgctgaactccagcgagctcgcctcgctgtacaaggcggtggagatgtaaatggctgacctcaacgtgagcaacatgccagaaggcgggctgattctcgcggtcgacgggccttccgggaccggcaagtccaccacgtgccgcgccttggccaagcggctggacgcgaagtacatcgacaccggcgccatgtaccgcgtggctacgctggcggtgctgcgcgccggcgtggacccgcaatcgaccgacgaggtgattgccgtgacccgcgagctgcccctgactgtgtcggacgacccggattccaccgaggtgctgctcggcggcgaggatgtctccggtgagatccgcggcccggaagtcacacgcaacgtctcggcggtctccgccatcccgcaggtccgcgagaacttggtggcgcttcagcgcaacctcgcgcgcgatgcccaccgggcgatcgtggagggaagggacatcgggaccgtcgtgcttgtcgacgcccccgcgaaagccttcatgaccgcctccgccgaagtgcgcgcgaagaggcgctacgaccaggacatcgccgccggccgcgaggcggattttgacaccgtgctggccgacgtacaacgccgcgatgagctcgactcctcgcgcgccgcaagcccgctgaagccggccgacgacgccgtgatcatcgacacctccgacatgtcccgcgaggacgtgctggaggcactgatcgagctgattgaaaggagcgccaagtgagcgactcacgcgacaacgagcgcgtcaacgacactgacgagcaggagacccagttctttcagccgggtattgacgcctccgggtacgacgatgttgaggagcagtacctcggcgtcggcgacgcggagttctacgaccccgatttcgaccccaaagatttcgacgatgccgactttggtgaccccgacttcggcgaggatgccggcgacgacgacgcggagtacaccgacgaggagtgggccgagatcgagcgcgcgtacggcgtgtctcgcccggatgtggtcgaggaggcgctgccgaccgtcgccatcgtgggacggccgaacgtgggtaagtcgacactggtcaatcgcttcatcggccgccgcgaggccgtggtggaggaccaccccggtgtgacccgcgaccgcgtcagctacctcaccgactggggcgggcgccgcttctgggtgcaggacaccggcggctgggacccggatgccaagggcattcacgcggcgatcgcgcaccagtccgaggccgcgatggaaaccgccgacgtcatcgtcatggtggtcgactcccacaccggcatcactgaaactgactccgtgatggcgcgcaacctccagcgctccgaggtgccggtgatcctggtggcgaacaagttcgagtccgagtcgcagtggggcgacgtggccgagttctactcgctgggcctcggcgacccgtggcccgtcagcgcactgcacggccgcggcggtgcggacgtgctcgatgaggtgctcaggctgttccccgacgtcccgcgcgccgcgaactcgatcaccgacggcccgcgccgcgtggctattgtcggccgaccgaacgtgggcaaatccagccttctgaacaagctgtcgaagaagaaccgctcggtggtggacaacgctgccggcaccacggtcgacccagtcgacgagctgatccagctcgatgagaacctctggaacttcatcgacacagcgggtcttcgcaagaaggtgaagaacgcccagggccacgagtactacgcctccctccgcactcgcggcacgatcgaagctgccgaggtgtgcgtggtggtcatcgacgcctcgcaggagatctcggagcaggaccagcgcgtgatctccatggtgctcgaggccggcaaggccatggtgatctgcttcaacaagtgggacctgatggacgaggaccgccggtactacttcgaccgcgagtttgaagagatgatcggccacttgagctgggtgaccaagatcaacatctcggcggagtcgggccgcggcctgcaccgccttgagccggcgatggcggaggcgctggagaactgggacaagcgcatctccaccggccagctgaacaactggctgcgcgaggcgattgccgccaacccgccgccgatgaagaacaaccgcctgccgaagctgctgttcgccacgatggcgacgacacgcccgccgaccatcatcctgttcaccaccgggttcttggacgccggctaccgccgctacctggagcgtaagttccgcgagcagttcggctaccacggcaccccgatccggatcgcggtgcgggtgcgtgagcgaaacccgaggcggcgcggctagtgcgccccgccatcatcgcgctgcacggcaagggcgacaacgggcccgactttgctgaggcgaccggtctcaccagggccgacgcggtgatctccgcgccgacggggaaggggctagcgtggtcgccggccccgtacgccgcgaccacgctcgagcaggatgcggctcgcatcggcgagattgtggacggtttggtggccaaccacgaagccgacccggcgcgcatctacctggtgggcttctcaaatggcggcgggcttgcggtgtcgctgagcacgatgagcacactgggcgagcgtttcgccggcgtcgcatctgtatcggcggcggtgcgcaccacgccggatgagatcgccgccacgcccaacgccgtagattacttgaacatccacggcacgtgggacgatgtcgtgccctacgccggcgagacccgctcgccgtacagcggtgagcaggacgacaccacctacggcgcggtggctgtcacggaagccttcacccgccgaaacgcgggccgcgcccgggcagagcacatccccgtcgagcgcatgggccatgagtggcggccggagaccaccgccaccatcctcaagttcttcggcattcaggcgagcttgtagacaaacgcgtcggtgcggtagggcagcggcagaagctggcccggcgcgaacccgagccggtcgtacagataccagcgcaagttgtcggccactttcgcgcgcgtcgcgccggaagcccccagccagtacgagcgcgtccgcgcgagcgcctccagcgcctcaggcgtgacaggctggatccacttcgtccgcaactcgcgctggaggagccattgcttgccgacgtccgcgtaaaacccctccctgtgcacatcacctgagtggctaatgcgggagtaccgcagcacccacgggtgcgtgacgtcgagcgtgttccagcacagtacaagcgaggcgccaggtgcggcgactcgcgcggcttctccacttgcggcgccgacatcgagccagtgccatgtttgggcgcaggtgatggcgttgaaggtggcgtcggcaagcggcagtgcctctgcttttgcctcaaccaccgcaacctccggcaaccgggccgcgagcacctgggacatgttgtgcgagggctcgacggccaccacccggcggccgggtgccaccagtgcctccgtgagtttgcctgtgcccgcgccgatgtcgaggacgtgcgagcgcccggcgatcagctcggcgacttcgggcggataggaagggcgaacctcgtcgtacgtgtcggcgccgcgggtaaacgccccggcagtgaactgcctcgcggcagcgtcgcggaaagccggcgcgtccttcgcgctcggcttgaagttgcgcggggtagcttggcgagggtccgtggtcacagcatgcaaatctagccgtgtagcctgacacctatgcaaagggcggtgtcactgattgttgcctcggcgctcgccgcggcgagcctgaccgcgtgcgacatgccgtggtcctcctcgcgcctggacgatgtgcagcaggcggaggaagtgcaacccctgccggcgcagacttcggccgcgttcacgaccgcgcccgcgacagcggagcccttgaaggagagggactaccgccacaccgtcaaggtggacaagcgcgaccgcgagtacctcctgttcgcgcccgaggacgccgccggaaaagatctgccgctgatcatcgcgttccacggccataccagctctgcgaagaacttccacaaatccagccatttcgaacgcgcgcaggcagtggtcgtgtacccggacggcgtggcgaagaagacatctttgcacgcggagccgaagcaagcgtgggcgccggcttggtacgccgacacctcacccgaggaggacgccaagttcgtcgacgcgatcatcgcgcaggcggtgaaggaatatggcatcgacccgaagcgggtctacatcaccgggttctccaacggcggcgggttcgccgcctacctggccgcgacctaccccgagaagttcgctgccgcagcgatcgtgggcgccgcggtgcgcacgccggaagaggatctgcgcacgggcctgcccatcccgctgctcatgatgcacggcgccgacgacaagaaggtccccaccacgggctacacctcgcccgtcccggagccgccgggcggcaccgacgaggtgctgccggtggagaaggtgctcgaggcgttccggatccgcaacggcaacgacggcgtcgagtacgtcaagatcactgagtgggggcacgcgtgggcgacgcctagttcgcggatgccgttcgacaccaccggcagagtgattaagttcttcggcatcgaggacacctacgcccagctgcccgacttcgaataatctccactattctatccgggtgcaattacggggtcttttgagtgccgcggccggcttggtgctggtcgcgggcgccgttgccgcgtgcgcgaattccgccgatcagccggactcgctggagcggttgactgacgcggctgtttccccggcgccgcccgccgccgacaccgccgcgtggagtccgcaggcgacacagcaccgcgtggtcgacgccggtgggcacaggcgcgagttcatcctccacgttcccgcgggtgccgagcagcgctcgaagctgccggtcatttttgtcttccacggctatctggaggaggcagcaaccatccgcgagtactccggcctcgacgccgctgacgcgctggttgcctacatgcagggggtggacaacgcgtgggcgccggctccctacgctgcgacgtccggcgagcaggacttggcgtttgtcgacgccgccttcaaccagctcacccacgacttttcagtcgaccgcgcacgggtgttcgccgcggggttgtccaacggcggcggcttcgcggcgtacctcggctgccagcgtccacaagagttcaccgccgtcgcaacggttgcgggcgccttttacgaaaaggtctcagaggggtgctcgatgatcccgatgaagcacatcgacttccacggcaccgccgacccggtcatcgcgtacgccggtggtagccgccacaaccacgtgtacgactcgacggcagagctcatgagcgacgccgcggagcgcaaccggtgcgatccccagccggttgagaggattgtctcgaacgacatggtggagcagcgttgggttggctgcgacgcggggttggtgcactaccgcatcgtcggcggcgcccacgtgtggcccggcggcggcaaggatccctccacaacggtgccctccggatttgccacccgcacgatgctcgagttttttggcgtcccgtccaccagtgccgcaaccagcgggttttagtcaagtgctcacagtggtgtaatctggcggagctgcgaaagcagcgatcgggctgtggcgcagtttggtagcgcaccacactgggggtgtgggggtcgcaggttcaaatcctgtcagtccgacatttttcttttccgggggctttagtcgatgggtgcgacgcgaaccgggtttccgtcggggtcagcaacgacgaaggtcgtgccgaacacttcctcgtacggctcgcgcagcacggtcacgccttgctccttccagcggtcaaacatggcggcgacctctccggcggggacgttcaagcacacctctgcagtccgagcggtggcttcgttcagcgaatcggcgcttcccgtccacagggcgagggacacgccttcagcgagcgcgaacgtgacgtagcggggggaaacgaagtcggtgtcgaggcctagaaggtcgcggtagaaggcaaccgaagcgtcgatatcggaagcgtagacgatgaagacgagttcgcggttcacagttacgcaacgtacacccacgcgcccgcgcggcgctcaaaacgggatcgctcccgctgcacgccgccggggtagtaggcggcgaactcgacatacccttcggagtcgaacaacccgcccccggttttgcccagaatcaccaagcgggtgaacggctcgccaccgcgactgatctcaagtgcggcgggccgcgtctcgggcgcccaggtgcgcagcaggtaatctgcgtcgcccaccacgaaagcggtgtagcgagagcgcatcagcgcctcggctgtgggcgcggcggcgcccgcgtggtattttccgcagcactgcttgtacgcaaagccgctcccgcacgggcaggacacgttttcgcccgccacttagcgcttcgaaatgtgggccttgccggcggcgcggttactcgcgcggcgctcggcaatggtcgctgtggacaccgtggtctccacagcgtttttctccacgtagccgtcgaccgtggacgcggcgccggcggcgcgaagtgtctcagcctgggcaggggtcacgtcgccgtagagcgtgatctcgcgcgtgaaggtgccgtcgccgttgtgggagacttcaacgcggacgtcgtcaagcggcatgcccttggcagcttccctgacagcttgggagcacgacgttgcgagcgcggacatgaacaggccggtggtggtcaccccctggcccttgccgccgctgttcttcggccggtcggtggtgatggcgcggcccgaggttcgcacgacgtcgccgtacttcgtgccgcgcgcggtgtaagagattgcgttggtgtcgccggtctcttccgcgatgaattccggcacgatgtactgcttcgcccagctgccgatgatgtccgcggcgcgctgcgcagtgccttcacgggtcagcaggtggtcggccttgtccagcgccatcagcgacttggggtagcgggtgagctggaaaatggtctgtgcgttgtcgatgccgacggtgacgtcggtcggggagtgcactagcaacagcggcttgcggagcttcggcaggtacgtctcagggttggttacggcgaggtcctccaagaactcgcgcgaaatgatcagttcacgccctcccagcacaacgggcaccgagccgttggtatctgcttcgccgatcttgtcggcgtagtgcagcaccgagtgcgccgggtcgaacggggcaccgatcgtggccacgcacttgatcatcttcttcagctccgggcgggtggctgcctgcagcgtcgccgcaccgccgagggagtggcccatgatgagctgcggggctgtgaagtgctcgtccatccactgcgcaaccgcgacaatgtcgtcgacgttctgggtaaacgaggtgtctttgaactcgccttcggactggcccaggccggggaagtcgaagcgcagcgtggcgatgccgtgctccgtgagccgttttgcaatgcgcgacgctgccggggtgtgacgcgacccggcgaaacagtgggcgaaaatggcgtaggcctgcgctggagcgtcgggtcggtcgatcgtggctgccaacatcgtgccgttggacgacggcactttcacgttcagtgactgcatacggctaagaataaagcacgttgcgagatgcgttgcgcctcgacttaccatggtgggaatgacgcgcacgcaccccgcgcggcacgcacgacgaaaggacggcacgcacgatgggcgcattcgactggttctggaaggccatgggctcgtcctccgagcgcaacaacaagaaatcgaagggggttgtcgcggcggcgcacgggttgatcccggagctagagcagcttgacgacgcagcgttggccgccaccgtgcgcgaaaccgtggccggaggcgagatctcggataagccccggttcttggcgggcctgtcggtggcctcctcgcgcacaatcgggttggtgcccttcgaggtgcagaaccaggcggtgcttcgcctgctcgagggcgacgtgatccaaatggccacgggtgagggcaaaacgctggtcggcgccatggccgccaccgggtacgcgctgacggggaaacgggtgcacctgatcacggtgaacaattacttggctgagcgcgacgccgcctggatgcgcccgctggtggagttcttcgggctcagcgtggccgcggtgacggaggcctccgcacgagacgagcgggttgcggcctacgcctgcgacgtggtgtacgcccctgtcacagagatcggcttcgaccacctgcgcgacaaccagatcaccaacaggcagcagacggtgcaacttcctgccgatgtcgcgctggtcgacgaggcagactccgtgcttgtggacgaagcgttggttcccctcgtcctcgccggctccgagggcactcaacaggcggccgggcagatcaccgccgccgtggcccaactcgccgagggcaccgattacacaatcgacgctgacggccgcaacgttttcctcaccgatgacggcgcagggaagatcgagcggctgctcggcattgattcgctgtactccgacgagcacatcggcaccaccttggttcgcgtgaacttggcgcttcacgccaaagcgctgcttatccgggacgtccattacatcgtcgccgacggcaaggtcgcgctcgtcgacgcttcccgcggccgcgtcgccgaactgcagcgctggcccgacggcctccaagccgcggtcgaggcgaaggaaggcctcgcggtgtccgagggcggccgcatcttggattccattaccctgcaggcgctcatgcgccgctacccggtcgtctgcggcatgaccggcaccgcggtcgaagcgacagaccagctgcgctcgttctacggcctgcacgtttcggtcatagaccgcgccaacgagctcgtccgcttcgacgaggccgaccgcgtctacgccacgatgggggagaaaaacgccgctatcgtcgaagaaatcgcgcacattcacgcgaccggccaaccggtgctggtgggcacccacgatgtggcggaatccgaggcgctggccgaggcgcttcaggcccgcggcatcgaggtcaacgtcctcaacgccaagaacgacgctgaggaggcgcgcatcatcgctgaagccggcgacaccggccgcgtcaccgtgtccacccagatggccggccgcggcaccgacatccgcctcggcggcgccgacgagcgcgaccacgacgaggtcgccgcgctcggcgggctcgcggtcatcggcaccgcgcgacaccgcacagcgcgcctggacaaccagctccgcggacgcgccggccggcagggcgacccgggcttgagtgttttcttcgtctcgctcgaggacgacattgtcaaagttggcggcgccgacgagcaagtcaccgcgcgcccggacgccgacggcgcaatcgactccaaccgtattcgccagttcattgagcactgccagcgagtgaccgaaggccagctgctcgagatccattcgcagacgtggaagtacaacaagctgttggcggatcaccgcgagatcctcgacgagcgacgtgcggcgctgctggacaccgacgctgcctggcgggagctcgcccagcgcaacccgcagcgcgcggcggagcttgaccatttgccccgcgaggtggttgagcaggccgcccgcgacatcatgttgtttcacttggacgatgagtggtcggagtacctcgcgctgatggacgacgtgcgcgagtcaatccaccttcgcgctatcgcgcgcgaaacgccgatcgacgagtaccaccgtattgctgtgcgcgagttcaaagatctggctaaccgcgcggtggacctggcgggggagacgttccagaccgtcgacgtcgacgagggcggagcccacttggcggacgccgggtggaagcggccgagctccacgtggacctacatggtctccgacaacccgctcgccggttcgggcaattccgtgatctcggggatcggcaacattttccgctagcttcacggtgaagcgcgcgagccggtattatggccaacgactaattgcacgacccatgagttgcttggaggatccaatgagcgagaccacgggaaccccgcagaatcaggtggaaaccacctcggttttccgcgctgacctgctgaaggagatggagacgggggccacgggctccgcggattcgtccaccagctcggagaacctgcccgagggggcggcactgcttgttgtgaagcgcggtccgaacgcgggtgcccgattcttgctcgatcaggattgcaccaccgccggccgccacccggaggccgacatcttcctcgacgatgtcacggtgtcccgccgccacgccgagttccgccgcaaggaggactctttcgaggtggtcgacgtgggctcgctcaacggcacctacgtcaaccgcgagccgcgcaactccgaggtgctctccaacggcgacgagatccaaatcggcaagttccgcctcgtgttcattacgggcgagaactaaccttcgtcgccccccagcgccccaggagccggggcgcgccctttctccccaaccttcaacctcgaggaaagattgagcagtcttgagcgcaattcctaagacttccgcgcccacgcgcgcggccgcgaagccggcaaaggcggcgaagaccatgtcgattggtgtggtcttggagcagctgcgcggcgagttccccgacgtcaccgtgtcgaagatccgcttcctcgagtctgaggggttgatcaccccgcagcgcaccgcctccggttaccgccgcttcaccgacgaggacgttgagcgcctgcgctacatcctggtcacgcagcgcgacaactacctgccgctgaaggtgatccgcgagcagctcgaggcgatggacgccggaaagttgactgccgtcacccctgcggaagcggaacccgtcgtctctccggagtcgttccgcccggccgccccggtccgcctcaccgacgtcgagctcgccgagcaggccgacgtggacgctgacttcgtcgaccagctgattcagtccaccctgatcgccccggacgccgcggggctgtttaccgccgacgacgtccgcgtagtcaccaccgctgctgcgcttcgcgggtacggcatcgacgcgcgccacttgaaggcgttgcgcaccgcagcctcccgccaggcagacctcattttccaggtgacggagccggtggccaagtccggcaagcattccgcgcagcaggaggcggaggagatcggccgccaaatgtctgcgctcgtggtgtcactcaacgcggcgctggtcaaaagcgagttgcgccgctccacttcccgctagcgccatggagcagctcaagctggtcggggtgttctccgtcggccccgagaacttcccctgcgcactgctcgaatgggaagagggtaaccgcttcatccccgtgtggctgccggcgctgcagggcgcgatgctcgccgctcggttgagcgactgggaaccggacgatccggacatctacgaggtgctggcccgcgtcgcgcaggttggcggtgtggagatcacgcactactaccagggaaccttccacacggagctttcgcttgtcgacggcaccaaacattccctccgcatcgccgacgctctcctcgtcgccgtgcaagccgacgtgcccatcgaggcggacgcggacgtattgcaccactcctcgttgcgcttaagcgctcgcgacgcgaaggattacttcggcttggatcttggcagtggcgacctcgaggctgaggacgaagccacgctcgaccccgctgagctggaggagttcatgcgcgaactgggcctaggggacgacccaggcagcggcgactaaccttcaagttgaggttgagacttccggcgtgttgcgcatgtgacgcttgaccttaggtctaggctgattttaaataagcaataggccaaatggtaaacaccatgggagtaattacgtgatgacgaacgacgcggaaacaccggtgcaggaatcgctgtttgatatcggcccgtctgacgaggtggggtaccgggtcccgatcgcctgccaggttgccggcatcacctaccgccagctcgactactgggcccgcaccaacctcgtccgtccgtccatccgcggcgcgaagggttccggttcgcagcgtctgtattccttcaaggacatccttgtcctgaagattgtcaagggcctgctcgataccggcatctccctgcaaaacatccgtctcgcggtggataagctgcgcgaccgcggcgtgaacgacatcgccgagatcaccctggtttccgacggcaccaccgtctacgagtgccgcagcaacgaggagatcatcgacctgctcaacggcggtcagggtgtgttcggcatcgccgtcccgcagatcatgcgcgagctcaccggcacgatctcttccttcccgtcggagcgcgtctacgccgacgccgagccggagaacgtggttggcatcgacgagctcgccgcccgccgccgcctcaagtcctcctaatctctcaaacctgccgcctcccgcaccgcgcgcgggaggttttctgctgcctgggcggcctcgacgtcgaggtggatgtcggcgagcgactgcagcgcctggtctttcgccaaatcgccgacgtgcaccaccgagaactcgaccgcgtcgcccgcggcggcgcggatctcctcgacgaacgcgtcgtcgcccgactctgctgcgtccgcggtaccggtggtgataagcacgatccttgtggtgccgtctgcgtcagcaagcgccgctacagccgcccgcagcgcttcgcgggtctgcggctggccgccggtagtgaaacgggtcacgacgcgcgccacctcctcgccgtcggcggccagcgccacattgcggcggtagcccttctccacccctgggctcaacggggaggagtagttccacagccccaccgcgtgcccgtcggcggctaccccgcgcgcggcggttcccacggcttcctccgcggctgccatgaacggtgccatcgcgtcggaggtgtcgagcacgaacagcgtgtcgtagacatcgccgtcggtgatcgttgcgccaccggacggcagcgctgccgcccataccagctccggcaccagcggctgcgcgggttggccgggctcgaagcgctcggcagcgaacctggcgaagtcctgcgctgcgcgcgcctgattctcgtcgacggtccctgcagcgttgaggggaatcgccgcgtactccaccgaagcttccagcggcgtgaactcgcgaccttcgggagcattgcttcccgacgccgccacccactccccagcgcccctctggtttgtcagggcctcgacggcctcgttcggcccgcccgcgagaacgaaggccaccactgctgacgccgccgactcagccgcggtgccggtggggaagctgacgctttgcacgtcggggcgctccgccttcaccgcgccgctcacccccactgggtcggcgtacaccgtggccgggttcgcgaccgcagcggtgcgctgcgcttcggccagttcttggtgggtgatggcggtggcgggagcgaggtacaccgccgcgtcttcaagcgagtcggtgacgaccggctgaatgcagtactcccgtaccgtcggcttcgatgctgcgtacgctccgatcagctccgcggccaccgccgggttcgccgtcgccacaggcagggcgagatcccccagcacacagggctcgtccgtggcggcaaccggggcctcgtcgtcgccgcggttcgcggcgaaccagacggcgccgccaacgagtaggagtgccgcgacgagggcgaacacggccccgccggaaagtgcgtagttgttcttaccgctggaatgccgacccatagctgcatagcttagctggcgagcagaccgtccaacagggcgatgagacgggcgcggatcggcgcggcccgcgctgacagctcgcgctggcgggcgacgtactcggccttgccggcgggcgtttccaccgcgacgacaccgagaccgagcccagtgcagtcatagggcgaggcctccatgtctaagcggcgggcgtcgaccgccagctcgaacgcatcgaggaggagctcacccggcgccgcgggacccatcttcgcggcccacttgtacaggtccatcgcgacgtggacgcaccccgcctggtcgctgtcggcctggtcgtcgcgctcaaggactgtgaggttgagcggtttcgctgcgggtgtgaagaagcggtacgcatcgaagtgcgtgcactttagctggtgcgattccaccacggcgtcggttgcggcgctgccaaggcgaagggggaggtcgtggcgcggcgcgtcccggtagaccattgcccattcgtgcatgccgaagcaatcgaagtggctcggacggtgctccaccccgcgcagcagcgcgcgtattcgttcacagtcgttgcgccgcttcgccagaaacgcgtcgcggtcgaagccgacgctgccatcggggtgcgtggtgtaaaagggaagggttgcgtggggggaggcgtgggcgtcggcaagcactatgccccaacccgggtgccaccgcgaaagctggctggcgcggaaagggtagtagtcgaagaggaagtcccacactgggtggcgctcgccgcgcgtgcggcgcgcaaggtgcggacgcgtgtaccgcccagcgcgcgtctcgtgctctgcaatggctttgcgccacgcttcgggcgggaggctagtcgtcctcatgcgtccagtcgctcaccgtgcccacgtactcctcgatgatgtcctcgagcgcggcgacgccgacgaggtcgccgttgtcgcggacctgggccatgtgggcggagcggcggtgcatgctcgtcagtgcgtcgtcaagcgtctgcgccccgtcgacaatgctcagcgggcggatgcggttgaccggcaccaccgggttctgctccggagaatccatgaggtcgaggatgtccttgacgtggatgtagccgaccagcacgcccggcgcgcgctcaaccgggaagcgggagaagccggtgtcccggacggtgtcctccaccaaagacagcgggatgccgcgggaatggtacgggagcgtcttcagctcgtcgagggggatcatgacctccttgacgttgcgcgattcggtgcgcagcgccttcgccagccgggctgtttcctcggcgtcgagaaggccttcctcgttcgactcccggatcatcgtggccagctgctcctgatccacagtggattccagctcgtcgcgctgctcgatgccgaacgccttcagcgtcttgcgagcgatccagtttaaaaactcgatgatcgggcgggtgagcttcatccacacggcaaacgcaggcgtcagcaccatggcggtggcctcggggccggcgatcgcgatgttcttcggcaccatctcaccgaacatgatgtgcaggaacgagatgatgatcagggcgatcacgaacgagaccgggtgcaaaagctccgggggcaagttcagcgatgcgaagggcacctcgatgtagtgcgcgatcgcgggctcagccaccttacccagcaccaacgacgcgacggtgatgccgaactgcgctccggcgaggtatatcgagaggtgttcgatggcgtagatcaccgcgcgggcctcctccttgccttgggcgaggagggactcgaggcggtcgcggcgggaagacaccagcgcgaactctgttgcgacaaagaacgcgttgaccgcgagcaggacgacgattaaaaggattgccacaacaacgttcatcgcaagctcccttccgcgtcagcctggagttgtgctgcttgctcgggggtaatcggggacaggattgccttgtcgacgcggcgttcatccatcacagtgacgcgagcgagccagaaaccgtcgccgcccgaggtgagcccctcttgaaagctttgcggctgggtgccgggcagcaccgctcggtcgccgacgcgcggcacgcgcccgaggctggccataacgaggccgccaagggtttcgtacggcccgtccggggcggtgtagccggtcttcgcggccaagtcgtcgaggcgcaccagccccgccacctcccaggaggtgccgaacttttggaagtcgcgctccgactcgcggtcgtcgtactcgtcgtaaacctcgcccagaatctcttccacgacgtcctcgatggtgacgagcccctgcgtgccgccgtactcgtcggcgacgagcactacctgcgaaccggcagagcgcacccggttgagcacggagtcgccgtccagcgtgcccggcacgaacggcaccggccgcgccatcgcggacagcttggtcgtggagcgctcttctctcggcacgttgaacgcgtccttgatgtgcaccacgccgatcgtgtcgtctagatcgccgcgccgcaccgggaagcgcgagtggccggtgtcgcgggcgagcacgatcaagtcggcgacggtgtcgtcggcgtcgagcgagtcgatggtggagcgcggcgtcatgacctcctctgcggtggtctcaccgaagcgcagggagcggtcgatcaccgccgctgtttcggcgtccagaccgcccgcttcggctgaattgcgcaccatcgcgccgagctcctggcctgacctcgcggaagcgagctcgtccgcgggctcgatgcccatcttccggaccacccagttggcagacgcgttcaaagcgttgatgaaccacttgaacacctgattgaaggcgttcaccggcgggacgacgaaccgagccgtgggcaacggctcggtaatcgcgatgttcttcggcaccagctcgccgaagaccatagacagcagcgtcgcgataactagggcgaggatcatcgccactgtttgcgacgcgctctcgccgagtccgatcagctcgagcaggggagtgaagtactgtcccagcaccggctccgccagaaaacctgcagccagtgtcgtcaccgtgatgcctagctgggccccggaaagaacaaacgagaggttggcgtggtcgcgggccacggccttggccgtcgcgtcgcccttctctcggacgtgggcctcgatcgtcgagcgctccaggccggtcatggcgaactcaatggcgacgaacaagccggtcgaggctgtcagcagaatgaatccgagcagggaaagaatggatatgaaaatgtccatgtgcgtgggctaccgcgttagcgtgagcgtctcctgtttctctgttggccacttcgctgaccgccatgttgaccgccgcggcgcggtttcgctggtgcttgcgactgggattggcccgggggcggcaacggtgcgcccgccggaacacgcgcgccggtaattttagtcaactcctccgactccggtgagacccgcacttcccgcgcgtcgaccccagctttgcgcagcagagccgccacgtctttctgctgctcatcggttacgagggtgaccacggtacctgacgtgccggcgcgggccgtgcgtcccgcgcggtgcaggtaggccttgtgctctgccggggggtcgatgtggacgacgagggagacatcgtcaatgtcgataccgcgggcggcgatgtcggtcgccaccaggacgggcgtggatccgtcagtgaagccgtcaatggcgcgcgtgcgcgctccctgtcccttgtcgccgtgcagtccctgggcgttgatgccgacgcggcggagtttcttcacttggcggtcgacaccgtgcttggtgcgcatgaacatgatcgtcttgccgtcgcgggcggcgatgcgttccaccaccgcgccgcgttccttgcggtcggtgaccaacaggcggtagtgctccattgtgtccacggcagcttctaccggtgcggtggagtgcgtcaccggctggtgcatgtagctgtccacgagtttctgcacgtcgccgtcaagcgtcgctgagaacaggaggcgctggccgtctcgcggggtgcggtcgagcagcttgcgcacctggggcagaaagcccatgtctgccatctggtcggcctcatcgagggcggtgatctcgaccttgtcgagaaagagcttcttctggttgatcaggtcctcggcgcgccccggggtggcaaccaggacgtccacaggggaggcgagagcgcggatgtggtggttgatgttcacgccgccgactacctcgatgacgcgcaggcccacggcggcggctgggtcggcgaggcggtcgctgatctgggcggcgagctcgcgcgtcggggagagaatgaggctgcgtgggtgacccggcttggacggtgcccccgccaagcgagcgatgatcgggagaccgaacgtgaacgtcttgcctgagcctgtgggcccgcggccgaggacgtccttgcccgccaaagcgtccgggatcgccgccgcctggatagggaaaggttcagtgatgccctgcttagtcagtacggaaactatgtctctgggcagccccaggtcggcgaacgaagtcattacgacgatgttaaacgctctccgccctgtttcctagtagctctagtacgacagctcctcgcgctcgccggaccacgtggtgtggaacgtgccttccatgtccacgcggcggtaggtgtgcgcgccgaagaagtcgcgctggccctggataagcgcggccggcagacgcttggcgcgcagcgaatcgtagtaagacagcgaagaggcgaacacgggtaccggaaggcccagccgagtggctgccacgaccacgcggcgccaggaatccaccaggcccttctccagctcacccttgaagtacgggtcaagcaggagcgacggcagatccgggtcgttctcgtaagcctcggtgatgcggtcgaggaacttcgcgcggatgatgcagccgcctcgccagatccgggcaaggtcgcccggcttgatgtcccagttgtgctcctgcgagcccgcgttgatctcgtcgaagccctgcgcgtatgccacgagcttggaggcgtagagcgcccggcggacgtccgcgatgaactcctcgcgctccatacccaggtcctcgagcgtcgacagctctccagcaggcagacccacctcctgcgccgcttcgcgctgcgctaaggcggatgacagcgcgcgggcaaacaccgcctcgccgatgcccgtcgtaggcacgcccaaatcgagggcctccttgacggtccagcggccggtgcctttctggccggcggcatccacgatgacgtcgataaacggctgccccgtgcgagcgtccttctggcgcagcacctcagccgagatctcgatcaggtacgagtcgaggtcgcccttgttccactcggtgaagatgtcggccatctcctcgggctcgatgcccgccgcgtggcgcaaaaggtggtacgcctcgccgatgacctgcatgtcggcgtattcgataccgttgtgcaccatcttgacaaagtggcccgcgccgtcgggcccgatgtgggtcacgcacggcacgccgtcgaccttcgccgcgatggattccagcaggggacccaaggtctcccagctctcggcgggaccgcccggcataatcgacgggccgagcaacgcgccctcctcaccgccggaaatacctgcgccgacgaagtggcggccgcgctcagcgacctcgcgttcgcggcggatagtgtcggtgaacagcgagttgccgccgtcgatgatgatgtcgccgtcatccatggcggaggcgagttggtcgatcaccgcatcggtcgcggggccggcttgaaccatgatgatcgctttgcgggggcgctcaagggacgcgacaaactcctcgatggtttcggccgggatgaagttgccgtcgtggccgtgcgcctcgatgaccgcgcgcgtcttctccggcgagcggttgtagatggccacggtgtggcctctggaggcgaagttgcgggccaaattcgagcccatgacggccatgccgacaacaccgatttgtgcgaggggagcgcttgagttggtcatgaacgccagtctacgtcgctatagttgcggccatgacgcaactcccggaggtgttgaccgagccgatcggcgaccgcgaactcactgctcaacagctcgctgcgctcaacgcggcgaacgtggggtttgcgcagctcgttgggctcgagatcacgcatgcgtctggggccctgcttgccgggcgggtcggcgtgggggagcagcatttgcaggtggcgggaatcgtcaacggcggcgtcttcgcggcgatcggggagacgctcggctccgccgccgccatcctcactgcgggcgcccccgccattgggatgagcaacaacacggatctcttgcgtagcgtcaccggcggcaccatcgaggcagaagcccgccccgtgcacataggccggcgcacgcacttgtggcggatcgagatgcgcaacgacggcgcgctagctgccgtcaccaacctcaaactgttgattccgtaggttcgcctacagccacttgttgcggcggaaccaccagaacatcagagccatcaccgcgaacataacgatcaaaacgacggggtagccgtacttccagttcagctccggcatgttcgtgaagttcataccgtatacgccggcgatcatcgtcggcgcggctgccatacccaccacggctgagatcgtgcgcatgtcggcgttctgctgcatggtgactttcgccacggaagcgtcgataagcgagctcaagcgctcgtcgaagccgagcagctggtccgagacgatcgtggcgttgtcctggacgtcgcggaagtaggaacgcagggcctttcgcaccatgtccttgttgttggtcaggccgttgcgcagcgccggggcaagcggatcgatggcgtggcgcatctccaagatctcacgcttgtagttgtagatcttgtccacgttgatcatctggttgggagtgaaaacttcgttctccagctcgtccacgtcgcggctgagcgcctcgccgacacgcaagtagttgtccaccaggtagtcggccacgatccacgccaccgcactcgggcctaggaccaccaggtcttcttcttcctcgagcttggctgtgagatcgggcaacggggcgttgtggcggatggtgatcgcgaagtttggcccggtgactacctggacttcgcccgtggaaatgatctcgcgggcgtcagccacttcctcgtcgtcgcggtagtggacggagcgcacgaccatgaacaactgctcgtcgtagcggtcgatcttggggcgttggtgcgcgtccacgatgtcgtcgacgatcaagtcgtcgaggtcgaagaccgccgcaacgcgctccatctggtccacgctcggcgcttttagcgacagccaaacgaacgcgttgtcgtgctgctccgccatctcgagcgcctggggaacgcggtagttgttgggcagccgtttgccgtcgacgaagacgcggcagaagtcgacggaccgctcaatcggaaccgggacgtaggcggggggcgcgggtttcttcgctttcggacgggtgagcgggatgcgtggcggcatgggcttcgagccccctttcactcgtgcgaggggctacaggccgcgcggcctgtagcccctgtgcggagggagaacgcgcactccgcggtgcgcaggacgattaaggtaatactacgcctttggcgcgggttagaaaacagtcagcccgcgcgagcggaagaccgagcggacgtgctcgaccgactccaaagacgggggagtaacatccttaagctcgtagtcgagcccgatcttgtcccacttgtcggcgcccatattgtggaacggcagaacctccacgcgttccaccgtgcccttccagcgcgaaacgatgtccgccacgcgggccacgttttcctcgccgtcggtaagacccgggacaagcacaaaacgaacccacaccttcttgcccttctcgtgcagccggtcgccgaaatcaatcgttggctggagatcgcgggcggtgacgttcttgtacgtgtccggatcgccggatttgacgtcgaggaggaacaggtcgatgttgtcgagatcctcgtcggtcagccgagcgccgaggtagccggaagtgtcaaccgttgtgtgcactcccgcgtcgtgcaccgctttgagaagccgtcgcgtaaacgcaatctggaaaagcggttcaccgccggagatcgtgagaccgccgcccgacgccttgaagaccgccttgtatcgcagcacccgcttcaccacatcgtcgacgcgttcaagggtgccttccttcatctccatcgtgtccgggttgtggcagaacttgcaccgcaacgggcagccggagaggaagatggtcattcgggtgccggggccgtcgacggccgttactagctcccacgagtggatgagtccgatctcgccggtacgtcgggcgtcgagcagctcggggcgggtgatttccaagtcgtccgtggaaagaccgcctaaaccggcggcgacgccgcgcacgcgctcaccctgttggggctcgagcgtgacgacgccgctagtaccgtcttgagccattacgcacccttgtggaaggtacgggagatgacgtcgcgctgctgctccttcgtcagcttgacaaagttcacggcgtagccagacacgcggacagtcaggttcgggtagttctccgggtgctccatcgcgtcttccagcgtggactcgtcaagcacgttgatgttggcgtggtagaggccggagtccatgttgttcgcggagcgggatgccttcatgctggccagacgctggtcaaaggtgggggtggtcattttctgtgctctccttcggtaggaaaagtgagtgggggaaactggttaggcgggctggatggccgtgtcggcgttgtccatgatgaagccggcgtcgagaacaccgaccaagttggacacctgctcgtccttgtcgcggccgaggcctgccggggtgatggtgttggtcagggagatgccgtcgagggcgtcgttgtagtccaacttgcccacggacagcatggaggcaaccatgccgtggttgtcggctccgttctccgggttcgcgcccggcgcgaacggggtaccggccttgtggccggacgggaaggatccggttgccttgccgtagaccacgttagaggtgatcgtcaacaccgactgcgtcgggatggcttcgcggtacatcgggatcgccttgatcttctgcatcacggtgtggaccacagttgcggcgatgtcgtcagcgcggtcgtcgtcgttaccgtagaacgggaactcaccctcggtgacgtagtccacgaccaagccggtttcatcgcgcaccgggtaaaccttcgcgtacttgatggcgctcagggagtcagcaacgatggacagacccgcgatgccgcagcccatggttcggatgatgtccgagtcgtgcagcgccatctcgatcgactcgtatgcgtagcggtcgtggcagtagtggatgatgttgagcgcctcgacgtaggtgccgacgacccagtccagcatctcttcgtacttctgccagacttcgtcgaaatcaagcgggccgtcgccctcgatcggagtgtggtcgccgtcggtgatctgcttgccgctgacctcgtcgcggccgccgttgatggcgtacagcagtgccttggctgcgttgacgcgcgcgccgaagaactgcatctgcttgcccacctgcataggggagacgcagcaggcgatcgcggcatcgtcgccccacttgtcgcggatctgcttgtcggattcgtactgcagcgacgacgtctcgatagaaatcgcggcgcagaattccttgtagccctccggcagggacggatcccagaagatggtgatgttcggctccggagccgggcccagattgcgcagcgtctgcaggaggcggaacgaggtcttggtgacttggtggcgcccgtcctcggagaagcccgcgtcagtccaggttgcccagtacgggtcgcccgagaagatctggtcgtagtcctcggtgcgcaggaagcggacgatgcgcagtttgatcacgagcgcgtcgatgatctcctgtgcctcgacctcggtcagggtcccgttggcgagatcccgctcaaagtacgcatccaggaagggggagaggcggccgatcgacatggcggcgccatcctggctcttcacagaagcgaggtaaccgaagtaggtccactggaccgcttccttggcgttcgttgccggtccggagatgtcgaagccgtaatcggcagccatcttcttgagcttcttcagcgccttgatctgctcggcgtgctcctcgcggtagcgagcccagtgttcagagaagcccttctccaaggaggcgtccttcgccttctgcttctcctcgatgaggtagtccacgccgtaaagcgcgacgcggcggtaatcgccgatgatgcggccgcggccgtaggcatcgggcaggcccgtcacaatgtgggaggagcgggccgcgcggatgcgcggggtgtaaatgtcgaagacggcgtcgttgtgggtcttgcggtactccgtgaagatcttcttcacgtccgggttgacctctttgcctgcctccttgatggcctgctcaaccattcgccagccaccgttgggcatcattgctcgcttggtgggggtgtcggtttgcaggccgacgatgacatcgtcgtcttcggagatgaatcccggtttgaacgcgtcgatgtctgcgggagtttcggtgtccacgtcgtaaacgcggcgctcgcgctcgacggcgaggtagttcttatccaggtggtcccacaggcggagcgtcttttcagttgctcccgcgaggaacgatgcatccccgtcgtaaggggtgtagttgcgctggatgaagtcgcggacgttaatttcttccgtccacggaccaggggtgaagccttcccacgcctggttctggatttgcggctctgtagaaacagtcacaattgcacggtccttcagttgaagattctgaaatgttccggcggttgcgcttgcccattcccatactcaaagttttaaagcgcttaccgcttgccattcagtatacgagggtgaccatctcgaaagataatatgattgacgtgagcttaggcacattaaaaaccgcccggtgacctgctgcgacgcggttaccgggcggtgacgtgtggagttttagttgttctcggctttgttctgccgggctaggcgctgctccagctcgccgtctgtggacgccagattgtagcgacgcgtgccgagggcgttgcgcagccaggtgtaggcggagacgacgcggctgcggttcgtctcgaggaactgcgcgtggacgatcagccacatcagccaggcgatgaagccggtgaactcgaccttgccaatcttcgccacagcgttgaagcgggagatgatggccatggagcccttgtcgaagtagtcgaacggctcacgctggtcaggctccacctcgtgggcaacctgatccttgatcaggttgcccacgtagtcgcccgactggatcgcgacctgcgcaacgcccggaagcttgttcaggctcatcatgtcaccgatgatgaagacgttgcgcttctcgcccacggagcagtccgggttgacctgcacggtgccgttgcggttaacctcgacgcccgcctgctcggcgacaatgcggcccaggggagaggcttctacgcctgcggaccagatcttggtcgcggcctggattgtggtctcctgctccgtcttcgtgtccttgtaggtcacggagtcggcgtcgacattgctgaccagagcgttgaggacgacggtgacgccctcgcgctcaagctggcgctgagccttcttgcccagtcgcttgccaaacggggggagtacctgcggcatgccgtcgataagcacgatcttggctgcctccgtgctgtaggagtactcacccttcttcagggtgcggtgggcgagctccgcaacctggccggcgagctcaacaccagtcggaccagcgccgacaatgacgaaggtgagtagcttctcgcgctcattcgggtcggtggcgtgctcagcgcgctcgaacgcgtcgttgatgcgcgcgcggatctccagcgcgtcgtcgacagtcttcatgcccggcgcaaactcggcaaagtggtcgttaccgaagtatgactgacccgctccagccgcgaggatgagggagtcgtaggagaactcgagagtttcgccggcgtcgagggcggttacagtctgcgcgtcggtgtcgatggtctgcacgtcagctcgcacgacgcgaacgttgtcctggccgcgggtgagctggcggacggactgcgcgatctcgccggacgacaggatgccggtcgccacctgatagagcaagggtgcaaagaggtggtggttggtgcggttgatcagagtcacgtccacgtcagcgtccgcgagcgagcgggccgcggagaggccaccaaagccagcgccgataatgacgacgtggtggcggttgccagcggggcggatgggccgatctgccatgggttttatctccttgaaggaagcgttcagaataccttcgtagatagtacgccccatagtgcgatccgtcacagtttcgtgtgcgtgggaaccggcccgcccgccaccgcggccgttactatcgatcgggtgatgagctctgatgacgggtacgaccacctctcggccattgatccgcagacgtggcccggcgtcgcgaccgttcctagggtgcgcgccgagtcgctacgagcgcaacgcgcggaggcggcgtttgcggccgcggcgagccgggcggggcttcggcttgacggcgacgagcccgatctccgcgtccacaatgacacggtgttcacccgtgtcgcagccgccggatgggtggggctgttggagggctacctggcaggagagtgggagaccggcacatcagacgggctggtggatgtcctgcgcgcactcgtcgcggcaaactaccaccctcgcacgccgcgcatccggccagtcgaagcgtccgcagggggagagcagccggccgaattgatttcccattactccggcgacggcacgagcccgttccagggccatttcgcgaccggtgtgccgaccacccagcgcaagatggtgaaatctttcgcccccggcgccggcaggggcagtgagcccgccaggcattacgtcgatgtgacggaatacggccacccgctcgaggtggaccgtgcggacctcgcggacgcgcagcagcgcagcgggcagatgcttatcgacgccgcccaaatctccaccggcacccacctccttatccaaccaaactgcggcgcgaccgtcttgcttgaggcatcgcgccgcggagcagccgtagactgcgtcgtctctgacggcggcacgaaacagctgttgtccgaccagctcgtcctgcaaggcgttgaccagtctgtctgcgtcattacggaagccgagattgagcaccgcttcgcctacgacgcgattgcgtcgttcgagcacctagagacgctggcgccggcggaccagagggtgtggttgcgggagtccgacgccgttctggcgccgagcggacgaatcgtcgtgcagtccgtgctggcagaggactccctgtcagctgcagcgaaggcgtccctgatgacgctccgggcgtacgtttggccgggcctgtcgctgatgaccgccgagcagctttccaaactcgttgatcgaaacaccggcctgcgcgtcatcgcagagtcgcgcgcgccagagcaccttgccgagtcgctcaagctgcagcgcgccacattcgagacgcaccttcgcgacgccgccgcagacggattcgacatcgtctaccgcagactctggcgctggcagctcgcactccgtgaagcgctcacgcggcaggggatgctgaatctggctcaagttaccatggtgcgccggagcagacgcgggagataagccttacttgacataatgtacattatcggacatttatcggtagtggtgtggaagtaggtgcactttcaacctcaagtaaacggtattatgcgcggcataatcgccccagggatccctcgccctcaggcatggccaccccgcggttattccgtcacgttacgtaataactgctactccttggtcaggttcaggcggatgttgatctcgccttcctcggcgatcttcgcggcaacaagctccggcgtttccacgccgtagtcgagacggttgatcggtacgttgccggcgatgaccaggttgtcgcccgagcgggcgacgtcgaaggtgtgcgtgatcgaccgggtctcgccgtggatcgtcatgtcgccggtcagttcgatctggctcacggttccgttgccgccaacgctggaaatgtccgcgggctgagtaagcgcgaacgtggattctgggaacttgtccgtgtggaagatcttgttgcgcacgttgttgtcgcgcacgtcgctgtcagtggtgatgttggtcatgtcgacaacgatttcgcccgcggtaaccgtggaatcagcgatggtcacgtgacccgacacgccttgggtcgagccggaggtctcgcggcgctcgcccggcaggacttcgttaaaggtgaatccggcggctgagcggttggctgagggccggttcgacaccgtccactcgccgtcaacctcggttgttgcctcgcgcagcgccgagtcgtcgatgcccccggtcttcacgcccgagccgagcatgtttaggaacagcggaaccatggcaacgagtactgcgagcacgatgaagatcgacaccgcgacgatcagcactgtctgcttcttcttctgttgggccatggtctcctacctcaacttctcaattcttacggctagggtaactaattcgtcacaaaggtgacgaatttcagagggttctgccccctcggtcaccgcggtctgtacgtcctcggcggcgcaccgcaactcgtacaactcgtcccggatctcgtcgacgcgctcgggccgcagcacgatcgatccctcagtgatcccggtgttgctgacgctgttgcggtgctcgtaggcgcgctgcttacagctgggtccgcagtacttgcgtttgcggcccctcccctgctgttcagcgagctcgcggccgcaccactggcagacgggagcgcgcttgttcgagctaggtgtcgcggctgtcacggcgattcatcgtagcagggaacaatcgcgccacctagaccgttataatgtttcgactgatagctaccaaccgaagggaagttgaacagcatggctgatcgtgttctgcgcggaagtcgcatgggtgcagtgagctacgaaaccgaccgcgatcacgacctggcgccccgccagatggcgaagtacaagaccccgaacggcgaggtcttcgaggtgcctttcgcggacgatgccgagatccccgaagagtggatgtgcaagaacggccaggtgggcaccttgatggaaggtgaaggcgtcgaggcgaagccggcgaagcccccgcggacccactgggacatgctgctggagcgccgcagcattgaagagctcgacgtccttctggaggagcgcctcgagcagctgcgcaagcgccgccgcaacgcggcgaagatggcgaaggagcagcaagcctccgaagaggcgtaagctcagctacttccgcagttcccgcactgcgacgcgggtgaactcggtagccgctgctagcctatctctgacggcatggacggcgcgggacggcagctgcggcacctttgagtgggcaagctcgtgcttgcccactttcgctatttctgcagccgcgttcgcggcgttgccggccgcgcccttcagcttaccgcccgcctttggcaggccagagtggcggtactcgtagctggcggtcgaagcgatctgcttcgtgaggtcggtggcggtggcgacgcgttcagacgcgccccacttcgtcacctcggccagagaggtgacggcgaagctcgggtcgagcttggactcgccgagcttgcggtcctcgaaggtgatcggcacctcgcgcacatcgaagccgtcgccaatcacccggtgcgccacctcaacctggaagatgtagcccttctcggacagcgtgtccaggtcgatctgctccagcacttcgcggcggaacgcgcggtagccggcggtcatgtcaccgacttcgtcgccgagcgctagagcgacgtagcggttgcccagcttggacaaaaggtaccggctcttcggccagttcttcacctcgccgccgtcgacgtagcgggatccgatggcgaggtcggcgccgtttgacagggcgtcgataagccttgaaagctcctccggcgcatgcgaaccgtcggcgtccatctggcaaatcacctggtagtcgcgctcaagcgcccagcggaaccccgcgcggtaggcggccatgagaccttctttaccgcggcggtgcaggacgttgacctcgtcgtgctcggcggcgagctcgtcggccttgtcacctgtgccgtcgggcgagttgtcgtcgacgaccagcacgtcgacgtcgtcgttggcggcgaggacgcggccgataatcagcggcaggttctccacctcgttgtaggtgggtatgatcaccaacgtcgagttcgacacggtggtgctcctttatcgttgttcaagctgtgtacccgaagcagcatactcgcgcctcgtggtggtcagcgcggtgaccgctacggcgaggcccgcgataacaagcagccactccaccgcggagccgatgtgcacggccggggtaacgcggtcgcgcaggggtagctcctccaccagaaacgcgggcgtaaaaatctccgagtgctgggagaccgtgccgtccggatgcacgatggcggagacgcccgaggtcgcggcgacgatcacggcgcggtccagctcaatggcccgcaggcggctcatcgccagctgctggtacgtcatgtctgtaaacccgaaggtggcgttattcgtcggtgtcgtcagaatctgcgcgccgtttcgcaccgcgatgcggtacgcggggtcttccgccacctcgtaacaagtggcgatgccgacgttgacgccgcccatcgagacgacgcccgggccgtcgcccggcttgaaatcgccggccaggtccacgaggtcggagaagttgcggaagaagtcgcgcatgggcatgtactcgccgaacggctggaggaaccgcttgtggtggtagtcccccgccccggtatcggggtcgaagacgaccattgtgttgcgcgcgcccacctcgtcgcgggtgagcgtgccgacgagcaccggcgcgtccaccgcgtcgaccgcctcagccacgagcgctgcggcctccgcgtcagcgaacgggttcacgtcggacgagttctcgggccatatgacgaggtcgagggggttgttgcgggtggcgtcggcaagcatctgcgtctcgtgcacgtggtttgccagcaccgccctgcgctgcgcgttgaagtccagccccatgcgcggcacgttgccttgaacggcggcggcgcgcacggtgccgctattctgtccgctttcaacatcgtggacaccgagccctgccaacaacccgagcgcgagcggaccgatcgcgcacgcggcggcggttgcccgtgcccggccgttgcgctggaccgctccgatgaaaccggcccccgccagcgccgccgcgaacgtgaccagcgcaggcccgccccacgacgcgagcgcggcgagcggcccgttgatctggccccaggcgaggcgcacccaggcgaacccgccgaagggaaacgacgagcgcaggaactcaaccgcgacgtacaccagcgcgaacgccgcgaagccgtagcgccaacgagcgaccagtacgccgaagacgccggtcaggatgccgtagagcgcgaggaagatagacagcgcgatgtacggcatcgcgccgacgaactcgccgacccacggcagcagaaagagatagcagaacagcgtgtgcgtaaaccccagcagcgcgccgtacccagccgaggggcggctggtgcgccacggcgccagcgccaaatagaacagcgcgatgccggcgatgccgaggaggaagtacccgtgcggctcgtacgagaggtagaccagccacccggcgatcgccgcgaagccgaagcgtaggaacgcgtccacttacgccccgcttccggggcgcctgcccgcctcaggcccgtcctcgccggggctgtccatgcggtacatctcctcgagttcctcggcgtcgatcacctcgtgcgactgagcaggctgcgtgaacgagccgtaactggtggtgcgcttcgccagcggggaggcgttgaagacctgcatgctgaagtcgtcgattttgcgctgcgcgcgtgtggtgatgccgcggcgaatcaacccgcgcgtgggcggaaacaccgtcaacaggcccaagacagtggagacgaaccccggcaccacgcacaggcaccagcccaccagaagcagcgccgagtcgccggcgagctggcctatcgacgtgcggccctgcgcggcggaagacagcgcggagcgcatggagaggctggtcgcgacgccgccgagcagcatgcacaaaaagatggcgaggaacgcccaccccaggccgatccatttggccacgccgatgaaggcgaggacctcaacaaagaaataagcgaagaagatcagcggcatgcggcatagattaccttggcgcgtgacgccacagccgacgcggcacccgccgcatgacgaaggcaagcagggccagcgaccgcgggatccagacggtggagcttttgttgcttgtcgacgcagccaccaccgcatccgccaccacatcaggagtcaccgacaacggcgcaggcttcatcccctcagtcatcgacccgatgacgaacccggggcgcgccgtgatcaggttgagcggggtgccgtggaggcggtccgctagcccctggcagaacgcgtcgaggcctgccttcgtcgagccgtagacgtagttcgcccggcgcgcccgccacccggcgatggaggagaacgtgaagatctcgccgcgctccaattcgtccgccagcacggtgagcatggacgcctgggctgtgtagtcgaccgtggcgatgcgcaccacctcgcgctcgtcccgctctgcgagctcctggtcccccaggatgccgaacgcgacgatggctgtggtcaggtctggaacggatcgcacgagctgccggtgtgatgagaagtcagtcgcctcaaaggtcacgcgctgtacgcggcgggcgccggcgtcggcaagcttgtgctccacttcatcgagccgggagatatcgcgcgcggcgagtacgacgtcgcggcccgggcacagccgaagcgctacctcgccgccaatgtcgctggtcgccccgagcagcagaattgtcccctggctcaccgcaggctcctggtcacgttgttgaggcgccgcgctccaccggcctcgagcaccacgatgtcttcgatgcgcacaccgaacttgccgggcagatacaccccgggctcgattgagaaggccatgccttcccgcagcacggtgtcgttgcccgcgatgataaacggctgttcgtggaccgcaagcccaatcccgtggccgaggcggtgggtgaaccgctggccgtaacccgccgcgtcgaggcactcccgcgcgaccgcgtcgagctcgcctgcggtcatcccgggccgcgcggcgcccaccgcggcctcctgcgcgtcgagcacagcgcggaaggcatcagcgaactcctcgcccgcgccagcgccgccgaccacgtacgtccgcgtgcagtccgagtggtacccggatgaaagcgtgccgccgatatcgactaccaccgggtcgcccacccgaagtgtgcgctgcgagaactcgtggtgcgggttcgccccgttcgcaccggagccgacgatgacgaagtcgacgctatggtgctcagctgcgatcagttccgtgaggtcctccgccacctgcgcctcagtccggtcgggcagaagcagctccggcacttgcccgtggacgcggtcgatcgccgcgccggctcgtgccagctcgctgatttcaccctcgtctttcaccgcgaagtccgccgccgcaagctgggcgtcgcccaccttcgcctgcagctcaaacacgtggtccgctgtcagcgacgcggtcagacgagctggcccagggggcaggtgctttgcgacgatcccgtacacatcctcaccatctccccacccaaccacgtcaacgcccaccagcgacgcctcgttcgagaccgtctccacatcagtcagcggggcgaggagggttagcgcgtccttcgtcaccaccagggcggtgaggcgctcatgcgagctgccgtgaaaccccgtcaggtacgccagctcggcacccgcgccgaccacgtagcccccgcccccgctcacctgctgctgcagcgccgcgcggcgcgcggcgtagacctcgtcactgaaaaacggcatagcgacatcgtaggtcgataccattggcgaagtgcacttctccccggcccaccttgtccgcatcaccgcccccggcggctactgcagcggaactctcatcgggccggagacagtgctcacgtgcggccacttcctcgcgtccgcggacgcggcggctgtgcgttgcgctgtgtccggtgttacgcgccgcgcccgcgccgtcgagttctactcccacaccgacatcgcggtggtgcacctggactcccccgtggagacggcgcagccgtttccccggtttggtaccccgccgaaaccgttcacacccacagtgaccttcggctttggcggccgcgcccgccaacccgcagcccgcgtcggcaggttcattactacgctgccgttcgcggtctcgcgcagcggcaccaccgtcgtgcgcccggcaggactcatcgcgaacgccccgcgcgcgatcaagggcgattcgggcggccctgtgatcgcagacggccgggtcgttgccgtgcagtccctcattctggacccgttcggccgcaacctcgggctggccacggtgtcgcttctcagctagttgccaatcgccaccacaccgcggcggatcgcttcgacggcgcggctcgcgttgcgccggatctcgtccgagtacccggtgttgtggatctgctccagtagatcgatcacctggcggcaccagcggacgaagtcgccgggggtcagttccgcgcccgattcggccgccgcggcgagcgcgtacccgagcggcgccccggccgtccactggtggatggacagtgcgaagccggcatccggcagcctcgtcggcggcaggtggtggcgctgctcgtcggagaccagctcgccgtagatgcgctgcgtttcgttcatcgcctcggccatccgctccgtcgcggcctctggagagccatgagtggacttgcgattctcgaacaccaccatcgatgcgaccccggccagctcggccgggtcgagatcgtcccagatgccgcgcttgaggcactgcgccaccaacaggtccgagacgttgtggatgcgggcgaggcgctcgccctcgtcggtgacctgcgcctcgccgtcgacaacctcgacgtagtccatctcagtcagcagcccaatgatgcgctcgaagtggcggccgagcgtgtcggtgctggaatccacccggtccttcacgcggataagcttgcgctcctcgcgcaccagctcctcaccgacgcgcgccagcatctcgcgctttgctgccggccactcgtgcgccgggtggtgccggatcgcctcccgcagcgcgaggacctgcttgttcgggcgggtccgggcttgctcccgcatcttccggggcgctgtgaagttgccgcggtgcagcatgtccacaacctttcgcgtgtgcttcctcggttgctcctgcatgtgccgcggcaccttgatccggcccaccgggatcggcgggttgcggaaggtgtccacacctatgcgccccgaccagccgcgctcggtagtgacccacggccttgggtcgtcggggcgacccgccggctgaacaaccgcggcgagttccggcatcttgttgcccggaatggcgatgacttcgcccacctgcaggcgagccagaatcttccgcgtttccacctcgcggtcactcagcgaggcccggcgcgcttccttctccgcgtccgtcaggtcgcgccgcagctgcaggtactcgaccaacagttcggcagggtcgtcgccctcgcccacgggcagcgcgtacgtcgccacgtcgcgctcgagctgctcgcgcagcttgtccaccttggcctcgcggcgctcgatgtcgcggacttcaccaaccacggagcggtccgtttggaactgggcgaaggactgctcgatgagtctgatggagtcctcgtagccgttcatgccgagcatgttgatcgccatgttgtagccgggcgtgaacggggagatcagcgggtaggtgcgggtcgacgccagccccgcgacctcgcgcggatccatcgcgggtgcccactgcaccaccgcgttgccgatgtggtcgatgccgcgacgcccagcgcggcccgtcagctgcgtgtactggcctggtgtgaggtcgacgtgcgcctcgccgttgaacttcaccattttctccagcacaacagttcgcgccggcatgttgatacccagcgccaaggtctcggtagcgaagacgaccttgaccagcccgcggacgaaaagctgctcgacgatgtgcttgaaagcgggaagcatgccggcgtggtgggcggcgaaaccgcgcacccacgcggtgcgcagctggcggtagttcagaacttggaggtcttcttcgggaatgtctttcacgccgtcgtcgataatcgccttgatctgctcctgctcttcgggtgtggtgagctccttgcgcgagcgcaggcactggaacagggcgccgtcgcagccggcgcgggagaagatgaaaatgattgccggcagcatgtcgcggccttgcagggcttggactacttccggcctgccgacggggcggacccggtcttgtccccgctccctgccgctgcggcgaccggccgcgcgggaccggaacccccgtccctgctcgtagtcttctcggccctcgtcgtgcgatccctgctcgatgcgggcgatggcgtggacgaggtcgtcgttcacggtgtcttccccgggttcaaaaagcgggaagatcttgcggccgaccatcatgtactggctcagcggcactgggcggtgctctgagacgatgatggcggtgtcgccccggacggcggcgagccactcgccgaactcctccgagttcgacacggttgcggacaagccaatcaggtttaccgagtcgtccaagttgagaatgatctcttcccacaccgcgccgcggtcgatgtcggcgaggtagtggatctcgtccatcaccacgtgcgaaagccggtcgagctgcggcgacttcgcgtagatcatgttgcgcaggacctcggtcgtcatcaccaccacgtcggcggagccgttgatggacacgtcgccggtgagcagccccactgcgtcgctgccgtgctcggcgacgaggtcgtggtacttctggttgcttaaggctttaatcggcgttgtgtagaagcacttggtgccccgcgacagcgcaagggcgacggcgaattcgccgacaattgttttgcccgatcccgtgggtgcgcagaccagcaccccgcggtccgcttcgacctcggtgcacgcctcgatctggaacgggtcgagcgggaacggtttctgcgcctggaattccgcgaaaaaggacataccccctagagtacgtcttcgaaaatatccttcgctggggcgatgggggctggccgctcgatcggctcggggcggatcgcttcagaggcgcccgtgctgccgctggccggagcaatcggggcggttgagatcggcccggacgcggtctcgtcgtcaaggtccatccactcagggcgcgtcgactccttgcgcctgtcgttgaaccggcagaactggaacgccagctcgaccaggacaaccatggacgtgccgagcgcgaccatggagaaggggtcctggcccggggtcatgaacgccgcgaagatgaacaggcccacgatgatcacgcgccgcttgtccttgacgtgctcgtagcgcagcacgcttgcgaggttcagcatgaccacgatcagcggcagctcgaagctcacgccgaagacaacagtgaggccgagcaggaaattgtagtagctctggccggtcaagccgccgacctgcacctcgccgcccatggtcatgagcacgtaaaggccctggtcgaggacgaagtaggcgagcaacgcgcccgcaatgaacaacaacaccgctaacgtgacgaaggtgaaggtgtagcggcgctcgttcttgtgcagacccggcgtgatgaagttccaaatttgcagcagccacaccggcgacgcaagaacgagaccagccaacgcgcccaccttcaggcgcagcatgaacatttcaaacgggctggtggccagaaggcggcaggaaccgtcgtgggtgaagtccgcgcgcagttcctgcgggaggttgcagtacggtcggcggatgatctcccctagcggcatcgtccccgggatggcgttttgataccagatgaacccaatcaccgtgccgacgacgatcgcggcgagggagacgatgacgcggcgccggagctcctgcaggtgctcaacaagcgtcatctccccttcgggattggccttgcgcttgcgtgccacgttttagagctggcggggctgcgtttcgggacggtcccagaaatcatcaggttgcgcaggttgtgcggtctgggtcgcgctgcgggcttcctggctcggcggcagctcaccctggcgtgccggggctgggtcctccatgtcctcgcggcgcatttccttgacttcggacttgaaaatgcgcgcggagcggcccatggaccgagcaagatccggcagcttgttcgcaccgaaaagcagcaggataatcagcaggataatgaggatttcactgggtccgaggttcggcatggacgttatcctaacacgctccgcgcggcctcagcccgcgcctcgacctcgcgcgcaaggcttgcggggctgaccaactgcacgcggtcagcctcgctcaggcagaagcggaccaaccagtcgtcgctgccgtagcgcatggtcgccggcagccacccctcccgctcctcggagccgagctcgatgtccttgtagtcggcgatccacgccgcgtctgagcgcaccttcagttccgccagtttgcgcgtggccaggctaaaggggtcgtccggatcgaacgttgggctcgcgccctccggcgtctgcgccggcagatcgctcagctccacttcgcggatccggtcaaaccggaacacccgcagctgatcaccgtgccacgcgcgcaggtaggtgtgcccgtcccggtggaaaatgtcgatcgggctgacggtgcgggtggtcgtcgcgtcggaagactgcgagtagtaggtcagcgtgagctgctgccctccgccgagggcttgccggatcacgtcggcgggtgaatcggacggggtttgctgcgcgtcgtcgataccagctcccctggccaccgcgcggattttcgccgctgccgacgccacggcagcgctgtccacaagcccgggcatggtttccaaagactcgagcaaaagcagcaacgcgctcgcctccgtgggagtcaagcgcagcggcttgtctaacccctggctgtcgataatccgcacactggcccagtcgtgctgcaagtcgatcatctgaccgccgtgtttgcccacgccggacaggtgcagcatgttgagatcgtcgcggattgtcaccgggtcggagcccaagtcgcgcgccatctccatgacggtggagtcggggtgcttctgcacgtacgccagcaggttgagcaggcgcaccgtgcgctcttgccgctcgtgcttcgccgacaccattactcctgccctcccacgcggctcagcagcgccacgacgtcgcggcgaacctcctcgggttccacggcagtcacgttcggcgcctgcgccgcaatcgttcgcactagccagtcgcggtccacgccgctcagctgaatcgtgtcgccgtcccgcttaccccggctcgcgagtgcatcgccggtgccgggggttagggtgacggtggcgtcgacaagcttggagctcagttgcttttcgacgatcccctgcaagtcccccgaggcctcccgaaaaccgtccgcgccctgcactccggcgacgttcgaaattttgcgcacgcggaacacccgctcctggcccctgtcgaggtcccatccgacgaggtaggcgcggttgttcaacggcacgatcccccaagggtccaccgtgcgccgctggacctgcgctcccggcgcgggcaggaaatcgaacttgaggcgcagcttgttgcgcacgcccgccacgagtttgcgcagcgtctcggggtcgaggcgggtgatgtcgttggacactgacgccaacaccggtgcgtcgaacgcccgcgttgcgccggaggcggcgagcttcgtccatccggatcgcgcgaacgcgccgaggttcgccccctgcgcaaggtccgcggcaagaccgacgacggtcgcctccgcctcggtgagctccacgggctgaagctcgtattggtctttgttgagccacagttcgccgtcttcaagctggatcggcacccacatggagcgaagctccttgacatcgcgcttcagcatgatctggaaggcgctagcggagttgccgtcgtagccgtccacgttggcgcgcacccactctgtggagcgggggcggtcggagccgagcagcgcgaacaccaagttcacgtggcggcggacggcgtcgcgttcactcaccgccggtgacctctgcgataagggcgtccacgcgctcgtcctgggtggcgaacggatcgagcagttccacgcttgtgggctgcgggcggttgatcttcaggtgcacccagtcgacgttataatccgcgcccgcttcccgcacggcgtggaggaattttcctcgcaaagctgcacgcgtggtcgcgggtgcctgcgccacggcctgctcgatggtttcgtccgtggtccaccgcgtggcgaggcctttgcgctccagtaagtagaacagcccgcggtcgcggttgatgtcgtggtacgtcaggtcgatctgggcgagcttcgggtggtcccagtccgcgccgagcttgtccttgtagcgggtcagcagcttgcgcttgattacccagtcgatctcggtgtccacgcgggagaagtcctgggaggcgatcgcgtcgagggtgcgctcccacagatccaccaccttggccatgtccgcgttcggtgtcccctcgtccgggcggttctccaaccagcgcttcgcggcgctgagggtttgccgttggacgtcgagtgcggtggtgaggcggccgtctttaagcgcaagctccgtggcgcccgtcggatccgcggcgatatcccggatgtggctgatcgggttttccagctcgaagtccggcaggtcgaagcccgcctcgagcatctcgatgaccagcagcgtcgagccgatcttcagcgcgaaggtgggctcggacatgttcgagtcgccgacaatgacgtgcatgcggcggaaccggtgtgaatcgccgtgcggctcgtcgcgggtgttgatgatcgggcgcgtgcgcgtggtggccgaagacacgccctcccacacctggtcggcacgctgcgagataacgaagcggcctttctggatcatgccggcgccgcagatgagctggcgggtgatcaggaacggtaggagctgcttgccgaaggatttcagcgccaggtcgcggctgatcaggtagttctcgtgcgcgccgtacgagttgccggcggagtcgacgttgttcttgaacaggtagacgtcggcgccgatccggtcggcggccagcgactcgaccgcctttgccgcgagctcgctgaagattgcctcgcccgccttgtcgtagttgagcagctgggtgaccgagtcgcactcggcggtggcgaattcggggtgcgagcccacgtccaaatacagcctggagccgttcgccgtgaagatgttggagctgcggtgcttcgccaccaccgggcggaacaggtagcgcgagacctcctccggcgtcaacaccgccttgccgtcgcggtaggcggcgaccccgaactcggtctccacccccatgatgcggcgggggtacatctactgcccgcccttttgcacgaacgagcggacgaactcctcggcgttggtgtccagcagcgcgtcgatctcgtcgaggagatcgtccgtgccctgggtgttgatctgcgcctgcgattgttcgaggtcttgctcctcgccgtcgtcgccgcccgggtagccgaagatctgctgctgattagccatgctgtaaccctaacgcgtcaatgagctcgtgcaccccatgagctgcgtcgagcgcgtcgccgacggtttccttggtaaaggagtcgatcgtatccatcggcacccgcaccaactcgtcgcccacccggaagatgatcgactgccagctggccgcagcgatgtcctcgccgaactttgaggtcacacgcccgcggaagtacgcccgcgagtctttcggcggggtcaccgccgcgtgctcgatctccgcggtactcaccatcgttttcatccgccccttgcgcaccagcgcgtggtacagcgacttctcgggatcgatgtcggagtactgaatgtcgatcagctgcagcttcgggtccgcgatatccacgccgcgatctacatactgcttgatcagcgcccatttcgccgtccaatccaggcggtcggccgttgaaagcgggtcgcgttccaggtcgtcgaggatctcgccccagagctggagcacttgcttatcgacgccccccagctcccccaacgccccacaacgatcccgatactcccgcaggatggcggtggcggagaggaggcgggcgtcggcaagcaggagctcatgggtgagcgacggatcgtgcgagacctttttgatctccgcgaccggattcttcagcgcaaggtccgagaaatccaccccggcctcgatcgcgtcgatcaccagcttggtcatgccgactttgaggaagttcgcgtactggctcatgttggcgtcgcccacaatgacgtggaggcggcggaaccgctccgcatccgcgtgcggctcgtcgcgggtgttgacgatgccgcggttcagcgttgtctccagggagatctcctgctcgaagaaatccgcgcgctgcgagatctggaaccccgcccgctcgttcgcctgcccgatgcccacccggcccgcgccgatgatgacctggcgcgtgacaaagaacggcatcagcgcctgtgtcaggcgctggaagtcggtgtcgcgggagtagaggtagttctcgtggctgccgtaggactggcccttgccgtcgacgttgtttttgtagaacttcaacggcgggcacggctcgtgcttgttcagcacgctaacctgctgttcccagagctggcggaccgcggcggccgccttgttcaagtagatgtcccccgctgcgtcctgcaccatcgcgtcgaacgcgttcgaggtctccggcgccgagtactccgggtggccgtggtcgacgtagaaccgcgccccgttctcggtcaccacgtttgcaacgcccatcgcgttcgggtccaccaccggcaccgtgcggtagcgctggaggtcgaacccgcgcgtgtctttgagtggagcctcctcctcgtagtcccaccgcgaccgcgccgccgtgtgcagcgccgcgtacgccaccaccgcgtgcgtggaggtgagcagcgggctcagcgtcgggtcgtcgggacaagtgatgccgtactcggtctcggtgcccataaaacgtgccatgggtcaccagcctagtggggggcggaaattatgcgaggcataataccgtctacttgaggttgagggcgtatcgaacgtgtgggcggtgctgttgggggtctggtatccgcaaaaccccaggggattatgcctggcataataccctttactttaggttgaaggttgctttctcttcatgcgaacgcgtgttctaattcgtggcttcgtgtgttaggtgcgttttgtatggtgtatccactccgtccaaaaggaccttgaaacaaaggaaacatagccatgaccagcacgattaccgccaccgatttcgacgtcaacgccaaaccgccgtcgaagcgagcatatgagatcgcagatgcgatcaggcgctctcaccagagggcgaacatgacgaaatcggaccttctcgagcagatagcggagtttgacgccagcgatctcgcctactcattcggcgcggtgagcaccgcaagctggctcgcccgcgagttgcactacccggtccccactgcctacgagtacgtccgagtggcgcggaaactccaggagtttccgatgctcaagacggcgtttagctatggcgagctggattacaccacggtgcggctgctgctccggtacatcaatgagcgcaacgagagagggctcctcgtgctggcaaaggaactgacgtttaccgagcttcggcgcgtcctcgccggcgtcgaacccgaggataaggatgacgatgaaaagcccgacgagccgtatctggacgcccacactcgcgacgacgggatgatcgccggtagtttccttctcccaccagtcgagggcgagaaattcaaggctgccctcaagattgcggaactggcatcctacggggcgcaagagggtgacgagaccgaacctcctaaagaggcgtgccctgcgaagatggtggacgagccgcgccccaatccggggatgagtgcggagaagatcctccggccgccgtcgcggttcggggcgccgctgaagtcagcgatgtacgacgcattcgtcaccatgatcgacatggtgcgcacgaacccggtcagtccccttcgagcgcccggcgcgcacgtgaacatcatgtgcacgacggacggcagggcgtggatgccctcgaacccgcaggctccgtcgagcgcgatccggcagtacctccacaacgcgctgggccgctggcacatcatggatggcaaggggctcacgctgaatatgggtagacagcagcggttcgccacagatgcgcaggttaccgcgctgctcgctcagtgggagtaccagtgcgcgatgcccgggtgcaaccactcgcggtttatggagatccaccatattcacgagtgggtcgatgggggctcaaccgacatcgacaacctgattcccctgtgttcaagctgccactcgaaggtctcgcacggtcttgcgcacatcgccaacaacagcgggtacatcgagtttaggttcctcgacgggtcccggtacgtcgccgagggccggagcctgcctaagcgggtggaggacttcgaaggtccgatggtcctcgaccccgacgaggtgacctttggctagaggttgagggttaccagccgcgctccgcgagacggtgcggggcgggaaggtcggcgacgttgatgccgaccatggcttcaccgagcccgcgggaagcctgggtgacggcggcgatgtcctgccagttgcgggtcgcggcgaccacggccttggcgcgagcctccgggttgccggacttgaaaatacccgagccgacaaacacgccgtccgcgccgaggtgcatcatgaacgcggcgtcggcgggggtggacacgccgccggcgacgagcaggggcaccggcaggctgccgtgctcggcaacgtaagctacgaggtcgtagggcgcctgaagctccttggcggccacatagagctcgtcgcggtttcctgcccagatcgcctgcaggccggcgatctcggaggtgatcttgcggatgtgcttggtggcctcggagacgtcgccggtgccagcctcgcccttggagcggatcatcgcggcgccttcgttgatgcggcgaagcgcctcgccgaggttcgtcgcaccgcagacaaacggcacctcgaagtcgcgcttgtcaatgtggttgacgtagtcggctgggcttagcacttccgactcgtcgatgtagtccacgccgaggtgctcgaggatcttcgcctcgtacacgtggccgatgcgcgccttcgccatcaccgggatgtcgacggcgtcgatgatgccctcgatgaggtccgggtcgctcatgcgggcgacgccgccctgggcgcggatgtcggcggggacgcgctcgagcgccatcacagcgacggcgccggcgtcctcggcgatacgggcctgctcgggcgtgaccacgtccatgatcacgccgccgaggaactgcttgtttacttcggaaaaatcagccatgcgaacaagtctgtctatccaactggtagattccaagagccagttctagatagtttctctgtaccagttggaggggcacagtgcttatcgacgtcaccgcgaaccacccgctgccccttcccgcgcagatcgcggccggaattcgggccgcggtcgctgacggcagcttgatgccgggggacgcggtgatatcgacgagggcgctcgcggcgcagctcggggtctcgcgcgggaccgtggtcgccgcgtacgaccagctgattagtgagggctacctgcttgcgtcccagggggcgccgactcgagtgcacccggagctgcccgcggcgagcggccaggctggtgcggcgggtggggttgaggtggcgttggcaagcaacctgctgctgtcgctgaaacctgcgccgagcgctgcgggcggcgtgcggcctgcggcgtggcgcgcggcgtggcgggaagcagctgcggagccgggtgggcctgtggacaagtcggggcagccggagctgcgggaggcggtggctgaacacctgcgcctcacccgcgggctgaatgtcgcgccggggcagctggtggtcagcggtggctcgcgcgaggggctgatgctgatcctggccacgctcgctgcgcagaccgggcggcggttgcgggtgggcgtggaaagtccggggcacccggggctgcggcgcatcatcccgatgggtgggcacgagctggttgaatgcgccacggacgtgggcggaattgaggtggcgcacctgcctggcggcctggacgcggtgctggtgacgccagcgcacctgtacccgctcggcggaaccatgccggcagcgaggcgtgcacagctggttgagtgggcggtgcgcaccggcacggcggtgattgaggacgactttaacgcggagctgcactaccggacggcgccccagccgacgcttgccgcgcaggcgccgcagggcgcggaagtgttcacgctcgggacgttttcgacgcttttgtcgaaggagttggcggcggggtatgtggtggcgtcggcaagcagcgcggagagcttggcgcagacgcgccgggtgctggggatgccggtgagcgccgtgacgcaacgcgcggtcgcccacctgctgcgcggagggtacgtccggcgcaacacgcgcgcggtgcacgcgcggctggcggcgcgccgcgacgtgctcgaggccgacctgctcccggcgctgcgggggatgggcgctgcggcggaactgtccggggcggtcggcgcagacgccgtggtgtccttcgcgtccgaggagcgcacggccgaattcgaggcgctactcgcgcaagccgggtacgaggcgggccggctgccccgcgcactgatcttgagtttttctcacctcgacgaggcggagttcgcgacagcggtggcaacgctggagcgcctgaccagccaggcgtagatcgcgccggtgatgttgtgcagcacggcggccacggcgccgggcagcgcggcttcaggggcgaagaacttgccggccatgccggacgacaggccggcggattgggtgcccacctcaaccgcgacggtgcggcggtagctttcgggctggccggtgagtttggcggcgtagtagcccaggacgtagccgagcacgttgtgcagcagcacggcgaggaagacgatggcgccgacctgcagcagcgcgtccttgttcttggccaccgtcgggaagaccacgccgccgatgccgaggatggagatccacggcaggaccggggaaatcttctccatccagctgtccagcacgtagcgcaggacgatcccgccgatgaccgggatgagcaccgtttgggcgagggtcttggccatacccgcggcatcgacgtcgacattctcgccggcgagcagcagcatcacgatcggcgtcatgaacggcgcgacgagcgtggacacgctggtcattgcgaccgacagggcgacgtcgcccttggccaggtaggcgatcacgttcgaggaggtgccgcccggcaccgagccgagcatgagcaggcccaccgcaagcgccgggttgaggccgagcagcttagcgacgaccaccgctcccaccggcatgatgacgaattgggcaacgacaccgatcagcaccggcactggccgccgggcgacttccttgaaatccgggatggtgagggtgagccccatcccgaacatgatgatcatgaggaagtacgtgatgtactgcgtccatggcagaaacggcgccggaaagaaaaacgcgattatcgacccaatgaggatgaacgcggggaaagccgcgacggcgagggctgccgaacgatccgccgcctcttcgcgagtggtcacagtgacctcctgtccgttatgtgggactgaagtcccgccttttgagatggaggctactgtacgggatcggtcagcacttccgcagcgattacgcgttttccgtggcggcccgtgatccgcgcccactcgtcggggttggcggtgttcggcatgtcctcgctctcgtcctgctcggcgcgcacggcggcgcgcaagtggtcggcggtgacgccgcttgccgcacccgcgatgtggtccttgatcgcgagcttcttggcgcgatcgaccacgttggcgatcatcgcgccggaggtgaagtcgtggtagtggagggtttcggtgctgccgtcgacaagcgacagctcgacgaacgggcgcggtgcgaacatggcgtcgactgcggcggcgatgagtgcctccggggtgtccgcgagcgggatgtccggggtgatgtagcgggagaagatgtcggcggcctcttctcggttggggcgcgagacgcggatcttgatgtcgaggcggccggggcgcaggatcgccgggtcgatgagctcctcccggttggtggcgccgatgacgatgacgtttgcgatgccctccacgccgtcgatctcggtgagcagctgaggcacgaccgtggtctccatgtcggaggagacgccggagccccgggtgcggaagatcgactccatctcgtcgaagaagacgatgacggggcggccgtcggaggcgagctcacgggcgcgctcgaagatcagccggatacggcgctcggtctcgccgacaaacttgttgagcagctctgggcccttgacgttgatgaagtgcgcctgtcccccgtcgccgatgcgctgagacagcgagttggccacggctttcgcaatcagcgtcttgccgcacccgggcggaccgtaaagcagcaagcccttcggcggcgcgagctggtaatcgcggtagagctcggggtacgcgaacggcagctcgacggagtccttgatggtgtcgatctgggagctcagccccccgatgtcgtcgtaggtgacgtccgggacctcttcgagcgaaagctggttgacctcggtcttggcaatgcgctcgaaggcgaatccggatttcaagtcggcgagcaccgtgtccccagcgcgcgcctggtccacaagcggctgcgccagctggaccaggtgctcggtgccctgggtgtcggcgacgaccgcgcggcccccgtcaatcttttcaatcagcgtgacaagttggccggttgtttcgtagccgcatgcttcgacgatgacggtgccgtcgccaagccggacaagcatgcccggcgcgagcgcatccggtgcgatagtcggggcgatcttgacgcgcatctggcgacccgaggtgtagatctccgcctccatgccgcggggcgcgggcgcgaggtagatgccgtaggtcgaggcgggctcggccagcgcctcaacttggccgtagaggctgttgagcttgtcgcggctggatttcagcagctcggcgagtttcttgttgcgcgcgccgagttcctggttgtcgcgcttgagctggcgcagctccggtccgaaggcgtcgtcttcaatcatggggccaagcttatctacgcgccctgcgctgcggacgcggcggcgtcacaccgtcggccaagcggcgcgtccacaccaggaacgcggtgtgcgcgttcatgcgatgctcggggcgggtggcaagaccctcgaccttccactcgcggagcagcgtctcccaggcgcggggctcggtgaagcacttggcttcgcggattgcctccatgatgttcatcagctgcgggacggtggcgacgtaggtcatgaacaccccgcccggaatgagcaggtttttgaccgtgtcgatgaactgccacggctcgaccatgtccaagatgaggcggtcgaccgggccgccgaggtcttcctgggtgacctcgccgaagtcgccgaggcgcggcgaccaccaggcgggctcgccgccgaagtactcggccacgttgtcgcgggcgaaggcgaggtggtcgtcgcggatctcgtaagagaacacgtggccttctggcccgacggcgcgaagcagcgacatagtcagcgcaccggagcccgcacccgcctcgagcacgcgcgcgcccatgaagatgtcgccttcaaccaagatctgggcggcgtccttggggtagatcaccgcggcgccgcggggcatggagagcacgtggtccaccagcaaatggcggaagcagaggaagtccgccccaagggtggactgcaccacgctgccttcgtcggagccgatgatgtcgtcgtgctcgacaatgcccttgtgggagtggaactggccgcccggcaccagctcgacggtgaagtggcggcgcttcgcgtccgtcagctgcaccttgtcgccggggcggaacttgccggagtagttgctgatcatggtggtctacgcccctttgtagtaagcggtgagcgcctgttggaaccaggcttggtccttgagcccgacgagttcgcgggcggagtgcatggcgagaagcggaacgcccgcgtccacggtcgggatccccagccgcgtggcggagatcgggccgatggtggagccgcagggaacgtcgtttctgcccacgaaggtctgcaccggcacactcgctgcggcggccgcgcgggtgaacacggcctgcgtctcggcgtcggaagagtagcgctggttggcgttgatcttcaacaccggacctttgtttatcagtggccggtgcgtcgggtcgtgcttctgcgggtagttcgggtggacggcgtgcgccgcgtccgccgagatgattgacgacgccgcgtagagctccagcgggtcgcccagttcaggggcaagctcagcggccagcttcgccagcacgcgttccagcagcggtccgccggcgcccgtcgctgaggctgagccgacctcctcgtggttgaaggctgcgagcaccagcacgtcctcggcgtcgtccaccgcgtcgagcagcgcagccagcgaggcgtgcacgctggtgaggttgtctaggcggccggcggcgagcgtctcgcccaccaccgcgggtgcttgcgtgtccacggagatcagctcgtgggagatcaccgctgctgggtcgacgccggcagcggcagcaatgatctcgcgcatcgactcgtcgacgcacagtacgggctgcatgtgggcctggcggtccagctctggcacgtccccgcggtagaggtggatcgccaggctgggaacgcgcgcgatggcgggtgtgcggatgaggtggctggtgccgtcggcaagcgaaatgcgccccgcgaacgcgagctccctatccgtccacgtgtgcaacagtgggccgccgtaaatctcgacgggcagctggcgaaacccctcgccggcgaattccgcgccgggtttgagcatcagccctggtgaatcggtgtgcgatccgacgatgcggaagcgcgcccgtggtgactctggcacccaccaggcgatcactgcgccgccctggacgtgcacgtgcccgccgggcgtggtggcggtgtcttcggtgaatccggctgcgacgcacgcgtcgcggacggcctgcgctgcgtggaaggcgctcgggctggcggagataaactctgcgaggctagtcatgcctttaaccctagtgctgcgatattgttgccccgatgtctctcgccctctccccctcccgcgccggtgattaccagcagtgtccgctgatgtaccggctcaaagtcatcgacaaaatccccgagccgaagtccatccaccaggtccgcggcacgctcgtccacgcggtgctggaagagatgttcacctggccgcgcgaggcacgcacctaccccgcggcggtcaaacgtctcaagccggcgtgggagaggatgcaggagcaagagcccgcgtgcgcggagccggtggaggacgagatgcagttgcttgtcgacgcccgcgccctcctcaaaggctacttccacatggaaggccccgaacgcttcgacccgcacgcccaagagatgcgcgtcgaagcggtgctgcccaacggcgtgcccgtgcgcgggttcatcgaccgcgtggacatcgctccgaccggcgaggtacgcgtggtcgactacaaaaccggcaaaatgccgctgccccgctacgccgatagcgcccggttccagatgcgcttctacgcgctggtgtactggcgcctcttcggcgtcatcccggcccagctgaagctcatgtacctgaaggtcatggacaccatgattttcaccccgtcgcgcgaggagctggagtacttcgaacgcgatctcggcgacctgtgggcgaaaatcgtggccgacggcgaggccgggtcctttcgcccgcggcagtcgcggttgtgcgactggtgccccttccacgacttgtgcccggtatacggcggcactcccccgccgtacccgggctggccgtcagaataggccggtaatcgcgccgttttcgtcgacgtcgatgttgttggcggccggcaccttgggcaggcccggcatggtcatcacgtcgccggtcagcgccacgatgaacccggcaccggtgcgcggaacgaggttgcgcacgtgcagggtgtggccggtcggcgcgccgagctgagtggggtcgtcggagaacgagtactgcgtcttcgagatgcacgccggaagcgtgtcccagccgttgtctttcagcgtctgcaggtccttcagcgcggcggccgagtactgcacgtcgtcggcgcggtagatttcgcgcgcgatggtggcaatggcgttctccacaccgtcggccgggtcgtagagttgggccgccgtgccttcggagtagttttcgagcagggtcttggcgagctcgattgcgccgtcgccgcccttggcccacacctcggactccgccaaagcgatgccgttttgctgcgcccagtccttcacgaagtcgcgctcggcctgcgtgtcggaggtgaacaggttcaacgagaccaccggcgtgaccccgaatttagccacgttctccacgtggcgctcgaggttgtcaatgcccgcctcaagcgcctgcaggttctcttcgtccaggtcctgtttgctcacgccgccgttgtacttcatcgaccggatcgtgcagaccacgacggcgcccgccacgtcgaggccgccggcgcgcgccttaatgtcgaagaacttctccgcgccgagatccgagccgaagccagcctcggtgagcacgatgtccgcgtagcgctgcgcggtgcgggtggcgattagcgtgttgcagccgtgcgcaatgttggcaaatgggccgccgtggatgaatgccggagtaccgcccagagtttgcaccaggttggggttgatagcgtccttgagcagggccgccattgcgccctcggcctcgagctggccggcggtgaccggctgcttgtcgtaggtcaacccgaccgtgatcgcggcgaggcgccgcttcaggtcggccaattcggtggcgaggcccagaattgccatgatctcggaggccgcggtgatcgtgaaaccggtctcggtgggcacgccgttgcccgcgccgccgaggccggtgaccacgccgcgcagcgagcggtcgttgacgtcgaggcagcgctgccacgtcactcggcgcgggtcgatgcccagcgcgttgccttgctggatgtggttgtcaataagcgcggcgagcgtgttgttggcagcggtgatggcgtggaagtcgcccgtgaagtggaggttgatgttctccatcggcacgacctgggcgtacccgccgccggcagcgccgcctttaatgcccatgacggggccgagggacggctcgcgcagcgccaccatcgccttgtggcccagcttggccagcgcgtcggtcagcccgatcagcgtggtcgacttgccctcgcctgccggcgtgggcgacacgccggtgacaagcaccagcttgcccgggtgcgagtccggaacctgggtggtgtccaccttggccatgtacttgccgtatgggatcagtgcgttagcgtccacccccgctttcgcggcgatggcgtcaatcggttccagggtgtgggcttgggcaatttcgacgtcagatgggatacctgtcatatcggactagagtaccgcagcgcccaacacgtacccgaggcctacggcgatggcgatgcaaatcacgcccggcacaaggaaggggtggttgaagacgtatttgccgatgcgggtggatcccgtgtcgtccatctccacggccgcgagcagcgtcgggtaagtaggcagaacgaacagcgcagacacggccgggaaggcggcgacggcggtcagcgggctgaccccgatcgcaagcgcggccggcataagcgccttggctgtggcggcctgcgagtagagcaggcacgctgcgaaaaagagcaccacggcgagcagccacggctgcgtctgcagcacgtcgcccgcgatcgcctggatgtcctcgatgtagaagttgatgaacgtcgtgcccagccaagccacgccgagcacgcacagcgaggcagacatgccggacttgaacacctgggtgccgagcacctcaacagcctggttcttgctgatcagcaggatgacggcggcagccgccaacatgatcgccataatcgcctcgttgcggggcacgctcggctcctggatgaggccgacctgatcagagatgagcgtggcgtagatcatcacgaccgcaatggcgatgaggaagacccagacggatgcccgggcaccgggcttggtggttgcggcggattgggcggctggcggggaaaccaggccgtcgttaagccgctgctgatacacgggatcgtcctcgaggtccttgccaaggcggttggccacccaggcggtggggaagatggcgataaaggtcgcggggatcatcacagccaacagctggaggtagcccacgccgagcggctccaggatggacgccatgaacaccacggcggcggagattggcgaggccacaatggccatctggctggctacgacggccaccgacagcggccgcgacgggcggaccttgccctccttcgccacttccacgatcaccggcagcgtggagaacgcggtgtggccggtgccagcaagcacggtcatcagccaggtcacgatcggcgcgtacagggtaatccgcttcgggttgcggcgcaggaagcgctcagccaggtggacgaggtagtccatgccgccggcgagctgcatcgcgctaatcgccgcgatgacgcacatgatgatgccgatgacgtcgaagggaatggcgtcggcagtaacggggacgccggtggcgccaaggagaaggactccgaggccgccggcgaagccgatagccacggagcccatgcgggcgcccaaaacgatggcgcccaaaaggatcgcgagacggatgaggaacagcatgcactgatcatgtcacgccgcttgcccgcccaaagttagcaaatagtgtgatctacaactagcgctcgtcctcgtcgatgtacagcgcgccgcggtactcggggtgcatgaggttttccttgctcaacaccttcttcagctcgtcttcggtcatgagctccttttccagcaccaagtcgtagacgctcctgcccgtcgctgccgcctcgcgaccaatgaggtccccggcgtggtggccgatgaccgggttcaggtaggtcacgatgccgatggagttggtgacgtacgcctcgcacgcctccttgttggcggtgatgccttccacgcacttctcgcgcagggtccgcgccgcgttggcgagaaggttaatcgactcgaagagcgactgggcgattaccggctccatcacgttgagctgcagctggccggcctcggcggccatagaaaccgtgacgtcgttgccgaacaccttgaagcagacttggttgaccacctccgggataaccgggttgaccttagccggcatgattgacgagcccgcttggcgctcgggcaggttgatctcgttcaggccagcgcgcgggccggaggacaagagacgaaggtcgttgcagatcttcgacagcttcattgccgcgcgcttgagcgccgagtgcatcatgacgtacgcgccggtgtcgctggtggcctcgatgaggtcgggcgatgcctggatgttcagcccggtgacctcacgcaacgcggtgaccgcctggtcgcggtacccgctcggcgtgttgatgccggtaccgatcgcggtcgcgcccaggttcacctcgagcagggactcggcggcggcgctgatcgtcttctgctcctccgccaggttcgagccgaacgcggagaactcctggccgagtgtcatcggcaccgcgtcttggagctgggtgcggcccatcttgatgatgtcgctgaactcgtcgcctttcgcgcgcagcgatttctgcagcccgtcgagctcgaccagcaggcggtcgatggcgtagtagaggcccaagcggaacccggtcgggtacgcgtcgttggtggactggctcatgttgacgtcgtcgttcgggttgatgacgtcatacgagcccttctccttgcccagtatctcgagcgcaacgttggccacaacctcgttggtgttcatgttcaccgaggtgccggcgccgccctggaacacgtcggagggccactgatccatgcagtagccctcatccagaatcttgtcgcacgcagcgatgatcgcctcggccttgtccttcggcagggtgtggaggcggcggttggcgatcgcggttgccttcttcacctgcaccatgccgcggatgaactctgggaattcgttgatcgtggtgcccgagatctggaaattgtctacggctcgcagggtgtggacgccgtagtagctttccgacggcaccgcgagcgtgccaagcaggtcttcttcagtgcgtgtagtcatagagcccattgtacgggccccatgacaggccaggttaggccaggttacagccgtgcgatgcgcagctgtgtggccaaaatgccctcggcgccgatgctggcgaggtcgtccatcacccggttggcgtcggccttcggcaccatagcgcgggcagcgacccagccctcgcgctgcagcggagagaccgtcggcgcggaaacgcccggggtcaccgcgaccgcgtcatcgaggttggcccgcgcgatgttgtagtcgaccatgtagtagttgtgcgccgtcaggatgccggtgatgcggctgaggacgcgctggtggtcgtcgttaagcgtcacgcccccgcgcttgaccaccacggccgcactcgccatgatcggctcaccaaacggggcaagcccctgctggcgcagcgtggcgccggtggacaccacgtccgcgatcacatccgcaacacccagcttgatggcgatctccaccgccccatcgaggcggatcaccgacttgggctggatgccgcgatcagcgaggtagtcctgcaccaggtgcgggtaggaggtggcgatatttttgccctcaagctgctcgatcgtccagctctcgttctgcggcgcggcgaaacggaaggtcgacgaggcaaagcccaagtcgagcacctcctcgacgtccgcgcgtgagtcagcggcgaggtcgcgccccgtgataccaaggtccaagtggccctgggcgacgtagatagcgatgtccttcgggcgcaggaagaagaactcaacgtcgttctcctcgtcgagcacgttgagcgccttggacactccgcggcctttgtagccggcctctttcagcacggtcatggcgtgctcggacagcgcgcctttgttcggaacagcgatcttgatcatggtgctaaagatacttgtagatgtcgtcggtggtcagtccgcgcttgatcatcatgacctgcgtccagtacaaaagctggctgatctcctccgccagctccgcgtcggactggtactcggcggcgatccacacctcgccggcctcctcgatgaccttcttgccgatgaaatgctcacccttgtccagcgcctcaacggtgctggatccggcgggtcgctcggcggctttctgggtgagttcagcaaacaggtcgtcgaagtttttcacggtggttaatgctagcccacagcatccgcgtaccacccgacaacatccgcggcaatcgccccttcgaagtttgccgggttgaagcggtgcacgcatgcgggcacgtcctccgccaagcccagcaccacgcagccagcgtccacggccgcggtcatcccagcccaggagtcctcgaagacaaggcactcctcaggttctgcgctcgctcgcctggccgcttccaagtacatgtcgggggcgggtttcgggttcgcaacctcgtcgccggtgatcgagtcggtgaagaagtgccggcccatggcgtcaatgcacctgtcggccagcacgcgctcggtgttggtggtcacgtacatcggcgtgcccgccgccgccagcgactccagtacgccgcccacacccgggttgaggtcgatgccgccctcaaaaagctgcgccatgcgattgaacatgaaggtgcggtagtggttgacgttgacgtcgacaagcgaaagccctgcgtactccgcaaggatccgcagggtgttgtcgaagctgccgccaacggtaagctcccgcacctccggcgtgatgcggcggccgagctcctccgagagcgcgtaggtggcctcgccccacagcggctcggtgtcgatcagcgtgccgtccatgtcccagaagatggcggccggggtgctactcaaaatcgggcagctccgcaagcgcctcgtcggtcgcacccgtggctgcgcacgcgcggaagacgaaggattcgatgtcggccttctcctccggctcgagcacggcgaaagcgtacttcgtgttgaactcgtccaagttggcgtagaacggggtcaccacggcgaccagctggtcgccttccggatcgtcgccgatgacgtcgagcgcgtcgaggaacatctccatgatgtgcttgagctcgggcagcacgttcgcgtcgaacggctcgtcccagagctccttgtcatcgtcgttaaggtaagcacccgaggcaaaggtgtgcaggtcgtcgatgaattcgtcgacgtcaggctggaactggctgcggatcgaggtcatggccttcatcttcgtcgattcgctctaaatccgcacgccaagcaggccgtcgatcgcggctgcgaggatgccgtcgtgatccccctgagccttatcgatcacctcgagcgcggcaggcgtgtccaggtcgttggccagggcttttcgcagcttatcgacgccctcctccacgtcctcccgcgccacctcgcgctgcaagcgctcacgccaagaggccagacgctcctgcgcggcattgagggcctcatacgagaagtcgcggtcggcgcggtagtgtccaccgaatactgcaaggcggatcgcggacgggtcgtagccctcgccactcagcttgtgcacaaagaccaggttgccgagcgacttcgacatcttcacaccgtcgagcgcgatcatgccggtgtggacgtagtggcctgccatgcgcgcgacgttgttggcggcctcagcgtgcgccgcggagaactcgtggtgcggaaaggcgaggtcgttaccgccgccttggatggcaaagtgctcgcccaagcggttcgtcgcaatcgcggagcactccacgtgccagccggggcggcctgggccgaacggggattcccacgccggctccccctcgcggtggccacgccacaacagcgcgtccagcgggtcgcgcttgccttcgcggtcggggtcgccgccgcgctccgcgaagtacgaaagcatcgtctcgcggtccaggttggactcgtagccgaactgctcggtggcggtaatcggcgcgtagatgtcaccgtggtcgagctcgtaggcggcgccggaatcgaggagtttttgcaccatcaccacgatctcatcaacggcctccatcgcgcccacgtaatcctgtggcgggaggacggaaaggacctccatgtccgagcggaagaggtcgatctggctggtgcccagctcgcgccagtccaccccgtcgcgctcggcgcgctcgaacagcgggtcgtccacgtccgtgatgttctggacgtagtgcacgtcgtggccgttggccagcagctgccggtacaccaggtcgaaggtgaggtaggtcgccgcgtggccgaggtgcgtggaatcgtacggcgtaatgccgcagacgtacatccccacccgctcaccggaggtgtcgaccggtttgaccacctggtccgcggtgtcgaacaggtgcagcggaacaggtgttccggcaacggacgggacttcgggcacgggccaggattgcatggcggcaagcctacaggctgttcttaatagggctgcatcacgccagttgcgagaagcagcatcacgataagccccagcgggatgcggtaggcggcgaaccacgcgaacgagtggttggagacgaacttcaaaagccaggcgattgagatgtagcccagcacgaacgcgacgccggagccgacgagcagctgcatgccggaggccgcttgccctgcctgcgggtcaaaggcgtcgggtagtgagaacaggccggaggcgagcaccgcggggatggcgagcaggaaggaaaagcgcgtcgccacctctcggtcgaggtcacggaacaggccgcccgagatggtgccgccggagcgagagacacccgggatcagcgcgaggcactgccacaagcccatagccaccgcgtccttcatcgtcagctcgtcgaacccgcgggtcttcttccccacccgctcggcgaggatgaacacgaaggaaaacaggatgagcaccgtggcggtgatccagaggttgcggaagttctcgcggatgagatctttcagcagcacgcccgcgaggcccaccgggatagtgccgacgatgaccatccaccccatgcggtagtcgcgcccccgcttttccgggttggccaaaccggtgaaccagccggtgaggatctgccaaatgtctttggcaaagaaaaccagcacggcgagctcggtgccgagctggatcaccgcggtgaaactcgcgccggcgtcctcgccccagaacagctccgagacgatgcgcaggtggccggatgaggacactgggaggaactcggtcaggccctgcacgatggacaggacgacgacttggagccacgtcatggtttcagtcacggcatgcaacactactctgggggctgtgaagaactcgcgcacacgcaacgccgcagcaatcctcggatcactgatggtgctttccgccgccgcgtgcggcaaacccaccgatatcgtcgacgagctcgccgtggacatgggtaacgccaccccggtcgagtcccctgccgcagcgaacccggacgggcgcgtcatcgattttgagccggtgcgcgacttagacaccaccgagggcctcgttggcgtgcgcaccggcgatgcgctgacgatcggctctccggcagagctgggaagcggtgaagccacccgctacgagctttcccccgagtgcggggatgcgtccgccaacgccggcacgttttcggttgcgtgcggaaacgtcgttcgactcttcagtgcgggcggcgaagatagcgtgcaggtggaagtgccggtgacggcggcgacggtggcgacctctggtgaggtgctcgtcggcagcgacaccgagcgcaccgtgtgggtgtaccgggacggcgaaatggtgaagaagatcccggtggcgcgcgagaccgaccagattcaggcagtcgcggttgagggccagccagacactgtggtgcgcaccagccgcttcgacaccacaatccaggaccttgactgggctggagggcgacagggcggcactctccgcgtcgggctcggcgtgggcaagatcgccgctggcgaggacgggcttgtgctcgccgccgacgccaccggttcgcagctgttggtctacacctccgacgacatcatccgcctgcaccagatggcgccggtggccgaaggcccgtgggacgtgacctgggaccgcacgcaccgccttgcgtgggtgtcgtcgaccgcgggcaacgttgctgccgggtacgacatctcccgcggcgtgccgcgcgagttggtcaaggtggagacggttgctgatccgcaaagcattgtttcgcttgacgacggcagcctcatcatcgcctccgccacaggcggaggactgcaatttgttgacgccgcggacatcgtggcaaagagtaaggagtgagcacggtgacgttgtacgacaaggctttgaaggtgatgttccggatccccccggaacagatccacggcatcatgtccgtggccttgggcctgttgaacgtggccaaaccgttaaaccgcgcaatggaaaaggtggtgcgtgtccacgatccggtgctcgagcaggagctgttcggcgtccacttccccgcgccgctggggcttgcggcgggcttcgataagaacgccaccgcggttgacgcgtggggcgcgatcggcttcggttacgccgaattaggcaccgtgactccgaagccgcaacccggcaaccctgccccgcgcctgtaccgcctgcccgcggacaaggcgattttgaaccgcatgggcttcaacaacgacggagcgctcaccgtcgcggagaaccttaagggccgtcgctcaagcgacgtggtgggcatcaacattggcaagaacaagacccagaccgacgcggtggcagattaccgcgctggcgccacgctgctcggcccgctggcggattacgtcgtggtgaacgtttcctcccccaacaccccgggtcttcgcgatctgcaggccgctgacgaactgcgcccgatcttgggcgcggtcaaggacgccaccgacacccccgtgctggtgaagatcgcgcccgacctgtcgaacgaggacattgacgcggtcgccgaccttgccgtggagctggggcttgacggcatcgtcgccacgaataccaccatctcacgcgatcacctcaccacccctgccgacgaagtggccgcgatgggcgcaggcggcatctccggagcgccgcttaatgaccgagctcttgaggtgctcgagcgcctccacggccgcgtcggcggcaagctcgtcctcgtcagctccggcggcatcatgaacgccgagcaggcgtgggagcgcatcgctgcgggcgccaacctgctgcagggctacaccccgttcatctacggcggcccgggttggatctacaacgtgcacaagggccttgcgcagcaggtgaagtgccacggcttgaacaatatcgccgacgctgtcggcagcgggctcacctggaaaaacgcctaaggatcagcgcgcacaacagcgcgccgactccccagagcacgagccacatcgtcggtgccacagtgagcactgtgttcggcaggagcatgccgattgccaatagcgcgacagcgctgcccagcgcgattagctgcgatcgcgagccgggctgcgacgtgttcgatgtggcgaacgcgccgaagataaccgaggctgcgacgatcgcgacgaagcgcgaggtgatgtcgaacaccgcctcgccgcgcatgaccgcgagaaacgcgaagatgaacaacaccacggcggtggcgatgaacgccccgccgacgcgaagttgaatcggtgccattcgctagaacttactcgttctcgaaccatccccaggtgatggcgcggccgagcgtgtggaagtacaggttgaacccgagctgggtggggttcgcgatctcttccggatcgaactcggtgtccacggcgtggacggcgtacaggtagcggtgcgggccgtggccggccggagggttcgcgccgtagtacccctttacccccgagtcccccgcgagcaccacggcaccgacgccgtggccgtcttccgacccagcgccagccggcaactcggtcacgtctgccgggatgttgaacgccgaccagtgccagaaaccggaggccgtcggcgcgtccgggtcgaagcacgtcacagcaatggtcttggtgccctccgggacaccggaccacgtgagttgggggctcaccgcgctgtcgccggtgagtttctccggcaatttctcgccgtcggcgatgtcgtcggagctcagctcgaacgccgggacgtccttcaggggcgcgtacgggtcgggtccagggaaacggtctgaaacgtaagaagcagtcatggcttcactctacctggagcacgcatcactcattctgaactggggatttggtactcccacacggccgccctatagttatgcgagtgcccggccgaaaggccgaacaaacacccaaagcccgggtggcggaatggcagacgcgctagcttgaggtgctagtgtcctattaacggacgtgggggttcaagtcccccctcgggcacaatgtgaccggcgttgtacgtgatttggacgtagaacgccggtttcgtctgtggtgaggaaggtgcggcaagatgcagcggttgggcgtccgccgaatcgtgttgctcgtgtgcctagccgccgcgttcatcgccgcttgggtgctgctcgaggtgcctccgctggcggtgatgcggcaatgggcggaggccgccggcgcctggttcccggtgctgttttggctgttgtacgtggtggtcacccagttcccgctcccccgcaccatcatgacggtctccgccggcattctgttcggcacggtcgccggtatcgccatcgccatcaccgccacgaccgtttccgcggtgatctcccttgtcctggtccggtttctgttccgcgacttcgtcgcaccgcagcttacccaccccgcggttgagactgttaaccagcgcctcgagcgacgcggctgggctgccgttgcgagcctgcgcatggtggcgtttatccccttttccgtgatgaactacgccgccgcgctgacccgcgtgccggtgctccccttcgcggctgccaccttcgttggctccttgcccggcacggttatcacggtgctgttcggtgacaccctcaccggtgaggccaaccctgcggtagttgtgctgacagtggtgctcacgctggtagggctttcgggcttgcttatcgacgcccgcgtgcccctcgacggctacactcaatcgacatgattggcgtgcacgcaaggtaccgaggacgcgacaagcggcgggccgaggtcgtcgcacgctccgcggaggcgctcgccacgcttccgggcgtgtcccccttcgaggtggtgggtgtagaagacatccgcgccgacgtggacacccccgagcacgcgctcaatctcgtgatggcgctgctgtcggacggcgactgggccatcgggttgggcattacgtcccacggccgcggcgtgcacgccgcgagtgatgcggtaggaacccgccccgcgcaagtgaaggtgaacgtggacacccgccacccgggtaccgcagccgacgacattgctgcggcgttcgcgcttgtgggacacgtgctgcacaagcgcaccttcgaggggcgcgaagcgacggcgctcgtgcgcagcggcatgaaccagaacgaggcggcgcaggcgctcggcatctcgaagcaggcgatgagccagcgcctgcaggccgctggctggcaggcggagcaggccgggtggcagctcgcgctgaacttgattactcgggctgaggcagatcgagccgacggctgacctgctcgatttcctttaccggcgccggctccggcgccggggtctgggtcgggtctggcgcgtcgacgtgcttgttggcaaccgcccgcgcctcggcgagcgcctttgctagctccgggtcagtggaggtgtcgaaccactcctcagggttttcctcgccggccatctcgcgggtttgctcgtccacgcgctcagcttcgtagcggaacaccccgtcctggtcttgtttggcaaaagccttggcgaactgctccagcgagttgccgaactgggacggaataagccacatcgtcgccgcctcgttgccggcgatcttcggcagctggtcgagatactggtaggcgagcagctccggagtgacgccggaggacttaattgcggcgttgaccttctggatcgccttcgcctcgccctgcgcctccaagtacttcgcggcgcgctcaccctcggcgcgcaggatcatggcctgacgctccgcctccgcgttgaggatcgcggcgtgcttctcgccctccgcggacaggattcgggcctgcttctcaccttctgcggtcttaatgtctgactcgcgcttaccctctgccgtgagaatcatggcgcgcttctcacgatccgccttcatctgcatctccatggactgctggatggacggtggcggatcaatggccttcagctcgactcggctaatgcgcaggccccacttggcagtggcggcgtccagctctccgcgcaggcggcggttgatggtttcacgggaggtcagcgtctcctccagcgtcatgccgccgaccacgtcgcgcagcgtggccaccgagatctgctccacgccgaccaagtagttgtccacgccgtagatggccttggctgggtcgttgatctggaacgtcaccaccgtgtcaatcgccacggtgaggttgtcctgggtgatcacagcctgcggcgggaaggacaccacccgctcgcgggtgtccacgcgggcgcgcacgcggtcgatgtagggcacgagaagcgtcagcccgcctgagacggtgcgcgtgtagcggccgagccgctcaatgacggcggcttcgccctgcgggatcagcttcacggaagcgaacagcagagagacgacaaggataaggacgacgaccaatatgattgcgggacccatcgattacttctccttccacacgacggcgacggggccgtcaatcgcagatacggtaacacgttcgccggacgctagggtttcgcctggatcgaggcagcgggcggaccacaacgacccgtcgataagcacctgccccctgctgcctgacacctcttcaaccacctgggctggcgagccgaccagcgcacgcggcgactcgtcgtagaccggcggggtgtcgaggcggcggcgcaggtacgggcgcaggaagaaccagaaaccggcggaggtgacagcgaagacgacgacctccgctgtcaacgagatgccggcgagcgcagccgccgccgtggtgagcgcacctgcggcgagcatgagcagcgtcagctcgccaacggcaagctcgagcgcggcgagtaaacctgcggccgcgaaccacaccaaagcacccatgcccaaaacgttacacggtgctactacatctccaggtcgctcttcgaaagttccggagtggtgacgaaatcgactagccgctccaccgcgccgatgagcgtggaatccaggtcgcggaaggtggcaaccgagctgtagacccggtgccacccctccttcgggtccgaccacccaaggcgccggcacacgcccgttttccagtcctcgccgcgcggcacctccggccaagcccggatgcccacgctcgctggcttcaccgcagcccaaatgtcgatgtacgggtggccggtgacaaggacgtgctccccgacatcggcgacgaggcgcgcctcttttgttccctcaatcaggtggtccgccagcaccccgatgcgggcatcggggccggggccgaactccgcaagccgggcggggaggttgtccaagccctcgaggtactcgacgacaacgccctcaacccgcaggtcgtggccccacaccttctccacaatcgcggcgtcgtggatgccctccacccagatccgggacgggagcgccaccttcgccttgacgttctcgactttccgcgagccggagttagaccgtttcggcccctcctccttcggcggcaaccacctcgtcagcgtgacgcggttgccttccaaaaggaacgcgccgggcagcatcttgaacagcctttgcacgccgcgccggtcctctaaccgcacgaaatcgccgtcgtaggtccgctcaaatccgacgactgcgccgacgaactcgtcgccgacaatctcgaccacaatccccggctccgcagggacctgcgggtaggtgggtctgcggttgcgctcgtggccgtgaaaaatgtccatatcggcgatcaagtctatccgctacaatcgcgcgaatgcagacgcgcgccgaagtgtattctccgctccagaacaccgctgtgtggctggccgcatggctctataacgtggagtcgacagacgacacggtgcaggcgatcaccgacctcggcggccggcacagctaccaggatttcggcgtcgagccgctgctcgcccggctgcgggccaccgcggcgcttgattcccccgggcccgtgatccgcctgctgctgtgggggccgggtcaggctgccggcttgcgccccggcagccctgcctacgaggcgctgacccccgcgggtgcggtagccgtgctcgacaggggcgggttggcgcacgtgctcgtgcccgagtactcgccccgcggcgtgtcgtggcgctggttcgaggagagcgagcggctgccggaacccgaatggctttccccgggcgaagccgacgcgctgttgtcccgggcgacgaacgaggctgccgatctgatcgaggccgccggcggctcgcggaaggaccttccgaacccgcggcttgccgtggggtcattggccgacttctacgacaccccgggacttcccgccggcgtcaccccgcgcgccgcgaaactgttcgccagggccgaccgggtggcggcgactattgaaacggtgactgaccgcctcgaggaccacactttcgacccccagctgttcgctctgtggcgccacatccgcactgcgcgcatggcgggcgtggcggaagcggtcatggactacgcccgcgagtacgcggcgagctagcggcgcaggttagccgcgggcggggcggcgcaccggctcgcagcagtgcgggctgcacggcgagccgttaacggtgcacccctgcaccgtcacggtcgaaagcgtctggggctcggtgccctgggcgacgcattcggcgatgtccacgatcatctgagcgaacgccggttcaagcccgactgtgtcgacgcgttccagcgcaacgccccgcgcctcgcacgcctggcgaagttcggtgtcgagatcccaaaccacctccatgtggtcggtgatgaacccgataggtacgcaaaccaaggtgtcgaagtgctcctggttgtcaagctcttcaaggcggtcgaccacatccggctcgagccacggcgtggctgggttacccgagcgcgactgccacaccacttcgtaggtgccaacgcccgcggcctctgcgaccaaccgcgacgcttctgcgacttggcgggagtacaggtgctcgtcgccgggcccgccagccgcggtgtcggcggcagtggggacagagtgcgctgtgaacagcacacgcgcggagccttcctgcttatcgacggcccctttcaccttcccagccatcaactcaataaaagttgggtgtccgtagaactgccagagcttggtgtagtcgatctgcggggtgacctcgcgcagacgctgaatgtcctcgtcgtactgccggcacgccgaatagccgccccacgcgctggtggcgaggaccagcacgtttgtccggccgtcgtcctcaagctgcttcgcggtgtcttcggcaaacgggtgccagttgcggtttccgaagtagacgggcaggtcgtgaccgcggccggcgagctctgcctcgatgttgcggatcaactcgcggttctgcccgttgatcgggctgacaccgccgaagtggaagtagtgctcgcccacctgcgccagacgctcgcggggaatgccccgcccgcgggtcacattctcaagaaacgggataacctcgtcttctccctcggggccgccgaaagaaaggacgaggagtgcgtcataaccagaaagcgccataaatggtcattctaaagcagccggactgccttaggagacatattcgcccaacgcacaggcaccacggaaacattctggccggactgcggcgcctcgatcatcatgccgtcgccgaggtagatcgccacgtgctgggagccgccgggaccccagaacaagaggtcgccgcgctgcgctgaggaggggtcgatctgcgtgccccgctggtactggtagccggtgtagtgcggcagcgaaacgcccgcgcccgcgtacgcgtagagcacaagtcccgagcagtcgaaacccttcaccgagccgccgttaaggccagtggtcgggccgttcgcgtctccgccgccccacacgtacggggtgccgaccatggacatggcgcgggcaatcgcggtctcgacaccggaagagttcgccggtgcgacagtttcacggatggtctcagtcactgtctccggcgtgaccaccttcggcagcgcgctgatcaacgtctccgtcggggtctcgttggagccggcgacacctacaccggattgaaaaccgccggcgaaggcagagacgatctcggctgcggagtaaccagagacgttcgcaccggagctcaatgaaccgagcgcgggtgccgcgtacgggtcagcgaacgtggcgtgcggagcctgggagtagcccaccagcgcggaggctgcagcgatgctggaagcctgctccactgtgtcttccggcgaatcctcgcgaagggtttcggcggtggctaccgcagcagcgacatcgtcctcgctgggcgccggggcatccggcgcgagctccgccacgcgttcctgcacggcctcgatgatctcaggcgcaacctcggcctcctcgggacgcgtctcatccgcgtccgtctcatcggcctgccccttgtccgcctgcgcctcgtccgcgttatcggcctctggcctcacctctgcgagagaatcctgggcgtcggcgagatctgcttgcgctgcctccaactcggcagcccgggcctccagtgctgcagtggtctcctccagcagttgctgcgcctcggactgtgagacttcggcatccccggccgcggcgtcggccagctgcgccgcctcgcgggccagcgaggcctcgttcgcagcctggatacgagcctgctccacggcctcgagagcggactgcttctccgcggtgcgttggcgcaggaaccgggcccgctcgagcgcgtccttctggccgttctttcccccgaggtgctgcagcggagcggattgacccgcggaacggtattgcgacctcgtgatctcgtcgagatcagcacgggcccgcttgacttccgcctcggcttccgcgagccgctgctccgcagtctcaacaccgcgccgggcctgctcagcccgcgcctgcttatcgcgcaagtcaaccagtgcgcggttcacgctttcctggatagcgccaatgtcgagcgcagcctcgtcgacgcccgcctgggcgcgagacacggcagctaccaggtcggcagtggactgcgtcgactcctgggctgcggcgaacggcgacagcgacaaggtaacggcactagcgaccgttgccgcgatggtccgcgggtgggcggggcgaaaacgccgcacggatgtgaccacgagggtgctcctcacagcgcacgccaaagcaggcgtgcccaactgcgtccgcgacgcccgcgcgtgactagcgcaccggcaacgggacagggcttgcgccttgacgtgcgtcttcaaagttgactactgatgcgcggatcgtgaatcggcggcaagcgcaacggcgcgagagtttttcagtacttggcgtgcttccccacatgcccgaactgcgtaggcggcacgcttgactagagcgtgctgccgatgaaactcaagtgccttgcatagacttgcgccgacccacgagccgacatacgcaccttacgtcacgaaatcatctcgattcgctttcaatctcttcagtcacagcagtcaaggcagttccactgacggttcctggggctgacctgctggttccattgttagaaagaagcggtgtgacaatcgtcacaccgcagtggtgctggagcagctgtttgaaacgtcagccctagtggcttgaccttctggtcgcggcgactgtcgcagcgataatgagcgcgactgcgaccgtcaccgcgacagcaaacgcgccccagggaacgctgaacgcgctcgacgccgcgtagaaatcggccaaaccggcaactggatcctgctgtgcggccatcgcgcgctgaccttcctcaacctctgcgcgcgaaagggtgtcgctcaccccgatcgcaacgtggggggtgcgcacaatcacggtgtcgagcccggtctcgttggccaagtcttgcgcgagatcgcgcagttgcggcacgtgctccggggtgtggtcgagcaggacgatcccggtagcgctatcaagcacctgccccatcgcctcgcggacctgtgccgacccttcctcctcacggccgaaagcggccccagaggcgcggagctggtcggcgagtgttgcgaagttggcgtagatatcggtcatggcgaagacacactctaatcggaatccaaaaacattacgggcgtactgttagtatggcagtggaactgtggcgcctggcttagaattgacggttgaccgccacgggtcgcacaacccataaacgatgagaattggagctcataatggctgaaagcaagaactccttcaacgccaagaagacgctcgaggtcggcgataagtcgtacgactactacgcgctcgacgcagtcgaaggcatggagaagcttccgtactcgctgaaggttctgggcgagaacctccttcgcaccgaggatggcaagaacgtcaccgctgaccacatcaacgcgatcgcgaactgggatccgtcggcagagccttcgatcgagatccagttcaccccggctcgcgtgctgatgcaggacttcaccggtgtgccgtgtgttgtcgacctggccaccatgcgcgaggccgtgtcctctctcggcggcaacccggatcaggtgaacccgctcaacccggccgagatggtgatcgaccactccgtgatcatcgaggcgttcggctccaaggacgccgaggcgaagaacgtcgagatcgagtaccagcgcaacgaggagcgctaccagttcctgcgctggggcgccgagaacttctccaacttccgcgttgttcctccgggcaccggcatcgtccaccaggtcaacatcgagtacctctcccgcgtggtcttcgacaacgagggcgtcgcctacccggacacctgcatcggcaccgactcccacaccacgatggaaaacggcctgggcatcctcggctggggcgtcggcggcatcgaggccgaggccgccatgctcggccagccggtgtccatgctcatcccgcgcgtcgtcggttttaagctcaccggcgagatcccggccggcgtgaccgcaaccgacgtggtgctgaccatcaccgaaatgctgcgcgagcacggcgtggtgcagaagttcgtcgagttctacggcaacggcgtcaagcagatcccgctggccaaccgcgcaacgatcggcaacatgagcccggagttcggctccacctgcgccatcttcccgatcgacgaggagaccatcaactacctccacctgaccggccgttcccaggaggacatcgaccgcgtcgaggcgtacgcaaaagctcagggcatgtggctcgagcaggacgcagccgaggcggagtactccgagtacctcgagctcgacctgtccactgtggtgccgtccatcgccggcccgaagcgcccgcaggaccgcatcctgttgtccgaggcgaaggacaccttccgcacgcagcttccggactacaacaccgcaggcgagggcaccgctgagccggtccgcgcgacgaaggtcgacaccgtctcctacaacgagtcgtggccgggcaacggcgagtccgcggcggctggcgcagagggccgcgcgtccaagccggtgatcgtggagtccccgcagggcggcgagtacacgatcgaccacggcatggtggcgatcgccgcgatcacctcctgcaccaacacctccaacccgtcggtcatggtgggcgctgcgctgctcgcgcgcaaggccgctgagaagggcctgaagtccaagccgtgggtcaagaccatcatggctccgggctcccaggtcgtcgacggctactacgagcgcgccgacctgtggaaggacctcgaggccgtcggcttctacctcaccggcttcggctgcgcctcctgcatcggtaactccggcccgctgccgagcgagatctctgaggcgatcaacgagtacgacctcaccgcgaccgcagtgctgtccggtaaccgcaacttcgagggccgcatctcccccgacgtgaagatgaactacctcgcgtccccgctgctggttatcgcctacgcaatcgccggcaccatggacttcgacttcgagacccagccgctgggccaggaccaggacggcaacgacgtgttcctgaaggacgtgtggccgtccaccgaggagatcgagtccaccatcgcgtccaccatctcccgcgagatgtacgaggcggactacgccgacgtgttcaagggcgacgagcagtggcagggcctcgacatcccgcagggcaagaccttcgactggagcgaggactccacctacatccgcaaggctccgtacttcgacggcatgccggaggagccggaggcagtgtccgacatcgagggcgctcgcgtgctggcgaagctgggcgactcggtgaccaccgaccacatctcccccgcttcctccattaagccgggcaccccggctgctgactacctcgacgccaacggtgttgcgcgccaggactacaactccttcggctcccgccgcggtaaccacgaggtcatggtccgaggcactttcgcaaacatccgcctgcgcaacgagctggtggacgagcagggcggctacacccgcgacttcacccaggaaggtgcgccgcaggcgttcatctacgacgctgcgatgaactacgagaaggccggcatcccgctggtcgtcctcgcgggcaaggagtacggcaccggctcctcgcgcgactgggccgcgaagggcaccaacctgcttggtgttcgcgccgtcatcgccgagtccttcgagcgcatccaccgctccaacctgatcggtatgggcgttctaccgctgcagttcccggagggtgagtcccacgcctccctgggcctggacggcacggagaccttcgcaatctccggcatcaccgccttcaacgagggcgacgaaatcccgcgcaccgtccacgtcaccgcgacgaagaacggcggcgaggctgtcgagttcgacgctgtggttcgcgtcgacacgccgggtgaggctgagtactaccgcaacggcggcattctccagtacgtcctgcgccagatggtgaagagctagtaccaaacccctatttagggccactcggtgggtattcaccgggtggccttttaggtgccgtcgacaagcaagaaagcccttttacatatgccgattgtcagcgaatccgagcttgcccgcaggcggcaggagattatcgacgccgcgcgcgtctgcttcgcccgctacgggtttgagggagcgaccgtggcgaggctggagcaggcaaccggcaaaacgcggggggcaatcttccaccacttcggtgataaagaatcgctgttcctcgcgattgtcagcgaggacgcggagcgccaggccgaggtggtgtcgcagcgcggccttgttgaggtgatgcgcgagatgctgcgccaccccgacgagcacgactggtacgtgaccaggagtgagattgtgcggaagctgcgcaccgaccccgattttgaggggcgctggcgcgagcaccaagaggtgcttgaccgcgcggtgcgtcagcgtctggagtcgaacgatcaggtgcgccacgacgtcgacctgagtgtggtgcagacctacctcgagaccgtgctggaagggttcatcgtgaggctggcagccggcgagccggcggagcagctggaagcgatgctggacgtcgtggagcagtctgtgcgcggctgaaagctgggaggcttatcgacggccccaattccgagaaagtagaccaagcggtatagaatgttccgcatggctcagctgctctttctctccctccgcgacggcgacatcggtcccgacgtggcgcgcgcggagtaccgcgacgcgcttcacgcctccggcctggcggaggtggagatggagcaccgcgtgctcgacacaccctcggcagcgattggttctctggaaaacgtcagcggcgtgatcgtgggcgggagctccctgaacgtgaccaacgctgaggcggggcgcggctacagcgcttaccagcagcacattcactcccagctcgcgcagctggtcgagactggggtcccagtgtttttcgtgtgcttcgggctgtcgtggctcgtgcacaacgccggcggcgagatcaggcacagccacgctgaagattccggccccacgaccgtgaacgtgacggcagccgggcgcgaggacgtgctgctcgcggcggcgccagcgacatttacggcgctgaccggccacacggagaacccggagactgcgggtggcctgcccgactcgttgacggtcctagccaccggccccggcgggatggtgcagatcgtgcgctatcgcgacaacgtgtgggcgacgcagttccacgccgagatggacgccgacgcgatgcgcacccggatggacttctaccacgactacggctacttcgctgcggaggattacgcccgcatcgtggccgatctgcccaaccacgacgtcgccgcggcgaacgggctgctgcgcagtttcgttggttactgcgcgtcctcgagcgcgctggctggctgctcgccgtcctcaaactcgtaggggttctccgggaacggctccccgcggtttacggctgcggcgatgacttcggccacgagctcgcgcgaggttttcgaaccttcgggcatatctccgttgatgtgggcgagaccgttggagggtgcgtcggtaagcgccgtgggccccaggatctggttcgggaactccgcctggagcaggcgcttgtcgacggccttcttactctccacatacgcgtaccacgacccgccgtcgtcgtccgtgctggcgtgagcagcgccggcgtaggagacgttgacaaggaacggggcgtactcccccagctcctcgagcgcgtcgatcattgtcagggcagcgtcgcggtccaccgcgtaggtcttctccgcgctgccgccgccggcgccggcggaccacaccaccgtgtcgaacggagtgagcaagcgcgcccacccctcctggtcgagctgcgtgaggtcctgaacgatcacggcggcacccgcctccgaaaggcgcggggcgtggtctgggttgtgcaccagcgcggcgaccttgtggcccgcctcaacaagcatcggcacggtgtggcgcgaaacgttgccgccagctcccaggacgagaacataggaggcagtcggggcgtcgttttctggatgtgtcatgggccccaccgtacgtcaatgggtactatttttgcccatgtacgcaatcatcaccacaaccggcaaggaccgcgtcggcatcatcgcagccgtcgcgaacgcggccgcagagcgcaacctgaacatcgtcgacgtatcccagacgctgatggacaacttcttcaccatgatcatgcgcgtggagctgccgaccgcgggcggcgagccggtcgacatgggcgatctgcaggcgcacctcgccgccaccgggcagcagctcggggtggacgtgcgcatccaggcggaggacctgttcaccgccatgaacgagatctagggcgcggggtattcacgaactatggcgactgatttcgacttcaaggctggccgcatcctcgacgtcatccgcatgatcgaggattaccggctggacatccgcacggtgaccatgggcatctcgctcatcgggtgcacccgcgcaacgatggaggcgaccgcagacgcggtgtacgaccgcgttatggaacgcgcccgcgacctcgtgcccgtttgcgaaggcatcgagcgcgagctgggcatcccgattgtgaacaagcgcatctcggtctcccccatcgcgctggtggccgccggcgccgagggcaacccggtgctggtggcgaaggcgttggacaaggccgcggctgagctcggcgtcaacttcgtcggcggctactccgctctggtggaaaagggcgcgaccgaggctgacgcccgcctcatccgctccatccctgaggccctgtccaccaccggcaacgtgtgcggttctgtcaacgtggccacctcccgcgccggtatcaacatggacgcggttgccgagatgggccgcgtgatcaaggaggctgccgaactcaccgcgaacgagtcctccatcgcctgcgcgaagctggttgtcttcgccaacgccgtgggcgacaacccgttcatggccggtgcgttccatggcgtcgaggaaccggacacggtcatttccgtcggtgtgtctggcccgggggttgtcgacaacgctattgggtcgctggagggggcttcgcttaacgacgtcgccgaagagatcaagaaagccgccttcaaaatcacccgcgccggccagctggtgggcaacatggctgccgagcgtctcggcgtgccgttcggcatcgtggacctctcgcttgcccccaccgccgagatcggcgactccgtggcgcacattctcgagcacatgggacttgaccaggtgggtacccacggcacgacggcggcgctggcgctgctcaacgacgcagtgaaaaagggcggcatgatggcctgctcgcgcgtcggcggcctctccggctctttcatcccggtctcggaagaccagggcatgatcgacgccgtgcgcgccggctccatcacgatggacaagctcgaagcgatgacgtcgatctgctccgtgggcttcgacatgatcgcaatccccggcgacacctccgccgaactgattgcgggcatgattgcggacgaagccgccatcggtgtcatgaaccacaagaccaccgccgcccgcctcatcccagtacctggcaccaagccgggcgacgaggtcaacttcggtggcctgctcggctacgccccggtgatccccgtatcgcaggtgggcaacgacgcgttcattcgtcgcggcgggttcattcccgcgccggttcacggcttccgcaactagccttgctagcgatccccgcccaggctatcctgtacgcaatcctgtacgttttttcggctgagggagacgtgttgtgaaagtcatgtcgtacaccgagtcgcgcgctaactatgcggaagttctcacccgagtggtggaggactgcgaggaggtggttattacccgttcgggccacgagccggtcgtcgtagtctccctcgcagagtacgaagcgcttaaagaaaccgcctatctcctcgggtctcctaggaacgcccgtgtactcgaagaaagaattgcacgggtcgatcgcggatcggtcttggaacgcgcgttgctcgaggatgactagtgctcatctgctgggacccagacgcatgggaagagtattgcgattggcagacccaagatcggcgcatgcttaaacgcatcaatgcgcttataaacgatatttgtaggaacggaaacgagggcatcggcaaacccgaacgcctcatgcacaatctgactggctactggtctcggaggatcaacagcgagcatcgcttgatctacaaaatcgacgaggccggtgtcaccattatttcctgcaaataccactacggtgactagccccgtcaaagttaacgctttttgcccaccgtaaagtaggccagccagcccagtgtgttcactgcggggatagtaactccccagagccacttggggccgcggagggaacgtgcgtcggcacgcgcgagattccagagtgcggcactcttgccgacggtgtcgatgcctgcgagaatgcccacaatctttcgctgctccctggacatggcgttccagccgtcgcgaagggtgtcgagaatagtgtcgttcgaagccatgcgtctgatcgtacgcgagcgcaggcattttaagaccgtgtactagattcatgtgaatgaccgtcgatcgtcctttcctgctgctcagcactcgtcctgaggacgctgcgtctgccgaggagtacgcatccttcctctctaaaatgcgcatcccggaagaggcgctggaacaaaggcgcgtcgaatccgctccactcggggacgtcgacctggataagtactccggagtgctcctcggtggcagcccattcaacaacaccgatgaggtcaagagcgatctgcagcttcgcgtcgaacacgagattggcacgctcgtgcgagagatcatcgagtgcgacttccctctcatgggcgcctgctacggcatcggcatggtcggcggtgctatcggagcgcggcttggcagcgagtacgccgaggaagccgggatgatcgagattctccttaccgaggacggtaaacgcgacccgctgctcgacggcctacccgattccttccctgctctcgtcggccacaaagaggcgatcaccgaactaccgtctgaggcgacactgcttgtcgccggctatgcctgcccgacccaaatgttccgagtgaaagagaacgtctacgcgacccagtttcacccggagctcacagcccaggcgctcgaggcgcgtctgcgcctctacgctcacttgggctacttccgcctcgacgtgttcgacgacattctggcgaccgcatacgcgcacgattactcctggtccaaccggatcctttacaacttcgcggagcgctaccgccagttttagggccggttcggggttccgggaaaggtttgcgccgctctaaagccgctttaggtcgcccccgcagccgttatcgtctccttcgggcttgcgtttcaccgtctcaaacaacgcgttgtgtgctggcggtggcgcatcttccgaacgcgcaatgacggacatcgtgccgtccgtttcgaggatgatcgcctgcacaccgtcgaggctggcggtaccgctgatgcgcaccgcctgcaggatctcccgctgtgtcacgcgctcggcgcgcatcgtgtcggtgaggaagtcgccgccgtagtacaacagagcggggtcggctttgataagccgctcgaacttgctcgagcgaaaggcgaggcgagagatcgtccattgcgccagaaggagaaccaagatcgcggttacagactgcgcgagcttaaggtcctccgtcgtcaacgtgctagcgaagattgatccgatcgcgacagtgatgatgaagtcgaagatgttgaatttcgacaatgaccgtttgccgctgatccgcagcatggcgatcaacgtgacgtagatgatgacgcccttcaccgccgtggcggcaagggtcccccattcgctagcgagaatgcccggcatcaggctagctccacaatttccatgtattcgtcgctccacaggtcttcgtcgccctcgggcatgatgatgacgcgctcaggctcgagtgcgcgaacggcacccgggtcgtgggtcaccagcaccaccgcgcccgtgtaggtcttcagcgcgtcgagcacctgctcgcgggactgggggtcgaggttgttcgtgggctcgtcgagaagcagaacgttggcgcgggaggagacgagcgtcgctagcgcgaggcgcgtcttctcgccgcccgaaagcgtgcccgccggctgctcgagtttgtcgccggagaacatgaatgcaccgagcaggccgcgcaggtcctgctgccccgcgtccgggcaggcctcgatcgtgttctcccacaccgtcttatcgccgtcgatcgtgtcgtgctcctgggcgaagtagccgatcttgaggccgtggccggacactaggccgccctcgccgtctgtgcgctccactccggctaacagcttgagcagggtcgtcttgcctgcgccgttggtgccgaggacgaccacgcgcgagcccttgtcgatggctaggtccacgccggcaaagacttccagcgaaccgtacatcttggtgaggcctttgccgtacagcggcgtcttgccacagggagccggttcggggaaagagatggaggcgaacttgtcggcaatgcggacgtcgtcaagctcgctcatcatgcggtcagcgcgggcaagcatctgcttcgctgcggccgccttcgtcgccttcgcacccagcttcgccgcctgcttctgcagcgcggcggccttcttctccgcgttggcgcgctcgcggcgccttctcgcctcgtcttccgcgcgggccttctggtaggtagagaagcccatgttgtacacgtccgcctcagcgcggacggcgtcgaggaaccagaccttgttgcagacgtcgtccaagagctcgacgtcgtgcgaaatcatgatgaggccgccctcgtgctttgacaggaagtttcgcagccaggaaatggagtcggcgtcgaggtggttcgtgggctcgtcgagaagcagcgtcgtttcactcttgcccgagccggagcgcgatgcgaacagaatctgggcgagctccacgcggcggcgctgaccgccggagagggttctcaacttctggtcgaggactcgctcaggcaggcccaagttgtcgcagatttgcgccgcctctgcgttggcctcgtagccgccgagcgcctggtagcgctcctcaaggcgcgagtacttcgcgatcgccttgtcgcgctcagcgccctcggtggtttccatgatctgctgctgtttggccatggagcgctgaatctggtccagcccgcgcgcggagagcacgcggtcgcgggcggtttgctcgatgtctccttctttggagtcctggggcaggtagccgatctcgcctgagcgcgtcacggagccgccgtatggctcggtctcccccgccaggatgcgcatcgtggtggtcttgccggcaccgtttcggcccacaagcccgattcggtcgccgggctgaacacgcaggtgctgtcccggtgccgaaagcagggtccgggcgccgacgcggacctcgagatcattggtgacaatcacggtatcaccttacaagcgaggtcaaatggcctgttcactagcagggatcgacgtactccgcggcgttgctcaggagccggccgttgcccccgtaggtcgctttggcccggcacattgcgtcgacatcggtgccgtagtcgatgtagatcgggtacacattgtggccgtcgacctgtgcccgcagtgacgggcacgcgcccggaaccgcgaaacgaaccggctccccgctcgggtgcatcatgagcacctgctgggcgatgtcatacatcgcgccgccgtcgttgccctcatcgatgaccgagtcgagaatcaacaccgcgcgcccgtcacaagccgggtacgtcgcgacctctccggcctccccaagccccgcggacacaatgacgccgtcttgcaggtagtagttcgatccgccagtctgcgacggggtcggcgctccctctgtcaccgtctcagtcaccgtttccgtcggagacgccggcgacgatgacgtcgagatcggggtggcgaccaccgttggctcctcaattcctgacgagctgcagctagcgagcaacaccaacgaggcgagtgccgtggccgcgccgaagacgcgtaaaggcaaatgcatggctcacacgccagctacaccgcgaaaccgagggcgcggagctgctcgcgcccttcttcggtaatgaactgcgggccccacggcggcatccagacccagttgagctccagctcgtccgcggcggtgttctccagcacggagatgcgggcctgctcctcgatgacatcggtgagcgggcacgcgggcgaggtcaacgtcatgttgatcaccgcgatgttcttgccctcgcgctcctcaatccacaggtcgtacacaagacccaagtcaacgacgttgatgcccagctcagggtcgatcacgtcgcgcatgaactcctcgacatcgcccgcgagcttgagctgctcctcggtctgctccgggcgcttcgctgccatatcttcagccatgggttagtcctctctcttctctttcgcttcggcggtcgcggcctcaaaggccttccaaccgagcaaggcgcacttgacgcgggcggggaacttggccacgccggcaaatgcgacaccgtcgccgatgagctcggcatcgccttccaagttgccgcgggaggtaatcatttcctcgaacgactgcagcttcttgaacgcttccccgatcggtttgccgatcagctcctccgccatgacggaggtggacgcctgggaaatggagcagccaatggcgtcgtaggagatgtcctcaacggtctccccgtcctcagacagctggacgcgaagcgtcagctcgtcgccgcaggacgggttaacgtggtggacctcagtctcgaacggctcgcggagcccggcgtgctgcgggttcttgtagtggtccaggatgacttcctggtacatcgattccaaattcatcgtgcgaaaaactccttcgctttgctaatcgacgcagccaacacatccacttcctccaacgtgttgtagaggtagaaacttgcccgggacgtcgactgcaggtcgagcccgcggtgcgcgggccacgcgcagtggtgtccggtgcggatagccacgccctctgcatcgagcacctggccgaggtcgtgtgggtgcacgccgtcgaccgtgaacgcgatcgcgccgccgcgcttgtcggcggtgaggggtccggcgatggacaggccgtcgataagctgcatttgctccagtgcgtacgccgtgagctcgcgctcgtgcgccgcgatctcctccatcccgatctcggtgaggaaatcgacagccgcgccgagaccaaccacctgcgaggtcatctgggtcccggcctcgaatcgctgcggggccggcgcgtaggtcgaatggtccatgtggacgacctcgatcatggatccgccggtgagaaacggcggcagttcgttcaggtgcttggagtacaccacgccaacgccgctcgggccgcacatcttgtggccggagaatgcggcgaagtccacgtcaagcgcgtggaagttgacgggcatgtgcggcaccgactggcatgcgtcgagcacggtgagcgcgccgaccgccttcgcgcggcgcaccatctcctcgacgtcggcgtgcgcgccggtgacgttggactggtgcgtgaacgccacgaccttgaccgagtcgtcgagctcgagcgagtcgaggtcgatgcgcccgtccgaggtcattgtgtaccacttgagcgtggcgccggtgcggcgcgcgagctcctgccagggcaccaggttcgcgtggtgctcgagctcggtgatgacgatggtgtcgtccgaggtgacctgcaggtcgccggcgcgggagtcgcccagcacgtaggcggtgaggttcagcgcctcggtcgcgtttttcgtgaacgcgatctcgtcgccgcgcgcgcccacgaaggccgcgatcttttcgcgcgccgactcgtaggcgtcggtcgcctcctcggccagctggtacgagccgcggtgcaccggggcgttgcagccgaggacgaagtcgcgctcagcatcccagacgcgctgcggacgctgggaggtcgcgcccgagtcgaggtacaccagaggcttaccgtcgcggatggtgcgccccaggatggggaactccttgcggatggcgtgaacgtcgaaactcattagatgaacttctcgtagccctcggcctcgagctggtcagcgagctcggcgccgccggtcttcacaatctttccgtcggcgaagacgtggatgaaatccggcttaacgtagttcaggatgcgcttgtagtgggtgatcatcagtacgccaccgttggtctcgtcctggtagcggttgatgccctcggagacgatgcgcagcgcgtcgacgtcgaggccggagtcggtctcgtccatgacggcgaacttcggcttgagcagggacagctgcatgacctcgtggcgcttcttctcgccgccggagaagccttcgttgaccgagcgctcggagaaggagacgtccatctgcagcgcttcgcgcgccgagttcagctcggagacccactcgcgcagcttcggcgcttcaccgcgcacagcggtcacagccgagcgcatgaagttggaggacgacacgcccggaacctccaccgggtactgcatggctaggaagaggccggcgcgggcgcgctcgtcgatgtccatgtcgaggatgttctccccgtcgagcagcacctcgccgtcggttacctcgtacttcgggtggccggccagcgtgtaggccagcgtcgacttgccggagccgttcgggcccatgattgcgtgagtctcgccgccgttgatcgtcaggttcacgcccttgaggatcggcttggcctcctggccctcctccgtcggcaggacattcgcgtgcaggttcttgatttccagagtggacataagtcagtacttcctttagttgttgttctgctcgagctcgccggctacgcgcgcgatgagctcctcgcgcaccgattccaccgggatttggttcaagacctcattgaagaagccgcggatgatcaggcgcgtcgcctccgcctccgggatgccgcgggaacggaggtagaacagctggtcgtcgtcgaagcggccgacggtggcggcgtgacccgcgccagcgatctggccggtctcgatctccaggttcggcaccgcgtccgcgcgggcaccgtcggtaagcaccaggttgcggttcgtttcgtaggtgtcggtgcccttcgcgttcgcgcggatcagcacgtcgcccacccagcaggtgcgggcctcgggcaggccggaagaggggttgccctggagcgcgcccttgtacaggacgttggagcggcagttgggcactgagtggtccaccagcatccggttctcgatgtactgaccgtcgtcagcgaagtagacgccggtcagctccacgtcggcgcccggcgcggcgaaagtgacgcgcggagtcaggcgcacgatctcgccgccgaacgccgcgacgctgtggcgcagcacggagtcgcggttcacccggatggattgctggccgatgtggatcgcgccgcggtcccagttggtgtccaccacggcgttgacgtgggagccctcgccgatgtgccagttcacgttgtcggcgtggatgccggtgcccgcgtagcgcacgataaccgtggcctgagaattgcggcctgtctcaacgagaatgttgctgaacgtggtggcatcctcgccggcaccggtgatggtgatcacgatcggggtgtcaagcattgcctcgtccggcacggagatgacagtgccgcgctcggcggacgtccacgcctgggcggcgacgcggtcgaccggaccgccggccacccgcaggcgctcgtcgctggaatcgaggtggtcgacggtgacgttcgacggtgcgtcgacaagcacctgctcctcaacctgcgccgggaacgtgccgtcgtgcaacccgcgcagcctgcggagcgggatgaagcgccaaacctcgtcgcgcccgcctgggaccgggaagtcggcgacgtcgaacgactggaacaggtcgcccttgttgttgtgcgttgttgcgtttcctactggcgtggtcactagcccacagatccttccatttgcagctcaataaggcggttcagctcgagggcgtactccatcggcagctccttagcaatcggctcgacgaagccgcgcacgatcatcgccatcgcctcttcctcggcaatgccgcgggacatgaggtagaacagctgctcctcgctgaccttcgacaccttcgcctcgtggcccagcgtcacgcggtcgttgcggatgtcgttgtacgggtacgtgtcagaacgggaaatgtcgtcgaccaagagcgcgtcgcattccacgttcgacacggagtggtgcgcgttcgcgttgacctggatcaagccgcggtacgcgctgcggccaccaccgcgggcaacggacttcgacaccaccgacgaggaggtgtgcggagccaggtgcaccatcttcgcgcccgtgtcctggaactggccctcgcctgcgaacgccacagagagcacctcgccgcgggcgtgctcaccagtcatccacacagccgggtacttcatggtgaccttggagccgatgttgccgtcgacccactccatcgttgcgccttcctcggcgcgggcgcgcttggtcacgaggttgtaaacgttgctcgaccagttctgaatcgtggtgtagcggcagcggccgcccttcttcacaatgatctcaaccacggcggagtgcagagagtccgacttgtagatcggagcggtgcagccctccacgtagtgcacgtacgcgtcctcgtcgacgatgatcagggtgcgctcgaactggcccatgttctccgtgttgatgcggaagtaggcctgcagcgggatatccacgtgcacgcccttcggcacgtagatgaaagacccgccggaccacactgcagagttcagggcggagaacttgttgtcgccggccggaataacggatccgaagtactcctggaacagctccgggtactcgcgcaagccggtgtcggtgtcgacgaagatgacacccttttcttcgaggtcctcgcggatctggtggtagaccacctcggactcgtactgagcggcgacgccggccacgaggcgctgcttctcggcctcggggatacccagcttgtcgtaggtgttcttgatgtcctcgggcaagtcgtcccagctctgggcctgctcctcagtggagcggacgtaatacttgatgttgtcaaaatcaatgtcggaaaggtccgcgccccaggtcggcatcggcttcttctcaaagatctcgagtgccttcaggcgctggttgagcatccattccggctcgttcttgatgccggagatgtcgcgcaccacgtcctcgctgaggccgcggcgagccgacgcgcccgcgacgtccgagtcgtgccacccgtagttgtaggcgccgatggagttgatgatctcgtcatcgttcatcggcgtctcaaggccgggtgcgggagttgctttcgtcattgtgtgtccgctccttagctttgaaagctcgttgttgtctggttttttcgctgccctgcgtaaggctggttcacgtccgttaacggaatgttcgtcgtgcaaattccgttgccgtccgcgatcaaggccagcgactgaatgtggctgcccacaagctctgcaatgagctcgtgctctgcttcgcacagttccgggtgctcggccgcaaccgcggcaaccgggcagtggtgctggcacagctggatgcctccggcggccttggtcacggtagtggcgtagccgtagctctccagcgcggaagcgacatctttgaccacgtcctccaccgcgccgtcggtgctcacacccgcaaggatcttccggatccgggcgctggcgaggtcgcgcaccgcttcttggccgccaaggttctcgatcacgtccaccgcgtctttagcgaggtcgccgtacccggtgccaaagtgcgcgcggccggagtcggtaaggcggaagtgtttcgccgggcggccgcgcgttgcttccgccccggcgacggcgttgggttcgcattcctcggcaatgccctccaccaccagcgcgtcgaggtgcctgcgcaccccagcggccgacagttcgagggcctcgcccagttcggtggcggtgaccggcccgcgcttgagaagctgcgacatgaccgcgcggcgggtctccccaacatttgttcgctcagccattgcctcacctctttccagcgtcgatttctcagggccttttcacaacactagtgtgtgctaaatgatttcgccgcagcgggtcgggggaacccaggagcatttcgcttatcgacgccacgccgtctcctacaatctccccgcgctcgattccctccctcaccacggggcccttcgagtggtgggccttatcggcgctgtgatcgtcgccctcggcggctggcgcggcggcgcccttccggcgaccgcagaggccaccgacaccgaggtaatcgtctccaacgcggcggtgttcgtcggcgcagccgttatggtcgctgcgtggttgggcatgggaccccgcgccgcgcgcggcgatgtgcgcgacagtgtgaccacgttcttgtggtggtcggcacccctggtcgtcaccgccccgctgttttcccaggacgtgtactcctacctcgcgcagggcgcggcggtgcaccgcggcttggaccccttctcgggtggacccgtgaccctgctcggacgcggcgacccgctggcgcagaacgtgccgaagatctggtctgactcccccagcccttacggcccggttgcgctcggagtgtccgcggcgatctcggtgctctccggcgacgacgttcgcgcggcgattatcatgcaccggctcgtcggcattgccgcgctactcgtgtgcgcgtgggcgctcgccgcgcttgcccgccgccgcggcgtatccccgggatccgcgctgtggctgggtctgcttaacccgttggtggtgctgcacctggtcgggggaatccacaacgaggcaatcatgctcgctttcatgcttgcaggcctcgaagtcggcctgcgggcgctcgacgagggtgccgtgcgcagctggacgttgttcaccgcctcgagcgcgttgatctcctgcgccgggctggtgaaggtttccggtttcatcgcgctcggcttcaccggcatggcgctcgcccgcgtgacgcgcccgcgtctcggaactgtcaccgcagtcggggcagcggcactcttccagctcgccgctctcgcctctaccgcggtagtggtcgcggcgatcgcccacaccaccaacgggtggctgttcgtccaaggcggcgcggccgagatccgcagctggctgtccatgaccaccgaggccgggatcatactgagcaacgtcggcgagtggctggggcttggagaccacaccgacggtctcatctcgttcacccgcggcctcgggttcaccatcgcggtcgcctacatggtgcgcaagctgttcgagacgctcaacggcaagcagcatccggtgcacgcgatgggtttatccacgctcgttctcgtcgcgctgttccccgtcgttcagccgtggtacccgctctgggctatcccggcgctcgcagcgagcgagcggcggttgcttgtgcgagcaggcctcgccgtcttcagcgccgctatctgcttcgtcgtccttccccttggcagctcgatggagccgaacgaggtcgctgtggtctacgcgggcgcgttcgcctcggtggcgctgatcgccggcgcggcgtggctctggttccggcgtaggacgcctgcgcgactacactgacgagccatggaaaacgcgctggttgtcaccgatgtggtcaagcgcttcggcgaaaaggtggcggtcgacggtttgagttttgccgctccgcagggccaagtcctggcacttttgggcccgaacggcgcaggcaagtccaccaccctggacatgtgtgaaggtttcgcccgccccgactccggtgagatccgggtcctcggcattgacccggccaagcaaccgcagaaagtgcgcgagcgcatcggcatcatgctgcagggcggcggttcgtattcgggcgtgacagtgcgcgagatgctcaatctcgccgcgtcgtacaacgtcgacccgcacgacccggattggctgatcgacctgctcggcctgcgcggggtggaaaacaccacctaccgcaggctctctggcggccaggcgcagcggctctcgctcgccctggcgattatcggccggcccgagctggtgtttttggacgagcccaccgccggcatggacgcccaatcccgtgccgctgtgtgggacatcatcaccgcgctgcgccgcgacggcaccacggtcatcctcacgacccatctgatggacgaggccgagtccctcgccgaccgcgtcgtggtgattgaccgcggcacggtcgtcgcccaggggaccccagccgagctcaccgcccacgccggctccccaaccaccacggtgatcacggcctccccactcgaccctgacgccctcggaagccagctcgcccccttcggttgcaaagtgcgcgagacccgccatcagcactaccgggtgttgggagagatgacccccgccgctgtttccgcggttgcgctcgaggcggagcggcaaaaggtgcagatcacggacctgcgggtgtcgcaccgcacgctcgaagacgtgttcttggacgtcaccgggcgccagctccgcagttagatccggccagacgagaagagaaggagtccagcatggagacaagcccgcagctcgaccacggcgttttctcccccgccccgcggcgggccaccttcagccaaatggctgttgcgcagggcaagatcgagtcgaagctcatgctgcggcacggcgagcagatcctgctgaacctactgatcccggcaggtctgcttatcgctgctgctgtggcgccggtattcggcgacatcgatttcaacacccttgtgccgatggtcttcgctgtcgccgcgacctccgccgggttcaccggccaggccatcgcgctcgcgttcgaccggcgctacggcgctctgaagcgcaccggcgcatccggggtgcctccgtgggtgatcatcgcaggcaaaatcatcggcgtgcttgccaccgtagccgtgcagatcgcggtgctgggtgcgcttgcggtgttcctcggctggcgcgtcagcctcgttggtgcgctcgccggccttgcggttttgctgatcggcgtggcggtgttcacctcgctcggcatgctcatgggcggcaccctgagctcagaagtagtgctcgcgctggcaaacctcatctgggtcgcgttcatgggcatcctcggctgggtggcgtattcgggtgatgttgcccacgccggctggtggaacgctgtcccgacggtggctctggccggtgcgctcacacaggccctccacgtcgccttcaacgcctgggcgtggctttcgctggctgtctggggtgctatcggcgtcggcggcgccgagcgctggttccgcttcgacggctaggtgtttggcccccgcgcgcgatagactgccccgaaacaacgagcatcaaacaaaagttggagaggttcgacagtgagcaccaccgcgcccgcgacgaacggcggcgatactgggttggcggctgaggggccgtcgataagcttgcagcgcacgcttgcgatgatcctgctggtgtgccagggcggcattacggtgaccgggtcgctggtgcgcgtcaccggctccggcctgggttgcaacacgtggccgctgtgccacgagggctcgctcgtgcccgttgagggcgcggcgccgtggattcaccaggcgatcgagttcggcaaccgcctgctcaccttcgtcgtcgccgctgcagccgttgccgttctgctggcagtgaagaaggccgggcgccggcgggagatcaagaccctagcctggatttcgctgctcggcgtggtgctgcaagccgtcatcggcggcatttcggtgctgctcgacctgcgttggtggtcggtggccgtgcacttcttaccctcgatggtgctcgtctgggtcgcggcgatgctgtacatgcgcgtcgccgagcccgacaacgccgcgccaaccgagcgctaccccaactccgtgcgcacgctggtcgtgctcgctgccgccgcgctgtgcctggtgctgatcaccggcaccatggtcaccggctccggcccccactctggagactccggcgtgggcatggaaggccgcctcgagctcgacacggccatgctcgcctacgtccacgccgcgtgcatgtacgtctacctcatctgcactctggtggctgtctacctgctgcgcaagcacaacgcgccgaaggacgcgttcaacacctccttggtgctggtggcgctcatcgtcgtccagtgggccatcggcgtgacgcagttccgcctcggtgtgccgcgctggaccatccccgcgcacattgggatgagctccatggtggtcgctttttccgcgttcttgtactcgcacgggaagcgcaggttgcctacgctgaagtgacatgaaggcaatttatgtcaccgagcacggcggacccgaggtattgcgctacaccgacgtggaggcccctgagccgacgcaggagcagttgcttatcgacgtcgcgtttgccggcatcaactacatcgacacctacttccgctccggttcctacccgcaggatctgccgtacatccccggcaccgagggctgcggccgcgtcgcgcacgaccccaagggggagatcgcggagggcacgctggtggcgtggaaccgcggacccggctcatacgccgagcaggtcgtggtggaccgcggccgcgtcgttgccgtgccggagggagtcgacgaggcagtcgcggcctccatgctgctgcagggcatgaccgcgcactacctcaccgagtctgtctaccccgtcaccgaagacacctcgctggttgtgaccgcgggcgccggtggtgtgggcctcatcctcacccagatggccgcggcgaaaggcgcgtcgatcttctcagttgtctccaccgaagagaaggctgagctcgcccgggaggcgggcgccacccacgtcttcacctacgcggacgacttggcggcccagatcaaagacgcgaacgacggccgcggcgtcgacgtggtcttcgacggggtgggaaaggacacgttcgatttcgcgctcgaggtgtgccgcccgcgcggtctcgtcgcatctttcggctccgcctccggcgacgtggagcccttcgagatccagcggctgaaccgcgccggctccctcttcctcacccggccgaaactagacgactacaccgcgtccgacgacgagttccgcatgcgggcccaggcggtcgcgcgcggtgtcgaggacggcacgctcacgttccgcatccacccgccttacgacctcgccgacgcgaagcaggcgcacgaggacttgcaggcgcgtaaaacaaccggttcggtcgtcctgcgggtcagcgagcagtagctgacggcgccgtcaagctacagcagcgtgggcaggccgagcaccgcgtccacggacaggccgaggaagagcgccgcgaggtagttgttcgacaggatgaacagcttcagcggcttgaccttctcccctgccttcacgccgctgtaaagcttggtcgcaaccacaaggaacacggccccggacacgagtgcggtgatcaggtagatccacgacgccgcgggcacgagaagcagcgaggtggcaacagtgagccacgagtagaccacgatcttgcgcgtggtctcggtcggcgtggccacgacaggcagcatcggtacgttcgcgcgggcgtagtcgtcgcggtacttcatcgccagggcccacgtgtgcggcggtgtccagaagaagatgatcatgaacatcaccacggcctgccaccagtggtccggggagccgtcgtggacgttgtcgcggatgaccgcccagccgacgaggacgggcatgcagccggccgcgccgccccagatcacgttctgccacgtcctgcgcttcaaccatttcgtgtagacgaagatgtagaagaagttcgtgaaaacgatgaatgccgcggcgagccaggagttgcagacgaacccgagccagagcaccgaggcgatgagcagggcccaagcgaagaccgccgctttttccttggtcacgcggtggcgcaccagcgggcgggcgcgcgtgcgccccatcttctggtcgatgtcgtagtcggcgaccatgttgaaggtgttggcggcgccagcgcccatccagccgccgaagagggtgcccagcacgagccagaggtcaacctcgccgcggttggcttggagcatggcggggatcgcggcgacgaggagcagctcgatgaccctcggcttcgtcaacgcgaaatacgccttgatggtctccaacacttctccttcgccgtggcgtttgaaaattcattcttaagggcgcagcggagcgcccccgcatcattccttcggttgatactaaccccgacccgcctctcgtacggaatcggacacgtcccccaccgctcgcctcgcgctcacggtgcggggagggagcttgtaggatttgtatgaccttcactgcccccacgagacccaagcgaggaaactgtgaaccagccgacgctgcccgagccgcttcaggctatgaccgtccgcaactaccccaaggactggaccgatacggacacccgcgcggtcgacacagcccgcgtcctcgccgccgacgccgtggagcactgcggctccggccaccccggcaccgcaatgtcgctggcaccgctggcctacaccctgttccagcgggtgatgcacgtcgacccgcgcgacaaggactggattgggcgcgaccgcttcgtactctccaacggccactcctcgctcacgcagtacgtccagctctacctcggcggcttcgggttggagctcgacgacctcaaggcgcttcgcacctgggcctcgaagacgccgggccacccggagtacaaccacacagaccacattgagatcaccacgggccctctcggccagggcctcgcctccgcggtaggcatggccatggccgcccgccgcgagcgcggcctgctcgacccggacgcagctgccggcgaatcgccgttcgaccacttcatttacgtcatcgcgggcgacggctgcctgcaggagggcgtcacctcggaggcgtcgtcgctcgccggcacccaagaactgggcaacctcatcctgttctgggacgacaaccgcatctccatcgaggacgacacgcagatcgcgttcaccgaggacgtgctgaagcgctacgaggcctacggctggcagacgctgaccgtcgagtccggcgaggacgtcgtcgctattgagaaggctgtcgagaaggccaaggccgaaacggctaaaccgaccatcatccgcgttaagaccgtgatcggctaccccgccccgaccatgatgaacaccggcgcggtccacggcgccgccctcgggcctgacgagatcgcccgcgtcaaggaggtgctcggcttcgacactgaggcgaccttcccggaggaggctgaggtcatcgcccacactcgcaagctgggcgagcgcgcggccgagtaccgcagcgcctgggaggagaagttcaccgcgtgggccgagcgcaacccggagcgcaagcagctgctcgaccgcctcatcgcgcgcgagctgccggccggctggggcgagggcgaacttgccttcccgacgtgggagccggacgagaagggtatcgccacccgcaaggcgtctgaatccgccatccaggtcgcggcaaaggcactgcctgagctgtggggcggctccgccgacctcgccgggtccaacaacacgttgatcaagggcgtggcgtccttcggcccgcgctcgatctccaccgacatcttcaccgccgagccctacggccgcaacctccacttcggcatccgcgagcacgcgatgggctccatcatgaacggcatcgccctgcacggcccgacccgcgtctacggcggcacgttcctgatcttctcggagtacctctaccccgccatccgcgttgcggcgctttccggcatcgacggctactacgtgttcacccacgactccatcggcctcggcgaggacggcccgacccaccagccggtcgaaacgctcgcggcgctgcgcgctatcccggacctcgcggtgatccgcccggcggacgcgaacgagacttccgcagcgtggaaggcagcgctcgagtccaaggagcagccgaaggcgctcgcgctgtcgcgccagaacctgccagtgctcgaaggcacgaagcagaaggcgtttgagggcgtggcgcgaggcgcgtacgtgctcgtcgaaggctcgaaggccaccccagatctgatcctcatggcctccggctcggaggtgcagtacgcggtcgaggccgccaaggtcttcgaggccgagggcaccgcaacgcgcgtggtgtccgtgccgtccatggactggttcatggagcagggcgacgactacatcgacgaggtgctcccgcgcgaggtgaaggcccgcgtgtcggtcgaggccggtgtctcaatgccgtggttccgcttcctcggtgagcacggtcgcgccgtctcgctggagcacttcggtgcctccgcaccgggcgccgagctgttcgagcgctttggtttcaccaccgacaacgtggtgcgcgtcgcacgcgagacgctcgactgcgtggccaacaaccgcaccgtcccgaccagcgagcgcgtcggcgataccgagtccgaaccaacccgcggcgacggcaagtaactgccgcacgaaaggaaccgaacaccacatgaccgcgatcgatgatctctaccagctaggcacctccacctggctcgacgacctctcccgcgagcgcatcacgaccggcaacttggcgcaggtcaagcgcgacaagtccatcgtcggcgtaaccaccaacccggcaatcttcgcaggtgccatgtctgccggcaacgcctacgacgagcagctcgccacgcttcgcaaggaaagctcgcttgccgacgcagcggtgtacgccatgagcgtcaaagatgtccaagacgcctgcgacgaattccgcgacactttcgagcgcaccgggggcaaggacggccgcgtgtccatcgaggtcgacccccgatacgccgccgacgaggagaaaaccgttgcccaagcagcggaactgtggaagcttgtcggccgcgagaacgcgatgatcaagatcccggcgaccgacgagtcgctgccggcgatcaccgcctccctcgccgagggcatttccgtcaacgtcaccctcatcttctctgtggagcgctaccgccaggtgatcgaggcctacaaacgcggcatcgccgaggcggccaagaacggccacgacgtgtcgagcattcactcggttgcgtccttcttcatctcccgcatggataccgaggtggacaagcgcctggacgccatcggcaccgatgaggcactggcgctgaaaggcaaggcgggtatcgcgaacgcccggttggcgtaccagctcttcctcgacgagttctcggacaccgccatgaccgaactcccagccggtgcgaacaagcagcgcccgctgtgggcgtccaccggcgtgaagaaccccgactaccccgccgacatgtacgtcgtggaactggcgggcccggatacggtgaacaccatgccggaggcgacgatcgacgccgctatcgccggcgaccgtgtcggcggcgacaccctgacgggcaccgccgaggcttcgcaggctatctttgaccagctcgccgccgccggtatcgacgtcgaggacgttgtggacgtactggagcgcgagggcgtggagaagttcgtcgacgcgtggcaggaactgctcgacaacatggaggaaaacctcaagtgactcgtccgaatccagcgccgctagcaaacccgctccgcgccttggacgacacccgcctgccccgcatcgcaggcccgtccggcatggtcatcttcggcgtgaccggcgacctcgcgcgcaagaagctgctgccggcggtgtacgaccttgccagccgcggcttgctgccggccgggttcaccctcgtgggcttcggccgccgcgagtggtcgaagcaagacttcgaggattacgtccgcgaggctgtgacgtcgtccgcccgcaccacgttcaacgagaacgtctgggcgcggctcgcagaaggcatgcacttcgtcaccggcgctttcgacgacgacgcagctttcgacaaactcgctgcccagctggaggagatggacgctacacgcggcacgggaggcaactgggcgttttacctctcggtcccgccagagcacttcgccaacgtcgtccaccaactcgaccgctgcggcatggcggcgcaggagggggacaacggcgcgtcgcggtggcgccgcgtcatcatcgagaagccgttcggacacgaccgggaatcggccgtcgagcttaactcggtggtcaactcggtctttcctgagaacgcggtcttccgcatcgaccactacctgggcaaggaaacggtgcagaacatcctcgccctgcggttctccaacgagatgttcgagccggtgtggaacgcccactacatcgaccacgtgcagatcaccatggcagaggacatcggcctcggcgggcgcgcgggttactacgacggtatcggggccgcgcgcgacgtgatccagaaccacctcatccaactgctcgcgctggtggcgatggaggagccgacgtcgttttccccgcggcgtctcaaagcagaaaagctcaaggtgcttcgggcgacctttcccgtcgaaccgttctccgagaccaccgcgcggggccaatacactgccgggtggcagggctccgagcacgtggtgggtttaagggaggaagagggcttcgacccggaatccaccacagagacgttcgcggcctgcacgctgcagatcaactcgcggcgctgggctggcgtgccgttctacctgcgcaccggcaagcgcctcggtcgccgcgtgacggagatcgcgctggtgttcaagcgcccgccctaccagcctttcaccgagggccaaacagatctcctcaccaacaacgccgtagtgatccggatccagccggacgagggcgtgctcatgcgcttcggctccaaggtgcccggatcaaccttcgaggtccgcgacgtgaacatggacttttcgtactccgaggcgttcaccgagcagtcgccggaggcgtacgagcggctcatcctcgacgcgctgttggacgagtcgagcctcttccccaccaacgacgaggtggagcgcagctgggagatcctcgacccaatcctcaacttctgggccgacaacggccggccggacgagtacgccgcggggacgtggggcccgaagtccgcgcacgacatgctggcgaaagacggccgcgaatggaggcgcccgtaaatgatcctcaccctgaagaacacgaccacgcgcgagatcgcgaacacactggtcgcggcgcgcgaaaactactcgctcgccaccggccgcgtgctcacgcttctcgtagccgtgagggcaatcgacgacgtcgacgcgatcctttccaccttgcgcaccgccacccgcgagcatcccgctcgcgtcctggtgctgatcatcggcgatccggcagagccaacctcgctcgacgctgaagtgctcgttgccgccgacgccggcgcatccgaggttgtggtgatgcggctgcgcggcgagctgacgaaccacctcgacgcggtggtgactcccctgctgctgccggacaccccgatcgtggcgtggtggccgaccacggccccggcgtgccccgcgcaggcgccgctgggcaacattgcgcagcgccgcatcactaacacccaccacaacgtgaccggcaactccctgctccgggtcacaacgggctacaccccgggtgattcggacatgatgtggtcgcggattacgccgtggcgcggagtggtcgcctcggcgctggaccgctgccccgacgcgcagatccgcgcggtgaggatcaccggctgcgcccaggacccgagcgtggatgtcgccgctggttggctcgcctcggcgttgaacgtcaccgtgaccagggcgtcgtccgagcggcctgctgaggacgcggcgcagatcgaccaggtgaccttcatcgccgacatcggcgagatcaccgtcgaggtcgtcgacgcccacacggtcaaagtgtcggtgccgggcaacgccgacgcctttgtcgcgctcagcgcccgcaccgacgcggagtcgctcgccgaagagctgcgccacctcgactcggacgcgacctacggcagggcgctcgccggactggcgcaggtgcaggaggcgtaaagtgcggattcttaggttcccagagctttcctcgcttatcgacgccaccgcgtcccgcctcacctccctcgtccgcgacatccagtcctcagcagacggcggcctccacggcgacggcgtggcccgcctcgtgctgaccggcggcaccgccggcatcgcgctgctgcgccgcctcgctgagcccgaactgtcggagcagatcgactggtcccgcgtccacgttttcttcggcgacgagcgcaacgtggcgcccacgcaccccgattccaacgaagggcaggctcgcgaggcgctgctggaccgcgtcggcattccagcgcggcacatccacggctacggccttgacggaggcccgatggacgaggcggtcgcgcgctacgctgaaacactcaacgctgtcgcaccgcaggggttcgacctgcacttgctcgggatgggcggcgaaggccacatcaactcgctgttccctcacaccgacgccgtgcgcgagcgcgaccttattgtcatcgctgtctccgactccccgaagccgcctgccgagcgggcgacgttgaccctgcccgcggttgcgcgcgccgagtgcgtctggttcctcgtctccggccaggagaagtcggaagcggcggcagcgctggctaccggagccgatcctgaggaatggcccgccgccggcgccaagggtacagccgaaacagtgctctatgtcaccgaggacgcggctcctccccagtcgtaactggacaaacaaaaagcttcccgcatggtgcgggaagctttttactgtgcataccgtctactacggcgtgaccggcgcggcgtacgtctggatcaggttcagcgcgatgatgcacgcgatccaaataatcgccagcaccaccgtcacgcggtccaggttgcgctcgaccgtggtcgagccggacaagttcgcctgcacgccgccgccgaagaggctggacaagccgccgcccttgcccttgtgcagcaggacaaagatcgtcatcaggatcgaggagatgaccagcacgatctgaagcgcgagcgccatgcggttgaaccttcctaggttggagaccgttagtgtctaactttggccagcctacaccaccgccgcccgcccctaggaatcagacacggctactgaaccgcttgcgctgcggcggccgcgagcttggcaaagtcatggccgtcaagcgaagcgccgccgacaaggccgccgtctacatcgggctcgccgatgatctcggcgacagtgtcgaccttcaccgagccgccgtagaggatgcggatactgtttgcggtgtcctcgtctgccaactcgcgcaccagcccgcggatagcgcggcacacttcttgcgcgtcgccggcggaggctaccttgccggtgccgattgcccacaccggctcgtaggcgatcacagttcgggcgagctcttctgcgctcaggcccgccagcgacgcgcgggtctgctccaccacgtagtccacgtgctcgccggcctcgcgcacctgaagcggctcgcccacgcacacgatcgggtggatgttgtgctcgagcgccttcttggctttcgcggcgaccagctcgttgttctctgcgtggtactcgcggcgctcggagtggccgacaaccacccaggtgcagccgagacgctcgagcatggcggccgagatctcgccggtgtaggcgccgttgtcgtgcgcggagacgtcctgcgcaccgaaagtgatctgcagtttgtccccctgaaccagcgtctggatggagcgcagatcggtaaacgggacggtcaaggcgacatcgacaaactcgtagccgtccttcgggaaggcgaacgcgagcttctgcgcgctctggattgcctcgaggtggtcgtggttcatcttccagttgcccgcgatgagcggtttgcgtgccatggtgatccttcctagtcggtcagtacagcaacacccggcagctccttaccctcgatcagctcgagggaggcgccgccgccggtggaaatgtgcgagaagccgtcttcgtcgagtccgagggtgcgcaccgaggcggccgagtccccgccgccgacgacggtgaacgaaccgttgtcctcggtcgcggcgatcatcgcctcggcgacggccttcgttccgtcggcgaagttctcgaactcgaacacacccatcggaccgttccagaacacggtcttcgagtccttgatcgcctcggcgtacgcggtcgcggactcaggtccgatgtcgaggcccatccagccctcagggattgcgtcgaggccgacaaccttcttctctgcgtccttggagaactcaggtgccgcagcgacgtcggtgggcagcagcagtttgtcgccgtagcgggcgatgagatccttgcaggtgtcgaccatgtcttcctgcagcaaggagttctgcacgttgtggccctgggccgcgaggaaggtaaagcacatgccgccgccgatgatgaccttgtcggccttctcggccagcgcctcaatgacaccgagcttgtcggagaccttcgaaccgccgagcacgacaacatacgggtgctccgggttgtccttcacggacgagagggtttcgacctctttctccacgaggtagccggcgtaggcgggcaactgcttcgccacgtcgtagacggaggtctgtgcgcggtgcaccacaccgaaaccgtcagagacgaacgcgccgttgtcggcggccagggcggcgagctcggacgcgaactcggcgcgctcggcctcgtccttggaggtttcacgcgggtcgaagcggacgttctcgagcaggaggatttcgccctcggtcaggccgttggcgcgctcgtgcgcgtcctcgccggaaacgtcgcctgccaggggcacgaactggccgagacgctcggacagagcctcggcgaccggggacagggagtatttgtcgttcacttcacctttggggcggccgaggtgggccatgacgatgaccttcgctccgtcgtcaagcaatgccttcaaggtcggaatggaggcgtcgatgcgccctgcgtcggtgatgttgccctcgtcgtcgagcgggacgttgaagtcggagcgcacgagcacgtggcggccgtcgacaccttcctccaacagctgcgcaagcgttttggtggccatgaaaatctcctcagtaattctccgtgttatgaaaacgggcccgcagccacgccgcgagccccctttgttgacaactgtgttgcggttacagcttatccgcgacgaacttggtcaggcggatgtactgggaggtgtaggaccactcgttgtcgtaccacgagatgaccttgaccaagttgccatcgataacgcgggtcatacctgcgtcgaagatcgcgccgtgcgtattagcgatgatgtcggaggacacgatcggatcttcggtgtactccagcgccacgcccaggacctcgtcctgcacggcgttcttgaccgcctggttaacctcctccaccgtgacgtccttgttcagagtgacggcgaggtcggtggcggagcccgtgatcgtcggcacgcgcatggcgaagccgtcgagcttgccctccaggttcggcagcaccagcgcgacagccttggcagcgccggtggtggtcggcacgatgttctgagctgcggcgcgggcgcggcgcaggtccttgtgcggcgcgtcctggatgcgctggtcgccggtgtaggcgtggatggtggtcatcagaccagactggatgccgaacgcctcatcgagcaccttggccacaggggccagggagttggtggtgcaggaggcggcggagatgatgttctgctcgccggtgtaatcggtgtggttcacaccccacacgtacgtgccgtcgacgtgcttgcccggtgcagaaatgatgaccttcttcgcgcccgcgtcgaggtgcgccttagcatcgttcgcgtcggtgaagcgaccagtgcagtcgagcacgatatccacacctgcctcgccccatgcgaggttcgccgggtccttctcagcagtgacctcgatgcggcggccgtcaacggtgatggattcctcgtcgtacgacacctcgcggccgagctgaccgtacgtggtgtcgtatttcagcaggtgggcaagcgtctcgttgtcggtcaggtcgttgatcttgaccacttcgaggtcgccggcatactcgtccaagatgatgcggaacgcggagcggccgatacgaccgaaaccgttgatgccaatgcgggtagtcatgccttcaatctcctctgggttgaatattcgttgactcgttggacccaccgcggcgcatctcgttggcagtgtttgcctaggcgctaacggcgctcacgatggcccgtcacaacccagtgtaaccagctggccccgcagctgcaggggcaaattggagggtgatctgtctaacgctaatccgcgccgccgctgccgttggcggcctcggctgccgcggcggaggtgtccggaagatcgagttcgctggcgcgcttatcggccagggacagcagacggcggatgcggcccgccacggcgtctttggtcatctgcgggtcagctaaccggcccaactcctcgagcgacgcgtgccggtgctcgactcgcaggtagcctgcctcagccaaatgctccggtacgtcgtcgccgagaatttcaagcgcacgctcgacgcgaagcgcagccgtcgccgcggcttgcgccgagcggcgcgtgttcgcgtcgtcgaaggtggcgaggcgctggcccgtcttcgcggtttgttgccgggtgacccgcttttcgtcccactccaagcggctgcgctgcgcgcccattcgggtcagcagtacaccgatggtctcgccgtcgcgaataaagacgcgctcggtgccgcgtgtttcgcgggtcttcgccgcgacccccatgcgccgagcgaggccgacaagagcgagcgcggcttcctgcccggggcacgctacgtcgagcgaagccgtgcgacctggctcggttaaggaaccccgggcgaggaacgcgccgcgccacgcggcctccaccgccgccatagatccggaaatgacctgacgtggcatacctacgacggggtggccggacggggtaacgagtttcagccggcggatcacgtcgtcggtgcggctgtccacgatgacgtggtggcgggtttcgcggctcgcgctgccgggctcgacggtttcaatccggcatggcgtctcgcaggtttcctcgagcagggcaccgagaaggtcggcgacggcgcgctcagcgaagttgcacaccagcgcaaggccgcggggggtggattcgtaggcgccggcaaagcggatgagcgcggttgcttctgccgcgcgggcttcagcggaggtccgcctcacgcccagaagctcatctttcacctttgcggtcagcgccaccgtcggatcctttccccttcacaattgccgtcgagacagtctagcttgcctgcaaaacctcgagcagcgcggtggcgagcttctccggatcgtgcctgttcagccctcggccgtcggcgtcggcttcccgcacctcgcagaagcagatttccgcgcccgccaccgcagccgcgcggcgcaggttgtcgcgctcgccctcggtcaagctcaacgtgctatcggcgatgaagtagtcgacgcgcagctcaggcgcgtggcgctcaaagacgtgcaggtggcgctcagtagtgaaaccaggcgtctcccccgcctcaggcgagaggttcagaagcaccgcgaccttcgcgtccgtctcgttcagcgctgtcacaatctcaggaacgagcaggtgcgggatcaccgacgaaaaccaggaaccgggcccgatggtgaccagatcggcgttgcggatcgcagcgaccgcgtctggggaggccaccggcttatcgggcagcacgcgcacccggcgcactgtgccgggggtcgtggcgacggcgacttgcccgcgcacggagcgcagcaccctcgggtcgtcatcaagacccgcgacgtcagcttcaatctcgagcggtgtcgggcacacagggatgacgcggccgacggatccagtccaacccgctaccacgtcgagggcagcttgcatcgaccccagctgttcgttgaggccggcgagaatcaggtttcccactgcgtggcccgccatcgcgccgtgaccgccgaagcggtgctgcaacgtgtcgcgccaaagatctccgtcgccgttcgccgcggtgagcgaggccagcgccatgcgcaggtctcccggcggcacgatgtccatttcgcggcgcaaacggcctgaagagccgccgtcgtcggcgacggtcacgattgcgtcgatcgtggttgcgttcgcgagacgggcagcttggagggtttggtaaagaccgtgcccgccgccgaggcaggcaatgtggaacgaagacacgagtgaatgtaccgcctttagtgccgctcgaggtcgcggtggatcacgctgacatccacatcgccccgctgacggagcctgcgcccgatcgcttcggatacggccaccgaccggtggtgcccgccggtgcagcccacgccgacagtgatgaagtccttgccctcgcggcggtaccccgccagagtgctgctgagcaaatcgacgaagttgtcgacgtattccttcgcgcccggctgcgtgagcacgtactgcgccacctgctcatccacgccgcggtaatcgcgcagttcctcaatccagtacgggttggggaggaaccggacgtcgagcacgatgtccgcgtcgcgcggggagccgtgcttgaagccgaacgactcgacggtgacgtgctggcgaccgacaggcaactcgccgactgaagcctccaccgcgcggcgcaaatcgtgcaccgacaggttggtggtgtcgatgatgatgtcggattgcgcgcgaagggtctccagcagctcgcgctcgcgggcaatgccggtctcgagcgtggcgttgccctgcaacgggtgcgtgcgccgcaccgagtcgaagcggcgtatcagcacatcgtcgcgcgcctcgaggaagagcacgaacggcgtgtagccgcgttccttgatgccgtcgatggtctgcatgagcgagccgttgaacacgtcagcgcgcacgtcggtgaccacagcgagccggtcgacaggcgaatcgtccgccgcagcgaggtcgatcagctcgagaatcagttgcggcggcaaattctgggagacgaagtaacccttgtcctcgaaaactttcgccgccgtagacaggccgccaccggaaagtcccgtgatgatcaccggtcgtatctgatcgcgcatgaaaaatatagtagtggaaaacgacttgtggatcttaagtgcgcaagtggtcgaaaatcgtctgggcgagctttggcccgacgcccttgacctcctgcagctcctccacgctcgcttccttcatcttcttcaccgagccgaagtgcttgaccaagtcggagcggcgagcgggcccgagacccggcaccccatcgagggcggaggcgcgcatccgcttggagcgctgctggcggtggtaggtaatagcgaaacggtgcgcctcgtcgcgaatctgctggagcaagtacatgccctcggagttgcggggcaggatcagcggctcgtcgtcgtgcggcacccacacctcttcaaggcgcttggcaagcccgatgagctgcacgtcgacaatgccgagctcgtcgaacaccgcttgcgcggcgttgacctgaggcttgccgccgtcgacgatgaacagctgcggcgggtacgcgaagcggcgcgaggacgattggctgccggtagtctcgacgtcggcgtcttcctcgtcggtgaacgtctgctccgcggccatctcgtcggggttagccaacttgtcctcgttgtagcgcttaaatcggcggcgggtgacctcggcgatggagccgacgtcgttcgaatggccgtcgcccgcggcttccttaatgcggtagcggcggtagtcgttcttcttcggcaggccgtcctcgaacacgaccagcgaggcgacgacatcggtgccctggatgtgcgaaatgtcggtgcactcgatgcgcagcggcgcctcgtccatcatcagcgcgtcctggatgtcttgcagcgcctgcgagcgcgcggtgagatctcccacacgcttcagcttgtgttggtgcagcgcctcggccgcgttcttgtgcaccgtttccatcagcgcgcgcttatcgccgcgctgcggcacccgcacctccaccggcccgccgcggagcttgcccagcagcgattcaacatcgtcgagctccgcgggcaggacctcgacgaggatgtcgcggggcacaggcatcggaggctgcaccttggcgcgcgattcctggtccaccccgcggcggcgcaccttctgcgcttcgatgcgcttatcttcctcttcttcctgggcggcgcgctcgacggcgtcggaatagtactgcacgaggaagttctgcatgagggtcggcagcgctgggtccttctggccttcctccagacgctcgagcgagccaggctcgtcaccggtcttctccaccacccagccgcgctgggaacggatcctgccgtcgcggacggtgaagatctgcacggccgcttccagctcgtctgaagcgaacgcaatcacgtcagcgtcggtgtcctggcccagcacaaccgtctggcgctccatcactttgttgactgcgccgaggtcgtctcgcagccgcgcggccttctcaaactcgaggttctccgccgcctcgttcatttgggcggtgatgcccttgaccagagcgtccgtgcgcccagacatgaaccccatgaatccttggacgatttcgtcgtactcggattccgtcactctcccgacgcacggcgccgagcatttgtcgatgtagcccaaaaggcacggccggcccagctgttcgtggcggttgaacacgccgttcgagcacgtgcggatcggaaataccctggtgagcaggtcgagtgtttcgcgcaccgcccaagcgtgggaaaacgggccgaagtagcgcacccccttgcgcttcggtccgcggtagaagaacgcccgcggatagcgctccttcacgctgaccgcgagcatggggtacgtcttgtcgtcgcggtacatgacgttgaaccacgggtcgaagcgcttgatccacgtgtactccagctggagcgcctcaacctcggaactgacaacggtccactccaccgacgcggcggtaaacaccatctgccgggtgcgcgggtgcagcgtctgcggcggctggaagtagttgttcagcctggctcgcaggcttttcgccttacccacgtagacgactctgccgttggcgtcgcggaacttgtacaccccgggctcagtcggaatggttcctggtgctggccggtaatctttcgggtttgccactgtgcgctggtgcttcgtcctaatcttctggcatgtacttcgcctcgagcacgcggaagtcctcgacggcctgaatggcgcgttccttatcccccgcctgaatcgcccacagcgggacgtactcgaagtctggcaactcgaggcgcgccatccgcgagcccttggggaagttcagtccgtacaccaggacccacgggtagaagcgggtgccgatgatgttgaccacctgcacgccgtccgcgttggctcgcacccgcggccgagtcagcgccacccacgacagcgcggaaatgatcagccccacaccgacgaacgcgaactggtcgagactggtgagcgtaacgcccgtgaactcggcgttcactacggcagccataaagatgtgcaccgccatgacgacgacgatccacaccgcggcgacgcgcttcaggtgcgaagagcgcacctcgtactcccacggcttgtccgtggttgccgcgtgcgggtcgagcgcggtgaggtaggcaagctcccggtcctccagttggctttggtgcgatgcttttccgctcacgtctacccgcttcccttcgccgccttgttgacggcgccttcatgttggttgtgtggtgatcctagcccttcagcggcaaggagcgaactttgcgcagctccaccgccgcgccgagggcggcgcggacggcatccgcacccttgtcctccttggcgtcctcgccgccggcgcgctcgatcgcctggtcctcctcctcgacggtgagcacaccgttgcccacgggggtcgcctcgtccagggcgacgcgggtgagcccggcggtgacggagtcgcacacgtactcgaagtgcgcggtctcgccgcgaatcacgcaaccgagcgcaaccaccgcgtcgtagcggcgggcgcaagcctgcacgacaaccggcagctcaagcgcgccgtcgacgaagtaagtgtccgcctttaccccgaggccgcgggcagtctccaaggcgcgctgcgtcatctgctcgacaacgcccgcgttccaacgggtagccacaactgccagggtgagtccttcggcccgtaactggtactcctcaggtgctccggtggacgacatgtttttgctccttcgcgtcggcgtttgatgcttcgagtgtatgagagcagtctatgcgttcgcctcagggtgctcggcgagccactcgcccactgcgggaagatcgtgtcccatccggtcgcgcttggtgcgcaggtagcggatgttctcgtgcgacggcgccacttcgatgcgcactcggccgctgatgcgcggccctgcaccgtcgagcgcggccaccttgtcagggttgttcgtcatgagctgggcggaaacgaggccgaggtcggtgaggatgtgggcggcggtggtgtactcgcgggcgtcggcaagcagcccttgctcgaggttggcgtcgacggtgtcgaaaccttggtcctgcagccggtacgcctccagcttgggcaaaagcccgataccccggccttcgtggccgcgcatgtagatcagcacgccgcggccggcgttgtggatgcgccgcatcgactcgtgcagctgcggcccgcagtcgcagcgcttggaggcgaagacgtcgccggtaaggcactcggagtgcacgcgcaccagcacgtcgtcttcaccggccacgtcgccgcacaccagcgccacgtgctccacgccgtcgatgccgcttcgatagccgtaggcggtgaattccccgaactcggtgggcaggcgcgcctcggtaacgcgggcgaccagttgctccgtgcgcttgcggtaggcgatgagctgctcgatggagatcatcttcaacccgtgggtgtcggcaaaacgacgcagctcgtcgaagcgggccatgtcgcaggggtcatcctccgaaacgatctcgcacaaggcaccaaccggccggcaccccgccatccgcgccaagtccaccgccgcctcagtgtgcccgtcgcgggtcagcacgccgccttcgcgggcgcgcagcggcaccacgtggccggggcgggtgaagtcggccgggaccgattgggcgtcggcgaggcggcggatcgtctccgcgcgggaggtcgccgagatgccagttcctcccgtcgcggcgtccacggtcacggcgtaggcggtgccgcgcacgtcctcgttgcggaccaccatcggcggcaggtcgagggcggtggcgcgggcgtcttcaagcgaaacgcagatgtagcccgaggtgtagcgcaccatgaaggcaaccagctccggggtagccttctcggcggcaaagatgagatcgccctcgttctcgcggtcctcgttgtccaccacgacaacggcctcgccgcgggcaacggccgcgaccgcctcttctactggatccaaacggttaagacggtcggggttgctcatacggcgcaatgttagccccgcaccattttctcgacgtacttggccacgatgtccacctcgaggttgacggtgtccccctcgcggagcttgccggcggtggttgcggcgagggtggtagggatgagcgagacttcgaaccagccctcgccgacagccgacaccgtgagggatgtgccgttgacggcgatggagcccttctccaccacgtagcgctcgagcggagccggcagcgagaagcggaacacctcccagttatccgacggggttcgagcaaccagccgcgcagttgcgtcaacatgcccctggacgatgtggccgcccatgcgctggcccgccgcaagcgctcgctccaggttcaccgcagaacccacctcgtactctccgatgcgggagcggttcagactctcgcgcatcacgtccgcgcaaaacgcggtgtctgcgagctcaaccaccgtcaggcacacaccgtcgacggcgatggagtcgcccggctgcgcatcggaggtgaccagcggcgcatccacggtcaagcgcaccgcgtcaccgagcgcttccagcttgacgacgctcccctgctcctccaccaacccagtaaacattttcgtctcacgccttccttttcatctcaaagatcacgtcgtcgcctaaaagcatggtgcgcaccggttgaaagcggcgggcatctgcaagggtttgcgccaccggtcccgccagcaccccgcggcccgcgcccaaaaacgccggcgcgatgtgagcctggaccatgtccaccaaatcagcagcgaggaaactgtgcgctaagtgcgccccaccctcgagcaggacgtcgcgggcgccggtctcccacagcgcgctcagggccttatgcggggtggcgtagcactcgtaaccgcccggcacctcgcctgcggcggcgcgcgagccgatcactaccctgcgcggctgccggtcgtaaagcgtgccgtccggtttccgggcggtcagcttgggtttgtcggcgagcgctgtgcccgatcccacgatgatcgcgtcgcgggtcgcgcggtcctcgtgcacccacacgcgcgccttgtcgcctgtgatccactggctggtgccgtcggcggcggcggtgaaaccgtccgcggtggccgcgtacttccacgtcaccgccggcctgccgagacgcaccgaggtaagccacggctcgagcgcgccgactgcgataggcaggtgcgtcaccttgacaccgttctcgcgcaggtgttgcgcgcccccggcggcctgcgggttcgggtctgccgtgagatacaccacctcggccacgcccgcgcgcacgagcgcctccgcgcacggcccagtgcggccggtgtggttgcagggttccagcgtcacaaccgccgtcgctgaacgggcgcgttcgcccgccgcgcgcagcgccacgacctcggcgtgcgcgccgccggcgggttcggtggcgccgcttgcgatggggttgccgtgggcgtcgataagcatgcagcccacaggcggattgggcgacgtggtgccgcggaccgactcgcccgcctggatcgcggcggatgcggcctcggcgaggcggctaggaagcacgtgcctcacgcgcgagcgcgcgcagccgctccacggcctcggccgggttgtcggcgccgaacaccgcgctgccggcaacgaacgcgtccacacccgccgcagccgcctcggcgatcgtctcgctcgaaatgccgccgtcgatgccgataacggtgtcaaggccctgctccgcgattgcgtcccggagctgcaccaccttgcccagcacctccggcatgaacttctgcccgccgaagccaggctcaacgctcatcaccatgacctcgtcgaagtgctcgaggctgtccaggtacggctcaaccggcgtgccgggtttgacggcgaacccggcctgcacgccgaggtccttgcattggcgcgccgcggccacgtggtcacccaccgcctcgacgtggaacaccatccggtctccgccagccagtgcgtaggtcttgaaccacctctccgggtcctcgatcatcaagtgcatgtccaagaactgctcggtgaccgcgttgaccgcgttggtcacatcgggcccgaacgacaagttgggcacgaagtggccgtccatgatgtcgacgtgaatcaggtcggcgttggcaacttttcgcacgtcgtcgccgagcgcggcgtagtcggctgcgagaatcgacggggcgatgtagatcatggtgcttagggtagcttcctcaaaacggcgaagaacatcgcgtcggtgccgtgccggtgcggccacatttgcacgcttttgtgctcgccgacgtcctccatacccccggcgaactggtgggcgtcgagctcctcgacctgcccaagggcaagttgcttgtcgacgatcccccgcgtctcccgcacatccggactgcacgtcgagtacacaatcaccccacccgggcgcgtcaggcgcaccgccgaggccaaaagttccgactgcagtgtgttgagttcggcgatgtcgcgctccgtctttatccagcgcgcctccgggcggcgccgcagcgctccgagcccggaacacggcgcgtccaccagcacgcggtcgaagctcgccttttctaacccggggtcgcgcccgtccgccacggtgaccttgaccgggaggtcgccgaccgcctttcggatgagctcagcgcggtgcggcgcgacctcaaccgcggtgacccgcgcgccgtcgatcgaggcgattgagccgattagtgcggccttgccgcccgggcccgcgcacaggtcgagccaccggccttgatcgccctcgaccggcacctcagccagtgcgcgggcgatgagctgggaaccttcgtcctgcacaccggcgaggccctcgcgcacctcctgtaactggcctgggtcaccttcgggcaggtagaccgcgtacggggagtacttgccctcttcaccgccggtggtcaacgcgagctcctcggctgtgatctcgccggggcgcgccacgaggtggacgatggggcgctccgagtctgccttcagcgcggcgtccagctcagcgactgcgctttcgcccagcgcggctgcgaagctggcggcaacccagtcggggtgagcgtggttgtggtcgaacttctccaaccactgcgccgccggagtgcgcgcgatggatcgcagcacgccgttagcgaagcctttggccttctcttggttcgccgcctccaccaagcgcaccgaggtgtcgaccgcggcgtgatcctccacgcgggtgtagagcagctggtaggtaccgagccgtagcgcggtgagcacctcggcgttgatatcgttcaccggccgcgacgagttcgctccaatgacctcgtccagcacgcccatggtgcgaagcgccccgtacgttagctcggtggcgaacgcggcgtcgcggcccttgatcttgcgctctttcaacagccccggcagggtgaggttcgcaaatgccccgtcgcgggtgacgcgcagcatcgtctcgaaggcggcctcgcgcggcgcgtcgccgatcgaagccgggcgcgccttcacgctgtaccgcgtctgctgcctgggcgtcgtgcgcttttcaccgcgaggtccccgcctgccgtctgctctcgacctgaatccgccgctcactcgaataccacgcccttctccgcgtcctcgggtttcatgccgcgcgcccagtcagccgcgttcatcatcttcttccccggcggctggacccgcgtcagcgcaacgtctgcgctgccggtgcccaccagcacctgcttcttcgacgcgcgcacctccccgggggcgagctccgacgtctcctgcgcttcgacgcgctcgagtttcacccggtctccgccgagagtggtccacgcgccgggcgcggggctgaacgcgcgcactacgcggtcaactacccctgccggttgcttccagtcgacgcgcgccatctcgggcgtgatcttgccggcgtaggtcccctcggtcggctggggcgtgtgcgcggctgcgccgctcgcgagctggtccatcgcctctacgagcgcggcggcccctgcttcggcgagacggcccagaagttcaccggaggtctcacccggttcaacttcagtgcgcagggtgtggatcacgtccccggtgtctaagccttcatcgatgcggaagaccgtggcgccggtgacctcatcgccgtggaggatcgcgtgctgcaccggggccgccccgcgccactgcggcaaaagggagaagtgtaggttcacccagccgtgcggcgcaatatccagcatgtccgacggaatcaagttgccgtaggcgacaacggggatgcagtccggctcgagttctttcaagcgctcgcggatctcctcgttgtctttcagcgtatccggggtgagcacctcaatcccgtgctcggcggcgagctccttcaccggcgaggggtgcaggctgcggccgcggcccttcctcgcgtcggggcgggtcagcaccgccactacctcgtgctgcgagtcgataagatggcgcagcgatgccgcagccggctctggggtcccggcgaacactaggcgcatagaacgaacgtctccttgtagttgcagcttttaagcttggaaccattccgcagcgcggatctcggccatggcggccttgcgctgcgccggttccatccgtgtaaggaacagtaccccgtccaaatggtcggtctcgtgctggatgcagcgcgccagtaaccccgaggcgcggatcaccaccggccggccgaactcgtcgacgccgcgcgcgagcacgtcctggtgccgtgttacctccccgcggacgccggggaccgaaaggcacccctcggaaccggtctggtaggcctcgccgaccggttgccacacggggttgatcagcaccccgcgcatgccctggcacccgtaaacgaacacgcgcttggcgacgccgacctggttggcggccagcccgacgccgcgggaggcgtccatcgtcgccaacatgtcccccgcgaaagcccggatggactcgtcgatgcggtcgacctcctgcgctcgcgtcgtgagcacggggtcgccgaagtagcgcaaacgcaacaatgccatgcgcccacgctagccgatgtcaatcgggttgacctgcacccgcaggggcagatctaccttgcgcgcaccccggctggccactcctgcgcgtagcgatttgcccagcgcgtcgcggcctgcaagcggcgagcgcaccagcatgcgctgcgccgggccgtgggtgtgtgtatcccactcccccggcagccccgcgccggggggcaggtcgacggggcccaagagttcggaatgctccggcagcgtggtgtgggcgaagaagtcgtcgagggcggcgcggggggcatcgacaagcgcgacatgcactgcgggcgggaaacgcgcgtcgcgccgctgcgcgagctcaagcgctgcgaagccctcgacatcccagcggatcaggtgctgcaccgcggggatggaagggtccgcaacgacgaccacttccccgccctcggaggcgggttggacaagtgccgcggcccgcagccatgtcgtgaacgtgtcctcggttgcccgcaggtcgggacgctgcagcaacgcccacgtgtcgagcaggactgccgccccgtatccggcagcttcgcccgcgacccgcggctccgctcccggcgtggcgacgacgatcgcgggctttcggtcgaccatgtcgcggatcttttccccccacgaactgatgatgcggtgcttcggaaacgcccgcccgagctcctccgcggtgcgctcggtgcctaagaccacggcgcgcattttcttcgacccgcacgccgggcacacgtggtgcgggtccatgcgtccgcaccagcggcacgccggtgcctgcgcctcgcccccggcgggcaggccaagcgggccgttgcaccagcggcaccgcgacggcgcgcggcacaccccgcaagcgagcgcctggatgtagccagtgcgcggcacctggaacagcaccggccggccccgctccagcgcgcgcgacgcagctaaaaacgcagacgacggcaggcgggcctggcgggcgcgggggtcgcgctccagctcgaagtcggagtcgcctgcggcgtggatgcgcggtgctcgcgcccggaccgtgtcgcggggtgcggtcagcgagtgcgcccacccggactccaccagaagctgcgcctccgcggtccgggcgtagccgccgatgatgactgaggtgcgctcgatcggcgcgcgggtggtgatgacctcgcgggcgtggaaatacggctcgcgcgggtcaaccagcgaatcgtcgccgtcgaacatcaccaccgcaagccgcaggttctccaacggcgcaaaggccgcggaacgggtacccaccacaatgcgcgcctgcccgtgcagcaccgagaggtagcgcgagtagcgggcttgcggtccctgggaggcggtcagtgtggtcacctgcttcgcggagacatgtgcgcgaagcgccgcctcaagctggtcgacgttacgctggtcgggcacgacgatgagcgcggagccgccgtcgatcgcgactttgaccgcgagcgcggccagcgcctccgcccagctatcgcccggcgccacctgccacgccgcccgcgccacgttgccggccagcacggcgtcgacgaaactctcgccgaaggtgtaggcgctccacgacgacaggtccggctctgaaacctcgccgagctcgtcccagctggtggccgtgtccgtctcctcggccttggcgtggcgcgccgggatcgctgcgcggtagaggtcggagcgggtggctgcgtagcggttcgacagggcgtcgataagctgcctgagctttgccggcgccaccacctcgggcgagataacccgctcgatgaaccgcagcttgccctggtgcgtggactccgcggtgcgctccaggacaaccgcgtccaccaaccgcccagcgaaacggatgcgcactttcaccccgggtcgcgccgcagctgaatccgcctccgaaacgaggtagtcgaaggtgcggtccagatgcgcgagcccgatcagcggcaacacccgcgcgacggggtcggcggcgctggaagtcggcatggcgacgattctaagcccccggttggctaaagctcagaccaaggcgcatactcagttgcgaattgttttggaagtacctgtcgtacccataaggactgtcccccatgaaccgcgccgtccgcgccaccgtcgctgctgtctgctcgctcgcactgctcacccccgcgtctcacgcgctgccgagcgtgtcggacctgtcgagctccagctcacgcgcgacgaacgacgcctggttgcagggctacaacgcgctgcctgcccagctgcgcgaggccgtgccgccgcacctgcggcccgcccagcccgcgcctctgccggcaccgcccgctgagcccgagtacgaggccgcgccggagcccacgccagcaccggacacctgcgcgaactgcgtggcgatcaccttcgacgacggcccgggagcctacaccggccggctgctggacatcctggacgagaagaacgccaaggcgaccttcttcgttgtcgggcagaacgcgaacgccaaccctgcgctgatgcgccgcatgcgcgacagcggccacacggttgccaaccacacgtacaaccacccagacctgaaaaagcagtcggacgcggcgattgcgaaacagctcgacgacaccaacgcagcgatcgcgaacaccacgggtattaaaccgaagtggatgcgcccgccgtacggctcctacgacaaccgcacggtggccgaggcgaaaagccgcggccaagcagtagcggtctgggacgttgacacggccgactggcaacaccgcaattctgcgaagacctgcagcatcgccgtccagaactccacgccgggctccatcatcctgatgcacgatatccacgcccccaccgtcgacgcggtgccgtgcgtcattgacgggctgcgcgccaagggtctgcgccctgtcagtcttgaatacatggtgaaacaatccgagccgggtcgcgtctacacccaccggccgtaaagcagccagcctcaccgcgcccgcgcgttgcggccgttacagtgagatgccatgactacttcgacagcggtatctgacgacaccgaaagcgccgggcgcaccggctggcgcacggcgaccccgtgggtcatgatcgccacgtacgtcctcgcaccgttgctgatcatccccgcggcgggcgagcaatccgcgcccacagccgtgatcgccctcgtcttcggggcggctgcggtcttcggcttcgtcgacgggtggaccttccgcttcacgtggtcgctgccgattctcgccggagtcggtttctggctggcgaagacgctctaccttaacgacggcacgtttatctacctgctgggctgcgtcgtcatcgctgccctcgcgggcgcgctcggcagcgcggcgaaccgcgggaagggcgcacgcgcgtgaccatcgagacatgggtgctcgaccaccccgaacacggccgaatcgaggtgcgcgccgggttcgacagcgatttcctcgccctcgatccatcctggccgggcatgaccgacgcaggcaaggtgggcgtgcgcccggacgccgacgcctcgctttccgctcgggcgcgggcgcgcatgcagaatccgccgatgcggatggagtttcttgtcgacgccgcggtgcagcaacagtacgacgcggtagaaagcgggcgtttccctctctacggcgagggcgcgaaggagacgctttcaccgacgatatcgctcggtgtcgaccgggagaaaccccacctgaagatcacagcgaacgcgttcaaggacatcctcgccatcgattaccgcgagggctccactgtggtcgagttcgatcccccggctggatcccgcggcgcgaaacggcgcgataccatggcctccagctcgctgaagcgaacgctcatccccattgcagaggggctgggcaaaggcggttgggcgctcgcggtggtcctgctcggcccgctggtaggcaggctcttaaattggctgctgggcttcctgcccgactggcagctgcccgacatcacgctgccgcacgcggacctgccggtgccgaaactcccccagaccgcgctgccaactccgaacatcccattcccagagatcaccctcccgcagctgcctgaatgggtggggtggctcgccgaatactccaaggtgtgggtgccggtggtcatcggcatcgtggtcggtatcgtcgcgctgcgcaaccacaagcggtcagaggcggagaaggcgaggtggaacgccccgcgcggcgaggcgcccgaggaacgctaggccacgccggccgcacgcttgagctcgtcgaccttgtccagctgctcccacggcaaatccaaatcgtttcgcccaaagtggccgtaggtggcggtctgcgcgtaaatcggacgcagaaggtcgagctcgcggatgatggcgtcaggccgcaggtcgaagaccttctgcaccgcctgctggatggactcgtcggtctggccttcggccgcggtgccgaacgtctcgacgtagaggccgaccgggttcgcgcgaccgatggcgtacgccacctggacctcgacgcgctcggcgagaccagccgccacaatgttcttcgccacccagcgcattgcgtacgccgccgagcggtccacctttgacgggtccttaccggagaacgcaccgccgccgtggcgggccatgccgccgtaggtgtccacgatgatcttgcggccggtcaggccggcatcacccatcgggccgccgacaacaaaggacccggacgggttcaccaaaagcttggtgtcctcgttgtagaactcgtccagacccgcgtccttgactacccactccaaaacatgctcgcgcatcgcgccctcgagcgcttcgcctgtgaagtcgtcgtcgtgctgggtggagatgaccaccgtgtcgaggtggaccggggtgtcgccgtcgtaggcgaacgtgacctgggtcttgccgtccgggcgcagtccctcgacgatggcctcgtggcggacctgcgcgaggcggcgcgagaggcggtgcgccgtggcgataggcagcggcatgtactccggggtctcgtgggtggcgtagccgaacatcaacccctggtcgccggcgccggactgggcgaactcctcgacctcggcacctgcgcgcgcctcctgggaggtggtgacgccggcggaaatctcctctgactggtcgccgatggcaacgttgacgccgcaggtggtgccgtcaaagccaacctcggaggagttgaacccgatctccaccaagcggtcccgcaccagcttggcgatgttggagtacgccgtggtgcgcacctcgcccaccacgtgcacttggccagtggtcaccagcgtctctaccgcgacacgggacttcgggtcctggcgcagcatgtcgtccaagatggcgtccgagatcgagtcgcagattttatccgggtgcccttcagtcaccgattcgctggtgaatagccggtggaaagtgccagttgcagtgtcatcgtgaagagacaaggtagtcacgctttcaagtaatcgggtgtatcacccaacacactagaccaagctgtctaaattggcaacgctacgcgccgtacgtctcgatcgcgtcccagatgcgcaccgcgacctccatcttggtgccgtccggcacctccacctcggaaccgtccgctccaagcatccaccccgagtttcgctcctcgccgaacacctttcctcccgcgacggagttcaccatcaacaggtccgcccctttgcgctcgagcttcgcgcggccgttggccagcacatcgtcggtttccgctgcgaaaccgacaatcaccgctttggtctcgcgggcatttcgcttatcgacgatcccccgcaacacatcagggttctccttaagacgaagcgtgctcaacgcgtcgtccgcctgccccttcttcaacttcgaggtcgctaccctctccggccggaagtctgcgaccgccgcggccatgatgaccacatccgcctccgcgacgcgctcgttcatcgcggcctccagatcgcgtgtggagcgcacccgcaccacctccgcgccggccggtgtgtccagatcgttggtgtctcccgccacgacagtgacctgcgcacctcgctgcgcggcgatctccgccagcgcgaacccctgcttgccggaagagcggttgccgatgaaacgcaccgggtcgatgttctcctgcgtgccgccggcgctaatcaccacgcgtttgccctcgagcgtgcgagcaatcgggccggtcgaggcaactgtgcgagccagctccgcgatctggcgcggctcaagcaaccgccccggtccggtgtccttgcccgtcaagcggccgcttgctggctctagcacggtgatgccgcggctgcgcagcgtcgcaacgttcgcctgcgtcgcggcgttgtgccacatctccgtgtgcattgctggcgcgatgaccaccgggcaggtggccaccagcactgttgctgtgagcaggtcgtctgcgcggcctgccgcgatgcgggcgatcacgtcggcggtcgccggagcaaccaccacgaggtccgcctcttggccgacgcgaacgtgttggacctcgtccacccggctgaacacaccggtgtccactgggtgacccgacagcgcttcgaaggtggctgcgccgacgaagttgagcgcgttcggcgtgggtaccacccgcacgttggcccccgactccttgaagtcccgcacgaggtggcacgccttgtacgcggcgatgccgccggcgaccccgaccacaacctgaaaatcgctcatggggtccgagtctacaaaaaacggtgccccgcacccgcctcaagttgaggcggcgcacggggcaccgtaacgcttggaagggtttactggccctcttcgtgctccaagagacccgcctggatctcgcgcagcgcgatggaaagcggcttctcgcccggttcggggttcaccagcgggccgatgaactcgaagacgccttcgtcggagttctggtagaagctgttgatctggcgagcacgcttggccgcgaaaatgaccagtgcgtacttcgaggagaccttggtcaatagctcgtcgatcgggggcgcggtaatgccctccggttcgtcgtagacgcgctcctgctcgatcaccgcgtcgtcagcagcttgcgacagatcgtcggttacgttgctcacttacacctactcgcttgttgtgttggtcaaaattgccgcgattgcggcgactgtctggtcgacatcgtcgttcaccacgacagtgtcgaactcgccctgtgcgtcgagctcttccctggcagtgctgagacgccgttggatgacgtcctcggtttccgtgccgcggccggtgagccgctcgacgagcgcctcccacgacggcggcgccaagaacacggttgcggcttccggcattaggcgcttgatgttgcgcgcgccggcgaggtcgacttcgaccagcaccgggtagcccgcctccagcgcctcgttcaccgggccggccggtgtgccggagcgctgcaggccaccgtgaatgtcggcccactccagcatttcgcccgcgtcgatgcggtgctgaaagtcgtcggctgtgacaaagaagtagtcttggccgtcaatttcgcccggccgcggggcgcgcgtagtcatggacacggagaaatagaggttcggcacatcggtgaccaaacggcgcaccactgtggacttccctaccgcggacggtcccgcgagaacgacgagcctgccgcgtttcgtgccctcaaccacgtcgctttacgcctcgtagccgaaacgctcgagcagagcgcggcgctgacggtcaccgagaccgcgcaggcggcgggtctgagcgatctccagctcttccatgatctcgcgagccttcaccttgcccaccttcggcatagcctcgaggagtgcggagaccttggtcttgcccacgatctcgtcggtgtccgccttgtccaggacgtccttgagggtgatctcgccgcgcttgagcgacgccttcagctctgcgcgctgcttgcgggcctcagctgccttctcaagtgccgccttgcgctgctcatcggtcaactgtggaagtgccacgggttcctccaatgtttctaagttcttaagtggtccagtgtgatcaaccgtccccggctgaattgcaccgttgcaactcgccagctccggccaagtgtagcactcgcgaaaagtgctgccgggttaacacggcctgcgtttgaccacgtcaacggttcgacggaactaagctaccagggtttttcccgagcagggaatcaccccgcgtcgttttgctgttttcgcagttcacgcacctgtttccgcaggttgtcaacattcggcccagcttgcagcaccgagcgcgagacgctcgggaacaccacgtgcgcgctgctccccgccagccggtcggcgtcggcgaacgtggcgccctgggcacccacgccgggcatcagcacacaaccgttcagctcgctgagggcaggaggcttgacgacggtcgcccccaccaccactccaacatggccgacagacgccccatccctggctggcgcgttgtacccggcgcactcgtccaccatgtactgcgccaccgtgggcgcagcctcagaaggctcgcccagcggcgcactctggaacgcctctgcctccgggttggagttggccgccatcacgaacacgcccttgccgtgctcagcagcgagcacgatcgcaggatcgagcgacccgacgccgaggtacggcgtcagggtgaccgcgtccgcttcgaggggcgaacctggctggagccacgccgcggcgtagccggccatcgtcgatccgatgtcgccgcgcttcgcgtccgccacggtgagcgtgccggattcgcgcagcgccgccagcgtctcctccaggacggcgaacccggctgagccaaagcgctcaaagaaggcgacttgaggtttcaccagcgcgacctcgcccgcgaacgcctccacgcacgtcagtgcgaaggtgcgcaagccgtcaacggtgtcgggcaacccccaggcgtcgagcaggctcgcgtgcgggtcaatccccacgcacagccgcccgcgctcgccaccggcggcgacgagcatgtcaccgaatgttggcgcacccatgcgctactcctgctcgccggtgtggttgagctcctgcaggctcatcacgccgacctcgttgccccgcaacgcttcgatgccctgcaccgcggcagtcacaccttgcaccgtcgtcatgatcggcacgcccgcggcgacagctgcggcgcggatgtcgtagccgtcgtggcgcgcgccggcagaacccgcaggcgtgttcaggatcaggtcgatctcgccgtcgttgatgcggtcgaggatgctcttgccttcagcgccctcgcgaacctcggacgccttcagcacggtctcgcactcgatgccgttgcggcgcagcatctgcgcagtgccggcggtggcaaccacgttgaaccccatggtgtagaggcgctggatggggaagatcagcgtgcgcttgtcgcggttggcgaccgagacgaacacggtgccctccgtcggcagctcgccgaacgccgctgcctcagccttggcgtaggccacgccgaaggacggcgccaggcccatgacttcgccggtggacttcatctccgggccgagaatagtgtccagcaccttacccgccggggtgcggaagcggctgaacggcagcacggcctccttcaccgcgatcgggtgctccagcggcaacgagccgccgtcgtagtcggacgggatgagaccctcagacttcagctccgcaatggtggcccccatcatgatgcggctggcggccttcgccaggtgcacgcccgtggccttggacacgaacggcaccgtgcgcgacgcgcgcgggttcgcctcgatgacgtagaggatgtcgtccttcagcgcgaactggacgttcatcaggcctttcaccccaatgccgtgcgccagcgcttcagcagagcggcgcactttcgcgatgtcgtcggggcccagcgtcatcggcggcagggcgcaagccgagtcgccggagtggataccggcctcctcgatgtgctccatcacgccgccgaggtacacctccgtaccgtcagagagcacatccacgtcgatctcgatcgcggagtccaagaagcggtccaccagcaccgggtggtccggggtcagctcggtcgcgcggtcgatgtagtcgtggaggctctcctcgtcgtagacgatttccatgccgcgcccgcccagcacgtaggagggacgcaccagcaccgggtaaccgatgccggcggcaacctcgcgagcctcctcgaaggacgtcgcggtgccgtatgccggagccggcaggctagctgcctcgagcaccttgccgaactccccgcggtcctcggcgaggtcgatggcttcgggcgtggtgccgacgacgggcacgccggcgtcggcaagcttctgcgcaagccccagcggcgtttggccgccgagctgcacaatcacgccggcgaccggaccggtcgcgctctcagcgcggtagatctccatgacgtcttcaaacgtcagcggttcgaagtagaggcggtccgcggtgtcgtagtcggtggagacagtctccgggttgcagttgaccatcaccgtctcgtagcccacacgcgacagctcgagcgcggcgtgcacgcaggagtagtcgaactcgatgccctggccgatgcggttcgggccggagcccagaatgatgactttgtccttgcccgagatacccgtcgcgtcgacctcgctctcggcgtcgggatcgagctcgtaggccgagtacaagtacggagtcttggcttcgaactcgcccgcgcaggtgtcgacagtcttgtaggtcgggtggatacccagcgaccagcgcaacgagcgcacaccgtcctcgccggccaactcggggcgaagcactgcaatctgggcgtcggacaggccgtacgctttcgcctctcggaggagggaggcgtcgagaacgggggcgtcggcaagcaaagccctaaactcgacgagcgactcgagctctgcgaggaaccacgggtcaataccggaggcttggtaaatctcgtcgatgctggcgccgaggcgcatggccaactccacgtcgtacatgcgcttgtccgtgggcaccttgaggtcttcgagcaccgcctgcttgtcctgcgcgcgctcgccggcgaagtactcgtccggcttcgtccagaacccgttcggcttgtcctccatcgagcgcatgaccttgttcaggccctggatgtagttgcggccgatccccatggcctcgcccacggccttcatcgaggtgcccagcgtctcgtcggagccggggaacttctcgaaagcaaagcgcggcatcttcacaatgacgtagtcgagcgccggctcggcgagcgccgtcagcgcgccgccggtgatgtcgttttcaatctcgtcgagcgtgtagccgatcgccaggcggacggcgaccttcgcaatcgggtagccggtggccttagacgccaacgcagacgagcgggagacgcgcgggttcatctcgatgacgatcatgcggccgtcttcggggttgatggcgaactggaggttgcagccgcctgttctcacgccgacctcgcggataatggccttgccctgctcgatcatcttcgtcacctcgggctcggtcatggtgagcacaggagccacagtgacggaatcgcccgtgtgcacgcccattgcgtcgacgttttcgatggtggcaatggtgatgcagttgtcgtccttgtcgcggatgagctcgagctccatctccttccagccgaggatcgactcttcaatgagcacgttggcctcggggctggcggcgagaccgtcgccggcgatgcggtgcaggtcgtccatgtcgtaggccaaacctgagccgagaccgcccatggtgaacgacgggcgcacgacgcagggaaagcccagctccgcaaccgtgtcttcgatctcctccatggtgtagcagacgcgggagcgggctgattcgccgccgaccttctccacgatgtccttgaacttctggcggtcctcaccgcgctcaatcgcgtcgatgtctgcgccgatgagctccacgccgtgcttgtccaggatgcccaggcggtccagctggatcgcggcgttgagcgccgtctgccccccgagggtaggcaggatcgcgtccaccgggtgacccaactccgcttcgcgggccaggatcttgtccatgtactcgggttcgatcggctcgacgtaggtcgcgtcggcgaactccgggtccgtcatgatcgtcgccgggttggagttgaccaacgtcactcgcaggccctcgtctttgagtacgcggcaagcctgggtgccggagtaatcgaactcgcaggcttggccgatcacgatcgggccggaaccgatcaccatgacgtggttgagatcttcgcgcttcatttacttggtctcctcgctggcttcaacggtgatggtggcctgctgcgggccagtcttggaaaggtggcggaccagtttgcgggtgtccacgccgcggatgccggtcacgccttggttgcgcagctcctcctcaaaagagcgcgccgagcggtggttggatgtgaggcgagagacatcgcgcaccaccacggccgcggcggtgatcgagccgtccccggcactgtcctcgctgttccagccgacgttgccgatctggggcgcggcaaagactaggatctgtccggcacgctccggctcggtcagttcccgttggtagccgaacatatcggccgtgtgggtgcaggtgcctgcaatctctccggtgccagcttcagggcaggcgccgaacgcgaagcccgggaattcggtgccgtccgccagaaccagcacggcagggatgcggttgttgctcatgagaagtccttttccatgtgggtgatcttgccgcgcagccaggtggccacgactttcgcgttgaaatccatgccctcgtagggcgtgttcgacgccttcgacgccagctcgtcaccgcgggtggtccaggagtgctgcggatccaccagggtgaggttcgccggctccccagccgcgatgggccggccctggtcctcgagccgcaagatttcggcggggcgctcagacatgacctgcgcaacgaagcgccagtccgcgagcccaggttcgacgaacagctggtggaccaccgccagggaggtttccaagccgagcatgccgggcttggcgtgttcgaactccacgcacttgtcttcggagccgtgcggggcatggtcggtggcgacgacatcgacggtgccgtccagcaacgcttctcggagagcggcggtgtcgctctcctcccgcagcggagggttgacgcggtagacgccgtcgaaggtctccagcttttcgtcggtgagcagcaggtggtgcggcgtcacttcggcagaaacctcgatcccctgctgcttcgcccagcgaaggagggagacggtgccctcagtggaagcgtggcacaggtggtagcgcccgccgtagtcgcgcgtcatgatcaggtcgcgcgcgacaacggattcctccgccacgcgcggccagccgcgcaggccgaggcgcgcggcgttagggccctcgtgggcgcatgcgtcgccggtcatgcggtggtcctcggcgtgctgcgccagcaccacgtcgtgcgccttcgcgtactcgatcgcgcggcgcatcagctgcgggtcgtttacgcagcggccgtcgtcggaaaacatgcgcacgtgaccgcgcgccatgaggccgatctcagtgagggtctccccctgcaacccgcggctgatcgagccgaccgggtagacgtcgcacttgccgtaggcctggcccttctcccacacagcgtcggccaaaaacggctgatcgatgaccgggttcgtgttcgccatggtaaacacggcagtgaagccgcccttggcagccgcctcggagccggtggcaatcgtctcggtgtcctcgcggcccggctcgcgcaggtggacatgcatgtcaaccaacccgggaagcaggatgttgcccgcgcagtcgtaggcctcgtcggcgtcggtaaacggctgctcgctgaccgagtcgataacgccggcggcgacgtcgataagaatgttggttgcgtcctcgccgtagggccggacgttgttcaaagcgagtgtggtcacggcgctactcctttccttccagtccggtgttgccgctggccagcagcgtgaacagcacagccatgcgggtgtagacaccgttcgagacctggcctagcaccaccgcgttcgggcgctcggccacggcgtagttgatctccatgccgcgcagcattgggccggggtgcatgatcagcgcaccgtcgctaagccgatcagccctgtccttgctcaacccgtagagcgtggcgtattcgcggtgcgacgggaagaacccgccgtgcatgcgctcagcctgcacgcggagcatcatgacgaccgctgggtctagttcgatggcttgatctaggtcgtgcattacgcggcacggccagtgctccacacccagcagcaaaagcgtgggcggggcgaccagcacgacgtcggcgccgagaatggacagcaggtcgacgttggagcgagccacacgcgagtgcaggatgtcgccgacgatcaggacggtcttcccgttcacgtcgccgatgtgttggcgcatcgtcacagcgtcgaggagcgcctgggtggggtgctgatgctggccgtcgccggcgttgacgatggacgtctccggcaaccaggtgcgcaaaaggttcggcgcgcccgaggccgggtggcgcatcacgattgcgtcggcgccgattgcggcgagtgtctgtgcggtgtccttgagcgactcgccctttttcacgcttgacccggaagcggacacgttgatcacgtccgcgctcatccacttgcccgcggtctcgaacgaagaccgggtacgtgtggagttctcgtagaacagggtgaagatcgtgcgcccgcgaagcgtaggcagcttcttgatctcgcgaccgtcaagcgcctcccggaagcggtctgcctcgtccatcagcccgatgatctcgctgcgagagcagtccgcgatgtcgatgaggtgtttcattttctattggccctccttggtgagggtgacgccgtcagtggcgtcgatcggagtcaggctcaccgtcacgtcttccgtcttggcggtcgggatgttcttgcccacgtagtccgcgcggatgggcagctcgcggtggccacggtccaccagcacggcaagttggatggcggctgggcgcccgatgtcgcgaagcgagtcgagcgccgcgcggatggttcggccggagtacagcacgtcgtcgacgaggatgacggtcgcgccgtcgatctcgccggggatgcgggtgggcctcagcgcgcggtggggtttgtcgcgcaagtcgtcgcggtaaagggtcgtgtccaagctgcccacgggcactgcgacacccgaaaactcttcgatcgcgtccgcgatgcgctgcgccagcggtacgccgccggacgggatcccgagcagcatcacgttgggtattttgtcggcgtcgagcgccgtcttctcgatgatctgatgggcaatgcgcgcaatggtgcgcccgacgtcggaagccgtcaacagctccactgtcgtgcgatcttggtcgcttcgtttgtcgctcaccggacctccttccccgcctctctgtgcggaatttaaaggatgtcttcttcgtttcgggtctattctcgaaagaccgcttcgaagtttagcaccgatagttccctcctagtagatcaagaaagtgagcggcgacaagctatgggcatcgacgcaacccacctcgtgccggctgatactgacaccgtttggaagtggcactcgaggccgggtgcgctcgagcgcttgacgccgccgttccttcctatgcggccggtgcgccaggcgcagtccttacgcggcggcaccaccgtcttccagcttccgggcggcttgaaatgggtcgccgagcaccaaatcgacgggtacgttgcgggcgagcagtttgtcgacgaagccgcgaaccggccgatcaggtacgcaacagggtggcgccacacccaccgattcgaggaggctaagagcgttgacggcaccgctgccacgctggtccacgactcggtcgagtcgcgggtgcccgagttcgcgctgcgccccgcgtttgcgtaccgccagcgccagctggttcaggacatcgagttcttgcggtccctgccggagaccgagccgagggtcatcgcagtgacaggggcttccggcctggtcggcagccacctgcgcgcgcagctgtccaccgccggacatacggtgatcggtctcacccgcggcgaggccggccccggcgagcgccactgggacccggacaaccccgccgcagacctcctcgccggtgtcgacgccgtcgcccacctcgccggcgaatccatcatgggcaggttcactgaagaaaagaagcgcaagatccgcgactcccgcgtcggcccgacgaggaagctcgcccagctcgcagccgacagcggcgttgcagcgttcgtctcggcctccgcagtcggttactacggcacagacgccggcgacaatccgcacgtcgagtccgacggcccgggcaagggctttcttgccgacgtctgcgcccagtgggaggaggccagccaggtaggcggactccgcgtggtgaacatccgcactggcctcgcgctatccggagcgggagggcttttgcccgtgctcaaggcgtcagtgaacgcgggcgcgggcgcaaagttcggcgacggcgacttctggatgtcctgggtctcgctcgacgatctaactgacctctacactcgggcgcttctcgacgacatcgtctccggcccgatcaacgccaccgctccgaacccggtgaccaacgcggagttgtccgcggcgctggccgaagtgcttcaccgccccgacttcttcagcattcccgcattcgggccgaagctactgctcggtgcgcagggtgcgaaggagctggctttggccgaccagcgcgcagtccccgcccgcgctgaggaggcaggctgggcgttccggtacccgacgctcggggcggcgctgcgccacgagctgggcaaggagacgctgctgggcttcgccccggggacggtgtcaactggcgttgatagcgggtaactcgggggcgtttcgcgtttccccaggtcgccgctcggctggttgagagttacccgctatcagcgcgcggcggcggctaagctgcggcggctagctgccgcccccggggcggtgttgttagctggcgttgatagcgggtaactcggggggcgttacgcgtttctgcaggccgccgctcggctggttgagagttacccgctatcagctcgcgccagcggctatcagctcgcggcggctagctgcggcccccggggcggtgttgttagcttgcgttgatagcgggtaactcggggggcgttacgcgtttccccaggtcgctgctcggctcacggggagttacccgctatcagcgcgcggcggcggctatcagctcgcggcggctagctgcggcgaagctcgcgcataagttcggtgagctcgccgccgccggccatttcccgggttagctcgtcaagactgacttcgctgcgcggcgcgtcgagcacctgcctgcctagctgcaggatggtgaagcggtcgcccaccaaatacgcgtggtgcgggttgtgggtgacaaacaccacggccacgccttggtcccgcgccgccgcgatgaacttcagcaccatcccggactgcttcacaccgagggccgcggtcggctcgtccagcaccaccacgcgcgcgccgaagtagattgcgcgcgcgatggagatcacctggcgctgcccgccggacaggtttcccgcctcgacgtcgacgtccgggatgtccacgcccatccgcctcaactgttctgaacagatgcggcgcatctcagcctggcgcagcaggccgaagcggccggtgagttcttggccgaggaagaagttgcgccacacactcaaggaatcgaccagcgcaagggtttggtgcacggtggcaatccccgcgctcagtgcgtcgcgtggtgagctgagggtggttggggtggcgtcgataagcacctgcccctcggttggctggtgcaaccctgccaggatcttgatcagtgtcgatttgcccgcgccgttgtcccccagcacgcaggtcacctcgccggggttgaccgcgaggttgacgcctcgaagggcctgaaacgcgccgtagtccttggtgacgccgcgtagctcaatgactgccatggatcagcgccccttggtgaagttggcaaacgtagtgttggtcagcaccgcaaacagcaacatcgcgccgaggaagaacttgaaccagtctgggttccaccctgcgtagacgatgccctggttggtcatgccgaagatcagcgcgccgatcgcggtgcccacggcggtgcccctcccgccggtcatggcgcatccgccgattaccgcggcgatgatgtagaggaattcgttgcccaccccttggcccgcctggatcgagtcgaaagcgaacagcgtgtgcatgcccacgaaccaggcggcgaacccgaccgtcatgaatagcgcgatcttcaccttgcgcaccggcacgccgacggcccgggccgcgtcctcgtccccgccggatgcggtgatccagttgccgaacttggtcctcaacagcacaaccgacgcgacggcgacgaaaagcgcccaccacaccaccattacgctgatgcgcacgccacccacggtgaaccagccggcgaagaaccggcgcgcggagggaaacccctccatgtccgcgatcgtcggcgtagcaacctggccggtgacgagcttggttacggccaggttcaacccctgcagcatgagaaacgccgcgagcgtgataaggaagctgtcgatgccggttcgcgtgactagatagccgttgagtgcgccgatgcccagcgcgatggcgagcgatatcgccgcccccacccacgagttgaggtggaggttgtagttgagcatcgtcgcagcgagcgccgcggtggtcaccgcgacaccggaagataggtcgaactcgccgccgatcatgagtaacccgaccgcaagcgcgacaatacccagcgtggagctcgcgtacaggatggtcgcgatggcctcgagcgagcgaaacgccggggcgaccgccgtaaacagggcgaaaaggacgactaagcccagcaggctggcgagctcgggccggcggacaacgcgcgcaaccccggtgctggagcggagtcgatcgtcgccggtcaccgcaaacccgccttcgcggcgtcggcgatgacgtcgacgtttcccgcgtcgacgaaactcgggccggtgtacacgggctgccctccgccaagcgccgcgccgttgcgtttcgccagccataacgagtccaccgccaggtacccctgcacatacggttgctgatccaccgcccacgccacgcgaccgtccttgatcgcgccgacaagctcggcgttggtgtcgaaggtaacgacctgggccccagcgcctgcctgcgcgaccgcctccgccgcccgcagcgccaccggtgcctgcaaggcgaagacggtgtcgaagctcgcgtcctgcgcgagcttcgacgtgatggtcgactgcgcggaggtgaggtcctgcccgttgacgtagagcagctccacccgcccgtcaaggccagagcgcacgccgttgcagcgcgcctcctgagatacgttgccctgctcgtggatgacgcagagcacgttgcgcttgccctcgtctttcaaccgctcgcccgcggcggtgccggcgacggtttcgtcttggccgaagaacccgctcaacccgtagtcggcgtaccggtccatgccggcgttcaacccgacgaccgggattcccgcgtccacggcactttgggccgcggggccgatcgcgtccgcgttcggcagggtgacagcgatgccgtccacgcgggcgtcgacagccgaacgcaccagattagcctggttcggtgcctgggggtcggaggagtacctcagctcaatattgtccttcttcgcggcgtcctccgcgcctttgcgcactagatcccagtacgtgtcgccgggggcgccgtgggtgaccatagcgacgacgtagcgcggagtgtccaccccgcccaccgcttcacccgccgggacgctgcggggagcaccgcctgtcgccgagcaccccgctgcaagcgcgacaccaagcgacgcaagcattgcggcggtcttcttccagattgttctcacggttccatcttggccggtggcgcccggcaatcccctcttgtcgacgctctgaaccgatacagaagctgttgggtacccttaggggccatgactgacccgcttgagacagcgccagatccaaacgaggtccgcgacatcgccctcgccgacgtggtcgcgatcctcgaggacgagagcctggagtaccggctggaagaggcggtacttcgcaccggattcgtcaacgccgcgatcgcgttcacgatagaagaccacaagctgcttttcgaagcagcttggcgaggggcatttgcgcttgccgacgcctcctccctcctcttcgccaccaacgagtacaaccaaacccgcttcaccccaacgctgcgcttctttcagagcgacgaggacacgctcatggtgaccggcgttcgtgcgatcgatattgggcggggtctgagcaccaaccagctcggcaccttcgttctcacctcgatcaacgccgccatggaggcgttcgactttttggcggcgtccttccccaccgccgtgacctgggaggagacccgatgaccgcaccgaagctcgtgaccatcgaccgcatcgccgagacatgcgctgcagcgggcatcgacatcaccccggacgcgaccgggcgcgcagcccacggcacccacgagggattacccttgctcgtggtgctcttggactccgtgtttatcgtgcgcgcagactccgcgaccgacacccccaccgattccccggacgcgacgtactacctcgccgcgaacgaggtcaacaccgcgatgatgggtgcccgcgcagtggtggcgaacaagggcgaggtaaacgtcattcgcaccgaagccgaagtaccctgcgctgccggcctgacagacgagcagctggcgttcgctgcaacccaggcggttgcctcggtggttgaggcgcacaacgccatggtggtcatgtgcgagcagatccgcgcggcgcgggaggccgcagctgaggagggctaggactcggcgaggcgccgcaactccacctcggggtcgaagtcagcttcgggccagtcgaggcccagcgagacaagcgcgtcgcgcaagagagtcttgacgacggtgcggcaatacttcttgttgtccgacgggatgcagtaccacggcgcgacgtcggtggacgtccgagtcatcgcgatttggtaggccgccatgaactgcgaccacagtttccggtcgtcgatgtcgctggggttgtacttccagtgtttcttggggttctcgatgcggttgcgcaggttttccgcctggaactcgcgcgagatgtgcggcatgaccttgatgattttggtgccgcgggcggccagatcggcctcgaagtcgacgatggcgccgtaacgacgctcgatctcctcaggcggcgccatctgcttgactcgctgcaccagcacgtcctcgtaatgggagcggtcgaagaccgagatctggccgggcttcggaaggtgcggctcaaaacgccacaggaagtcgtgggacgcctcctcttccgtcgggcgcccgaacgcttggacgtgcaccccctgcaggtccatcgtctcgccgatgacgtggcgaacaatgccgcccttgccggcggtgtccatcccctgcagcaccaacagaattgatccagcgtcctcgttgcctgcacggccgttggcgtacagcttctcctgcagctcgtcgagctcggagtcgaggcggtggaacgcttcgtcgatgtcgtcactgccttttaggccaggcgtcgaagcggggtcaacgtccgcgagctggaagttcggcccgaccttgagagattgggcctcctcagagctgagcttcgccatcgccctcaccgtcagtatcggcgtcgacttccccgggcgcatccgcggattgcgcctgcgtgatcccgtcgagcatcgcgtggatgtacggcggggcttggttgccagagtactccgttgccatctccagcgcgttcgcgatagcgatcgccggaggcacctcctcgttgaacaggatctcccaggtggcaacgcgcaagatctggcggtcaaccgcaggaagccggtgcagctcccaatcacggtcgaggaaacgttcaatctggtcgtccagatcatcgagcttctcagccgcgccgcacacgatatcgcgggtgtagtcggcgatcggcgcaactgcgttttgcgggtcgcgggccagctcggtgcggtcttccacgatcgacaccgggtcgacgtcgcgggtttccgcctcgaagaggatgtctactgctctgcggcgcgcgcggtagcgggcgccgtgacgtttgtagtcgggcattagttgttcacgcgggagaggtactcgcccgtgcgggtgtccaccttcactacgttgccggtctcgaggaagagcggcacctggatctcggcgccggtttccagcgttgctggcttggtgccgccggtggagcggtcgccctgcaggcccggctcggtgtgctcgatgcgcaggtccacggagatcgggagctcgccgaagagtgcctcaccttcgtggaaagacacctgaacgcgcatgttctcaagcaggaagcggcccgcgtcgccgaacgcttccggggagagctcgtactgctcgaatgtcttgtcgtccatgacgacgaagttggtgccgtcgttgtacaggtaggtcatgtcgcggcggtcgacggtggcggtctctaccttcacaccggcgttccaggtcttgtccacggtcttgccgctgacaacgtccttcagcttggtgcggacgaaagcggggcccttgcccggcttcacgtgctggaactcaacgatctgctggagttttccgtcaaccttcagcacgagaccgttcttgaaatcggcggtagttgccacgggggtacctcccaaatagagaatgcgagcaaacaccgcaatgctacagcacgatcaaatccttcgggtattcggtaatcacccgcggcgccccgtccgtgattacgagcgtgtcctcgatccgcaccccgccgcgtcccggcacgtagatgcctggctcgatggtcagcgtcatgtccttggccaactcgcccttgcctgtcgccgcggcccacggcgcctcgtgcacctcaaggccaacaccgtggccggtggagtggacgaagtactcgccgaacccggcctcgtcgataacctcccggcaggcgcggtcaacgtccgcgagcgcggtgcccggggtggctgctcgcacgccagcgagctgggatgcgagggtggcctcgtagatctcgcgcaggaactcctccggctcgccgatcgcgaaagttcgcgtcatgtcggagttgaagcccaagcggtgcatgccgaagtcgatcgtgaccaggtcgccctgctccagcgcgcggtcgccggctgagtggtgcggcattgcggagttcggccccgaggcaacaatcgtgtcgaaacttggccgctccgcccccagcgtgcgcatccggtactccagatcggcggcgatctcgcgctcagagcgacctgagcgcaccccgccttcctcgatcaacgccgccaaggcctgcgccgcaagctccgcagcctcggtcaggcgcgtgatctccaggttgtccttggtcaggcggatgtcttcgataacgccggtgaccggcaccagcgtcaccccctccgggcacaccttctcaagcttctccagcgcggtgacgctgaggtagtcggcctcgtagccgatgcggtagccgtcggcgacgccttccagcaactccgcgttcagctggcgcgtgaccgtcgcctcgatgtccggcacctctgcggcgatctgggtggtgtagcgcccgtctgtcgcgatgcgcgccgagcggtccttgaacaccatgagcgccgcgttggagccggtgaagcccgagaggtagcggacgtgcaggaggtggctgactaacaggccgtcgaggcgcttcgcggccagctcagaggcgagcttgcggcggcgggtttcaaaacgggtgtcggccatggacatggtctatcgctcctttgctaaatactcgagtgctaggacgtaaccgcgcgcgccaaggcccgcgatcacgccgatcgccagcggcgacaggtaggagtggtggcggaacggctcgcgcgcgtggacgttggagaggtggacttccaaaaaccccgcgccgtccgcaacctccgccagggcgtcgcgcagggcaaccgaggtgtgggtccagccgccggggttcacaatcactggccacgcgttatcggctgcctcgtgcacccactcaagcatgacgccttcgtggttggtttgacggaagtcgacctcgacgccgagctcggcggcgcgggcgcgcaccatttgctcgacgtcgtcgagcgataaggatccgtagacctccggctggcgcttgcctaggcggttcaagtttggtccgttcaggacgaggatcgtcatgagtggcctgcctccttctactggcgcgtcaccgcggcgtacgcggcgcgcatttcgtccacagtcgcgtcttcaagccgggtgcaggaaccgagaccgtcgagcaccacaaagcggatccggccgtcgcggttcttcttgtcgtgggtcatggcctcgtagagctcgtcgaaggcgtccgggtcgtaggtcaccggaagaccgacggtggcgaggatttcgtggtggagggcgtacagggggtcgtcgataagctgcctgcttcttgccagctcggcgacgaacatcatgcccaccgcgacggcgttgccgtggcgccagcggtactcctcgcggcgctcaatggcgtggccgagcgtgtggccgtagttgaggatctcgcgcagcccggcctccttcaggtcctggccgaccacgttcgctttgaccgccacggagcgctccaccagctcctcccagtgcttgtctgcgccgtcgcggtagagctcgaggatgaccgggtccgcgatgaagccggtcttgatcagctctgcagagccggagacgatctcctcctcaggcagggtgtggaggcgttcgaggtcgatgaacaccgcgtccggctcgtggaacgcgcccaccaagttcttgccggcggcggtgttgatgccggttttgccgccgacggcggcgtccaccatggccagaagcgtcgtcggcacctggataaccttgatgccgcgcatccacgcgctggcgacgaaaccagcgaggtcagtcgcggctcccccgccgaggcctacaatcgcgtcttgccgcgaaaaccctgccgcgccaagctcgtcccatagctcgccggcgacgctgagcgtcttgccgctctcggcgtcggggacgggcagcagcagcggttgcacgcagacagcctcaaggtcgctggcgattgcacgggcgactgccgcgagcggctgttggtagacgacggcgaccttgcgcgctcccgtggatttcgcgtggccggccacttcacccgtgatgtcgtagccgatgtggatgttgtagggattcggtcccgtcacttcaatcgtggccaaaatcgcacccctattccgtatcgatgaagctcaagacctccgcaaccacgcgctgcggcgggcgggagtcggtgcgcacccggtggtccgccacctcgcggtagaacggctcccgggtttcgagcaggttgcggtagtgctcctcgcggtttgcggcgttaagcaccgggcgtgacgtgtcgtttgcggtgcggcggatcccctcttccggggtgacgtcgatccacaccacggtgtgccgctgcagcagggtgcgggtggactcggtgagcaccgatcccccgcccaggctgaccacgccgccagtcgccaacgcccgggcgacgtagcccgcctcgagcttgcgaaactcttcttcgcccagctcggcgaagacctcgccgcagggcttgccctcaccctgctcaatcagcgtgtcggaatccaccagcgggaggttcagcgcgctggccagccggcgcccgatggtcgatttgcccgcgcccggaggcccgacgaggaccacccgcgggaaggaattcaccatctgcacaccttcgtgcgcaggccgtgcctgctcctcgggtgtcttctcgggggcatcaatcatcatcgatcaccttcctcgggcgccgcgtcaaacgccaggcgctgggccacatactcgttgtaggaggctacattgcggcgcacctcttcgagggagtcgccgccgaacttctcggtcaccgcgcgcgcgagcacaagggcgaccattgcttccgcaaccacgcctccggcaggcaccgcgcagacgtctgagcgctggtggataccggtggccgcgtcgccggtggccatgtccacggttttcagtgcgcggggaacggttgagatcggtttcatggccatgcggacgcgaagctgctcgccgttggtcatcccgccctcgagcccgccggcccggttggtgaggcggcgcagctccccgtcttcacgcaccatctcgtcgtgggcttgggagccgcggcggcgggcttcttcaaagccgtcgccgatctccactcccttgacactctggatgcccatgagcgcactggcgagctgcgcgtccaagcggtgctcgccggaaatgtgggagccaagcccaaccggcaagccgtcgacgatgacctcgatgatcccgcccagggtgtcgccgtccttcttcgccgcctcgattcgggcgaccatgtcctcttccgccgctttgtcgtaggcgcgcacgggagaggcgtcgatcgcgtcgatgtcggcgaacgtcggcctggggccgtcgtatatcgcggactcaccgatagacaccacgtgcgagaacacctcaacgccgagcgtttcacgcaggagggaccgcgcgacggacccagctgccacacgcgccgcggtttcgcgggccgaggaacgctcaagaaccgggcgcgccgaggtgaagccgtacttgatcatcccggcgtagtcggcgtggcccgggcgcgggcgggtgagctgggcacctcgaccggaccccatcgccttcgccacttccgggtcgtccatatccaccggctccgcggacatgatggtggtccacttcggccattcggtattgccgatctcgatcgcgatcgggctgccgattgcctgcccgtgcacgataccggtcagaagggtcagctcgtcggcctcaaacttcatccgcgcgccgcggccgtagccgaggcggcggcgcgagagctggtgcgcgacttcttctttggtcaccggcaccccggccggcacgttctcaacaagcgccacgagcgcctgtccatgggattctccagcggtggtccaacgaagcattgctgcattgtctcacacagcgccgatgaagagtgcattaacgaacacgagccaaaaggcggcgatcatggacggtccatgcggcacctcgcgcttgcccgcggaaaccgcaaccaggcaggtgaacagcgcggacagcaccattgcggccaccaccgcacccgggccggtggagaaggcgagcgcgacgccgagcggcagcgcaagcttaatgtccccgccgccgatgccgcgcccgaagaacaggtaacaggcgggccacgcgaacccccagagggcatatggcttaacgacgcatcccgcaaccgcaacagcgcacgccggcaacgtgaggacgtcggggaggcggtggcgggtagcgtcgacaagcaaaagccccaacgaccagcaaagaaccaacccccaccccatagctggcagcttagcgctgcgctgccacgtgtgtgaagagcgcggcgcgcattgcctcgcgtggggcgtccactgaagtgaactgctcgaactgggagtacgactggcctgcaagcatgctcaggcccccgacagcgtggtagccgtggctggcggcgcgtaccgcgagcggcgtcggccacgggttgtagatgacgtcgaggatcggcgcgtgggcgagatcgttgacgtggtcggcgacgccggcagacggcacagtcgagatcaccgcgtcggcagccatggtcagaccggcgatgtcggtgcgcgcgtccagcggcgcgaacgcgacgtccatcccctcggtcagcgacgcaagctctgcggagcggtcggagcggttcagcacggtcacgtgttcaactccgagggatcgcagcgcccacagcgccgggcgcgcggtgccgcccccgcccacgacgacagcgctggtgatttgctggccgcgcatgagctcgtccagcgcgatgagcaacccctcgcagtcggtgttgtcggcgcgccacgtgtcagcgcccgtgcgcacgagcgtgttggcggatccgatcgcgcgggcgcgctccgtcacctcgtcagcgaagtccagcgccgcgaacttggcgggcatggtgacggagaaaccgcggtagtcctcccccgcgccttcgacggtctccggcagcgcttccgcggtgcactcaatgcgggtgtactcccaacccgaaaggcccgctgccttataccccgcgttgtggagcactggggaaagcgagtggctgatcggcgagccgagcacagccgcgcgaaacgtcatcgctgcgagtccaaaacgccgttctggatggagcgctcggtgtcggcgaagtgctcttccagggtgtcgttgaacaccgtggtgccgtccttgtcgacggtgacgaagaacagccagttgccctcagccgggttctccatcgcctcgatcgcttccatcgacggcgaggagatcggcgtctgcggcaagccgtccatggcgtaggtgttccacggggtgacgcggccgcggtcggcgtcggtggtcgcaacctccacagacggcagatcgtagttcacggtcgagtcgaactggaggcgcatcggctcatccaggcggttcaggatcacgcgggcaaccttgtcaaactctcctgccggcgcctcgcgctcgaccagggaggccgccaccagcagctcgtacggcgtcagcccgatcgcctgggcgcggtcgacaatgccagagtcgttgtagagcttggccgagcgcgtcaccagatccgtgatgatctcctcggcgcttgcctgcgggttgatgatgtagtcgcctggggcgatgagaccttcgaggcgcttcgcgtcgccttggcgggcgtttaccgtctcgagcgcccactctggcacgccgagcgatgccgcgtcggcgttggcggcgaccttgttcaactgctcaatgtcgacgcagccgttcatgttgtcaccgccgcaggtcacgtcctgaatcatcgagaggatgccgtaacgggtctggccgccgagaacgttgatgtccatcagggtggcgccgccgtacaccttcagcggggtgaccatcttgtccgggtcgacgagcgcggccacggcggcctcggcgctcatctccccctgcaggcggtagaacccggggtggatgttgtcggattccgggttgttcgccgcggcagtctggaacgcgccgtcggatgcgacaacgccgcgttccacgagctccggcccgagcgccgaaatcgtcgagccctccttgatttccacgacctgctcgacgccgttgccgtctccggtgaaatcgtccggggcgccgttctggcgcgccaccgcgatccatgcgataaggccgatgatgagcagaatcgaggcgatcagcagcgcagcgctgcgtgtccgcccttgggcgcttcgtcgggtggtcacgattcgttctcctttagataggtgtttcgcccgtccaaccaagattggaggatctcgacagcggccgcctgatcgatgaaagaccgcgcgcgcttctccgacgttcccgcagcgcggatcgcctgggaggcaacgacggtggtgaggcgttcatcggccattttcacaggcaacccggtgcggcgcttgatgcggaaggcgatttccttcgcgtgcttgacactcttcgagccgttcccctgcaaatctcgtggcagacccacaaccacctcgaccacgtcgtagtcgttggtgagctgcacaagacgatcgatgtcgtcgccgtcttggtccttaaagccagtgacccgaggcaccgtttcaactgcggtggccaaacgcgcgtcacggtccgaaaccgcaacaccgatgcgcacagtgccgacgtcgacgccgaggcgtcggccgttaccggggtcgtcgacccctggcgcatctggctgtaccttcatcgtcatcgcctttcgggttgggctttccaaccaaactaatgctggataacgcctgaacgtacccgaaacgccgacttgggtgtaaccaattcgttacgtggctaccggccaagttcctcgcgcacggctgcgagcgcttggtcaatcccctcgggtgcggagcccgagccctgggccaggtccggcttgccgccgcccttgccgccgacgtacccgccgacgagtttgaccaggtcgccggacttcacaccgttcgccacggcatcctgggtggcagcaaccgcgtacgctgccttgccgccgtcgttcgacgcgagcaccaccacggcatccccgccgttgagcttgccgcggatatcacctgccatcgtgcgcaggtcgccggtgttgattccgtccggcaagtggacggcggcaagcttgcggccgctggggagggtctccgccttgcgggcgatgtcgcccgtgttggccaaaagctgcgcgcggtgcagggcctcgatctccttctcagccgcgcgcaggcgctcggtgagctgcgcgatgcgctctggcagctggtcgctcggcgtcttcagctcgctggccaggccggaggcaagcgccgcctccttggagaagtagcggaaggattcgagacccgagtacgcctcgatacggcgggcccccgaaccaaccgaggattcgccgagcacagcaaccgggccgatctgggacgagtggtccacgtgcgtgccgccgcacagctcgatggagaacgggccgccgatctccacaacgcggacgcggtcgccgtagttctcgccgaagagcgccatcgcgcccatcgccttcgcctcgtctaaggacgtctcgatggtgttgaccgcgaagtcggcgtcgaccgcctggttggtgatcgtggcgatttccgccagctgctcatcggtgagttggtcggtgtagttgaagtcgaagcgcaggtagccgggcttgttcagcgagcccgcctggaccgcggtggggccgagcacctggcgaagcgccgcgtggatgaggtgggtcgcggtgtgggcctggcgcgcgccgtggcgccacgcgccgtcgacctccgcggtcaccgtctggccgaggtccagcccgccgttttgcaccgtcgccttgtgcacccacagcttcttgccgattttctgcacgtcgttgacgtccagcacggtgtcgccgaccagaagacggccgcggtcagccatctggccgccggcctcggcgtacatcggggtgacgtccaggatcacctccacctcgtcgccttgggcgacctcgccgaccttctggccgtcgcggactaggccgatgacgttcgcttcgtgcaccagctggtcgtagcccacaaacttggtcgggtgctcgtccacccacttgcggtacagcgagtcgtcgcggttacccatcttcttggccttgttgtcggcctttgcgcggtcgcgctgctcctgcatcgcggcatcgaaggcctccatgtccacgtcgaggcctgcctcgcgggccatctccagggtcaggtcgatcgggaaaccgtaggtgtcgtgcagctcaaaggcctgcgcgcccgtcatcacggtgctgccggcggtcttgagagcctcagccgtttcgtcgaagcggtgggtgccggactccagggtcttggaaaatgcgcgctcctcagcaagagcgacgcgcaggatgcgctcgcggttctccgcgatctcggggaacgacggcgtcatcgtgtccatgatggtgttcatgagcggctgcatcacctcgccggtggcccccagcaggcgggcggaacggatgatgcggcgcagcaagcggcgcaggatgtagccgcgcccctcgttggacggggtcacgccgtcgagaatgaccatcatggcggtgcgcgagtggtccgcaatcacgcggaagcgcacgtcgtcagccgggttgccggtgtcgtagcgcgtgccggtgagctcctgcgccacgtcgattacggggcgcaggaggtccgtctcgtagacgttgtcgacaccctgcagaatgcacgctacgcgctcgacgccgaggccggtatcgatgttcttcttcggcagctcgccgaggatctcgaacccgcccttcttgtcgccggcgccgcggatggactccatgaacacgaggttccagatctccatgtagcggttgtcgtcggcaagcggaccgccctccttgccgtactccgggccgcggtcgtagtagatctccgagcagggaccgcacgggccaggcacacccatggaccagaagttgtcctccatccccatgcgctggatacgctcagctggaacaccgacctcgttctcccagatgctggcggcttcgtcgtcgtcggtgtagacggtcacccagagccgctccgggtcgaggccgtacccgccttcttccaccgagccggtcagcagcgcccacgcgtgcttgatcgcgccttccttgaagtactggccgaaggagaagttgcccgccatctggaagaaggtgttgtggcgggtggtgatgccgacttcctcgatgtccagcgtgcgcacgcacttctggatggaggtggccaggccgttctcgaacggcggggtctgctgacccaaaaagtacggcttgaacggcaccatgccggcgttgacgaagaggagtgtcgggtcgtcgaggatcagcgacgcgctcggcacctcggcgtgaccggcctcgacgaagtggttggtgaaccgttcccgaatctcatgtgtctgcacggggtgtacgtcctttcagctgattggaaaatccggcataactctaccccgctagttcccgcgcaccatgcgccggagcctgccaaggtactcgctgatgcgtttctcggccccgtggtcggtcggctcgtagtacacggcgtcttccaaaccgtccggaacgtactgctgctccaccactccccggggatcgtcgtgggggtacttgtagccgacggcgtggcccagcgccttcgcgccctcgtagtgtccgtcgcgcaggtgcggcggcaccggccccacgcggccagcgcggacatcctcctgcgcccgcgtgatcgcctggatcaccgacggcgacttcggcgcggtggccaggtggatcgtcgcctgcgccaaggtgagacgagcttcgggcatgccgatgaactgcaccgcttgggcggcggcggcagcggtctgcagcgccgtggggtccgccatgccgatgtcctccgaggcgtgaataactaagcgcctggcgatgaaccgggggtcctcccccgcctcgatcatgcgcgcgaggtaatgcagcgcggcgtccacgtccgacccgcggatcgatttgatgaacgcgctggtgatgtcgtagtgctggtcgccgtcgcggtcgtagcgcaccaccgcgcggttgacgttttgccgcaccacgtcctcggtcacggtgccgcccgcgggcaccgcttccgcggcagcctccaaatatgtcaacgcccgcctcgcgtcgccgccggccaaaagggtcagctggtcgagggcctcaccgtccaccaccacgtcgagcgcctcgtccacggcgcgacgcagcacggcgcggatgtcgtcgtcgctcagcggctccagcttcatcagcagcgagcgcgacaacagcggcgccaccaccgaaaaactcgggttctccgtcgtcgcggcgaccaggagaacggtgcggttctcaaccgccgcaagcagcgcgtcctgctgggtcttagagaaccggtgaacctcgtcgatgaacagcaccgtcttctcgccgcgcacaaggtcgcgccgggcctggtcgatcacggcgcggacttccttcacgccagatgacagcgccgagagcccgacgaagttctgccccatcgtctttgcaatcaaagaggcgatcgtcgtcttacctgtgccgggcgggccgtaaagaatcacactcgccgcgccggatccttccaccagccgccgcagcggtttaccctcgccgagcaggtgctcttgccccgcgacctgttccagggtctgcggccgcatgcgcgcggccaggggtgcgtcgctcgagacttcgaagaagcttgagccccgctggcttatcgacgcccccttatccgccccttcatccccaaacaatccgccttgcgtcatcgccgcgtctgtctccgtctacgccaaccgcgcggcgacctgggccgcaaaatcagagataaccaggtaggcggtgtcgcgcccggtgcccgcgtagctggcgagcgcgttgaacgtctcgcgcaggtcctcgcggacaagttgctcctcgtcggtaaacggcccctgagacgccgggcgcagcacgtcgcccgaggcgtcgaagtcgagctggtccaccgcttcggaggtcagctcgaggccagcgcgggcgaactccgcggcgagttcggtgtctgcctcactcaactgccggaaagccaccgggttgagcatgctcagactagacagcgcccagccgatcatcgcgcctgtgatgcgggcttgcagcgtgtcttcgtggttgagcagcggccaggtttcgcgcacctcgcgcaaccaagcgtcgatgaacgcccccgccgcctcgtcgctgtaaggccgcggggagacgtagagcgggaaccccgtcaagacgaaggcgacgtcgaaagacgcatcgcggaaacctgcccactcgtagtccaggaactgggtaccgctcggtgtgtacaagacgttgtcggggctcagatcgaagggggtaaacgcgcgcaagccaccccgcagcaggcgcgactgcaggttcgccgccgcgaccgacacctccgccggaacgtcaaaaccggcgtttgccagcatcgacagtcccaagcggattcggtgggacagcaaccgatcgcgcacgcgctgcacttgctgcgcgtctgtctctgcccgcgtcatgcgcgcgaacaagacgtcgaaggcctgctccttgccggcggtgccggcgtgcatgcggccgagcgcggtgccaaggttgcgcaggatgttgatgtgctgctcctcgtcagcgcgctccagcatctccgcgagggtgtcgcagtcgccgacgtcggagagcacgatcatccgctcgtccatgtcgtaggccagcagcaccggcccgggccggacatcgctgctgagagacgtcgcgaattgatacgacaccacttcgcgtagaaacgcagcgtcgtcaagcgggaagcccgttgtcggcgcgtgcttgaccaccaccgaacggtgctgcaggaacgggttcgttgccaccttggcccggtagacggccgcgacgccggaaccggacaggcgggccacatcccccagtttctgcgtgccgccgtagcggcgggtcaggatgtcctcagcgaccgcgatcgccgcgtcctggtccatgtgcgctacctactcggcggtgccttcagccggcgccttcttcggcttgaagtccacaccggtctcggcgcgctgggctgcagggatcgggcccggtgcgtcggtcagcgggtcgacgccgccgccggacttggggaacgcgatcacgtcgcggatcgagtcgaaaccgccgagcaggctgacgatgcggtcccagccgaacgcgatgccgccgtgcggcggggcgccgtactggaaggcgtcgagcaggaagccgaacttctcctgcgcttcctcggcgccgatgcccatcacgtcgaacacgcgcttttgcacgtccgcctggtggatacggatcgagccgccgccgatctcattgccgttgcagacgatgtcgtaggcgtaggcgagcgcctcgcccggctccttgtcaaaggtgtccaggtactccggcttcggcgaggtgaacgcgtggtggacagcagtccacttggagtggcccagagccacgtcgccggaagccgttgcgtcagcggccggctcgaacagcggcgcgtccacaacccaggtaaacgcccaagagccctcttcgatcaggtccagcttgcgggcgatctcgccgcgggcggcgcccagcagcgcgcgggaggccttggtgtcgccggcggcgaagaagatcgcgtcgcccggcttcgcgtcgacgtgcgctgcgattcccgccttctcctcgtcggtgatgttcttcgccaccgggccagtcagctcgccgtcctcctgcaccaggatgtacgccaagcccttggcgccgcgctgcttcgcccactcctgccacgcgtcgagctggcggcgcggctgggaagcgccgccctgcattacgacagcgccgacgtactcggcctggaagacgcggaacgtggtgtccttgaaaaactcggtgcactccaccagcgggatgtcgaagcgcaggtcgggcttgtccgaaccgtagcgctccatggcctccttgtaggtcatgcgcggaatcggagtctgaatgtcgtacccgataagcttccacaactcgaccaggatctcctccgccaacgcaataacgtcgtcctggtccacgaaggaggcctcgacgtcgagctgggtgaactccggctggcggtcagcgcggaaatcttcgtcgcggtagcagcgggcgatttggtagtagcgctccatgccggagaccatcagcagctgcttgaacagctgcggggactgcggcagcgcgtaccaagaacccggcttcaaccgcgcgggcacgaggaagtcgcgcgcgccctccggggtggagcgggtcagcgtcggggtctcaatctccacgaaatcgtgggagtcgagcaccctgcgcgctgcctggttcaccttcgcgcgcaggcgcatcgcgttcgcttggcgctcgcggcgcaagtcgaggtagcggtacttcaggcgggtctcttcgcccacctcggaagacgatgcgtcctcgatctggaacggcagcgcagcggacttgttcagcacttccagctcggtcgcgttgacctcgatctcgccggacgcgaggttcgcgttcgcggagccttccggacgcggctcaaccacgccggtgaccttcaccacgtactcgcttcgcaggtcgtgggcagcctcggctacctcggactcgcggaacaccacctgcgccaagccggagcggtcgcgcagatcgatgaagatcacgccgccgtggtcgcgtcggcgcgccacccagccggtaagggtgacggtttgtccgtcgagttctttgttcaagttccccgcaaggtgagtgcgcagcacggcttaatccacgtccttccacgtgatggcaaaagttaacgggcaagagtctaccgcgctgggttaccaacatgcgttggggatgtttggcagaatgcttgccatgacgtttagaggcaatgccagccagggcgcgaaccgccgagtgcagaccagtgtcggcggtggccgcggagccgcgggaggcggcgcgggcggactcctcgccctgccgttattgctcggcggcggcggaatcgggtccctgcttatcgtgctgctgctgttcttcctgttctccggcggcggcaattccacccagtcgcaggcgccgggtacagaccagggcggctacaacttggaccactgcgacacggccaacgccgccaacgagtacaccgactgtcttgccgcggcgacggtgatctccgtcgacgaggtgtggtcgcgcgtgctgccggagcaggccagcctcgagtaccgcgagccgggcatgcacatcttcaagcgcgacgtcaccaccggctgcggctacgccaccgcagacaccggcccgttctactgcccgcgcgatgagaccgcctacctcgacgtctccttcttcgaccagctgcaccagctcggcggcagctcgggcccgctcgcgcaggcctacgccaccgcccacgagatgggtcaccacatccagaacatcgagggcaccctgggcttgagcgattataagaacccgggcgaggattccgccgccgtggccatcgagctgcaggctgactgctacgccggcttgtgggcgcactacgcccagcaggacggcagcctcgagtctgtctctgaccagcagttgaacgaggcgatccaaaccgcgcaggcgatcggcgacgacaacattcaacgccgctccggcggcgaggtcgacccggacgcgtggacccacggttcctcagagcagcgcggcgaggcgttcatgtcgggctaccagaccggcaagatgtccgcctgcgacacgttgaaccgcggcgtctacaacagctaagcgccagcgcgatggctacccaggaaactgccgcggccgcccctcccagccgggctgtcgagttcctcgcctcgttcaacgagatcgagggctttctccgggacgcactggaggcaaagaaaaccgactcattcaagtggatgtgcacccaggcggccaagagcggcgtgctgacgcgtgggcaagcggacgacctgaaggagttcgctgaactccgcaacgccattagccacggtgagtaccgggacttcaaaccgattgccgagccgcttgcggaaacagttgcggacatacagcgcatccgggactcgctcatctcccccacgaccgcgctgcaggtggtcggccaagatcagcgggtggtgacgttctcgcccgacgccgcaatcggcgaggcgctccgagcgctcaccgagaccggccacacccagttcccgatctacgagggcggcgagtgcgtaggactgctcaccacgaacgccatcgcgcgctgggtcgccgcggagctcactggcggcgaggtggcggaatcgaccaccatacgcgaggcgctcaaactctccggccagcacgaccagccggtgtttctgccccggacagcacctgccgccgccgcggtggaggcgctcaccaccccccttgcatcgggtgcgctgccgcgcctcgccatcatcacagagcacgggaacaaggatcagcgccccatcgccgtcgtgggcgctaccgacatccccgcgctgtcagccacgttctagcaccgccaaaggagggctcatgacaacttcgacgaagccggcaaggaaacgcaacaccgtcagcgtgatcgaccttttctccataggcatcggtccctcgtcatcgcacaccgtcggcccgatgcgcgcggcgcaggcgttgatcgaggatctcggcgtccagccggcgaaagtgcgggtcgagttgcgcggctcgctggcggcaaccggtgtcgggcacggcaccgaccgcgcagtgctgctcggtcttgtcggctacactccgacgaccaccagcgccgacatcgccccgaagccgggcgaaccgatctcgccggaaggcgtgatcgaaggccccaccggcgaggtggcatacgagatggttttcaacccactccctgtggccgagcacccgaactgcctcgtgttcgacgcctgggacgcagacggcacccagctggtcagcggcaaggagtacttcagcatcggcggcgggttcatcctggatcgcgcgggcatggagaagcaccgcaacgaaaccggtgtcgctgccgtcgcgcacaccgacgcagtgccctaccccttcgacacgggcgccgacctcgttcggatctgcaacaagacggggctgacgatcgcggaggtgatgcgggccaacgaggagcacatccacagccggactgagctcgatgcgcacctggacgccgtgtgggacgtgatgcaggagtgcgtggcccacggcctgaaaacggaaggcacgctgcccggcggtctcaatgtccgccgcagggccaaccgtctgcaccggctgctcaccgccgagtacgaggcctcgacggcgcgcggtctggatgcgatggagtgggtgaacctgtacgcgctcgccgtgaacgaggagaacgcggcgcacggccaggtggtcactgcccccacaaacggcgcggccggcatcatccccgcggtgatgcactactgccgagatttcaccgacgattttgaccgggagcgcgcgcacgagttcttgctcaccgccggcgcgatcggcgcgattatcaaaaccaacgcgtcgatttccggcgctgaggtcggctgccagggcgaggtcggctcggcgtcttccatggcagcggccggcatgtgcgcaattttgggcggcaccccggcgcaggtggaaaacgccgccgagatcgcgctcgagcacaacctcggcctaacgtgcgacccagtgggtgggctggtgcaggtgccctgcatcgagcgcaacgccatcggcggggtgaaggcgatcaacgcggcccgcttagccaagcttggcgacggcaccaacatcgtcaccctcgacgacgtcatcgaaacgatggcgtcgaccggtcacgacatgatgaccaagtacaaggagacctcgatgggcggcctcgccgtgcagctcggcctgcccgtgagcattactgagtgctaatcgcctcgatcaccgcagcggcgtcgagggcgacctggcgctgcgagtggtcgtgcagatccttgagcgtcacctcgccgctttcgagctcgcgctcccccagcaccagcgcatagtgcgcacctgagcggtcggcgcctttcatcgcgcccttcaaacctcgcccgccgtaggacatgtcggcggcgatgccggcggcccgcagggcgtcgacaagcaagctcatgcgctccgaggcctcatcgccgatggcgaccccgaaaacgtcgacgcgcgagtccacgccctccaacgtcacgccctcagcctcgagtgcgagcacggtgcggtcaacgccgagtccgaagccgatgccggagaggtcttggccgccgatctgcgccatcagaccgtcgtagcggccgccgccgccgatgccggactgcgcgccgagcccgtcgtgaacgaactcgaaggtggtcttggtgtagtaatcgaggccgcgcaccatgcgggcgttgatgacgtacgccacgcccatcgcatcgagcgtcgccgtcacggtgtcgaagtgggcgcggcaaccgtcgcaaaggtggtccagcatgagcggcgcgtcggcggtcatctcgcggacctcgggacgcttgtcgtccagcacgcgcagcgggttgatctccgcgcggtggcgtgtttcttcgtccaaatccaggtcgaagaggaacgcctgcagcttctcgcggtatgccgggcggcactcgccgcagcccaggctggtcatctcgaggcggaagtcggtcagcccaaccgcgcggtagcagcggtccgcgagcgcgatcacctcggcgtcgagcagcgggtcgtcaactccgatagcctccacgcccacctgctgcagctggcggtagcggccggcctgcgggcgctcgtagcggaaaaaaggcccgtagtagttgagcttcacaggcaagtagccgcgatctaagttgtgctcgatcactgcgcgcatgacacccgcagtaccctccgggcgcagggtgaccgagcgctccccgcgatcttcgaaggtgtacatctccttactcaccacgtcggtggactcgcccacgccgcgggcgaacagcgtagtgtcctcgaacaccggtagctcgatgtgctggtagccggctaagcgggcttggcgggcaaactcgtcgcgcacgcggatgaacgtggcggatgccggcgggacgtagtcgggcacgcccttcggagcggaaagggcctggaacttcttctgctcagtcacaacgattgagcttagcgtccgcggttggcggcgcggaggtacgggttggacgcccgctcagcgccgatcgtggtagccggcccgtgaccggggagcacggtcaacgcgtcgtcgagttcccacaccgggccgcggagcgactgcgccatcgcgtccgggtccgagaactccaagtcggtgcgccccacggatccgttgaagaggacatcgcccgaaaacaccagctccttacccaccagcagcacgcagccgggcgaatggcctggtgcgtggcgcaccgagagctccatcccggcgagctgaagcgcctcgccgtcgacgatgtcgatcacgcgcgcaggcgtttccatacggctggcgttgaacgccgcgcgtccggcgctgggtaccgacgtttctccggcgagcatgaacgcgtcgtccgggtgcatatacacgtccaccccgagaccggcagcgtcgcgcacatggtccaagtggccgtgcgtgcacacgacagcggtcaacgtagcgccctgctcttcgaactggcggcgcacatgctcgcctgccccgagccccgggtccaccgcgaacccttcgcgcgtttgatcattaatcaccacatagcagtttgtctggtacgggccgacgacgaatccagcgatgttcatgcatgcgatactatttcaccgttcaacacccgttgggcgcacgcacaacgcaatccacgagggaatcgaggtctggtcacggtggctacgaatgaagagcgcggcaagcaggcgctttcgaacctggagaaggaactgaactcgcgagaccgcaagcagcgccagcgtccgtgggtaacggcagcggcatcgctggctgtcatcgcggcgctcggcggcggcatctactttgcggctacccagaacagcgacgaggacgtgaccgcctccgaggagaccacggagtcaaccgcgaccgagaccgaagagtccaccttcgacgcgtccgagtatgaggctctgtcaaccaagcgcgccgtcgcgctgcccgccacggtgaactgcacctacaccgaagacggcgacgacgcgaacttcgtcggactcccgccggccgagggtgtttccaccgagggcaccgtcaccgtggacctcgaaaccaaccgcggcccgatcggcatggaactcgaccgctccgtctccccctgcactgtcaacgccatcgagtacctggctcaggacggttacttcaacgacactgtctgccaccgtctgaccacctccgacgggctgaaggtgctgcagtgcggcgacccgagcggcaccggcgccggcggcccgggcttccagttccccaacgagttccccaccgacgaggttatcgacgacgtggatctctcggccctcggtgtgccggaagatgcctccgacgaggagaagcgccagtacgcctccatgatgttgcaggatccgaagcgctacgagcgcggcacgatcgcaatggcgaacgcgggcatcgacaccaacggttctcagttcttccttaactacggtgactcggttctgcccccgctctacacgtacttcggcaagatcagcgacgaaggtctagacaccttagacgcgatcgccgaggtaggcgtcgaaggcggcgcgtccgacggcgccccggcagaagaagtcaagattcaaagcgcggcggtgaagtagcaagcacgcgaatacgacccttgcggattcataagggactgttaggatactcaaggtcacaagaagacgccgccaaaagattggacttcccatgcagtaccgtaagagcctcgtcgctgccgccaccgctgccgccgttctgacctcgggcgtttccgttgcgcaggcgcagaccccgcaggtgaacaaggaaacgacggccaaccagaccacgaacaagaagaacgagtcgtcttccagcaacggcaacaagccgaccgcgaaggagatccaggactggatcgctgtggctaccgcgcttgtcggtctgctcggcaccatcgcggcgttcgcgcagaagtacctgcgcccgtagccactacggttcgctcgatcgccccagctcttagctcggggcgattttgcttatcgacgcccctgccaaacagctaacccgccaccctctccttcgcggagacagtggcgggttaattggtttcttaagctaacgcttaacggccgaggtaggcgatcgggccgagcaactggtcgatcgggaacgcgaagatcagcgtgagcacgctgaggacaccgacgaccgcggcgatgatggcgccaaggttcgcatccgacgagccggaggtctgagacggcgcagccgagtcagacttcgcaacggtcacgggcatcgtgatgctggtttccttgtcggtcgtgatggtcagcgtctgctcaccggacacacccgccgggatgtcgatggtcacggtagcgcgcccctgctcgccgtagcccttgtcggcgtcggtgacagtgttatccaccttggccgtcgcttcagcgccgccgatcttcacggtgacgttctcagccttcggctcaccctcggacgagtacgacagcgaggtcagcttgatctcgttcttctgcccagccttcaagccaccttccggcagcaccacgccgacatccttttggccggaacgaactgttgcgtcgcccgactccaggtagtcgacgaacgcctggaggtcgttgtagccgacatcgttgcggtcgcggaagttctccgcgcccaagaagccgtcacccccgtcgaagaggaaggtggaaccagcgacggtgtagtccttgttcggatcgacctccttaccgttgatggtgatgctggtgatcttctcgccgcgcggagcctccgggttgtaggtgtaggcaacgttgtccgacaggcctaggtcgaggcgcggacgaccggacttcgcggccgcttcctcgctctgccactggttctcaagcatctccttgatcgcagcgccagagacggtggccacggcaatgttgttgccgaacggctgtacgtcaaacgcctgtttgtaggtcacgtcaccttgggcgaggtcctcacgaacgccgcccgcgttcatgatgccgaaatcaatgtcctgagcgaggaactccgacagcgcggcaaccgcagactgggcgatcatgttgttcgcagtcgattcggtgccgcggttggagcccggagccgcagccgggttggagccgcgcttgaaatcagcgtcaatcgtcgccacaacctgattgccaagaacatcagcctgctccttggccttggccacgatatccgcaaccgctgcgtcaggctcgatacccagctcattcaggtgcgaagcgtcgtactgctgggcgtccttcttcacgatcttcttctcggccttgtcgtaggtgagaaccaggttcgtgacaaccttgccgtactcctgcgactgggcaaagggcaccggagcctcgaggtcaagacgcttgatgtggtcgtcgccgccgaaaacgaagtcaacgtactgctcgttcagcttcgctgcgctggtgtgggcggggtcgtggatgagcgcgataacgagatcagccttgccatccttcttcagcttttccgcctcgacgttgacctgctcagcagagtcagtgatgttcaggtccttgacgttggccgggttcgacttcgaaactgtcaggttggaggtggtgccaacgagggccaccttgacaccgtcgacgtcaacgatctcgtagggcttggtctcgcgggtgccatcggtcttgaacacgttagcgccgagctgggtgatggtgccgtcaacctcggtgcccgggacgattcggttcatcaggtccgcgtaacccttgtcaaactcgtggttaccgatagccgtgccgttgaccttgatcgcctgcaggaactccatcgtgtacttatcgtccgagatggccgacacgaacgcggagccaccctggttatcgccggaggtggtgacgagcgtgttggggttctgctcgcggaggtagttgatgatgcctgcgacgtttgcggcacccatctcgtcgcctgccttcggagtgacttccccggtttccctgttcttgctcaggttcgcctcgaggcggccgtggaagtcggtgatgttggcgatgttaaaggtgacctggtcggcctcagcggcgaaggcggccggagcgccggtcaggacaacggcggtggcggtggtggcggcaatcaggttgccagcgcgacggaacgagaacattgaaactccttggcaggtggtacaggtgattcacctgtctttgtaacctcacaaaaagtttcctgcaggaagctgccagggccttgtgattgcgagctggggcgctaacttcaccgacacgaaaaattcatgtaccggcaacctttcgggggttgctgaacgctacgccgtcacacggtagatgtcgaagacaccctccacgttgcggatctggttcatgatcgatcccagctgcttgacgtccgacacttccaccgttagacggaccgtcgcaatccggtcctcgctcgcttgcgacgatagcgcgacgatgggcagcttctgctcgctgagcaccccggtcatttcggcgaggaggccgtggcggtcgagcgcctccacttggaaggtggcgagggtggcgctgccgtggccggtggagttggcccacgcgacgtcgataagccgctccggctcctccttcagcttcgccgcgttcgtgcaatccgcccggtggactgaaactcccccaccgcgggtgacaaaaccgaagatggcatcccctggcaccggctggcagcacttggccagcttcgccatcacatcgggcgagccttggacaaggatgcccgggccgtcgctgcgggaggcgcggtgaaccagttccgcgattggcgtgcgcgaagcgagcgcatcgattgcctcgtcctcgttgccgaacatctccaccaacagcttcgacacgtgttgcgccgagacgttgccggcaccgatcgcggtgtagagcgcgtcaacgtccgggtagtgcagctgcgtggccacgcgacgcatggattcagccgtgaacaggcggtgcataggcaagccaccgcgctgcacttcggcggcaagggcgtcgcgccccgcctccaagtgctcctcgcggcgctcttttgcgaaccactggcggatttttgccttcgctcgcggcgagacgacgaattcctgccagtcacgcgacggacccgcgttctggtcctttgaggtaaagatctccacccggtcgccggattccagctccgattcgagcgctaccagcttgccgtttacttttgcaccgatgcagcggtggccgacctcggtgtggacggtgtaggcgaagtccaccggggtcgatccggcggggaggttcaccacatcgccctttggcgtgaaggcgaagatctgctggctggtcaggtcgtagcgcaatgagtcgaggaactcgttcgggtcggcggcttccttctgccaatccaaaagctgacgcatccacgccatctgatcgacttcggcctggtcgcccttgtgcgaacccttagtctccttgtaacgccagtgcgcggcgacgccgaactcagcgttgtagtgcatctcgtgggtgcgcacctgcacctcgagcggccgaccagtgtccgtcatcaccgtggtgtgcagtgactggtagaccccgaacttggggttggagatgtagtccttgaatcggcccggcattgctgagtagatcgcgtggaccacgccgactgcggcgtaacagtcgtggacgttgtccaccagcacacggatgccgacgaggtcaaagatctcgttgaaatcgtggccgcgcaccaccatcttctggtagatcgaccagtagtgcttcggccgccccatgacttcggcctcgatgccgttggagcgtagctcgcgctgcagctgcgaggtgatctcgttcagcgcccggtcacgcgaaggtgctcggtcagcgacgaggcggacgatctcctcgtatttcttcgggtaaagaatggcgaaggctaaatcctccagctcccacttcacgctcgccataccgaggcggtgcgccagcggcgcgatgacgtcaagggtctcgcgagccttcttcgcctgtttttccggcggcaagaaccgcatggtgcgcatgttgtgcagacggtcgccgaccttgatcaccagcacgcgcgggtcctcggccatggcgacgatcatcttgcggatggtctccgcctccgcggccgcgcccaaggccaccttgtccaacttggtcacgccgttgactaagcgggcgacttcggggccgaactccgattcgagctgctcgaggctgtactcggtgtcctccaccgtgtcgtgcagcagcgctgccacgatcgtggtcgtgtccatacccagctccccgcagattgtggccacggcaagcgggtgcgtgatgtagggatcgccggatttgcggtacacgccttcgtgcagcgtctctgcagtttcgtaggcgcggttgagcagttcaacgtcggccttcgggtggtaccggcggtggatcgacagcagcgggtccagcaccgggttcgtcttcggccgcccgccgccggtgagcgaccgggccaaccttgccgaaacgcttcgcacgctcggcccctggcgctttacaggacgatcatgcgtcaccgccgtttacccctccccgcctactggcccagcacgacaagcttgccgtcgccgagcttttcgcgcccgccgagaccctccacttcgaggacgaccacgtagcccacgactttgccgccggcgcgttcaatgaggtcggttgccgcgacgagggtgccgccggtggccaacacatcgtcgacaagcacaatgctctttcccgcaatgtccatgccgtccgaggggatctcgagcgccgcggtggagtactccgtggtgtactcctgggtgatcaccggcgggggcagtttgcccttcttgcgtatagcgaggatgccgaggcccatctcgtaggccaccgcggagccgagcaggaaaccgcgcgcgtcgagaccgccgacgaggtctgcgccgagctcgcggctcgcctgcgccatttcgtcgatgacgatgttcagcgcgtccgggtcggccagcaccggggtcaagtcctcgaacaggacgccctcctccgggaagtccggcacgcgcctgatcttgtccgcgagcgcttccttagccgactggtatttgttggtttctagagccatggcttttcttacgtttcgtccttgtgtgtggggtgatcgccgcgctgccagcggtttacgttccaaccgatgccagacaaacctgtgtacgcaactacgttactcacctcgcggtcgatcgcgaacgtcacgggctgggcaatgagcgggatggtgggcaagcggtcccagaggaagatctcctgcgcgcgcagcacgcccaggttgtccgccttgttcagcgcagccgggaagctggtcatcgggtcggcggggtagataaacgcgtcgatggtgccatctgccgcgacctcttcgccccactcgccgatctcggcgcggggcaggtctgcgagcgattttccgtcgccggtggcgtccacgattgtcacgcccgcgggctcgcagctgcgccgcatcgcttccaccatcgcggcgtaccgcttactcggatacgcgtaaccgatgcgcacctccgcgccctcgagggcacgcgccctctccacgtccacgtcgaggcgcggctgcacagcgtcgtcgaggcgtttcgccagcgggtcgtcgttctgcagaacgtgcagcggcgccaccggcaccgctatgccagccgcactgctcgcggcatccgcaacggcgcgggggtcgatgcagcgcgacagcgcctgtcggttctcctcgaccgcccacgtacccacctccgggaactgcagcacctcggtcagctgccccgcgacggtggaaacctcaaggcggttgtcttcggcgttcgagtcaaaccattcgggtgtgtggtcgcgcaggtcgccaacgacgagttccccgctttcggcgagcgccccggcgtcagccgaacccggccacaccacgatttcgggctcggccggggcgtcgccgtaatagtgctcgttggcgcgcagcaccacttccccgtcatcgccgacgcggtcgatggtgtacgggccaaaggacgtctgcagctcttcgtcgaagttgtccaggttgaagctgccgcgccacacgtccgcgatcgggcgcaggcggtcggcatcctccgattcaagctcttcgacaagttcatcgacggagagctcaagttgctttgcgacggcatgcgccggcaacaccgtgccagcctcaaacaatccgcgccaacgtgcgccgcggccctccttgaagatgaccgtgaagtctttggagccgggcgtgcaggtcagttgagcggtgtcgtcgaaaagcggcatgcttgagccgaacagcgctgggtgcgtgccggcggtgaacgccagaaggtagtcggaacaggtaaccggcgtgccgtcggagaacaccgcctcctgcgacagcgagtagttcacgcgccgctcggggcccggcaactcttgggtggtgaccaggtccgtgttcgggatcatctggccctgcggcccgggcacgtacacgcccgggtacagcgctgtcgaaagcagctgcgcctgggtggaccggccctcgagagtacccgcgttggtggtgaccagcggcgtggagacgaggtagccgaagcttgcctcgtctgcgccgtcgtcgatccccgcgcacgcggtcaagcttgtcactgcggcggccgcgagcgcggctacgcctttgcgcatcgtcgttttcatcatccgcctaccgggcgttgggcctccacgtggtggagccgcccggtatctcctggtacggggcgatgtcgtcgctgacgtccgcgcggcgcgacaccggtgcggtgacggttcgcttcccggacccgccgcggctgtcgccgtccgtgtccacgtccgcgtctgcgtccgggccgtctgcgcggtagcgggccacgtcctcgttgtggagctggtacttcctcttgcgctccatcaaggtgaccagaagcggcgtagcgaggaacagcgacgagaacacgccctcgatgacgccgatgagctgaatcagcgcgaggtcccgcagcgtgccgacaccgagcatccacacggcgacgaccatcagcgcgacaatcggcagcgccgagatgacggaggtggaaatcgagcgcataacggtttggttgagcgccaggttcgcctcttcggcgtaggtggagcggcgcgagtccagcacgccggcggtgttctccttcaccttgtcgaagacgatgacggtgtcgtaaatggagaacgtcagcacggtcaacagaccgatgatcatcgccggagtgatctcaagtgcgaagagggcgtagatgcccatgatcacgacgccgtcgacaagcagcgcaaccatggctgcgatggccatctcgcgctgcaggcgcagtgcgacgtacacagcggccgcgaggaggaacacacccatcgcgagcagcatgcgtttggttatggtgtcgccccacgattcagacacggtcgagtcaccgatcgcgtcggggcttgcctggccttcctggtcgagcggctggtgcttctcgtagatcgcctgccgggcctgatcgatctgctcctgcgtgaggtgctgagagttgatttccagcgtgcgcgcgtcgcccgcgccgacgatctgggtcagctcgggggtgactccggtggcctcggtgaaggtctcctccacatcctcggcgaccaagtcgccggccggcatggcgatcttcgtgcctccctcgaaatcgatgccgaggttgaaaccgcgcgccagcatcgccacgatcgagatcgcggccaacgcgagggtgattgcgtaccacgtcttgcggcggcccacgaagtcaatcgcgccctcacgggtgtagatgcgctcgaaacggccgacgtttacgtccggggttgcagcggtagtgattgcgctagacatggcttagtgctcctcttcaatcacgtcgggggtgcggggggcgccggtcgcgcgggccgcggcgcggttgcgctcgcccactgcgaacgccttgcccatgccgttgaccgccggcttcgaccagaagccgctacgggaggcgatcacgagaagcggcgccgtgaccaggaaggtgaccaagaggtcgaacacggtggtcagacccatggtgaacgcgaagcccttcacgtcgccaacggctaggaggtagatgatgacggcgccgatcagggtcaccatgttgccggtgacgatggtctccttcgcacggtcccagccggaggcggtggcggagcggaacgtcttgccccgtcgcacctcgtccttgatgcgctcgtagatcaccacgaaagaatccgcggtggtgccgataccgatgaccaaaccggcgatgccggacaggtccagcgagtaaccgatccagcggcccagcagcaccagggcaccgtagacgagcagcccagcggcggcgagggtgaccagggagatcaggccgtagaggcggtagtaagcgaagacgaagatagcgaccagcgcgagaccgaccaagcccgcgtagatgccggcctgcagcgatgccaagcccagtgacggcggcacagtcatggcggtgccgcccggctcgccgttctcgcccgcaaacgacagcggcagggcgccgtagcggaggttgttggccagcgtctcagcctcctcctgggtgaaatcgccggtgatggatgtggcagaaccgaccggggtggcgccttggatcactggtgcagagatcacctgcgagtcgagcgtgatcgcgatctgctggccgagcagcgacgaggtcaactgcgaccacgtctgggaaccgttgtgctggccgtcctggctgaaggcgaagctgatttccatctgccctgtctgcacgttcgggccgccggtgatcggcctgctggtgtcaatctgctcgccggtcagtcgcgggccgtcggcgtcggtgacgccggtgagcagcggcacctcatcaagcagcagcacctgcccgttggacgggtcacaggcgaccagcggcagcgtttcgtcgtcggagccggcgagctggtccacctgctggccgaagcacttcgactgcagcagcaccatggaggcgaactgctgcgtcgggtcggcagactggcgggtctcgcgcagcatctcagtcacctcctggcggcgctcagctgccccaacggggccgttcggctccggcagcggcgtagcgtcgattgcgggtgccgtgggagctgcggcgtcctcgccctcggtctcgccctggggtgcgaagacctggttcaccgcagcctgagcctccgcctgggtgagcacgcccatctcgacccattgagtcgcggtgttgacaagcacctgttcagcggtggccggatcacccgccggcgcctcgagtaccgggcggaacaaaagctgggaggtctgaccaatgttgcggacctcggaggtgtcgtcgcccgcggcggtgatcacgagcgtgttgccgtcgaccacgaccgacgcaccggacacgcccataccgttgacgcggttttccaagatgttgcgcgcgtcttcaagctgctcgcgcgtcggttcggcgccctgcggcacgagggtgacgcgggtaccgccctgcaggtcgatgcccagtttcggcgacgcttgcttgtcgccggtgaaaaacaccagggaatagacggcgatgacgataagcgcgaacagcgcgagcgcccgtgcgggccaccggcgcgccgagccgttagatcgccgagtgtttgctgacactgagctttctcctcaactttttcacgtttttctcctgtccggcgcccattgacccgcggacatgcacaacggaacatgctacggcatgcccgcgcgacgttttaagcttggcccgcagcttccgccgggccttcctttgcgccctccaccgggtcggcagaagcggcgacggagtcgcgtttcagcacgccagcggaatccatcgctacgacaacaccgggcgcgatctcgacttgaaacacctcgccgtcgacgccgactaccgtgccgtgcacgccggccacggtgacaatcgcgtcacctgggacgatggacgcacgcatctgctgcacctcctgggcgcgcttgcgctgggagcgcatgagaagaagcgggggcaggacgaacaggccgagaataagcagcattgtcagaagttccatgccgcatatcctctcatgtgccgggatgaaggagatttagaacataccgagctgccccggcgcatccggcgggggcgtcatgccgaggtggttccacgcgctggccgtggccacacggccgcgcccagtacgggccatgagaccggcgcgcacaaggtagggctcgcacacctcctccaccgtcgccggttcttcgccgacggcgatagccagcgtgttcacgcccaccggcccacccgcgtgcccgcggataagcgaatccagcacggcgcggtcgaggcggtcgagccccagttcgtccacgtcgaataccgccagcgcggcgcgcgccgcagcgaggtccacatgcccgtcgccgttgacgtccgcccagtcgcggacgcggcggagcaggcggttggcgatgcgcggcgtgccgcgcgagcgggaggcaatctcaacggcggcgtcgctgtcgatgttcacgccgaggatgcgcgccgcgcgcgccacgactttggtcagatcctccacactgtaaaactccatctgcgcggtgaacccgaaacggtcgcgcaacgggccggtgagcatgcccgcgcgggtggtcgcgccaaccagggtgaacggcggaatctccagcggaatcgacgtagcgcccgggcccttgcccacaatcacgtcgatgcggaaatcttccatcgccatgtagagcatctcctccgccggacgagcaatgcggtggatctcgtcgatgaagagcacgtcgccctccatcaggttcgacagcatcgccgcgagatcgcccgcgcgctcgagcgctggtcctgaggtcatgcgcaatgacgtgcccagctcctgggcgatgatcatggccatcgtggtcttgcccagcccgggaggtccagaaagcaaaatgtggtccggtgtcacgccgcggcgtttcgcgcccgcgagcaccaagttcagctgctcccgcaccttcggctgcccgatgaactcgttgatcgacttcgggcgcagggtcttctctacgtcgcgctcgtctgcctgcgcttgcgcgtccacaggcgaatcaaccggccgcgtgtagcccgcaggcagctcgaactcggtcctttccacgtctgacatcggctacttcttccccaacgacgtcaacgaggcgcgcaacagcgcactttggtccatctccgcattctctgcgagcagctgctccacgacagggcgcgccgccttttcaccgaagccaagaccaatcagcgcctccacaacttgttcggaggcaaaggagctggtgctgcttgccgacgtcgcgcttcccgccgcgcccgccccctccggagcaaccgcggcaagtgcgtcgatcttgtccttcagctcgagaactatccggtcagccatcttcttgcccacgcccggaatcgtctgcaccgccttcgcgtcgcccgcggcgatcctgttcgccagctcccccggctcaaagaccgcgagcgcggcgagcgcgagtttcggaccgagccccgtcaccgtctgcaacttgtggaacatggtgcgcgcgtccgcgtccgcgaacccgtagagagtcacgctgtcgtccttgaccaccatggatgtcagcaccctgcgggattccccgcgaaccagtttgcccaacgtcggcggtgtggcgaggaagcggtagcccacgcctgcgcactcaatcaccgcatggtcgaggccgattgcgataacttcgccgttgagggagtcgatcatgctgtcgctgtcctttcgccctgcgtcccaagtgtcgtgcgggcgattaaaggcgcgcgccagcagtggcacaccgcgatcgccagcgcgtccgcggcgtccgctggctttggcggctcactcaatccgaggatgcgggtaatcatgttcgtcatttgcttcttgtcggcgcggccgttgcccgagacggccttcttcacttccgacggagtgtactggtgcaccggaatatctcgctccgcggcgcagagcaccatcacacccaccgcgtgcgccgtgtgcatcacggtggagacgttcccgcgctcgaaaatacgctccattgcgacgacgtctgggcggtactcgtccatccagtcccctactgcgcgggacaaccgcaggagacgctccggcagctcagcggtggagggtgtgcgcaccacacccaccgagaccggcaggatctgccgcccccgcccggcttggacgacggagagaccgcaccgggtcaaacccgggtcgatccccatcacgcgcagcccttcgagattcaccacacatatgttctaccacacgggtctcacacgtagtcgaggtcggagaaaccctcgatgtcgcgtctgccgtgctggtagatctcgtcgtttgccgctccggaaaaatcccccacccagtcgccgtcgctccagcgcaccggaacgcggccgacaaggagatcttcgtccttgtccaactggtcagcggagaagaacaccgcgacctccacgacgacgtagtccgtgtcgcattccacgaccctgtaggcgaccggcgccggcatcgtgaggaaccggtggctggggtagcctgcgggatcgttaaacccgccttcgtcgcgcaatgttgcagcgagggcggaggtcttcgaaagctgctcgtacgactcggccgcaacttcgtcgccgctgttcgggtggaacgtggcggtgttgatcgcggcgagcaccgcgcccgccggcgagtgcgcgtatccgcgagggatggcccggaccgtcttggtcgggccggcttggtcattcaccaccatgtagcgggcgttgacgtactgctgctgggtggtgcctttcaggccgtcaaaatcgccgcacgaaccgggtcgcagcgcggacgcatcgggcaggtcgccgtcgtgctcaattggggtccacgccgggcggcccagaaacacgtcgggagcgtactcgccgggcttggcgtgcacgctgtcgtcgacgcctccgggccagctgcgctgccggttccccacgagcgcacccgcattcaccggcgggtccaccgtgtctgctgctggggcaggttctgggtcagggctctgcgcaatgctggtgaacaaggccggctgcgcttccggcacaccgcgcccgccgtcgggcacagagcacccgcccagcacggtggtggtcaggacggcagcagaaaaggccgcggcaacgcggcccgggaggcgaaaccgcaacgcgacctagtcctccaactgctccgcgacgtcgtcggagatatccatgttggtgtagacgttctggacgtcgtcggactcctccagcgcgtcgataagccgcatcatcttcttggcgccttcgacgtccatgctcacctgcacatcggcgcggaactcctgctcggaatcttcgatctcgatgccttcggccgcaagcgcctcgcgcacggcggcaaggtcggtcggcttgcaggtgatctcaaattcctcacccaagtcgttgacctcttcggcgccagcttcgagcacggccatcagcacgtcgtcctcggtgagctcgcccttctgaatggtgaccacaccggtgcgctcgaacatgtagcccacagagccggactcgcccaggttgccaccgttcttcgtcatcgcggtgcggacttcggtggccgcgcggttgcggttgtccgtcaggcactcgatcaaaaccgcgacgccaccaacgccgtagccctcgtacatcaccgtttcccagttggagccgccggcgatctcgccggatccgcgcttgcgggcgcgctcaatgttgtcgccgggcacggaagccttcttagccttgcggatcatgtcatccagcgttgggttcgcggacgggtcgccgccgccggtgcgggccgccacctcaatatccttgatcagcttcgcccacaacttcgaacgcttcgcgtcgttcgcagccttcttgtgcttcgtagtcgcccactttgagtggccagccatcacgcaccccttacttgctcggagacatgtatcggcctgccagtatacgcgcgggcgctatttcccccgcatcggaacttgggtggcgccggggcgcaactgccgggcgagtccctcctgcgccaccaaggcgaccaagtcgccgccggcgttgaagaggcgcccctgggtgagcgcgcgcccgcttgacgccgaaggcgaactttgctggtacagcaaccaatcggtcacgcgcaccgggcggaagaaccagatcgcgtggtccagcgacgccagctgcacttgcgcgccggggtgcgcctgcagggacgagtacagtagcgtcatatcggacatgtaggtcagcgcgcaggcgtggaacgcgtcggtgtccagggcggttgccgcgccaggcacctcaagctcctcgcggtagcggaaccagaggcaccgtccgctgacgatcttggggccggctggcgcctcctcttggggcacaacccggatgtcccactccctaaaatccttctccgccccgggcactcccgagggaataggaccaccggccggaattgtctctggcccgggcacggggggaaacggctcggcgtgctcgggtccgacgtctgcgtggtggtggaaactcgcggtgagcgtgtagagcaacgtgccgccctggaacgcctcgacggtgcgggaggagaagctgcgtccgtcgcgaagccggcgcacccggtacaacgtctcttgatcagcctcccctccggcaaggaagtagctgtgcagcgagtgcaccgttttgctcccttccaccgtggcgctcgccgcggcgagcgcttgcgcagccaagtgcccgccgaaggtgcggacgaagacgtcggtgttcatcgccgggccgcggaaggtgtccccgccgtccgccgcaacgccaagcacgcggcgcagttcggatgtgctcatagctcggcagattaccagcgggtccgctacttaccccgccgccatctggccgagcgcggcgtactcaggcagggccgctgtgccgcccaaccgcagcgtgcgcaccgcgggtcgcaggcgcagcgcgcgcgtatcagccacggcgtcgttgtaaaaccgcagggcgagcatcacgcgcgtgtcagcgtcagcaatctcgcgctgcgctgccgccgcgaccgtgccctgatccaaggccgcggccaccaaggcgccgagctccgtctcccggtcaagcctggaggcgagatcgcgcggacccatgcgcacctcctccgccgcccgcgccgcggctgcgagctccggcagcgttgccgcgatcaccgcgcagcgcctgtcgagggctgcctgcagcgcgtcgcgcgagcgatccaggcggatgtgcagccggtcgaggcgggtggcggtcgactgcgcccacagcgcgagcgctgtcaaagccgctgcgaggattacccaccagacagtgctcacctttgcaccgccactttctcgcccgtggccacggtctcgtacacggccatgatttggtctgcgactgtggaccagtcgtactgctgtgcgcggcgggcacctgcgtcgatgaagttgttgcgggtgccgggggcgtcgataagcaactgcaactggctcgccaacgccgactcgtcgccgaccggaaacagcaacccggcaggctggtgcgctcccgcgtcgcacaccgcggcgaacgcctcaatgtcgctcgccaccaccgcgcagcccgcggccatcgcctccaccagcacaatgccgaaggactcccctccgaggttcggcgcgacgtagatgtccgcgcggccgaggatcgcggccttctcctcgtcggtcacccgcccgacaaaatccaccccagccacgctgcgctcccggcccgcacccatcaccgtcacccgcgcaggagcatcaagcttatcgacgccccccagcatcacatccagccccttcctcggctcatccaagcggccgaggaagacgatttccacctcggacgtatcgttccggggaccgcgcgcagcgctgaagcgctccgtgtccaccccgttcgggatgaccaccgggtccgtgcccacctgctccacctgccaccgccgagccatctcggagaccgcgatgcccccgcggatcttctccaagttgcctcgcagcaccggcagcgccgccttcaacgccaccgaggaggtggcggaggtgtggtaggtagccacgatgggcccgcttgcccagcgcaccgcggcgagcgagtagctcgtggcgttcggctcgtggacgtgcagcacgtcgaagtcgccgtcctcgatgaactgccgggtcacccttcctacgtgcgggccgatcgagaggcgggcaacggagccgttgtagggcaccgccactgcgcccccgccgcgggtgacgtacgcgggcaggccggtcccggcggaggcaggcccaagcacctgcacgtggtggccgcggttggtcagcacttcggccaagtcgagcacgtgggcttggactcccccgggttcgtcgaaggagtacgggcagaccataccgatgcgcacgcttagaccttctttcgcctcggtttccaatcgctcggccacacgggttgcagcatatgccaatccgcggggtgggcggcgatgttagttgcgaacgcgtcagcgacgcgctggacggttggcccaagctcgtccacctcgaccggtgggtcgactttcagaccccaccccgggccgttcgcgtcctcggtgaaccacgagtgcacaaccaaaagctcagcgccagtctcgatagcgagcttggcgggcccaacgggaaaggtggtcgcctcgccgaagaaggtcacgggcacgcccttgccgccaagatcgcgctcgcccaacagacacacgatgccgttgttctcgagcacctcgcgaagccgcgggaacggcgccgcgcctccggtcagtggcagcacttcgaaaccgagggactcgcggaaatccacgaacgcgtcgaaaagcacctccggcttgagccgctccgcaaccgtggtgaactgcgaatagtgcttggtcagccacagccccgcgaagtcccagttccccgagtgcggaagggtgagcaccgcacccttgcccttagctagcgccgcatccaggtactgggtaccgctgacgccttcggtgtagcgggtgataagcgcctcgtccttctcgatgcgcggcagccgaaaggcctccagccagtagcgggcgtaagagcggaccgattcccgcactagctcgctggtaacgtgttcggcgccgacgaccctggtgaggttgcggcgcaactggtccatgccccggccgttgtcgctcaccttgtccgcggcgagccggaacgctggtgcggtcacggcgtacggcaacgcgccgacgagtttccacccggcgatgtagccgtacgcgctcagcgcgtccttgtaatccacctacgcccccggcggcggagggatcttcacttgtgctttcggatcgcgcgctgcgtagatcagacgctgaacaacggtgaacaccgaaccagcgagaagcagccacaccgcaacctccaccgcgtgcgcaacgccgaagccctcgagcccgatgccgaccagcgccacgatgaggcgttccgggcgctcgacgagaccgccgacgatcttcaaaccgccggcctcagcgcgcgctttgatgtagctgatggtctgagacagaacgaggacggccaggctggcggccacgtgcgcggggtgggcgtggtcgacgtagatcagccacatcgcgatcgcgccgaagagagcgccgtcggtgatccggtcgcagctcgcgtcgagcgtcgcgccgaacgcggttcccccgccggaaagccgcgccatcgtgccgtcgaccatgtcgaacaaggagaacaggccaatgagcacagcggccgtgatcaggtggccgctgggaatcagcgcacacgccagcagcactgataccgcggtgccgagcagcgtggtcgcgtttggggtcaggccggcgccgagcatgccgcgggcaaccggttccacgaaccgcttcgccggcttgcggccgtgcacactgagcatgtcagttgtcccttccgttcgcgtccgcgatttcacgccatccgtttgcaagcagctgcctcgtctcgcgcagcagctgcggaagtactttagtgccgccgatgaccgtcatgaagttggaatcgccggcccaccgcggaaccacatgcaaatgcaagtgttcggacaccgaccccccagctgccttgcccaaattgagccctacgttgatcgcttccggctcggacacgtgcttgagcgtgcggaccgccatcttggcaaagtccatgagctccgccgtctcctcaggcgtcaagttctccagctcagctaccttacggtagggcaccaccatcagatggccggcgttgtacgggaacaggttgcacacggcgtaaacgtgctcgccgcgcgcgatgacaaggccgtcttcgtcgtccatttccgggatggcgaggaacgggtcctcactcttctgcggcattgacgcgatgtagctggagcggtacggcgcccacaatcgctgcagccggtcggtgtcgccgacgccgacgtcctcgtacggctcggccccgctggcctggccgctacgcgcgtcgcgcaccgacgttttcctcgttcggctgctcgttgttcttctcggccgcccagtccgcgatgagcgccaccgcttcatccacaggtacgccgttgatctgagagccgtcgaggaagcggaagctcactgcgttggcttccacgtcgcgctcgccggcgagcagcatgaaaggcactttgccggtggtgtgcgtgcggatcttcttctgcatgcggtcgtccgagtggtcgacttctgcgcggaggccgcgcgccttcagctgaccgatcacaccctcgaggtggtcgccgaacgcgtcggcgaccgggatgcccaccacctggtgcggggcgagccacaccgggaaagcgccggcgtagtgctccagcagcacgccaaagaaacgctcgatcgaaccgaagagggcgcggtggatcatcaccggacgctgcttcgacccgtcggaggaggtgtattcgagatcgaaacgctccggcaggttgaaatccagctgcacggtggacatctgccacgtgcggccgatcgcgtcgcgagcctgcacggaaatcttcgggccgtagaaggccgcgcctgccgggtccggcaccagctcgagaccggacttggtggcaacggactcgaggatgctggtggagcgctcccagatgtcgtcgtcgccgatgtacttctccgggtccttggtggacagctccaggtagaagtcgtcgaggccgtagtcctggagcagcgagataatgaactccagcacgctggtcagctcttcctccagctgatcctcggtgcagtagatgtgcgcatcgtcctgggtgaagccgcgggcgcgggtcagaccgtgcaccacacccgacttttcgtagcggtagaccgtgccgaactcgaacaggcgcagcggcagctcgcggtaggagcgcccgcgggagccgaagatgaggttgtgcatcgggcagttcatcggcttgacgtagtagtcaaccggctgcttggtcacgttgccctcgtcgtccacctcgccgtcgagcttcatcggcgggaacatgccgtccgcgtaccaatccaggtggccagacttcttgaacaggtcgcccttggtcacgtgcggggtgttgacaaagctgtagcctgcggccacgtggcgctcgcgggagtgctgctccatcaccatgcgaacgatgccgccgtccgggtggaacaccggcaaaccggagccaacctcatccgggaacgagaacaggtccatctcgttgcccaagcggcggtggtcgcgcttctcggcctcctcgagcatggtcatgtactcgtcgagcttctcctgcgactcccacgcggtgccgtagatgcgctgcagcccagcgttggactggtcgccgcgccagtacgccgcggacgagcgcgtgagcgcgaacgctgggatgtacttggtggtgggcaggtgcgggccgcggcagaggtcgaaccactccacctcgctggtgcgcgggttcaagttgtcgtagtaggtcagctcgccggcgccaacctcggtcgcctcgtctgagttggggtcgacgttgcccttgtcttggatcagctcaagcttgaacggctcgtctgcgaggcggtcggcagcttcctcctgggaggcgaaaacgccccgggagaatttttgcccttgcttaatgatcttcttcatccgcttctcaagcgtcttcagatcctcgggcgtgaacggttcttctgtatcgaagtcgtagtagaaaccgtcgttgatggcggggccgataccgagcttggtgcccgggaactcagcctgcacggcctgagcgagcacgtgtgcgcacgagtggcgaatgacggcgcggccgagctctgtgttcgccgcgatcggcataaacgtcgcggtctcgtccggaacgtgcgagaggtctttcaggttcccctctgcgtcctgaaccaccacgaccgcctgctcacccttgttcggcaggttcagctcgcgcattgcggcgccgacggcggtgccggcgggaacctcgaacggctcgaactgaatgatttcggcggtttcagctgctgcttctgccatggataaggtgcgctccttttgcgctcgtgggaagcgtcatacctggacgcgccccgtgtacagtgcggcctcagattctactccgagttctacccaagaaccgactggccccagtagctgtcgcgcccgccaccggtgccgggcggcacgtagtacacgctcgaaccgatgtgggtgatccactcgttgagccggtccgcctcgtccaagcgctcaagcaccggggtgaactgggtgtcggggtccttttggaaggcaatgaagataagtcccgcgttcgacagttcgccggagccgggcaccggcggcaggttgtagttgtaggggcggcgcttgaagcgctgctccgggtggtcctccggagccctcgaacgggccatgtgggagttccggtcgatcacgggaagcccgtactggtcgaccgcgtcgaagttgggttcgtcgaactcctcggtgccggtaagcggcgccccgctagcaagcgaacgccccacggactcctcccttgagctgcggtcgagcttttcccactcgtcaaggtgcattgctattcgacgcaccaccatcgacgtcgaaccgtcatccccaaacacctgctcgctgtattcagcctcggtgtaggggttcacggtgccgtcgacttgaccgaagaggtttctcggcgtctggcctttggggatggcgccgtaggcgttcatgaacccctgctggacccaggcggtggtgacgtaatccgcggccgcgcgagtcatgtgccgcatcgcccacgcgcacatcaccggatcgtccgcgcaaatctgcagcgcaatatctgtctgaccccacgcggggtcgagctcgtcccgacccagcgccggaatatcgtggagccaggcaggcttgtccactcccgcgatgtcaaagagacgctcgccgaaaccgacggtgaacgtcaggttggcgggccacgtgttcatctcggtttcgaggctaccgagcggagtgcgccctgacgccagctcgcgcgcgtcctcgctccacaaccgcataagccgctggatgccagcgcggtccaccccctcgttcaggttgaacccgaccaggttcagggcagcctgcgtgagggtttcaatgcccgcttgatgcgggccgtcgaaggcgacagtggccgactgcagcggttctcggtcgggttcggagttactcggcaccccggcgggcgcattcgggtcctcgccggctggagcgcacccgctgatcgcaccagcctgtgcgacagctgccccaatacccgcgatgaacccccgcctagaaaccgccatgacgctctatccctctagtggctgtgcccctcgtgcttctgcatctggtcgccgtagtcctcctcgccggcggccatggtgcgcaccgcgagatccggtatctccaccgccgacccgtctgcgagctggagggtgagggtaagcgtgtcgcctgcgtgaatcggctctgcatagtccatcaccatcaagtggtcgccgcccggctcgagttcgtgggaacccccggcggaaatggtgatgccgccgcccttttcctgcatcacgccgtccttaacctcgtgaatctggttcttgtttccgccgagcgaggtggtgaagccggtgatcgtaatctcactgtcggtgtggttacgcagggtgccgaagattgaagtcatgtcgttgccgtgctcggtacccgcgtccgccttggcccgcaccgttcctttctccagcgtgaccgcgtcaccagagggcgcggcgtgctcgccgcggtcttgagctgacgtggctgcggtgtccagggtggttgcggtgtcgctcgcgccgcacgccgcagcggtgccggcgagcacagtggtcagggcgaccgcggcgaatgtctgcaacgagttgggcaacgattcttccttctagctgttgtgggtgtcgggatcggggtccaggatggtccgctcctcgagcttgcgggcctggcggcgtttacccaccgcggcgatggccacgccagcgatgacgacgaggccgatgattgacaaaagcagggtgcggttggagttctctccctggtcggcaatactcggttcccccgagttcgcgtcctccgcgctcgccgcagccgtttcggtagtcgccgagccgtccggcgcgtaggtgaaggttgtcgttccctttgtggcgtggccgtcggaggacacgatctggaacccgatctggtactcccccggctcagcggcgaaatcgcccggcaaatcgagcaccacgtcctggccgcggacatccggctcgccggtgtagacgatatcagccccgcctccaccaacccgcgacagcgccaccgtgttgaaaccgtctttcggctggccggagaatgtcagttcaagcgttgaagggaatgtcgccaccacctccccattcgctggcgagccgccgataacggcgtcgtgagcgccagctgccggagccagaagcagcgcggcggccaccccggtcgccgcggccgagcgcgggaaggacacattcataagcgatctccttttgcgttgctaggtaagttagtcgcctctcccccgaggttagttcccgggggtgcagccgcccggcaacgcaaaaccccggacgccgcaggcgcccggggcaatgtttcgtggtcctagctgggatcgaaccagcgacctttccggtgtgaacggaacgctcttccactgagccataggaccgaacagggaagtactttacacagtggccggcgcgggaccgaatcgcctgctcaacccgaacattccgcggtcggacactaagtcaggccgcacttttcacaagccttcgcaaccctgctcagatcacattcgtgtaattcacccgttacgccggttttgctggcgatttgtctatctcgggagcgaacggttaatgttctatctcgcacaatgcagatgcggatgtagcgcagttggtagcgcatcaccttgccaaggtgagggtcgcgagttcgagtctcgtcatccgctccaagtcccctagcgggacttcacccgcgcgattagctcagcgggagagcgcttccctgacacggaagaggtcactggttcaatcccagtatcgcgcacagagatcccctgcgggatctcgacgcggatgtagcgcagttggtagcgcatcaccttgccaaggtgagggtcgcgagttcgagtctcgtcatccgctcaagtactttccacgtacttcggagcgaaagcactccacccggtggattggtcgagtggttaggcaacggtctgcaaaaccgtgtacacgggttcgattcccgtatccacctcaactaatcttcatattccccgcgcgattagctcagcgggagagcgcttccctgacacggaagaggtcactggttcaatcccagtatcgcgcacaaagatccttcgctcgaggggtcttgccgctgttttcaggcgcggcgtgcggatgtagcgcagttggtagcgcatcaccttgccaaggtgagggtcgcgagttcgagtctcgtcatccgctccatctcacgggggttaaggttgcttcatgcacggagcagaccttaacccccaaattgatgccctgatcggcccggtgcaggcaccagccaggcgcgagctgcgcatcgtcggcgccaacaccctcttcggcgggttcgcccgccgcggcacctccggagagttgggcaacgacaccgacgcggcgctcatcaaaggcctgcgcgaatgggccgatgtcatcctggtcggctccggcaccgtgaccgccgaagattacggcccgtcggacacgccgatggccatcgtgaccgagaacgccaacctcgacccggggctgggagtgctcgggggcaagaagatcctcctcatggctcccgaccgctcgtttgcgagagagaaaaccaagcagaagcttgcacagcttgccagcggcaacgtgtcccccgttcccaccggcagcgggagcctgagcgaggtcgtcgcggcgctgcacgcccgcggtttcaaccgcattctctgcgaaggcggtccgagcatctacgccgatgtcgttgccgctggcttggcggatgtgctgcatgtgacgttggatccgtcgataagcagcgccgacggccccttcggcctgcctttccccgactacccccgcttcgagcaccgcttcgtgctggaggacgctaccttcacccgcgactcgatgctgttctgccgttaccgggcgctaaggtgagcgcgtgactttctggaccgctcccgcacccgtcggcacgcgcggcagcgccgcggctgcggccaacgcgatggcgtggccggccgcggtcgtgctcatcgtgcaccgtttggccgtgcttgcccgcacaggctcggtgaccgacgacttcaccaccgtctggtccgccgcgcggcggttcgtcgagcgggtgccggtgtacagcgaggtctaccaccacgtgaacccgcactacctttacaaccccggagccacgctgctgctagcgcctctggggctgatcccgagcgtcgacgcggcgcgaccgtggttcatcctcgccaacgctgtcgccatcatcgccgcgctggcttggctgacgctactgagcgggcggagcctgcgctcacctgtgttccccgcggcgctggcgctcggattcgctaccgaggccgtgaccaacaccctggtgttctccaacatcaacgggattctgctgctcgcgctcgtggcgttcatcgcgaacatgatgcgcggcagacagatcgccgcgggtgtgatcatcggactcgccattacggtaaaaccgatgttcctgccgctgcttgtcttgccgttgatgcggctggagtggcgcgccctggtggccggcgccgccgttcccgttgcgctcaacgcgatcgcgtggccggtgactcccggcgccggcgactacctgacgaagctcgtgccctacctcggcgtcacgcgcgactacgccaactcctcgctcgccggattcgctgtgtacttcggtatgcctgagatcctgcacaccgcgctgtttctagttttcggcgcctcagtcgccgtcgccgtcgccggtttagcccgctggcgctacagcgacccgtggctctgggccacgatgacgtcgggcgtgctgctcgccggagtgtgccttctctcctcgctggggcaggcgtactactccatgatgctctttcccgcgctgtttacggtgctgcacaaggcttctccgatgcacacacccgcagcctggctgggtgcgattttgtgcctgtcccccttgagctggatcacgccgcacatgcccgctgccggtaggtggctgaccacgttcttgcccaccgccggctgggcgacgttcatcctcgccgccgcgacatgggtagtgtgtgcacatgaccgattacaagaattggaccaacgaccagtggcgcgagaagctctcccctgaggagttccacgtcctgcgcgaagcgggcactgaaccgccgggagtcggtgagtacaccaacaccaccaccgaaggcgtctaccgctgccgggcctgcggcgaggagctgttccgctccaccgagaagttcgagtcccactgcgggtggccgtccttctactcccccgctgacaccgacaaagtcatcgagcgcgaggaccgctcccacggcatggtgcgcaccgaggtgctgtgcgcgaactgcggctcccacctggggcacgtgtttgccggcgagggctacaacacccccaccgacctgcgctactgcatcaactccatctcgatgacgctcgaggaagcgtaagcagacccgcgccctacggcaggatctcgatgatctccgcgatgtcggagacgcggcggcccgtctggaacgggatttcctcgcggacgtgcaggcgcgcctcggtgtagcgcatcgtgtgcatgagctcctcgatccgtgtcagggtcggcgcctcgaacgccagcatccactcgtagtcgccgagagtgaaggattccacggtgttggcgcgcacgtcggcgaagtcgcgggcggccatgccgtgctccgccaagatgcggcggcgctccgtcggctcgagcaggtaccagtcgtaggaccgcacaaacgggtacaccgtgatccagtcgcccggttcctcgcccatgatgaagctgggcaggtgcgacttgttgaactcggccgggcggtgcagcccgttgccgatccagctcacttccaccagctggccgagggtggtggtgcggcggaagtcggcgaacgctttctggatctgcgagaactcttcagcgtgccaccagatcataaagtccgcgtcggcgcggataccggtgttgtcgtaaatgccgcggacggtgacttccccctcttcctccaatttggcaaagaaggcctgcgcctctgcgatcacctcggaacgttcggcgcctagcgcgcccgggatcgcccggaacaccgcgaactggaggtagcgctggacagcgttaagggaatcgaaatcgagcttggccatggcaggcatcctttctccggtagccggaatcaatcgaaagtcgtattcgatactaccccgagctcgacggcgcgcctccactgaatcccgcctgtggtggatagcttaagtttctgtgaagcaatcggaatcctccactggccacggccccgcgccggtgagcactataggcgcccgcggcgcggcaccggacgacaaggctcccgcggcgaccccggaagagttcaaagccgctgtggaatcgatgcacgccgcccgcctgcgcccggagatcaccctcggttcgattcgcccgccgcagcgcccagccccgttcagccacgctgtcggtctcgaagtagaccgcggcgacgacgccgatgcggctgccatgaattccgagggcgacgcgttcggccgcctgatccttttgcactcccccgatgccgaggaagcgtgggagggctccatgcgccttgttgcctacatccaggccgacatggacgacgcggtggctgcggacccgctgcttccagacgtggcctggcagtggcttaacgaatctctcgcagacaccggggccgggttcaccaacctgggcggcaccgtcacctctacggcgtccgtgcgcttcggcgaaatcggtggccctccgcgggcctaccagcttgagatgcgcgcctcatggaccgccgacggactcgacttggctccgcacgtcgaggcgtttgcaagcgtgctggccctcgtggccggcctgccgccggagggcgtcaccgagctcgggcgccgctagccgcccgctttttctcagcaacctgtaaagtaacccctcgtggagaaacgcccggcctacgagcttgttgacacccccgaggggtaccgccgcgcggccgccgcgctggcgcagggccgcggcccgtttgccgtcgacaccgaacgggcgtccgcgtaccgctacgacgaccgggcgttcctcgttcagatccaccgccgcggcgccggcaccttcctcatcgcgcctgaaggtcaccgcagggaggtggaagcgatccttggccccgtggtcaacgacggagactggatcatccacgccgccggcgaggacttggctagtttggcgctgctcggcctgcaccccggctccctcttcgacaccgagctcgcggcgaggttcgctggtttcgaccgcccgaacctggccgcggtggtggagcactacaccggtgtgttgttggagaaaggccacggcaaagaggattggtcgctcaccccgctgcctgaggattggctcgactacgccgccctcgacgtcgcgtacctgcacgacctagcagagtcgctcgcggaggagttggaccacgccggcgtcctctccttcgccgcggcggagttcgaccatctcgtcgaaacgcgcagcctgaagcccgcaccccggcgcacgtggcgcgacttgaaaggagtcgcctcggtgcgctcgccgcgcggcctgcagatcgcccgcaccttgtacaacgcccgcgctcacgaagcgcgccgcagcgacgttgcccccaactctgttcttccgtcccgggtcgttgtcgcgattgcccgcgccgagccggccacacccggccagctggcccgtatcccgggttttcccgcccgccggcgaggtgccgcgcagcactggatgagctacgtggagcaggcgcttgccgacgacccgacgtcgtttcccgcccccgcggtccgcgaccgcagcaaacctccaacgaaggcgaactgggagcgcagccacccagagaactttgctgcgctggaggaagcgaaacagctgcttggcgacgcctcgcgcgacctcgggtttccccccgagatcctcctcacccccgcgattctgcgcgaggtggtttggcgcgcccatgcgaccgacgacacgcactcggttgtggcgtcgctgatgtcaagcggggcgcgccagtggcaggccgaaatcgccgcgccgctgattgcgaaggcggtacaagcgcacccgcactaggagcagttaccgatcagccaaaccggccgcccactggcggatctgctccgcggcgctgactgcgtcaaggccgtacatggcgataatctcgccgcgggaagcgtgctgcgggaagatgtcaggaaaggcaaggtggcgaaccggggtatcaacctcggcggcggacaacgcctcggccacggccgagccgacaccacctcgaaccacaccgtcttcgtacaccacaaccatgtcggcgccagccgccagatcgagcacggcaggtgccaccggcaccacccaacgggggtcgatgaccgtgcagcggatgccctcggcatccagctcctcggctgcggagagcgcgtactccgcaaacgtgccgaccgcgacaatcagcacttccaggtcgtcctcggtgcccggtccctccgggtgcgcggccgggtagcgcaacacgtccacactgccggcgatacgctcgattgccgggatgtcctcgctcacgctgcccttgggaaaacgcaccacggtcggtccgtcctcaacggcgatggcttcgcggaactcctcgcgcaggcgctccgggtcgcgcggcgccgccaccttaatccccgggacgatggatgtcagcgccatatcccacactccgttgtggctcgccccgtctgagccggtcacaccggcgcggtccagcaccacggtgacgggctggttgatcaggccgacgtccataagcaactggtcaaacgcgcggttcaggaacgtggagtacaccgcaaccaccgggtgcatgcccccgagcgccaaccccgcggcggaggcaagcgcgtgctgctcggcgatgccgacgtcgaagaagcgctcgggaaactgctccccgaagggggccagccccgtcgggcccgccatcgcggcggtgatcgccacaatgtcgtcgcgctcgtggccggccttgagcagctcctctgtgaacaccgacgtccaccccggaggcgcctccgcgagcgcttcaccggttacggggtcgatgacgccggtggaatgcatctggtccgcctcgtcgttgaccgcgggcgcgaacccgtgccctttttcggtggctacgtggatgatcagcgggccctcgtaggtgcgagcgtaagtgaacgcgttaacgagggccttcaagtcgtggccctccaccgggccgacgtacttcattccgagctcggagaacatctcggtgggcaccacctggtgcttcacgcccgctttgagcgcttgcagcgcctcgaacgtgcgctcgccaacccagcccatggacttcagcgtcttcttgccggactccatcacctcgtcgtaacccggctgaatcctgatctgcgcgaactggtcgcgcagccgcctgaggttggccgcgaacccgccgatggtcggcgcgtacgagcgcccgttgtcgttgaccacgatgaccacgttgcggttgccctcagcgatgttgttcagcgcctcccagcacatgccgccggtcagcgcgccgtcgccgaccaccgccaccacgtggtcgccgccttcgcctttgagctgcttcgccttcgccaaaccgtccgcgtaggacagcgccgccgaggcgtgggaggactccgtccagtcgtgctccgattcggcgcgcgacgtgtagccggacaggccgtctttttgccgcagcgtgtcgaagtcgcccgcgcgcccggtgagaatcttgtgcacgtacgactggtgcgacgtgtcgaaaatgatggggtcctggggcgaatcgaacacgcggtgcagcgcgatcgtcagctcaaccacgcccaagttcgggccgagatgcccgccggtggccgaaactttttcgatgaggagctgccggatctcatccgcaagcttgcccaactgatcctgaggcagggctttgagctccgccggcgaaccaatcgtgtctagcaatcccacggtatccatgcgctccttcgctctcggtgcttccgaacaatcgtacacgcggagaaagcgcgcctaggaaactggttcgagcagggcaattgattcgaagtggtgggtgttggggaacgcgtcgacaagcacgatgctcccaacgccgtagccggaagcccgccacgcagcaaggtcccgggcgaaggtggcggggtcgcacccgatgtggataacgcgctcgggccgcgccgctgcgacggcggccaccaccggctcacccgcaccagcgcgcggcgggtcgagcacaacaagcccagggggcttcagcttgccgacgcttgcctcaaccttcccagcgaccatctcaacatcgaacgcggccagcccccgctgctgcgccgccgtcgccgccggcgagtagtccaccgacatgatgtgcgcgccgcctgtcgcctccgcaatcgcggggacaaacgcgccgacgccgccgtagagatcccacgccaccgggttggcgtagtcgccggcgccccagctgcgaatgatctccgagtagacctcgggcgcgcgcacgtgcgcctgccagaacgcggtggccgggaagcggaactccacgccaccgatgcgctcggtcacctcgccggtgccctctacgacgttttcgatagcttccacgcgccggccgcgctgcacacgcgcggtttccacgacgtggcgcgcacccgcggcgtcgatcacggcaaccacctcgctgcccggggtgaagcgctggtccagatccatgagccccggcacgggctgggtgcagcgctgagacgcgatgacgtcgccggagcgggcccggcgcacgcccgcgcggcccgactcgtccacgcccaagcgcacgcgggtgcgccaacccaacgtcggttgaagcgtgcgcagcgcgatcccgccggcgaggtcgtcatcgcgcacgccggcgatgctggccagctggccgcgcaacacgtcgcgcttgagctctggttgggcagccgggttgatgtggctgtagtcgcagcaaccggcgccggcggcagcagcggggcacgcgggcacgacgcggtcttctgacgcctcgacaacctcggtcagctcggcgcgcgcccaccgcttcttcgacttggtgatgttcgcctcgacggtgtcgcctgggatggcgccggggatgaagaccacgcggccgtcctcaagctggcctatgccctcgcccccgtgggcgatgcgggtgatgtggatcggcactgactacccgttgttcttcgcgttctgctccaggatctggcgcagcgcgtcagacagcgcgttcgggttgcccgcctgcggagcctgcccctgcgcaccctggccctgcgccgcgcgcgcctgcacggcctgctggacctgggcagcgagctgctgcggcaggacaaccggcagggagttgccggcaagcaccgggtcctcgccgcggtagacgaaggagcgcgcgataatctcgcggcccaactgcgccatcgcgtcctcgcggccggtcggcgcggcaagggtgacgcggtagagccagcgcgggccctccacgccgatgatgcggatcacgccgttggagccggtgccgacgacctccatgccccacgggccttcctcgtagtgcattggcatgccctcgttgcgcatgccctcgccgatctcctctgcagactcctcccacagcccgccggtgcgcggagccgcgaacgcgaccggggtgaagcggccgtgctgggtgacgatgtggaccatcttcgggccctggtcccccatctccacctgcacctgggtgcccttcggcatcggcacgcgcaccgagccgaggttcagggtggcgtcggagaagtcggtgaagtcgaagtcgtcgatgttgacggtgtcgccgtcgaaggggccggtggagccgttgaccggatcgtaatcggtgaggcgcgaggtgcccggcgcggcttcgagcggcgcagcgtccagcggggcggcaaccaactcagcggcggcctcctctaccggggccgccggcgctgccggctccgcggggtctgccggtgcggtgtcctccaccggctgcggggcctcaaccgcctccggctgctgagcgtcttttttcttcttgccaaacggccaaaatgccatggtttctccaaaaattttgttgctgctcgccgatgtgttgctgggttcgaccttagtcgcccgcttgcggcgggcgggggacgtggttagtgcgtgccggtggagccgtagccgcctgcgccgcgggcagtgtcgtcaagctcgtcgacctccacgaaatccacgagctccacccgctgcaccacaagctgggcgatacgcatgccccgcgtgatctcgatagcgcgctcggtgtccgtgttcagcaggcacaccttcagctccccgcggtactccgcgtccaccgtgcctggagcgttaacaatggtcagcccgtgcttggcggcaagacccgagcgcgggtggatgaggccaacggtgcccatcggcagggcgacggcgatgccggtgccgacgagtgcgcgctgaccgggtgcgagggtgaggtcttccgcggagtggagatccgccccggcgtcgccggcgtgcgcgcggaacggcaggggcatctcggggtcgagccgcttcacgtgcaggggctcgaggtcggtcagggggccagctacggtgtcgtgttcgttcacccggcccaccctactaaggtttgatgcgtgtccaacaacgtttctccgcaggtgctctactcggagcggcagtgggtgccgtggtactggtgggccgcgggcctcgggctcgcgctgctcatctccgcccagttctcgctcaaccggaccttcgtgtggttcatcgtcccgctggtggttgtcggcggcctgatcggctggttcttgttctggctgtccaaaacggtggtgcgcgtggagcaggacccggacggcacgcgctggctgagcgtcggcgaggccaacctgcccagtaccgtggtcgcccgctcaatggtggtgccggcgtctgcccgccagaacgcgctggggcgccagctcgacccggcggcctacctggtcacccacacctgggttccagagcacgtgatcttggtgctcgacgacccggaggatccgaccccatattggatggtctccgctcgcgatcccgaggcggtgctggcggcgttcgtgccgggtcaggtggatgacgggcgaagcgtctagcagggcgtcggaaagcaaccaaaagcaaaccccggccgcggatccgtgagaaggatccggccggggtttgcttgtggccctggattactcgcagtcgaggcagatcatcgagccgtccggctcgacgtgcgccaggcgcttgcgcttttgcaccaggaagcacgatgcgcaggtgaactcgtcgtcctgacggggtttgacctcaacgttgagctcctcgccggagaggtcctggctgggcagttcaaaaggctccacaatttcgccgtcatcatccatgctgctgccggcgacttcagccgccttgagcccctcgagggaatcggtctcgatgtcgtcgtccatccggcggcgcggcgcatcgtaatcagtagccatggtgagtgtcctccagcggtgtgaatccttgcgcgaaactgtgcgtagcccgcgccatttcagcggaatactaaaacaccggattcgttctgtcatcacagcaggtcagatcactgttaggggcagtgccgcgacacttacagcgccgctatagggcaggttgcgcccgcggactccagcaggtcgaaaaagtcctcccacacccgcggcgccgaggcgatgaccggctcgccgcggcccgccccgtccgcaatgcccgggtggcgcaccacggcaccagcctcggccgcgatcaccgccgctgccgcgtagtcccaaggatgggtgccgtgctcgtagtaggcgtcgatgcggccctcggcgaggttgcacagatcgagcgccgccgagccgatgcgccggacgtcgcgcacccgcggcaggatcagccggagcatctccgcctgtttcccgcgccactcggcgtcgtaggagaaccctgtggccacaagggccgtgtccgtgtcctgtttgttcgacgcgcgcaagcgcgtgtcctcgccgccccggcgcacgaacgccccctcgcccttcgccgccgagtagacgtcgccgctggccacgttcaccacgcaccccgccacgaactctccgcgcaccgcagcacccaccgataccgcgtacgcgggcaacccgtaaaggaaattgactgtgccgtcgatggggtcgatcacccactgcacgctggtggtgccgtcgacattggcgccctcctcccccacgatcgcgtcgttgggccgaagcgcccgcagccggtcggcgatatgcgcctccgccgccctgtccacggccgtgacaggatcgacagcagaagtcttcgtttcagtcacctgcgcgatagatccgtgcttggacaagaaatcgcgttgctggaccacgaggtcggcggcgctgaccgcaaggtccgcgcagatgtccttcagttctgctggggtcgggatcgcgttggtctccatacgcccatggtgccagggttatagacttacgtggcatgacaggaaccaacctcgcggccggcgtcgatgtcggcggatccggcatcaagggcgcaattgtcgatttggaaaccggagagttcattggggacagggtgaaaatcgcgacaccgaagcccgccactccggaagcggtcgcggaggtggttgctgaggttgtgggcctgctcggctgggacgggcccgtcggcgtggcgctgcccagcgtgatcaaaaaccagatcgcgcagaccgcagcgaacatcgactccgcgtggatcggcaccgacgtccaccagctgctcgcgcgccacctcaagcgcgagcgcgtcgccatcctcaacgacgcggacgccgcaggcttgggcgaggttgcgtttggcgaggacaccgcacgctccggcgccgtcatctttctcacgttcggcaccggcatcggctcggcgttcttcgcaaacggttccctgttcccgaacaccgagctggggcatttgcttatcgacggccacgaggccgaacacctcgcctcctccgcagtcaaagacaacgaggagctgagctacacgcagtgggcggcacgcgtcgacacagtcctcgcagagttcgaccgcttgtttaacccgtcggcatttatcgtcggcggcggtatctcccggaaggccgagaagtgggtgccgaagcttaccgtcgacgtgcccgtgatccccgccaagctgcgcaaccgcgccggtatcgtcggtgcggcaatggctgcgtgggacgacgtgaccccgtagttataacgacacgctccgcgggtcggtggaatagccctatcagtaacgctgttactatggctgttctgagatgcgggacgtcaatgtgccgtaccctgggtttcccaacccggttggtgggtgcggctgaacgtgaactatccgacaggcgaaagggcgtacgtggtagccaaggaagcagcaggcaacaacaccgtcgacgacacagaatcaaccaccggcgacgtggttgagcgttctgcgaagaagacggcgaaaaagaccaccgccaagaagaccgccgccaagaaaacggcgaagaaggccaccaagcggaccacgggctcggccgccgacgcgaccgtcgaagacgtgaccgcagcagcggccaccgccaagaagacgacgaagaagaccacccgcaagaccgcggcgaagaaaaccaccaagaagacgacgaaaaagactacgcgcaaggccgccaccaagccggcggcggaggaagcggaagcgccagtcgaagacgttgacgcgaccgcggccgaagacgatgtcgacttggacgattccccggacatcgactacgacccggaactcatcgacgaagacgacgagtccttcgactccgacgaggtggttgatgatgtcgacgaggtagatgacgtcgacgacgaagacggggacgaggacgacgaggaagaagacgcaggcgcttccgtctgggacatcgaggattccgcggccctgcgccaggcccgcaaggacgcacagctgaccgcttccgccgactcggtgcgcgcttacctcaagcagatcggtaaggtggcgctgctcgacgccgagcaggaggtttctctggccaagcgcatcgaggccggtctctacgcgcagtaccgcctcgacgagatggaacgcgctgccaaggagggcgacgcggaggccaagctcaccccgatgatgaagcgggacctgcgcgctgtcgcccgcgacggccgcaaggcgaagaaccacctgctcgaggcaaacctccgtctcgtggtgtccctggccaagcgctacactggccgcggcatggcgtttctggatctgatccaggaaggcaacctaggcctgatccgcgccgtggagaagttcgactactccaagggctataagttctccacctacgccacgtggtggatccgtcaggcaatcacccgcgcaatggctgaccaggcccgcaccatccgaattccggtgcacatggtcgaggtcatcaacaaactcggccgcatccagcgcgaactgctgcaggatcttggccgcgaacccacgccgctggaacttgcgaaagagatggacatcaccgaggagaaggtcctcgagatccagcagtacgcccgggaaccgatctcgctggaccagaccatcggcgacgagggcgacagccagctcggcgacttcatcgaggattccgaggcggtcgtcgcggtcgacgctgtgtcgttcaccctcctgcaggatcagctccaggacgtgctgcacaccctctccgaacgcgaggccggtgtagtccgcctgcggttcggcctcaccgacggcatgccacgcacgctggacgagatcggccaggtctacggcgtgacccgcgagcgcatccgccagatcgaatcgaagacgatgtcgaagctgcgccacccgtcgcgctctcaggtgctgcgcgactacctggactagcagcacgtttgccgcgccgcggccgcttaccagtctcgcaggtagtcgatgcgctggcgcagctgctccgcgttgcacagcgcggtcggcggccccccgcacgcgttgcgcgcttcagtgtgaatcgcgccgtggggccggcccgttttccccgccacaatcgccacgcgggcgttgagctccttgcgcagctccgggatctcgtctgacgcaacgctcgggccctgcccgcccgccgcgtcaggctgcgttttccccaccggttctccgtgcaggcgcgcccgctcacgctcttcccgctccgcggccttgcgagctttctcctccgcctcgcgcgcgtcgagctggtcgctttgccgcttgcgcagcagcgttttcacctgctccgcgtcaagtaagccgggcaacccgaggaaatcctgctcctcctgcgagcccgcaacggtcggggtgccgtaggtggagccgtcgaaaatcagcgaatccagctcggcggacgcgccgatcgcctcgtagttgggcgactcgtccggctcgttctgcgtccggttcgcctgctccagaagctcgtccgaccagcccgactcccggtggggtttgccaagcacatggtcgcgggagacttccatctcctccgccagctgcaacagcaccggcaccgaagggaggaacacagacgccgactcgccgggcaggcgcgaacgcacgaagcggccaatcgcttgggcaaagaacagcggtgtggacgcggaggtcgcgtacacacccacggcgagccggggcacgtcgacgccctcggagaccatgcgcacggcaaccatccactcgtcggtggagttggagaattcgtcgatccgctcggacgcccccgcctcatcagaaagcacgaccgcaactggtgtggagctgagcttctccagaatccgggcgtaggcgcgcgccgtggttttgttcgtcgcgatcaccaacccgcccgcgtcgggcatgttggcccgcagcttcagcagcctcgtgtgcgcagccgtaagcaccgcggctatccagtcgcccttcgggtccaaagcggtgcgccacgctttcgctgtttgctccgcgttgagcggctcgcccagacgcgccgagtactcctcgcccgccgaatccttccactgcgcctcgcccgagtaggcgaggaagaccacggggcgcacgacaccgtcgcgaagcgcctccgcgtagccgtaggtgtagtcggattcggacacgaggtggccggcaccgtcctcggcgtagcgcacgaacggaatctgcgagtcgtcggagcggaacggcgtaccggtcagcgcaagtcggtgttcaacgtcgttgtacgcctcgtagacgccgtcgccccagctcttggagtcgcctgcgtggtgaatctcgtccaggatcaccagcgtcctgcgcgcagaggccaccgcgtggtgcttgaacgggtgcatgcccacctgcgcgtaggtgaccacaaccccgtcgtacgccgcgttgactgccgaggagttcgtgaagttggggtcgagcgagagcccgaaccgcttcgccgcgtccgaccactggtgcttcaggtgctcggtcggcacaacgacgatgatgcgctgcaccttcttcgcctcgtacaaacggctggcgagcgtgagcgcaaaggttgttttacccgcgcccggggtcgccacggccatgaaatcgcgcggcatggtgcgctcgaactggctcagagcctcctgctgccatgcacgaagcgtcggcatggtcaggctcacttgcggcgcagccccttgtaaatgcgctcgcagtcagcgcacaccggcgagcccggtttcgcttgcttcttcaccgggaacgtctccccgcacagtgcgacgaccatcttgccggagatggcggagtccacgatctggtccttcttcacgtagtggaagaacttcggcgtcccgtcgtcggtggtcgacgatgtgtcttctcgtaaatcagtgcgctcgagcgtcttcgtcgtcgtattcacgctccccatcatgccccacatcccgtccggaaactaagccggaggcgctacgctggcaacctatgagcgcttcggaggaacacgtccacggccccggcacggtcgacgtcgaagcagaaccaactgccccgcgcaagaaacggacgcgccgcgccaaccgcgcgctgatcaccgacgccacgttctcccccgagcagaaccgccgctcgcgcgagtcgcagtacctgctgctgcagggcatccgcctaccgtttatcgcactatccatgttggccgcgttcgtgtggcacaactggtggctcgccgctgtgtttttcgtcgtgagcattccgctcccctggatctctgtcatggtggccaacggccagggtgaagttcgcgacgcccggtcgaaaaacgtgtacaagccggcgcttgtgcgcgaggagcagcggctggaggaagcccggcgcgcgcagctttccgcgggaggaaaggcgggcgcgcccactatcatcgaccacgacgaacgctagtttttgaaggagctttcatgactaccgaaccccccgcgcccgagctgatgtgccagcttgcggacgtactgctgcaagcgtccttcaccgcggacggaatcgcggcgcacttgggccccgacgccaccgacgcgctctaccgcggggagccgggcgtggtgctccgcgccacccgcggcggcacccaactcgaccagctcatccgcttctttttgctgcgccgcccgcttcccggtaaccaggttgcggaaatgctgggcgccaagctggggctttcgcttgtcgacgccgcctttttctcccccaccgcctccggcgacatcgccgtcaacttcgatgtgcgcccgcacgtgatcgcggggcgcgagcgcctcgtggtgtcggaccgcgacgcgtcggtcaccgatatcgttcctgggcgcgatcacgtgttgggggtgggcgcggcgtcgataagcctgctctccgcctcgccctcaagccctgtcgagcgggtgcttgacctcggcaccggttccggcgtgcaggcgctcgcccaggcggacagcgcggtgcgcgtagtcgcgaccgacgtgcacccgcgcgccatcgcgctcgcccgggcgacgctcgccgccaacggcatcgacaacgttgagctgcgcaccggggcctggttcgagcccgtggccggcgagacgttcgaccggatcgtggccaacccgccgttcgtggttggtttgccggaggtgggccacgtctaccgcgattcggggttgccgctggacggggccaccgagctggtcgtgggcgaggcgccgagctacttggccgccgacgggaccgcctgcatcctcggggcgtgggtgcacacgctggatcagccgtggcagaaccgggtggcgtcgtggctgccgtcgaccggggtcagcgcgtgggtgctgcagcgcgacgtggtcgaccccggcatgtacgtctccacctggctgaaggacgagtcgctcgacccccgctcccgcgcggccgtcgagcgcaccgagcgctggctcgaccacttcgacgagcacaacgtgcacgcaatcggcttcggttgggtgctgctgcgcaatatcggcgacgccccgtccgaaatcaccgctgaggagctgcggcacccgttcaccgatcccctcggccccgaggtggaggagtacttcctgcgcgccgcctggctgcgcggccgggacgccgacggggtgctgggcagcaccttcctggtgcggccgggcgtggccgtggaggaagtcagcgtcaccgacgacgagactggcatgggttttgcgcccaaggtgtgccgtgtgacccgcaccgacgggccgcggttcagccacgacgtggacgaaggcctgcgctccctgttggccggcctgcacccgcaggggctgccgttgcgcgacgttatcggcctcctcgccgcctcccgcggtgtggtggacgacgcggatatcgcgtcgctcgaggattccgctgtgagcgcggtggtcgatctgatccgccacggcattgtcattcccgccgagatcgcggaggtggtctgagcgtgaaagctgttttaacccgcgtctcaagcgcgtctgtcaccgtcgacggcgaggtcgtcggcgccatcgactgccctgaaaccggcggcatcctagcgcttgtcggcgtcggcgccgacgactccggcacggcgtgggagacgatggttcgcaagatcgcggagctgaggattttggacggcgaacgctccgtcgaggacgcaggcgcgccggtgcttttggtcagccagttcacgcttctcggacgcaccgccaagggccgcaggccgtcgtggtcggacgccgcgccgggggacgtcgccgagccggtgatcgcgaaaatcgctgacgcgctgcgggcgagaaatatccatgtcgaagagggtcgtttcggggcgaacatgcaggtagcaagtgtcaacgatggtcctttcacggtgcttgtcgacgtctcgtagacaaccccaacccaccgtggtaagaaacacatagcgttgttcccccgggaacaaattttctgcccggtgcgttgaacgggtggatttgaaggacctgttttcgaggaggcagcaccacatgactcagccggatcatgccaccgctacggatagtgaggaagttgaccgtggcagccgccgaaaccagacaaacgacaacccgtcggcggacttagtccgcgtttatctgaacggcatcggcaagaccgccctcctcgacgcagaggaggaagtggagctggcacaacagatcgaggtcggtctgtacgcgcagcacctgctggatgatccggaggtgcacctcacccgcgcgaagaagcgcgacttgaagattctggccaagcagggccgcaaggctcgcgcgcacctactcgaagcgaacctccgcttggttgtgtctttggcgaaacgctacaccggccgcggcatgccgcttctggacttgatccaggaaggcaacttgggcctgatccgcgcgatggaaaagttcgactacacgaagggcttcaagttctccacgtacgccacgtggtggatccgccaggcgatcacccgcggcatggcggaccagtcccgcaccatccgcctcccggtccacttggtcgagcaggtgaacaagctctcgcgcatccgccgcgagatgtaccagtccctcggccgcgaaccgacgaacgaggagctcgccgaggaatcgggcatcccggagtccaagatcgagatgctgctgcgccagtcccgcgacccagtcagcctggatatgccggttggcgccgacgaggaggccccgttgggggacttcatcgaggacgctgaggcgaccgacgcggaggacgccgttgtctccaccctccgccacgacgacatccaggacatcatcaacggtctcgagcagcgcgagcaggacgtcatccgcctgcgctacgggctcaccgacggtgtgccgcgcaccctcgaccagatcggccgccagtacggtctctcccgcgagcgcgtgcgccagatcgagcgtgaagtgatggcgaagctgcgcgccggcgagcgcgccgaccgcctgcgcgactacgccctgtaagcaggttttcgccttctcggcccgctgcctttttcgcggcgggccgttgtcgtgcgcgccgaccgcccacccgaacttcgctaaagttacccgtaaccgccccacccttgattttgagaggcagaagaagacgcatgcgtgatctcgtcgacacaacggagatgtatctgcgtaccgtgtacgaacttgaggaagagggcatcactcccctgcgcgcccgcatcgcggagcgcctcgagcaatccggaccgacggtgtcgcagaccgtcgcccgaatggagcgcgacggtctcatcgtggtcgagcgcgaccgctccctttccttgacaccggcgggccgcgagctggccaccgcggtgatgcgcaagcacaggctcgcagagcgcttgcttaccgacgttttgcagctcgacctatccaaagtccacgaagaagcctgccgctgggagcacgtgatgagcgatgaggtggaagcccgcgtcgtcgctgttctcgacgaccccactcgctcccccttcggcaacccgatcccgtcgcttgaccagatcggcgggccggcgactccgcgcgagcagcacggcacccgcgcctccgatctccgtttggagaagcccgccgaagtcacggtcgtgcagatcagcgagatcctccagcagggcaccgtggttcagcaccccgtagtctcgctgggttcactcgtcggccagcgggtcacgctgaccccgctggacggcggcggcgtcatcgtcaccaccgcctcgggtaacgaggtggagcttgcaccggagttcgcgcacgccctgcgcgttgagttagcgaggtaggaaagggtatgaaactctgtgtcaccggcggtgccggctacgtcggcagcgtctgcgccgctaccctgctcgaggccggccacgaagtcgtggttgtcgacgacctgagcaccggcaaccgcggggcagttccggccggcgccaccttcgtcgagggcaacatcgtcgacgtgatcgacgacgtcttcaccgagcacgccatcgacggcgtgctgcacttcgcggcccgctcactcgttggcgagtctatggtcgagcccgcgacgtattggcacgacaacttcgaagtgtcgctgcacctgctcgaccgcatgcgcgcccacggcgtgaattcgctggtgttctcatccaccgccgcgacctacggcgagccggatcagaccccgatcgtagagaccgccccaacgcgcccgaccaacccgtacggcgcttccaagctcgccatcgactacgcaattacctcctactgccaggcctacggcctcgccgcgaccagcctccgctacttcaacgtcgcgggcgcctacggctccatcggtgagaaccacatcacagagactcacctcattccgttggtgctgcaggtggcgatgggctaccgcgacaagatcatgatcttcggcgacgactggcccaccaaggacggcacctgcgtgcgcgactacatccacatccgcgacctcgcggacgcgcacatactcgccctcgaagcgaacacgtccggcacccacgccatctacaacctcggttccggcgacggctacaccgtgcgcgaagtcatcgacgcctgccgcgaggtcaccgggcacccgatcccggctgaggtggctccccagcgcgccggcgaccccgcagtgctgattgcctcctcggcgaagatccaggacgagctcgggtggaacccgacgcgcaccgagcttcaccgcatcgtgcgcgacgcctgggagttcaccaaagaactcggcgacgcctcccacggcgcgcgctaaaccgcgctaacccagcacgtccctccacgtcgcgtcgcagccggagcgggcgctctgcagtaagccttcatgctcgccgccgcgcagcagctggtcgaggatgtaggacagggagtgacccggcacctcctcctgggcacacatgagggccacgcttgcccagttggcgagcttgagcttcacggcgatgacggcccacacgctcagcgcgttcgcgcggatgaccccctcgaagttgcgggcgatggtgagcatcaccgcgccggcctccttcgggtggtccagcgccgtgttgaacaggctgtcgcgcagctgcgagcgggtcagcatcgtcgcgacgcgctccatttgctgcgtgctggtgaacacgtcgtcgaacctcaggtgctccgccccgccgacgagggggtgcggcggtgcggacgccaggtcgacgcacgcctcgagtgcgagatcgcgcgccgcactgggattggcctcgagttgctcgatcaggttatcgcccaggtggtagcagtgcgcggcgccagatgccgccgcctcttggtccccccggcagctcgcgtcgaaaaacgcccgtgtgtcgtccttgcgcaactccggcagcgccccttgtgcaagcagcgcgcccattgtcggctgctgcatgaccgacgccacggtgccgccgacccagtcgtcgccgaagcctgccgtgaccagctcccccggcggcggtccgaacacgaggctgtacggggtgccgggggcgatctcggagacgtgccagcagacgtcgacaagcgcaagcccctgcgcatccttcagtgcgtagagcgcttccaccgcatccaacgcgaggcccgagttcggaatgcgggtgaccaccaccgccatgtggccaatggcgttgtgcgtgtccacctcatccacggcgtcctgcaggttgccggcgtggcacagatcggtgcgcagcaccgggccgagaactggttcaccgctttcgtcgtcgagccacaagctcatgattacggcagattcttgcgggtagtagcctagaacccccggcagcgaggcaatgaagtcggcggggccggatagcgtggtgtctgggtgcatgtattgagtcatggttattttgacttccagttcccccttgcggttccgcttgcccgcaatctcgctgaagctgtggataacttgcggggtgggtgctggcagccgaggcaccgatccggcacaataggtgctttgaacttcgtggttgctgggtgcaaccctgtggaatgttcgcagcggcgaccacgttgtcgaaagggaatgcgcgccatcaagggcgcccatcttcggatcaggaggcacaccatgtcggacgaacgccgcatgtacgaactcgagtatcctgcgccatcagtcggcgagggtgctcccgccgggcccgccctcatcatcgccatgcagggctacgcagatgccggccacgccgtcgaaggctctgccgaccacctgaaggccgcgctggagtcgcgcaccgtagccaccttcaacaacgacgagctgatcgactaccgctcccgccgccccgcagtgacgttgagccagcacgagatcacccagatcgacgagcttgagctagacatgcgcgtgctcaaagacaacaccggcacgccgtttctgctgctctccggcccggagccggacctgcgctgggaagcgttctcggaggccgtagctgacctggcggaacgcttcgacgtgtcgaagacgatctgcttgtacgccgcgccgatgggtgcgccccacacccgcccgctggtggtttcggcgcacggcaacagcgctgagctggtcggctccatgttcacgttcgacggcatggtgaccatccccggttccgccgcgattttgatcgagcgcgagctgcacaagcgcgggcgctcggttgcggggtttaccgcccacgtgccgcactacgtcgcttcctcgccgtacccgcacgcgatgtaccagctgctgcagtcggtggaggattccacacagctgaagttcccgctgcgcgcgctggagcaggacatgaagaaggtggcgcgccagctcgcggagcagacctctgcgtccgaggaaatcacgcaggtggtgcagtcgctcgaggagcactacgacgcggagatggaggactaccgcaagcgcaacccggaggccatgatgccgggtgaggccgagctgccgagcggggaggagatctctgaggcgttcgagaatttcctttcggccatcgaggaccgggaccgctcgagggagctgtccgacccctacttcgttgaccccgacgaagacggcgctgacgggacggacgagaacgagtgacactctctgacttcctcccagatctcgccgacgttcccgaatcgctctttgaagacgcggtgtgggactcgttcacccagtggacggttgagcggggtatctccctctaccccgcccaggaggaagcgtcgctcgctttgctcgcgggcgacaacgtcatcctcgctaccccgactgggtcgggaaagtcgatggtggccaacgccgcgcacttcatcgcgatggcgcgcgggcagcgcacgttttacactgcgccgatcaaagcgctggtgagcgagaagttcttcgccttgtgcgagatcttcggtcccgagaacgtgggcatgatgactggcgacgccaccgtgaacggtcacgccccgatcatcgccgcaaccgctgagatcgtggcaaacatcgcgctgcgcgagggcgcgaacgcccgcatcgaccaggtggtgatggacgagttccactactactccgagccggagcgcggctgggcgtggcaagtgccgctgctcgagctgccgaacgcccagttcctgctcatgagcgcaaccttgggcgacacgcagtggctccaggacgacctgaccgagcgcaccgggcgcaccaccacgtatgtgggcggctcgcagcgcccggtcccgctggacttccactacgtgttcacgccggtccacgagaccgtggaagagctgatggaagccggcaaggcgccgatctacatcgtccacttctcccagcgcgaggcgaccgagcgcgcccaggcgttgacgagcatgacgctgatcaccgccgaggagaaggcgcgcatcgccgaagagatcggcgacttccgcttcaccacctcattcgggaaaaccctgtcgaagctggttcgccgcggcattggcatccaccacgcgggcatgctgccgaagtaccgcaggctggtcgagaggctttcgcaaaccggcttgctcaaggtcatctgcggcaccgacaccttgggggtcggcatcaacgtcccgatccgcacggtgctgattacggggcttgcgaagtacgacggcaccaagagccgcatcttgaagtcgcgcgagttccaccagatcgcgggccgcgccggtcgcgctggctacgacactgaaggcaccgtcgttgtcgaagcgccggagcacgagatcgaaaacgtcaaactgcggcgcaaggcgggcgacgacccgaagaagctgaagaagctgcgcaagaaggctccccgcgacggcgaggtgtcgtggtcggagaagaccttcgaccgcctcaccaccgcggagccggaggaactcaccagccagttctccgtgtcgaactcgatgctgctcaacgtcgtcgcgcgtcccggcgacggctacgagcacatgcgccacctgatccgcaccaaccacgacacccgcgcaaagcagaaccgcgacatcctgaccgcggtcgagctgttccgcgggctgattcaggcaggcgttgtggagcgcaccccggattcacccgcgttccgcccctacacgctcacccgcgagctcgacccggacttcgcgctgaaccagccgctgtcccccttcgcgctggcgttcctcacgctgctcgacccggagtcggacacctacgccctcgacgtcatctccaccttcgaggcgattctggaggatccgcgccagctccttcaagcgcagcagaacgtggagcggggcgaggaaatcgcggcgctgaaggccgaaggcgtcgactacacggaccgcatggcgatcatcgaggacgtcacctaccccaagccgctggccgacgagctggaggaggcgttttccacattcacggagtccaacccgtgggcgaaggagtttgagctgtcgccgaagtcagtggtgcgcgacatgatcgagcacgccatgacgttctccgacctcatcgccacctactccctggcgcgctccgagggtgtggtgttgcgttacctgaccgacgcgtggcgcaccctcactcattccatccccgagtcctacatgaccgatgagctcgaggacatcgtcgtctggctcggcgagctcatccgccaagtcgactcctcgctcattgacgagtgggcgcacatggcagacgaggacacccccatctcgagggagaccctcgaccgcgaactcgcgtttggcgtggaggacccgagtgctttgaccgcaaaccgccgcgcgttcacgatcatggtgcgcaactacttcttccgactcgtggagctcttcgcctacgaaaaggaggaccagctcgtcgacatgctcgcctacctcgacccggacaacacggtggattggccggcggcgatggacgactacttcgacgagtacgccgacctcgacctcggccaagacgcgcgcgggccggagtacttccgcatcggcgaccaagccggccggtactgggacgtcacccagatcatcaaagacccggacggcgacaacgccttccagcttcacggcgtggtcgacttggatgcctcggacgaggcgggtgaggtgcggctgagggagatacggctgcgtcgttaagcaaaatgctccgcagcgcgcgggcgtggattatggtgttggaaatctcacccgatctaccaccgtgataaggagcacacaatgccggaccttttggtcaaccacacgccacccgagcaaaccagcgatgtcgatgcggttgtccaagccgcgatcgcgcgcgcccacagctggatggaggccaccgcagaagcggacgccgacgacgcgcagacgcagcaacttgccgagatgcttcgcgacgacaacggcgtacgcttcaccatggacttcgtcgaccgcgtcatgcgccccgaggacaaccgcgttgcggcgaacgcactgcgctccattacccgcggcgtcgacgcgtcgttcctcggtcagatcaacgccctgctcgtcggcgccggcgcgttcgtgggcccctttttgccgttcgtggtcgtgcccgcggcgcgcgcccgcctgcgccagctcgtcggccacctcgtgctcgacgccgagtccgacgccctcaaccagctgctcgagcgcgcggagaagcgcggcgaacagctcaacctcaacctgctcggcgaggctgtcctgggcgagaaggaagcgaccgaccgggccgagcgcacgcttgccctgatcaagaacccgcgcgtgacgtacgtgtcggtgaaggcgtcgtccatggtctcccagctcaaccactgggattacgacgagtgcgtccgccaagtcaaagaccgcattcgcccgctctaccgcgctgcgcgagaccgcagcccgcaggtgttcatcaacatggacatggaggagtaccacgacctccacctgaccatcgacgtgttcacgcagctgctcagcgaggaggagttcaccgattacgagggcggcatcgtgctgcaggcgtacctcccggacacgctcggcgccctcgagtatctagccaagttcgctcaggagcgcgtcgccgccggcggctccaagatcaagatccgcctggtcaagggcgcgaacctgtcaatggagcgccaccacgccgaggtcaagggctggccgcaggcgccgtacctgaccaaggacgaagtcgacgcgaattactaccgcctgctcgactacatcctgcgccccgagttctcagacgccgtgtccatcggcgtcgcgtcgcacaacctgttcacttcagcgctggcttacgagcttgcttatcgacggggcgttacccccatgatcgactctgaaatgctccagggcatgtcgccggcgcagcaagcaatcgtgcgcgaggtctacggccgccagatcctctacacccccgtggtgcgcaaggaggatttcgacgtcgccgtgagctacctcgtgcgccgcctcgaggagaacgccgcgccgcagaacttcctgcacgcgctgttcgcgccgaagaccgccgagcacgacccgatcaaggagcaagaagacgtcttccgatgggcggtggccaaccgttgggaggtgcgcgacgggccaaaccgcacccaggaccgcactacggagaccggccgccacgtggccgaggcgtctgcggtgacgggccgcttcttcaacgagccggacaccgaccccgcgctggccgcgaaccgcgagtgggcgaagcagcacttggcgaacccgccggcggtggacaccggcgaggagatcgcggacccggcgcagattgcggaccacatcgagcgcgcactgaaggcgcaaggctcgtggggcgcgctcagcgccgacgagcgcgcgaacgtgctggaggcgatcggcgacgagatcgcgcgccgccgcggcaactttgttgcggtcgcggcgcacgaggcgggcaagaccgtcgaccagtccgacccggaagtttcggaggcgatcgacttctgcgactactacgcggacagcgcgcgccggctgggcgatatcgccgccgagttcgagccgaacaagctcaccgtggtcgtgccgccgtggaacttccccgtggcaatcccgacgggcggcgccatggcggcgctcgccgcgggctcggcggtgattttgaagccggcgccgcaggtgacccagtgcggcaagctgatcgtcgattgcgcccacgccgtcttcgaggcccacggcatcgacctcgacaccctgcagtacgtgcgcgcggacgagggcgaggcgggcaaggcgcttctgaccagcgacgccgtcgactcggtgatcctgaccggcgcgtccgaaacggcccagctgttcacgtcctggaagccggatctcaacgtgatggcggaaacctccggcaagaacgcgatcatcatcaccccggccgctgacccggatctcgcggtgaacgatttgtacctgtccgccttcgggcactcgggccagaagtgctccgcggcctcgctcgccatcctggtcggcgcagcaggtgagtcggagcgcctgatcaaccagcttgtcgacgcagtctccaccctcgtcgtcggccccggcaccgacctttccaccaccatgaacggcctcatcgagccgccgggagacaagctcgagcggggactgacccagctcgagcccggcgagcgctggctgttgaaaccccgcaagctcgatgacgagggcaagttctggaccccgggcatccgcgacggcgtcaaaccaggctcgtggtaccaccgcaacgagtgcttcggcccggtgctcggcatcatgcgcgccaaggatctggacgaggctatcgagtggcagaattccaccggttacggcctgacggcgggcatccacacgctcgacggcgacgagatcgccacctggctcgaccgcgtcgaggcgggcaacgtctacgtcaaccgtggcatcaccggcgcgatcgtgcagcgccagccgttcggcgggtggaagaaatcctccgtcggccccggcgcgaaggctggcggcccgaactacgtggcacagatgggtgtgtggacggatggggatgggaaggtggcgtcgttaagcgtgagcctctccccggccatccgggagcttttggaggagttcaagccgcacctcgagccagacgattacggctggctgtcgcgcgccgcggagtacgaccagcgcgcgtgggaccaggagttcggccgcgaccacgactttgccgggcttcgctccgaggcgaacatcttccgctaccgcacgccgctcgagccggtggtggtgcacgtgggcaggggctacaagcttcgcgacgtctaccgccagcttcttgcttccaccatcacgggcacgccggttcgggtggtggcggaccgtgcgatcgcaggcgagctcgaggcggcgggcgtgcgcgtcgacgccaacgcggtcgccggaacgccgtcgcgcattcgcgccgtgggcgaggtgccggaagcgctgtacggcgatgttgccacgcacgtgtttgacgggccggtgcttgtcgacggccgccgggagctcctcccctacctcctcgagcagtccgtgtccgcgacgttgcaccgcttcggcgtgatccacgacccggctgggctgcgcgagtcctagccgcaaacgcagtttgaagcgcgaaaaatcccgtccgaaattcttccgggcgggattcttagcgtcttaggtttcgcgggcgctagcgcgcgtcctccacgatgaccacctgggccacggcctgaacgacggcggcaaccttgactgcctcccagacctgctccttggtcaggccggcctcgcgcacctcgttcgcgtgcgcgacggcgcagtgctcgcagccgttgatggtagacaccgcgagcgaccacagctcgaagtcggccttctcaacgccgggcttcgagatgatgttcatgcgcaggccgaacttcacctgggagtagtcgtcgccgagccagttcttggcgcggtaggcgacgttgttcatcgccatgacggtcgcggcgccgtacgcggcctcgacagcctcctcggagaggtgctccttggcctcgtcggcaatctcgctgatgacggtcgcgttgcgggtcgccgccgcggatgccagcagggtgccccaaagctgctgctcgctcagctcgctcgagcgggtgagcgagcccaagttcagcttttggtccttggcgtactccggcagcgcgccgcgcaggttctcgatcgacattgttattcgggcctccttttacttcagggagtcctggaccacagccatcttgtcgatgttcttggtcgggtcgttcttctgccagtcgcaggcgcagacctcctcagactgcagcgcgtcgagcacgcgcagcacctcgtcgacgttgcggccgacagcgtccggggtgacggaaacgaactgaatcacgccatccgggtcgatgatgaaggtagcgcggtctgcgacaccagctgcgttctccacgccgagggcgcggatcaggtcgtggcgcacgtccgcgaacatcgggaacgggatgttcagcagatcctcgtgggtggcgcgccagttgaagtgggagtactcgttgtcggtggagccgccgagcacctgggtgtcgcggtcctcgaactcctcgttcagcttgccaaacgcggcgatctcagtcgggcacacgaaggtgaagtccttcgggtagaagaagacgaccttccacttgccttcgtacttctccagggagacgttctcgaagtagtcgtccggcgaagcggcgttggcttccttcaggttgccgcccttcagcgcaatgaggtcgaactccgggaaacgctcgccaacggtcatgataggcatgtcaatcctccatctcttgggttccagcgatacatctcaagtgtgccacagatccgatagccggacaagaaaaacttatggcgctgcggtattctcataggcatgtccaataaagattacaggccgacgctcgcccagctgcggacgttcgccaccatcgccgagcacaagcacttcggcacggcggcgaccaagctgggcatttcgcagccgtcgctgtcgcaggcgctggtggcgctggagagcggcctcggcgtgcagctgattgagcgctccacgcggaaagtgatcgtgaccccgaccggcgagcagctcttgccctacgccaaggccgcgctcgaggcagcggacgcgtttgtggtgcactcgcgcggcggcgacggcacactcagcgcgccgctgaccatcgggatgatccccacgatcgcgccgtatcttttgccccacctgctgccgctggttcgcgacgagttcccgcaggcccagccgaaggtggtggaggaacagaccgcgcacctggtgagcaaactccgcgacggccttatcgacgtcgccgtcctcgcccttcctgtcgaccagagcgggctcgaacaggtggagctctacgctgaaccgttcgtcgttgtcacccccgaggggcacccgcttgcggggcgcactgatctcagtgtgagtgacgtcggcgagctggagcttttgctgcttgacgacggccactgcctccgccaccaaatcctggacttgtgccacggcgctcaggtcaaccccacctcaacgtcgctgtctgtcactcgggctgcgtcgctgaccacggtgacgcagctggtgatgtcgggcatgggctcgacccttttgcccgtctcggcgctggaggcagagtgccgccggccgaacttgcggatttcgaccttcgcgccggattcgggcgcggagcggcgcgtggggctggccttccgcacgtcgtcgtcgcgccgcgcagatttcgccgcactcggcgggcttgtcacccgcgcctacgaggcggccgccaacaacgcgaaggatatgctgccgtaaatgtacgaatcgctgaccatcgccgacgagcgcaagttccgccgccggctcaagaacgcgaaaactgacgaggcgcgagagacgattcgcgccgagatggccgaggccgcgcaggtcgtcgccgcgcgcgacgctaccgtgcccgccatcacctacccggagggcctgccggtttccgcccgccgcgacgagatcatggacctcatgcgcgaccaccaagtcgttgtcatcgccggcgagacgggctcaggcaaaaccacccagattccaaagatgctgctcgagctgggccgcggccggcgcggcatgatcggccacacccagccgcggcgtatcgcggcgcgcaccgtcgctgagcgcatcgccgaagagctgggccagcaagtcggcgagtccatcggctacgccatccgcttcgacgaccgcgtctcccccaccacttcggtgaaactgatgactgacggcatcctgctcgccgaaatgcagcgcgaccgcttcctcaacgcctacgacaccatcatcatcgacgaggcccacgagcgcagcctgaacattgacttcctcttgggctacttgaagcggctgctgccgaagcgccctgatctgaaggtgatcatcacctccgcaacgatcgacccggaggcgttcgcggcccacttcgccgacgctgacggcaacccggcgccaattatcgaggtctccggccgcacctaccccgtggagatccgctaccgcccgctgatcgagcaggtcgaaaccaaagacggcgtcaaagacgtcgacaccgacatgatcgacggcgtgatcgacgcatgcaaggagctcatgcgcgagggcaagggagacattttgtgcttcttcgcctccgagcgcgacatccgtgactgcatggaagccattgagaagcaacactggcgcggcgtcgaggtcgtgccgctgttcggccgcctctccaacgcggagcagcaccgggtgttctccccgcactcggggcggcgcatcgtgttgtcaaccaacatcgctgaaacctcgctgacggtgcccggtatccactacgtggtggacacaggccttgcgcgcatctcgcgctactctacgcgcacgaaggtgcagcgcctgccgatcgaggagatctcgcaggccagcgccaaccagcgctcgggccgttccggccgcaccgccgacggaatcgcaatccgcctctactccgaggagaacttcgaggcccgtcaagagttcaccgacccggagatcctgcgcaccaacctcgcgagcgtgatcctgcagatgatctcgctgcggttgggcgacatttccgagttccccttcatccagccgccggaccagaagtcgatccgggacggcctgatgctgctgaacgagctcggcgccatccgcgacggcaagggcggtgcgccggcgctaacggacatcggccgcgacattgcgcgcatcccggtcgacccgaagatggcccgcatgctggtggaggccaaccgcttgggcgtgcttgacgacgtcaccgtcatcgtcgccaacatgaccatccaggacgtgcgcgaacgcccgctcgactaccaggcccaagccgaccaggcgcacgcccgcttcaaagacaaggaatccgacttcctctcggcgctgaagctgtgggattacatcaacgattcgcgcgacgagctgtccggcaacgccttccgcaagcggatgaagcgcgagttcctgcactacatgcgcatccgcgagtggtacgacctcgtgcgccagctgcgcgacgtggagcgccagctcggctggtcgcgcgccgagaacgtcgccggcgagcgcgacgcagacgcgatccacaagtcgctgctcaccggcctgctctccaacattggcgcacgggacggcaactcgaaggagtacgacggggctcgggggacgcggtttgtggtgttcccggggtcgtcgttaagcaaaaagccccctgccttcctcatggccgccgagctggtggaaacctcccggctgttcgcccgcgacgtggcgaagattgagcccgcctgggtcgagcacgccgccggcgacctgctgcgccgcagctactccgagccggtgtggtcgcgcaagcggtcagcggcgatggtgcacgagaagacgatgctctacggcgtgaccatcgcgcgcgaccgcctcgtgccgtaccaccgcgtcgacccggacggggcgcgcaacatgttcatccgccacgcgctgatcggcggcgattggaatcggcaccacctgttcatcgagcacaacgaggcgctgctcaacgacgccgccgccgtcgaggagaaggtccgccgccgcggcctcgtcgtcgacgaggacacgctgttcgacttctacgacgccaaactgcccgagacggtgaccaccgcccggcatttcgactcgtggtggaaaaagcagcgccacgcggacccgcactacctcgacttcgacccggcggcgctgttgaccgacgacaacctcgacacgtccgaggaggcgttcccgccgctctggcgccaaggcacgatcgattacgagctgcgctacaagttcgagcccggcgccccgttcgacggactcacggtggtggtgcccgtgccgctgctcgcgggtttcgaagcggacgggttcgactggctggtgccggggctgcgcctcgagctggtcacggaactcatccgcacgctaccgaaggcgctgcgcaaacacgtcgtgccggtgccggacttcgccgcccgcgcggtgccgctgctcgacgaggagcttccgcttgtcgacgccctctcaaacgccctgcgcgccgccggcatctccggcgtcaacgggaccgacttcaaccccgcggcgctgcctgaccacttgaaagcgacgtacgcggcgattgacaagcgcggcaacatcatcgaccacgacaccgacctcgccgcgctgaagcgcaggcaggcgggcaaaatccgctcgtcggtggcgaagcgcgccgctgccagcgcctcggaaacggtaaagaagtggaccgccgacacgctcggcgcggtgcccgaaaccgtcaccacagtcatcgagggcaacgaggtcgacgcgtaccccgcgctcgaggtcacgccggacggcgtaaaggtgtcggtgcacccgacaaaggcggccgccgacgcgtcgatgacgacggcaacgttgacgctgctgcttcgcgagatccccgtgtccgtgcagcagatgacgaaggggctaccgttgcgccacaaggtggccgtggaccattacccgcacggcggcgcggagggcttggttgacgacgcccgcgtcgcagtcatccgcgacctcatgctctcgcacggcggcgcagtgcgcaccccggaagagttcgacgcgcttgtcaaggagatcaagccaaaggttcctggcgaggtgcgccgcatcgtggtggggctcgcgcccgcgctggtggagtacgcgaatatgcgaaccgaactggcgaattgggaaggcccggcgatcgatgacatgcgctctcagctggacttctacctgccgaagcacgcaatcaccatccacggcgcggaccacctgcaacacctgccgcgctacattgaagcgatgcgcatccgcttggaagacatgcgcttggacccagaccgcgacgccgaccgccagtcggtcgtcgacgagtcgaagcgctacctcgaggcgcgtgtcgcgaaactgcctgcgagtgtgcggaagtctcgcgcctacaaagacatcctgtggcgcatcgaggagctgcgcgtcagcctgttcgctcagcggctgggcacgccgcagccggtgagccagcgacgaattgagaagctcgccgacaagctcgggcgctgataccgggcgctagaattccgaacggtcgcgcctgcgcatgaggcggatctcggactcgaaatcgtccgcgctttcgaacgacttgtacacggaggcgaagcgcaggtacgccacctcgtcgagcgcgcgcagcggttcaagcaccgcgaggccgatctggttcgccggcacctgcgagctgccttgagcgcgcaccgtctcctcaacttgctgcgcgaggcgcttcagcgcgtcgtcggacacgtcgcggccctggcaggcgcgacgcacacccaggataagtttgtcgcggtcgaacggctcgctgaccccgttgcgcttgaccactgtcagcacggctttctccaccgtggtgaagcgccccccgcactccgtgcactcgcggcgtctacggatcgcggcgccgccttccaccgtgcgcgaatcggtcacgcgcgactgctcatgatggcagaacgggcaaaacatgacctctatcctagcgcgccgcttccaagacgctgctgggttgaaccggcgcatcccccgcgccgaacgcgccgccgaagagcgacccggcgatcagcgccgccgccatcagcccgccgagggcgagattatcgcgacgctcgcgacccggttcgaacccgtcgtgctgcggaagagcgcggccaccggcaggggcagccgttcgctccgccgttcgattcgcgggcgctaacgttcgaacaacggcacgttcgcccgtgcgggaactcccgcggttgacgtcccaaacctccgacgccggtgcgccgccgtacgggtaaatcatggtggtcattgcttatctcctctcattcaactgggccaaatactaactgcccgcccaacacgggcgccggttcgtacgctcacctgttctaacgcccacatgttcgatttatagcacaccggtggagaatatcgaacacacttgcttagcgtggtagcttcgtcgataagcaactgccccaacgtccaaggagaacgcatgccgcgcaagaaggcggacccgaacgaactcgacatgagcgctctctccgagcgccagcgccgcattctgcaggtaatccaggacgcggtcgtgctgcgcggctacccgccaagcatccgcgagatcggcgacgcggcgggcctgcagtccacctcctcggtggcgtaccagcttaaagagctggagaagaaggggttcctgcgccgcgacccgaacaaacctcgcgccgtggacctgcgccacctgccggaacccgtgaaacgaaagaaggcggcccccgccgaaaccccggaagaggcgtcgagcccgcggtttgttccggttgtcgggcagattgccgcgggagcgccgatcctggcggaggagaacgtcgagacgtactacccgctgccggatgagctgctcggggacggtgacgtgttcatgctcaaagtcgtcggcgattccatgatcgacgcggcgattctcgacggcgactggctagtcgtgcgatcgcagccggtggctgaagaaggccaaattgtcgccgcgctgatcgacggcgaagcgacggcgaaagtgttccacaaggacgcgacgggcgtgtggcttcttccgcgcaacgaggccttctcccctattaagggcgacgacgccgagattatgggcctcgtcgtgtctgtcttccgagcactgtagcagcgatgcaggccgaggaacgccgccgccaaatcgccgcgctgaccgccgttgaggggcgggtgagcgttgcggagcttgctgagcgcttcgacgtcaccgctgaaacaattcggcgggacttggccgcgttgaacgacgaaggggtggtccagcgcgtccacgggggtgcggtggcgagccagggatatatgacgtccgagtttccgctggctgcgcggttgcgctctgcgcttgatgcgaaggaggcgatcgcgagggcggcagcggcgtttttgccttcggagcccggcaagtcaatttttctggattcgggcacgacgatcagcgcgttggcgcagcggatagcgttcctgccggaggcgagttcgtggtcgattgtgacgaactcgctgccggcggcgctggagctcgccgaagccggcgtcggcgacgtgcagcttctcggcgggacggtgcgggccattgcgcaggcggtcgtgggtgacacggcgctgcggacgcttgcgcttttgcgtgccgacgtcgcgtttgtcggcaccaacgccctcacagtggaccacggcctatccaccgccgacgcgcacgaagccgcggtgaaggctgcgatggtaaccaacgcgcgccgcgtggtggtgctgtgcgactcgacgaagctcggcaacgactacctggtgagtttcgccccgctcgacgcggtggacgtggtggtgactgactggggtgctccgcagtccttggtcgccgatcttgagaggcacggggtcaatgtcgtcatcgccgacagtctctagactggttgtcactgcaactgatgttcgcgcacaacgaaaggaccccatcatggcttccaagacggtgaaggttggctcccacgtgggcctgcacgcgcgcccagcgaccgttatcgccgacgccgcgggcgagtacgacgacgaagtcattctctcgcttgtcggaggcgacgatgaggacgaaacggatgccgcctcagcgctgatgatcatggcgatgggcgccgaattcggcgacgaggtcaccgtcacctccgacaacccgaaggccgtcgagtcgatcgcggcgctgatcgagcggaacttggacgacgcttaggagggcgtcgtttagcggtactgcccctcgccgatggtgtcgtagatccagcgcatgatcgggtacaccacgatgatcccgacggagcccaacgcgatgccttcaagggcaacctggccggcgtgcagcgtgaggttgccgatacccacgatcagcgccaccgccgcagcagtgaggttcaccggatcggtgaagtcgacgcggttgtcctgccagatgcgaacgcccagcatgccgatcagcccgtagagcaccaggcaggcgccgccgagcacgcccgctggaatggtgaaaataacggcgccgaacttcgggatgaacgccaatacgatcgcgaacaccgccgcgacccaataggcggccgtggaatacaccttcgtcgccgccatcacgccgatgttttcggcgtaggtcgtggtgccggagccgccgaaaccgccggcgagtgtggtcgcgatgccgtcgccaatcagcgctttgccctgcagggagtcgaggtcgcggtgggtcatctcggacaccgccttgacgtgaccgacgttttcggcgatgagcaccaccagcacgggcagcgtcaccagcacagccgaaaggcggaactccggcgtgtggaaggcgggcaagcccacccagggggcggcgccgatggtgtctaaggcggcgtcgtcaagaccgcccgtcagggcggcgaaaacccaaccgacaaccactccgatgaggatggacagcctggacgccatcccgcgcgcggcaacggtgaccagaacgatggtcacaagcgtgacgccggcgaccgccggctgcgtctccacgttcgccacagccgtcggggcgaggttgaaaccgatgagcgccacgatcgcgccggtgaccacgggcggcatgacggcgtcgatgacgcgcttgccggcggcctggacgatcacgccgacgaggatgagcgccaggccggtgatcagcacgccgccgagctgcgcacccatcccgtactgctgcgaggcagtcagcggggcgatgaacgcgaacgacgaaccgaggtagctcggcagcttgttctttgtcagcagcaggaagatgatcgtgccgaggccggagaagagcagcgtggtgttgaccgggaacccggtcagggtgggcacgaggagcgtggcgccgaacatagcgaccacgtgctgcatgccgatgccgatcgtgcgcggccaggagagccgctcatccggggcgacgacggcaccggggctcacccgtttgccgtcgccgtgcagcgtccaaccaaatcgtgtcgtatcgggagtgcggggcgtttcattcacggggagccattatcgcacccgagcggcgcaatctcctaccccgcgggcacgcgcggtccgaacaggagctccatcgcgccggggcggttggcgggtagaaggtgcccggtccaggttcggtaggccggcccgccgcggttcatcacgatgcgaccggcccgccgccgtcgtttctgccagccgggactcgcatcatcggggtcgtcgttgttgatgcggttgtggtacgagcacagcaccgccaggttcgaaatgttcgtctcgccgccgtgtttccacgcagttacgtggtgcgtttcgcagtggtcggccggcaaccggcacccgggtaccgcgcaaccgggcgacaccagcgcggctaaggtgcgctgcttggtgttggcgcggcgctgggtgcggtacaagttcactgcgccgtgctcggggtggaacagcgccacctggagatcgcaagcgtggtgcaaagccaggtattgggcgccggtgattgaggtgccgtcggtaagcatgagctccgtgtcgtcgcctgcgccctgcagaatagctacgtgcttatccagcggcaccagcacgcagggctgcggcgcagctggcgcgatgccgccgcctgagttctcgaacaacgaccagaacttctcctccatctgcggccccgcgggttgaccggggtcgagaccttcacgcaggcggtgctcaagatcggcgaggcgccgctcgtccgaaccaatgtggaacccgcgggtgccgcaccgggagcgggtgaacgaagcctgcttcttgtacggcttctcctcaaccggaacgagttctttcgcgcgctgctgcaaatacttgtacgagcggcgcgactggagcagctccacccgcagcgcggcgcgttcagcagcatcagcgacgagcttgagcttcttctcaatgagcaccagctgatcgagcgggaaccggcccgcacgcgccagcgacaccgcctgacgctgcagccgcacgtaccgcgtgggcccgaagtacgcgttgtgcaccgcctcccagtcccccgcggtcgacgaagaaatgccggcggcaagcgccgcgccgcggtcgaagccctcgagggcatcgaccgtcaacgcggcgatcatgctggcaaacggggtcatggccaagacgctagaggcgcaacaacaccaagtaaagggccccctccgaaattgtggataaccccgccgccgcgccgaaatcttctccacaatgcgcagctgaagtacattactccacatggaaattctgatccgcagcaccaaagaagaagtcggcgccgccgcagccgacctactggagcccacggttcgggcgggaggagtgctcggcttagcgacgggctccacccccaccccgacctaccgagagctcacccgccgccacgtggaagagggcctgagtttcgggaactgcaaagcgtttttgctggacgagtactacggcttacccgcaacccaccccgagtcgtactacgcgacgatccggcgcgaactaaccagccacatcgacatcgcggacgctgacgtgcattctctcgacggcaccgcggcagacgcggaggccgcggctgcggcgtacgagcgcgcgatcgctgccgccggcggcgtcgaccaccaaatcttgggcatcggggccaacggccacatcgccttcaacgagccgggcagccccctcgattcgcgcacccgcgtcatcgacctgcacccgcagacgatcgcggacaacgcccgcttcttcgacagcgagggggaagtgccgcgccgcgcactgacccagggcatcggcaccattatggaggccaagcgcattgtgctcatcgccaccggcgaaaacaaggccgatgcggtgcgcgcgctcatcgagggcccggtcaccgaggactgccccgccagcgcgctgcagcgccacgagaacgtcgcggtcatcctggacgaggcggcagccagcaagctcgtctaaggggagacgacgaactcgcggtgttggtcggcgaggatgcggggcaggcggacgtcgataagcgtgccgtgctcctcgtagctttctgaacgcacggtgccgtgctcgtgcagcagtgacacgacgtcgccgcgcgtgaagggcaccaacatcgtcacgtgctcatcgagggtgttgaggaacatctcgatcttcgcctcgagctcgctaatcccctcgcctgtgagcgcggagacgaagacgacgtcgcggccggtgcggtcgaacgcgtggcgcagctcagcgagcacgaccggatccgcctcgtcgatcttgttcaccaccacgatttccggcggcagcgtctcgcccgtgtcgcgcgtgatctcggcgagcacctcgcccaccgcctcgatttgcttcagcgggaacgggtccgagccatcgacgacgtgcagcacgaggtccgcgccggcgacctcctcgagcgtcgatttgaacgcctcgacgagctgggtcggaaggtggcgcacgaagccgacggtgtcggtgaggacgacggtgcggccgtcggcaagctgagcttttcttgtcgacgggtccaacgtcgcaaacagcgcgtcctccaccagcacacccgcatcggtcatggcgttgatcagcgaggacttgccggcgttggtgtagcccgcgatcgcgatcttcggcgtggccgatcgcgcgcgctgcgcgcgtttcacctcgcgcgacgtctgcatggcgcgcagctggtggcgcagcttcgccatctccgtgcgcaggcgccggcggtccgcctcgatgcgcgtctcaccagggccgcgcaggcccacgccgccgttcgaaccggcgcgtccacccgcctggcgcgacaggttgccgccccagccgcgggtgcgcgtgtagaggtactccatctgcgcgaggctgacttgcgctttaccctcgcggcttttcgcgtgctgggcgaaaatgtccaaaatgagcatcgtccggtcgatgaccttgatgttcagcgcctcctccagcgccaccatctggccgggcgagagctcgccgtcgaagaccacggtgtcggcgccggtcgcctgcacgatctcgccgagctccttgaccttgccggagccgatgtaggtgcccgggtccggcttgtcgcgcttttggtacaggatgtcgagcacctcggcgccggccgtttccgccagcgcggcaagctcgagcatgttcgcctccatctcggcggtggtgccctccgtccacgcgccgacaaggataacctgctcaaggcgcagcttgcggtactcgacctcgaaaccgtcttgctgctcctcggcgcggatgtcggtgccgcgggtgaggcggcgcagcgcgttgcggtcctcgaggtcgagggcgccggtggttgggtccgcacccggctgcggggcgttgtgcctaaacgcgcgggcgagcagctcgtcgtgggcgtcgttggcgtcgtgggttgtctgagtcattcagtccttatgttctttggcggttcacgattcttcctaccccatctaacccgcgcctgcccgcttttcttccgccggggtgggcgggaggtaggatacggccgtatgagcgaaactctggtcacggaccttgctgctatcggcctcggctttacgcgttggcaggacgcggtggaggcggcgatcgcctccaacaggctcgctgtcaccggcgaggtccgcggcggccagctgatccagtactccgacccgtcgggcgcgcagctgaacatcctggcggtcgaaccgttcgcaacgttcgcgggcttcgagtccatcacgcgcacctacgcgcacatcacgccgctgagcgacgtcgtcgcgctcgccgacatcatcgatccccacggcaacaccattgcttcagtcacggtgaacctcgcgcaggagccgttgcttgtcgacgaagcgcccctccaatggcaagagctctcgctgaccgccctcatgctgtcggtagaggtgcacgactcggtcgacgcgtacttggcggatcacccgggtgaggttgtgggtgaggtgcgctctgggggtgcggagggcatcgctaagcgtgctcctcaagcccctgatgcgagcgccgagttttctgcgcgcgtgctggaggcggagttccgcacctcgcagctgaccgggcagcgttttgtgcacgcgacggtggacgcggcgttcccgttcgacgtgtgcctgcccgaagggttgctgccggacggcgagttgccggcgcacaacagcgtgatctccgggtctgccctgctcgtggggtccatccccacgcctgccggcggcggctgcggcggttgcggcgggtcttgcggatgcggcgggcactaggctaggcgggctctagtgaacgcatccgaccgcgacttaacccgcgcccttgtcggcgcgctcacgctcgcggccgtggtcatgctcgtggtgctgctgcgcctgcccgggcttttactgtcggtgctgctggtcgtgggcgtgctggtgtttttccgcatgcaccagacgacccccgaagtcgccgcgatgcgcgcgagcctgagttacgcgcgcgacgacatctgcgaggtgctcgacgcctacgaccagctccaaaacggcgcgagcgcggccgacatcgccgaccgcaccctgcactaccccgccctagcgaacccggacaactccgtaccggaggtcaacgagttcctgctgcgcgcttcgtctgcgcgccgttttctttcgcgcatcgacacgtatttagaggaccccaccgtcgaccgcgcgcagctcgaacgcctgatcagcgtcgccgaccagcgcgccttcgagctgcagagcgcgtgggacgaggcgcgccgggccgccaagcagatcggcccgggttagggctcgcggtttggtgttgggcgctgcaggcccagctcggtgatagcgggtaactcgcgctgggttttgcgttcccgctggtcgcagggagccgggttgcgagttacccgctatcaacgcgtggggctgtagctcccacggtttcggggtggtggcgacctgcgattttacccctcgtcgatacggtgttttccgttgggagctacaggatcggcgagctcgccgcgggcgacgatggtggacgggccggtcatgacagcgcgggtaatgccgtcatcctcggcgatcgcgacgtcgatggcgccgccggggacgttgacggtgacggtgccggtggcggtgccggaggtaagcgcggcgtcggcaagcgctgcttgcgcggcggcgacggtgccggtgccgcaggagcgggtctcccccacgccgcgctcccacacgcgcatgtggacctcgccgtcggaaagctcggtcagcacctccacgttgacgccctccgggaagaagtcgtggtcgaacgacggctgcgtgaactcgagcgccgccagctcctcagcagtcagccccgggatgacgcacgcgaggtgcgggttgcccacgtcgacgccgatcccggcgaactcgaaatcgcccatcgaagcagtggacacgcccgtcacgtccacagcgcccatgccgaccgacacaaccgcgtgcgtcggcgtggcctcaagcacgcggatcgtcttcacaccggcgcgggtgtccacgtcaaactcagaggccgtttccaacccctcggccaccaacacgtgggcgaaggcgcggatgccgttgccgcacatctcagcgacggagccgtcggcgttgcggtaatccatgaaccagacaccgcctcgccgaacgacacgcagcaaaccgtcgccgccgatgccggcgcggcggtcgcacagaaacgcgacctgcgaaggtgaaagcgtcagctcgtcgtcgacgtcgacgacaacaacaaagtcgttttcggtggcgtgggctttgatgaacttcacgaaagggagtgtagcgcggcgtcgacaagcaatggctcccacgcgtccagccactgcacccgcgggtcccgattgaaccacgagcgttggcggcgcacgtagcggcgtgtgccggtgatggtttgctcgtgggcgtcggcaagcgaaagctccccctcgagatgcgccagcacctgcgcgtagccgatcgctcgccccgcggtggaatcgcgcgtcaggcccgcgtcaaccagcccgcgcacctcgtcgacgaagcccgccccgaacatttgccgcgtgcgcagctcgatgcgcgggttcagccacgcggcatccgtgcgaagccccacaatccgcgtgccccagcgcggcggcgcgtccttcggcggctgcgacgcctgaaacggccgacccgtcagcgcaatgacctccagcgcgcgcacggtgcgccgcgggtccttgtcctcgatgacccgcgccgccgccggatccacctgcgcaagctccgcgtgcagcgcgtcgacgccgatcgacgcaagccgcgcctcgtagcgcgcgcggacggcggggtcggtggggggaaacgaccagtcgtcgataagcgactgcacgtacagcatcgaacccccaaccaggatggggaccttgccccgcgcggcgatctcctccaccgcggcgaccgcgcgccgctggtaatcggcgacactcgcggtgcgcgtgacgtcccaaatgtccagcaggtggtgcgggatgccgccgcgctcttccggcgcaagctttgccgtgccgatgtccatcccgcggtagagctgcatcgaatcgacgttgaccacctcgccgccgagctcctgcgcgagcgcgatgccgagggcggatttgccgctcgccgtcggcccgaccaccgctaccggcgctaccactgccacacccccacgtacctaccgacaccgagcgtcgcgtcggaggcgatcaactcagcgcgcttcggcgtaagctgcgcaagctcgcgccagagcagttgcttatcgacgcccccctcaagccccccaagcgcccctccggcgatgaaccgctcgagtccctcgtgcgtagcttgcgcgccgggctggagcgcgagcggcgcgcgcgctgtgagacccgcggggccgtcgacgaccacgatcgtgagcgcgtccgggtcaaggggttcgacgtgctcgcgcgtttcgcggtactcgcggtcgcctgcgacgtagcgcgccagcagctcgccgaggtagttgccgccgccgacggtgacgtgcggcgcgccccacgcgtggaagctaccggtgtgggcggtgtacgacgcctcgtcgagcgtggtgacgatgtccacggggccgcgatgcgctcgggccgcctcgcgcgcggcggcgagcagccgcgccgatgcctcgtcggcgggcgcgagttcgggcaccagcgccggcgagccgggcatgatcaaaacggtcgcactcatcgcccccaccctagtcagggaaatgctgcaccggcgctaccgctgcgcgctaagctaaatcgatactggcagccgcgtcgcgcggcactgaagagacgaagcgaaaggatgcgcgtcccatgacccacccgaacgaggacaaccgccccaccccgaagcccggccccaagccgggtccgaaaccgggcccgcgccctggggccaccccggcaccggcgccgcgcgagacgcctgcgaagttcgggcgtatcgacgacaacggcaccgtcttcgtcacccgcggcggcgtggagcgcgagattggttcatggcaggcgggtacgccgcaggagggtctcgcccactacggccagcgcttcgacgacattgttaccgaggtgcagcttctggagacgcgcctggcggcgaacccggaggacgcgtcccagatcagcaaaaccgcaacggcgctgcgcgactcgctcgctgacgccgccgcgatcggcgacttcgacgccctcgaggcgcgcctgaacaaggtcatcgccgacacggacgaggccggcgcccgcgccaaggaagcgaaggcggcccgccgcgccgaagcgatcgcgcgcaaggaaaccctcgccgccgaggccgaggacctggccgagaactccaccgactggaaggccgcgggcgaccggattcgcgacatcctcgaggagtggcgcaccatccgcggcatcgaccgcaagaccgacgacgcgctgtggaagcgctactcccgcgcccgcgacagcttcaaccgccgccgcggcgcccacttcgccgagctcgaccgcggccgcgcgcaggcgaagcaggtcaaggaggacctcgtcgcccgcgccgaagccatcaaggactccaccgagtggaacgagaccgcccgcgctttccgcgacctgatgcaggagtggaaggccgccggccgcgccccgcgcgacgtggacgacaagctgtgggagcggttccgcgccgcccaggaccacttcttcgacgcgcgaaacgccgtcaacgccgagcgtgaccgcgagttcgaggcgaacgcccaggccaaggacgcgctgctcgccgaatacgattcgctgatcgacccagcggccggcctcggcgccgccaaggcaaagctgcgcgagctgcaggacaagtgggaagagatcggcttcgtcccgcgcggcaaagtgcgcgagtacgaggacaagattgccaagatcgagcgccgcgtgtccgacgctgaggattcccgctggcgccgctccgaccctgccgcccaggacaaggtgaaccagttccaggcccgcgccgacgagttcaccgcgcaggccaacgccgccgaggcgtccggcaacgccaagaaggccgccgagctgcgcgagcaggcgaagcagtggcaggagttcgccgacgtcgccgcgaaggccgcaaacgagcgctagtgcccgcactgcactttgtccccggtgccgccgacttcaacgaggcagtcaccggggcgtacgccttttcggccacgctcgcgatccaagacatcaccggcctggccacctctggggtgacgccgtcgcacattgcgaaacgcctcgagggctccgcggaatccgaggcgctgctgttcgcgctcaccagccgcaccgcgccgcgcccgctcggcccactcggctacccgcagctcactcccgacgacctcctcgatatcgacgcgtgggtcttcgtctcgctgcccctccttgaagacctctcggtactcgaagccaacgtcaccctcgacgcggccatcgcaccgctgcccggcgaaccggttccggattcaccctggcaggaagcattcttgcttatcgacgccctgtcacactccctccaccgccccacccgccaactgtgggtcacgcactcccccggcgaatggaccccacctggcgccctcgaacgcgggtacgctgcggcgttccgcgaagatcaagcggtgttcgacgctgacgcggcgctcgcgctgcctgcgcatccccaccgcatcgacgtgttcgagggccccgggttcgcgggcttcaccgcgcccgctacgtcgctcagcgacgacgccgcccagttcgcgaacctgctcacctccgcctcccgcgactacccacgcggcgacctcgtgatggacaccatcacgtgggacctgcagaggatcatcgacgccggtgagcgcctgggcgaccgcggcggccggcagctcaccggcgtgtgccgcgcacgcacggcagacggggccgagacgatcgttgggctttgcgaggccgtccactacacctccgacgccgacaccgtttgcgagcttggcctcatctacgtcctccccgagtaccgcggccgcggcatcggtgaggcgctcatccgcgaaacgatcgcggccgcccgcgcacgctgggaaaagctggacacggtgtacctctcctaccccgccgacatcgcggcggcgcagagcatcgccgcatcgcttcacgcggacacggtttcctccaccaccgcctggcagcgacgaggtacgtaacgggctactgctgtttgtggcggcgggcggcgcgggcgcggcggtcgtcgacaagcagcgggttcccgctgtgcgattcggtggcagcgcgctgcagctgggcaagctcgtcgctttccggcggtgcgctctgggtgctggacgcctcggctcggcgggtgattgccggtacgtatgcgaaaacggcgatcaccacctcgaccaatgcaacgtaaaagccagggccgtggccgatgtcgaggagcgccgtggtgttgcgcagccacatggacagcaccgcgaacacgagcgacatcgcggtgagcacccaccccacggcggcaacgcggtagcgcttcgtcagcatcgccacggtaccgagtacgcctaacccgataagcgagaaccacgcaaaaaggtactccgcgatgttcgcgcctgcatcgcgcgcagcgtcggttgccgcgaggaattgccaccctcgcgcagacccggcgaaaggaaggaaaaacgacacgacaacgccggcggcgcaggtgaggagggtgggtttgaaggggccgtcggcaagctgtgcttcggtcactgtggtgctccgatgcgtagcgtcggcaagcctaagcccactcccgtggtggtgggcacctgaccgatctcggagttatcgccggccttcgtgcggcggtgctcgtggacgccggaatccgcgatcaagaagtgcggtttggcgtcggtgacagtcacggtgacgtaatcgccggggcgaatcccctcgttgccgtcgagcgagaagtgcaccaggcggccatcgcgggcgcggcccgacatgcgctgcgtgcggtcgttcttccggcccccgtcggcctgcacgagcaactcttgctgcgtgccgaccagcttcgcgttctcttccgcgctgatgcggtcctgcagcgcgacgaggcgctcgaagcgctcctgcaccaccgccttcgggatctggtcagtcatctcggcagccggggtgcccgggcgcggcgagtactggaacgtaaacgcggaagcgaagcgggccttctccaccacgtcgagggtggactggaaatcctcgtccgtctcgccggggaacccgacgatgatgtcggtggtgatggcggcgtgtggcagcttctcgcgcacctcgtcgagaatcgcgaggaacttcttcgagcggtaggagcggcgcatgtccttgagcaccttgtcggagccggattgcagtggcatgtgcagctgcgggcagacgtttggcgtctccgccatggcgtcgatcacgtcggaggtgaactccgccgggtgcggcgaggtaaagcggacgcgctcgaggccgtcgatctcaccgcaggcacgcagcagtttcgaaaacgcggagcggtcgcgcggggtgtcctcgtcgacgaagttcacgccgtacgcgttgacgttttggccgagcagcgtcacttcggacacaccttggtcgaccagcgcctggacctcggcgaggatgtcgcccgggcggcggtcgatctccttgccgcgtaacgacggcacgatgcagaacgtgcacgtgttgttgcagcccaccgacaccgatacccagccagcgtacgacgactcgcgcttcgccggcagcaccgaggggaaaacttcgagcgcctcggcaatctccacttgggcctcgtctgtgacgcgggcgcgctccaggagcgctggcagcgcagataggttgtgcgtgccgaagacggcgtcgacccacggcgccttcgtgatcacgctgtcgcggtccttctgcgcgaggcacccgccgacggcaatttgcatgccggggtgctgctccttggtgtgcttcagctgacccagcgagccgtagagccgcttgtcggcgttgtcgcgcaccgcgcaggtgttgaagacgactaggtcgggggtgtcgccggcgggggcggcgacgtagccggcgtcttcgagcatgcccgacaggcgctccgagtcgtgcacgttcatctggcagccgaacgttcgcacctcatacgtgcggttggtagtagacacggcacgagagtctaacgccgcgacgtggtcaaacgaaaacgtttgcgcgacaatggtgggcaactgttttgctgactcaggagtttttcatgcaccgtgccatccgccgcgccgcggcgtccgtcgttaccgccgccgccgcgctcacccttgccgcttgctcaggttctgacggcaaccccgaggccgagggcttgctggcgcggattgaatccggcgaggtcacagtcggcatgcgcgaggacaccagcgcgatgggcaagttggacgaggcaatcgcaacccacgtcatcaacgcgatcgcgaaagaccgcggctgggacgcgcccgagatcacgtgggcagagacactgccggcgaagcgcgaggagatgctgacaagcggcgaagtcgacatggtcgccgcggcgtactcgatttaccaggagcgggcggagaaggtgagcttcgccggcccgtacgcgattacgcaccaggcgctgctgatcgcagccggcaacacggagatcgacgggctcaacgatttgcgcggcaaggtggtctgctcggcgaccggctcgtggtcggcgcagatgatcctcaccacgcaaagggacacggaggtgcgcgaacgcgacacctacaccgagtgcgtggacgagctgcgcagcggccgggtcgacggcgtgaccacggacgagctgatcctgcagggctacgccgctaacaacccgggcgagttccgcatcgtggagctggtagaccgcggcacgccgctgaccatggagcgctacggcatcggcgtgcgcaaggacgacacgcaggtcacagacgagatcaacaaggcgcttggggcaatgcttgacgacggcaccttcgaccgcctcaccgccacccacatgcccgacggcgtagaggtggaaaaggacgtgcccggggacctcgcgtacttgaactagggcgagatctacgtgaggcgggcgatcgcgtcggcaagcgcgtcgatctgctcgagggtgtgcgtcgccatgacggtcacacgcagcatcgccgcgccgcgcggcaccgttgggtagcggatggcgggcacgaagaagccctcttgacgcagctggctcgatgcgagctgcgcggcgcgttcgtcgcccacagggacggggatgatcggcgtgggccactgccccatcccgagccggccagcgaggtgggcgatgttgcggtgcagggcgggcaccgggctttcggcgctgtcgatcacgccgatcgccgcagtcacggcggcgcaggtggcgggcgtgggtgaggtggagtacacgaacggccgagccttctgacgcagtagcttggcgacgccctccgaccccaacaccgcgcccccctccacgccgagcgccttcgacgccgtggcgacgaggatgtcgggccgcgcttgcggatccgcacccagaccgaagtgctcgatcactccgcggccggtggcgcccagggtgccggtgccgtgggcgtcgtcaaccatcagcgccgcaccgtatctgcggcatagcgcaaccatgcccgggacgtcggcaacggtcccgtccatcgagaacagcccgtcggtgacgacgaggacgcgcgtcgccggctccgccgtgtgcgcggcgaggagctcctcgaggtggctcaagtccatgtggcggaagacgtggacccgcgcgcccgcggctttggcgaggcggcagccgtcgatgatgctggcgtggttgcgttcgtccgaaagcaccacaagctgcggcgacgccagcgtgtgcagcaccgcggtgttcgcgtggaacccggaggaaaagaacacggcgtccgggtagcccgtaaagcgcgcgaacgcctcctccacgccccggtgcagttcggtggtgccggtggtgaggcgcgagccgccggagccagcaccgtagacctccagagcgcggcgggcggcgacgaccacagccgggtgctctgcgagaccgaggtaattggatgaggagaagaggatggtgggcgcggcgtcgataagcgcactcggctcctgcgccgaggaaaacaccgcgggtgtgcgctcgaggccgtcggcgagccaggcggtgagcgtgtcgtctgcggcggtgtctatccagctcaccgctgccccaccaccacgggcgtgtgctcgaggtactccacgaggtcgcccggctcagccacgacgaacacgcggcccccgatcggggaaccggccggcttcatgttcgggatgcggacgtagccgcggcccgaggtggcgaggtagccggtggtgtagtcggggtcgtcggagatgcacacctccgctagcaccgccgggtggtgcgcaaccttcgaggccagcaccagcgcctcggagacgcgggccttgccgtccgtgtccgggggcgcggcggcatccatgttggtcacgcgcacgccgcgcttgtggtcggcctcaaggcgggcgccggttgcggcgcccatgagcaccgccccacgcatatcccgcacctcggtcagcagctgccacgcgcgctcggcgtggacggtgtggtcttcgagcatccccaccaccagctcgcgtgcctcagcgggagaggcgcactcgagctccgtcacgggcaagaacgggacgcgcacaattgcttcttcgtcgactgcagccaccgtgacgtgaatttcgtccggctggcccttcgggtgggaaagtgcgcgccgcgtcatcgcgtcgcacaccccgccgacgcggtcggcgtccacgatgcgctcggcgccggagacgtgcacgccgccgcggctggaacgcattttcacgctgaacaacgacatgcgcctcagtctaaggcgcgggcctactcccccgtgagcgtttcgatccgcgcgtccaagctctcccgcgccacccgcatcgttagctcgctgccgtagccgcggcgggcaaggacaccgacaacacggcgcagcaccttgtcgtactcggcgcggtcggccggtggtgctttgacctcgcgcgctttcttctccgccagcgcgcgggcctgcgcttcctcgtcagcgggcgtcacctgcgccaaggcctcggcgcggatgtcggcggcgactcctttctcccgaagttccaagtccagcgcgcgggtggatttcccccgggtgcgcgagcgctggcggacccattcggaggcgaagaaggcatcgtcgataagcaaactgctctcgagtgaatcgagcacctcgtccactaacgcgggctcgaactccagcttgaggaggcgctcgcgaagctcgtggcgcgaacgcgcgcgctgatcgagcagtagcagcgcccgcttgcgtatcggtgcgagctcttcctcccggcgggtgtcgaagatctccccgccggtgaagttctcgatcgcctcctgcagcttggcgatcttgtctgggttaggcgagctcgccatcgccctcgtcgtcatcgtcgaaatcgatgttcggaaccatgtcgatcgcgtcgtccgtcagggcgtcgtcctcagcgctttgccccgcgtacttgcccacgccgagtgcctggaagatcttgtcctcgatctcgtcggccagatcagggttgctcttcaaaaacaggcgcgccttctctttgccctggccaagctggtcgccctcgtaggtgaaccaggagccggactttttcacaatgccgttgtccacgcccatgtcgatgattgagctctcgcgcgagatgccctcgccgtacatgatgtcgaactcggcgaccttgaacggcggagacaccttgttcttcaccaccttcagcttggtgcggttgccgatggaatcctggccgtccttcagcgtctgaatgcggcgcacgtcgcatcggaccgacgcgtagaacttcagcgccttaccgccggtggtggtctccggggagccgaacatcacgccgatcttctcgcgcagctggttgatgaagatcgccgtcgtgcccgagttgtacaacgcgccggtcatcttgcgcagtgcctgggacatcaggcgtgcttggaggccgacgtgactgtcgcccatctcgccctcgatctcggccttcggcgtcagcgccgccaccgagtcgatgacgatgatgtcgatcgcgccggaacggaccagcatgtccgcgatctcgagcgcctgctcgccggtgtccggctgcgacaccagcaggttatcggtgtccacgccgagcttcttcgcgtaatcggggtcgagggcgtgctccgcgtcgatgaacgcggcgatgccgccggcgcgctgcgcctgggcgatcgcgtgcagcgccacggtcgtcttaccggaggactccgggccatagatctccacgatgcgcccgcgcggccagccgccgatgcccagcgccacatcaattgccgtgttgccggaggagatggactggatcggcgggcggttttcctcgcccaggcgcatgattgcgcccttgccgaagtccttctcaatcatcgccagcgcggcgtcgagcgcgttctggcggtcgttgccggccgccgcggtctttttcttcgttgccatgtgtttctccttgtcgctttcagctattagacgtccgccgccaccgcttcggttccatcactctggcggtttgacctgcgggacacagtagaggccggtgcaaacattgttgaagatacacgcacgcgtgttcgaaatcctattcgacacaccggttcaacacgccgctaccaccccggccggtccaccccgagacggcggtcctccggcacgtcgaaggagtcgcacaacccctcccagacaacgcggggatcgacaccactttcgataagctccgcggccgtcttgtcgctctgcggcagcacttgcgactggatgatccactccgcgcgctccgcgccgaactcgtctcgcacgagctgatgaaattcggtcaatcgcatgccataaaacctacaggaggtactgttttcgccatgacttccgctgcaggcgcacctactccgcgcgccaacaacaccgcggccgacatcgcgtacatcgcggtgtttgccgctatcatcatgatcctcggtttcgtcgccatcccggtgggcgcggcgggcgtgccgatcgtgctgcaaaacgccgctgtcattctcgccggcttggtcctcggacgccgccgcggcctgctcaccaccgcgctgttcctgcttgtgggcatggcgcttccggtgctcgcgggcggtcgcaccaccatcagcgctctcggcggcgtgacggtgggctacctcgccggttacctggtcgcagcgtgggccgccggcgccatcgcctaccgcgcgccgtttagcaacaaccgcggcgcgaccatcgccgtgctggccctcgccggctacgtcggcctcttcctcgagtacctcttcggcgtgttcggcatgatgtggcgcctgtcgctctccttcggcgaagcgtgggcagcccaggtgccgttcttccttcccgacgcgctcaaggtcgccctcatgatcgcgatcgcggcggcggtccacgcagcgttcccggacctgcgccgcacgcgctagaccatgcccaccattgagttccgcggcgcggcggtttcctacgacggccaaaccgttcttcaccccctcaccgccacgctcaccgagcgccgcatcggcatcatcggttccaacggctccggcaaatccaccaccgttaggctcataaacggtctcatcgagcccaccacagggcaggtgcttgtcgacgccctgtccccctccaccaacggcaaagaagtccgccggcgcgtcggttttgtcttctctgacgcagaatcccagatcatcatgccccgcgtggccgacgacgtcgcattctccctgcgccgcttcaagctgccgcgtgcggaggtcgacgcccgtgtcgccgcagttcttgagcgcttcgggcttaccgacctcgccgggaactcgccccacaccctctccggcggtgagaagcagatgctcgccctcgcctcggtcctggtcatcgagccggagaccattatctgtgacgagcccacgacgctgcttgacatgcgcaaccgccgccgcatcatcaacgaacttgaggcgctcgaccagcaacttatcgttgtcacccacgacctcgccatgctggaggatttcgatcgggtgctggtgattaacgacggccacctcgtcttcgacggcgccccagccgaagcaatctcctactacaccgacctgatggacgcatgattcgcgaactccctttgggcgtttacgtcccaggaaacacgctgctccaccgcgccgatcccgcgtggaagtttgtggtgctcgtcgtcttcatcgtgctggcgtcgtttttgccgagccaaccgtggcacgcaatggctttcatgacgctcgtggttgtctgctacgcgtgggctcgcatccccatggtcaccgcgtggcggcagttcgtgccgctgctgcccatcctcgtgttcttcggtgcgttcctttggtggcaaaacgggctggggcagatgctgacgagcttgatcagcctcgtcgccaccttcgccgccgcgaacctgcttaccctcacgaccaccgtggaggagttactcactgccctcgataggtcgctgcaacccctcggccgcgtcggcgtgcgcgtggagctgatcagcctcaccatcgccttgacgattcgcctgatccccctcatgctgcaaacggccaacgaggtcctcgacgcgcgcaaggcgcgcggcgccgggttctcgttggccgcgttcggtatccccctggtaatccgcgctgtgcgccgcgcccgcatgatcggcgaggcgcttatggcgcgcggcgcagtggactagacgcgcttaggcgacgagcttgcgcgcctcttctatgatcggcgccgcctgcgggtaggcgttcgcaaccgcgtcggcaagcgggccgaagatggcagcccagatgccacccagcaccagcgccgggatcaggatcgccgccgccaaggagccgacggtcgaaccgacgacgaactggctgctgttagagctgccagccgagccctgcggcttcggagccggcgcaacgacagtcgtaggaacaacaacggtggtcggcacagtcaccgtggtgggaaccgcaaccgtggtgggaaccgcaaccgtggttgggacctcaatcgtcgtcgggacctcaaccgtggtcggaacctcaaccgtggtcggaacctcaaccgtggtcggaacctcaacggtggtcggaacctcaacggtggtcggaacctcaacggtggtcgtcacgatgacgcagtccttcgagaccaccgcgatcgcgccacggagtgcgatgttgttggtgtggccgtcatcggcccacaggtagcgggtcgtggtggtctgcttgccatccacgcactcgcctacctcgcggcgggcagcaaagccttcgttggcgaagttatcggtccctgcggggcggttctgcaccttggagacctctttgaactcggtgccgttgtgtgccaggaggatggattggccgaagcacacctcgtcgcaaagcactcgcagctccttggccgaatcctcccaatccagcgccatgacgcccttgaacggggacttgtagcgctggacgagcttggtggagccgttgtctccgagctcaacgaagaggacttcgccggaggactcgacgccgacggcgtacaggttggtgccgatgcctgggatgtaggagatcgcctccaggcccgagttcgcgccgaccttgccggtgtgttcggcgaggttccactcgtcggtagccttcagctcgccgctggtgccggtcggcaggtcgaagcggagtaccgacgggcgggagacgttcttgtcgtcgttgttgcgctcggtggcgacgtagatcgcgccgtcgtggccgatggtgacaccctccgcatcgggggtgccggtgccgtcttggtagcgcagggtccaagtgccggcaacggtgtaggtgtcgttgtctgcgtcgtaatcaagggcccagagggaaccctggccgttgttcacgatccaggcgcggccgttctcgtcgaagtcgacgccggacatgtcctcgatgttgaagtcggcgccgaggtcgatgtccttgatctcgagggcggcgtgcggccacgcttcggcctcgagcggcgcgggttcggtgtacgcctcgttggcggcctccggtgtggcgttggtgttgacgaaatcgccggtaccgtccgggatgcggcccagggtgtcgggggcatggccctcccaggtgtgctggtccacgagctccttacctgggttgaagaggcggacgctgtcgttgccgccaagaccaaagcccttttgcccgccgagtacctcggtgccctcggtgtagaagcggtagaaaccaccaggctggagctcggtgccggcagggataacgagcggatcgtgcttgtcattgtcatcgagcacgaaccactgtgagagatcgacgacctcgttaccggtgttgtagagctcgacccagtcgccgaactcatcgccgttggattcgatctcgttgatcaccacggttgaggccagcgggatgtcatcttggttttccacgatggcgacgttggccgcgccgcgcgttgccttgccggtcaccgcgaagttgcctgtcatgtccgggaggcggccccacgaggtgttcgcgccgttgtgctttgcgtgctcggcatacttgaacgactcaagcaggttgccgtcggcgtcactgaggttgacctcgtcaccattgcccagcccaaagcccttcgaaccgtccggggtgaatcccttttgggtgtcgaagacgtaatagccgccggagggaatcaccgtgtcggggagcacgatcggggcatgcttcggatcatcgtcaaccacggaccagccgccgatattgacgtcgccatccgtgggattggcgagctcgacccagtcggactcggcgccgtcggaaacgacctcgttaatcacgacgcgcagctgttcgttggcggcctcgcgggtggggcgcaggctcttttccagcttgtcgccgacgcggatccacgaggtcttcgtgccgtggacatcggcgtgcgcgttccagctctgggtgtcgacgacggcgccggaagcgtcgcggatggtaatctcatctcccttgcccaggccgaagcccttgcttccgtccggggtttgcccctcttcggtgtagaaggcgtagtacccgcctgcaggaaccacggcgtcggacgggaaagtaattgcgacggatttcttgccgctgtcgatggcggtccagccgccgatgttgatgtcggtgtcgccggggttgtacagctcaacccagtcggccacggggtcgccgttggtgacgacctcgctgatctgaatctgctggtcggccgcggccgcgccggggacggtgagaaaggtaaacgccagcgccgcggtgacaggagccgcgaggacagcgtggaaacgggaaagcgccatagaacttccttggtgtgaggtgtgaacaaggttctcgccaaggctatggatgctcggtaaacgttaagtgtcaccgaggtggctaacgggtgaaagaacgcgaaacccccaacgcggcgggtggccggttgggggtgggcgtcgacaagcttaaccttctccgcgcagctcacgcatgcgctgcgcgaccgcgtcgtcggagatctgtgctcccgccgggttggctgcaccggtgttggaggcgccgccctgctcgatcgccggcttggcaccggaggtgagctcaccggccatctcagcgcggatttgctcgaggcggccgtggcctgccatctggatgccggcctgctcaacctcagccatgcggccctcaacggagttctgcgcaagctccgcggcgccgagcgcgttggcgtagcggcgctcgatcttgtcgcggacctgatccaggttcgggcccgatgcagtgatggagttcatctgctgcatggtctcggagaccttctcctgcatcttcgcctgctcgagctggctgagcagcttggagcgctccgcaacctgctgctgcaggtgcgcggcattgcgctcgacggcctgcttcgcggcgccagcctgctgcagcgcctggtcgtgcagctgcttggtgtcctcgacaccctgctcagcggtcaccagctgggctgcgaacgcctcagcggcgttctcgtactcctgcgccttctggttgtcgccggctgcgcgggccttgtccgcgagctggagggcctggcgggtgttcgcctgcagcttctccacgtcctcgaggcggcggttgagctgcatctccagctggcgctggttgccgatcacggcggcggcctgctggctaagcgcctggtgctgacgctgcgcttcgctaatagcctgctcgatctgcaccttcggatcggcgttttcctcgatcttgttgtcgaagagcgccatcaggtagttccagaatttcttgaacgggttcgccatggggcgttctatacctttcgtgggagaattcaacgagttctgcattcccactgtagacgcgaagcgcccgccacgcttgcgccaggtattacacctcagcggcagccggggtggtggcgctcagttcatcggcgatagacgtcagtgacaggttcgacacggcttcgagcagcaggtccgcaacggatgtgtcgagtgcctcacagatcgaggcgagtacttcggatgagacttccttgcggccgcgctcgagctccgaaaggtagcccggggacacgagcgcttgggaagcgagttcgcgcagcgagacgcccttgtctgcgcggtaggcgcgcagtgacatcccgatcgcctcgcgcaacagcggctctttcgcccgccgcgccggagcaatgcgggcagggtcgagcgtgagggtgcggtcgagtctcggttcggcgagcagcgttgtagtggtcatcgttagtcctaacggtccgcgcccgcggtttgttcccgttcgatcgcgcgcagggctccgagcagcgcagcctcaacggctgcggcgcggatctcgttgcgctcacccgtgagcacgcgcagcggctccgcggagccgggcactagggcgtagcggcccgcctcggccggcaggagctcggcggcgagcgacgacgcagtccagttcggtccgctcagcccgatccacacctcccccaccgggtggccgtcttgaaggtcggggccggcaacgccggtgagcgcaaccgcccagtccgtgccgcaggcttttcggcagccgcgcgccatctcgcgggcgacggtcggcgagaccgcgccgcattcttgaatcacagcctcctcaacgccggcgagtgccgtcttcaagtcggtcgcgtaggtcaccagcccgccgcgcagtacgtccgaggcaccggggacgctagccagcgtcgcggttgccaaacccgcggtgagggattcgcaaaaagagatggtctggttgcggttgcggagggcgtcgataagcaaactgctcgtggtcacttgttcacctttcctgcgtcgacgaggtactgcacgccggtgattaccgtgaccaccgcggcgaggatcataacgacaagcgtcggggtgtccatccacgctggcagcgggcagaggtaaaggccgatgccgacgctttgcagcacggtcttcagcttgccgcctttcgatgccggcaccacaaaaccgcgccgcagcatcaccatccgccaagcggtgatgcccagctcgcggatgacgatcacgacggtgatccacaccggcagcgtggacgcgatgttcagcgcgaccatcgcggtaatcatcagcgccttgtctgcgatcgggtcggcgattttgccaaagttggtgactaacccgcgggcgcgcgcgatgtcgccgtccagcttgtccgtaatcatgagcgcgacgaacacaccgaacgcccaccaccaacgctgatcgagcaccagccacgcaaacacggggatgaagatgatgcgcaggctggtcagcacgttgggcaggttccaattggactgtgtggccgtagcgttactcacgcttcccaccctagactgcctgacatgaaatacttcgcttgcacctacacatatgtagacgatggtgaacttgtcggcgccacccgccccgcgcaccgcgagttcatcgcgtcgcagctctccctcgggcgcgtcgtcggctccgggccgtacgtcgacggcgggcaggcgctgatcattatccagctgccggacaccgccacgcaggccgacgcggaagcgatcatggatcaggatccgtacatcgccgctggcgcgctagccaagcgcgagatccgggagtggaacccggtctcgaacatcttcagctaagcgctacttctttccgccgcggctcacgtgcaggtggtcggtctcccgcgagccggtcgcagtgtggtcgcccttgcccgaagtcgccgggtcgtcgatccactcgatgtggtggccgtggcggtccaccttgcggcggttgccatggtcgtcgaagtcaatgtggtagctcgggccctcagggtccttcttgccggccttgacgtccgcgcggtccttcagcagcgatgcgatcgcggttactgcgagcacgccgacgatgacgagcagcgaggtcacggtgccgaactccggcacgttcacgccctcgccgccgttgatgaacggcaggttgttctcgtgcagcgcgtggaacagcagcttgatgccgatgaagcccaggacgatagccaggccgtacggcaggtacaccagcttgtccaacagcccgttgagcaggaagtacagctggcgaagaccgagcagggcgaacgcgtttgccgtgaagaccaagaacgcttcttgggtgatgccgtagatcgccgggatggagtcgaaggcgaacatcacgtcgatgaagccgatggccagaagggcaacaaacagcggcgtgacggccttcttgcccgcctcggtctgcgagaccaggcggtcgccgtggtaggacttcgtcaccggaataacgcggcgcagcgtcttcaccacgaacatgtcattcgggtcggtttccggctggtcggtcgcttcgtcgtacaccagcttgatcgcggtgtagagcaggaacgcggcgaagaggtagaagacatcgctccacgcctcgatgatgaccgcgcccagcaggatgaacagcagtcggaacaccagcgccatgacgatgccgatcagcagcaccttctgctggtacgcgcgggggatcttaaacgcgcccatgatcagcgcgaacacgaagaggttgtccaccgatagcgacagctcagtgatgtagccggtgtagaactccaccgcgtgctggccgtcccacagccaccacacgatgccgccgaaaatggcggccatggccatgtagaacagtgcccagccggcggattccttcacgctgggttcgtgcggcgtgcgcacgtgggagacgaaatcaaagatgaaaaatccgaggatcaccactgaagtgatgagccagattgacacaggaacgtgcacgtcgacctccggtctagagttacaaaaaacgaccggaggtctcccccacctgcgttaggtcaggctgctcggaccggggccgttgcttatcgacggcaccgtgctgacgattccgagcacttgcggggtactcccctccaacgtcaggccacattaccacgcgcggcgacgttctagaacgcgccgccggtggggttgtaggtagcggtgacagtgcgggtgtcgtcatcagcgggtgcgctttcaggcccctgctcctccttaggtgcctcggcggggtcggcacccttgatcatccactggatggtctccagctcctccggcttgaccagcacctcgcgcgccttcgagccctccgacgggccgaccacgccgcgggtttccatgaggtccatcaggcggccggccttggcgaaaccgatgcgcatcttgcgctgcagcatcgaggtggagccgagttgggaggtgacgacgagttcgacggcctcgaggaggtcgtccatgtccttgccgatttcctcgtcgatctgcttggcttccgcagccttgtcctcggtcacgccttccacgtagtcgggctcgtcctgggacttcgcggcctcgacgaccgcctggatctcctcgtcggtgacgaacgcgccttggagtcgctgcggcttgcccgcgccctgcgggatgaacaacccgtcgcccatgccgatcagcttctcggcaccgccctggtccaggatgacgcgggagtccgtcagcgaggaggtggcgaacgcgagacgcgacggcacgttggtcttgatcaggccggtgaccacgtcgaccgacgggcgctgggtggccagcacgaggtggatgccggcggcgcgcgctttctgggtgatgcgcacaatggaatcctcgatctccttcggcgccgtcatcatcaagtcggcgagctcgtcgacgacgcagacgatgaacgggtaaggccgcatctcgcgctgggatcccggcggcgcggtcagctctcccgagcgaaccttgcggttgaagtccttgatgtggcgcacgcgcgcggacttcatgtccatgtagcgctgctccatctcctccactagccactgcagcgccgcggctgccttcttcggctgtgtgatgatcggggtgatcaggtgcggaatgccctcgtagggagtgagctccaccatcttcgggtccaccaggatgagccgcacttcttccggtgtcgcgcgggtgagcaaagacaccagcatggagttcacgaacgcggacttaccggagccggtggaaccggcgaccagcaggtgcggcatcttctgcacgctggcggcgacaaagtcgccctcgatgtccttgcccaagccgatgagcatcgggtcatcttctgaggcgaccttgggggcgtcgaggacgtcgcgcagcctcaccatctcacggtcctggttcgggacctcaatacccaccgccgatttgcccggaatcggggtgagcaatcggacgttgtctgtcgccgccgcgtacgccaggttggactgcaggttggtgatcttggagaccttcacgcctgggccgagttcgacctcgtagcgcgtcactgtcgggccgcgggagaagccggtgacctgggcgtcgacgcggaactcctcgaagacgtccgtaatcgcctcgatcatccggtcgttggcttcagtgcgggtcttcggcgcggagccggggatgagcagatcggtcgacggcagcatgtagtccgaatcgcgcgcaacgcgcttcgcctgctgctgcgccggctgggcaggctggttctgagcctgggccttctccacctccgacttgggcgtggaagcaggcacagctgcggcgtcgatgccgctacgtgcgacgatggccttgcgcaccgcctcgcgcgagctctcgaccgcgtcgggctgttccgcatcgctttcgggttcttccggctcgcgtgcgggcggttccggctcgcgggcgggcggcgttgccggcctctccagcacctgcgtttcgttgtgctccggctgccgcggaacgatttcagtccgaggagcaggcgcgggcgcgggagtcggggtctcttcgacgtcgtcggcgaagtcgtagacctccggctcttcgttcgccgggtagttctccatcggggtgcgccgcggcgctggcggggcaggcggcgtggcgcggtggcgccgttggcgaggtgccgacgccggcgccggtgcgctctccgcggccgggcgctccgcgcgcggccggcgctcgcgcccctccgcaatatcgtcgaggtcgcgatcgacgtggccgtacgggtcgttgccattgtcgcggtcgccgtctgcggcggtgctgtcttcgcgattgaacgccttcgagaagaatccgacgatgtagtcgtagaactgccggacggtaatccccgtcgtcttcaacgctccgtagatgatgagcagggtgagaagcggcacggccacaaacggggtgaacgcgacggagagtgcgccgccgacaaaggtgccaattgcgccgccggcgatcttgcgcgattcccaatccgcgggcgtgcccgcgaaaacgtggatcatgccgagcattgccaccgcgatgatggaaagccccaaggcgactcggccgcgcacctccatcggggtgcgaacgttgagcatcagcgcgatcgccgcgccaaccaagaccaccggcaggatgaacgcgcctgcgccgatcacccagtggcacgcctgcgcaatggcgctgccgacgggtccagcgatatccatccacaccgacgcgccgataatggcggcgagcccgattagcaccaagccccacgcatctgcgtgggcggagacgtcaccttcagtgctgcggctgctgctgcggcgccggcgtttcggcttctcctgttcttcgtcctcgtcatcctggccctcgaacggatcgaggtcgtcttcctcctgctcatcgcggcgcttgcggcggtttgcgccgatgctggaaaaggcagatccaacccagcgccctgccgagccaatggagttgccgaccaccttcgtggcagaccccacccgctcgtccgctgtgtccgacgcaaccagagatgaggtcggggggtgcgtcatcgacacaggcgcaccgtagtcacgcgagcgggagtacccgccggtggtgtggctgcggggcgcggtcgacgagcgcgtcgagcggggagccgaatttttgacagacatgcatgtaactttaatacctcaagtcacattgcccacacgcgccacaccggcgcaggcgggttctgatgcgcccaatcagatccgcgaggagccagcccggtacaacaggttgttcagctccagctgcgcacgcagcccgaacgagatcaccggcgcgaagaacttcaccacggggtcgttggtgatgaccttgccgtagggcatgtacgacaactccgttgccttttcgccgtcgatgtagcaaccccacataccgcctttggcgttcatgaggcagagcaccgaatcctgatcgaactggccgagcacccggacgccgcggacgttgctgtcccggtacctcgggtccccgaacttcaccacgtcgtagctgcgccactgggtggcatagcccggttcgaaagggacctcggtgccggcgggaagcggccgcccacccgtccaatcagtgccgtcctgcgcgtgagcaaccggggataggacagcgacggcgcaaactagcgccgccgcggttttggccgtggtcttcatctacactccgcgttcgatcgcttctagttcggcggtgttgccggtaagggtgacgtcggcaaccgagcgccccgacacccacagcagcaactcccccggctcgcccgaaacccgcgcgacgttgtcgccgcgctccgccacgccggccttgccgccgagcgtgaccggcgggaggttcggcggcgtgagcacgacggggatctccgctttgcggaacgccatcaggccgaagcgcttcgcccacgtaagcagttccttgttcacggccgcgctgaactcgcgcgggttgacctctcccctgccccggcgcacgtcctcgtggtggatgaaatgctcggcggtgttcatcttggcatcgatcggcctcagcgccgcgggaggaccggccgcccactgacgcacgacatcctcgtacgggcgggcgagctgcttgcgggtctccgcatcaagcagttgcttagcgacgggcacgaaaatccccgcagccgccaacggcttccgctcgcggataaacaagtgggcggccaagtcgcgggtctgccacccttcgttgagggtgggtgcgtcaggtccgacctcgatgagcagctcgccgaggcgctcgcgttctctctgggcaaaagtcatgcgcccaagcctatctagaacgacgacatcgagctgaggcgcccgagcggcgagtacgcaattctgtcctggatctggaaccgcagcttgaacagcggggcgaagaacgccaccaccggatcggtagtcacgcggcgaccgttgtgcgcccaacccaggtcggtcacctccgtccccggcaaggcgcacgcttggacgccgcccttgttctccgcgcagaagatcttgtcgccgtcgaagcggccccacacctcaacggattcaccgtcgttgggctggcctgggcggaccacgtcgaactccctccagtaggtaccgtagcccagttcgtagggcacgggctcgccgggagcaacgagacggctcgcggcacccgcgggagcggcggcgagtgtgagggcggtgactgccgctacgccggcggcgagaagcgtatcggtggagcacataggaaacggccttccgttcgagatgagttggatctacaacctacatctttagtggacggaaggccgttacgcttagcggttgcgtctagagcgactctcgggaagcgtgcacgtcatcgtcgtcgtcatcaagcggcaggaaatccgcagccatcgggacgatggtcggcagaatcaccggctcgcgcttgtacttctgctcgatgccacgggagaccttgcggcgcagctgctgcaccatacgcagcgggtcgttctcaccctccgccgcgaggtcgttcatgacctgctcgacgccctcgacgaccttcttgttgaagtcgcgatcgtcgtccgaccaaccagtagtggacacggtcggcaccgaaagcaggcgacctgtgcggtcgtcgatcacgcaggtaatcgagacgacgccgccggaagccagcgaggtgcggtctgccagcacatccgggtcgacatcgcccatggtctcaccgtcgacgtagagctggccgacctggtactggccaaccaccttgatcttgcccttggtcatgtcaaccacgacaccgttctgcgccagcgcggtgttctccgggcgcacgcccgtggaaatcgccaactccttgttcgcgcgcatgtggcgccactcgccgtgcaccggcatagcgcaggtcggtcgcgccgcgttgtacagcgcgagcagctcgccggcgtaaccgtgaccggacgcgtgaacatgagcctcctggttggtgatcacgttcgcgccaatctgggcgaggttgttgatcactgcgaacaccgcttcctcgttgcccgggatgagcgacgaggacaagatgatggtgtcgttgtcgcggatggtgatctggcggtgctcgcggcgcgacatgcgcgacagagcagccatcggctcgccctgggtcccggtggtgatcaacaccgtcttgtgcggcgccatcttcgcggcttcctcgatcgggatgatcgtgcccttcggcgccttgagcaggctcatcttctccgcgatctccatgttgcgcatcatggagcggccgttgaacgcaaccttgcggtggttagcgacggccgcgttaatcgccatctgcacacgagcaacgttggaggcgaacgacgcgatcaccacgcgctggcgggcctggccgacgaggcgggtgagcgtttcctcgatacctgcctccgaggccgagatgcccggaatggtggcgttcgtggaatcgcacatgaacagatcgatgccctcgtcgccgtagcgcgcgagcgcaggcacgtcggtcggcttgccgtcgtacggcgtctggtcaagcttcacgtcaccggtcatgacgacgtggccggcgccggtcttaatggagacacccaggcactcggggatggagtggttgacgtgccagaagcgcacgcggaacgggccgacggtgatgtcggaatccttgttcacctcgtgcagcttcggcttctggcggtgctcctgcgtcttcgccgcgatcagcgcgttggtgaagcgcgaggagtaaatcgggatgtcgtggcgcagcttgagcagccacgggatcgcaccgatgtggtcctcgtgaccgtgggtgacgatcaaggcctcgaccttgtccagtttgttctcgatcggaccgaagtccggcagcaccaagtccacacccggctcgcccgagttcgggaacaggacaccgcagtcgacgatgaggaggcggccgtcgtactcgaagacggtcatgtttcggccaacctcggaaatgccgccgagggcgtagatgcgcagcgtgttcttcgccggcttcggcggcgccggcagccgcttggtcaggtcgttgccctgcatctgcttgaccgggttgcggcggtcccggccttcgccgccgttgttgccgcctccattgccgccgcggccgcgaccgcggcgtcggctgcggccgttgcctccgtttccgccgtggttgccgttaccgccgtggttgttgccgccgcggttgtggttctcgctgccgttgtcgttttgacccgcagcagcgttgtcgccgccctcccgggcggcgggggtctctggcgcctggaaaaccggctgctggtctgcaggttccggcgggccagccttgcgcgtcaccttgcgggcgcggttacggggttcattcattgttaaaggactccagccttttccatgtcgtctcggagagccgcaatctgttcctcggtcgcagctgcgacgggaagcctcgggtctccaacttcaatgccctgcaggcgcagagctgctttagcgaacgtgacgccaccgagcaccgcttggtgtcgcgcgagcacatcgatgacgttggcgttgatttcccgcgtgcgggcgaggtcgccggcctcgaaactcgtgatcatttcccggagtgcgccaggcgcggcgtgcccgacaacggagataaacccggtcgcgccgacagcaagccacggcaggttcagcgggtcgtcgcccgagtaccacgccaggtcggtgccagcgatgagctgggcggcctcgaagaagtcgcccttggcatccttcaccgcctgcacggtctcaagcttcgccagctccgcaatcgtcgcaccgtgaatcggaacaccagacctgcccggaatgtcgtacaggcagatcggcaggtcagtggcctgggccacggccgtaaagtgcgccaggaggccggtttgcgacggcttggagtagtacggggtgacaaccaaaagcccgtccgcgccagcttccgcagacttgcgggccagctcgatggaggtgcgggtgttgttggtgccggctccggcgatgagcttggcgcggtcgccgacttcttccttgaccgcagtaagcaccgcaatcttttcttcaactgaagtcgtcggggattcgccggtggtgccggcgaggacgagagagtcgacgccgttgtccacgaggtgggcagctaacgagcgcgcggcttcaaggtcgacgtcaccgttcgcgtcgaacggggtgaccattgcaacgcagacggtgccaaaggtttcagctccgcggttagctttcagtgatgtgcccatggggtaacagactacccccttgccccggcgacactcacttcaccacgcgagccggtgtgtgcttaggcaatgtagggactggtggccatccgggtgccgtcggcgaggtcgctgatgaggaagtcgctgaagaggactggcgcctcgccgcgaagcaactcgaggcaggccaccgctaggctccggatttcgacgtccgcgtgctccgaagcccgcgccgcgatgaaggagcgccacgcgcggtagttccccgtcaccacaaagcgcgtctccgtagcgttgggcagaatcgcgcgcgcggcttggcgggctttcttcgcgcgcagcagcgcgttcggctcggcggccatgttttcctcgagtgcggtgagcagctcgtcatggacgaagcgcgcctcgtcgaccgcgttcaagaacatgcggcgcagctcctcgtcgtccgcgatcgcctcggggacgactacctctccggcgccagcgtggacgtagcgctgcgagagctgggagaacgaaaaatggcggtgccgaagcagttcgttgcccgcgacccgcgacagaccgcggatgtacacggtggcggtggcgtgctcgagcagcgcgtcgtggcccacgtcgatgatgtggcgcaggtaggcgtcgtttgccctggtgtgcgggttgggcttgtcccaggtttcgtagcacgcccgacccgcgaactcgacgatcgcttctgcgtcggtggcggtctcgtctgcctgccactcgattccggagggcatgcggaactgcgacgccgcgatcaactgcacgtcaagcgtcgacgattcagccatctacagccccaggtaggcgtcgaggccaatggtcagccccgggtgctccgccacctggcgcacgccggtgagcacgcccggcacgaacgactctctgccgtaggagtcctggcggatggtcagagactggtcgcgggtgccgaagataacctcctcgtgagcaaccatgccggtcatgcgtaccgcgtggacgtgcaccccgtccacgttggcgccgcgggcgccgtctacggactgctcggtggcgtcgggcatcgggtccatgcccgcttcgagacgggcccgggcaatgccctgcgccgtcttgatggcggtgccgctcggcgcgtcgagcttgttcgggtggtggtactccacgacctctgcagactcgaagaacggcgcggcctgcttcgcaaacgccatagtcagcaccgccgagatagcgaagttaggcgcaatgagcacgccgacgccgtcggcatcagcgcaccactggcgcacctgctcgtagcgcgcctcgtcgaagccggtggtgcccaccacgcaatggatgccgtgctcgatgcagaacttcaggttgtccatcaccgcgctcggcgtggtgaagtcgacaatgacctctgcaccgctttccacaagcaggtcgagtgaatcgtccgaatcaatctccgcgacgagccccagatcatcggccgcctgcactccggcaacgacggcggaaccgacgcgcccctttgccccgaggactccaacttttatagccacgacccctaaaaacctccgctggctcatatagtggtgggtatgaaacgatcgtcgataagcataatgctccttgcttcgctcgctttgactgcctgcgggcaggcttccgtgccggagccggcgaccgtgacgcaggtgagcggttcaaccagcgttgcaacgtcaaccgtgaccgaggcggttaccgaggaagtgaccgcgacgcagaccgagcagaccaccgtcgaaccggcagacgccgccgcgacgaagtccgccttcacactcgacaccgtccgcatcccctctgagggcaaccccgagttggtcatcgaggacgtgcgcgccggcagccacgacgggttcgatcgagtcgtgttcgagtactcgggcccgggcaagcccggcgtgattgcgggctacaacccggatcctcgccagcaggcgtctggctacccgctcgacgtgcccggcaacgcgtacttagagatcatgattcagggcacgcccatgatgatgatgtccccgcgcgaagacctgatcccgaccgggcctgtcggcgttgctgcgggcggagtcacctcagtggtgcacggaggcgtgttcgaggccgacacccagtacatcatcgggctggaccgcgagcggccgtaccaggtgtacatcatggagaatccgacccgcgtcgttgtggagttccaaaagtgaacctgacctcctggttaggaatcggctttgtcgtcctgctggtggcgctcggcgcggcggcgcttggtgcgacgctgaggaagatcagcaagtccgacatggatgacgcgtcgaagtcgaagtggggattgttgatcgggctctcccctggcgcgggcttgtacgcgtggcaccgcaaggacgagctgatgggtaacggcgacggcgagcaggattcacggcgcgccgagctttaaaccccgcacgtgcccgacaacccggtgattccgctcggactaggccgctggtgacccgtgtctcaggcgcgactgcgacgtgttacggttcacatgtaggtagtccccgttgccgccgagcgcgcaacccgaagattgaagcccgcatgtccaacgacactcccgaatacaactacaacgaagacggcaagccggagcacggccacgtgacgaaggacttcgactcgctgggaaagttcgacgacgctggtaaccgcggcaagcgcgagctcaagcgcgcgccgctcggcccggattccctgctgtggcagtggggcgcagacaaccgtatccagctgctccgcggctacaccggcgtgctgcagaacatgcaccctgccatcggccagtcgcttctggatcactcgaagttcttcgaagagccattctcccgcctcgagcgctccaccccgcagatcatctactcgatctacgacgacggcacccgcgcgaagcagattcgcgattaccaccacggcattaagggcaagcttcgcgacggcagccgctaccactccctgaacccagacgtctactggtgggcgcacgcgaccttcgtttaccgcgtgatctgggcgcaggagcttttcggcaccccgttcacccacgaggagaaggaccagatcgtccgcgaaggcgtgacttggtgggacatgtacggcatgtcggagcgccccgtcatcgacaactacgacgagctggtcgcctacatggaggagatggaagacacggttctcgagcgcaacgagaccgttgacttcgctctgcgaaccgctcgcgtcgaaccggtgaaggcgccggacggcgtgccggaggctgtgtggaaggtgatctggaagccgctgatgaactcggtgatctggctgacctacggcaccttgagcgataagcagcgcgagatcttggatctgccttggaccgagaaggaccagaaacgcttcgaccgcgtggcaaacggggtacgcaagctcttcgagatcctccccgaggacaagcgctacatggagcctggccgctccatgatgatcaaggccggcatgatcgacggcgagtacaaggagccgaagctcgcgggcccgtacgtccaaggcggggaggcctcagcggaagccgggaagaccaatgacgccccgaaggccgcgggcgcggcgttgccgtcgcgcaagaccgcgctcgcagtcgctggtgccgcggccggtgtcgcagctgtgcgccgagctcgccgacgcgggaagcgccactaaggcaacttcaccacgaccccacattcaccgcggcgatcaaacgggacgagatcaacggaacattcccccgctcgctcacggatgtagcctgcgtgaatgtggcagatcatcgcatccggcgcggcgccatctgcgttgataaatgggcatgccctgaggcccactatcttgttttcccggaggtgcgggtcgaagccgagctttcgcagttcttgcaccgccgcacccagtgggtcttcgtactccatccacgttgcctcccttgggcggtccgatgggaggacgccccttccccacactcgcccgagctcttcagcgcgagtaattgcagccgagccgtcggtagattccgagccgcagagttgacctgcaagtacctggatgagctggacgtattcgtttgccagctccgatggttggggcgagcgaatcgaatacttcagccacggtcgacctcgatagggtgtctcctgagcctctgcggtgacaacccccgcatcgatcaacccgtcgaggtggcctcgcacggtattcggatgcgcagctaccgcctgagcaatctcggacacccgcgctgcgcctccgcattcacggattgcttcaatcacctcgcgttgtttagcgctggccgctgcagcttcttctgtcgccgcgtatgccgggcgcggcccggctccctgaccccggttgctctcatctctgaccactgtggacctccgtagcttcgcgcgtgtttgcccctacaccagaaatagtacgatgaaagccgtgaaaaatgatgggttcgcggcacaccgcaggtggcacagggtacttgcgggggtggtcatagcctggctcgttgccgccgtgtgcgtgaatgctgcggcgctaggcccaagcagcgcaccggtctcgcactgggcacgcgtgcacaccctgacaatcggggcaatcaccaccgcaatcgtcgggtactccgcccactttaccgcgacactcacacggggtccgcagccctcatacgtccagctaggcgcggagatcgccatcatccaagtgagtctcgtctggttcctgctccaccccgtctggactacagcaaactcggttttcgccgccacggtcgccgccgtcatcatctggcacgtgcgcacgctgacacgaatgatccgccgcgccttcaccaaccaccttgcggttaccgcgtgggcctatgtcatcgccggttgcttgcttcttgttgctgttaccctcgctgtgttggcgcagtactgtcgcaatcacgacgcattcatccacgcgcactcgcgcgcagccgtgtggggattcgcctggactgctgtcctcggcacctcattaaccctgctgccgacgctcactggaggacacgtcaatgtgaaagcccgcactcgttgtccacaggcgctgatcattcacgggattgctgtagcgctcgctgccacgtgtctcgctgcaggactaccgcgatcagcaggtgcatggctgctcatttccgccgccagctgcgcaagtctcatactgccgacacttgtcgaagtggttcacaaacacaccccacgaaacgcctcagccttgctcctgtggttcggtgttgtgtggctttttgcctgcctcgtgggcgacgccgtcttgctggccgctggtcatcttccacccagcctgacggccgggatcgccgttgcattgctcggcgcggggcttggacagacgctcctcggcgcactgtcgcacctcctgccagtgctcacagggcggccagcagccaaagagcacttggttcgcggtttggtggctcgaattgccctgatcaacgctggtggatgtgcggccattgcaggctttccggtggctggtggcgctgcagtagctgtagccggtctctggcacaccgcgcaattaggtatctctctcaagaaagcgagccaagacgcatgacacaacccagcccctcccacaccatgcaaagcaagaaggcatctcaccgcaacggcgctgtggcgtgggcagttgttgcgcttcttgcggttggcgcagtcggcggaaccctgctggtagacagctccggcccaggcccggtgcgaggacaagtgatccaagatgtccgaattaacggcatgagtttcgagcctgcaagcgttgtggttgactccagcacccctgtcgtcctgcggatcacgaacgacgacgaccgggagcacaacctcaaactcggcgatgggttctctggcccgatacaccctaacgacaccgttatcttcgacttcggcaccttcgaagccagcgagcaggggtggtgcgcgaaggcgggacacaaatcgatgggaatggtctacgacgtcatcgtgcagtgatcactgcacgctgcacctttacgcctcgcaccatgagcggcaagaacgcaacgaggcaaccaaaagccacgaggctgcacaggattgcggcgacagagttctcaaccgcaagccagcaaacgagcgcagcgttgaaaagcacagcccgtgtcacacctgcccgattcagttctgcgaggcctgcgcgggtggctgtcggcccacctcccattgtcgtaggcagaaggtaactcatcgtcccgaagagcagctgcgccgcgaaaccgagtagcaaaggaatcaccggcatctgaaggccgctaaggctttcccccgaggtaagaagcctcgcagcaaacgacacgcagaagacgaaaagccacgtcacagacgcaagagcagacaggctccagtaagtaacccggcccttccgctcgccgcgcaccccaagcagcgccgaaatccacccctgcagtgcgtatgcccacgaagctgcatacacaagcatgccgatgcccgctgtcaccccatggccaccgacaacgccggcgaccgccaaccccagcccagcgcaccctgcaatgagcatggctgatggctttccgagcgtgccgttgatacgccacatcgcgggaaacagcacggtcaatgacccggccgcggcgaaccctacaaacccgaagacattcagcatcacgtgcgccaacagcgcacggttctgccaagcgccctgcagatcggagaccagcagcgctcccagcaacgctcctacaaccaggcatccggcagatgcaacgtaaaagtcaaccgccggccggaaccgttgatgaggtcctgccgcccgaatctgacgcgcgatgacggccccgtgccacgccagaacacccgccacacctgcggctcctgcggcggagatccaccatgcccactgctgcgctggccctggcagcattcccaccaagaccagcacgacacaaaggttgagcagccgagagcggagcagctgagcgggacgctcgctgtcatccagccggcggtgcaaaaaacgctcagtgaggttctgcgaccaaacggtgattgagttagtcaaaatcccgagggcgaagatatggatcagcagccaccgggaacttggaacgaatgggtggacgagaccgacaaggatgaacaccaagatccaaaccgtaaccggtcgggacacgcggcgatgccagacccgaggactccacttgtcggtctcagagggatgatgaaggccaccgtgatctgtcataccttcaaaggtatcaatctgacggtgattactacggaaccaaccgtaaaaaataggcggccggatagccacccatttttctaccgccctttactcctcgccgtcctccactgggaccagcgagatcttgccgcggttgtcgatgtcgcggatctccacctcgaccttgtcgccgacgttgatgacgtcctcgacgttttcaacgcgggtgttgccgcccaagttggagatgtggatcaggccgtcggtacccggcaggatcgagacgaacgcgccaaaggcaaccgtcttgaccacggtgccgaggtagcgttcgccgaccttcggcatctgcgggttcgcgatggcgttgatgcgctccaccgccgcgtcggccgccgagccctgcgttgcggagacgtagatggtgccgtcgtcctcgatggtgatctcggcgccggtctcctccgtgatggagttgatggtcttgcccttggggccgatgacctcgccgatcttgttcaccggcacggtgacggtggtgatcttcggagcgaggtcgctcatctcgtccggaccgtcgatgacctcagccatggtgtcgaggatcgtctcgcgggcctcgcgcgcctggttcagagcgcttgccagcacgttggacgggataccgtcgagcttggtgtccagctgcagggcggtgatgaactcgcgggtgcccgccaccttgaagtccatgtcgccgaaagcgtcttcagcaccgaggatgtcggtgagcgcgacgtactcggtctcgcctttgacctcgccggagaccaagcccatagcaatacctgcaaccggggccgccagcggtacaccggcgttgtacagcgacagcgtcgacgcacacacggaacccatggaggtcgagccgttggagccgagcgcctccgaaacctggcggatggtgtacgggaactcctcgcgcgacgggatgaccggggtcagagcgcgctccgcgagcgcaccgtgaccgatctcgcggcgcttgggcgaaccgacgcggccagtctcgccggtggagtacggcgggaagttgtagtggtggatgtagcgcttcgactgctccggcgtgagcgaatcgatgtgctgctccatcttcagcatgtcgagcgtggtaacgccgaggatctgggtctcgccgcgctcgaacaatgcggagccgtgggcgcgcgggatgagctcgacttcaacttcgagatcgcggatgtcggtgacaccgcggccgtcgatgcggaagccctcggtgaggatcttctcgcgcacgatcttcttttgcaccgcgttgtacgccgcgcggatctccttagaggcggctgcgagctctgcggtgtcgtcgtcgtcgatgtcgaacttgtccaggagatctgcttcgatctcctccatgtacgcgttggactcgttctcgcgctcggccttgccggcgatcgtcatgatcttcgaaaggcgctttgcagccttcttctccaccgcgtcgtaaaccttgtcggagtacgccgggaagagcggaaactcctttgcgtccttcgcggcctccttggccagcgcggcctgggcctcgcacagcgtgcggatgtacggctttgcagactcgaggccctccgccacggtctcctcggtcggtgccgggtagccgtcgcgcaccagctggaccacgttcgcgccagcgccagcctcgaccatcatgatcgcgacgtcggactcagtcttgcggccgcgacggcgctcgacaatgcggcccgcaaccaccatctcaaacagcgctcgctcgtgctgcgcgtggttcgggaacgcaacccactgtccctcagggtgcttgtcatcggcgatcagcgccatgcgcacgccgccgaccgcgccggacaccggcaggccagacagctgggtcgcagcggacgagccgttgatggcgacgacgtcgtagtactcctccgggtcccagctcataaccgtcaccacaacttgcacttcgttgcgcagacccttgacaaaggtcgggcgcagcgggcggtcgatcaggcggcacgccagaatcgcctcggtggacgggcggccttcgcggcggaagaaggagccggggatcttgcccgcggcgtacatgcgctcctcaacgtccaccgtcagcgggaagaagtcgaagccctcgcgcggctggttggatgcggtgacggtggcgagcatcatcgtgtcgtcatcgaggtaggtggtcaccgacccgtcggcctggcgcgcgagctggccggtttcaaaacggatggtacgggagccgaaatcgccgttgtcaatggtggcgaccgcttcagtaatgccgtaatcctcgtcgacaaagacgtcgtacgagttcttcggggtaaacgtgctcaaaaaattctctccttaggcgatcatcgatgccgccgtaacgtgctctgactgttgaacggtctcacataatagcagctcgcatgcaaaacgggcccgcccccgtgaaggagcgggcccgtagagcctgaaaaacggcggcgcgactagcggcgcagacccaggcgagcgatcagggagcggtagcgctcaacgtcgttctcgcgcaggtacttcagcagaccgcggcggcgaccgacgagcagcagcagaccacggcgggagtggtggtcgtgcttgtggtacttcaggtgctcggtcagattgttgatgcgctcggtcagcagcgcaacctgcgcctccggggaaccggtgtcggtctcgtgcaggccgtactccttgaggatttcggccttcttctcagtgctcaaagccatgaggaactctccttgtatttcagttcgcactcgtgatgttttcttgcgccccaactgctgcgaaccacagtcaaagccgagaggcgatgttaccgtgcagctgtgccggcagccaaaccggtcaggcgttgcatgaactcttccaagaatctgtcgacgtccacgccgactgccacgtgggcggtcttgaccgggtcgttcaaccgcgtctcgtcgccgatggtgcggccgcgggtctccccctcggtgtccgttttcatgttgatgtccaaggtggtgaccaggctcgggtccacggcgacggcgacggcgagcgggtcgtgcaggccgcagccgccgaggtaaggcgcggtagtttcgtacgccttgatgtagtagttggtcgccgccgccaggaagtcgccgccggcggtgccaagctcggaccacttcgcagtctcctcagtggtcaaaagcgtctgcaacgtgacgtcgagaccgatcatggtcacgtccttcgcgcggcggaacagcaggtcggtggcctcggggtcctggttcacgtttgcttccgcccacttcgacacgttacccggcacggtgagcgctccgcccatcatgacgatgtgggcgcgctcggcgaaggtctcgctggcttcgatggcagcggcgatggtggtcgacggacctgtcggcacgatgaccaagtcgtcgccgtacttctccaccgactcgaccaagaagtccacggccgaggtctcctccaccgcgcgcgagggctccggcagatccgcctcccccacgccgttcttgccgtggatgaactcggagatctccagcacctcgaagctgtccttggcgcgggcgtgatcggggccggcgaagaccggcacgtcaccgcggccgaacagctccaggatggccagcgtgttgcgcacgccggtctccaccaacacgttgccgtaggtgccagtcacgccgatgaggtcgagctcctccgagccaagggcgtaggccagggcgagcgcgtcgtcaatgccagtgtcaagatcgagaatgattttgcgggtcatggcacccgactctacgcgctggtctcacgcaccgaggatctcgcgggtgcgggcgacgtcgcggcccatgtgctccaacagctcgtcgacggagtcgaacttcaccatgtcgcggacctttgccacgaactcgacgcgcgccaccctgtcgtacagatccgcgtcgcggtcgagcacgaaggattccacgctgcggcgctcgtcgccgaaggtggggttcgtccccaccgagattgcggccgggtagcgcacgcccggttccatatcgccgtcgatccgcgcgtcgtcgacgatggtcagccagccggcgtacacgccgtcggcgggcagcgccgcgccttccggcacgtactggttcgccgtggggtaccccagctcgcgcccgccgcgcccggcgccccgctcgattgcggagacgacagagaacggccggcccatgtagtcggtggccacgcccaggttcccccctgcgagctggtcgcggatggcggtggagcagatgcgcacgccaccgtcgtcaagcagctgcaccacagtgacatcgacgccgtacttctcccccagcgacgtcatggtttccggcgtgccctccgcgccgcggccgaacgtgaagttccggcccaccacgacgtgcttggcgttcaagcgcccggcaagcgtgtcgcggacgtaagactcggcgctgtctcctgcgagttcgacgcggaagtcgatcaccacgaggtaatccacgccgagctccgcgatatggcgcgcgcgctctgcaaacggggtgagttccgcgggtgccgtttcgggcgcgaacacggtgcgcgggtgcgggtcgaacgtcatcacgacgctttcaagccccagctggcgggcggtgttgaccgcctgggtgatcagcagctggtgaccgcggtgcaccccgtcgaagacgccgattgtgactacggttccgtccgggcgtccgaaatcgtggggcacctcggccagaccgcgcataatcttcacgcgacatagagtacggcatactgaaaaaccatgaccgatcccctcgaagcatctggcatcgtgattgtggacaagcccgcgggcatgacaagccacgacgtggtggcgcgcctgcggcgcatctttggcactcgcaaggtgggccacgccggcaccctcgaccccatggccaccggtgtgctggtcgccggcatcgaacgcggtacgaagctccttgctcacctcgtggccgaggagaaggtctacgaggccacgatccgcttgggcgcgtcaaccaccacggatgacgctgagggcgaggtcctttcagcggcggatgcatcgcacgtcacagacgaggcgattgcggcgggcatcgcggcgctgaccggcgacatcatgcaggttccggcgagcgtgtccgccatcaagatcggcggcaagcgcgctcacgagctggtccgcgagggcgccgaggtggcaatccccgcgcgcccggtgacggtgcacagcttcgactacaccgtccgccgcggcgagcacctcgacatcgacgcgataatccgctgctcctccggcacatacatccgctcgttggcgcgggacctcggcgcttcgctttcagttggggggcatttggttgctttacgacgcaccctagtcggccccttccccatcacccgtgcacacaccctgaaggacttggaagcgcacccggcgctgacgctgacgatggacgaggcgctcaccaccgcctggccggtgctagacatcacccaagacgaatacgacgcgctcgccatgggcaagtggttggagccgagggggctttccggcgtgcacgcggctaaaggtcctgacgggcgcgtcgtcgcgctggtgaaggagcagggcaagcggctcgcaaccaccttcgtcgcccgcccgtcgacgctgacgtagcactagataaagaacgccgacgcgatcacgtacccgccgcgcaccacccagcggccctcgaagtacggcgcgggggcggggcgggcaagcagctgggcgacaaacgtgccgtcggcgcgcagggcaatctccgcctcttcgaaccccagccagcgcctagtcagcgggaaccagcacttgtaggtggcctccttcgcgcagaacagcagccggtcggcccacgactggcccgcggccatcatcgccaagaccgactcgcgctccgccggcagcgcgatctgctccaaaacaccttccggcagcggctgcgcgggttccgcgtccagccccattgagcgcacgtagcgcgtcggtgccgccaccgccgcgcgcaggccctcggtgtgcgtgagcgagccggtgaaaccttttggccacagcggcataccccgctccccgcgcagtatcgcccccgccgtggtcaccccgagctctttcagcgcctggtgggcgcaccagcgggcgtcgccgaactcgcccttgcgcatgtcgagggcctccgaaacctgggcgcgttcactcggcagcaggtcgcggtagttggtcaggtcgcgggcgtcgtcgttgcgcaggtacaccacgcgcgcggcgggcggaaacaggcttacgtccctcatcacccctccacctccatcaccggatacgggaaggcaaggggcgggtgctcgcggtgctcccactcgcgcgggtagccgagcgagacctcaatgtgcttcaccccgtcgacttgcatgacccccggcatgtgcaggtggccgtagatcaccgccttggcgttgtagcgcttcggccaactgcgcgtgtgcctggtgccgcaccacagcgcgacttcggaccagcgcatcttcagcgtcggctcctgcacaagcggccagtggttaatcaggatcgtggggccttcgatccgggacagccgcttggtggtgtacgcgaggcggtcccagcaccacgcccggacgtcgacgaaaggggcgatggcgaactcgtccgtcatcatgatgttgcggcgccgggccgcggcaaccgcctcctccacgctcatgccgggtgcgcggaaggagtagtcgtacagcgtgaacagcgggcaaacggttaccccgccgaagaccgggtaggggtcctccggggtgatcacacccatctcccgcatggactgcaccaatgccgtgtacttgtcgcgtccccggtggcggtcagcggagcgggagaacagctcgtggttgcctggggcccagatgaccgtgtcgaatcgctcgttgagcttagccatgacccggacgatcaagtcgcttcgctcagcgacgtcgccggcgacgatgagccagtccgacgggtcggtcggctggatctcgtcaatgcgcggggaattcgccttcaccgccgcgtgcaggtcgctcactgcccacaaagtggtcatggaaggtttctagcacacagcgcgaagtctcggccgcgcagccggccgggttaggcccctgtgcgcgcccaccgcatcgacctgaaccgcagccacacgcccaccaagcggaagacaatggacagcaggtggccagtccaaatccccgtcagcccccagccgaactggacggagagaagcgtcagcggcaggaacccgccgagaactgaagcgatggtgaggttgcgcaggaacgcggcgtcggacgcgccgagcagcacaccgtcgagggcgaaaaccacgccacccgtgacgaccatggcgatcaagagccaccacggcacgcgaagctccgcgaacacagcggcatcgctcgtgaacaacgactggatcggccgggcgagcagcgcgaacaccgcggcgagggcggtggagaacagcacggagaaccgcgtgacctgcaccccgacaaaacgggcctcgtccacgttgcccgtgccgagggcggaaccggtaaacgtctgcgccgcgatggccaaagaatcgagcaccagcgtgagaaagttccacagctgcagcatgatctggtgcgcggcgagcaccgcgacgcccgacctgcccgccacggcagcggccgctaggagcgaaatctggaacgacagggagcgcaggatgagatccctgcccaacaccagctgctgcttaatcacgctccaccgcggcgcccagctgccgccgtagcgcaactgctcccggatcagcaccgcgaggaagaaccccgctgtaatccccatgccaatgacgttggctacggcggagccgaccagcccgtaccggctgaccagcaccggcaagaggattgccccgggcacgagcccgcacagcgtgagcatgaacggcagccgcgtgttctgcacgccccgcatccacccgttgccggccatgatgaccagggtgagcgggatcgcgaacgccgccacccgcatccagcgcgcagcctcggcggacgtggctgcgtcgttggtcaaaaacatcgcgagcggctgcgcgaagagcatgactagcgcagcgagcagcgcgccgacagcgagggcgacccaggtggcttggacgccctcagcgacagcgtcgtcgcgcctgcccgcgccgaacatgcgcgagcttcgcgcggtggtgccgtacgacaaaaacgtcagctgggtggtcaccgtggactggatcgcggtgccagccgccagcgcggccagctccccggtgccgagacggcccaccaccgccgtgtctagcagtaggtacagcgggttcgctgccagcacaccgagtgcgggcagcgacaacgtgaggatctgtcgcgcggtgatcatggcagcgcagcgagcagctcgcgggtgatcacgtcttgggtgccgtaggcggaataccccgccgccggcacgtgcccgccgccgccgagcgccttcgccacctgggacacgtcgatcacggacgaccgcagcgacacggcccagtagcgcggcgcttgctgcttgaacaccacgccgacgtcggaaccctcaagcgctcgcgcgtagtcgatcactgcctcaactgcagtctggctcatgcgcgccagcgactcggccggcaccgcaatcaccgcaaccgtgagtcccttctcgcggtagatctgcatgtccgcgagtaccgagcccataatcttcaaatcgatggcgctcatcgaatccatcagatcgagggcgatctggcgcgtgtccagatcgaactgcatgagctcagcggcgagcacgtgcatccgcgcggtgccccaccggaagttgcccgtgtcggtgaccagccccgcgtacaggcagtacgcgatatcccggtcaagctcggcacccatgtagcccaacaactcgcgcaccagcgtggtggtcgactccgagtcaatgatgaggttggtgccgccgaagccggggttcgtctcgtggtggtcgatcaccacgacacgggacgggtcggcggcaatcgcgtcctgcaccaagccggtgcggtcaagggaggcgcaatcaacggtgaccacgagcgcgtcgtcaggcaacgagcccccgtagttgattgctcccacacccggcacggtgtccaggttggacgcgtgcgggtaggtctggccaatatgcacgctggtgtcgatccccagccgcctcagcccgaacgccaagccgcaagctgaacccacggcgtcggcgtcgggtttgacgtgggccacgaccgccaccttcgcagcgccgagcagccgcgaacttacggcctcgaactgcgcggcgtgcgcgggaaacagtgagtccatttccgcgccctacctacttctccccgtcacccttgtacgggttggaactgccggcgggcgtggcgttggcgcgcagccgagcggtttcctcgtcgcgcgcgcgggcgcggctgagaagctcttccatgcttgccgacgccgccggcacctcgtcgtacacaaacttcaacgtcggcgtgaaccgcacgttgagctggtccccgacaatcttgcggatctggccgcgggcgcggttgagcgcttccgcagccgaatccaggtcgggctcgtcatcgatgttgcgcccgcgcacggtgtagaacaccgtcgcgtcgtgcaggtcgccggtgacgcggacgtcggtgacggtgaccagctcgagacgcgggtcttttacctcgtgctcaatcgcggtcgccacgatctgctggatctgcttggcaaggcgctgtgcgcgcgggttctcacccatgactcctccttgtgtgtcggtttcccacctggaaggtacccgtgcggcgtaaaactagccgcgcgggacctcgaccatctcgtacgcctggatgatgtcgtccacctggatatccgggtaggacagcaccatgccgcactcgtagcccttcgcaacctcggtgacgtcgtccttctcccggcgcagcgagtcgatcgtcgcgtcgggggtgacgacgttgccgtcgcgcaccaggcgcaccttcgcaccgcggcgcaccgcaccgtcggtgaccatgcagcctgcaatgaggccgacggcggaggccttgaagatctggcggatctccgcctggcccaggtcgcgctcctcgtagatcggcttgagcatgccgcggagcgcagcctcaacctcctcgatgacctggtagatcacggagtagtagcggatctccacaccctcgttgttcgcttcctccgtcgccttgccctcggcgcgcacgttgaacgcgacgatgacagcgtcggaagctgcggcgagcaggacgttggtctgggtgacagcaccgacaccgcggtcgatgatgttcacctccacctcgtcgtccacctcgatcttgagcagcgcctcctccagcgcctccacggaaccggcgttgtcgcccttgatgatgaggttgagctggctggtttccttgagcgcctggtccaggttctccagggagacgcgcttcttggtgcgggcctgcatcgcagcgcggtggcgggcatcgcgctgcgcggcaatctggcgcgccacgcggtcgtcgtccaccacgagcaggttgtcgcccgggccggggacgccgttgagaccttggacctgcaccgggcgggacgggcccgcctcttcgacgtcgttgccccactcgtcgaccatgcggcgcacgcggccgaagttgccgccgacgacgatggagtcgccgacgcgcaacgtgcctcgctgcacgatcacggtcgaaaccggaccgcggccgcggtcaaggtgggactcgatcgcaacaccctgcgcgtccatgtccgggttcgcggtgagctcaagcgctgcgtccgcggtcagcaggactgcctcaaggagatcgtcgatacccgtgccctgcttggccgagatgtcgatgaacatggtgtcgccgccgtactcttccggcacaaggccgtactcggtgagctggccgcggatcttgtccggctgcgcctcgggcttatccaccttgttcacggcaaccacgatcggcaggtccgccgccttggcgtgattgatcgcctcaacggtctgcggcatcacgccgtcgtccgcagcaaccaccaagatggccaagtcggtggacttggcgccgcgggcacgcatggcggtgaacgcctcgtggcccggggtatccaggaaggtgatcttgcgtggctcgtcctcgagggtcacctcagtctggtacgcgccgatgccctgggtgatgccgccggcctcgcccttgcccacgttcgcgcgccggatcgagtccagcaggcgggtcttaccgtggtcgacgtggcccatgacggaaaccaccggcgggcgctgttcaagcgcttcctcgccaccgatgtcctcaccgaactgcaggtcgaaggactcgagcagctcgcggtcctcgtcctccggcgagacaatctcaacctcgtagttgatctcggcgccgagcagctgcagcgtctcttcggagacagactgcgtcgccgtgaccatctcgcccaggttgaacagcgcctgaacaaggttcgatgcctcggtgccgatcttctcggcgagatccgtcagggtcgcaccttggcgcaggcgcacggtcttgccgccgccgtcgggaagacgaacgccgccgatgacgttcggtgcgtgcatctcctcgtactcagcgcgcttctgccccttggacttgcggcgcttgccgggtgcgccgcccggacgcccgaaagcgccggcggtgccgccgcggcgaccgccgcggcctccgcggaaaccgtcgcgcggggcgccacccgggccgccctggccgccgccgcggccgccgcggttaccgccctggccgccgcggccgcggttcgggcccgcagccttggacggcatctgggtcggcgacgggtgcgcagccatatcggccggcgacgggcgcgagccgcgctcgccgctcggacgcggggcaccttgcccctggccctgtcccgggccgcggccgcggccagcaccctgctgcgcgccaccacggccgccgcccggacgcggggcgggacggccgccgccgctgttggaggagaacgggttattcgctacgcgcgggcggccgcccggcttcggcatcggacgcggcatcgcattgcccgggtttgcggactggccggaccctgcgcccggcttcggggcagcaggcttgggcgctgccggcttcggagcacccggcttagccggcgcgggcttggcggcaggcttagccggcgcgggtttcgcggctgccggcttcggcgctgcgggcttggcagcacccggcttcggggctgcgggcttggcagccgcaggtttcggcgccgcaggcttcggagccgcaggcttggcggcaggcttggccgccggcttctccgccgcggcggcaggcttgggcgccgccggtttggcggctgcgggtttcgcggccgcaggcttcggggccgccggtttggccgccgccggcttctgcgcgtttgcgtttgcggtcttgtcggccgcgtctgccttctcaccgccggcttgcgcctcgtagtgggcgcgcatcttcttcaccaccggcggttcgatggtggacgaagcggtcttgacaaactcgccctgctccttgagcgtggcgaggagttccttacttgttacgccgagctgttttgccagttcgtgaacgcgtagctttccgggcacgtgtctccttggttgttggctaggagtgcgcgcccttcgtagttacacaaaaagcgacgtacccctagattggtcagtgactttcatcgctgatgctgcttcatggtcgcgtactcatcagtgttcggtcttcctatctgtatgtgggtctctatgtgggtcgctaacgtactcacgtacatgactcacgtccacaagggtggacaagcgaagcgccctggcgaacgcccggcgttgctccgctagctcaacagcttccggcgtcggtataatccacgcgccccgcccaggcagcctgcggcgggggtccgccagcacgcggccggggtgttccggatcctgcacaacccgcagaagctgggtgtcttccaccttctggcgagtggctatgcaggtccgcatacggatgggcatgcgcataccttcgctggtaacagtttgtaagccgtcgcctagaatacgccacgttacgccgaaacttctaacccgcggcccccgcggcggttaagcgtcgtcgccgtcggcgtcggaatggatgtcgatcttccagccggtgaggcgggcggcgaggcgggcgttctggccttccttgccaatggccagggacagctggtagtccggcaccacgacgcgggcgacctgcgcctgggcgtcggtgacctcgacactgatgaccttcgagggcgcgagcgcgttaccgacgtaagtcgccgggtcctccgagtggtcgatgatgtcgatcttctcgccgccgagctcttccatgatcgcggtgacgcgcgagccgcgcgggccgatgcaggcgcccttagcgttgacgcccttcaccgtcgggcgcacggccaccttggtgcggtgccccgcttcgcgggcgatcgcgatgatctcaacggtgccgtcggcgacctcgggcacctcgagggcgaacaaaccgcggacaagttcggggtgagtgcgcgacaggttgacggtgacgtcgcggtcaccgcggttgacgccgactacataagccttaatgcggtcgccgtggctcagttgctcgcccgggatcttctccgccggcagcaaaataccgtcctgcggctcgatctctgagccgatttccaccgcgttcaccccgcgggcttccttgtacgcgtcgcgctggaccacgccagagacgacctggccctctaagtcggcgtactccgagtagacgcggccaacctcggccgaacgcagctgcttcttaatggcgtcgcgcacggcgacagcgccgatgcgggagaagttcaccggggtgtcgtcgtattcggagagtacttctccctcagtgtcgtgctctgtcacgatgaccgagacgtcgccggttgcggtatcaatgtcgattcgcgccttcgacccgtcgtcgagcgggtgctcgcggaagtccttgtacgcccacaacagtgcggacgcaatcgtctccagcagagccggaaccggaatcccctggttcttctcgatggccttcaaggccgccatatcaatattcacttgtcacctcttcaaacgggagttccgccagctccatctcctctgccggcggattgttgaactcaatttctaccaccgcacccgccaattcagaaactgcgcgaggggcggcttccggctgtttggcaccggagctgacaagcgcaacctgcgtctcatcctcgcttagcgcgccgatgcggaacacctgctcgccgaccgccactaaacgcccgcggttgcggcgccagtgacgcggctgcgtcagcggcagatccacgcccggggtcgtcacttcaagggtgtagccggctccaaagttgaggtcgccggcgtcctcgcgtgcgtcgaaaagcgcggaaagctcctcgctgacctcctccagctcatcgagcgtggggcgggaatcgctgtcgagcgcgacgacaacctgggacttcgcccccgctttcgcggtgcgcacaccctccacgtccatgccgtaggcggcggcgaccggctcgatcaggcgcgtaagttcttcttcggaagggaaagccatgcgctaaagcctatcgtgtagcgtttgagcagtgaaaaagctgttcgccctgcccgcctgccttcttgtcgctagcacggtcgccgggtgtaccgtgatggacgtcgtcggcccgcgcccgaacgcggagatcgtggctctggcgcgacaggcggcggctgatgaggcggcgggtagcgaactgcggggggcgcagaagcaggcgcttgttaacgaggcgttgcgtctctgcggcaccacccctcaaggcgaaaccccgtcgtcgtgcagcgtggagctcggggaacttcccgcggccgcagacaccgggtcgttggtcgcaatgaccgctgaggcggcgaagcgggtaccggaggattccgtggacctcgtcgtcgcgcaggccatcgacgccgcggctgcgggaggcgtcgacctcgaggacgcccatccgggcgcgaacgaactcgacgccgcggaccccgccgacgccgcgtcgcagaaagacatcttagagcgggaatacgcgttccagtacggtctcggggtggccaaggcgttcggcgacgacgcgctggcggaccgcattgtggagctcgaccgggcttcgaaggagcgggtcgcggcactagttgaaagcgtcgacggggacacccctgagacggttgccgccccaggctacctcatcggcgacgccgagcagccgacggatgaggcctcggcggcagcgctggtggagcacctgcgccagaacctggtcgacgagtggcgccacaccgccgccgcggcgaacgacccggcgtggcgcgaggccgcgatctggctcgcagcccacgcgcagcgttcgtagctaacccgcgcgtagttagcccgccagcggcgcagtttccttgcgcaccagctcgacaacctggtcgacgatgcgctctgccggtacctcgagggtctcgccgccgcgaatgcgcagctccacgatgccgtcggcgaacgagcggccgaggatcaccacgaacggcatgccgagcagctcggcatctttgaacttgacgcccggggagactttggggcggtcgtcgaaaagcacctcgagccccgcggcatcgaattcagcaaccagccgctcgccggcctcgagcgccgcggcgtccttgttcgcgaccgcgacgtgcacctggtacggcgcgatggcgaccggccacacaaggcccttgtcgtcgtggcgctgctcggccacaaccgccatcatgcgggagataccgatgccgtaggagcccatggtgggcacggcgcgcttgccgttttcatcgagaatctgcacgtccatcgcttcggtgtacttgcggcccaactggaagatgtggcccagctcaataccgcgggcaagggccacggtgccattgccgcttggcgacgggtcgccttccttaatctccgcagcctcgatgaacccgtcgacggtgaagtcgcgcccggccacgaggccgacgacgtggcgctgcggcgcgtccgcgcccgtgatccagctggagccgtcgaccacgcgcggatccgccagcaaccgcaccccgttggccgcgagcgcgcgcgggccaacgtaacccttgaccaggaacgggttgtttttgaagtcctcgtcgcttgcgagctcaaacgtcgcgggctcaaggctcgcctcgaggcgtttttcgtccagttcgcggtcgcccgggatcaggatgccggtaagttgcgggccgaccgggttgccgtcctcgtcggtggcgcgcgggtcgttgaccttgaccatcatgcacttgagggtgtcggaggcttggaccgcgcgaccgtcgacaagcagctgctcccggttcgcccactcgaccagcgccgcgatggtttcggacgcaggcgtgtcgtactcggtggcctccggcaggcccgcgatgtcgcgcgcgggcggggcgaccgtggtcacggcctcgacgttggcggcgaaatcacccgcggtcgagacgacgaacgtgtcctcgccgttgtcggagtacgccaaaaactcctcggaggcagagccgcccatcgcgccggaggtggccttgcagatttcgtagcgcagaccaacgcggtcgaagatgcgctggtaggtggcgcggtgcttggcgtaggactcagccagcccctcatcggtcatgtcgaaggagtagctgtccttcatcacgaactcgcggccgcgcagaatgcccgcacgcgggcgcgcctcgtcgcggtacttcgtctggatttggtacagcgtgacgggaaaatccttgtagctggagtaaaggtctttgacctgggcggtgaacatctcctcgtgcgtggggccgagcagcatgtccgcgcccttgcggtccttcaggcggaacaggtcgtcgccgtactcggtccagcggttcgtcgcttcgtacggctcgcgcggcaaaagcgctgggaagagcaactcctgcgcgcccatcgcgtccatctcttcgcgcacgatgccctcgatcttgcgcagcgtgcgaaggccaagcggcagccaggagtacacgccgggagccgcgcggcgcacgtagcctgcgcgcacaagcagtttgtggctgggcacttccgcgtcggcgggatcttcgcgcagggtgcgcaggaacagggaggacaggcgtgtgatcatgtcaggaaattctagcgctagggtttttggcatgctcatcgtgctgccaccgtctgaaaccaaggctcccggcggtgccggtggcccgatcaccgtctcctttccccagctcgacccggtgcgcgagacgcttatggggcagctcgccgcaagcgacgtcgacactctcatgaccgagctgaagatccccgccggcaagcgagcggaggcggaggagaacctgacgttgcagtcagcgcctgtcatgcccgcgatcgagcgctacaccggcgtgctgtacgacgccctcgatgcgccgtcgcttccagccgctgcgcgccagcggttggcggtcggctcggcgctcttcgggcttgtgcttgctaacgaccacgtgccccgctaccgcctctccgccggttccaagctcggcggacggacaatgcgtgcgtggtggggcccgcgcgttaccgaagtactgcaggcggaggatttcgtcgttgacctgcgttcgggcgcttaccagcaacttggcccagtacccagcgcggtgaccgtgcgcgtagagcaggccgacacaggcaaggtggtcagccacttcaacaaacgctacaagggggaactggcgcggaccctggcatttgccactaccccaccgagttcagtcgacgatgttgcggatgcggcccgggcaggcagtttgaacgtgctggtggacggaaacgaggtgacgcttaaggtgtgagaacggtgcagtacattcgatgaccatgccgttgcgccgcgctcttccaatctccggaatcatttacctcgccgttctcgcgttcgttgccgccaggtgggacgcaattccggacccggtgccgatgcacatcggccccggcggtgaagtggatcgatggtcggagaagaacttcctcagcgccaccgcggtgacgtggatcggcgtcgtgatttccgcggcgatggcgctgtgcgcgccgaagcagagcctggccgcggcgcggcgcgagccctccgacgaaggcaccctacccaacgacgcgctgccctactcggagtcggcgtcgcagcgcgcgcagcatctcatcgataccaccaatacattcttgggaacgctgcttatcgccaccagcatcgtcttggcgctgacccaggtcatgatgctgtttcccgagatcgtctcgcccaccctgtggtgggtctttttcgggttgtacatggtgggggttgtggtggcgtcgataagccttgcccgaacatcccgccggaacttcgacgacataccggcagacgcagatgagctgcaacgcgtggacgcgctcaagcgggtggcgtcgatgggcttgtatagtcagccgcgcgaccccatggcggtggcagtgctgcccggtgagcccggcaagctgcagatcaactcggcgcacccggcgggcaagcagcagctgcgccggatgggcatcggcatcggcgtttcgatcgtcctcgttgtgctgctggcggtgatcgcgtgacggcgccccgcacgcaacgccgcggcgcgctcaaactggcagcggccatcctcatcgcactcatcggcatcgcggcgatcgcgttcaccgtcaagacgtggcaggagcgcaccggagacacggtggtggtgagccggattgtggacggcgacacgatcgatatcgagcgctcgggcgagacggttcgcgtgcgcttgctcaacatcgacaccccggagaaagaggagtgcctgttcaacgaggcgaccgagcacctcacgatgctcatcgcccccggcgaccgcgtctcactggttcacgacgtggagcgccaggaccgctacggccgcgaactggccggggtggttacagccgacggcacctttgtcaacgaggtgatggtggccgacggtttcgcgcgcgccgtggaatatcagccgaacacccgctttacccggcagatgcgcgacgcggaggcccaagccaaggccgctcgcaccggcatccacgccgtgcccaccgagtgccttatgcccaccgagatcgcccgcgacgcgcttgcgcgctaccagggtgacccggacccgttttacctcgacgtgatgcgcgacgcggtggacaacacgaacaacttcacctaccgggaccaggcgattgcgctgatcgacagcctctaagccgatagcctttaaggccatgagcgacttgaacgaggcacgggccatcctggataacgcccgacatatcgaggtcttcaccggcgcgggtatgagcgcggacagcgggatcgcgacctaccgcgacgctcagaccggcctgtgggagaacgtggacccgcaggcaatggcgtcgatagacgcgtggcgcatcgacccggagaccatgttcgcctggtacctctggcgcgcacacctcgcgcagcaggccgagcccaacgccggccacttcgccatcgcccgctgcccgaaaacctcagtgaccacgcagaacatcgacaacctccacgagcgcgccggcagccacaacgtcgtccacctgcacgggtcgctgttcgagttccgctgctccgagtgcggccgcccctacaccgccccgatcgagctgcccgaagggccggtcgaggcaattaccccgcccgcatgtcccgagtgcggcggtgcggtgcgccccggagtggtgtggttcggcgaggcgctacccgacgacgcgtgggcggaggccgagcggcgcatgaaaaccgcggacgcgctgttgatcgtcggcacctcgggggtggtctaccccgccgcgggcctgccgctcatcgcccacgcgaacggggtgccgatcgtcgaggtcacgccaatgcgcaccgacctgtcccacctggctgacgtggtggtcgaggacaccgcggcgcgcgccgtgccgcagcttattcctacttcgtcgcccgcagcacagtaaacgtcgcgtcgcgggcgacctgctccaccgtggtgaatctgcgctccacctcgccgcggtagcgcaggtgcgagttgtgcaccaggtacagctgcccgccgggtttgagcattcttatcgacgcccccagcaactccctcaccaacgtcgcatccaccgccgtgccgtcgtggaagggcggattgagcgcaaccgtgtcgaaggactcgccggggaacttcgaccccgcgtcgtcccacgtcgcgttcagcccgttggcgcgcgctgaaagcactgcgtcggcgtcggagtccgtggcgaaagcgttcatgccccgcgtcaccgagccgttgccgcagcctaagtccagcaagcggccgggatccgcgggcaggcacgatcgcagcagctcgccgccgcggtccggcttcgcacctgagaacacaccgccgatcgcggtgagaccgttgactgtcaccggctcgtacgcgaccggcttggggccttcggcggcaaggcagcggaacttgcctcggccgcgcgaggccgcgacgcggtcgaacgactcagccagcacgtcgttcatgccccgcgagaggtgcttgttgttgccgccgaaaacaacacgaagcggcgcaaaaccgctggaagcgagcgagcgcgccacgtagtccaagcgaccgagcgccttcggcatttctcccaccgccacggccggcccctccgagccggcgaggaaaacgtccagccgcacgtcgccggcggtcgccgcgccgagcgacgccgccgactggctgcgcgcgtagtcggggtcgagaaacaccaccgggttgcccgcgcccagcgcggcccgcgtgaggtcgagggtggggtcgtggcagatcagcacggtctcgcccggcgcgatctgcgcggtgtcgaggatcaggctatccagcgtgcgcaaggccggccacctccccgaagacgtagacggcgggcgcggacacgccctcggcctccatgacgtcggcgagcgtttcggcggtggcgaagaagacccgctggttggatgtctcgccgtcttggataacggcggcgggggtggtggggttcaggccggcgtcgataagcgactgccctatggcgcgcacgttgcgcacccccatcaccaccacgatggtcccgccgagcgtggcaagcgaagcccaatccaccagcgacttgtcgtgcccgggcggcaagtggccggaaaccaccgtgaacgcgtgggtgaccccgcgctgcgtgaccgggacctgcgccgccgccggcacggaaatcgccgaggtcaccccgggcaccacgtcgcatgcaatccccgccgccgcggccgcctgcagctcctcgaacccccggccgaaaacgaacgggtcgccgcccttcagccgcgccacgtgcttgccctcgcgtgcgtaggagaccaacagttcgttgatgcgctcctgcgccacctgcttcgcgtacggcagcttggccacatccacgacctccttgccgtcgatgtcgataaactccgcaagctccgcggcgggccctaagtggtcgacgaggatgacgtcggctgcctcaagcgcgcgcagacctcggatggtgagaaggtcccacgcgccggggccgccaccgacaagcgtgatgtggcctgtactccctgtactcatggcagaacagtttagggtgagaccatgcaaccaccacagctcgcccacacgctcgctgaccgcttacccgaattggcgcacgcgcagccgcccacgcgctttgaaaacccgaagctcgtggtgctgaacgagccgctggcggccgagctcggcctcgacgcaggttggttgcgcacggacgagggggtgcgctggctggctggttcctccggcggccacgccatggcgtatgcgggccaccagtttggacagttcgtgccgctgcttggcgacggccgcgccctccttctcggctcccttccccacgcagacggcacgccccgcgagatccagctgaagggctcgggtccgacgacgttctcgcgcccgggttctgacggtgtcggggccatcggccccatgcttcgcgagtacttggtctccgaattcatgcacgcggtgggcattcccaccacgcgatcgctggcggtagtcgacaccggcgaacacgtcgtccgtcagcagggccgcgtacccgggggcatcgtcgtgcgtgtggccgcgttgcacctgcgcgtcggcagcgtgcagtacgccgcaacgcagtccgccgagctagtggaccaggtcgtgcgcgccgccggcttcgactcccccgccgcgatgctggacggtgtcctggacgcgcagctttcgctcgttgcatcctggatgcgcatcgggttcgtccacggggtgatgaacacggacaacaccgcgctatccggcgaaaccattgactacggaccgtgcgcgttcacggagacgtatgacccgaacgcggtgttctcctccatcgacgcgcaaggccgctaccgcttcggctaccaaccttccatcgcggtatggaacatcgcgcggcttgccgaagcgttgcttcccgtcatggaccaagacgcggcccaggctgtgctggcggacgcgcaggagcgttgggaccgggcatggaatgccgccgtgccagacccggctgcgctggcggcggcgggagacctgttcacccacgccggcatcgtcttcggcccccgcaacggcatgcttgagcgggccattgtggaagcggaacagaacggcaactacgcgccgtacttcgagcttctttccgcgaccagcgacccgttcaaccccgacgccggcccggaatggatgaaggcgcccgaaggcgccttcacgttccaaacattctgcgggacctaagaccccgccgcgcaggactcggctacttggccgtgccctgcccgtccaagtggcgctccacatccaggcccagagtcttctgggtccacgcccactgctcctcgtacgccgcgcggtcgcgcttcagcgacttgccgtaagtcgggaacatctcgtggagcttgtcgccccagtcgatcatgcgctcaccgaagcagcgctcgagcagctcgagcatcgcggccggggtgatcgacgcacccggggacgcgcccaggatgccggcgatggtgccgttctggtcgttgaccagtgcggtaccgaattccagcgagccgaagcggggggcagcggtcggcttgatcacctgcacgcgctggccggcgacaacctcttgccagtccttcgggtcggcctccgggtagtactcgcgcagcacttccatcttgccgtcgaagttgcggaagacctcctccaccaagtacgtgaccaggttgaagttagtggccgcaacgcccaggtacgacgggatgttgtccgggcgaatcgacttaaacaggtcgaggtaggaacccttcttcataaacttcggggtccagccgccgtacgggccgaacagcagcgactgctcgccgtcgaccacgcgcaggtcaaggtgcggcacggacatcggcggggcgccgaccttcgccttgccgtacaccttcgcctggtgctgggccacgagctcctggttggtcgtgcgcagccacataccggagatcgggaagcccgcgtagccgcggacctccggaacacccgctttgcgcagcaggtcgagcgcgtagccgccggcgccgacgaagacgaagcgtgcgcgggtgaccttgcggtcgccgttgcgcaggtttttcacgctgaccttccagaagttgccctcgcgcttaatgttggtcacttcgtggccgtagcggatgacggtgccgttttccttcgcggagtccaagaactgcttggtcagcgcaccgtagttgatgtcggtacccgcgtccgtccaggaaatcgcaaccggctcggcgtcgaagtcacggccctgagccatcagcggcagcatgcgggcaaactggtcgcggtcctcggtgtactgcatctgcgggaacatgtggttcgcgctcagcgcgtcgtagcggcgcttcaggtacccgatctggtcttcgccctggccaaacgagacgtgcggcaccggattaatgaaggcgctcgggtcggtgagcacgccgttttccacgcggttcgaccagaactgacgagagagctggaacttctcgttgatgttcatggccttggagacgtcgatgcggccgttcttctccggcgtgtagttcagctcgcacagcgcggagtggccggtgccggcgttgttaaacgggtaagaggactcctgggctgcgccgtcgagacgctcgtagatcacctgagtccatcccggctccagcgcctggagcatcgccccaagggtcgcactcataatgccggcgccaacgaggagaacgtctacctcgtcgtcatagtggtctttcttctcagccattgcatgtcacctgtttcatttcagatcgtgttctggtgctgtcaagggtaatggtttttcactctacgcttatataacttggctccggctaatatcggtcgcatgagtgcgccgatagacccgacgtttcaaccagacatcctcggtgacggcttcgagcaggcggttttgcccatgggcaaggatccggacaccggcacagacgtccgcgccgtcctcgtccgcgcgagcgtcggcaacaaacacgccgacaagaacaagccggccctgctgtgggtgcacggcatgtcggactactttttccaagaccacgtcgccgactacttcacagatctgggctacccgttctacgcgctcgacctgcgccgctgcggacgggcgcgcacgaccggccagcgctggcactacaccctcgatgtggctaactactacccggagctgactgccgcactcgatatcatcacccgcgaccaccccggcgtgatccccatggcccactccaccggaggcctcatcgtgccgctgtgggtggatgagctgcgccgcgaggatccgaagcgccacgcgcagattaaaggcatggttctgaacagcccgtggctggacctccagttcaacccagtagcggtcgcagtgacccggccagtcatcaacacgctcggccgcgttgccccgaaactacccctgccgcagggcggtctcggcgcctacggcgcttcgatctaccaaggtgagcacggcgagtgggacttcaacacttccatgaagccgctcgacggccaccgcaagtacctcggctggatccgcgctattaataaggcgcagcagaagatccactccggcgaaatagacgcgggtgttcccacgttgaccctcgtgtctgcgcactcgtacctcggcgaggactactcccccgccgctgacaccgccgacacggtgctcgatgtggatcagatccgcaaatgggctcctgaaacctcatcccagaacgaaacaaagattatcgatggcgcccgccacgacgtgttcctgtccgaaccgttcgcgcgcgaagtcgctttcaagaccaccgccgagtggctggagaagatttaaacgacatggacaccacgcactacgacctcatcatcatcggcaccggctccggcaacacgatcatcaccgaggactacgacgacaaacgcgtcgccatcgttgagaacggcaaattcggcggcacctgcctaaacgttggctgcatccctacgaagatgtacgtgctcgccgcggatacggcctaccaagcgcgcgaatccgagcgcctcggcatcgacctcgagttcaaaggcgccgactggcctgccatccgcgaccgcgttttcaccaaccgcatcgacctcatcgcagcgggcggcgaggagtaccgccgctccgacgcgtgccccaacgtggacgtctacgatcagcctgcgcgcttcgttggcccccgcacgatcgagaccggcaccaaagaaggccccgccacgattacggcggaccaggtactgctcgccgccggctcgcgcccgttcatccccgattgggcagaaggactggattaccacaccaacgaggacatcatgcgcctcgagaagctgcccacatccctcacaatcgtcggcggcggcttcatcgccatggagttcgcccacgtcttcgaggcgctcggcaccgacgtgaccatcgtcagccgctccgcgctcctgcgcacgctcgacgaaacgattcgcgacgaattcaacaccctcgccgaaaagcgcttcaacgtcgtgcactccacggttgaatccgcccaccagaccgaggacagcattgagctgctgcttgccgacggcaccaccgtctcctcccagcaccttctccttgccaccggccgcgtccccaacggcgacgaactcgaagtgcagaacgggggcatcgaaatgcttccgaaccacagcgtgaaggtcgacgagttcgggcgcaccaccgccgagggcgtgtgggcgctcggcgacatctcctcgccctaccagctcaagcacgtggccaacgccgaagcccgcgccgtcggcgccaacctgctggccgccttcgccggcgaagagcccaccatgaccatgccgcacgagcacgtgccatacgccgtgttcacccacccgcagatcgccaccgtcggcctcaccgaggagcaggccgtcgcagccggccacgacgtcaccacgaagatccagcgctacggcgacgtcgcgtacggctgggcgctcgaggacaccaccggcgtggtgaagctcgtcgccgacaagcagtcgggccgcctcctcggcgcccattacatgggtccgcaggcctccacgctgattcagcaggcgatcacaatcatggcgttcgatttggacctccgcgacgttccccgcaagcagtactggatccaccccgcgcttgctgaggtcaccgagaacgccatcctaggactcgatctggacttcgccctcgcctaacccctacccccacatgagggggccatgcggggcccctccgtcagcaggcatcgcctttgcccacgcccacgttacttttccaaggtttagatacttcactggacgttacctgtgaaaaatattgtgtggtggttgcacgttgctctaaggacattgctacagtagtgcacgacactcggtcagatggagccggtactccagatcgagagcctccgggccaaggtcgccagatcaagttcggatgacttgtaaaaactagaagtaaggatttcgtttcatgcgtaacttccgcaaggcagccttcgcaggcgccaccgccgttgccgtggcattcggctccaccgcagtcgccgctgcagacaccaccgagaacacccaggagttctcccacactcgcgttcagaacgttccggcggacgcagagtctgacttccgtaccaacgttggccacaaggtcgaggcttggtacaaggacgaggagggcaacgtcatcgccaccggcgtcaacaaggacgagttctacggcgagtggactgacgagacccccgcttggtccaagatcctcttcgttggcggtatcgctgcgatggtcagcgcggttatcggcctgatcgttggcccggcttacaacttcttcgtccacggcccggcagctttctaagcctcgctcatccacaaactaagatttcttgaaagaaggaaaatatgcgtaacttccgcaacgcaaccctggccgtggcgaccgctaccgctgtgaccttcggtggcgcagctgctgcaggtgcacaggaggcagggaacaccgaccagtcgtccgtcgagcagaccaactcctcccagcagaacggctcttcccagtcggctgatgacaataaggattacttcatcgtcgactctcacggtaagaccaaggacgaggacgaggttccggcttgggcgaaatcctggaacaccgcctccatcgtggcctccatcggcgctgttattggcctgatcatcgctggcttcaacttcgcttcctacaacggctggatcaacttctaagatcgccgttcgctaactgcgaagctattgcgaaagctcccgcccttcggggtcgggagctttttcgtgccggcgggagcctgcgctcccggggcggctacgcgcccagcatgtgctgcccagctgcgaggtcggcatctgggatcgtgaggatctcgttgccgtcgtcagtgatcaggatggtgtgctcgaactgggcggtgtactcgccgtcgcggttctgtaccgtccagccgtcgtcccagatgtcgtacgggagggcgccgaggttgatcatcggctcgacggtcagcgtcatcccgggctcgagaatgtcggtgtaggcgtcggagtcatagtgcagcaccacgaggccgttgtggaacgtggtgcccacaccgtggccggtgaagtcggtgaccacgttgtagccgaagcgcttggcgtaggactcgatgacgcggccgatgacgttgatctgtcggccgggcttggcggccctgatgccgcgcatggtggcttcgtaggtgcggtccaccagcaaccggtgctcctccgccacctcgcccgcgaagaacgtggcgttggtgtcgccgtggacgccgttcttatacgcggtgacgtcgatgttggcgatgtcgccttcctgaatcaccgtggtgtcggggataccgtggcagacgatctcgttgagcgagatgcacgaggacttggtgtagccgcggtagcccagggtcgacgggtaggcgccgtggtccaagaggtactcgtggatcacgccgtcgacgtagtcggtggtcacgcccggtttgatctctgcgccgccgacggcgagcgcgttcgcggcgatcttggatgcctcgcgcattgcctcgatggtctcgagggtctgcacgtgcggctcgccgacgttttcctggacgtcgtccttccaggcgtactcggggcgctcgatcgacgcgggcactttcctaatcggggtgggttttcctggggtcaactttccgcgtggattcatgcggtcaatgttaaccccgggcggcgtccaggttcgaaagcatcgagctcgtcagcgccacggcggcttcggatccgccgcctaagacgacgagggtggcaaaggcgatgtcgtcgtcggcgcggtagccggtgaaccaggcgtgggatccgcctgtgatctcggcttctccggttttgccgtagacgtcgccaaacgaaccaagccctcctgcggtaccccctggcatcaccaccgccttcatcaaccgccgcaactcgtcgattgactccggcgacggtgggtcgacctgctcccccaccttcgtctcctcgccggcaactaagaacggcaccggcatcgagccgtgcgctgccgtagcggataccagcgccatgccgaacgggctggccaggtcgtacccctgtccgtagccggcctcggtgcgctccagcggggtgtccccgactggaatgtcgccggtgaccgtgtcgatacccgggatggaaaagtcgaccccgaggccgaactgcttgccgacgtccctcagctcccccggagccaacttcgtcgagatgtccgcaaacgtggtgttgcaggacctcgcgaacgctgtctgcaaaggaacgctgccgaggccgaagccggcgtagttggtcacgatgcggccgtagatgttcatggtgccggggcacggcaccgtcgaatccggggtgagcccctggcgctggaggcctgcggccgaagtgatgatcttgaacgtcgaccccggcgggtactgacccatggtggccaagttgcccttgcggtcggcggcgggggtttgcgccacggcgaggatgccgccggtggaggggcggatcgccacgatcatcgcctcttggccggcgacgggctcgagcgcttgttcggcggcgcgctgcaccgcgtggtcgaggctcacgctcactgccggcgacgggtcaggctcgacgcgctcgacctgctcgaactcggcgccgttctcgttgaccacggacacgctccagccgggctcgccgtccaagtcgtcgccgacgagcgcgccgatgcgcgccatgatgtcgggggcgaaggtggggtcttggttcaccatcgcggcttcctcgttgaggcgcacgcccggggcgttgccgagagctgcctcgaaggcgtctttcgacgtggcggggatgacggtgacggagtaggtggattcggcggaggcgagggctggggtgagggaggcggcgtcgataagcgcaatgctcctgtccccctcgtgcgcagccgcgagtgcctccgcgatgcgctgagcggtctcgggggcagaacgcattgcggacgggtcgaccagcacgcggtatgcgacgcccgggcgaagcagctccaccccgtcggaggacacgacgctggcctggtgcgccgggattgcccggagttcgaggtgctggttggcgccgaggcgcggatgcaggatggacggctgccagcgaacggtccactcgtcggcgacctgggtgagcgtcatgttcgcgtcgtaggtgtaggtacgctcgcgcgggagctgccacgacatttcgtaagtcgccgtggcgatgttgtcggtttgcgagacgtccttcagctgcgttgtcagcccctcggcctgcagcccctcccacgtcgttgtggtggagcgctgggcctctgccggattgtcgacgcccgcggtgaaatcctcgcgcgcctcaagcgctttgagaaacgcttccgcgaccggctccgcggagttcggccgcggggtgcagcccgccgcgctcacagtgagaacgatgctggcgagcagggcgaaaaggcggcgcatggcaaaaacgtagcagcaccggccgtgtgatcggtgctgctcaggaggtgttgcggaacgtctagcgcgtaaccttgacctcggccttggcgccagcgacctcctcgaggccctcctcctcggcgatgcgcagcgcgtgcgcgatgagcgtctccacaatcttggcctcaggaacggtctccacgacttcgcccttgacaaagatctggcccttgccgttgccggacgccacacccagatcggcgtcgcgcgcctcgcccgggccgttgacaacgcagcccatcactgcaacgcgcagcgggaactccataccgtcgaggccggcggtaacctcttcggccagcttgtacacgtccacctgcgcgcggccgcacgacgggcacgagacgatctccagcttgcgcgggcgcaggttcagcgactgcaggatctggtcgcccaccttgatctcctccaccgggtcggcggaaagggagacgcggatggtgtccccgataccgtcggcaagcagggccccgaatgccaccgaggacttaatggtgcccatgaacttcgggccagcctcggtcacgccgaggtgaagcgggtaatcggtcttctccgcgagctggcggtaggcctccaccatcagcaccgggtcggagtgcttgaccgaaatggcgatatcgccgtagccgtgctcctcgaacaggccggcctcatagatcgcggactccaccagcgcctcaggggtggccttgccgtacttctccaacaagcgtttatccagagaaccgccgttgacgccgatacggatcgggatgccggcgtcgcccgccgccttcgctacttccttgacgcggccgtcgaactccttgatgttgcccgggttcacgcgcaccgcggcgcaaccggcgtcgatcgcggcgaagatgtacttcggctggaagtggatatccgcgatcaccgggatcggggacttcgcggcgatcgcgggcagcgcttcagcgtcaaccgtcttcgggcaagcgacgcgcacgatgtcgcagccagcggtggccagctgcgcgatctgctgcagggtggcgttgatgtcgtgggtcttggtggtggtcatcgactgcaccgtgatcgggtggtccgaccccacacccacgccgccgaccatcagctggcgggtcttgcgccgcggcgccaaggtgggcggcgggccttcggggatacctaatccgatggggagactcatgcgcactagattagcaccgcggcgcacgggcgcgacgcggcggattgggcggggtttagaagatgcggaccgggttgatcacgtccgcaaccatgacaaacacaccgatgatgagcagcgtcgcggccatgaagtaggtcagcggcatcagcttttcgtagttcaccggctcccccgggccgagcccgcgggcacggcggaaaaggtcgcggatcttctcgtagatgatgacggcgatgtgcccgccgtccagcggcggcagcggcacaaggttaaacagcgccaggaagaagttcaggctggccagcatcatgaagaacacgggccacatgctgcgctcagccaactcgccgccggtgcgcgaggcgccgatgatgctgaccggcccctcgacgtcgcgctccgcgccgaagacggaggcgatcacgcccgggattttgcccgggaatgccgccagcccatcgaccgtggcgccgagcatctcgccgctgaagcgggcggtggccgggacggcctcgagcgggctgaactgcttcaccgcgtccttgattggtgccgcccccatgccgatcgctccggcgtcgaactcctcgccggtctgcgggttaatgcgtttgacgttttcaaccgccacgtcaaacgagattgcttcgccgccgcggtcgacctcgatggcgacgttctcgcccgggcgggtgatgacgtagtcgcgcagctgcacgaacgactcgatcggggtgccgtccaccgcgagcagctcgtctcccccgcgcagtcccgcagcgtaggccgggccagagccggtgcacgcagcaagggtttccgcatccacttggtctgaggtgcacgtcagctcgcccacccgaagcgtgcggtcggcgtacgggttcgggatacccgaggacacggcaacaaggtaaatgatcacgatgccgatcagcaggttcatcacgatgccgccgaccatcacgcagatgcgctgccacgccggcttgttcaccatcgcgtgcggcgcctcctcctcggtgacggggtccatcgcggtcatgccggcgatgtcgcagaacccgccgaacggcagcgcagcgatgccgtactcggtgtgtccgcgcttggtcgaccacaccgtgggaccgaacccgatgaagtagcggcgcacccgcatgccgaaggcgcgggcggtgaacatgtgacctgcttcgtgcagggcgatcgacgccgcgatgccgagggcgaagatgaaaacgccgagaaaacccatgcgctacttccccgccagagccgcaacggcagcttcggcgtgctcgcgggccgcctggtccacgcggacaacgtcatcgaaggtagccggcacggttgcgaacgcgtcggcgcgctcgagcacctcagcaatgacgtcgacgatctgggggaaggcgattgccccggcgaagaacgcgtcgaccgcgacctcgttcgctgcgttgtagatcgccgggtagggatcgccccgcttcaccgcgccgcgcgcgagctcgaccgcgggaaacgcatccgcgtccagcggctcgaaagtccaggagtgggcgtgggtgaagtctaaggctggctgcgcgtcagcgacgcggcccggccacgcgagcgcgtgcgcaatcggcatcttcatcgacggcggcgacgcctgggcgatcgacgcgccgtccacaaacgtcaccatagagtggatgacggactgggggtggacggtgacgtcgataatctccgggtcgatgccgaagagcagcaccgcctcgatcagctccaagcccttgttcaccatcgtggccgagttgatcgtgttcatggttcccatcgaccacgtggggtgcttgaccgcctgctgcggggtgacgtccatcatctgctcgcgagtccagccgcggaacggcccgccggaggcggtgagcacaaagcgcgacacctcttcggcgcggcccgcgcgcaggcactgcgccatggcggagtgctccgaatcgacgggcactaactggcccggcgccgcggtgtcgaggacgagtcggccgcccgcgacgagcgactccttgttcgcgagcgccaggatcgcgccggtctcgagcgcggccagcgtcgagcgcagcccggcagcgccgacgagagcgttgagaacgacgtccgccggctgcgcctcgatcagcaaagcggccgcctcgtcgcccgtgagcaccttaccgccgagcgcctcggacacctctgctgccgcgtcctcgcgctgcaccgcgacctgcgaaggagccaaaccgaactcgcgggcttggttgattacagcggccgggttgctgcccgccgcggcgatgcccgcgacctcgaattcgtgtctgttcgcagcgatgacttccagcgcctgcgtgccgatggagccggtggacccgagaatgagaatgcgcttcacgcccgccattgttccagccgcggtcgaactttcggaggtttagggggtattaggtcgcagatgcggggatagctgtgcgacaatggagcgagattttgaactcgagtttgtcaacaaaggagtttggctgtggcccaccacgctcaagagaaggcaccgcaggtgtacaacggcgtttccgaggcagatgtgccctcagcccgtttcggctggagcgaggtcggccgcggcgccgtgcagaccgccggctggatctcggtgctggttctgctcgcctacaacttcggcaaccaccagggccacgtcgagacgatctggctgatcgcgctcgcggtcctcatcgctctcggcttgatccttcacgccacttccccgaagctcaaccaggtgcgcaccgtcaccgcccacaacaagccggtcggccaccaggagccggactgggcgtacgaccagaagacgctctccggcgtttacgagaacctggacgagcgccagctgcgcgcactgaatatcgacccggctcgcgtggcgcacctgcgcgccccgcagcgcgaagtcaccacccacaccacgaccacggtgcgcgaggccgagccggccgaggtagtccgcgtcaagccgactgagacccgcacccactaagcgtcgcacttcctggcgcaagactaaagcccggtccccgctgtggggccgggctttgtggtgcttgggatggggagaaaaaagggggcgtcgataagcctgatgcccctaacccgccttctcctccgcagccagctggccgcaggcggctgcgatctcctgtcccttcgtgtcgcgcaccgtacaggtgaccccctgagcaatgacgcggcggacgaactcgtcctggcgcgccctcggcgaggcgtcccacttcgaacccggagttgggttcagcggaatgaggttcacgtgcaccttggaaccgagggcgcggtgcagcttctgacccagcatgtccgcgcggaaatcctggtcgttgatgtcgcggatcagcgcgtactcgatggagacgcgccggcccgacttgtccgcgtagtagcgtgcggcgtcgagcacctcggcgacctcgtaacggttgttcatcggcaccagctcgtcgcgcagctcgtcgtccggcgtgtgcagggaaaccgcgagcgtgcaggagaggtcctcgtccgcgagtttgcggatctgcggggcgagaccgacggtggagactgtgacgttgcgttgcgagatgccgaagccgtcgggcgacggctgcgtgatctggcggaccgccgagaccacgcggttgtagttcgccagcggctcgcccatacccatgaacacaatattggacaggcgcgatccttccgcagccatcatcgcggcggcttcgcggacctggtcgacgatctccgccgtggacaggttgcggtccagcccgccctggccggtcgcgcagaacgggcaggccatgccgcagccagcctgggaggagatgcacaaggtggcgcggtcggggtagcgcatcaggacggactccaaaagaatgccgtcgtgcaggcgccacagcgtcttcgtggtgtcgccgttgtcggtctccacctgccgcaccggggtgagcaaagtgggaaacagcgcgtccttcaccgtctgccgttgcgcctccggcaggtcggtcatggtcagcgggtcggcctcgaacttgccgtagtagtggcgcgcgatttggtcggcgcggaacttcggcaagccgagctcggcgatggcttctttgcgctcgtccttcgtcaggtcggcgaagtgcttcggcggcatgccgcggcgcggcgccagaagctggatctgagggacgtcgcccttctggctcgtctcgcgttgttcagtcggctcagtcataatgccgcgtattgttgcacgtcacgcgctcgggcggcgaattgcagcttacagcgggttcatcagcgcggccgcgttgagcagcacgtaggtcgcacacgctgccggcagcatgccgtcgaggcggtccatcaggccgccgtggcccggcagcaagttcgacatgtccttgatccccagctctcgtttgaactggctttcaacaagatcgcccatggtcgcgcagacgaccagcgccgcccctaagacgatgcccatccaccacggtccgttgatcaggaagtggacggcgactacgccggtgacaacgccgaagatcatcgagccggcgaaaccttcccagctcttgttcgggcttaccgccggagccatcgggtgcgagccgaacatgaccccggccgcgtaccctccgacgtcggaggccacaacacagagcatgaacgcgatgatgaagtgggatccggggatgccgccttcgtcaataagcgaaatcagcgccgcgaacgacccgaacagcggaatccaggtcaggacgaagatgccgactgccgtgtcgcgcaagtagtgcaccggttttgcgtcccggccgttgtggaacaggcgccagaacatgaggaacagcaccgtgatcgcgaacgcggcgaccaggcctgcggtgctgtagagcgcggaggaccagatcatgatctgccccagcacgataagcagcgtgcgcggctgctggtagccggcttcgcgcaggcgcgtgagcacctcccacatggcgagcgccaccgcggtggcgacgagcgggtaccacgctttcggcccaacccacaccgcagcgatgacgagcgcgccgagaatcacgcctgtggtgatcgcggcgcccaaatcgcggcccgggttgtttttcggcttcggggcacgcaagtgcaccgaggggcggcgctgctcctcggctgtttctgcgcgctctgctcggctctcggtcatggggtcctagacctccatcaactccgcttccttcttggccaccaactcatcgatctgagccacgtagctctgggtggtcttgtccagcgccttctccgccgtctggacctcgtcctcgcccgcgtcgccatccttctggatcttcttcagcgcgtccatgccctggcggcgcacgttgcggatagccaccttgccgtcctcgcccttctgctttgcctgcttgaccaggtctttgcggcgctcctcggtcagctgcggcacggtcacgcggatcacgtggccgtcatcggtcgggttcacgccgaggtcagagttgcggattgcctcttcgatgtcgcgcatggtcgaggggtcgaacggcttgatcagcagcatgcgcggctccggcaccgaaatggtcgccatctggttaaccggcgtcggggcaccgtaaaagtccgccatcacgccgttgaacatggccgggttggcgcggccggtgcggatggaaaccagctcgccgcgggtgtgctccacggacgaggccatcttttcctcggagttcatcagcacgtcatcaatcatgggtcaatccctactttccgttgctaaacgtatcgcccttaatctaccagcgggcgagcgtcctagactgttgccatgcaccaccccgccttcagcttcttcgccgacgaaccgctgcggggtgcccccggaggcaggctggacgggtggtggatcccggtaaaggactccaccaacgtgcgcgggtggcccactaccgacggctcgccgcaccgggcccgcaccgcgcggacgaccgacccgattgcgcagaagttgctcgccgcgggcgcgaccatcccggccaagacgctgacgtccgaattgggcgcgacgtgctacgcggagcggccggacgtgcctgtgctcgaatcccccgcctaccccggccgcacacccggcgggtcgtcgaccggcgccggcgttgcagtgagcttaggcctgtgccgcgctgcgcacggcaccgacgcgggcggctccatccgcgttcccgccgccgcgtgcgaggtcatcgggttcaagttcggcggtgcctcgctcgcagccgacgggttcctcgcgcggagcacggcagagcttcgtacggtgctcggctggccgccgcagcttgaggtgccccgcaggttgcgcattgggttgcttaccgacggcctgtttacacccaccaccctccaacccgagcgcggcgacgccgtcaccgcctgcgcgtcaacgctggcgaaacggcacgacgtcgtcgacatttcgcgatacccgcaagcatgcgcaacctacgagcatttcacctcgctgatcacctccagcttccgcaagctcgaccccttggacagcgagtacatcgcgtggatgaaagagaccggcagcggtgtaactgccgcgcagcttgcagacgcggtggcgcaccgcgcagagcttcccggcatcctcgccgcagcgtgggatgtcgatgtcgtgctctcccccaccctcgcgtacgacccgccggctatcggctacttcccgtctttgcctcctgaggagagcttccacgcgcagacggagtggtcgccgtggtgttctttgttcaacatgctccaagcccccgcgcttgccctcgggccggtgcaccttggcgcggtcaccgcgaccgggcgggagctcctcgccttggccgatgagctccgtcccgcctgagcgcgttacgcgaccagcgtgcccacctgctcgccggagacggcgcgcttgatgttgccctcctccagcaggttgaacaccaggatcggcatatcgttgtccatgcagagggagaacgcggtcgcgtcggcgaccttgagccccttctcaatcacttcgcgcggggagatctccgagaaaagcaccgcgtccgggttcacgcgcgggtccgagtcatacaccccgtcgaccgccttcgccatcagcaacacttcgcagccgatttccagcgcccgctgggcggcggtggtgtcggtggagaagtacggcatgcccatgcccgcgccgaagatgaccacgcggcccttctccaggtggcgggcggcgcgcagcggcaggtacggttccgcaacctgcgccatgttgatggcggtctgcacgcggcagtccacacccatttggccgaggaagtcctgcagcgcgaggcagttcatcacggtgccgagcatgcccatgtagtcggagcgggcgcggtccatgccgcgctgctgcagctcggcgccgcggaagaaattgccgccgccgatgaccacggcgacttgggtgccggcgttgtgcacgtcggcgatctgacgggcaacgctttccaccacgtcagggtcaatgccgaccttgccgccgccgaacatctcaccccccagcttcagcatgactcgcttgaaaccagtgcggttggggttgatgtcagtcaccgggaaatgctccttcgcgcggatgggcctgcaaaatgttcgcagccgatcttagccccgcgcacacctaaggtaggaaccggccgcgcgccaccggccggggacggcaaaaccccgcacccaaccggccgcgtgcgcggcaagtttcaagggtgcggggtgtgcgggtgggcagcgagtgcgccacctggcggctacttaggcctggccgacctcgtagcggacgaagtcggtgatctcgatgccgctttcttcagcgaactgcttgacagtcttcttggagtccgccagcgacggctggtcgagcaggacgacgtccttgaagaagccgcccatgcggccctcgacgatcttggcgatggcagcttccggcttgccctcgttgcgggtgatctcctcctggaccgcgcgctccttctcgatcacgtcagccggcacagcctcctggttgaggtagcgggccttcatcgcggcgatctgcagagcaacctggtgcgcagcctccgcgttgtcgccggtgtacgcaacgagcacgccaacggccggcggcaggtccgcagccttctggtgcaggtagacctcgacattgtcgccctcgatggtggccgcgcggcgcagttccagcttctcgccgatcttggcggagaggcgctccagcacgtcgtgcgcggtctcgccgttcacgtcagcgttggccagctcctcctgggagtttgccttggcggcggcagcagcctgagcgatctggtctgcgaggtccttgaactcctggttcttggccacgaagtcggtctcggagttgatctccacgatggtgttgccggacacagcaaccagaccctcgagcgcgttgcgctcagcgcgcttgcccacgtccttcgcacccttgatgcgcaggacctcaacggccttctcaaagtcgccgtcggtctcctcaagcgccttcttgcagtcgagcatgccggagccggtggtctcgcggagcttcttgacgtctgctgcagtgtagttcgccattcgggcgattcctcctcaagtagtggggaaaggtgtttaacgttagaaagactagccgaagacttttgcctcggcagaaatagggggcgcaagcccacgcaaaaagccccgcgcgaggcggggcaatttcgtgcgaaggcgctacttaggcctgggtggcggactcggtaccagagatctggatgccctcgtcgaccttgccggtcttgttggctgcctcagcctgcttggcctgctcagcagcgcggacagctgccggctgctcaacctcctcgacaacctgcggggacgcagcctcagcggcggcagctgctgcagcagcctcagccggagcaacatcctcggaggacgcagcctgcgctgcggccagggaagcctcagcctggatcttggcgtcgctgtcgccagcggcgtcacgagctgcggcgagctgacgctcctcgcgctgctgcttgccctcgatgacagcctcgcccacgatgtgggtgagcagcttcacggagcggatagcgtcgtcgttgcccgggatcgggaagtcgacttcgtccgggtcgcagttggtgtccaggatggcgacaaccgggatacggagcttcttcgcctcggagatggcgatgtgctccttgttggtatcgacgatccacagtgcggacggagccttggtcatgtccgcgatgccgccgagcacgcgctcgagcttgatgcgctcgcggttgagcatcaggacttccttcttgccgcggcctgcgtagccgtcctcggctgcgtccatcgcctgcagttccttcatgcgggcgattcgcttggacacggtctggaagttggtgagcatgccaccgagccagcggtgggtgacgtacggcatgccgacgcgctccgcctcttcctggatgggctcctgagcctgcttcttggtgcccacgaagagcacggtgccgccgtgtgcgacggtttccttcacaaactcgtacgcctcatcgatgtaggtcagcgtctgctgcaggtcgatgatgtagatgccgttgcggtcggtgaagatgaagcggcgcatcttcgggttccagcgacgcgtctggtggccaaagtgcacaccggcgtcgaggagttcgcgcatggttacgactgccatgggaatgtctccttcggagaataatcgttcggttttctagtggtcgtgttgcgcgggtttttatcccgcgccctggcaccgggctagccctgcacccctttcgagggaccgttgctgagctggtcttattcggcgcgcgtagtcagccttcgcagactgccgggataacaatacccagcgcgggctggaaaacctaattgatcagcgcgattgtggataactcggttgccgcccgcacggttattcacaggcgcaggggcatcatgctttacgacgcccccttcaacccccacactatccccatgcaataccccgccctcaccctgttgagcgccgccctcaccgccgccctcttcacttttaccgccgcgcccgccgccgcctgggtcgacccgaccaccggcaacccccacccgacaaacgtggcccgccgcgcggatatccccgagaagaactggctccccggccaccgcggcgtggacttaggtgcccgccccggcgcggacatcctcgccaccgaggacggggtcgtggcgttcgtgggcgtgatcgtcggcaccccaaccatttccatcgaccaccccggcggcatccgcaccacctaccagccggtgcacgcgcgcgtggccgttggcgaccacgttgtcgaaggcgacatcatcggcacacttgcccgccccgcgtcccagttcgcccgcgagcacgccggcctgcactggggcgcgcgcaccggccccgaccactacatcgacccgctgagcctcctcgagccgccgcgcatccgcctcaaaccgctcgacccgtctcaggcgcgcgggtgagcttggtcgtagaccttctttaagcgctgcgccgagacgtgcgtgtagatctgggtcgtttgcaaactggagtggccaagcagctcttggactacgcggatgtccgccccaccctcaagcaaatgggttgcggcggagtggcgcagcgagtggggagtcacgcccgccgcgtcggcgtccctcgccgattgctcaacgatgcgccgtacctgccgctgatcaatgcgtttgccccggcttccgagaaacatggcggcctcgctgtcggggccggctagcttcggccgcgccatctccatccactcgcccaccgcgtcggctgcgggcccgccaaacggcacgacccgctgcttgttgcccttgccggtcacgcttgccacgccgcgcgcgaggtcaacatcgcctaggtctaaaccggtgagctcaccgacgcgcatgccggtggcgtacagcagctcaaggatcgcccggtcccggcacgccaccgggtcgttgtcgtccgcgccttccccgcccggcgcgcctgccattgccgcggcggtgtcggggcgcacgacggttggcagcggacgcgagatctttggcgcgacgaggcgtgcggcgacgtcacattccaggtagccctgtttgtacgcccacgtggagaatgcccggaccgcggcggtgcgccgggcgagcgtggagcgtgccttgccctcgctcacagcaccagcgagccagagccgcaggttgtccagggtgaattcggcgaaggagtcgaccgagccttcgagcgttgccaggtcggcgaggtaggcgcgcaccgtgttgtcgctgcgaccgagcaccaaccgcgcgtgctcggcgaagtcttcagccgccgccgatacctgggtcatgcatcaggagtgtaatcccgccacttccgttacgcggcttcgatcgacgcccgccgccacaaccgccgctccctgaccaccaactgccgctgctgcaattccataagcaggtgcacggtcagccccaggctcaggccggcgaccgccgcgacttcctcagcttcacgcccatcgtcgccgacgggcggcagcgagtcgtagacccgcagctcgttgtgggaaagctgctgcagcggggttggcgcgaacagcgcctccatcggctcgcgcgcatccgttgcgccgacgggccccaacagctcgtggatgtggtcggcgctcaggacggcttgcgcgcggccgtcgacaatagccaagttcgtgcccagcgacgactggctcattatcgagcccggcactgccatcgccacgcggttgtacgcgatgacccacttcagcgtgttgagcgcaccggaccggtagcccgcctccaccacaaccgtacccggcgtcagcgcggcgatgaggcggttgcgggtgaggaatcggtggcggtcgggggtgactccgggaggatactcgctaatcactgcaccgccttcggcgacgacgcggttgaacaggcgctcgttgctgcgcggatacgtcaccccggccccgcacgccgcgatcacaaccgacggcgcggcgttcgccagggccgtgtcgtgcgcgacagtgtccacgcccagcgcgccgccggagacgatcgtgtagttgtgcttcgccagccccgcgaccaggttggcggtcgcgccgtgaccgtcttgggtggcattgcgcgtgccgacgataccgacggactgggcaaacaacgccgcgaggtttgtctctccccgaacccagagcgcgtggggttcgcaacccccgtcgacgatctcagcgcccggcgcgccgaagctagcctggattgcctcgcccggccactccggtgaatccggggtgatgagggtgtagccgtaccgctgcgccgtctccaagtcggcgaccgggtccgctagccggtagcgggcctcggtggcgcggccgaggccgccgagccagcttgcgcggctgcgcactccgtcggtgatctcgtcggcatcgcgaccggcgcgaagcagggcttgcaggtgcgggttcgggccttcgatgacacgtgaaaggtaggcccaagattcaagcttgctcacgccgccacccctgcccccgtcgcaccgcgaagcgtcagcgcctcgtcgatgtgctccatgtgcggggtgtcttcgccggagagatccgcgaccgtccacgcgagcttgagtacccggtccacaccgcgctgcgtgagcgcttggcttttcagcatccactgcagcgtttgcgccgcggcttccaccggcggaaagtggcggcgcaggaaggccgaatccacccgcgcgttcacggccgcgttgaggcccgccttcgaccacctggccgccgcccgctcgcgggctccggcgacccggtcgacgatctcggccgacgtctccaccccgacggggctaagtacggcagactgcgcggtggtggtgaggaagatgtcgaggcggtcgcgcagcggccccgagacgtttgccaagtggcgggagcccgagcggcacgtgcactcggcacccgatttgccgcaccggcaggggttggcggccaagatcagctggaagtcggccgggtaggtaacttctcgccggttgcggcggtgcactacctggcgcttctccagcgggatgcgcagcgagtcgaggacgtgggcgctgatctcggacgcctcgtcgagaaacagcacgccgttgtgcgcctggcttaccgcgccgggccgtggcgtgccggatcccccgccgatgagctcgactctggtcagcgacgggtgcggcgcaacaaacggccgctcggcgacgatctctcccctcgacacaccagccgcggaatgcagcgccgtggtctcaatctgctccgccaccgtcagcggcggaaggatggaaggcaagcgttccgccagcatcgattttcccgatccgggcgggccgaccatcatcacgtggtgcccgccggctgcggcgacctcgagggctttccgctcgaagagctggcccgccacgtcggcgaagtcgggggctgccggtgccgcagcggactcccgcggcacgtcgatggcccgctcgaggccgacctcaccgcgaagccactggtagacctgtggaagcgtgtcgccgagcagcacgcggcgctggccgagcagcgccgcctcctccgcgttggcgcgggggacgatgacggtgtcgaagtcgaactccggcgcctggccgcgcgcccgttccgcggccagcagcatgggtaggacaccctccacgcgcctcagcgagccgtcgagggcgagctcccccatgatgacggtgcgccccaaccgcgcgtggaccgctgggtcgaggctagccaccacgctcagcgcaataggcaaatcaaagtggctgccggccttcggcaagtgcgccggcgagagcgacaccatgatcttggtgcgcggccacggcaaagccgtgttcgcgatcgcggtacggatccgctcgcgcgactccttcaccgccgcgtcccccaaccccaccatgtgcatccccggaagccctgggcccacgttggtttccacggtgaccatgtgggcgctgaccccttcaaccgtggcggttagcgtgctagcaagcgccatcttcgaccccctcgaagcggagcatcgtgtactcggtgaagccagcgccgtcgaagacgacctcgcagacgtcgaagcggacgtccacgtacccaccgtgcggagatcggtcgagccactccccggcgcagcggcgcattgtgagaagcttcttggcagtgacggattccgccccgccgtactcgttactgcggcgggttttcacctctaggaacaccacggtgccgtcgggcgcggcgaggaccgcgtcgatctcgcctgcacggcaccgcacccgctggttcagcacctggtagccgtgctcggcgtaccacgttgcggcgaggtcctcgccgaaacggccaagggcgtactggtcagcaacggcgctatccgggtggccaacgttttccgccaccgtgccgtgtgtaacgcgcggcatgccggtggcgggtgtgcgggtgaggcttaacgtgtggtgcgacatgaatcgctcccccttcgtttcatcgtgtgcggtatgtaaacgggatttatcgggagcagaagaaaaactgctccatcctgttagaccgatgaaacgggtgcgcggttcccccgaaccacgaaaaagcgcgttgcgctagcgctgcgggaaggcgatctccggcttatccagctcttcgatgttgacgtccttgtaggtgatcacgcggacgtagcggacgaagcgcacggcgcggtacatgtcccacacccagcagtcggacatccgcacctcgtagtagacgtctttgccctcggtgtgcggaattagctcgaccgcgttcgcgaggtagaaacgccggtcagtttcgaccacgtaggagaactggctggccacgtcgcggtactcgcggtagagcgacagctcgacctcagcttcgtaattgtccagctcttcggcgctcatctaccgcacaacccctttgtaaacctcgttggcttcacggacgtttgcataactataacggtgctcgctactcgcaccgtggcggcgcaccgcatccatatgcaccgccgtggagtagcccttgtgcttctccaacccgtactccggaaagtccgccgccatctcagcgatcagctggtcgcggctcaccttcgccagcacgctcgcggcagcgatgcaacgcgcggtgtagtcgccgccgaccacgggtaagtgcggcacggctaggccggggatggcgaagccgtccatgagcacgtattgcgctttggggatgagtcccgctaccgcgcgacgcgccccgtcgtagttcgcggtttggatcccgcggcggtcaatctcggaggcggggatgtggatgacggtgtgggcgagggagaggttcacgatggcgtcgaaaagcaatgcccttttcccgacagaaagcttcttagaatcagtgagcccctcgagcggcggcagcggcttggtgggaaggatgcacgcggcgacggttaaggggccgaagcaggcgccgcggccggcttcgtccacccccgccacgggtccgagccccgctttctccagcgccacctcgtacgtgcggagctgcttcaagcggcgcacgctagtgttggatatccgggttcgccacgttgccgaaacggctgagcgggaacaccacggcctgcacccggccgcgcaggttctcgcgcgggatggtgccctggtactcgtcgcccaagtggtagcgcgagtcggccgagttggtgcggttgtcacccatcatgaagtagttgccgtcgggcacctggaccgggccgaagtacgcgccgccgcaggcctcggaaccagtggtctcgtccaccgggtaggtcggcggcgacagcacgtacgactggtcgatcggctcaccgtccaccatcaccgccgggtcgcccgcctggcaggacacggtttgcccgccctctgcgatgatgcgcttgaccaaggtgttctcatccttcggcacgagccccacccaggagccgacctcctgcatgccgcgcacgaaagcgttggacgagcggttggagtagaaaccggtgttccacgagtcggtgcccttgaacaccaccacgtcgcccggcttcgggtcgttgaagtagtagctgactttctctacgagaatccggtcgccgctgccgttctcgccgtggagggtgggttccatcgaggcggaggggatcacgtacagccggccgaggaacgtctggatgacgaacatgatcgcgagcgtgagcacgatcaccgcggggatttcgatgtaccagggcgcctggttgtcgtccttcgcggccgtatccccggcgcgttctgcggcgcccgcttcttggcgctgcgcggactggtcgttcgggaagtgcggttcacgttcggtcgagaccggttcattcgggttggtcacccgagatactctacacccgccgcgccgcgcaacctgcatcccacctgcggttttctcttctgcaggcaggaacgcgaaaacccgctcaccagcagcctcgtgcgtggtgagcgggttgaaaacgcgtgaagattagcggcgctccttgatgcgggcagccttgccgcgcaggtcgcgcatgtagtagagcttcgcgcggcggaccttaccgcggcggacgacctcgatcttctcgatgttcggggagtgaaccgggaaggtgcgctcaacgccgataccgaaggagatcttgcggaccgtgaaggtctcgcggatgccgccgccctgacggcgaacgacgaagccggtgaagacctgggtacgggtgacagaaccctcaatcaccttgacgtggacgtcaagggtgtcgccggggcggaagtcagggatgtcgtcgcgcagctgacctgcatcgacaaggtcgataatgccgttgctcatagtgaagcaatcctttacatgtacggacagaggacccagtggcgctggcgctcaaccatgctctcctggttcgtatcgtgtgcaataacctccgataccttacatatcggccggtcagttaccaaatcccgcccgcttgagcgcgtcgctcatcgcgttggaggctgtgccgccgtcccggccggagcgcgcgcgaccgccggagcggtttccagaccggttgccgcggcccttgtcgcgttggccgtttccgccaccagcgccgccgcgtttccccttcggtgccggctggtcgtctagccgcatggacaggccgatgcggcttcgctccacgtcgacatcaaccaccttcaccttcaccacctggccggagcggaccacggcgtgcgggtcttcgacaaaccggtcggcgagctgggagatatgcaccaggccgtcttggtgcacacccacgtccacaaaagctccgaaagcggccacgttggtcacggtgccctccaggatcatgcccggtaccaggtctttgacctccgtgacaccctccttgaacgaggcggttttaaactccgggcgcgggtcgcggccgggcttgtccagctccgcgataatgtcggtgaccgtcggcacgccgaaggtgtcgtcggcgaaatcagcgggccgcagcttggtcaacaccgcggagttgccgatcaacgcatcggtggccagcccagccgattgcgcgattcgcttgaccaccgggtaggcctccgggtgcacggccgaggcgtccagcgggtcagctccgccgttaatgcgcaaaaatcccgcggcctgctcgtaggccttcggccccaggcgcgacactttcgtcagctctttgcgggtgaaaaacgagccgtgctcgtttcggtagtccacaatgttgcgcgcaatcgttgggctgatgccagcgactcgctcaagcaggggaaccgaggcggtatttacatcgacgccgaccgagttcacggcgtcctccaccaccgcgtccagcgacttagccagggcggtctggttcacgtcgtgctggtactggcccacaccgatcgacttcgggtcgaccttcacaagctccgccagcgggtcctggaggcggcgggcaatcgacaccgcggagcgcagcgagacatccatgtctgggaactcggccgcggcgatttcacttgcggagtacacggatgcgccggattcggacaccaccaccggggtgggccgcgccccgcccgcctgggcgatgaggtcggccacctcgccggcgagcttctccgattcgcgcgaagcggtgccgttgccgatcgcgatcagctccacgccgtgctctgcggcgaggctggcaagctcggcgcgcgaagcgtcccagcggttctgcggctggtgcgggtagacgatcgtggtggccaggaccttgcccgtgccgtcgaccaccgcgcacttgaccccgtttcggtaccccgggtcgagcgcgagcgtggcgcgctggccagcgggggcggcgagcagcacgtcgcgtaggtttgtggtgaacacctccagagcgccggcttcagccttctctttgagccgcattcgggtgtccacgttggccgagaccatcagtttggtgcgccacgcccagcgcacagctttggcaacccactcgctgtcgtgcaccggcaggtcgaagtgcttggcaatcatgccctcgtacaccgcgtcgtcccccgcgtcgagctgcagcgcaagcacaccctcgttctcgccgcggaagagcgcgagaatgcggtggctcggcagcgtgtcgaaatcttccgagaaatcgaagtagtcggcgaacttcgcgccgtcacgctccttgccctcgaccacgctcgcgcgcatcgtgccggtttcgtacacgcggtcgcgcacctctccgaccaagtctgcgtcgagcgcgatgcggtcgaccagaatcgcccttgcgccctcgagcaccgatttttcgtcggggaacccctcagaggtaaaccgtgcggcgaaggtttctggggtgttgctgggtgcgtcgataagcagctgcaccagcgcttccaaccctgcctcgcgcgcgatgtccgccttcgtcttgcggcgcttcttgtacggcgcgtagaggtcctccagacgcgccttcgtgtccgcggcggcgagctgggcgtgtagctcgtcggtgagctggtcgccgatcgcctcaatgatcgcttcgcggcgctctgcaagctccgtgaggtagctgttgcgcgcttcgatgtggcgcagctgcgcgtcgtccagcccgccggttgcctccttgcggtagcgggcgataaacggcaccgtgttgccctctttgagcagggtaagcgcggcctccacctgggagtctcgcaccgaaagttctgtcgcgattgttgctgcgatagtcattcggcacagtgtagcgacccgctcacacacccctcgtggcaccgcgccactgcaaccccttcggcagcgcctgagccaccgcatccgtcgcggcttgaagctccagcgctgtccgcccacgcacggtgattgccgtggtgccgtccgcccgggtttcagcctcgatcgcatccggctggtagccagctttgcgcaaacgcctgcgcatctgcttttcgacgccccctcgaacctccccagccacctcaatctcagtcaccacagcccgcgcgtgaagcgcgaagtggtcttccgtgctcaacccgccggcggcctcgaccgcttcaagcaggtccgggcgcaccgcctgcgtgcgcttcagcgacgcctccctccggtacgccgccaccttcgcgtggtcgccggaggcgagcaccgccggcgcctcgatgccccgccagacccggggcttggtgtagctgggtccttcgagaagcccgtcggagaagctgtcgtcctcgtggctttcggcgttgcccagcaccccggggatcaacctggtcacggcctcggcgatcaccagcaccgccacttctcccccgatgagcacgtagtcgccgatggagacctcgcggacgcggtagcgcttcgccgcgtcggtgaacacccgctggtcgatgccctcgtagcgcccgcaggcgaagacgatgtggtcttcgttcgaccacgcctgcgcgtccgcctgtctgaacggagcgcccgccggggtgggcacgatgagcagcggcaggtctgcgtcctcgccgtcgcgcacgtcgcgcttctcgtagccccgcgcggctgcgccttggacatcgtcgtggcgcaacttgtcgtttctgtgcgcggcggccgtgtcgaggcgcacaccgccgcggcctgcggccacgtcgtccagcgccggtccccacacctccggcttcatcaccatgcccggtcccccacccagcggcggcgcgtcgacggacttatggttgccggtcgcccagtcacgcaagtcgtggacccccacctctaggatcccctgctcgatcgccttgcctagcagcgcgtgtcgcagcggttctaggtactccgggaagatcgtgacagcgtcgatcctcataggtcgagcagcccctccggcggggtgatggtgagaaaaccctcgtccaaatcgacctcgggcacgatgtccatcacaaacggcaccagcacctcccggccttgatagtcgacctcgaggatcttgcggttgggtgtgtccatcacgccggtgacttcgccgatctccccaccgtccatacgcaccttcaaaccgatcagctcgtggtcgtagaactcgtcggaatcctcctcgcgctccagcggcggtgcgtagaacttcatcccacgcaggctgtccgcggcggtgcggtcaggcacctcctcgaagctgacgaggagccgctgctggtgcgggcgcaccgtcttcacggtgagatcttgttctttgcccgtctggcggccgtgaagcacctcgcccacggcgaagcggacgtcagcctcgtcggtgagcacttcgacagccacctcacctttgacgccgtgggacttcacaaccttgcctatcagcagcttcatgacgtgcaagagtagcaaaacgacaacacccgccctcgcccacgcttgcttgcgtgggcggggcgggtggagctttgtgcggcagcgggagcttagttctcctcagccgcagcctcagccggagcttcctcagaagcctctgcctcggcgttctcggcagcctcagcggcggcagcggcctcagcctcggcagcagcctttgcctcggcatcttccttagccttcttgcgcttctcggtgatcgcctcggcggtcgggccgttgttggcctcctcgagcgccttgttgaacagctcgagcttggacggcttctcctcggccaccttcagggtgccctcggcgccctcgatgcccttgaacttctgccagtcgccggtcaccttcagaaggttcagcaccggttcggtcggctgcgcgccgacacccagccagtactgagcgcgctcggagtcgatgcggatgagcgacggctcttccttcgggtggtagatgccgatgttctcgatgtagcggccatcgcggcgggtgcgggcgtcagcgacgacaacgcggtactgcgggttgcggatcttacccatccgctgcagcttgatctttacagccatgctgttatttccttacggtcactgggcagtacagacacccgccgcttgtcgacgggccggttcaacccctggattcacctgcgcgtgactggccgaacggacgtatccggcttcggctctgacgcaggatctgggcaagtgtagcctgtgacgaggctgaatcccaaaccgactaaggttctcttaatgaccactcaggcgcacacggcgggacggaccgcgaagggctcgagcgcataccgcgtcgacctcgacggtctgcgaggatacgccatcgcgctggtggtgatcttccacgtcttcgtcggccgagtttccggcggcgtcgatgtcttcctttttctctcgggctacttcttcctcggcgggcagctgcgctacgcccttcgccccagcccgaacctgaacccgtggtggccgctgtggcgcaccatccgcaggctggtcccggcgctggtggtggtgctcttagcgacgcttacgggcgtcctcctactcgcccccgagctcatgagcgacgaacttgccgcgcagttcaccgcctcgcttttgtacttccaaaactgggagctgaccgcgcaagacgccgcctacgccgcggcgagcagcgccacgtcgccgctgcagcacctgtggtccatggcagtccagggccagttttacctcttcggcatcgtcctcggcacgcttgtcgcagtgctcgcgacgaagacgaagctcggccccgaagccgcccagcgtgtggccgtcatcgtcctgtccgcgatcaccgtcgcctcgttcatctgggcttcccgtttcgggctcgtgggcacacctgcgaactactactccaccttctcacgcgcctgggagctctcgctgggtgctctgctgtcgttcgtgccagcgcgaatgttcatccccgccccagcaaacgggttcaccgccttcgtcggcgtcatcttgatctccatcaccggcgtagtgatcccgacctcgctcgccttccccggcccgcttgccctggtgccgctcacgggcgcggcgctgatcatcctcagcggcaactccagttccgtgtctacggtgttgtcctcaaagccaatgacgtggctcggcggcgtggcctactcgctctacctctggcactggccgatgctgatcatcgtcaccgcctccggagggttcgacaccccgccaccgctgattggcgccgccgtcatcgcggcgtctttggcgctcgctcacgtcacgcacatgcttgtggaggaaccgctgcgccagcacggcaagcgcccgctcgccaccgactccccggtgcgcgacgcacggaagacgctgcggacccccgcaggcattggccgagcgagcggcggtgccgtcgtcgctggcctcttcgtcggcgcactgacgatccagccaacgtggaaccaccgcgtggaccaggcggaccggccgctcgatcccgccacataccccggtgcgctcgccctgaccggcgcggaagtgccggacgtcaagccgcagccggacccgagcctgattgccggcatctaccctccgatcggagagcaggactgcatgatcttcttgccggcggcacccgacgcgatgccgcgccccgactgcgtctacggcgatgtaaacgcagaaaccacagtggtcatggccggagggtcccacatcgagccgtttgtgatccccctcgacatcttgggcaaggaacacgggttcaaggtggttccctacgtgcgccaggagtgccccttggtcgttggcggggaggaccgcttcgatattgtctcggaggtgtgtgccgagtggggggagaatgtgtggcaggaggtcgtcgataagcaacctgccctggtgatttccacctcgacccgtcctgcgggccacgctggggccgtggatacgtcggtggatacggtgcccgatgcctacgccaacctgtggttcaacctcgctgaagccggcataccgtttctcgggctgcgtgacaacccgtggttcttcgatcagttcggcaacccgatggacccgaacttctgcatcgtgtccggagacagcgagcgcaactgctcgatgccgacgagcgaggtctaccccgagtccgatccggcagcgggctaccttgacggcacgaacaacctcttctccgtggacacggcgtcgtggtactgcaacgaggagttctgcccgccgcagatcggcaacgtgtacgtctaccgcgaccagaaccacatctcgaacgcgtacgcgcgctcactcgcaccgctgctgtgggcggagatgcagccgatcttcgaccagcttggtatcgcccataattaggttttgtggctgcgcgattggcggggaccagctagaagaacttgcccttccccatgcgcttcatcgcctcgttgaagtcgaggttgttgaggtcgagtccctgcatgcctgccggcagctgctcctggagcttctccagctccttcgggtccggcatcccgcccggcataccaggcatgcccggcatgccaccgggcatccccgggaacccagccggcatctgcggcatgccgccgccctgacgcttcggcggcttgcgcttgccgttcttgcccttgcggcccttcggcttcttcttcgtcgcggagcgcccgcccatccccggcatgccggagagtccgaactggctggccatctgccccatcatcttcttcgcctcgaagaagcgctcaacaagctggttgacctcggcaacagtgacgccggagccgttcgcgatgcgcttgcggcgcgaggcgttcaggatcttcgggtcgttgcgctcctgcggcgtcataccgcggatgatcgcctgaatgcggtcgagctgcttctcgtccaccatgtcggccatctcgttcatggccttgccgcccggcatcattttcagaaggttgccgatcgggcccatgcggcggatcatcagcagctggtcaaggaagtcctccagcgtgagctcgccagaggccagcttgttcgctgcggcctctgcgtcctgctcgttgtaggtctgctcggcctgctcgatcagggagagcagatcgcccatgccaaggatgcggctggacatgcgctccgggtggaagacgtcgaagtcctcgagcttttcgcctgtcgacgcaaacagaatcggtttgccggtcacttctcggatggacagcgcggcaccaccgcgagcgtcgccgtcgagcttggtgaggaccacgccggtgaagtcgacgccctgggcgaacgcctccgccgtctgcaccgcgtcctggccgatcatcgcgtcgatgacgaagaggacctcgtccgggttgacggcgtcgcgaatgttgcgagcctgcgtcatcagcgtctcgtcgataccgaggcgaccggcggtatcgatgatcaccacgtcgttcttgttctgcttcgcgtactcgacgccctgcagcgcaacgccgaccggatcgccgtgggaagtacccatctcgtgcgcgtgcgagtcgatggacgtacccggatccggggcgaaggtgggaacgcctgcgcgctcaccgacgatctgtagctgctggacggcgcccggtcgctggaggtcgcaggcgacgaggatcggagtgtggccctgcttggacaggtgtttggccaacttgccggcgagtgtggtcttaccggcaccctgcagaccggccaacatgatgacggtcggcgggttcttcgccatgttcatccggcgggtctcgccaccgaggatgttggtgagctcctcgtcgacgatcttgatcacctgctgggcagggttcagcgcctgggaaacatccgcaccgagtgcgcgctccttgacgcgcttaataaaggtcttgaccaccggcagggagacgtccgcttcgagcagcgcgatccggatctcgcgggcggtggcgttgatgtcggcctcggtgagtttgcctttgccacgcaagccaccaagggccgtttgcaagcggtcggacaatgactcaaacacgtcgagtcctcctgtgaactaatcgcggatataagagcacatatatacggtgcaagttaacccgtcccagcctagcgcttgggtggtatgaggccgaaacacgagcaggtgcatgcgcgcggcgtcgaccgggtcggcggcagtgtgtccacctctaccggagggcgtccacctctaccggagggcgtccacctcggtaaggggggcgtctggcggatgacggaagtaccgcttcgggaaggcatatccgccctccttcagacgccctccttcatccgccccccctacttccgccttttgggatccggcgcaccacgcccctccccccctccgccgccccc

SEQ ID NO: 5 - DNA, 272157 bp, Corynebacterium cassirii
  source 1..272157: mol_type = genomic DNA
gcatgtgttaagcacgccgccagcgttcatcctgagccaggatcaaactctccacaaaaacatttcagtaaaagaaaccgagccgtgaaaagcccaaacccaaccaaaacaaaaccacccaacaaaaaacgttggactggcaatcctttgaaaaaacgttggccatgtatccgacgaggaaaaaccacaaccaacaaaaaatagtgaaaccatcacacgtcccaccgtccaacagcaccacccaaagaaaaagcagcactgccaccggcacacaccacaacaaaaaatcatggcgcacacgcacaacaatcacaccaaacaaaaaagtattggcacactatcgagttctcaaacaacacacgcacacccgcttcggaactttctaagcccctcggctgcggtagctcgcatcacgttactgggaatgttttttcctgtcaacccggcgttcattgcccggtttctcggagttcatgtccccgtaacctctatgctcttattttcgttcctccctgttcggaagcaacgggagaagatataaccatgcaatgagaatgtcagcaaatcaccagctcacgccgcctagtggtaggtcgcgatcggcccgtgcggcccgtcgatcacttgcaccggcgtattgaagatctcggtgagcaagtcgtctcgcatgatctgcgccggggtgccgaaggcggcgatggcgccgtctttcgccgcgcagatgtagtcggcgtagcgcgccgcaaagttgatgtcgtgcaggacgatgacgatggttcgccccagttccgtcgccgctgagcgcaagtgctgcatcatctccacactgtgggcgatgtcgaggttgttcaacggctcgtcgagaagcacatgctccgtttcctggcacagcaccatcgcgacgtaagcgcgttggcgctgcccgccggagagctggtcgaggaaccggccttccagcgcgttcagacccagaaagtcgatgtacttggaaatgatctcctcgtcctcatccgtgaggcgcccgcccgagtacgggaaccgcccgaaaccgacgagctggcgcaccgtcaacctggtcacgaagtggttctcctggcgcaggatggagatgaccttggctaggtccttgttcttcgcctgcgtcacgtcggtgccgccgatcgacaccgtgccggaatctaccgcgagcagtcggccgatcatggtgagcaacgttgacttaccggccccgttcggcccaacgagggcagtgatacccccggtgggaatctcgagattgacgggtccgatggcaacgtcgctgctgtagtccttgcggacgtctttaagcgtaatcacaagcgccccttccttaagatgaccacgaggaacgtgatcccgccgacgagttcgatgatgatggagaccacgccctgcgcgtagaagatgtggttcatgacgaagtacgcggccgtcaacacgcagtaccccagaagcgccgccatcgggaagatgaagcggtggtcgtaggtgtcagtgaactggtacgccaacgttgcgacgaggaacccgaggaacgtcatcgggccaaccagcgcggtcgagatggccatgagcaccgcgaccagcacaagggtgtagatcgagtgccagcggaagttcaccccgaggttgactgcggcgtcgcgcccgagccccatcacgttaagccgctgcgcgttcagactgagcagcacgacagcgaccgcgacaagcgggatcgccaccgggtagtaatccgggttagcgttattcaccgagccgaacaggcgcgcggtgagcacgtcgaactcgctcggtgtgagcatccgttgcatgaaggtggacacgctggccagccccccgccgatcacgatgccgaccagcagcatcgcgtgcatgttggcttggttgtcggttagaagccacgagtacagcagcaggctgagccccaccatgaccgcgatctggaagaggaacatttccagcgagcgagcgttgatcagccccgacgccccgaagaagaacaccgtcgcggtgtgaatggtgatgtagagggactcgaagcccatgatcgacggcgtgaggatgcggttgttggtgacggtttggaaggcgaccgtcgcaaaggcttggctcactgccacaatggccatcgcaagcacagatgctaatcgacgctgcgcaatcagccagtacgcccgagtcccaaactccaccgggttcttgtacgccagcaacccgaacgtggcgccggctgcaacaagagccagcaacgccagcaccatccagtaccgccgcctgctcgtcgcggactcgaacgcccctactgccctgttagccacgtcgcgtctgcctcacaatcagcgcaacaaacacgacggcgccaaccacgccgaggatgacggagaccggcatctcgaagggcgcgatgatggtacgcccgaggatgtcgcacacggtgacaatcatgacgccgagcaggcagacccacggcaggttcgaccgcaggtcgtcgccgcgcagcatgctcacaatgttcggcacgatcagccccaggaagggcaggttgccgacgaccacggtcacgacacccgctgccaccgccacgagcgccgtgccgaccagcacgatgcggtcgtaattcagcccgatcgtggtggcgatgtcttcgcccagcccggcagcggtcaaccggtccgcgtacacgaacacgatgacggcgacgaccgcgaccacccacagcacctcgtactgccccttgataaccgaggtgaacgagccggcaaaccagatgccgagcgactgcagcatgtcgaactgcaacgccaaaaacgtggataccgagctgaccaccgccccgagcatgatgcccacaatcggcacgatcaagctggagcgcagcgttacccggcgcaggaacgcgaagaagatcatcgtgccgacgaaggcgaacgcgaccgccatgagcatgcgcgtcatgatcgtgccgttgggaaacagcacgtacgacatcaagagcccaagccccgcccactcggtggtgcccgtggtggtcggctcgacgaagcggttctgcgtcaacatctgcatgatcagtccgcacattgccattgcggcgcccgcgagcaccagcgcgatggtgcgcggcactcgggtggttgcgaacatctcccagccgtcgtcggagcccaagatgtcgtactggccgacggcgagcgagagagctagcagtgcaaaaacgacgaccacggcaagcccgaacttccaactcagaagcggggggcgggtggtcgtcatcgtttccggcatcgtggtcttacgttagcgcaccgcgaggtgcggttactttgcggcctcaaacatgtcggcgagctggttgaggatctccgtgtaggtgaggatggactcgttggtgtaggtatctttcggcgcgatgtagatgtggttctccttcaccgcgtcgacgttctttagcgcggcggaatcgctgatgaccgacagcgcctccggcgagccctcgtcagacttggtgcccgcgtcgcggtcgagcacgagcagccagttcgggtttgccgcggcaatcgcctcgacggagatgtcgtcgccctggtggtcgtcggacgcgtcttgcacctcaagcgccggcgtgaagccgatgaggtcgaacagcgggccccacgtgcggcccttgcccggcgcgacgtagccgatctcgccgccggagacaatggtcgccatgacggtctgctcggggttgtacgcgtttcgcgcgcgctgcacagccttggtgaagtcgccgacgacctgctcagcctcggcctgcttgccaaagacctcgcccagctcgagcgtctggcggatcagttccttgtcaaagtcttcgttctcgcgcggctcgaagtcgagcaagacagcgtccggcaccagtttctggatgtcctcgtcgtacttctcgaagcgctgccccgagacgatcacgtccgggtcgacggcgacgatggcctccaggttcggctcgcggtggttgccgatgtcaacgatggagtcatcatccgaaatacccgggatcgtggtgggaaccagcgcgcgggcagctgcgactggcttaacgccccacgcgtcgagcagctcaaaggagcggttatccagggcaacgacgcgcttcggcggggtcggcacggtcttctcgccgtagttgtcggtcaccgtcacggtgtcaacggcgctgtctgcgctcgtagcggcgctgcctgcgctggtagcggccgaagtcgcagcagtctcgctcgacggcgtgttggaatcgagtgccggctcagcgttcgagcaggacgcgatagtgagtgacgaagctgccgcgagggcgataagcgcagtgcgcgaaacacggaacatgttggttcctctcctaatatggcctgacgttggtcgaatacgttcatcaacgtattgcacccatcttaagtaaggcaaaccttcgctttgttagagggtgcttagaagggggtgcccgataaggctgaaacgcggtacgattgttgttgacatatcaccaactgtctggagtgatcccacatgaaagctttcgggttcttgagtttcggccactacaccttcggtggccagcgtggcccgtccgcaacggagatggctgcgatccacctcgacatcgccaaagcagctgatgagatcggggtgaacaacgcgtcattccgagtccaccacttcgtgccgcaggcctccgccccgatgccgctgttgggcgccgtcgccgccacgacacaacgcatcgaggtgggcaccggcgtgatcgatatgcgctacgaaaacccgctctacctcgcagaggaagccgcctcgctctaccagcttgccggcggtcgcgtggccctcggcgtgtcgcggggcgccccggaagtggcagagcgcggctgggaggcattcgggtacaaaggcgaggccgcaaacggtgccgacgtggcgcgcagccatctcgaggcgttcatggcggcagtcgacggccgcggctttgccaccgccgcccccttagagcgccagtaccccaacatgttccagcccggctctaggctcccggtcttcccgctcgcgcccgagctgcgtcaacacatcttctacggctccggcacgcactcgtccgccgagcagaccgccaaagacggcctcaacctgatgtcctccaccttggtctccgaaaccaccgcccaaaccttgggcgagatccaagcggaccagatcagccgctaccgcgccgcgtggaaggatgcgggccacgactggaccccgcgcgtgtcggtctcgcgctccatcttccccatcgtggacggcaccgacgcgcaaatgttcggcatgcacgcttccggctccgaccacgtgggcatgcttcccgacgtcggcgcatccaccttcggtcgcacctacgccgccgagcccgacgcattgatcgagcagctcaaggctgacccggccgtcatggccgccgacaccttgctcatcaccatccccactgggatgggtgtggacgtcaacgtcaagattttggagaactttgccacgcacgtggcgcccgagcttgggtggcagccgaacactgcaggaccggtcaccgggtacaccatcgattaacacccatgcacaaagcaggaaacccgccggccgtaacgaccagcgggttttcctctcagtggagccgccgggaattgaacccgggtccttcaccaccgcgccagggcttctccgtgcgcagttcgcacaacgtctctgctcggccctccggatcaggcaaacatgtccggatgacgggcccagtcagtgaaaagtgtcccttccaagaccccactgacagggccggaaggcgagtcccctaagtcgacgccaggtaccggagcggggacatccccggcctgacggacacgcaggtcgcttgctctatttcttaggcagcgagggcgtagtcacgctgagagttcttctctgcgtttattgattgcagcgacgcttacggtggtctcctgcctgcaccggcacgcttcccctggctgagtagatgaagtcgaaaccaaatcgaccccgtcaactacgaagaaaacgtaggagtgaaaaccttaatgcacccccgcgttttacacaaggcctccacttaaataccgctcgggcgcacgcgcaggaactccacgacagcgtctggccccgcatcaacggccaagcgagcagcctttgccacgttcaccgcatccatcttcgggcggtcgtcgtcgccagcaagcatgtcggtgtcggtgcgtcccggatggagcgaggtgacgcggaccttgcccgcctcctcaagctggagtgactcggtgaacccgcggagggcgaattttgaggcgcagtacgcggagttggcctcgatcccgtggaagccggcaccggagttgatggtgatgatgaggccgtgggagcgtcgtaaagcaggaagcagctccttgaccagggtgactggggctgcgacgtttacctcgaaagtctcccgccactgctcctcggtgagttcctcgagcgggcccttgtgcagcacgccagcggcgaggacgaggacatcgagctgctcgaccttgcgcgcggccgcggtcagcgccgcggtgtcggtcaagtcgacctcgaacggctcggcgctcggcagcgcggccaccacctcggaggcgtcggacgaggcaccagcgtaaatgtggtgatccttgcccaactcctcagcgatagcgcgtccgatgccgcgggaagctccggtgacaagtgcggtttgctgtggcttcgtcatgccacccaccgtacgtgcgcaacgcggcgcgggtagctacgccttgatgcccttgagcttgcgaccgagatcgcgggtgatctctcggtcttcggtgcgtcgcttgatgtcgcgacgcttgtcgtaatcctgcttaccttgggcgagtcccagctccaccttggcgcggccgtctttcaggtagagcgacagcggcacgagggtgcggttgccggcgcgaagcttgccctcgagcgtgtcgatctcgcggcggtgcatcaaaagcttgcgggtacgacgcggcgggtggttcgtccagtgccccttcgagtactcggggatgtgcatgttgcgcagccacacttcgccgttgtcgatggtcgcgaacgcttcgacgagggaaaccttgccctcgcgtagggccttaatttcggtgccctgcagcacaatgccggtctcccagctatccaagatggtgtagtcatggcgagccttccggttcgtcgcgaggacgccggagttgctcgtctgtctcttcttcttggccataggggagctaactgtactacgcgccccacaccagcaccagttccgcagcgaggtgacgccggcgtgtaccgcctacttccgtacgtaggatcgcagcgcgacttgggctgcaagcccgccgacaatgacagccgcgagcccgaccagcggcatgactgaccacaccgccgaatccggaacgtgcgcgatcagctgggacgcgtaaaggtcacccagcatcgaatccaccaccgagcgtttgcccaccagcagcagcaccatgcccagcagcgcgccaagtgccaccgaaatcacggcctcgatcacgaacggcgcttgcgtgtaccagcgcgacgcaccgaccatgcgcatgatgccgatctgctctcggcggttgaaggcggccagctgcaccatgttgacgataaggaaaatcgccgccaagccctgcgcgccggcaacaatccaggtgacgttgcggaacgtgtccatggtgttcgcggcctcgcgcacggtatccgcctgatcagtaattacagtcacctgcggcagcgtggcgatctcactgatcggcgccgggtcggacggatccttcagcctcacgtgcaacgcggccggcagtgcctccgggctggtctcgcggacaaggtccggctcggaatcttcgaagagctccacaaaccgttcgtaggattgctggcgggatctaaacgtcacctgctccacgcgatcgtcggcttggagggtgtcccgcacctcccggcaggcctccgacgagcaatcggtgtcattcgccgagatctcctcgtcgagctccaccatcacttcgacgcgatctaagtacaacgactttgtctccgcggttgcttttgagatcaggatgccggcacccagcagggtcagcgtcagcgcggtggtgatgatcagcgcaatcgtcatcgtaatgttgcgcccgaggcctcgcaggccctcgcggaagataaatccccagttcatctagctcctcccgtacacgccgttttgctcgtcgcgcaccagtttgcccaggtccagctccatcacgcggcgacgcatgtcgttcacggcgcgcgcgttgtgcgtggacatgaccacggtcgcaccaaggcggttaatgcgcgaaagcagacccataatctcgtccgcggtcgagggatccaggttgcccgtcggctcgtcggccagcaccagtggcggtttgttcacgaatgctcgggcgatagcgacacgctgctgctcacctccggagagctcgtggggcattcttttgcttttcgacgccaaccccaccaattccagcgcctccggcacaagcttgtcgattcgctgctgcgacttgccgatcacctgcagcgcaaaggcaacgttgtcgtacacgttgagccgcggcagcagccggaagtcctggaacacgtacccgatggactggcgcagtttgttcacgtccttgcctttcagggcgttgacgtggaagtcgttgaaccagatgtcgcccgacgtgacgttctcttcccggatcatcagctgcagaaacgtcgacttgcccgacccggacggcccgatgaggaacacgaactcgtcgtctgcgatgtcgaaggtcacgtcatcgagcgcgggacgcgtcgatgtcggataaaccttgcttacgtggtcgaatcgaatcacgggccacacattacctgttactggtgtgacaggagaagtgttctgtgcaaatacgaaagagcttggccccgcgagggggtcaagcccttttttgcttcacgctcaccgcttacgcggccggcgcgattagtcgttgacgtagaggtactgcttgttcacaaactcgtcgagcgcgaacacggacagctcgcggccgaagccggagcgcttcacgccaccgaacggcagcactgcagagaagtactggccaaggttcacgtggatcatgcccgtctcgatctggtccgcgaccttgatggcgcggtcgacgtcgtcggagaagacagcgccgccgagaccctggtaggagttgttcgccagctcaatagcctcctcctcggaggaaaccttgtagatctccgcgaccgggccgaagaactcctcgtagtagggctccgaaccgaccggcaggtcagtcagcacagccggggagaagtaagcagaggtctcgtccatctcgccgccggtgcgaaggttcgcacccgctgccacggaacgcttcacctgatcgtccaggatctctgccgcgcggcgcgaggacatcgggaagtactcgttctcgcccgggttggacgggtcacccttcttgtaggactcggcgatggcgaccatctcgtcgacgaactggtcgtagatgtcctccatgacgatgatgcgcttgttggaggtgcaggcctggccagcgttgtgcacgcgcttgtcccacgcctcctgtgcagcggcgcgcacgtccgaggagtcgaggatgacgtagggatcggtaccgccgagctcgagcacaaccttcttcaggttgcggcccgcggtctccgccaccttcgcaccggcacgctcggagccggtaagggagacaccctggacgcgcgggtccgcgatgatggtctcgatctggtcgtgggtggcgtagacgttgatgtatacgccgtcgggcagaccagcgtccttcaggatctgctcgaacgcggcagccgacttcggggtgatctcggcgtgcttcaaaatgatgcagttgccgttcatcaggttcgggccggcgaaacgcgcgatctggtagatcgggtagttccacggcatgatgccgaggatggtgccaagggcctggcggcgaacgacggccttgccacccggcacgtcgaccttcttgtcggcgctgtgctcagcggcgttgtccgcatagaactgcatgatgtcgccagagaagttcatctcccactcgccctccgggatgggcttgcccatttcctcggcggcgatctgcgcgagctcgtttgcgcggtccttcagcagctgtgcggctttgccaacaatctcggcgcgctcctcgtacgaggtggtgcgccacgtcttaaacgcctccgcggacttggccaggatctcctgaatctcctcgtcggcggcgaaatcgaaggtttcgacgatctcgttggtcacggggttctgaactcggtactggttgctcatgcggtttatttcctttcgggaatgcttctttagtgttgtgaactatatcactacgcgcccgggttgtaagacccgtcgctcattttgatgccctcgtcctggcccatgtaggaggtctcctgtgtcagggcgtcgagaagcacctggtggttctgcgcaacctcgcgctcgagcgcctcggggttggcgcgcagcagatcgaaacgctcctgcaccatcggcaggcccagctcggtgaacgggcgggacgcagcgtggggcacgttgtagatgtccgcgacgtcgtcgccgtgcatcaggcgggttgcggcgtacatccagtcgtcgatggactcatccgggaacggcagcaggcccttgacgttggtgcggaagccgctgaacagcgcatccaccagcgcgtgggaggcgtcgttcgggtcgccgtccaccgtgtggatcgcgtcgatggtctcctgggaggcgtcgatgtccgtctcgtgctcgagcaggtcgctcggaatgccgagcatgtgaccgacgatccgccaaaggtagaacaggtcctgctcttcttcgacggtgagcttgtacccgaggttgcgcaggtaggtgaacgcgatgtacgtgaagtcgaaccacgtgcgcagcatgtcgaagtcgttgatcggcgcgccccactcgctgtagtccaggccgagcttggactgcacgcggcggacgtgcgcgtgcatcgcgcgcaccatgccggtgtggatgtagctgacgttgccgggcttgaggccgtccttgaggtagacggagtagatccagttcgtggtgtacgccaggcggtgcactgcacccttggtcagctcgccggtgttcaccagcacgtcggcgatcgacggtgcggagtaggtgtggatcagtgctcccgggccgagcgagaggttctgtgccagcaccgggatggatagcgcgacgcgctgaccgcgctcaaggcggtcccagtcgacgtcctcgagggaggcgttcatgtcgttgatgagcgcggcaacctccggcagggtgttctcgtcagccgcgccgcgggccagcgcgccgcgcaggttcggcatgacctccttgctgggggtgccgctggtgtagagcgcgtccgcaaccttgtcggtcgcccagaacgcctgctcaaagcgcttcgcgcgctcctcaccgaactgctcaacaaacgcgtcgcggtcgccgcgcgcgctcggccagtcggagcggtcgtagtgatcggcggccaacgggttctctgcgaaagtttgcgtcattgttctctccttttttcgtggggcgcggattagcgcctggcttccttcgagtcgtcgtgcaagctgtagttcgctttcacgcccggctcgttttccttgatgtaggtctcgatctggttcagcacgtcgctccacggcggcttgccgtcggcagccttcttccgcttcgcctcggcagcgcccggcagcttgtcacgcaagcgatacaccgcagcctcggccttcgccttggcggtgaacgcggccttccagtgcaggtacggggcgtcctcgaagcgagagcccttgaccatgaacttggtatcggcatcgccgatcacggtcgacagcgcgccgagcacctggcccggcatctgcgggtccagcttttccaagatgctcatcagcgcagtcgccacacgctcgtgataggtcgaggagtacccgccgttggcgtagatgaagtcggtcatcttgcgcatctcgtcgccggtcttgggaatcagacgctcctcggcgcccatgaggtggagcacccacgcccagtacatcgcgacgtcgtcccactccttgccagagtgggggcggccgaagaattcgtccaccgcgatcggcatcaatgcgaaccagccctcgccggaaaccaggaaggaggatccgatcgggcgaccaaacgtgttgtagtgctccttgccccacagcttttccagaccgcggttggcctgcgcgtgcagcagacgcacacgcacggcggctttcagcccgtcactgtagcggtcaaacactccctgcttacccaagtcgacgaagaacttgacggtctccagcgtgcgcgtcatcgcctggaactcgaacatgccggtctcaccagtggccgccgaggtgcggtcctccatcgtggtggcccagtatgcgaacgcgatggacaaaagctccgccgacggcgtgacgttgtagtacgcgatgcggccacgttccgccgcctcaaggtcgatccactctgggatgttgtccacctcggcgaagaactcgaccaactcgggagacgggtcggcaacggcgccaatgcccttattcagcgcggtctcgaagtcttcgcgggacttcttcgcgccgtcgcgcttaaacgcctcggcgagctttgcaccagtctcgtcggtttgccacatgtggtcgtcgagcagcttggtctgcaggctgccgtagccgtcccagctgtcggcgaccgtgtgccacctgtcgaagatgttgtggcgcagtgtcgaccacgacggggttttggtgcggcgctccggcgccggacgtagcggcatgccgtcgcggtagaagtagcggaaatcctcgtaagggttctccgacatcggcaggatttcgggctgcgagcccgtatcgcgctgcggttcggagtctattcgtgacgtcatcgtcatcctttcccgtcaagggggggcggggacacacggaaatgttttccagctaacattattggtattatgtgttgccggtcacttctcgcgtggtttgatggtaactgttacaccaacgcccggcaaccagttttgccgaccaatttcgcgaggaaacgagacatggacaacgccctgatccccctgacagtcgtggatgtggaccgcggcaccgcagacatcgccgtgatcactctgaccaccgccgatggcgcgccactgcccggttacgagccaggctgccacgctgatttccacctcaccgcaaagtccggtgaggagctcgtccgccagtactcactgttccccatgacgcccaacacctcggatgagggtcgctacggcatcacggtcaaagtcgagccggactcccgcggcgggtcggaagcgctctacaaccttgaggtgggcgacacgatcgatatctccacgccgcggaacaatttcgggctcgccgacaacgcgcagcactcgatcctcatcggcgccggcgtcggtatcgcaccgatttactctctggcccgcggactttcccgccaggccgcggatttctcggtgatttacttcgccagcagtgccgagcgcgccgtgctctcccacctgttcgacgagtactgcgcctacaaaacgcgcaacgtgttcgctaccggtgcccgcgagcagcagggacgcatcgtgcgcgaggcgctgcacccgctaacctccgtcgctggcgcaagccacctctacgtctgcggtccacaaggcttcatggaaacggtgcgcgaagtcgccagcgagtacctgccgtccgaaaacatccactgggaggcgtttcgcccggaggaaggaaagcttcagggcacggcgcttgccgacgcccccttcaccgtcaccttccgcgacgaaacgttcgccatccccgcagacaagagcgtcctcgacgtgttcgaagacgaggacttcccgatcatgtctcagtgcgcggaaggcacgtgcggcacctgcgtcatgcgggttgtcgacggcacgccagaccaccgcgacagcgtgttcaccgaggagcagcacgagtcgggcgcgttcgccacctgcgtgtcgcgcgcgctcagcgacaacctcacactcgagcgctggcgcaacgcgatctaacgcgccggctacaaaaggcgcaccatcgccacaccggcgagcaccatcgccaaccccacgatgcgcgccggggcaggcgcgccgcggcgcgctcccccgacccccatcgattccagcacctggccgcagatgatggttccggtgagggaaccgatcacggtggtgcctgtgccgagcatcggcgccagggtcgccccgccaaaaacgaagagcgcacccagcgctccaccgagccacatccaccacggcccaggctccacacccgtggccgccgcccggcgcggctgcggcagcacagcgacgagcaccgcaagcagaagcagccccaccgcgagcgaaatctggccggcctgcagcgggctgcccagcacgcggccgaggtggccgttgaccgcggtctgggtggacgaccccatccccatcaccacgccgaatgcgcggagcaaccactgcttggcgccgctcgcctttgcgggtcccgcgttgcggatgtccagcacgatggcgatcccggccaccacgatcgcggcgccgaaaaggcgcagcgctccaacggggacgcgcggcgaggcgaagaggccgaactggtcgataacaaggcccatcaacacttggccgaggatcggcaagatcacggtctggatcggtccgagctgcgggaagagcacgatgttgcccgcgatgaacatcacacccatgaacccgccgagccagatccaccacggttcggaagcggggacggcgaggttggggatgagcgtggacgtcgtcaagcaactcatgcccgatgcgacgaccaccgcaatgacaaacgagtaaaaggtcgccgcaagcggcgaccccacactcacccgcaaccgggtgttgatggctgtctggaccgggacaatcgccccgaccagcattgccaggatgacgagcattggctactcgtcggtcggaatcgtgtcgatcgtctccatcatcttcgccacgtagccggtgttgatgtcgcccgtgcggaacggctccgagttcagcagcatcgcctggaacgggccggtggtgacgacgccgtcgacggtcagctcatcgagtgcgcgaagggtgcggtcgatgcactcgtcgcgggtctcggcccagcagatcagcttgcccaccatcgagtcgtagaacggcgggatagtgtagccggtctcgatgtgggtgtccatgcggacaccgaacccgcccggcgcgcggtagtgctcgatcttgccggggcgcggagcgaagttctcgttcgggtcctcggcgttgatgcggcactcgatggcgtggccgcgaatcgtcacgtcctcctgggtcaggcgtagcttctggccggaggcgatgcgcagctgctcctgaatcaggtcgacgcccgtgatcatctcggtcaccgggtgctccacctggatacgggtgttcatctcgatgaagtagtacttgcgctcgatgttgtcgaacacgaactccacggtgccggcgttcttgtagcccacctccttgcagaggttgatcgcggcctcctgcaggcccgctcgcagctcctcgtcgatcgccggcgacggcgcctcctcgatgagcttctggttacggcgctgcgaggtgcagtcgcgctcgccgagcgcgatagcgttctccccatccgcgagcacctggatctcaatgtggcggatgtcggtgaggtagcgttcgatgtagaccgaggagtcgttgaacgcggactgcgcctcgttcatgatctcgttcaggtcgcgctcgagggtgtcctcactctccacgacgcgcatgccacgaccgccgccgccggcagcggccttgatcagcagcgggaaaccagtttccttggcaacagccagtgcctcgtcgaactcggtcaccacaccgtcggaaccggggacagttggcacacccgcgcgctgggcaatcttcttggcttcgatcttgtcgcccatgaggcggatgtgctcggacgacgggccaacaaagccgatgccctcgtcttcgaccatcttcacaaagtcagatttctccgagaggaagccgtagcccgggtggattgcgtcgaccttgaacgccatcgccgcggagatgatcagctccgggctgttgtagcttttcgcagcgtttgccgggccaatgcacaccgccttgtccgccagcttgacgggcagagagtcgcggtcgccctccgagtatgcgagcacgctcttgatcccgagctccttgcacgcccggatgattcgcagcgcgatctcgccgcggttagcgatgagcacgctgtccagcagctcttgttcagccatgggtactccttttggtcaggcttcgaaaaaggcttagttcggctcgatgaccatgaggggctggccgtgctcgaccgcatcctcgttctccacgaggatttccttcacggtgccggcgaccttggcctcgatgttgttcatgagcttcataacctcgacgatgcagagcacctggcccacctcgacggtgtcgccgacattgacgaaggcgggtgcgcccggcttcggggcggcgtagaaggtgccgaccatcggcgccttgacctcgacaccgttgccgctagccgccggtgcggccggcttttcctcagccggagccggagcgggagcctcagcttgcggcgcctctgtagccggtgccggagcaggagcttcctcggtagcgggagccggtgccggagcggccggcgcggccggagcagcctccggagccggagctgccggtgccggtgcggccttcaggtggtccagaccgcccggggtcttcgacatggcgagttcgatgtcgccgaacttgatgctcagctcctcgatgtccttggactggttgacccagtcgaggaggttcttcagctcgttgaagttggtggtgtcagacattgctacttctctcctttggtgaggttgacctcgaggtcgtcggtcttgaggtggatttggccggtggtggtgtcgtacagcttctgcacaaggccggtcagcgagccgcccggcacgccttcgccttggcccgcgcggccctcggcgacaaagcgcttcatctcgtcgacgttgttgcccggaatgttcgcgcgcagcaaaagcgtgtcaatatcgtcgtcggggtactgctccttcagcgccggcagcgccggcttgagctcggggcgctcttccttaatctccgaggaaccgttggcgataatcttctccagcacctccgggtcgatcggggcaagcggctcgccgtagtagccgagcgcgtacttcttgatctcgttcggcaccacggagtagcgctcgccggagatgacgttcatcacggcctgcgtgcccacaaactgggcaaacggggtgatcatgatcgggtacgcaagctcttcgcgcacacgagccgtctcgtacagcaagtcgtcgaagcggtcggacaggcccgcggttgcgagctgggactcgaagttggtgagcatgccgccaggcagctggtgcatgtagtggacgccgtcgtatgcgcgaggcttgccaacgggcttctgctcccggtcggcgatctgctggatcttcttgctcgccgcgtccacccgctcgtcatcgatgttgacggtgtagcccagcgcacgcaggtcgcgcgccagagcctgggtcgctggctggccctggccgttcgcgagcggagcgatggaggtatggatcgaatccacaccgagctcggcgccgtagatgtaggtcagcgggctcaggccggtcagggagtgggtgtggacctcgagcggcagctcatcgccgatcgcgctgcgaattgccgggatcagcgtcttcatgcggtccggggtgagcaggccaccggcgtccttgagcatgatgcggtcaacgtcggtgcggtcaaccagctccttcgccttgtcaatgtagagctggtcggtgtgcacggggctcaagcagtacgacaggcagccgtaggtttcggcgccgagttccttcgccaggatcagcgtgtcggcgatgttgtcgatgtcgttgagaccatcgaacgcgccaatgacacggaagccgttctcgtagagccgctccacccaggtgtgcagcacgtcatccggcaggaagtcgaaggacgcgaggttgcgggaacggatcatcgcccggaacttggtatccggcgccgcctggtgcaccaggcgtacgcgctcccacgggtcctcgcgtaggtagcggaccggaacgtcgaactcgatcggggcgacgaggtcgacgtgctcgaagccggcgtttgtcacgtcgtcgagcaggtcgaggatgtgctcggtgcgcatgcgcgttgcccagatggactggtgcgcgtcacgcagcgtggtgtcgatgatcttgatctcccgctcgctatccgcaggtcgtccacctgcggcgagaatttcagcgagggtttcagtgctcagttcctcaggacttagagcagccatagttacctccttatacaacgcttgacgcggtgcaagcgccgagcagactgtccgactcgacatcgcctacgaccgttggcccaaatgtaatcgcagacccattgcgcgggggagcgaattcacgtcacaaaaccgccgtgaatgtgttctacgtcgtagccggcctatcacttgcccccaaattggggtgcgcagggtgcacggccgttcgttcagcgaacgctttgacgtcaaaacgccagcaacttccgcaaccggaagccaatatccggtgagttaactaacttcacctcatgaaatgtgatcggcgttatagttttcgctcaacatccccaacacgtctaaaggaggaacccgtgacccaagcagcagtaccgccaccagccccatctcggcgccagatgggtagcacccacatcgaggcggaacgccccgcagaccgcaaatcgctcggcgccagcctgatcggccagcttctggagtggtttgagtggagctcctacgccgtctttgccccatttatcgccaaggccttctttgacaagtcggaccccacctcggcgttgctggcaacctttggcgtgttcgcgatcggcttcctcgtccgcccgctcggcggcatcgtctttggccgcatcgctgaccgcgttggccgcaagaacgtcctgatgatcaccatcatcatcatggcgctgtccgccgtggtcatcggcattatgccgacctatgagcagatcggtatctgggcctcagtcatgctgctggtcatccgcgtcctgcaaggcttcgcgcacggcggtgagtccgccaccgcgaacagctacatcccggagatcgcacccgccgcgcaccgcggcaagtggggctccatggtctacatgtccatcttcggtggctccgtcatcgcgttcaccctcggcggcatcatctcgctggtgctgacggacgatcagatcgcagcgtggggctggcgcatcccgttctggctcggtgctggcgcagctgtggtcgcgctctacctgcgccgccacatgaaggagtccgagcacttcgaggagttgcaggaaggcggcgcagccgactacgaccacctctccccgacccgcccgcagaccccgaagcgtccgaactgggtcaacatcctgctggtcatcggcatggtctcgggtgtgacgtcagcgcactacacctggacgtcctacgtctccacctacgcgatcacccacgagggcatgtccacccagggcgcttactgggtttccgtgttcgctcaggcctgcggcttgatcgccctgccgctgtggggttcgctgtctgaccgtatcggccgtaaaccggtcatgtacaccttcgccatttcgatcgcgctgctgcaaatcccgctcatgggcttcattgactcgcgcccgtggacgcttttggtctcgtccaccatcgccgtgatcgcggtcgcggccggcggcgcgctgctggcgccggttatggccgaggtcttccccacctcccagcgcacctcgagcatcggcttcgcctactcgctgtcggtcgctgtcttcggcggtaccgcaccgtacatcttccagtggttcacggcccacgacatgacccacatctcgggcatctacgtggtggtactgtgcatcctgaccctcatctccatgaagttcctcccggagacgaagggcatcgacctgcgcgacgcctagagtagacgcctagagaaccggcaacgccgagaacctagacatcagcccgctcgcaccgaatggtgtgggcgggctttattgtgtgtgacgggaacgcggataagcaggggctccttacgcctccgcctgggccatgcgccagcggatgccggcctccaagaatccgtcgatatcgccgtcgagcaccttctggggatcccccacctcgaactcggtgcgcaggtccttgaccatctggtacgggtgcagcacatacgagcgcatctggttgccccagctcgcgttgccgcctgcgccgagcgcgtccatctcggccttctcctcctggcgtttgcgctccagcaggcgggactgcagcacgttcagcgcgctcgctcggttttgaatctgagacttctcgttctggcaggtcaccacgatccctgtgggcaggtgggtaatccgcaccgccgagtccgtcgtgttgacgctctgaccgccgggcccggaagaacggtagacatcgacgcggatgtccgcatccgggatgtcgatgtggtcggtctgctccaccaccggcagcacctccacctcggcaaacgaggtctggcggcgcgcctggttgtcgaagggcgaaatgcgcacgaggcggtgcgcgccctgctccaccgacagctggccgtacatgtaatcgccgtggacgacgaaggttgcggacttaatccccgcctcctcggcgtaggagatgtcgtaaacgtcgaccttgtggccattcttctccgcccagcgcacgtacatgcgcatcagcatctcggcccagtcggccgcgtcgacgccgcccgcacctgagcggatgttgaccaccgcttcccgctcgtcgtactcgccggagagcatggtctgcacctcgagggaatcgatctgcgccgcgatatcagcaagctcgtcctcggcgatggaggtgtcaccctcctcctcggcgagctcgtacatcaccggcagatccgtcagcctttcgcgcagggaagtcacctttttcagcttcgcttgcacgttggacaggtcggaggtgacctgctgcgcgtgcgccgggtcgtcccacagactcgggtcgcccgcctgctgctccagttcgcggacgcgttcgcgcagctggcctaagtccatcacctgctcgatggtgccgagggtggcgtccaaatccgcgatgcgcgcttgagtgtccgattgcatagcccctaagtctagttggccgtcaaacagcgccggcgcggctcccctcccggcctcgccgtgtggggccaaccgctacacttgaaacttgcacctacacgggcgcccgcggcagcgggctgagatcgcgctgaggtttaccttgaacagccgcgcgagcaccgtcggaacctgtttggttagaaccagcgaaggaagtcaaaggagcggctatggccgacatttacgcgcaagaaatccaccccaagcacagctacgccccgattcgccaagacgggctcgaggtcccggagaccgcgatccagctggacgactcccccaccggcccgaacgagccggtgcacatttaccgcacgcgcggcccctacgccgagccggaggagggcttgcccgatctgcgcggcgagtggatccgcggccgcggcgacgtggaggagatccaggggcgcaagcgcaatttgcttgacgacggcacccgggctgccaagcgcggcgccgcgtccgaggagtggcgcggtgcaacgcgcccagtgctgcgcgcgaaggaaggcaaacgcgtcacccagatgcactacgcccgccagggcgtgatcaccgaggagatgcgcttcgtggcgctgcgcgagcactgcgaggccgagaaggtccgcgaggccgtggccagcgggcgcgcgatcatcccgaacaacatcaaccacccggagagcgagccgatgatcatcggcaacgcgtttttgaccaagatcaacgccaacattggcaactccgcggtcacctccaccattcgcgaggaggtggacaagctgcgctgggcgacccgctggggcgcggacaccgtgatggacctgtccaccggcaacgacatccacaccacccgcgagtggatcctgcgcaactcgccggtgccgatcggcactgtgccgatctaccaagcgctggagaaggtcaacggcgtggccgaggagctgacctgggagatcttccgcgacacagtcatcgagcaggcggagcagggcgtggactacatgaccgtccacgccggcgtgcgcctgccgttcgtgccgatgaccgccaaccgcgtcaccggcatcgtctcccgcggcggatcgatcatggccggctggtgcctcgcgcaccacaaggagagcttcctctacgagaacttcgaggagctgtgcgagatcttcgcgcagtacgacatcgctttttcgcttggcgacggcctacgtcccggctctgtcgccgacgcgaacgacgctgcccagttcgccgagctgaagactatcggtgagctgcgcaaggtcgcctgggaccacgacgtgcaggtgatgatcgagggtccgggccacgtgccgctgaacatgatccagatcaacaacgagcacgaggaagagtggtgcggcggcgcacccttctacacactcggcccgctggtcaccgacatcgcccccggctacgaccacatcacctccgccatcggcgccaccaacatcgccgccggcggcaccgcgatgctgtgctacgtcacgccgaaggaacacctcggcctgcccaataaggacgacgtgaagaccggcgtgatcacctacaagatcgcggcgcacgcagccgacgtggccaagggccacccgggcgcgcgcgagtgggacgacgcgatgagcaaggcccgcttcgagttccgctggcacgaccagttcgcgctgtcgctcgacccggacaccgcgcaggcctaccacgacgagacgctgccggcggagcccgcgaagacggcgcacttctgctccatgtgcgggccgaagttctgctccatgcgaatcagccaggacatccgcgacgagttcggcgacaagctggcggatctgggtatgcccaccgtcggcgccgaaactccggccccggaggcgaaggttggcgaggccgccatggcgcaggaattccgcgagcacggatcaaacgtttatcttccggaataatggcgtgagtgaacgctcacgtaactaccgccgaattcattgacacccaccgcgaggcggccgacgcgcagttggccgcctcgctggttgagcacgccggccagctcgcgctgacgatgcgcgcggccggcctcaccaccgacacaaagacctcggtctccgacgtggtgacggaggcggaccgcgccgccgagaccttcgtcgccgaggccctcgccgcgcttcgccccgacgacgggctcctgggcgaagagggcgccgcccacgcctccgccacgggccgcacgtgggtcattgaccccgtggacggcacctacaacttctcccagggctccgactacttctgctccgcgatcgcgctggcggagggcgacccggcagacggcaacgcgcttatcggcgcggtgcaccgcccggcgacgggcacaacgtgggtggcggacggcggggtggcgcggcgtgacggggtggcgctgggggtgttggagggggcgtcgataagcaaccaagccctggtcacctacctgcaccctgcgcacatgtcggacccggacatcctgaatacctggctgcgcgcggtgagcggcgcggcgacggtgcgcatgatgggcgccggcagcgtggacttggccaacatcgccagcgggcagatgggcggctggctgcagcactccgtggcagattgggattggctgcccggcaaggcgttgatcgaggccgcgggcggccgcgctgtgaaagtcgacgcgggcggagtgacttggtgcgttgccggaaacccgcaaatcgcctcggagctcgaagctagactgctaggccatgactaactacgcggacgacctcgcgctcgcgctcgagctgagcgacctggccgacacgattaccctctcccgctttgaggccgcggacttggccatcgaatcgaagccagacatgacgcctgtctccgacgcggacctggctgtggagcgggcgctgcgcgagcggctggcgcaatctcgccccgcagacgcggtgctcggcgaggagttcggcggcgacgtcaccttctccggccgccagtgggtcatcgacccgatcgacggcacgaagaacttcgtccggggtgtgccggtgtgggcgacgctgatcgcgctgcttgtcgacggccaccccaccgtcggtgccgtctccgccccagcgctcgcccgccgctggtgggcgtctgaaggcgcgggcgcgtggcgcacgttcggcggcaaggacgtgaagcggctgcaggtctcgcgagtgtccgacatcgcagacgcgtcggtgtcgatgtcctcgcttgagggctggcacgcccgggatttgcgggagaacttcatcgggatgacagatgagacctggcgcctgcgcggtttcggcgacttcttctcctactgtctcgtcgccgagggagcggtcgacatcgcagctgagccggaggtgtcgctgtgggatctcgcccccttatcagtcctggtcaccgaggccggcgggcggtttacctcacttgccggcgaggacggcccgcacggcggggacgcagtggcgacgaacgggctgctgcacgacgcggtgctggaccggctgcgttaacgcccgccggcgttcgtgcctttcggcgtcatggcaggcggaagtcgcccggcacctgcgccagcaccgcgtcggcgcgcgccgagccggtcggggcgtgcaccgggccctgcagcggcgtgtggcaggcaagcgcgaacggcggcgggaacatgccgccgttgaccagccccacaagccggtcgcccacaaagagcggcgcgccggagtcgccctgcatcgcgcacacctggttgacgttcatcgcctggtagtcgtaccaggtgatgccgcaggtcaccccggaggcgacacccttcttgcacacggtggcgccgggggccagcggcgccgatcccaggttgttgatggtcacgccgtcataggtgcgcgtgacctcggtgttcggcgcgagcgcgattaccgcgtagtccaagttgcggtcgacgtgggtgacgcggccggtctggcccaaagactgcgcgtccgcgtttaccaccgggtcgcccaccttggcgcagtgcccagcggtaatggcgatcttgcggccggtgttgtcgtagcccgccaccgcgatagtgcaaatgagctggtcctggcccgccccgacgtagaccggggtgccggggccgtagagtgcgttgccgcgttctacggcctgctgggcttcggcggggatgcggggggcgtcgtgaagcgagcccggaacgcggcgcagcaccttgtccgcaaacggcttgccggccagcgtcttcgccacggcgtccgtgcgccaaacgtagttcaggtccttggcggtgagctcctgcgccgcagccgttggggaacccgcggcacccgccacagcgatcgcgcacgccgcaaccgcggcagctacctggcgaaggaaacgacggcccatcacaaccccttttggtatctcgagcaacatagacaccatacgtcacacgcgggctaggctaaaccccgtgacacaccccgagttcaacactgagttcaagaccctcgacgacatgaccgcgcgcgaggcctacgagttgttcaagctccgagtcgacgtgttcgtggccgagcaggactgcccgttcaacgaacttgacgaggtggacgcggcaagcgacacgttccacatcctcgcccgcgacgcgtcgggcaggctggccggctgcgcccgcgtttttcccgaagtacgcgacggtgttccccacgcccgcttcggccgctttgtggtcgcaccgtatgcccgcggcaccggcgttgggcccgaaatcgtccgtgcgggccttgagttcacccgccggtggccgggcgacctggtcatcgaagcgcagaccgggctcgtcggctactacaaccgcttcggtttggtcgaggagggagaagagttcctcgacgggtcgatcccccacgtgctgatgcggaagcggcggagctagcggcgggggcggaacagcgcgctagcggcagacgacgtcacggcggagccgaccagcaccagcacggtgtagagcatcccagtcacgccgaccatctgcagcagccagccgaagaacagcgcgccgatgacggcgcctgcaatcgcaacaacccaacgcatgctcgccacgctaccagcacgctgctaaagtcagctggcgttgaaggggagtagctcaccaacggcgacttcgacacactggcgcgaccccgcgcccggagcgccggcccagcaccgcacttcgggcgagcgagaccttcggttcgtattatcgacgcaccgaaaggaaaccccgtgccgaacacaactgcgttaaacacaaccgcccccggcaacccgcgcgaagagcagcagctcctcgagcgattcatgaagatctcgctcgcggcctccatcttcgtcatcgccctgaagatctacgccgcgttcgttaccggctccgtgggttttttctccgacgcgctggaatcgctggccaacgtcgcggcggcgggcgtcggcctgtgggcgttgaaactctccgctaagcccgcagacgacaaccacaacttcggccacgccaaggccgagtacttcgctgcccaggtcgaaggctcgctcatcttggtcgcctcggtggccatcatcgtcacctccgtgcagcgcatcatcaccccggaaccggtcgagcagctcggcatcggcctgctgttttcgatcttcgccaccgttatcaacctcggcgtgggcgtgatgctggtacgcgccggccgcgcccaccgctcgagcacgctggaagccgacggcaagcacttgcttaccgacgtgtggaccaccgtcggcgtcatcgtcggcatggcgctggtctgggtcaccggctggcagattctggacccgatcgtggccatcctggtgggcctgaacatcctctacaccggctacaagctgctgcgcgaggccatcgaggggctgttgtcggagacgctgccggcgcaagaggtcgccgaaacggaggccttcctcgaccgctacgcaaacgacaacggcgtggcgttcacctcccttcgcaccaccgcgttcggccgccaacgcctgatcaacgtggtcatgcaagtgcccggcgagtggagcgtcgaccacgcccacacgcacgccgaccgcatcgaggaggggctcgccgccacgcttggcggggcggaaaccatcgtccacatcgagccgctcggggtggtcaccctcaccggtcccatcgaggtctagcaacggaagtcctgccactcagtaggctcgggtgcatggctgataagcatccagagaacacccccggcggcccgagcgtgaaagacggcgagctctacgaaaagctgcgcgaggaaggcaactcgaagtcgaaggctgcggcgatcgccaacgccgcggccagtgagggccggtcgaaggtgggcaagcgcggcggcgaatccggctcctacgaggactggaccaaaggcgagctgtacgagcgcgcccaggagctcgagatcgagggccgctcaaccatgagcaaggacgagctgattgaggcgctgcgtgagcactaacctggacctgcgctgctacttcgttaccgggcaaggccctgacgtggtcgagcgcgcccgccaggcggcactcggcggcgccggggttatccaggtgcgctccaagccgatctccgcgcgcgagctgtactcactcgggctcgcagtggtttccgcggtgcgtgaggtaagcccgacgacgcatgtgcttatcgacgaccgcgtcgacatcgccctcgccctccaacccgccggtatcagcggtgtccacctcggccaagacgacctcgacccgcggatcgcccgcgagctcctgggacctgatgccgtgatcgggctaaccaccggcaccgcggaactcgtgcaggccgccaacgcctacgcggacgtgctggactacatcggctgcgggccgttccgcgacaccccgacaaagaactccgggcgcatgcccatcgggctggacggctaccccgcgcttgtcgcagcgtccgatctgccgatggtggcgatcggggacgtcaccgccgacgacgcatgcgacctcgcccgcgccggcgtggacggcgtagccatcgtgcgcggcatcatgcacgccgacaacccgcgttcctactgtgagcaagtcgtcgctgaggtggatcggggccgcgccaaccggggcgtacggtgaaacgcatgagtcacttacgcgtcggcgttatcggcggcggcatcatcggcctgaccaccgccctcaccttggcggaccgcggccgttcagtcacggtctacgacccggcacccgccagcggcgcctcctggcatgccgggggcatgctcgcgccgacagcagaggtggtgtacaagcaggatccgctgtttcccctgatgaacgcggccgctgcctggtacccggagctgatcgagctggtggccaagtacaccgactcccccaccggctaccgcaccgacggcaccttagtggttgcgcgcgaccgcgccgacaacacccacttggaggagctcgccgcctaccagcatctccacggcatggaggtcgaccggctgcccacccgccaagcccgagcactcgagccggcgctgtctcccgcgctggcgggagcggtagagatcaccggtgaccaccaagtgcagccgcgcctgttcacccgcgcgctgatcaaggcgtgcgaagctgccggtgtggcattcgaccagacccgcgtcaccaacaccaacgacattgacgcagaccaagtggtcgtcgccgcaggccttggcgcagcaggtatcgcaggctggttcgagggcgttaacccgctggatcttcggcccgtctacggcgacatcatccacctgcgcgtcccggaccaccagtaccccctgcttaacagggtggtgcgcgggttcgtggaggaccgccccgtctacctcatcccccgcgaggaccgcacactgaccatcggcgctaccacccgggaggacgggcgcgccgaaccgcaggctcaaggtgtttaccagctactgcgcgacgccatcgaggtttgcccggcaatcgaggagtgcgacttcctcgaggccgacgcaggtgcgcgccccggctcccccgacgacctgccgtatctgggccgagtctccgagcgcgtgactgtgtccacggggtatttccgccacggcatcctgctcgcgggcatggcagcgcgctgcggcgcggatctggtggaacaaaccaccccgccgatatcgttggaagcctgcgacccttggcgccataggaggtaacaagatgaacatcacagttaacgatgagccacgcgtcaccgacgccgcgacggtcgaggccctcgtcctcgagaccctcggcgaagtgccggaggccggggttgcggtcgcactcggtggagacgtcgtgccccgctcggcgtggggtgagcagcagcttgccgacggcgccgtggtcgacatcctcaccgcagtccagggaggttaacgccatgctcgagatcggcggaaagacctttaactcccacctgatcatgggcaccggcggttccagctcccaggacatgctggaaaaagcgctggttgcctcggggacggagctgacgacggtggcgatgcgtcgtcacgcacaagcccccgcaaccggcgagagcgtgttcgacttgctcaaccgcctcggcatcgacccgttgcccaacaccgcggggtgccgcacggcgcgcgacgccgtgatcaccgcgaagctcgcgcgcgaggcgctcggcacgaactgggtgaaactggaggtcatcgcggacgaccgcacgctgttgcccgacatcgtcgaaaccatcgacgcgtgcgaactgctgatcgccgaaggcttcacggtgctggcctacacctccgacgacccggtggccgccaaacgcctcgaggatctcggtgccgcggcggtcatgccgctgggctccccaatcggcaccgggctgggcatcttgaacccgcacaacatcgagctcatctgctcccgcgccgaggtacccgtgctgatcgatgccggcgtcggcaccgcatccgacgcggcgctcgcgatggaactcggctgctccggcgtcctgctggccagcgccgtgaaccgctgccaggacccggtggccatggcgcagtcgatgaagcacgctgtcgaggcgggtcgcctctcccggcaggctgggcgcatcccgaagcgcgagcacgccgttgcgtcttcctcgtttgagggccttgcgagctgggcggattccgtactataaacgggtgcatgaaacgcacagccttcctcgctgcggccgccaccaccgcactgtcctgcctcgccgcgcccgcagcacaggccgtcacacaggtctcgtcctccccgttcaacccgcgcggtgttgactggccggccgactacgccaagctgccggcgcaggcgcccgtggcaacgttctcgaacggcgcgggcaccgcgcgctgcggcgtgtacaacgtggacggccagtcgtttgtgaagtgcctatccaccgttgattcgatgccggggcacatgtgctcccagcgaggccaggtgaacgccatgctgctgggcactggcgacgcgtgggactgcgcgaacccgagcgatttcgcgggcgcgccgccgattggcccgctgcaggttcgccgcttcggcgacatcgtggtctacagcgacgctcgcaataacttcatcgtcggctacgccaacctcacccgtgcggtgcgcgtcggcgagatcaacgacatctatctcgatcgcggccacatccaggcgttcaactcgccgcttcgtgggtcctcgatcccggctggctcttcgttctaacccctttcgtcccgcactcgtgcgcgtgcgctatattcaaacaatatattgattgtttgaaagaaggtccccatgcgccgcatacttcccctacccctcgctgccgcactcctcttggcaggctgcgccgataccgctgacaccgccaacacctccaacaccgcggcgtcgggggcaaccatcgacaactgtggcatcgaaatctcggtcgagccgccggtggagcgcgctgtcgctctcgagcagggctcgtcagacacgttgctgatgctcggcgctggcgaccagattgcgggcgtgggccatcagaaggacaacccgccggacggctacgacaccccggagatcatcgcgccggcgattcccaccgccgagcagatccgcgcggtggacgccgacttcgtctattcgccgttcgcgctggtctggacggcggattccgccggcacccgcgaggagtgggaccgcctcggtgtccgcacctaccagtccaacaccgagtgccacgattacggcgacaacacgggcaagtcatcgttcgacctgatcgaaaaggacatcaccgaactgggcgagatcttcggccgcgagtccgaggcgaccgacctgaaggcgaagctgcgcgacacggtcacaagcgccaaccaggcgccggacggcaccacctttgtcctcatctactccgctatcggcggtgccccctacgtcgctggcggcccgtcgatcgtgaccgagatgggcagcgcggtgaacatgaccaacgcgtttggggaggtcaaggaagagtggccgcaggtgtcgtgggaggccgtggctgaggccgacccggatgtgatcatcctggccgatctcccgatccgcggcgagccgggcgacacctggcaggaaaaggccgagacgctgaagactacgccgggcaccaagaacctcaaggcggtccaagacgagcgctacatcatcatcaacggcgtcaccacgtccccgtctgcgcgctcctaccagggcctgcagcaaatttcggacgccatcggcaacggaatcgcaggctagaagttgaagcgttccttagtgttcgggctgctctcgcttgtggccctagcgctcgccattgtcatctcgctgcccctgggctccagcggcatttcgctccgggatctggataatctctcgcccctgcagcgctccatcatcaccgagctgcgcctgccccgcgtgctgatggccgcgtgcgtgggcgccatcttggccgtgtgcggtgttgccatgcaggcgatcacccacaacgatctcgccgagccctacctgctcggtatctcctccggcgcgtccacgggcgcagtcatcgcgattatgttctccacgtggcagttcggcatcatcgtcggcgccgcaatcggcggcctggtttcgttcctgctcctgatgacgctgttgcgccacaccagagcggacgcgacccgcgtcgtgctcacaggtgtgcttgtcggctacctctttcaatcaatcacctcgctcgtggtcaccgcgtcgggcaacgcggaatcaacccgcggcatcatgttctggctgctgggggtgctctccgccgcgcggtggggaacgctcgtcgtggtcgcaatcgccggagcaatcggtatcgccatcttgtgggcgctttcgcgccacctcgatgcgctgacgcttggcgacgccaccgcccacaccatgggcgtaccagtggtcgccgtccgctacaccgtcctggtcgtggtctcacttctcaccgcagcgacggtggcatcggtcggcgccatcggcttcgtcggcctgatcgtgccacacgccgttcgtatggtcatcggtccgctgcacaagcgactgatcccgatctcggccattgtcggcgcactcttcctcgtcatcgcggacgccattgctcgcgtcgccttcgcaccgcaggaactgcccgtcggtgtcatcacggcgctgatcggtgtgccagtcttcttcgtcatcttgaaaaggatcgcgcgatgatcgaaatcgacgtgtctaccaaggtccgcgggttcgaactccatgtcgacaccacactcccctcttccggcatcgtcggcatcgtcggccccaacggctccggtaaatcgacgctgcttcgttccatggcgggggtccacgatttcaccgggagcattcttttcgacggcacgtcgcttacctccctcccccgcaaacaacgcgtgcgcacgctcgcttacgtcgcgcagagccacggcacgctcccggacctcacggtgcgcgaactggtggagctgggacagaccgcgggccacgggatcttctggaacgagtctcacgctgatgccgatgtgatcgaggaagccctcatccactccgacctcgtcgagcttgctgaccggccgttgcggaccctttccggcggccaagtgcagcgggcgatgacggcgcgtgcactcgcgcaggactccgagtatctgctactggacgagccgacgaaccacctcgacctacaccaccagtaccgcctgatggacatgctcgagcatgtggtgaccgaccacggcaccaccgtcattgtcgcgctgcacgatttagcgctagccgcacggtactgcacgacggtgcttgtgcttgacgacggccacgtagcagcactcggcgccccctcagaggagcttacgccagcgctgctgcgcgccaccttcggcgtggacgcaacgctgtcagccgtctctggtgagccttccttggtggtgcatggcccagtcacggcacgctaaggtagtcggctatgggtgatcacgagagctgggcggcagtgttcaagacgttgggcgataccacccggctttcgctcctcgacgcaatccacgacgcgggtgataaccagctcaccgtgacagacctggcggagaccaccggcacgcgcgtcgcaaccgcatcggccgcgcttcgagcgatggagaagatgggcaccgtcacgtccgtgcgagaaggccgcactatcttttacggcatcgcggacgagcggatccacggactgttgcactgggtagccgcctacaacgagtaggccggcataaggacgacgaagaccgcaacctcggtacccgaggctgcggtctttggcttgtgagctcctagtactggcgcaggtgcagcttgccctggccacgcaacgtggagcgcgcgatgttcgccgcggtttgcaccgcttccatcaggtgctcggtgcgggtacccactgcgcgcaggacaaagcccggaacgtcgcaggcggtgacggaggcctcgatctggtcgatctcagccagcgccgcgcgaacgttctcaatcaggtcctcgtcaatcttcgggtcgaagcacaacgcggtagcgaagtgcgtgttcgaccccaaaaacgtcggcgagtgcaaggtctcggtgtcgcgggtcggcatgatgcgcatgttgtccaccaacgcgagctttccgccaacgcgaacctctgagcgcaggtgcgcctgatgatagcggaactgactaccgtccggcgaccaccccggggtcacaatgtccgacaggaacgcgctcgcctccgggtgaagatccaccgtcatgtgctggcggaagtcggcgtcccggtacaggatgagctgatcgggaacgtactcgaggacggaacccgcgcccaccttgaaggcgatgttctgagagacgaacgactcaggcgtgcgatacaccttggtcgcggactggtccgtgaacaggatcgacgcaccgtcggcgacgtccaccgcgatacggtacgagtcgccaccgacgtagccgccgcccgggttcgcagtgatgtagtagacctgaccgctgtcatccaggtagtgcggacggatgatctttagtgctccagcgtggtactggcgcgtcgcgaccgacttcccaccactgatggcaatccccagctcgagagtgccagtggcaggttgatcggcagcgtgcccaaaccgctctgggggaatcgaccacatactagccatcgatgtcctgcatgagcacatcgtggcggatccagttcaggacctcgtcaagaccctcgtcggtcttcaggttggtcagcacaaacggcttgtcgccgcggaactgcttggaatcgtcggccatcacctgcagatcggcaccaacgtgcggagcgaggtcggtcttgttgatcacgaacaggtcggacttgatcatgccctgaccggccttgcgcgggatcttctcaccctgggcgacgtcgatgatgtagatggagaagtccaccaactccggggagaaggtcgcggacaggttgtcgccgccggactcgacgaagacaagctccagatccgggtggcgagccaccaggtcctcgtaggcggcctcgttcatcgaggtgtcctcgcggatcgcggtgtgcgggcagccgccggtctcgacgccgacgatgcggtccttcggcaggatgccttcgcgggcgaggatcttcgcgtcctcggtggtgtaaatgtcgttggtgattgcggccatcgacacctcgccgtccagcgcgcgggtaatgcgctcgatcagcgcagtcttgcccgagccgacggggccgccaattccaaccttgatcgttgccatagtgaaattacttcctttcttttaagacatgaacatgcgcgaacgcatgtattggtgctgcatctgcgcgatttccaggcgcgggaaggagacaccgaggtctgccacgtcgtgggtcagcgtctcctcggcgaagcccgggaggtactcgtagacgctcacaagaatcctctgaccggcgtcctggccgagtgggatcgcgcggatcgcgttctgagtcatcgagttggccatctgcatcaggtaggcgcgcactgcggtgagctcgtcgacgccggccgctccgagcacgagacccgcggcaatgccggggttgccgtagtagcggcgttcacgcaggccctgttcgtactcttcgacgagtgaatccgcggcgtcgataatccgtgcaaccttcgccatgcgcttgcccatcgcctgcatcgaggctcgcagctcaaccggggtctgggtagcgtggcacagctcgtcgagaagcgtaagctcttccttcgcttgttcgagcggcaagttcgccgcctgcagacgaattgcaagtagcacggacagcgcctcgccgtacgtggcctggtgcaaatagccgatcagccacttcaggtagctgtccggatcgctgacttcgtcgcgctggatgaatgtctccatgcctgcggagtgggcaaacgcaccggtcggcagggccgagtcggtgatgtgccagacaaccaggctggcgcgcacatcagtgggtatgttctgcatgacggaaagccctcggcattacgtagtccccacggtggtagttcacgccgacgtggtccaggtggtgctccaccgtgtggtcgtagcgcacgaccatgacctcggcgccaaaatcgctgtcggcgccgaagaactgcgcctgcaggtggcggttacccagcgagtgagccaccttcagtgcctcttcgatcgaggccggctgaatcaccagcacgtcgagcggggccatcgatgccacgatgacaccctggtcggtctcggcgaggatgtcgccgtcctcgagttcgcgcacggacttgtccagcttcagcccaagctcggtgccgccctcggtggtgacgcgctggatccgcttcagccggctctcgttgtcgaataccacgcggtcggcgacgtgcgcgttagcgccaaggtcgcggacgttaccgcgaagttcagtaacaatcatgttcaactcctttgaaaaaacgaaagcggagtggccgaagcctctccgctcacgctgggtttctagttcagactagctggttttcgccacaaggtctaactagaacaggaagtagcgctgtgccatcggcagcacctctgccggctcagacgtcaccttcttgccgtcgacggtcagctcgtaggtctccggatcgacctcgatgttcggcgtagcgtcgttgtgcttcatgtccttcttggagatgttgcgcatgttcttcgcctcgacgtacttgcggccgatgttcagcgactccggaacgcccgcctcgaatgcggctgtggacaggaaggtcaccgaggtgcgggcagcagcgtggccgtaggcaccaaacatgtcgcgcatggtgcgcggctgcggggtcgggatcgaagcgttggagtcacccatcacggagcgaacaatgaagccgcccttgagcacggtgttcggcttgacaccaaagtacgccggctcccagataaccaggtcggcaatcttgccttcctcgacggaaccaactgcgtgggagacaccagcggcgattgccgggttgatggtgtacttcgccacgtagcgcttgatgcggttgttgtcgttgccctcggagtcgccctcgagcggaccgaactgctccttcatgcggtgagcaacctgccaggtgcgcaggacgacctcaccgacacggcccatggcctgggagtcagaggaggtaatcgacatggcacccatgtcgtgcagcacgtcctcagcagcgatggtctcgcggcggatgcgggagtcagcgaatgcgacgtcctccggcaggtccgggttgaggtggtggcacaccatgatcatgtcaaggtgctcatccagcgtattcaccgtgtacggcagggtcgggttggtcgacgccggcaacacgttgctcagacttgcagccttcacaatgtccggagcgtggccaccgccggcgccctcggtgtggaaggtgtggataacgcggtcgccgattgcctcgatggtgttgtccacgaagccgccctcgttcagggtatcggtgtggatcgcgacctggatgtccatctcgtccgccacggagagcgcggtgtcgatggagttggcggttgcgccccagtcctcgtggatcttcaggccaatcgcaccagcacggatctgctcacgcagcgggttggcgtcggacgcgtggcccttgcccaggaagccaacgttgaccgggaagtcgcgggtggcctggatcatgcgcgtgatgtttgctgcaccagcggtaacggtggtcgcgttggtggactcggccgggccaacgccgccaccgatcatggtggtggtgccgttgtcgagcgcgacgcgggcctgttccggggaaatgaagtggatgtgggtatcgagcgcaccagcggtgacgatcttgccctcaccagagataacctcggtgctgacaccgatgacgatgtcgatgtcgtcctggatgtccgggttaccggcggcaccgatcttgatgatcttgccgtccttgatagcgatgtcagcgacgtagatgccggtgtagtcgatgatcagcgggccggtgatgacaacatcgggaacctgctcgtcgcctacccagcggctgttctggcccatgccgtcgcggatgaccttgccgccaccgaaggtgacttcctcaccgtagtgggtcagggacttctcaacgcgcgccacaaggttggtatccgccaagcggacgccgtcaccggtagtcgggccgtagagctcggcgtactgtttacgctccatctcaaatgccatgattaaatacctttctctttggtgccttgtgtttagtcgaccgggccgttgaccttggagttgaagccgtgaacctcacggcgaccaccgaagtcgacgagctggacggtgcggctgtcgcccggctccaggcgcacagcggtgcctgccgggatgtcgagacgcttgccgtgagctgcctcgcggtcgaactcgagctcggagtttgcctcagcgaagtggaagtgggagccaacctggacggggcggtcgccgcggttcgtcacctcgagggtggttgcctcgcggccctcgttcatggtcagtggcccgttatcagaaatgaagtactcaccagggatcatggaaaactctcttttcttagcggatcgggttgtgaacggtgaccagtttggtgccgtcggggaaggttgcctctacctgtacgtcggagatcatctccgggacaccctccatgacgtcgtcgcggctgagcacctcgacaccctcgctcatcagctgcgcaacggtcttgccgtcgcgcgcaccctcgaggatgaagtcggagatcagagccacggcttctggatggttgagcttgaggccacgctcttgacggcgacgtgcgacgtctgcggcaaccacgatgagaagcttttcctgctcacgcttggtcagtttcatttttgctccttatatttcgacggccccagcaagctactgctcgccggggatcggtaactagttacagcttgttcgggttgttcggaacttcctccggcgagtggccaggagccagtccttccctttgtagctgatccgacagattggcgtcggggttctcctcgcctgacttcttcttcttgccaaacaggattgcgaacaaaccgttctggtatgccaccgttgcaagaatcatcagcacaccgatgatctgcagcagcgacgggatctcaccgaacagcggcgccgcgatgatcacggaggtcacaggcgacagcagcaggatgccggcggacaacgtcgggtcgagccagacggtgccgtactggacgaaggtccatgccagtgcctggccgaagattgccagcgagatcagggcgatccagttaccagcggtcagcgggtcgccgagcgtggtctccgggttgacggacggcagcacgccgtcgataagcacaccgttcttgaagtcgaagccgccgcgggcggagaaggtgtgagcgatgatcgtcggtgcaaccatctgcgcagcagcggtgtacatcatcggctggatgtagagatccttacgagccgaggtaccggccttgcgcgagaagtagaggtagaacgagtagcagataccggaggtcagaccgaaggcagtacccagggttgcggtcttgatgccgtagatggtctcaggaccggttgcctctgcggtctgctcgaacacgccaccggtcagcatcacgccgaccgccatgatcggaacaagcacgaggaagaccggcgggatcttgtacttgtcaaagatcgcggtcagcatcggcacgatgatcacctggaggttcagcagaatagctgcgacacccgcgccgatgtagaagatggagtagttccaacacgtaaagtcgacacccaggaagagaccggagatcacggagtacatgatgctcctcttagtcaggccttccttcttcttcatctcccaaataccgaacgggaggagaataaggaagccaagagacacacggaggaaggcctggctggccgggtccatgttggcagccttcaccaacagaggagttgaggcgaggaatgcggtaccaagagcaagcaccgccagagctttgccgtgagacaccggtttgaccggcggtggcgtccggacacccgccacactgtttactgatgatgttgtcatggggttcacagtagataacttgtgtagtgacaccaatacgaaacgcattttctgcattttttacactaggtcataatttatgcaccgcgtttcccgagctgatcccgcatgcgagcccaccgtatacaagtcacacttccctataacgggggtagcaatggcgtttatggtgcagaaacagtacagatgttatttttcatcgcattttggtgtgccctttaattgaaactccaaccatgtatattttaatcaagcactcagttgattttatgcaggggaagtagactgtgggccgtgaatgtatcgacgctacccacctccgagctcgcgcgcacagcccgacagctcaacttgcccggattcggcatcgaacagcaggaacgactccgaggcgcccacgtccttgtcatcggcgcaggcggcctcggatgccccgtgatgcaaacgctcgctgctaccggtgtcggcaccatcaccgtggtcgacgatgacgtcgtctcgctctccaacatccaccgccagattctcttcggcgcctccgacgtgggccgaaagaaggtcgaggttgcggggcagcggttacgcgagctgcagcccgacatcaccgcgcatgcggtagacggcaggcttacggaagacaacattgtcgagtcgctgcggggcattgacatgcttatcgacggctccgacaccttccaaaccaaattcctcgccgccgacgccgccgaaatcaccggtactcccctcgtgtggggctccgtcttgcgctaccgcggcgacgttgccctgtggtggtccggccccggcgcccccagcgacggagtgggtatgcgcgacctctaccccacccagccggacccggattctgttcccgactgcgccacagccggcgtcctcggcgtcaccacgagcgtcgtcggcggcctgatggccaccgaggtagtgaagttcctcaccggagtcggcgactcacacattggccgcctccacatgtacgacgcgctcaccgccaccgttcgacacttcaacgtcactcgtgatccaagtcgcgagctggtgcgggaactagggacctacgcaggagtctgcgcggtgccaggcgctagcaccgaagcggctgatagtgaagggcagcacctcatcgaccttcttgcgggcggcgacgccgtctccttggacgtgcgggaaccccacgagaagctgctcaaggacatcgcgcaccccggagcaaacctccccatgagcgagcttgaacgcaccgccgaagtgctcgatactctccccgctggcgacgtcgtggtctactgcgcctcagggaggcgttcagcccggttcgtcgaggagttcgccgacgccgccgaggcacgcggacttaccctttacaccctccccggcggtgcgaaccgctggggtactgacctgctctaacagctcgtggtgctacgacgctatggggctacgacccacgtgtggggttgcgttgctatgcaacaagctcctcttggcggcgcaccgtagcgcgccgcacgaaccacgcggccacgaacgagaacgcgagcgacaccaacacgcccagatttgcgtccgcccactgctcgcccactagcggtagcaggtagccctgccagttgttccaggcggcctcatccgcaaacgcgttgaccacgaggccccagccaagcacggaggcgaccgccatgatggtaatggaggcccaatccaccgagccgtagcggcccgacggggaaaagagcgcggcctcgtcgtagtcctgcgtgcgcgtaaagatgtccgcgatgaggatgccggcccagctggcgagcggtacgccaagggtgatgaggaaagactggaagggcccgaggaagtcttgggcgtaaaacaccacccagatcgtgccggcggtgaggatcacgccgtcgacagccgcggcgaccggccgagggatattgatgccgagggtgatgagcgtcagccccgaagagtaaatgcccagcaccgccccggagacaagcgccagcaccgcggcgatgaggaaaggcacgagcacccaggtgggcagtatggtagccagcgcgccaatggggtctgctgcgatcgcgtccgcgagcgccgcgtcagagccggcaagtagtaggccgaagatgatcagcaccaccggggcgatcgcgccgccgaaggtgttccagaagacgattgaacggtcaggcgtgtcccggcgctggtagcgcgaccagtccgcggcaatattgatccagcccaagccgaagcccgtcattaccatcactagcgcgccgatgaccgaaccggcagagccggcggggatggaacgcaccgcgttaaagtcgatgtgggggatggtgagcatggcatagagcgcggtgatggcgccggtaatccaggtgaggatcgactgaaggcgcatgatggtgtgatagcccagcacggacgcgccgacgattagcaccgccacgacgagggtggcaataacctgcgtcactgtccccggctcagccccgagctggcgaattactgtggtagtggccagcaccgccatgatggacagaaaagtctcccacccgattgaggtgagccaagagacgatcccgggcactttctgcccgttgacgccgaacgcggctcgggaaaggaccatggtgggagcagaaccacgcttgcccgccactgcgatcagaccgcacaggaagaacgaaaacgtcacgccgaacgcggtgaccagcgccgcctgccagaacgagatgccgaaccagaggatgaatgagccgtaggagataccgaacacggacacgtttgccgcgaaccatggccagaagaggtctgcgggcttcgcagtacgctctgcctctgggacgatgtcaatgccgagggtttccacaaccggcgagttcgtgcctttcacagggctaaccgtactggatgctggggacttgctgaaaataatatttgcccggcaccttcggccccaccaacacccccagcgtcgttattgaaccgaggcgaagaacgacttcatgatgaagtacgactccttcagccgatgggccgtctcgaaacggtcccacatgtcccaggtgttgcgcaccggcgtggtcgcctgctgcgccacgtcgtcgccgtcaccgccggcgaacacgaagcttagcccagtgttgtcgacgaacttgctttcgtttacggacttgtcatcccacaggtccgcggtcacctcgcgccggctcgggtcgcgaaaattcattagcaaccacgggacgcgcacctccagcttaaatttgccggaggaccaagcgtagcccgtcaacgaattgtagttatctgcctcaggatcgccgttgccctcccgcagcgcacctgcctcgtactcctcaaaggggaaccattcgcccgtttctgcgtttcgcatctgcttgttcaacacgtagggtgctgttgcaaacttcaggcggagagccgtgacgacccagtcttcatcctctgatgctcgctgcgggtcggcgttctcaggcagcctcgaacacccggctgacgatcaccgcatccgggttcggttgctcgtaggcaaacatcgcgccctggcctttccgtaatgagtgcatcgcttccatccctttcaacgtccggtacgccgaggtccggtttttgaacgcccccttcggtccgaggatccgtttcagccgcccatgatctccttcaatgacgttattgaggtatttcacctgccggtgttccacggtctgcgggcagattccctctgacttcaactcggcgattgccctggccagggagggtgctttatcggtgttgatcacccgcgggaacccggttatcgtgttcgacctcagggtcttggccaggaaacgcttcgctgcggcgacattacgctttggggacaggtaaaaatccagggtatgcccacccgcggtgatggcccgatagaggtagcaccactttcccccgacccggatataggtctcgtccacccgccaggaccgggcctgccaatccgggacttgtcggtaccaccgggtctgcttgtccagctcaggagcatatttctggacccagcggtagatggtgctgtgatcgaccggtacgccgcgtccggtcgtcatttcttccagatcgcggtagctgagcccgtagcggcagtaccaccggaccgcccacaggatgttttcacgggggaaatgacgaccggagaagatgcccatggctgtgattatttcacgcaggtcttcctgtcgcccgaactttgcaacagcacccttttggcggtccaggaggtgtgcccaattggattacaagtacctacacacttgatcggtgctgcacgtttcagggtccgggtgtgcggcgtcctgtctgaggtccgcgatagtgtcgcgcagcacggagagctgcgcgatctgctgctcgatctcagcgaggcgcacgtcaagcaggtcgcgcacgtgctcgcagggcgcctggccgccgtcgcggatgtcgaggatctggcggatctgggcgagggtcagcccggcggcctggccccggtggatgaacccgacccgacccacggcatcctcggcgtagtcccgatagccggaggccaatcgctcggccggagggagcagccccgactcctcgtagaaccgcagggtcttggtcgtggttccggttgcttccgcaagctgtccaatcctcatgttcgccgattccccttccaatggccaccacacttgaccttccattgtactggaaggttcacaatggttccataggaacttttgaaccacagggaagagacatctggaatgacaaacgaaaagttcgatctggcgattattggttccggcggcggagcgtttgcggccgcgatccgggccaccgggctgggcaagcgcgtcgtgatggtggagcgcggcaccgtgggcgggacatgcgtgaacacgggctgcgtcccgtcgaaggcgctcctggctgccgcggaggcccgccacgtggcgttggattcggcccgcttccctggggtggcggcctcggcgggcccggtggacatgccggccctgattcagggcaaggccgcgctggttgaaagcatgcgcacggagaagtacgtcgatctggccgcggactacgggtggacgatgatctcgggggacgcgtcgttcaccggaacccaggacgcaccgctgctccgggtgatctccccggatggtgcagtgagaacgatcgaggccgggcactacctcgtggccactggctccgcaccctacgtgccccccgttcccggactggccgaggccgggtacctgacctcgacgacggcgatggaactggacgaggtgcccgaatcaatgctgatcctgggcggaggctatgttgccctggagatggcacagcttttctcccggctgggctcccgggtgaccatgctggtccgttcccggttggcctcgcaggaggaaccggaggcatccaaggcgttggcgggggtgttcgccgacgaggggatccgggtggtccggcgggccatggccgactccgtggcctccggcccggacggggtctcggtgacggcaaacgtggccggggacgaggaggtgttccgcgcttcccacatcctcgtggcactgggccgccgcccggtgaccgagggactggaccttgacgccgtcggggtgaagaccggcgcatccggcgagatcgtggtcgattcccgcctggccacgtccaacccgcgggtttgggccgccggggacgcgaccggccatcgggagttcgtttacgtcgcagcggcccacggcgccctggccgtggacaatgcgttcaccgatgccctggccgaggtcgactaccggcacctgccccgtgtcaccttcaccagtcccgccatcggggcggtcgggatgacggaaaaggaagctgtcgccgccgggatcagctgcaagtgccgggtcctccccctggagtacgtgccgcgagccgtggtcaaccgcgacacccgcggcttcatcaaggttgtcgcggaccgcgacaccggacggatcctgggcctctccgcggtggccaaggacgccggggaaatcgccgccgccggcgtctacatcctcgaagcgggcatgaccaccgcgcaggtcgccgccgcctggagcccctacctgacgatgtccgagggcatcaggatcgccgccaaggccttcaacaccgacgtctccaagctctcctgctgcgcctgagctgcagcccccactgccgaagcaaaggaatgccatgaccgccactgaccaggccctcacctatctgttgtcccccgcgcgctccggaatagacccggaattgttcgtgccgctgctgcggctcctggccgagggcgagcccgtcacggtcgccgaactggccaccgccagtggccggagcgaagacacggtccggcagggactggccgccgtcccggacaccgagtacgacgacgagggccgcatcatcggcctggccctgacgatgcggcccaccccgcatcgcttcaccctggccggggaacagctctacacctggtgcgccctggacaccctcttcttcccggccctgatcgggaaggccgcaaccattgagtcgacctccccgggtagcgggaccctcatccgggtgatgacggacgcggacggcacggtgacctccgtgcagccggccaccgccgtcgtggccatcatcagccacccgggcacggggccggtgcggtcatcgttctgcaaccaggtccactacttcgcctcccgcgaggacgcccagccgtggttggattcccatcccgacggcgaagtcctggacatcgaggcggcacaccgggccggtgccgccatggccgccgccctcctcgccgcggccgccacgcgggcccccgcggcgcaggactcctgctgctgagctttaaaaggccatgacatgacccagcacccagaacagccagacaccggccatcaacccgtccggcagaccggtcgccccgggcgataccacacactggccgcaggaatcggcatagcagcggccatgatcctgtgctgcgcaggacccatcctcatcgccgccggagccctcggcgcgatcgccggattcttctcaaatcccctcgtgttactcgcggccgccacggtgctcctggccgggatcatcgccgtcaccaggcagcgaaaacgccgcaggaccgacgactgctgccctcccgcatcccccgagcaccaccgcaccgaccacggcaccgcctgagtccccatccccattcctggaaggaaccaccagacaccatgacatacccgagatcccgccgttctctgtccgttccccggcccaggcacctcgcctccgccctgtttctgacagcggtcatggcactgacaaccgcctgcgccagctcaccgagcggcccgtcggccgcgccaagcggttcgtcgcccgacgcggccggtgccgttgctgttacggtctccgacattgacggcactacccggaccatcccggacggtaagcccgcagcactgttcttcttctctgccggatgcggtgagtgtgtggaaggggccgattccctgaacaaggcctccacggccctgggaagctcggccgactacctcctggtggacgtggacccccgagaaccgaaggagaccatcaacggattccgcgattacatcaaggcccctgagctccctgccgtcatcgacaccgaggccacactgaccacccggtacaaggtcacctctataagcaccctggtggtggtcgacgcgaagggcgacgttaccttccgggccaccgacccgtctgcggaaaagatccaagaagaactcaccaaggccggtgcccaatgacagccctgcttgccctggccttcgccgctggaatgattgccccggtcaatccctgcggtttcgccctcctgcccgcctggatagcccagaccatcggggacgcccggacgcgcccgctcgcgctgcgtctggcccacgggctccgggccgggctcgcgctcagcctcggcttcgccgggaccctggcagccttcgggctgatcgtcagcgcgggcgccaggaccctgatcagcgcagcgccctggctgggaatggccaccggggtgatccttctcctgctaggcctggccatgctcaccggactcacaccacggctccgtctgccggcctgggccacgaaaccccgcacacaagaagccgcaggggcaggtcacaaaaccgggcgcatggtggccttcgggatcggatacgccgcagcatccctcggctgcaccctcggggtgctcctggccgtgatcgcccaagcccaggccgtcgccagctacgccgggctgctcgcggtcttcgccgcctacgccgcaggctcggccactgtcctgatgctcgtttcggcaggcacggccatcgccggggccgccctcgggcgaagaatcaccggcctggccaagcacagcaaccgcatcaccgccttcatcctcaccataaccggcgcctacctcagctggtattggtatcccgccgccaccggcggaaccgcacaggccaacagcctcgccgtatggtcagccgccgccagcgcctggatcagcgacaacagcaccctgatcgcagccctcgccgcagccgtggtgctcgcatcggcattggccgtcctcaaccggcgcaggagactgcgcatcagacagggaacgccgcccacaggcgagggccccgggcaaagcggggaacccgactgctgcacaccaactccggacaacaactcgaccgaggaccggccaggcacgatcccgtagctggccgaggactcccaaaaagcaagggggagagggaaccttgcccatcttctggcaaacgaggcgcccgcctatcaggacaggttggtacagcggcatcaggccggaagtcaattcgtgcagagggcttcgggcaatccgtcaggagccctctgtaccgcccccgcaatgacgggaacgtcagtgtggtggacttcggaaagccacagtgacacccactagttgtactcgaccgtgacgttggtggcactttcggtcttgtgaaatagctaggcctcctggcttagtggagctgtctagttcttcactgccaggaggcctctacgcccaacggtaacgcccgcttgaccacgcatgcgagagcgttgctggtggccaggcaagctcatccatatcgatgtgaagaaactcagccgcatccccgacagcggcggttggcgagtccacgaccgatccgcgaccggaagacccgatcgggttcgaccacgtccatgccgctgtcgatgaccacacccgactcgcttatatggcccactagcggtcgcggagcgtcctgaaaacctaaagttttatgagacacccggcaggaactggaatgtgagaccgtttcatggggcaattggcctcctccccgtctcactaaagcgtctcgccctaagttgtcgcagggtggtgctcggtaggggtttgtgaggcataatcgagacatgaggcttttggggtacaccccaagcgaacaatttgtgaatgacaaaacttcctgttcgctagggttagttccaagactaacggaacagaaccgtcactgcctctggagatcactgaacagttgggggcgatctcaggacaaaaggtgggctatgcccgggtgagttcgaaagatcagaaccttgatcgtcagattgaacaactcaaggcagagaaggtcttcacctattacacggataaggccagtggtggatcgcgtgagcgccctggacttgatgaagcaatgcgatatgtccgtgcaggagatcagcttgtcgtcacgtcgatggatcggtgcgcgcgttcactgacggatctgtacgccattgttgacgagctagtcagcaaaggagtgtcggtgaagttcctcaaggagggacagacctactcaaaagactccaccccgatcgccaagctgatgctagggctgttgggttttgttcagttgggtatggccgtgaaagagctggatcaacaccgtgaaatagttgaaaaaaataaccccgcaggtttccctgcggggtgtcgttgttagaacggtgcttcgtcgttgtcggcgtcagcgccagccagggcggcgttcgccgcctcgcctccgcgacgggctgcgcgcgcagcggactctttcttggagtcgatcagctgcacggtgtcgatacgggcgaccagcgggtagtgcttcacaccgtccttgtcggtgtagacgtcggttttcagcgagtagctcaccgcaacgcgatcgccggagccgacgcagccgaacacgccggggttcttagcgtcctggacgtagccggtcagctccacgatctcgctttccaccttgccggtggccttgttcttgaaggtgttgcgcgcatagacgctgagtttcaccgtcgcgccaccgtttgcgtgctcgaacagcttcggtgcgcgagctgcgttgccgacgatggtgccgttgttgaaggggttggacatgttggttctccttacctgagtgggtgtgaattgccgtgcaatttgggtacttaagcagctgctttgctgctgcggggtggttgcgctgtcgttacagcactgcccagggcagcggtgtgcctgccgcctctaggtcgcgcagttcttgcgctgcgcccggatcggcgtcctcgccgtcgatgccgtcggcgagctggtagagcagttccaggtcggtgtgggtgatgtcgcgcatcacgtgcctccttgttcggattgatggtcaatccgtctgttggagacagctctgctgtctaggggtcgctcccctacctcgttgaggtgtctgtcgtcgcaagccacggccgacgagaaaaagaaaccccattgcattgctgcaacggggtgtgtggtgctactcggcaaacaagatcgtgcgggtcttctcggcgccttcgcggacaagctcgaccatccgctcgccctggccgttatcggtcagcttcgccaccagcgacgggaagttctcgtctggcccgatctcggtggctcgctgcgcagccacgccagctagtcccggctggccggtggcgtgcgcgagcactgcgacagtggcggtgagctgcgcccgcatccccggccagctggtcgggacagcgcgcataacctgctctatgaacgcaaggcccgcctgcgggtcatcgagcagcgctgcgagcagcgtgtctcgcaagcgctttgtagtgaagcatttcagcgccgatcgaacagcgcgcgtgctcggctgggttattcctgccgccgcctgctcgtattcacgctgcagcacgtcggagaacatgggcgggatatacgccagcgcgtcttcgatgatgtcggcgtgctcggcagcgtcgatgccgtgatcggtgctgttcaaccgtgcttcgatgtcgtctttgctcggctccggcagctctccggtgtgctctagcatctgccgcagcgccgccgatgcggcgacctcgccgacaacgccgtggcgcggctcgtcgatgagcggatgctggtacacagaccaccacgcagccccggtgacgatctcaggcacctgcaccaccccgagcagcggcggtaggtgcactgccccgctggtgaggtacgtggccgtctcgtcgaagatcggctgtgcaatgtcgtcgctgatcatgtacgcgataacagcgtcgagttcgaggtggtggacccacgctgcgaaccgctcgcggctttcggtgagctttgcaacagcttcgtccaggtcgaaccgcgcgaccgggccgaggcggacggtgtcgacgccctcgtcgtcgacgaagaacgcgaggatcagcgagttgttcgggtagaacccgaggatgccggggaggttcgcgaggatctcgccgtgggatgcaagcgtgtgggaatgagtggacatggcagtgctcctttgcacgaatacggggtgtacgtgggcaatcccgtattcagtccggctctgccggtcgcgccctgccacggcaccaccgcacctgaagcgtgctgagcgtcgctagcgcagcctgatgctcgctcgctgggtgcgagcgctagcgacgcagcattgttagatccccgcgtcgccgctggttaagcgttacctttggcgcggttgtgagacttgcacagcagttcgcagttgctttcctcgaactgccggctcccgtggcgttccttcgttgctgccgtcctagcaatcactaagcaatgcaccgaaaacctgcgccgcgtcgttggagcgtcgcagttccgtttggtgcaggattttgaccctagtgcaccagctagtgcaccaaatggcgatccgatcacaaaatgaagaaggcccataccagcgtttccactggtaggggccttatcttagtagcgggggctggattcgaaccaacgacctctgggttatgagcccagcgagctaccgagctgctccaccccgcgccgggtgatattcaatttcacctgctgccttgatcggcaacggtgatcactatacgtaccaacgcagaagacgccaaatcccctggccagatggattactggcgcaggggatggtgggtggccaccaaggttttgacgcgaggcgttagttctgcaggccctggtagtcggccaccgccttgtccagtgcgtcgagtgctcggccatagtcctcaaacgagccgtcgcgggcgctctcgagctggcggagggcgtcgttaatgttgctcaatgcttcctcggcgttcgccgcgcccgggacacgagcaggtgcctcgtcggccgcaccgcccgtctcgtcgttgacgtccggcgacgtcggggacgccatgtccgcctcggtacgggtgccagcggactcctcgtccaccacgtcaatgtcctgggctgcagacgggttgatacccacctgggacaacgcctgcgagatcgtcggcgcgtaacccacctggccgcggtagaacaccagcacgcgcaaaagcttcgggaacgcggattcctggtccttgcgctgcgagtaaatcggctcgacgtagaggatctcgccgccaccaaccggcagcgtcaaaaggttaccgttcttcaggtcattggtgccctcccacagcgtccggtcgcgggcgacctggtccgaggacatcagcgcgtcctgcgcctgcttcgggccctgggtctgcgtcgtggtgggcagcacgcgaaccgtgatgcggccgtaggtctcagggtcagacgagaccgacatgtgcgccgacaggaactcgcggttcagaccgcggtacggcgtaatgagctggaacgaggcctcgccggtctccggatcggaggcgacgatgtagtacggaggctggtacagctcgcggcggtcttccggcgcagttgggtcgttcggcacggaccagaatgcgtcgttgttgaagaagacgcccgggtcatccacgtggtagcgggcgagcagctcacgctgcaccttgaacaggtcctccgggtagcgcaggtggtcgcgcagcgcgtcggagatctcgctctcaggattcaccgtgcccgggaagatgtccatccatgccttgagcaccgggtccgactcgtcgaaggcgtagagctccacggtgccgtcgtacgcgtccaccgtggccttcacggagttgcgaatgtagcccaggttgtcgttgatgatgcgctgggaagtgccgtccgggttgagggcgtcctgcgttgcgtcggtaagcgtggtgcgcgtggagtacggcagctgggacagcgtggtgtagccgtccacgatccacttcacacgaccgtcgataaccgccgggtacgtcttggagtccgtggtcagccacggcgcaaccttttcaacacgttcgcgtgggtcgcggtcgtagaggatcttggaatcaccgccgacacggtcggacagcagcaggttcagctcctggtagcgaatcgcgtacgcgatgcggttcagccagttgccaatgttcacgccgccctgaccggtgtaggtgtaggtggcggtgtcagtgtcgtactccaccgggccctggccgttgtcgccgacgatggcgtagtccagcccgtcggcggcagaagcgatcaccgggccgtagtaaatccgcggctcgtcgacacggatacccagctcctcagcctggtcgctctcgcgcgcgatggcgttggtctgcaggtcggagacggtgaagatgggcaggccgccgcgggtcgagccggcgtcctgcgccgcggcgtcgaccgtgttggcctgggccgcgatgaagccgttgccgtgggtgtacacggtgtggcggttgatccagtcggcctggttctccgacaacgagttcgggtttagctcgcgggcggcaacaacgaagtcgcgcatctcgccgtcgaactcgtagcggtccatcgccagctgctcggggaagccgtagaagttgcgcagctgctgattctgggtgaacgtcggggaaatgatgtctgggtccaaaaggcggatgttggaaatggttgcctcgtcctgcgcaacgtcggcgttcgacgtcgccgattggccccagttctcctcgtaggcgaccttgtcgtccgtcaagccgtaggcgaagcgggtggcctcaatgttgcggccgatgtagtcgtactccttcgcctgccggttcggcttcacactgaactgctccagcagggccggccacacgttgccgaccacgaccgacgacactagcatcagcaccgtcgccagcaccgggatacgcagatccttgtacaccacggaggcaaagaaggcgatagcgacgaacaccgcgatcaccgtcaggatgatcttggccggcagcatcgcgttgatcgaggtgtaggacgcaccggtgaaaatgtcgttgcgcgcgtagagcagctggtagcgctccagccagtaggacacggctttgagtagcatccacagaccggctgtgacggcgagctggatgcgagcggatttcgacactgaacccttggcacccgtcatgcggttgccgacgcggatcccgccgaggaggtagtgggccaccaaaccgatcagaaacgccgcgaggagcagcagcgagagcaactcgacgatcgctgaaagcgcggggaggctgaacgcgaagaacccgaggtcgcggccgaactgcgggtcgttaacaccgaagttcgggccgttgaaccacatcaggaacgtgcgccagagcccctgccctgccagaccgctcaagatcgcgacaacgagcgggacccacaccagcagcgagcgcaccccctgctcgagctgggcgcgcgcacgggcgtccggcgcgaacgggtccatctcgtttttctgcctgccctgccaggcgaggcgcgccgcgaggtaggccaccgcgccgccgatagccccgaagatgaggaagagcagcaaccgggtcaaaatgactttgttgaacacgctgcggtagtcgagctcgccgaaccagaggaagtcggtgtacaaaccgaccagcatcggcaacaagaataagatgacgccgaggacaccaatggtggtccaaagccccttattcgacttccttgcgtttggacgtggcggcgtcacacgggtagccaatccttctccttttcgcgatggcttaggtcagtaggcttctagcctaaagagttcaacgattgaaaccgaagaagggttcccgcaatgcagcagcaagcgctcaacaaagcgatgatggaagccatcgagttcgtccacgccgaaggctgggacgccccgcccacgttgttcggcctcgtccccaccgcgcttctagtcgatcagctcgaagagctcgaacgcgaggacgactcgccgttgaccttggtcgtgcaggagcttccggcgcacatccgccccggttcagaggagctcgcggattacgtcgcccgggtagcgtggccgcgcgaagtggagggcgtgatcctcgcccaggagatcttgttccgcgacacctccgcagacacggacgagccgcgcccagcgcggttgttctccggagcactgcgtgacgacgacacgtttcaaacccttctgcaacttcgccccaccgacgaagagctagaagagggcgggttgttcgcgcaggaccggatcgagttgcgcggcggccccgacgtcgcgccgacggtgatcgccgcactgcagtacagcctgtcccaagatccggaagacctgctttagcgttttgcctgctttaggatgatggatgtgaaatttcctactcgcacctcctcggcggccggtgcggtcgcagctgttgctctggcaggcgccctgaccgcctgcggcgacgcggacacggattcgacggcggtggaggaaacggtggcgtcggcaagcacgagccccgaaacctcaagctccgccgcaacccccaccaccacctcgagcgcaaccaccagcaccgcggcaacgacaacgacgcgcagcaccacccccgccgcaccaacaagcaagaccgcggaaggcgcagccctggtcgaaacggtcgccgagcaattctccacccttgcacccgcttccctgttcgcgcagctcgacgagtgctcccaggccggcatcgccggatcttacaactgcagcggcaaagaagttggccagttccagttctttgactccgagtcgaaggctgcctcgaccacccagttgctcacggagctgcgctcctcccgcgtggtcgaagacaccggcaaccgggtcgtgggttggtctgtgctggcgaactcggcgatcatcaccgtggtggacaacgaagccggccaggtgatgcagcaactgatctccaccgacgagacagacccgcgcacccgcatctacgagcttggcctggcggaccaggtggaagaagtctccacgcccggcgggcacacaaccagctcggggacgacctcgccggcagcgacgtcctccacatcggaggccgccgagcccgccgctgagacgacccagcactaagccgcggctagttcgcgcaggaagtcactggtcggccagcggcaaaatcgtccatcgcgcgaacagcgtcgtccaagtcggcgaccttcgccaccgtcatatcacccgcgttcgccttcgctgcttccttgcagttgccctcgggcgctaggaagagctccactcccccgtcccgcgcacctgcgatcttgtgggtgatcccgccgatcgggccgacctggccagattcgtcgatagtacccgtgccagcgacaacgcgcccgtgcgtgagctctccgggcgagagcttgtctatcaccgcgagcgcgaaaatcatgccagcgctcgggcctccgacgtcgttgaggttgtaggcgacagagaccccgtcgccgggcgtggacgtcatcaaaattccgagcattgctgtgtttttgtccgcctccgaggcgccgagggtaacagttactggaacctcgctgccgccgcgggagaccgcgatctcgagcgagtcgcccggctgcttggagcggacaatctcctgcacctcaccgggcttcgtaacgtccttcccgtcgacgcgcgtgattgcgtcctcaggttgtaggtgcccgtcagcggcgctgccctccaccacgtcgtgaacgatgaccactgtgggctttcccaagtaatgcatcgccgcgaccgtggccgatgcctccgaggcgacaaacgcagcctcgttgtactcgcgcagctcctcttgcgtgaggtcgggcggcaacacctggtcgacagggacgatcgtgtcgtcggtggtgatccaccggctcagcgcctgcgtcagcgtcatgttggtgcgaaccgataccgtcgtcatgttcagcgtgcccgaggtttcgtcggtctcagcaccgttgatcgccacaacgggctcgccctgcacatctccgagggtgtcgaacatcggccccgggccttgcgccgcgtacggcaccgccagcgagatatcggtgccggggatgtggtcgaaggtcagcagcgcggtcagcgccgcgacagggatcgcaccccacgcgacagtggcccagcgcacgcgccgcacctcgtcgcccgtgtttaccccgccgaccgcaggttgcacttcacccggttgctgtccagtcacagcaggctagcttaacccagacggcgccgcttccagcgcgcagtggtcggcgctgccggcccagcagtgcttccacgtgctgttgaaccgtctgtactgtggtggggtatgagcaacggattcggattctccttccctaacgacgaccgcgataacgaccgcgaccgtgacaaaggcggcggagaccagggcaaccaaggcgacggcggcgccaacaacccgttcgccgcgttcggcttcgggggctttaacccgcagggcgcgtccggaggtttaggcgacatgctgaaccagttcggtcaaatgctctccggcatgggtaactcgatgaacactcaggcctccgacgacgcggtgaacttctccctcgccggccgcatggcgcgccagcgcgtggcaggcacccgcgcggtttccgccggcgacaccaaggccgttgaagaatcggtgaagcttgcggatttgtggctggacgaggcaactactctgcccgcttccggcacgaaggcgcaggcttggaactccgagacctggatcgacgagacgatgccgatgtggaagcgactggtcaacccggtcactgaccagatgaaccgcgcacagttggacaccatgccggaggaagcccgcgagatgatgggccccatggcgggcatgatgcgccagatgaactccatgcagatgggaatgaagctgggccacgctctgggtgaccttgctggccaagccctcacaggcacggacttcggcctgccggtcgccccgcgcggcgtcaccgccatcctgccgggcaacgtgaccgagattgccaagggtctcgaggtgccgggccaggaagtcatcgtctacatcgccgcgcgcgaagctgcccgccagcgcctgttccagcacgtgccgtggctggtcgagcgtttggtctccgccgtcgaggagtacgccgcgggcctggaaatcgacacctcccacatcgaggagattgcccgcaacctcaacctggagtccggcgacccgcagcagattcaggaggcgctgcagtcgctgcagggcgaggacctctccccgcgcgttggttcccgcaacgcggcggcgacctcccgcctcgagacgctgctggccttagtcgagggctgggtcgacgtggtggtcgctgaggctctcgacgggcgaatcccttctgccccgcagctggcggaagcgtgggcgcgccgccgcgccaccggcggatccgccgagcaggcgtttgccaacgtggtcggtatcgagctgtccgccccgaaggtccgcgaagccgccgagctgtggcgccgggccgaaaacgccgtgggtatcaagcgccgcgacgcggtgtgggaccacccagacttcctgcccaccgcgcagcatttggagaacccggcggcgttcattgacacgctgctggacgaccagccagacaccgatctcgacgctgagtttgccaagctcgaagaggagctgcgcgacaacccgacgctgaagcgcgaggacgacgacggcaaggacgacggccgcgaagacggcaccgaactgtaacaagccgggttacacgaaccgctgcagcgcctcgaggtaccctttcgctcgctcagagcgcggcgcacggtccgcccacgcccaaaactcgggcgagtgatcggggacgaacgtgtgggtgagctcgtggacgatcaccgcgtcgaccacgtagctgggggcaccgcgcagccggtcgctgatccggatatcgccggttgaggtggtacacgacccccacctcgagcgctggttcgagacccaccgaatcgaacggaacgacgcgcgcgactccagcacctgccggttcagcgcttcagcgcgaaccgcgagctgatcgtccgttgcgggtgtgcgcgacgccttcgcttggagccgggtaagcatctcagcgaccgcctcgcgttcctgcgccttggtcatacgctgcggaatgcggatttctgccaccccgtccactatccgcgcctgcaccgttttggtgcgcttcgcagagcggatcacgcggtaatcaatttcatctgcaggcacagcggttcattgtatgatgtcgcctgaacacatcggggggtggtttgcgcatggcgcgcgttaacaatctgtcgctggtccagctagcgaaaggcagcacggtcttccaacgggggccgaacctgttgcagttcggactcgacgccacgcgcacggggatcatcgaaaccgcgtgcgcgcaagagcttgtgccgatcatgcgcgcagcccgcatccccacccctgcccgccacctcaccagcgccatggcggaactcatcggccacgacgcggcgcgcagccttaccgcagacctcgtctcgtaccggatcctcgtgcccgccgagccgcgccacgtagcgctcatcggtgctagcccactcgcgaagcagctgtcggacttcctgaagacatgcggtttcgccgtttcgaccaaccttgagagcgccgactcgtgggtgccgcttgtcgcggtggaccagcttgctcacgcctccgcggtggctcgcatagcgaaacaccgctcaggccccgcaatcccagtcacgcacatcgactcccgcgtcatcatcggtccaatccgcctcgccccaaccgacccgtgccttatgtgcgcgaacgcgcacttcgaagacattgatgtgctgtggcgagcaacgctgactgagaacccccacggctcgcacgaccctgacccggtcgtcgcggcggcgggtgtggcggccgctgcgaccgtcatccgccgcgtcgccggagtaccagacccgccaggcgtgtccgcgcagtctgtctcacccggcgaaatcgtcgtgatcgaccctttcggaccgcgccctgtcacgacccgcgccgttgcgccgcatccgcggtgtcgagtgtgctactagcggtctgcgcctaatcccggaacggcgcgagcacttcgatgatctgggcgccgtacagctcgaccttcactggccccaccccgctgatcccgagcagcgacgcctcgtcgtacggcatggcctcggcgatcgcgataagcgtagcgtcggaaaacaccatgtaggcgggtttaccctccgcgcgtgagacgctcaaacgccattgcttgagcgcggcgtagacatcatcgtcgtaatccgcctcgcaggtggagtggcgccccaccgccttgtccgctggctccgacaagggcaaaccacacacccggcacaggcggctgcgtgtcaggcgctgcggtgatttctccacctcaagctccggcaccaagccgtccaagaagcgcgagcgggaccgggacttgcggccgccctcctgtcgggccagcgaccaggacatatggagatgctcgcgcgcgcgggtgataccgacgtaaaacagccggcgctcttcctcaatttgttcgtcgccggccttaatggcgtgcgagataggcaacgtgttctccaccaacccaacgaggaacaccgcgtcccactccaagcccttcgccgcgtgaaggcttgcgagcgtcacgccgtcaaccgcaggcggctgcttcgcctccgcgcgctgccgaagggaacgcagcacctgcggaaggtccgcggcttctttggaagtcacgatctcctcaatgagatctaccagcgcggaaagggcctgccaccgttctctcgcctgggcgccctcgggctcctgcggcgtcagcccgagcggggcgaacgctgcgcgcgcgaccttgacaggatcgttcggcagatccgttctgttcgcggcgcgggctagctggttaatcgcctccctgatctccccgcggttgaaaaagccctcgcccccgcggacttggtacaaaatgccggcgtcagccagcgccgcttcgaaagccgcggactgggagttaatgcggtacaacactgcgatctcgcgggcgggcacgccctgatcaagcagccgcctgattgcggcggcgacctcgcgtgcctccgtcggctcgtcgtcgtacgcgctgtacgtcggggcgggccccgccggccgcatgccttcgagttcaaggcgcgtgcccgcggcgcggccggtggccttggagatgaccgtattcgcgaggtcggtgatctgcggcgtggagcggtagtcccgctgcagcttcaccaccgtggcgttgtcgtacgtccgggcgaagttcagcaggtagtcgggtgtggcccccgtgaaggagtagatggtctggttcgcgtcccccaccacggtgagatcgtcgcgctggcccagccacccttccagcacgcgctgctgcagcggggtgacgtcctggtactcgtcgacaacaaacgactggtactgctggcggaactcctccgctacggcgggcacattttccagggccgcagcgacgtgcaagagcaggtcgtcgaagtccagcagcatgccctctgggctcgtcttctggtcttcgtagtggcggtacgcttgcgcaaccttctcggcgtctgccgggggcgtgcggttcaccgccgcaatgcgggtgacgtaatcgtccggcccgatcacgttcgattttgcccactcaatctcacccagcaaatcgcgcaccatttccttgctggagtccagtcccgccgcgcgagcggagcggcccaccagcgggaacttgttatccagcactctccacgggagctcaccggcgatgtctttccaaaagtacgacagctgccgcagcgccgcggagtggaacgtccgcgcctgaacgccgccgatgcccatcccccgcaggcggtcgcacatctcgccggcagcgcgctgtgtgaacgtcaccgccagcaccttctgtggtgctaccatgccctggtcgattaggttggcgatgcggtaggtgatggtccgggtcttgccggtgccagcgccagcaaggatgcacaccggtccgcgcggggcagtcgcggcgacacgctgatcgctgtcaagcaagctcaagtcaattgccactgcaagcctccttcaactccccgcgcgcccatttctcaatcaacgcccgagcgatagaacctgttttcgccaaggtcaacctcgccagatcggagcgcgtggcccagatgatcgatcccagctccccgtccagcggaccgtgcgcatctgtgtcgccggtgcgcgagtaaaacccgagcataagcgagcccgacatcgcccacggctgggagcagacataggagatgtcgcgcacgcgccgtcccgtttcctccaacacctcacgggaaaacgctgcctcagcggtttcccccgcatcgacgtagcccgcgatacaggtgtagtacccgggccggcggcggttctcgccgagaaggatccgctcgccgtcggcgtgctcaacaatgccgatcacgcacgggtcgatgcgcgggaaaatgggccggccggaagctccgcgtgcggcgccgtcgtttccccagttaagttcgctgccgtcggtaggatcgaaacgcattagttcgcgcgcgctcagcagcgccaccgcgcgggaaacaaccgggtcgctcgcgtgtgagcgggcgtcccccgtggtgaagctgatgtccgaagcgcgctggtctgtcaggcgcactgccaccacgccgtcgctgatgcgggcgtgggcggagggggtgttcggcgcagcgtcggcaagcagaagctccccttgcggcgtgagcgggaacgcgttgtccgaatcgatgagcaggtatttagtcatcgccgtggtccgtgggcttggtcatgcgcacgtagagcaagcggtcgcccggctcaacggtctcggcttccggcgcgtcgatgcggtatagctcgccggatcggaccacgccgagaacgatgtcagctaggtggcgggggttggcgcccacctcgtcgtctgcgatcggcctctcggcgacagcgaagccctcgtcggggctgagcaggtcctccatcatctccaccaccggcggggtgacggtagccaagccgaggaggcgaccggtggtctcggcggaaaccacgacagaatccgcgcccgactgcatcagcaggtgctggttttcgctctcgcgggcgctggccacgatcatggcgctcggcgcgagctcgcgcacagatagagtgaccaacaccgcggtgtcgtcggtcgacggcgcgaccaccaccgaacgggcacgggtgacgccggcgacgcgcaacacgtcagacttggtcgcgttgccgtgcaccgtgactaggccgcgcttctcggcggcacggagcgcaaccgggtcggtgtccaccacgaccaggctggagggcgacgcgccgtctgccagcagcgcgtcgatcgacgagcggcccttggtcccgtatccgatgacgatggtgtggttacgcacggtttgcctccactgctggatctggagcgttttgcgggaatcctcagtcagcacggacaaggtggtgccgacgaggagcatcaggaaggccacgcgggccggagtgatgatgaagatattgactaggcgcgcgccctgcgtgaccggggtgatgtcgccgtagccggtggtcgacagggagaccgcggagtaatacaaagcgtcgatgaacgtcagtgactccgagtacccatcccggtcgatgtagacaagtatcgccactgccacgatgagcagcgccgcgtacgcgaagcggcgagccatcagcgcccacggcgtgatgtgagcagagcgcggaatggagatgacatcggtcagagtgtcgaccggaacttcgaggtcgtcagagctcgaccgaaagagattcccccaggtcagcgcggacggtaatttcactcacgcctacctttctcaaagctatccattgcactgcggccatcttgtccgcccgaaggaaccttactccacgcttcggacacttcaggggtgatgagtgttacgagctcgtcagcatccgggaggtcgaccggcgcgtaatcctcccccgtgcgcacgtagaagaacatggcgcggacctcgcggccatcgccggtgattcgccgccacgcctcgcggtagaccgcaagctggagcttggcggcctccatgtctgcgggacgcggtttctgaccggtcttccagtcgaccactgtccaaccgtccgcatcctcgaatatggcgtcgatgcgcccacgcaccaccgcgtctccaagcgccagctcgaacggtcgctccacgtgcgctggtgtccgattcgcccagtggctggcctcgaacgacgccctgagctgctcgagcacagcgtggtcggcgtccgcttcgtcgtggccgggcaactcgttctcatccagcaacgggcgggcgccgtagagctcctccagccactcgtggaacgcggtgccgcgcttggcgaaggtgttcggcttgaacggcaccgggcgccgggcgcgccgcgcgaactgcgccgggtccgctcgcatggccaccacgtccgaggctgtcagctccgccggcacgacaaccggcaccccctcctggcgaagcgactcgtgctcctcaatgagcgcggtgacgtcgttctcccactgggtgaacagctgcggcgacgacgcgcccggtggcgcgggcatcgtcttcctggcttgcgcaaccatctcggctgcgttgaccttgcccgcctccggctcgagcgccggccaggtgccgcggcgctcaccgtcgacggcgttggcatcgtcagcttcaacctcatcagcaacccacgcgacgatgcactcgtctcccgcttggtctttcatctccgcgaagtgggcgtacggcgcgttgcctttgttcttgcccctgcgcttgaccttgccggcctcagcgcgcgacgcggtgaccatgagattcttcgcagcgcgcgtgactgcaacgtagaacagacgcgacgactcctcggcgagctcgtcgcgcacgctgtccttccacccgttcgctgctttctcgaactgggcgcgggtttccacctcggcgaactgggggaacagatccgggtcgccgaagttttcgtcctgcaggtacttcacccacgtcaagaacgtctcggccttcgcactatacgtcgcggcatcggcgtggagcaccgccacggtatcccattcgaggcctttggccttgtgcgcggtcagcagctgcacccggtcgtccttcaccacgacgttacccggcgcgaggccgtcctcgaaggtgcgcgcgagctcgaagtaatccagcagcccctccaagctggcaccggggtatgcggccacttcttccagcagccggtcgaggtgggtggcgcgcgccgcgctcggccgggcaagaacttcagttctgatgccgaagactgtgatgatgtcggcgaacagatcggatagtcgcttgcccagactgttggtgcgcagccagcgcagtttcgccgcgaggatctgcagccgcttatagccctcgacggagtagcgctccggctcaccgaggtcagcaaccgcgtcggcgagaccagccgagcgctcggcgcgggcgttgatctccgcagcgcgctgcacgatgtcgtccacctgcgcggtgtagcgagaccacgggtcgtcgccgaccagcgtgagctcctcggcctcctcgccccgctcgcgcgcacggagattcttggcgcgggcggccagcgcgttcaaatctgccaggccgagcccaaccgcgggcccgcccagaacgcggagcgcggcggctgagtctcccggacgcaccagcatggtggcaaccgccagagtgtccgccacctccgggatatcaagcagacccgccacacccacgatctcatagggcacgtcgcgctcctccagcgcctgcgcaacggcggcggtgtgcttgttcttgcggaccagcaccgccgccttcagcttctcccccgtctgctgggagtgctcgaagtgagccgccatctcgtctgccacaaacgcgatctcctcctcctgggtggcgaagtaaccgagtttcacgtcgcccgcgtccgcgccagggcgcggctgcagctgggccacagcgcggtcgtcgtcggtgccgaggatcgcgtccgagaccccgttggccaggtcgagcacttcaggggggttgcgccaagacgtggtcagctgcttcttcggcgccgcctcgccgcccgctagcgggaaatcctcgacaaacgcttccaagttcgccgcggtcgcgccgcgccaggtgtagatcgcctgcatcgggtcgccgactgctgtgacggtcagttccgggtcggccccctcgccgaacaagctgcgcagcagcacccgctgcgcgtgggaagtgtcctggtactcgtccagcatcaccacgcggaagcgcctgcgctggctctcgcccacctgcgcctggtcgcgcgccatcgcagaagcgaccgacatttgctcgttgaacgtcaccacaccccggcggcgaagctcctcctgcagtttcctcgccaacggcaggtacgcgacgcgctcctgttgcttggcgcgccacttccccatggtttgggagtactcgcccgtggtccgcttgttgccttgcagggcttcggtttctttcaggaaaatgtcggcgcgctcgatgatgctcgcctccgtggctagttcgttgcccatcgaagtcatcagcccgagaaggttgctcaccgccgtcttcaccgaggtgttgtcgctgccctcggcgaacagggtgccctcgtagttggtgacaacgtcggtcgcaatcgcgtggagctccgcgtccgtaatcagccgcgcgtccggttcgacgggcaccagcaggccgtattcgcggatgaggtcgccggcgtacgcgtcgtaggtggacacggtcggggcgatcacctccaagtgcttacccagctcaccgcccgggtcgagcctctgcacaagcgcgctgtctgcggccaagacagccaaccgatcacgaatgcgcttgtccagctcgcgggcagctttcctggtgaacgtcagcccgagcacttggtcggggcgcgcgtatccgttcgccaccagccacaccactcgcgcggccatggtttcggttttgccggctcctgcgcccgccaccaccagcagcgggccggggtccgctccaatgacgtcagcctgctgcggcgtcggcgggtactcctgctgcagcgcccgcgacagcgccaccggggacatcgtgttacgcatcggtgatcaccgttccttcaggttgcaccgggcacagtgcccggactttgcagtattcgcagtgggggccggtctgggccgtaagcgcagggcccgtcatcgcacccggcagcggctggatgaggttggcaaacgcgtcaagctcttcgtccgttttcgcgctttgctcgagcaccttcgccgtcttcgtcgtcgaagctgggtacaggagaacagcgctgtcgatctcgagcccgtccccgtctccgctgaccaccgactcgccgtcgagcacaccgtttcgaacagccagctgatacgccatgagctgggcgttctcctgcgcctgttccttcgtcggtgcgctcgttccggacttcagatccacgatccggacgcgtccctcgccgtcgacctccaagcggtccgagcggccccggatccgcagctcgggccccacgcgcacgtcgacctcagcttccacggcgagtgcgttccggttcgcctgagaaacgtcgagccagccgtcgatcttggacagcatccgctcgaaatcctcgaggtcgcgccccgccttccacgccggcccgtcttccatctggccgcgcgccgcaaccgctatctcgcgagctttatcccgttcgatccccctgcccagcgcctcgaaataggcgtgtgcgagcagccctttcaccatgtgcatggtttcgtcaagttcgaccatctgctccagcaccacccgcatcgggcattccaacagcccctcgatgcgcgagggcgacagggaggtccgcttcggcagggcttcgcttgtcgacgccccgccaatcccccaccactcatccgccgacgcccccgcgacgccagcatctgccaacctcgccagctgacgagctgcctgctcgtgcgcctccgacgggcagtccgggtcctgcagcgcccgccgcagctccgcaaccacgtcgtcccgcgacagcgtgcgcaccacgtacgcacttccacttgtcagtacctcactgacctcgcctgccgcagccacgcggcgaacctcgacgccgtgctcagcagcgaactcctcgacgaacctggaaggcagggtcacctcgtcgctttcctggtcgtcgacagcggtcacgagcaggtgcttagtcgccctagtggtggcgaggtagaagaggcgccgctcctccaccaaacgctcggccgagcggggaacgggaaccgctgggtcaacacccgcatcaacgaggtcgatgaggtcctcctgccggaacatcgtgcccgtctccccgagactcggccacgtcagctcttgcaccccggcaacgacgacgcgctcgaattcccgcccggctgcaccgtgcgcggtcatgagcgacaccgcgtcaggtttcgcggtgcggcggtcgcgcacaccggtgggcagctcctgctcctcaatgaactggatgaacagcccgatgcccgcggacgggcggcgctcggtgaagtcacccgccgcgtcgaacagcgccattgcggcatcgaggtcgcggtcggcttgggagcccgtcgcgccaccgcgcaaagccgcggcagacagccggccagacaacccggtggcttcccagatcgcccacagcacttcctcgacgctgccgcccgcatcgagcacgccccggccagcgtcgagcacactgcgcatccgggtgagaatgtcgatctcgcgctctgtgagcactccgccaaaatcgggggtttcggcatccctggacagcaggtcctggagggtttcctctgcccgctgggcgggctgcaacctgcgaaggccgcgaagcaggcggcgcagcgtgacggggtcggagccgccgaccggcccgaggatgagatcgcgccactgcgacggctgcagatcctcttccagagcgcgcaagcccagcaacagcgcgacgacgatgcgctgctgcgagagcaccacgtcggtggggtcgagcgcgaccgggacgccagcgtgcagcagggcgcgccggaccggctcgatcatgggggtcgatcgcacgataaccgccattgaggaatacgcctccccgccttccaaatgcgcgcgccggatcgtgtccacgatcgcggcgtggtgcgtctgctcgtccggcgcgacggcaacggagcgggctggcgttcgcttcgaagcccccaaatcgatcacgccgtgctcgagaccgccgaggtcggcgtagaacttcggcgacgcgccgcggaaacggaagacggactgctcagcatcgccgccaactacaccgagcgtggcgcgctgcaacaaacgcttcaccagttcggccgacgccggcgagaggtgctgcgcgtcgtcgacgatgacggtgtcccagtgctcggtcagctcacctttcaacacctcgcctaccagctcggcggcggaaaatcgcagcgcgcccgtcagcgacatcacctgccggtactcgcgctggaagtcgcccgcggctgcccaaataggaatcccgtgttggccgccgaggcgctcgaggtcttccggctcgagattgcgctcggccgcccggagcagaaaatctcgcagctggcgagcgaacccgaccatgggcagggctggccgcagctcttccggccagctcccgccgccgtcctctgcgtgcccctgcagcagttgacggatcacggcatcctgctcggcacccgagatgagtcgaatctcctgctccgtgcgctgacgcagcaacgcgaacgcgagcgagtgcacagagcgcaccataggctcgtctgcgacgtagcctgaagcggcgagcaaatccgagagctcggcgcgcagccgggcacctgattctttcgacgacgagatcaccaaaaccgagccgcgcgacgcggccgcggcagcggtgtcgatgagaaagctggatacgcccgagcctgcctcacctgtaatcttccacatcccctccgcgggaaggttccggccccattgccgcgcctgtgcgctgcgcgttctgggcacgaggtacgcccgcggcgttaccgctgcggggatggaaggaatgtctggtgagctcatagccaccatcgtggcacatcaggcaaacacgatctcccgaacacgccgcaaattcgcacgcgcgttcgattccaggtgcgcttctccagcctcccggaactcatacgccctgcgcactagctcgtcgatgcgcggaacgtgggcccagcggcgaatcacgcccgggtcgacagcggaggcgagcaaaccgtccacaatgacaatcgcggcggtgtacccgcgcggacggagcccggcagagggcacgagaccgattaacgtcggcggcaacataccgtcgaaaaggcagtggcgcagcatggaaaggtttgccaccacgccggaggagtcaacgtcgccatcggcccagacagctcggtcggcgtctgcccacacatcgccttcgcggggcgccgacgggggttgggaggggtgggaggtaagcgctgcgtcgataagcagtgaagcccccaccgcctcatcaatgcgcgcggcggtctccccctccgcgaactcgttcgccgcgaaaccgccgacgaccaaccgaccgtcggtcgcccgcacaggtcgagcgatgcggacaccctcaacttcgccggcgagcttctcccggcacttggcggaccagaccgccgtctcgaccgccggggagacaaccacgcggccgaagcgctgtccgccgtcccacgctggcgacatgtcctcaccgctaccctcaacctggaatgcgtgcaacacgtgttccggaatgcgcacctggttcctttccctcaaacgcttacagcacggccgggcgcgggtacggccacgggttatacctgcacgtatccgagttgtctgggtaaacctccgacgggtcaaagctgcgcagctcagcgttgttcacactcagcgtctgctgcatcatgatcggcgccagcgccccatcggacgggcacggcacgtgctcggcgaagccaagcgcgtgacccacctcgtggttgatcacgtactggcggtagctgcccacatcgccttgaaacggcgcggcgccgcgcacccagcgggactcgttgatcagcaccgtgtcctcgcctgtaatccgggtgcggcagctcgtctccaacccgagctcgcctccgcacagctcgcgggtggtctcaacggaggcgagacggatacgcagcgtcggctggtccgccgcggtcacatgctcgagcttgaagcgggggtcgttggtccaaccacgcgggtcaaacagcgtcgaatccaccatggcggaaaacgcgtcgttgccgccgtaggcagcggtgtcgacgccttcttccacctcgacgacgtagcgcaccgtaagttcggtaccctcgccgcccgatgcaccgggagcgccgacttcgaagaactggccagtccccttctcggtgaacggcccgccgggaggcagcatgttcacatcaagctcaccctcgggtagcgccgccggttcgcgcacgtcagcaccctccggcgccgactcggcgtgcccgtcccccggtgcgtcctgagcgatcgtgttggcggcgccgacgactggcccgtccgggttctgcaccatgttgatgatcacgaacacggtgatcacggccagcaccggaatcgcgtaggcgcgccagccgtagtcgcgcgcgagctgcacaagcttgccgtcgttggcgccgccgggcacggcagcgcgctgcaccgagaccggctcttgccggtctcggcggtcgcggcggcgcggctcctccgcctcccacgcactcggatcgtcgaaatcgtcccagtcgtcggcggcgtcagtgatgcgctgctgccgtttcgtcataggcagttaatctagcgcatgaagcccacagaatgggtggtcgccgaaccctgctcgacgtaaacaatgcgatccgtgcggatcaggtaattgcggcccttgtcgtcgctcagcttgatcaccggggtgccggcctcgattgcgcgctccacaaccgcggtcacatcctcgctgccctcagccgggcggataaccagttcacgggggctttcagcaagtccaatcttgatatccatgccgccattgtaacggtggcgcacacaccgcctaggctgccgagaacgcgcggggcaagcgtgcgcgggtcgcgggctaagatgtcggtgtgccgaacaacgccgaaaaccccagccagccgacgttcacctcgctcggcgtcgcagccgagctcgtcgacgcgctcgcggatctcggcatcaccgaagcgttctcgatccaagagctcgccatcccgctcgcgctcgacgggcgcgacctcatcggccaagcacgcaccggcatgggcaagacctacgcgttcggcgtgccgcttttagacagggtgttcgatgacgcagacattgctgagctcgacggcacaccgcgcgcgctcgttgtcgtccccacgcgtgagctggcagtccaggtgggagaagacctcgagcgcgccgccaagtacaccccggtgcgcaccgcgaccatctacggcggccggccgtacgaggagcaaattgaggcgcttcagcgcggcgtcgatgtcgtggtcggcacgcccggtcgcctgatcgacttgtttgagcggggggagctttcgcttgccgacgtagccgtgatggttctcgacgaagccgacgagatgctcgacatgggtttcctgccggacatcgagaagatctggggcgcggtctccgaggatgtgcagacgatgctgttctcagccacgatgccggggccgatcctcacgctagcccgttccaagatgcgccggccggtgcacatccgcgctgaatccggcgacgcgcccgcaacacactccaccacgcgccaggtggtgttcaagtcccaccggatggacaagcctgaagtggtggcccgcatcctgcaagccgacggccgcggccgcaccgttattttcgcccgcaccaagcgcaccgccgccgaggtggccgaggaccttgcgaagcgaggcttctcggtcggcgctgtccacggggacttgggccagaaggcacgcgagcaatcgctggaagcgttccgcgccggcgaggtcgacatcctggtcgccaccgacgtcgccgcccgcggcatcgacgtcgacgatgtcacgcacgtcattaactaccaaacacccgacgacccgatgacctacgtccaccgcatcggacgcaccggccgcgccggccactccggcaccgctgtcacgttggtcggttacgacgaggcccacaagtggcagatcatcgactcagaactcaacctgggcaaggccgcgctccccgagtggttctccacctcagaagagctgcgcgaggcacttgatattccggagtcggccaagagcagtgtgggcgcggcgcgtaaagtgcacggggcacggacaaaccaaccacgaggaggcagacgccggtgagccacaccctgcgccgcaccacgggcgacctcattgccagcggcgtcattgccgcgatcgcgctcgcgctcctacttatcgcgtttctgactgccccggtcaggtcggcgcagctcgatccagcacccgaggagttggagaatgtgggccgcttggcggtggcgccgacaaagttaagcgaaagcttccgcctgcccgaccacgcgcccgacaccaagccggtggtggtcaacggcgtgatcgtgacgtacaacgacggcgccgtcaccgcgacaactcctgcgggcgagaccgcctggacctaccaccgcccaaacgagctgtgcgcgctcagccaggcgtggggcaaggttgtcgccacctaccgcgacaacgcgggctgcggcgatgtggtggctattgacgctttgaccggccagtacgccggcacgcgctccgcgatagccccggacatggtcacatcggtctcctccaacgaccgcatcggctacgtgggctcgacgcgcgctgagctgtggcgctccgacatggtgcgcacggtcgagtacggctacgtcgaggcgccgcaggagccggacatgcagcccaaccgctgccagatcacctccgcgcttacccgcaccgagctgttcgcagttaccgagacgtgcgctgacggctccttcttgcgcctgcaggacgccacgcccgaagactcccgcaaaccagagatctacagcggcgtcgacatctccgaggagtcctacctggtcgcgatctctcaggacgcagcggcggtctacgacccgggcacttccgagatcctcacctacgacaaggaggggacgctgatcgcagcctcctcggtgccggacctaccggggccgttgacgctggataacggcgtgcaccctctgccggtcgccgacctaccgcaccacatgacctaccacgagggcgactacctggtgttgatggagccgtcgaaattggccgctaccggggtgttccaaggggccctcggcacagggttcgccgccggcgaccgcctgctctacgcctccaacggcggtatcgccgtagtggactgggacgcgaacgccgtcgaccgcatcatccccgtcgaccgcggcacctactcggggcccgtctccatcgattccgcgggcgccacgatcgtggagaaacgcggggacgaggtcgtcgttctagcggcgcaataagcagcgatacactcccagtgtgagtacgagccgcaaagaagcaaaacccgcacccgaccgcgagaccctcgagcgagacgcggcagtgatgcccccgctgatgcgctacggcgcgtatgttgtgctgctgcagtgcctcgccgtgctcggttacgtcgtttcgctgttgctgaaccagttcagcggcggcgagagcgtgcttgagtccgattcggctgccgccggatacgtcaacatcggcaccgcaatctttttgtccatcatcttcggcttcatcgcgtgggttgccgcagagacgctgcgcggccggccgcgcagccaaggcgccgtcatgctgattgagatgatcctcatcggcgtggcaatttacatgttccgcggcggcgcgccgtggatgggtctggccacgctcatcaccgcggtcttcacgctgtttaccatcctgcacccggccacccgccgctacgcggaggcccgctacgccgttgaccgcggccgcgcgtaggcccaagcacagccaaccggcagcagttggcgttgcggcgatttgacggtgcagaaaaacactcctcggtcccattgagcaccgtcatccgtggtcacagcggttttcacgccgtccccacaactccccacccccagatccatcgcccccgtttgctagctcaaccgagcgaaacgggggccttttctgtgagttgcatcacatttacatcgctacccctagcgcgatttgacgaatcgtgtcatcatcctcgggtagcaaaaacaacgggctggttacacagcccttaaccccaagccaccacggggttaacgccagggaaactggaagacgggtccagcaaggaacaccgcctagtgaactggaatcaaatcttcctttgcaacatccccgatccgtcggggttgaagtggtgcgcaactttcattgagacgtgtaaagaccgtaaggagtatttgacatggattggcgccacgaagcaatttgccgcgacgaggacccggagctgttcttcccggtcggcaactccggcccggcactgtcccagatcgcccaggccaagctggtctgcaaccgctgccctgttacctcccagtgcctgaagtgggcgctcgagaccggccaagacgccggcgtgtggggcggcttgtccgaggaggagcgccgcgcgctcaagcgccgcaacaaggcccgcgcccgcaagcgcgccagcgtcacggtgtaacacctaatttccgcgcctgcccatccgggcgatacagtaaacaccgatatctgccacacaataaaggaggcccacatgagcaagcgtggtcgtaagcgcaaggatcgccgtaagaagggcgcaaaccacggcaagcgccccaacgcataagcgctgagcaaccaaaagcgccgctctcacccgtctcagttcgggaaggagcggcgctttgttttacccccgctagcggtagcgcacctcggtgtagctcaccgcggtcaccgagatcgaggcgatgatccgctcgcgcagcggctcgggcgctttctgcccaccgcagcagtcgcgcacgagactgcgcacggctttctcggattcaaactggccgaagcactcggggcacgcctcgatcgcccggaggatctcagctgagcgcgcagccgtggtttcggggtcgaacagctcgttcaggagttgctgtgcatcttcgtcgcagtctgcgcagttgcagccgcggttcgggtctgaagttgccatctacttttcctccgatttcggccggtctaagccgatgccttgttcgtttgctacgtccttcaacatctcgcgcagctgttttcttccgcggtgcagccggctcatgacggttccgagtgggatatccatcacttccgcgatctccttgtacgccagaccctccacatccgcgtagtagaccaccatgcggtagtcctcgttcaaggcgttcagcgcctccgagatccgcgagttcggcatcagcttcaacgcctccacctcggcggattccagccccgtcgagtcgtgcgaggacgaggtgtagagctgcgagtcggtcacgtcctcggctgaagtgaccagcgggcggcgctgctttttgcggtacgagttgatgtacgtgttcgtcatgatccggtagagccacgccttcaggttggtccccggcgtgaagctgtcgaacgcgttgtacgccttcaggtaggtctcctgcaccaggtcctcggcgtcttgcgggttgcgcgtcatccgcagcgcaccgccgtagagctggtccaaaagcggcatggcttcttcggtgaagcgcgatttcaaatcgggctctagctcggtttcgggcatagtggtcattgtattgaaaggagtcgccatggccgcgcgcacccgcgctctcgaggccgccgccggcacgccgcacgaggtttacgagtacacaccgagccaggaccacttcggcgagcacgccgcggaggagcttggaaccgatcccgccaccaccttaaaaacgctggtgattgtcaacaccgccaacccgagggagatggccatgtgctgcgtcccggtcgccgggcacctctcgctgaaagccgccgcgaaggccctcggctggaagcacgccgagatggccgaccccgctaaggcgcagcgggtgacgggctacgtcgtcggcggtatttcgccgctcgggtcgctgaaggagcttcctttgcttatcgacgccgccttatccccccaacccaccgtcaccttctccgccggccagagaggcctctcgctcgcgatgtcgcctcaggacttggcctcgctgacgaacgcgaccttcgccgacatcagcgctcagtagacgccccagtcagcgccgcgtagtcgttgcgcacgttgccgaccgccttgtctgcctcgctccagataaacgttccggcggcccgagagggcgcgatcaactccgccgcttcctcggggctgccgtgcacccactgctcgatttcatctggcaagagaaacagcggaagacggtggtgcagccacgccatgttctcggtcgcctcggtggtgaccatcgtcgtcgacaagcggttaagtcccgtctcccacagggccgcggcgtagagcagccctttttccgggcgcacgtagtagggggtcttgccggcctcgccagctttccactcgtagtagccgtctagcaccatgagcccccggcgcgcctgaaacgcggagcggaacgacggcttgtccgcaacggtctcgccgcgcgcgttgaatagcggcgcgccggtctcgtccttcttccacgtcggcaacagcccccagcgggctgggtcgatgcgcgcgatggccccgtcgatacgaagcagcggcacctgttgcgtcggcgcgatgttgtagcgcggcggcggagtaccgtccggtgccttcaccgcgtccacgcccggcaggcccccgacctcctcgtacaggtcgtggcccgaggtgaaaagcacaaagcgtccgcacatgcctccattatgatggagcacatgacaaacctgtggcccgccccgttcgcctcggccccgatcacgcacaccgtcgagatcccggggtcgaaatcgatgacgaaccgcgcctacgtgctcgccgcgctggccgaaggagagtccaccattgtcggcgctctgcgctcgcgcgacaccgatctgatggagggcgcgctggcggctatgggggtcaccttcacgcacgagggcggcacgatccgcgtcacgccgggtcaactgaccggctgcgaggtggattgcgggctcgccggcacggtgatgcggttcgtgccgccggttgcggcgttcgcgcaggggccggtgcttttcgacggcgacgcctacgccaaaaaccgcccgatgagcaccatcctggacgcgcttcgcaaactcggcgtcgccgtggccggggactcgctgccgttcaccgtccacggccgcggcttcgccgagggcggcgtggtggagatcgacgcctccgggtcttctcagttcgtctcgggcctgctactctccgccgcccgcttcgaccgaggtgtgaccgtggtcaacaccgccggaatcctgccgtcgatgccgcacatcgaaatgacgctagcgatgctcgaagacgcgggggtgcacgtcaaagcagacgggcagcgctggcaagtcgacccccaaccgatcaagcccgcgcgattcgtcatcgagccggatctgtccaacgcgacgccgttcctcgcagccgcagcagtcaccggcggcaccgtgcgcgtgccgcactggccggtggacaccacccagccaggagacgtcatccgcctcatcctggagcgcatgggctgccgcgtcgagctgtgcgccgatggagccgactacaccctcgaggtggaaggcccggtgccgggcacgctcaagggcctgcgcatcgacatgagcgacattggcgaactcaccccaaccgtagcggcgctcgcgacccaagccaccacggtcaccgagctcaccggcattgcccacctgcgcggccacgagacggaccgtctggcagcgctcacccgcgagatcaacaacctcggcggcaactgcgaggaactccccgacggtctgcgcatccaccccgcccgcctccacgacggcacgtggtcgtcttacgccgatcaccgcatggccacggccggcgccatcatcggcctcaccaccgccggcgtcgaagtggaggacatcgccaccaccgcgaagacgctccccgggttcgaaacgatgtgggcgcgcatggtgaacgcggcggtggagggctagtgcgcggttttgccgactacgacgagtccgacgcgcgtgtgcgccccggcaagggctcccgcccccgctccaaggaccgcccaagccacgccgacgctgagttcggcatggtggtgacgaaagaccgcggccgctggggcgtggtcctggactccggcacgcaagtgacctgcatgcgcgctcgcgagctcaaacgcatctctgtggaggtgggcgaccgcgtgggcgtggtcggcgacacgtccggccagaaggacacgctggcgcggatcgtgaaacgcgaggagcgctcctcggtgctgcggcgcaccgccgacgacacggacccatacgagcgcatcatcgtcgccaacgcggagctcatgctgatcgtggtggccgccgccgatcccccgccgcgcacggggtttgtggagcgcgctctcgtcgccgcgttcgacggcggtgtcacccccgtggtgtgcatgaccaagtcggatctcgcggatccgggcgagttccagcgcgagatcgaggacctcaacgtcgcggtgtacgaggtcggcatcgatgaaccggtcgacgccctgctcgagctgatcaccgaccgcacctcggcgctgatcggccactccggcgtgggcaagtcaaccctggtcaacaggctggtcccggacgctgggcgggagaccggcgcggtgtccggcgttggcaagggccggcacacctccacccaatctgtggcgctgccgcttgccggcggcggctgggtgatcgacacccccggtatccgttccttcggcttggcacacgtcgccccggacgcgatcatcgatgtcttccccgagctcgccgacgccgccgagcgctgcccccgcggctgcacccacctcggccccccggctgacccggaatgcgcctgggacgagttcgacaccgactcccccatcggccgccgcgtccaagcggtgcgccgcctgcttcaggcgctgcactcgaacaacgagtgggatctaaagcagctcgatgaggaacggtagctcggtcgggtcgaaaaacgccatgtagttgtcttgggcgtcgcccacggcaagttcggcgtcttcgtcgccgagatcggctgcgtcgataagctgcactgctttctgcgttgcctcctcagcttccttgacgtcgacgtggatcgccgcaacgtccttcagctcgacgggggcatgcagcttgacgacggactcccccatatccggcgcgccctcagcctcagtatccaccgagatcaccacgcgccggtgcgggaacttctcctcgtccccgatggcgaggaggcggagggaggcaagcgccgcgtcgtcgaacgccactgcctcgatctcctcctcatcgcccgaggtgaagaattcggtgagctccggcgtggcggcaaaaccccagccgttgcgggcgtggatgagcccgttctcttcaagcgactccagcatcgcgaacgtcgcggggaggtagacgcgcactagaactcgccctcgatgtcgaagagggactggatctcgaccgagctgcggtcgaacgcggtgtgaaggatgccgatcatgccgtactccacggcggcgcgaacgttcatgatgtcgtcgtcgatcatgaccgcgtcgttcagcgcgacgtcgagggcgtcagccgcggcttggaacgcggcgcgctccggcttctccgccccaatctcgccgctgagcacgacagcgtccacatcgccgcggaactcccactcgcggatcttctcggcttcctccccctcagccgcctcgttggagagaatcgcggtggagaaaccgcgctcgcggacagccgcgatcagggtccgccaccgctgctggtcctccgggtcctggtccagcaccccggcgtagtcaatgatcaaaccctgcatcacatctccacttcgtcgtcgacctgcggttccgccccgcatgctcactttcttggacgcggtggcgcttcttctggccccgcgcgaacgtgcacaatactacctgtgtattaccaggcaccgggccaccagcacgtcaaggtcgtcgtaccgcgtgcgcaccgccccgatatcccccacgcccgcgctgcgcacgcgcttccgccgagccccatggccccgctggtgcgccaggcgctcgacgcatccttcgggcagcgcgaccccgagtccctcacgggcgcgttgttcgacctcgcggtccgttcccacgtgcgttcccgttaccgcttctcggacgcgaagggcaaagtgaccgtgacctcgtgccacgcccgcgagcgcggcgagtacttcggcacggttgaagtgggcggcaagccctacggatacgcggcccgcatccgcgcaggccgcctcatctcgttcaaggtgctgtagcgacttcgccctactcagccggctgctcgaactgcttgcgcatcataaacagctggcgcacggtctcctcctggacggcctcgttcatcgcgttgaacatgtcgccgccttccttctggtactccaccagcgggtcgcgctgcgccatcgcgcgcaggccgatgccctctttgaggtagtccatctcgtagaggtgctcgcgccacttggtgtcgatcaccggcaggatgaccatgcgctcaatgttgcgcatctgctcttcgccgccaatcgacgcgacgttctcctcgagctggtcgtactgggcctgggcatcgtcgacaagcgcctggcgcagctgggctggggtgagctcgcctggccggccgtactcgttgccgtcgataagctgctgtgcgcttaccgacgggccgtagagagcatccagcgcgttccacagctcgtccaaatcccagtcctcgacgtagccttcgcgcgtcgcgccgtcgacgtaagcgccgacagtctcgtcgatcatgcggcgcacctggcccgcgatgtccttggaatcgaggatctcctgacgctcgcggtagaccaccttgcgctgctcgttgagcacctcgtcgtacttcagcacgttcttgcgcatttcgaagttctggttctccacgcgcgactgggccgacttgattgcgttcgagaccatcttcgcctcgatcgggacgtcgtccggcacgttgaggcggttcatcatgttctccatggaagtgcccatgaagcggaccatcagctcgtcgcgcatcgacaggtagaagcgagtctcgcccggatcgccctgacggcccgcgcggccgcgcagctggttgtcgatgcggcgggactcgtggcgctcagtaccaatcacgtacaggccaccggactcgcgcacctggtcgccgagctgcttggaacgttccttcgccgccgggagctgctcgtcccacgccgcctggtagcgttcctcgtcctcgaacgggtcaagaccctgttcctgcagcttcgcgtcgagcaacacctcggggttgccgccgagcacgatgtcggtgccgcggccggccatgttggtggacacggtcaccttgcccggaagacccgcctcggcgatgatgcggccctcttcctcgtggtgcttcgcgttgagcacgttgtgctggatgcccttgcgggtgagcagctgggacaagtactcagagcgctcaaccgaggtggtgccgacgagcacgggctggccgttctcgacgtgctccgcaatgtcgtctgcgaccgcggaaaacttcgcctcctgggtcttgtagatcaggtcgtcgcggtccacgcgctggttcggcttgtttggcgggatcgccaccacgtcgagcttgtaaatctggtgcagctccgcagcctcagtttccgcggtaccggtcataccggcgagcttggtgtagaggcggaagtagttctgcagcgtgacggtcgccagcgtctggttctcgttcttgatctcgacgttttccttcgcctcgatcgcctggtgcatgccctcgttgtagcggcgacctgccagcacgcggccggtgaacgagtccacgatcaggacctcgccctggcggatgatgtagtccttgtcgcgctcgaagagctccttcgccttgatggcgttgttgaggtaactcaccagctgggagtgctccggcgcgtagaggttggtgatgccgagctggtcctcgacaaactcgacgccctcctcgctcacgccgatcgtgcgcttgcgctggtccacttcgtagtggatgccctcgcgcatgcgcggcgccagctgcgcgaacacggtgtaaaactggctcgagccgtcagccgggccggagatgatgagcggggttcgggcttcgtcgataagaatcgagtcaacctcgtccacgatggcgaagttgtggccgcgctggaccatctcggcgggcgagcgcgtcatgttgtcgcgcaagtaatcgaacccgagctcgttgttggtgccgtaggtaatgtccgcgtcgtaggcggccttgcgctccggcgggcgcatctcggagaggatgacgccaacctcgagaccaaggaagtggtggacgcggcccatcatctccgcgtcgcgcttggccaggtagtcgttcaccgtgacgatgtggacgcccttgccctcaagcgcgttcaagtacgccggcagtaccgaggtcagggtcttgccctcaccggtcttcatctcggcgaccgagccgaagtgcagcgcggcgccgcccatgatctgcaccttgtagtgcttctggccgagcacgcgccacgacgcctccctggcggtggcaaacgcgtcgatgaggatgtcgtcgagcgacgccccgtcggcaagctgcgccttgaactcgtcagtcttcgccttcagttccgcatcggtcaacgccgcatactgatcatcaagcgccatcacctggtcggcgatcttggccagacgcttcacggtgcgtccctcgccggcgcgaagcagcttcgttagtccttgaaacacgttaaagaaatccttttgtaggtttctgcaggtataccaacgaaccagtgtacccaccgctaccttgcaaccaggatgcagccggctgggaacttccttattgggcgaccggtgggcgcaggtgaatgaggtcgtccgattatgcgcggcataattttcgaacgcttgttctataacgtgcgatcgtatgttcgaggcggtttgtatagtgttcgcaccgatgtttcacctccacaattccccagccagagcaaggaaaccgccatgaccacaacgcttctccctccccgccgcagcaccgatgccaagacgatcgcgggtgagatacgcgaacagcaccgccttaccaacgtcgctaaggccgagttgttagaactgattgcccatttcgacgagcacgagttgtcggaggcgctcggagcgtccagcaccgttgactggctgcaacgggagctgcgctaccccgtctcaactgcctacgagtacgtccgcgtcggccgaaagttgcgggactttcccctgcttgccgctgcattccgcaaagcggagctggattacaccaccgtcaggttcctgctgcagtacatgactgcagccaacgaatcggatctggtggagttaggtcgcaccctgtgccacgcggaactgcggcaagcgctcgccggggcaccgaaggatgacgacagggacccggacgagccgtatttcaacttggacactcggtcggatggcatgtgggctggcgacttccttctcacaccgatgatgggcgaaatattgaaatcggcgctcaagattgcccagctggccaactacgacctcgaaggcgaggacatcgagggattactcaacgaagacgtaaaggccgtcatggagcaagaactgcgcgaaatgttcggcgacgcgctggtcgacgcgtgcgaccctcaggcaaccgccgaggacgaatgcgcggtcccgcgtcctgatattgaagaggcctgccccggagagcaggtcgccgcgccgcgaccagataccaagatcaccatggagaagctcttacgcgtccccacccgcttcggtgcagtggccaacgttgacctgtacaacgcgttcgtaaacatgatccagatggtccgtgcaaacccggtcaccccggtccgcgctcccggcgccaacgtggcgatcatgctgaccgaggacggcaaggcgtggatgccccagaacccacaagtgccgtcgtcggtggtgcgcgattacgtcgccaacgccatgtaccgcatgcacataacggaccccgcggggttgacgttgtcgtacgggcgcgaacggcgcttcgccagcgacgcacagatcggcgcgctgctcgatgtatggggccaccaatgcgctatgcccggttgcacgcatacccgcttcatcgagattcaccatattaaggagtggtccgaagggggtcggaccgatatcggaaacctcatccccctgtgctcaacctgccactccaaggtcagccacggactggcacacattacgcaagaagggcccgacttagagttcaggttcaaggacggcagccgcttcatctcgcgcaatcggggacttccggagcgcgccgccgactacgaaggtcccatgcgtgagtacgagttcaggtccgacctgtcgttcgagtagccgactatgccgcgcataaattatgccgggcataaaacaacccacaccctgaggtccaggatgcgggtggatgagaagagtcaggcgtaagcagacgttactgctcctcgcccccgttttcggcgatctcggactcagaggcgagcgcgatcaggccgtagtcgtaggcgtggcggcggtagaccaccgacgggcgctgcgtttcttcatcgatgaagaggaagaaatcgtggccgaccagctccatctcagacagcgcgtcgtcgacgctcatcggagtgttcgggtgcagcttgctgcgcacgatctggcccggctcgaagtcggcgaactgatctgcgtacgggtcaacgtcgtacttgcccggctgcgcctcgcggacgtcggcggcctcggcagcgagctcagcggcgacgacaccggtggacttgggcgcgcggtggcccgagcgggaaatctcgcggcgcaccttcaccttgcgcagggagcgctccagcttgcccaccgcggattcaagtgcggcgtagaagctgtcttccttcgcctcggcgcgggcgaggtggcccttgcccgaggcggtgatctggatgcggttggcctgcgcttcgcggcgcgggttcggctcgtgcttcagctccacgtgaaaggaggtcagcgaggggtcgagcttctcaatcttcgccagcttgccgttgacccgctcctggaagtgctccggaacttcgacgtttcggccggtgatggtgacttgggcggcggggctcaagccaacgttttggtcatactctgcagaagtcatgttctgcctcctcggaaggtagtaggaaccgggttcacctctgattatacagctggtcatgcggagttaatgtggttttcatgttatgccgcacataatgcgacgcaggctttcacatcggcgccgtgggctagcaacttttcgacgctcgcctgcaacgtcgcccccgtcgtcaccacatcatcgaccacaatgaccggttgggccggcactgcggagatgcgcacggcgttggcgaggttggctcgccgctgcgctgcgtcgagctccgactggtccgccgtgcgctcgcggaggctgagcactgggacaaccgatcgacgggtggaccggcagcacgcctcgacggggtcgccaccgcgcgccctcgcggaagacggccgcgtgggtgcgggcacgagcgcgcagctgtcgggaatgtcgccgcgcgcctcgaggtagtccagcgcagcgtccaggacggcaccgacgtggcggcgcacggcgaggttctcgcgctctttcatggcgagcaccaccgagcggtgagcgtctgcgtaggaaccgagcgcgaagactgggacgtggggcgaggtgggcgggaacacccgcgcaggagggtgagcgagttggacgcggcagtcgctacaaagcagctgccccggctcgccgcagccggcgcagtgacgaggcagcaacagttcggcgacgtcccccaagatccccacaactgcactagcttgccacagatcagcgcgcgacgatggggagcgcgcgaactccctgcaaaccaggcacttcgcgccacagtgggttgtcggcgccggtgttgggcagctgcaggatcgcgttggcgtcggtgacgtagagcatgttcggcgacgcggcgacggccaccaccggagccgagatgttgcccaccgacaggggcgcggcggaggagccgtcctgttctacgcgcagcaccggcgagacggagctcgaggtgcccacgatcagggaaccgtcgggctgccaatcggcggcgacgacagagccgccgaggtcgggcgcgtactccatcacgttgatgatggcgcggtcgccgggcgcccggcgggccacgattccggtgtagaggtggccgtcgatgaccatcaccacccgcgcgccggagcgcgacagccgcagcaccgagatgttgccgctgactccctctggcagctcggcgacaatctcctcgcttgtcacctcgccgctggcggcggagcgcacggagcgaaggatgcgggtgccgtcggcaaccgtccagacggcggaggccttgccttctaacgacggccgcgtgaaggtgcccgcctcgagcagctcgaacgactccttcccgccggagtccagcgacccggcgcgcaagcgggaagtgccctggccgtcggtgaagacggcgacccagccgccgctcgcggtgatttcggcgctggcgacgttgccggaggacagttcggagtttaagggggtgggcgaggcggcgtcgataagcgaaatgctcccgtcggtgagcgagtagagcgttgacgcgccggcggattgaaccaccgggcttaggtcggcgaagtcgtccgtggtcagggtgtcggcggaggtgagcaggggcgcaccgtcggcaagcagccgaaacgggccgttgatgcctgccgacgccagcgtccacaccacctgcgacgcgaagcgcccgcggtcttcctcgctgaccccgccgaaaccggagaagctgtaggcgccgtcctctaccccgaggtacgccgctccggcgggcaggatcgagctgagcgcgggctggaggcgttgcgacggcccctccatcagcagcgcgatgagcgcgctcggcagcgtctcgcgccgggagtagacccagcggcggtcggtcaccaactcttggccgcggttgtcgaagaaatagaggttgagcggctggtactggttgcgcagctcggtgcgctcgaggacaacacccggcggcagggaggagatgcgccactcaccgccgacctgctccatgtcgatcgtggcctcgtaggagccgcgctcggggcggaacgcgccccccgcgccgaggacgccgacgacgttgccgtgggcagagaagctgcggcgcccgcctgtgccgccggcgattgtggtcacaccgatgcggtcgacgatgagggtctccacgttcgggtcccacgtgcgcgcggcctgctgcgtcatgaacgcacgcgccgcctcgtaatccgacgaggggatcgcggaggctgcgtagaagtcgcgcagcagcaagtcgggctcgcggccggcctcgggggcgatcaccggcgcggcgggcgcctcggagttgtacgtgcgcagcacgtgcgggttcgaggtggacggcaagctcgcgcagctgctcaaaagcgccgtcaccgccaccacagctgtgagctgcgctcgcctactcctgcgtgcgagaaccgttcgcatcgcaatccacctccacagtgttctcgtcggcgccctccatcgcagcgcgcgcctctgccaccccgtccggttcgcccggtgcctgcagctcgaccggcgcgcgggcgaaaccttcctcgggatgcctcggcagcaccaggcggaactgggagcccacccccggcacgcccgccgcgtcgagcaagccgcggtgcagctgcgcgtcttcccgggcaatggcaagacccaaaccggtgccgcccgagtggcgcttgcgcgacttgtccgcgcgccagaagcggttgaacaccagctcttcctgcccaggtttcaggcccacgccgcagtcggtgacggtaacggccactgcctcgtcgttctgcgccagcgccacctgcacggggttgccctccgagtggtcgatggcgttggcgatgaggttgcgcacgatgcgctcgatgcggcgggggtcgccctcgatctgcatcgcgtctgcagggacgtcgaactcgaccgcaacgtccagctcttcggcgagatgctgggtttgagcccaagccgattcgatcggggcgcgcacgtccatgacggtgctcgccagctcagccacaccggcgtcgtggcgggagatctcgagcaggtcggtgagcagcgcctcgaagcggtcgagctcgcgggtcatcagctcggaagcgcggcgctgggccggctccaagctgtcctggtccgccgcgatcatgtccgcggccatgcgcacggtggtcagcggcgtgcgcagctcgtgcgacacgtcagaggtgaactggcgctgcaggtcgccgtactcctccagctggttgatctggcgggacagcttgtcggccatgttgttgaacgacagcgcgagcaccgccatctcgtcttcgccctccacaggcatgcgttcgcgcagatggcctgcggcgaagcgctcggcggtgcgcgacgcggagcgcaccggcgcgacgatctgctgcgaggcgagccacgcgatgccgaccaagagcacgatgacaatcagcgcggctgaggcgagcaggccccgcatgagcgcgagcgtggacgcctcgttgtccatgttggtaactaagtacagctgcaagttcggcacgtcggcgtccgtcggcgtacccacgatcagcgcgttgtattgcgagccgtcggcgcgctccacgacggcgaactggtaggccacgttgccctgggatacgtactgcacgagctgctccggcagccggtacgactccggcgaggtggtggtcaccccgacggacgactggaccatgatgacgggctcgtagacgttggccacgtccgagctctgctgggtgcgctgcgtcaggctcgcgcgagcggagtttaaccgggactgcagggacgaggtggcgctgctggactcgatctgctcctccaccaacacgcgggcgcggtcgatttccgcgctggcggcgtcgatcttcgtctgggcaatgcgctgcgagacaacggtggcaagtgtgaagccgagcaccagcatcaccacagtggagactaagagcaccgtgccgacgaagcgcagctgcagggaggtgcgccacgcttcggacatccgctcccccgcgccgcggagcgaacgggattccgccagcgctttcgcgttaggcaccctcggtctttcccgtcttgtaccccacgccgcgcacggtcaggatgatttcggggttttccgggtcgtgctcgatcttggagcgcaggcgctgcacgtgaacgttgaccaggcgggtgtcggtggcgttgtggtagccccacacattcgccagcagctcttcgcgggtgtgcacctggttcgggcgtcgagccatctccaaaagcaggtcgaactccagcggggtaagcgcgatctcctggccgtcgcgggtaaccatgtgctgaggcacgtcgatggtgaggtcgccgatgctgagcacctcggtcggttcgtcgtcggtgcggcgcagacgggcgcgaatacgggcgacgagttccttcggcttgaacggtttcgtgatgtagtcgtccgccccagactccaggcccaagaccacgtcgacggtgtccgtctttgctgtgagcatcacaataggcaccgcggactccttgcgaatctcgcggcagacgtccacgccgttcatgttcggcagcatgaggtcgagcaggatcaaatccgggttggaggagcggaacgccggcaccgcctcggcgccgtcggtcaccgactccgtttggaacccttccgcgtcgaggatgatggtgagcatttcgttgatggcggggtcgtcatccacgaccaaaatcttcggcggcatgtcggctccttactgctgctcgctacggcctagcgctttgtcgctctcgcgctgatggcatcgatgataaccgccggatcggcggtgaccagccactgactcgcccacgaccgctccgcgagcgcagcgtaggcggcgtacgtggcctcttggagcgcgaaatcgcgctcgtagcggtcgcgcgtgcgcgaatcgtcggcagcctcccggcgcgcggcgcgctccgcagccacctcggggctcgtgggcaccagcacttggagatccggccggggcaggctgaggcgctcgaactccagctcttcgacccaccgcacagcggtctcgtcgccggtgcgcgcccaggtgtaggccgcgttggaggcgcagtaccggtctaagatcaccgtctcgtccgggttacccgtgaagcggtcgagctcgcctttcaccccgtggcggtcgagggcgaagaccgcggccatgccgtaggccgactccgccatgtcgcccatttgcccgcgcagcgcggcctgagcgagctgagctgctgcggaatcctcgtagcgcgggaatgcgatggaggtggcgctgaggtggttcaacagcgcgtcgacaagcgtgtgcttgccggcgccgtcgatcccttctaccgcaatgatcatcgcactagtaccggtagtgctcgggcttgtaggggcctgcgacgtcgacgccgatgtactcggcctgctccttggtcagctcggtgatcgtgccgccgagggcctcgacgtggatgcgggcgaccttctcgtccagcaccttcggcaggcggtacacctcgttctcatagttcgcggagttggtgaaaagctcgatctgcgcgatcgtctggtcggcgaacgagttggacatcacgaacgacgggtggccggtggcgttgcccaggttcagcaggcggccctcggacagaacgatgatggcgttgccgctgggcagctcgaacaggtcgacctgcggcttgatgttggtgcgggtgacatcgtcgcggtgggtcagcgagtgcatgtcgatctcgttgtcgaagtggccgatgttgcccaaaatcgcgtggtccttcatgcgcatcatgtgctcgaaggtgatgatgcccaggttgccggtcgcggtgatgacaatgtccgcgtccgcgatcgcatcttcgacggtgactacggcgtagccgtccatcagcgcctgcagcgcgttgatcggatcggcctcggtgaccgacacgatcgcgccttggccgttgagcgcctcagccacgcccttgcccacgtcgccgtagccgcagaccagcaccttcttgccgccgatgagcacgtccgttgcgcggttgatgccgtcgatcacgctgtggcgggtgccgtagcggttgtcgaacttcgacttggtcaccgcgtcgttgacgttcatcgccgggaacggcagcaggccctccttggcgaagtggtacaggcggtgcacaccggtggtggtctcttcggtgacgcccttcacctcggcgccggtggtggtccaccgggtcgcatcctcggcgagcacctcgcgcagcatgttgtagaaggcgatctgctcgtcggagtcgccctcctgcggctgcggcacagcacccgcagcttcgaactcggtgcccttgatcacggccatggtggcgtcgccgccgtcgtccaagatcatgttcgggtacacaccgtcaccccagttgaacacctgccgcaggcaccaccagtactcgtccagggactcgcccttccaggcgaagaccggcacaccctgggggtcttcaggggagccgtgcttgccgacgaccaccgcggccgccgccgggtcttcagtcgagaaaatgttgcacgacgcccagcgcacctccgccccaagcgcagtcagcgtctcaatcagcactgccgtctgcgtggtcatgtggatcgagcccgcgatacgcgcgcccttcagcggctgctctgcggcgtactcctcgcgcagggccatgagccccggcatttcgtactccgcaagctcaatctgcttgcggcccgactcgtgcaggttgatgtcggcgatcttgaaatccgtcgttgccatgttcagtgtgcgctcctcaacagtgaatctgcttcttcacaaaccacaggccactgtagcgctaccgcccaacacggcggcgcgctaggacagcgcttcgatgaactggtcgatgtcggtgtccgaatcggtgtcctctgcggccgcctcgagcaccgcaacggccgattccgccagctggtcgctgatctcgcccgggttggagcggatgaacgggtacgcttcagcggcttcgccggcggagaacggcgctcccgcccagatcgcggccatcgtcgccgcggcgcggccgttggcgagctcctcgtcgctgggagcctcaccggcggcgagcaggacggcgtcgtgcacggcctcgaggatctcctcgggctccagatccaccagctcatcgaggaaatcgatgttcgcgtcgtcagcgaagatttcctggtcccacgtgctcaccttgtttcagctcctttgtgcgtagcgttccggctgtattaccggccacaataatttaagatccgcgccggacgtgttataaacgcgaacatagtgtcattccgcccaaggagccgcaatgagccacaaccagcgaggcattggcctgtttatggtcgcgggctccgtgctggccgtggtcattggactcgcggtgtggaacacttcaacgccgcagcgctccgtcaccgctggctacacccaggaagctgacgaggcggttggcagcgcggcgtatgtctcgtcgccgcagcgcacgccggcacccccgcagacccagccgcgcccgggcaagacagagagctcacgaagcgcggcgccgaagccctcctccaagcgcagacgcaccgcggacgccggctacgaccccaccgcacccgccggcgggacgggggacgaggctgccattcaagcagccccagcgccgggccggtaccgcatggaggatgacccgctggcgccgccgcacgcagtgacgtcgcagccgcctacggtgggcccgaccacgcactaccgccccaccaacgcgcggccggcggagcagcaggtgaccactgcgccggagcaaccgtccgcaccgcgcgctaccgcgccgacaccggcgtcgcagccgccttcaaccagcgtccctgagacccagagcccgcagacttcgcagccagcgcagcccacacaaccgacagaaccctcgcgcactgacgcgccgacgacgcccgccacctcaccggtagaaccgacgagcgcgccgcaggaacccggagacaaaaagacgctgacaagcggagaagcgcaaccaagcgctgaggccagctcggttgaggagccagccgccaccccggccagcgaggccccgagcgacgccgaatcagacgcggacgaggaaaacctcggcgggctcctgcccagctagctcaacaacgcacgcctcggcgctagcggggacccacaccgcagctcccggagcaatctcgagcccgcctaggcggatacgacccgccgtgcacaagacgactgcgggaccgtcgttgtccaccgcaagtgttgctcccccggcgagggggtgtcggctcacgcggaactcgtcgatcggcagctggtactcacacccgctttcgacctcggcggcggcgacgcgcgggtcgctcagcgccgtgaagtcgagcacgcgcgcaagttccggcacgtcgacgtgcttcgaggtcaacccgccgcgcagcacgttgtccgagttcgccatgacctccacgccgaggccgtgcaagtacgcgtgcggctgcccggccccgaggaagagcgcctcgccgggcgcaagcgtgacgtggttcagcatgagcgcgaccagcgcgcccacgtcgcccgggtaccgctcggacagctgcaaaaacgtctccgccacttcgaacatccagtctgccgccccgccggcgatgagctctcgggcagacacctcgacgccgccgagcagcgccacgcgcagacctgcaggcagcgagatcaacgtggtgaagacggcgcgaaggctttcctgcgggtcgtcgccgctgagcaacgcgctgtagcgctcgagcggaccgagcacgtcgaacagttcgcgggtgagatgcgtcggccggaacccggcgagcgccctaaacggcgtcagcgcgacgatgagttcgggtttgtggttcgcgtccttgtagttccggcgcggatcgtccaacgcgatcccctgctcgttctcccgctcgaaaccttcgacggcctgcgccttcgacgggtgcgcctggatcgacagcggctcgcctgcagcgagcagcttcaccaagaacggcagttccccgccggaggcgtccgccacccgcgcaccgagcgcggccacggggtcctcctcgatcacgtcgtgcagcgaacggccgccgacggtcgacggggccgcggggtgggcgccgaaccacagctccgcctcgggggtcggcgccggggactcggttccgcgcagctcggcgagcatggtgcgcgaaccccagggataggtgcgcaacgcgggctcgagatactccatcgggctgctccttatctccacatctcctccgccggcgggtcgaaggcggttacggcgtacgcgcgggtaaccaaccgcacgcactgggctaccgggccgaggcctgcgtcctcaaccgactcggcgcgcgtgttgggcgcggccgacgccgcctcggcggcagcgcccggcagcgcccacagaacggtcttcaacggtaccagctggaactcacccgcctggaactggtcgagcggcatctcttcgggcgcgacaaagcccgagacgaggccgcgcgccgaccatagttccgcggcgacggcggccaccgcacggcctacagccgtgctgcccaccaggccgtccacctcggcagcggaatgcgccaccagcgagtccgcggcgaaggcgcgcaactggcgggcagggttcaccgattcctcgcgctctggggagagggcggcgagatcgctatccacttgctcggcgatggcctccaagcgggcagccgcatctgccccgctgccggcaataacgtcgtacaccgcggtgactgccgcaatcgtgcgcgcgggcgagggacccgcggcggttggaagggcggggatggttgtggtggtggcgggggcgtcgttaagcaagggcccccgagcgggacctgcgaggagcacctcagccccgcggcctgaggcggtgatgagcgcgcgcgaatcggactcccgcgtcgcgcgctcgcccacgatcagcaccacgtcgagcgggccgacgtacgcgggcaactggtccgcaacacacaccggcagcttatgcggctcgcacagcgcgaccgccgcccgcgcaaccgccgccgcgagctggtccgttgcgatgaccaccagcgagcgcggctcgataccccccagccgctcgatctgaggcagcgcccccgccaccgcgcgcagctgcgcgccctcgtgggcgacgtcaaagaagcgaaccgtctcgcggtcgtagtggccggcaccggagtagtaatccatggccgcgagtctaggcagttacgcgcggataactccgagcacttcggcgaccagctcgtccaccgcctccgcggtcggagcctccacgttcaggcggagcagcggctcggtgttggaagcgcgcacgttgaaccacgccttagagtctttcagcgacacggtgaccccgtcgaggtagtccacgtccgaggcgcggtcggcgaaagcgtcgacgacgcgctgcatcgtcgcttgctggtcctccacttcggagttgatctcgccggaggcgacgtagcgctcgtactcagccatcagctcggacagcggcttgtcctgctccgccagcgccgcaagcacgtgcagcgcggcaacgaggccggagtccgcgttgaaaaactcgcggaagtagtagtgcgccgaatgctccccgccgaaaagcgccccccgctcggccatctccgccttgatgtaggagtggccgacgcgggtgcgcaccggggtgccgccgagctccgcgacgatctcgggcactgcgcgggaggtgatcaggttgtggatgatcgtcgcacccgagttctttttgagggtgcgcgcggcaatcagcgcggtaatcgccgacggggacaccggctcgccgcgctcgtccaccacgaagcagcggtcggcgtcgccgtcgaaggcgagcccgatgtcggcgccctgctcgggcgtgaagcgctgcaggtcaaccaggtttttcgggtccagcgggttcgcctcatggttggggaaggtgccgtcgagctcgaagtacagcggccggatgtccatgtcggagagcacagccggcaccgtcagccccgccatgccgttcgccgcatccacggcgattgtgagcggtcgcgtcaccggcaccagctcacgcaggaacgaggcgtaggcgccgagcacatcttgcttgtcgacgcccccctcaacacccgcatccgccccctccaactcaccggagagcagcagctcgcggatctcccccagccctgtgtctgtcgacaccggcgccgcccccgcgcggcacagcttgatgccgttgtactgcgcagggttgtgcgaggcggtgaacatcgcgcccgcgcagctctgggtgccggccacgaagtacagttcgtcggtgctggtcaggccaagtaccgtcacgttcagaccctgggccgcggcgccgtcggcgaacgccgccgccaactcgggcgaggacgggcgcatatcgtgaccgactgcgatccgggtctccccctcgcggcggagaatgtgcgcgaacgccgcgcccacctgccggacgaaatccgcatccaccgtctcaccgacgacgccgcggatgtcgtacgccttaattactttgctcaagcgctcgctggtgtaaaccatgcgggaaagcttagctttctgcctcgccttcaccgctcgacgggtcgggcaccacacgcaagtgggagcggcgcgccgcgcgctgcgctgccgcctgctcctccacgcgcttcgtgcggtgcaccgggtggttggaggttgccgggtcgttgaagtctttcgatggctggtactcgatcgggtcctgcgatgtgtccaccagcccggtggtcacccggcccgcctcgcgcacagcctcggcaagcgcggtgaggtcggactcgtccatggcgtcgaactcttcatcggtgatgtcgacctgctctacacgcaccatctcccagccgaccggggcggtgatgtgggcagagtggcgctcgcacaggtcccaggcgtgcggatccggcaccggcgctagcgggccgaccacagcggtggactcggcataggcgtagacgagcgtggccacagccggccggccgcagccgggcctgcaacaacgtcgaaaagtgctcacggcgcctaagtctaaacccctgcttgagttttcggggagtagcacgcggcgcgccccgactacctgtacgcgcgcgagccctactatctagccgtatgcgcaccgattcagctagccccctgcacctgcgtccggggcgcgaccgccacggccgcggcgcccgcggaccgctcgtgcccgtcggtgtcccccgctaccgcagccggtcgatggccttcgaccaactcgttttagagatgtacgcaccgctccacaacgcctacttcgaccagctcaccggcgtggatctggcggtggacatgattccgcggatgcgtctgcgcgcagacatgacggtgatgccggaagagatcgtcgccgatggccccgtgccgctcggccgcgtgctggaggctggtgtggaccgcaacggcaaccccacccgcgccaggttcgtcgtcttccgcagtcccatcgagcaaagagcccgctcgggagaagagcgggctgaacttcttacctgggtgctcactgcgcttgtcgcgtactacctcaacatggacccgcgcgacatcgacgaaagtttcccctggtaagtgctagccgagctgcttcttcaggcggcggcgctcgcggtcggagagcccaccccagataccgaaccgctcatcgtgctcgagggcgtactcgagacactcatcgcggacagcgcatgccttgcagatacgcttcgcctcgcgggtggagccacccttctcagggaagaacgcctccggatcggtctgcgcgcagagggcctgatcctgccattcctgctcgacggtgccgaacaactcatccagcgtcatgccccccacggccgcgccgcggagaaatgcgtcgtctcccatactccacgccctcccttcctccgttgtttttcaggtctgccggtcatccggtggattacacgcttgcgattcaacacgcatccactaaatagccgcaacctcgcccgcccgatcgagcacgaaaactatggttcccccagcgcgctagtcacaccagtcacacgcgtttcacccatgcgccttcaggggtagtcggcgggggtactacatctggtaggcacccccgccgaagttaactagtttggcgattcggcgtgtcgcttatgcatccggcgaaaaacgcacccccgaatctgggagttccacgcccggccagacgcgcatgccgccctcgagttcgcagcgggcgccgatgcgcgcgccttcgccgatgacgcaatccttcagcttcacgttggcgccaatagtcgccccggaggcgatgattgagttccgcacgactgcgcccggttcgacggtgacgccgtcgaaaatcacggagtcgtcgatacgcgagcccgcgccgatgaccgagccgcggccgattgccgtaccccccaccaagatcaccccggcggcaacgcccgcggacgggtcaaccagcgactcgccggtcttgccctcgagcagcggtgagtgggcaatcccgcggaccaggtcggacgagccctgcacaaagtcgctgggccggcccatgtcgcgccagtacgacgagtcgacgtggccgaggacccgggcgccgtcggaaagcaagcccgggaacacctcgcgctcgacactgaccacccgacccgcggggatctgctcgatcacctcgcgcttgaacacgtagcagccagcgttaatctggtcggtcggcgggtcctcggtcttctccagaaacgcgagcacgcgaccgtcctcgtccgtcggcaccgagccgaaagcgcgcgggtccggcactcgcacgaggtggagcgtgacatccgcgtcgccctcgatatgcgtgcgcagaatcgcggtgaggtcagcgccggaaagcacgtcgccgttgaacaccatcgccgtgtcgtagcgcagcttgtcgtgcacgttgcggatcgcgccgccggtccccagcgcctcctcctccaccacgtactcgatctcgagcccgaagtcggtgccgtcgccgaagtactcctcgaacacctcggcacggtacgacgtcccgagcaccacgtgcttcattcccgcggctgcgatgcgggccagaaggtggctcaagaaggggtagttggctgtcggcagcatcggcttcggggtcgacaccgtcagcgggcgaagcctcgtgccctggccgccgacgagaatgacggcgtcgacctcggctgggtggacctggcccgaggcctggtgtgcttgctcaaccatgctgcttccttttgtctggtagttacccgcgagcgagcgaaaccgcgctgcgcactttcagtccgagccacaatcccgcgcggatcggggcttgccaccagtgcgggtggcgatcgcgctggaaacggtacgcggaggcgtggtgcgccggcacggtgacccggctgtgtttgccggccacgtggccttgatcgtggaagatcaccgacgacgggcagtagaagttgtcccacccggcacggctcaaccggtcgccgaaatcgatgtcctcgaagtacatgaagtagcgctcgtcgaacccgccgacagcgtcgaacgcgtcccaccgcactaaaaggcacgcgccagagagccaccccgcggtgcgctgggtgtccatgtccgcacctttcttataggacgcggtaaacgggttcgacggccagatgtcgccgaacagcgcgtggccgataccgttgatcagcccgggcacctgccgcgcactcgggtacgccgacccgtcggcctcctcgatcctcggaccggtcgcgccagcgccgctcgcatcggcgcactcgagcagcttgtctacgctgcccggcgcaagctccacgtcggggttgacgatcaggaagtagtcggggttcaccgcgccgcgggcccgaagagcttgcagcttgccgacacccacgttaatcgccgctccatacccaatatttccgcccgtgggcacgaactcgacgttgtcgtgctcgcgcgccgccgcctgcggcaccccgtcagtggaaccgttgtccgcgcagacgagtacggtgcctgcggatgtcgctgccttgagcgacgagatcagctgaccgaggtggcggccgggcgaatacgtcaccgcgaccacggccagaggtgcttctgaggcggggccgcggttgctgtcaaggtgcaaagcgtcgatcacaatgcgggatagcttacccagcgctgcatgtcagcccgggcaggcgcgcgcactatactttccggctgtgacggacaactcccgcaaaggccaaccccgccgcgcgcgcagcatcgcacccgcgccgtcgcgtgcgcgcgacgtgagccaagcgggccacccggcggcgaaggccgtgctcgcctttttctccgccgccaccctattggtttccggcgtcgggtacgccaccgtcggccgcctcggcaaccagctcagcgcctcagaactggagatccagaccccgaagcgcgggggcaagggcgccaagaagcaagcgcttgtcgacggcgcggtggacatcctccttgtcggctccgactcccgcaccgacgcccagggcaaccccctgtccgaggaggagctcgcccgcctcaacgccggggtgtccgacggcgagatcaacaccgacaccatcatggttgtccgcgtacccgaagacggctcccgcgcaaccgccgtctctatcccccgcgacacgtacgtccacacggatgacttcggcaacctgaagatcaacggcgtctacgccgcccacgcggagaagcgccgcgaggatctggtcgccgccggcatgtcgcagggcccgcaacttgagcagcaggttgcccgcgccgggcagctgggtttgatcgaggcggtcgcggacctcaccggcgtggaagtcgaccactacgcgcaagtgggcctgctcggcttcgcgctgctgacagacgccgtgggaggagtcgaggtctgcctcaacaacgccgtcgacgagccgttgtccggcgcccacttcccggctggccggcaaaccctcgacggggcggaggcgctttcgtttgtgcgccagcgccacgacctgccccgcggcgacttcgaccgtatcgtgcgccagcaggcgtacatggcctcgttggtgcagaagacattgtccgcaggcacgctcaccaacccggcgcgcctgcgcgacctggccgcagccgcagagcgctccgtcaccctggaccagggctgggacattatggcgttcgcgcagcagatgtcggggcttgccggcggcgacgttacctttgccacgatcccggtgacctcggtcaacggcgtgggcgactacggtgaatccatcgtcaccgtcgacatcggccaagtgcaccgattcatggaggaggccgccaacccacctgaggaggagacggaggaggattccactgccgcatcggagtcagcgccggctgctgcggtgtttaccagctacgaggcctacgttctcaacgccggggcgcgccctggacaggcgggtgctgtgggcacgcaccttgagaaggaaggtctaactgtcgccagcgtctcgaacgccctggacggcatctactcgacctcccaggttgtagccgccgacccggcagacccggcggcggtggagctcgcccgcatgctgggcgggctgccaatcacctccaacgaaggactcgagccgggcagcctgatcgttgtggtggccgacgattacgacggccccgccgccatcgaggaagacggcggcgcggacgggactgaatacgccgagccgatcggcaccccgggcgaagacttcggcgccgcggagatcgcgcccgagttcaccgcggagggaacgggcccgcgctgcgtaaactaattgttctacgctgggcaggcatgagtttgcttcaaccgcttctcgcatccgaccccgcctcgccgcgcttgacggtgtacgacgaggaccgcggaacccgcatggaattttccgcgcagacgctggacaactgggccagcaaggtcgccaacatgctcgaggaggagttcgaccttgcagccggcgataccgcgcttattgatctcgcgcccagctggcagtccgccgtgatcgccctcggcgcctacaacgcgggggtgaagccggagtttgcggtgaagggagacgcgacggcgtcggcaagcacctggcccgtcgtctttacctcccctgaacgggcggagcagtggcctgccaccccggatgtcgtggtggtgtcggacgacccgtttggccgcggcgtggaggaagcaggtggcgcgctgcccgcgggcgcggtggacttcggtcccacggtgcggttctacggcgacgcctacttcggggactcccccgatctcgggcagtttacccgcaccgggtacggaccccaccgctacctgtcggcaccgtggagtaccgcagcgcagttcgaggagcacgttctcgctccgctggcggccggcggttctgtcgtggtagcgacggggctgataccggccgagcacttagaccgcatctcgcaggcagaaaaggtaacgcacttcttaactcaaggttaagtcgccagatccacccccatatttgggtaaacaccaaaaatggcggttctcgaatcttttgggttctacattgttagtcacctccgatctgacttgtgatccgaaaggccttttgaatgaaccgtcacgcaacccgcaggaccggcgcggccatctgcgcattcgcactgtcctccaccgcactggtggcttgctccaacgatggcgacaccgccggcaccaccaacgatgagaccggcgcaacaaccgccgccgcgagcgacgctgcggcgagcgacgccggcgaagaccgcggccccatcaccttcgccatgggccgcaacgacaccgacaagatcatcccgatcatcgacaagtggaacgccgagcaccctgacgagaaggtcaccctttccgagctcgccggcgaggccgacgaccagcgcgacaccctcgtgcagtccctgcaggccggcaacgccgactacgacgtgatggcgctcgacgttgtctggaccgccgacttcgcggcgaaccagtggctggaaccgctcgagggcgactacgccgtcgagacctccgacctgctgcagtcgaccgtcgactccgcgacctacaacggcaagctctacgcgctgccgcagaacaccaacggccagctcctgttccgcaacaccgacgtcatcccggaggcgccggacacgttcgccgatatcaagtccgcgtgcgaagcaatcgagaccgactgcctgaccacacagctcaagcagtacgagggcctgaccgtgaacacgctcggcttcatccacggctggggcggcgaggtcatcaacgacgctggccagccgacgatcgagtccccagaggcgaaggccggtctgcaggcgctggtggacgcgtacgaggacggcaccattgcgaaggcctccaccgcggcaaccgaggaggagaccaacctcgcgttcaccggcggcgagaccgcgttcgcgatcaactggccgtacatgtactccaacgctgaagaggctggcgtcaacttcgaggtgcagccgctcgttggcgagaacggcgtcggcgcttccaccctcggcggctacaacaacggcatcaacgtgaactccaagcacaaggcaaccgcccgcgacttcatcgagttcatcatttctgaggagaaccagctctccttcgccgaagcttcgttcccgccggtgcttgcctccatctacgacgacgcggagctgatcaaggaccacccgtacctcccggcactcaaggagtccctggagaacgcgaagccgcgcccagtttccccgttctacccggcgatttccaaggccatccaggacaacgcgtacgcagcgctgacctccggcaagagcgtcgacgacgcgaccaaggacatggctgcagccatccagcaggcgcagtagttcacacgcctcattgctaaacgctcacgcccgcgcggtttagaatccgttgcgggcgtgagcccatttctccccacgtgcaacgagaagggcgcgtatgagcaccgttacccagaagaagcagtccgacgtaggtaaggcctacggcttggtggctccggcactgatcgtgctcgccatcgttatcggctaccccatcgtccgcgctatctggctgtcgttccagtcaaaccgccacctcgaccccaagacgggcgtcttcgtcgacggtgggttcgcgggcctggacaactacttgtactggctcacgaaccggtgcatgagcccctccggggtggtgggctcctgcccgccgggcgttttgagcaccgacttctggccggcagtgcgcatcacgctcttcttcaccgtggtcaccgtcgcgctcgagacgatcctcgggttggcgatggccatgatcatgaaccacccctccaaggtgcgcggcatgatccgcgccgcggtgctcatcccctgggcgatccccaccgctgtcaccgcgaagttgtggcagttcatgttcgcgcccaacggcattgttaactcgctgctcggccagagcatcgcgtggacgacggacccgtgggccgcccgtttcgccgtcgtcatcgccgacgtgtggaagaccaccccgttcatggcgttgctcatcctcgccggtctgcagatgatcccgcaggacatctacgaggcagcacgcgtcgacggcgcaaacgcgtggcagcagttcacccgcatcacgctcccgttggtgcggcccgctctcatggtggcagtgctcttccgcaccctcgacgcgctgcgcatgtacgacctgccggtgatcatgatttccgggtcctcgaactcgcctacagcaacgatctcgcagctggtggttgaggacatgaggcagggcaacttcaactcggcatcagcgctgtcgacgctgatcttcctgctgatcttcttcgtggcgttcgtgatgatccggttcctcggcgcggatgtcggcggcgctgtgaaggaagaagggaagaggaagaagaaaaggcggcgtcgacaagcaactgctcaagacgctgaaccgctagacgcacgactgtcggaggctgcgcgatgaaaaaggtaggacacttcctcggtgtcatcttcatcatgttctgggggctcgccccgttctactggatgctaataacggcgctgcgcgacaagcgctacaccttcgacaccacgccctggccgacgcacgtgacgctggacaacttccgcgacgcgctcgcgacggataagggcaacgacttcctcggtgcgatcggcaactccctgatcatctccgtgagcacgactgcgctcgccgtcctcgtcggcgtattcacggcctacgcgctcgcgcggctgaacttccccggcaaggggttcatcacgggcatcatcttggctgcctcgatgttccccggtatcgccctggtcacgccgctgttccagctcttcggcgacctcgggtggatcggcacctaccgcgcgatgatcattcccaacatctcgttcgcgctgccgctgacggtgtacacgctcatctcgttcttccagcaactcccttgggagcttgaggaagcagcgcgtgtcgacggcgcgacccggggacaagcgttccgcctcattctgctgccgctggcggcgccggcgattttcaccaccgcgatcatcgcgttcatcaccacgtggaacgagttcatgctcgcccgccagctgtccacaaccgcgaccgagcccgtcaccgtcgcgatagcccgcttctccgggccgagcgcattcgagtacccgtacgccgcgatcatggctgcgggttctttggtgacgatcccgctcatcatcatggtgctggtcttccagcgccgaatcgtctccggtctcaccgccggcggcgtgaaggggtagccagtcttcggctggcgggctcatgccgctggctacaaccagctggggtctcggtgcgctacgcgccgagaccccaagattatgcgcggcataatcacccgcgcacctgcgcgaccagacggcgccacagtacccgggccaaggagtggggcaccgcgatgagttcgcgcgagtagttcttgatcttgctcttcgggtacccgggcggcatgggggcaccgaccaggtcgacggggatgcccaggtgccacgcccagacagcggtgcgagcgacgtggaagttgctggtgaccaccgtcaaccgcgcggcatctgggaaaagagcgcgggcccgctcgagattttcgttggtggaggtggcgtgcggttcaactacgatgtgctcgaggggaacaccccgctcggcaagccataaggccatgacctcggcctcgcctcgcccgctcaccacaatggggcggggtgcggcgttgtaaatcgacagcgctgaggttaaccgggaggcgagcatgcgactggggcggccgtcgataatccttgccccgaggacaacgatcgggttcaccaattagtcgccgagcaggcgctggcggagcgcgtcgtccttgcgctcgacgtcggcggcgaggtcggcctggtaggtggccatcttctccaccagcgcgtcgtcgcccgcgccgaggatgcgcacggcgagcaggccggcgttcttggcaccgccgatagacacggtggcaacaggcacgccgcccggcatctgcacgatggagagcagggagtcgagaccgtcgagatccgcaagcgcgcgcgggatgccgatgaccggtagcggcgtggcggcggcgaccatgccgggcaggtgagccgctcccccggcgcaggcgatgatgcacttcaggccgcgggtgtgggcgcttttcgcgtacgccagcatcttctccggcgtgcggtgggcggacacaacgcccacctcgaagcgcactccgaagtcgcggagcacctctgcggcaggcgcgaccgtgtcccagtccgaatccgagcccatgatcaggccaacaagcggttgcatacctcttactcctctcctgcggcgctttcgtcgcgccacgtcgcgttcacgatgaagtgcgcggcatcttccgcgacggcgcgcgcctcgaccaccgtatccgcggcgacgttgacgtgacccatcttgcggcccgggcggtggcccttgccgtacaggtggatctttgcctgcgggtagcggcgcatcacctcgatcacgcgctcggccatcggcatctccggatcggtgtcgccgccgagcgtgttcaccatcacggtcaccggcgccgtcggttccgtcgcgccgagcggccagtccagcacggcgcgcaggtgctgctcgaactgcgaagtcacgcacccgtcctgggtccagtggccggtgttgtgcgggcgcatcgcaagttcgttcaccagcagggtatcgccggtgacgaacagctccacggcaagcacgccggtcacgtcgagctcctgcgcgatgcgggaggccagctcgcgggcttcgcgctccagcttctcgtccaagcccggcgccgggctgatcgccacgcggcagatgccgccgtcctggatcgattcgaccaccggccacgccgcaatctggccggtgcggccgcgcgccaccatggcagacagctcgcggtcgaacggcaccttccgctcacccataagtggcaggtccagctcctcaaccagggagagcagttcgcttaacgacgcagggaaccacacccccttcccgtcatatcctccccgggtggccttcagacagacctgcccatccacctgctcccagaacgcctccgcgtcctcggcagtgttgatggcggcgaactccggcaccggcgcccccagcgcgttgaggcgctgacgctgctccagcttgtcctgggcgtagatgagcgcagacgggcgcggctccggatcgaggtcgttgtcgatcagcacctgcaggtgctcgttgggcacgtgctcgtggtcgaaggtgacggcgtcggttccttcggtggcggcttccaaatcctcgagcgaggtgtaatcgcccaggcgggcgtcggcaatcacctgcgccgcggaggcctcgttgcttcccgccagcacgcgggtctcaatccccagctcgatggcggcagtctgcatcattcgggccagctgcccgtcgccgatgatcgcaaccaccggcatcccatacgcgttactcactcccaacactgtagtcgcagttcgaagtaccatcgcacccatggctgaaactatccagcggcacacgatcttccagaattcgctgatgaccgccctgctcgacgggatctacgacggagagctgaccatcggcgagatcctgtcgaagggcaacttcgggctcggcacgttcgacgggctggacggggagatgctgattatcgacggggtgtgccaccagctcacctccgacggcaaagcccgcgtcgccggcctggagcagcggaccccgtttaccgtggtgacgaacttcgtcccgcggatccgcgtcgaggccccgcggggcatgcgccgctccgagctgtccagcttcatcgacagcgtagagccgagcggcaactacttcaccgcagtgaagatcaccggcacgttttcccacgtgtccacgcgcacggtgagcaagcagttcaagccctacccgccgatgtcgcaggcggtgggcgacgatgcggagcacaacttcaccgacgtcagcggcatcatcggcggcttccgcacaccggcctacgccaagggcatcggcgtgccggggtgccacgtccacttcgtcaacgacgaccgcacctcgggcggccacgtgctcgactacaccgtggacgacgctgtcatcgagctgtgccccggtaccgacatggagctgcacctgccgatcaccgcggaattcgcgggcggcaacctcgcgccggaggacttggacgaccagatccaccacaccgaggtgaagaactaggagttgatgatcttctcgacttgcttcggcttgcccacctggtcgaagaaaagcggccgctcgaagccgtagaccgaaagcgagatgccgccgccggacttgcgcgcagaatggatgtgctggcgggggatagaatcaaccgcgccacgcgggccgcgcgagagcacgcgccggtctgtgaccacgaaccggcggcgccgcgcgcgcgaaactggcacgataaagcgccagatcaccaccagcacccaccccagcacgacgaggttgcgcaccagcgggtcgagctcggtgttgacgtcgaaccagccgatcgcgatccacaccacgccggtgaccactaccgcttccagcagggggaagaccaacgtcgaaatcggcgcgctgacgtcggcgaggactacctcgtcctcgccgactgcaaagtcggcctgcctcgccactacgcttcgctcgggcggaggtggtggacgtcgccgacggcgtacggggtgccgtcgataagcaactcgccttggtcgttgatgccgtcgacggtgccggtgacttccccctcgtcgtcgctggtgcgcagctccagccgcacgcgctgaccgatggtcgcgcagaccttgcggtaatcctcgagcagctgcgggtcgccctcgcgccactgggtgaggcggcggcccatggcgttgaggatgtcgatggtgaagtcgtcgaagtcgacgtcgatgccctcgaggttgagtgcggtcgcggtctccacaggcaggtcttctgggcgcatcgccacgttgatgccgatgcccacaaccacccgcggcatgtccaggccggagaggatgccggcgatcttcttgccgcggatctgcacgtcgtttggccacttcagctgcgcctccggcaccacgtcggtgacggccacgcccggcgtaatggacagaaggccgaagtcgcccgggtgctccgaggcgtccagcaccatgctcatggccagctgcgatcccttcggcgtgacccactggcggcccaaacgtcccttggcgtcggtctgctcgtcggcgatcagcaccgtgcccggctcgccctcgcgcagcatgtccgcgttggttgaaccggtcgattcgacccaccgcacgtccggccagtactcggcgacggcctcctgcactgcctgcacatccttgatgctcatgggcactaagcctagcgccgagcacacccgcaacgcgcgtccccgtttcagcctatgctcggatttgtcccataaccccgagcacataggtaaaggtcatggcaaattcagaagcttcacagcaagagcaaaacgcgcaagatccgaagccgtcggtcacccaggcatccccggccggtgacaccgtgtccggcgcaccagcaggcgcggacaacccgtctgaggccaccaaggcccccgaggccgtcagcgtcaacggctgcccgttccactttggcgcctccgaaccggacccgcgcgcgcagcagggcgagtacctcaccacctcccagggcgcgcgactgagcgagacgtcgaagtcgctgcgcgccggcgagcgcggcccgctgctggtgcaggacctgcacttccgcgagaagatcacgcacttcgaccacgagcgcatccccgagcgcgcggtgcacgcccgcggtgtcggcgcccacggcgtgttcgtggccaacggtaaggcagaaaagatctccaaggccgccgtgtttaagaaggacaaagagaccccggttttcgtccgtttctccactgtgctcggctcccgcggctccgccgattccgtgcgcgacacccgcggctgggccaccaagttctacaccgaagagggcaactgggacctcgtgggcaacaacatcccggtcttcttcatccaggacgcgattaagttcccggacgttatccacgcaggcaagccgcacccggaccgcgagatcccgcaggcgcagtccgcgcacgacaccttctgggacttcgtcggcctgcacaccgaggccacccaccacaccctgtggaacatgtcggaccgcggcatcccgcgctctctgcgcatgatggagggcttcggcatccacaccttccgtttcatcaacgacgccggcgagaccacgctggtgaagttccactggaagccgaagttcggcgtgcactcccaggtgtgggaggaagcgcagatcaccggcggcatggacccggacttccaccgccgcgatctgtacgacgcgatcgaggccggcgccttcccgcagtgggatctcggcgtgcaggtgttcccggacaccgaggacgagatgttcgagggcatcgacctgctcgacccgaccaagatcgtgccggaggagctcgcaccggttgagatcatcggcacgatgacgctgaacaagaacccgcgcaactactttgaggagaccgagcaggtcgcgttctgcccgagccacctgcccccgggcatcgacgtcaccgccgatccgctgctgcagggtcgcctgttctcctacctggacacccagatctcgcgcctgggcggcccgaacttcacccagctgccgatcaaccgcccgcacacggcagtgaacacgaacttccgcgacgcaatgggccagcagggctcccacgtcggtgtggcgccgtacaagccgaactcgctcgacggtgggctgccgaaggaagcgacggttgaagagggtgcgtttatcgacgtcccgcgccccgtcgaaggccagatcacacgtgagcacccggtctccttcgacgaccacttctcgcaggcccgcctgttctacatctccctgaccgatgtcgagcaggagcacctcacccaggcactgtctttcgagctgggtaagtgctacgaggaggcggtgaaggtccgctacctcgacgtgctggcgcacgttgaccaggatctcgccgagacggtggccgacaacctcggcctgccgcacccggagaagcaggaagtggccgacgttgagccgtcccctgcgctgtcccagacgggcggcagctggcctatcgacgcccgccaggtcgccatcctgatctcctccgagctttccggcgacgacgccgaggctgtgggcaagcttgtcgacgacctgtttgccgccggcaccaccccgttcctggtctctgacaagggcggcaaggtcaccgtgggcggcaaggacgtttcggtttcccgcacctacctgacggcgagctcgatcgagttcgacgccgccgttgtggtcaacccgccggcgaacacggacgtcaacaccatgctgggcgagttcgagcgccacaagaaggcgatcgctgtggtgggcgcgtcaggcgcagcggccctggaggcagcgcgcgtggatgcggaccagccgggcatcgccgcagtggacaccgctgacgcggctgcagcccccgtgaaggacctgctggccggccaccgcgtctgggaccgctagggcgcgctagacccgcgctagacccaagtgcggaacacctgaatcccgccgcctgagccgaggacgcgcgggtcgatttcggggccgatgtccatggggatgagcttggacttgtccggcaacccggtggcctcgaaatcttctcgcgtctggtcgtcgaacaccaccacgaagcgggcgcccggcagggcgttgatgccgtcgagcagcgtcatcggcatctgcgcgtcgaagtcttcgccccacccggcgggcacgtaatccttcacatcgcgcggcagccacgcgtcgatggtgttgacgatgtggatggctgcgtcgctggtcatgtcctcgttcagcgtctccgcgagcttggccaggtgcttcggcatctcgtactccgggccgaagaggcttaagacaatgagcgatgggtagagctcgtcaatcacgctgcggcggtaaataccgtcctccaagaaccgcttgctgccggccacccagcacagctgcttcgcgtacgcgagctccgtgtagaagtcgatgggaagctcgccgcggcgttcagtggtgtacatctccaccgcctcaccgagcgtgcgcagcaggtggaatgcgtcgcggttcgtggtgaagcggcagaccaccgtcttgtcgtgcatgaggctttgcaccgtcacgcggttctcaagcgtgccgtcggggaacatgggcgcgggcaacaccatgcggccggtgacgttgaaatcgtcatccgtcacgtcctcgtcgcccaccatgcggatgctgacggcggtgtggtcggggatgcgggtggcctggaaatcttcctcgctctgacggtcgtccacaatcacgcggtgcggcgtgtaccccgcatccgcgtaccgcagcggcatccacgtctcgatgctctccacgaggtcggagacgcgcacgtagtcgaagttgcctgcctcggcctcacccagcctggccaagtggtacgccatggcgaaacgcgggtcccaggcagcgagcacctccaagttgctcgctgcgtggaagaggtactccttaatctgcttcgcggtcgtgtcttctgaatcgcgcgccaagtcgagcacctgcagcgtgttagctaagaccgcgtacgcgtccagcgactcgttgcgggcgtcttcctccggctcgtactccgcggtgaggtccatcaggtgctcggtgagcgcccgcgcgtactcgaggtgttcttccgtggcgtacccgccgccgcgcggacccacagagatttcagcctcgaggtcgacgccgtggatggtggtggaaaaagacagttgcttcgcagtcatagcgcctccctgggccatgggttggtggtcgttggtttacgcgttcaagtataaatttgagctctacacgccctttggctttctcgaacgggtggtctaactacggttgatggctgccggactactctggaggaatgcagttatccccccgcttcctcgtttcactgctggccggcgccggcgcgctccacttcatcaaaccggaaccgttcgatgacatcgttccgccgtccctgcccggcaaagcccgcatgtacacctacgcctccggcgccgcggagctcacggcggcggtgctgctggcctctccaatcctcggcccccgcagcaacgcagaccaccgccggcgttccgctgctatgcgacgagcgggcgggctgttctcggccgcgttgttcactgcggtttggcccgcgaacttctacatggcctggcagtggcgcgacaagcccttggcgaagaaggcggtggcgctgggccggctcccgctgcaactaccgctcattcgctccgcgtggcgtgtgtacaagcgtggctgaccaggatgtgaccgctggcgacatcgaggcggcgaccctcggtcttctcgcgcaacgcaagcccgagtcttccatctgcccctccgaggccgcacgtcacttgtactcggctgacaccgtggcgcgactacatggacgacgtgcgcacggttgccggcaagcttgcgcagcaacgtgttgtgagaatcacccaaggcgacgatgaggtagatttcgccagcgtgaagggcccgatccgtatccggcggggcctggactggcaggagccgtaagtcggaaaacgtttcggcccgatctacacttaagccctatgacttcgaaacccgacttgaccaccacagccggtcgtttagaagacctccgcaaccgcctcgatgaggcgcaagctccggttggtcaggacgctgtcgacgccgtgcacgccgccggctccgctaccgcccgcgagcgtgtggagcagctgcttgatagcggcacgtttgtcgagaccgacgcgctcgcccgccaccgcgtcgaggcgtacaagatgtaccgcaccaagccggccacggacggcgtggtcacgggttacggcctcatccaaggccagcgcgtgttcgtcttctcccaggacgcgacgatttttggcggcgcgatcggcgaagtctacgccgagaaggtcctgaagctgtacgagctggcgacgaagaccggcgtgccggttgtcggcatctacgactccgccggcccccgctaccaggaaggtatcgtcaccgcccacatgcaagccaagatcctgcgggccgtctcgcaggcctccgggctggtgccgcagatcgcaatcgttgcgggtgacacctcctctatcgccgcgacgacgatcccggtcgccgatttcatcatccaggtcgagggcgcaagcgtcgacgccgaggcgcacctgaccaccgcgaccgacacggaggcgattgagcaggcccgcgcggttctggggttcctgccgcagaacaacctcgccgcctccccgctgggccaggctgacggcggcaacggtgcggacggccccgatctcgatgtcttcatgcccgacaacgacgacgaagcctacgacatgcgcgacgtggtcaacgctgtcaccgacggcgacttcctcgagctcggcgcggagcaaggcgggagcgtgctgaccggtttcgcccacgtcgccggccgcgcagtcggtgtggttgccacccagccgaaggtaaccggaggcaagctgagcgcagacgccggccgcaaagctgcccggttcatccgcacctgcgacgcttttaacgttcccgtgctgcagtttgtggactgcccggggttcgcggacgaccaggcgctgagcggcgctgccgcgctcgcctacgcgttcgcagaggcccaagtcggcataatcactgtcatcacccggaaagcgttcggcgaggcgtacatggtgctcggttccaagggcctcggagcggacttggtcttcgcctggccgaccgcgcagatcgcgctttcggacgctgccacggctgccgaggcgatcggcacagacaccgccgagtacgaggcagagaatctgaacccctacgtcgcaactgagcgcgggctcgtcgacgcggtggtcgagccgtcgcacacccgccgccacgtgctcgaaggcctgcgcctgctcgagcgcaaggtcgtctacccgccggtgaagaagcacggcaacatcccgctctaaggagaacccttcaatggatatcgaagtgacgaagggtaacccgagcgcggacgagctcgaggccctgtcccagctgctcagccagctgcacaacgaggcgacgaagtcccagaccccggctgaccggaacgcttggggcgtcagccgccccggctaccaccaatcgccgctctacaacccgcacgcgttcggcagcgccgcatactactaaaaagttatggctggcaaaggcgtgcggttggtgttggcgtcgaagtcgccgtcgagaagcatgctgcttacgcagggcggtgtggaaccggtactgcggccctccgacgtcgatgaagacgccgtcatcgcctctatgcgcggggtcgagccggaggacgtcgtcgcggctttagccagggcgaaggccgctgctgctgccgaggagtttcccgaggatgtcgtggtggggtgcgattcgatgctgctgcttgacggcgcgctactcggcaaaccccacaccgtcgagcgggccattgagcggtggaaggcccaacgcggaaaaaccgcgcgcctgctcacaggtcacgcggtttcataccggggtcagtgggtggtggacaccgtcgccaccacaatccgcttcggggaagtctctgacgcggatattgaggcctacgcccgttccgggcagccgctggaatgcgccggcgcattcacactcgaagcgctgggcagctggttcatcgactccatcgacggcgaccccaccagcgtcatcggcctttcgatgccgctcttgcgccgaagcctttactcgttcggcctcgacgccagcgacttctgggcttaggccttgtccttttcgtactccaccagcttggaggtgttctgcgcggtcttcaccatcgccacgtagaactccagaccgatacgggcgaagaccaacgccagaaacgccactgcggtaccgaagatgaggtaaccgaagaggaagaggaaaccggtgccaacgccgtcagcaaagccggagaaggaagcgaagaggccgacaacccagcctagtgcgatgaacgccagcacgattgcgtagatgaccttgacaaagtcaatcgtgatgtagcggctgaaggagaagtcgaacagcgccttgaagaagccgtcgcggtcgccctttcccactttgcccggctgctggaacccgccctgcggagcgccgaactgcgccggctgctggtactggccctgctggtattggccctggtactgcgactgcgagtagtcgttttgaccgtactgggtctgcgcgtggccctgattctggccttggttctgcggcgggtactggccctgctgcgcgccgtactgcgcctggtactggtcctgctgctgaggttgcgaaccgtaaccggactggccgtagccggactgggagtaatcaccctgcgagtagtcggactggccgtactgcggctggccgtactggttgtaggactgagcctgaccgtagcccgactgggagtagtcggactgcgagtaatcggactgcccgttctgggattgcgcgtgggactgcgcgccccacgggttgtcctcgttcgacgagctggagctggaacccgaggtcgaagcggaggacgacgactcactggtgccccactcggaagatgacgcggcgtcgcccgtgccccactcggacgcagactcgctgcgggagaagttggtggtcggttccgaggactccgcgctgcggtcggtcaggtaatccggctggtcgttgttgtcgttcgaacccgtcgggttgtacggcgtagacatgtgctgtctccttacgtcttccgttaatgatttcggtacccaactgtagttggtggacagtaaggctgcctgtgctgcgcatctccgtacaccgtgcgcaccgtgtagacggcgcgcacggttctgcgcggcgcaagattatgcgaggcataaaacggtcaggttgaggttgagactgttatgccgcgcatacaggccgcgcatagtcccctttgcgcggaaaaaggcccgctgacacagtctccgggaatctcacccgaagctgcggtcagcggaccaataaacaggcgctagtaaagcggcgccaacttacgcgtgcttctcctcaacgcgcttgatagcctcatcagccaccatctcctggatgcccatgtcgagctcggaggtgaagccgacgcaggagcagttgatctcgccgaggacgtaggtgtcctcgccggtctcatcgtcgtcggcgagcatgaagtcagcggtccagatcagcgggatgttgtcgccaccgaggttctcggcgatgaccgggcgggcctcggcgaacatgtcgacgagctcctgccactcctccggcttctggtaggtgtacttcgcgccggagaacagggttgcggagaacgcgtcgccgccttcagccggcttcttgtgcacgacgaagaccgggtgcgggccgaccagcaggatgcggatctcgccctcgacaatgcgcggcatgaagcgcatgtcaaccagcatgccgttgtcgcccacgatgtactgctcgcagaagtccatgaactcgccgagctcgcggtcctcggtgtggttgtccacagcctcggtgcacttgagcttggtgtcgagcggcagcgcggtacccggctcgacagactcggccagctctgggtctgcgaggcggacgcgccagatgccggaaccggtggagccgcggttctgcttcagcacgcgctcgccgtaggacagggaggtcgggaaggtgttcttgaacgtctcgacgtcgtagtaggcggcggtgtcggacggaaccaggtcggtctggttcagcttcaccagcgcgtccttcgctccgtaggagatcatttcctcaggggtggacatgccgacaaggccagcttcagaaagtcgggtgagcaggtcgaagtagcccttctcgccgcccgggatgttgcccgggttcacgcgggagatgtaggcatcaaagttctcggaaacgtagttgaagaggtcatcgctccagtcggggcggtagtagacgacctcggagtgccagcccttttccttgatggcgttgacgatgggcatggtgtccttgcggtggccgtcgaaggacttgtcggagccgccctcaacctcgaaaactacaatcgctttcttcacgtgcgatccctttcctcgtaatggttagcattgtcaccgcacgaaaggcggcgcgggaaacccagttgttcctcttcaagggtatgccggaagtggtgacctcacaggacaggcacaaggtttagtgtttaacctcacacaccgcacaaacgtcccgcgtcagcgcgcttccccacgcgtcgtccagcgctggaaccacgtgcgcgctttttctcacaggtagtgttacctatagcgtttaacgtcggtatttacggttcagaagcgccagagttgaggagaccaaagtgggcatcgaattcgacagcagtccgcagtttcaaagcttcacccacccggagaagttcgtgtctgcggcgtggctgtccgcgcgccttggcaccccggggctgaaggtggtggaaagcgacgaggacgcctatctgtacgacatcggccacatccccggcgcagtgcgcatcgattggacccgcgatctcaacgacccggtcatgcgcgacctcgtggacgctgaggctttcgctgcgctcatgcgcgaccgcggcatctcccgcgacgacaccgtggtggtctacggcgaccgggcgaactggtgggctgcctacaccgcatgggtgttcgagctgttcggtcacccagacgtgcgtctcctcgacggcggccgcgacgcgtggatgggcgaagagcgcgacacgtcctacgtggtgcccgattacccggcgactgactacccggcggttgatcgcgcagattcaccgatgcgcacgttcgccgcagaactcgtcgggggtgttgaggacattcagcttattgacgctcgcacgcccgacctctacgccggcactaccccccagccgcagacgctccgccacgggcacattccgggtgctgtcaacgtgccgtggggccgctccgtcttcccaaactcgctgttccgcagcattgacgatatcgccgccatctacgacgatttcgaccccaaagcgcccaccgtggtgtactgccagcgcggcgagagttcggcgcacacctggttcgtgcttaagcacattttgggtttcgaaagcgtttcgctttacgacggttcgtggatcgaatggggcaacatggtccgggttccgatcgaagttgatcccgccgcgctcgcgcctgccgtaatagatgacgcggacgacgatatagattagataaatctattcaactgaccgtgacatcgagaagaaacggaaatttttcgtgtctgaattcaacaaggtgctgattgccaaccgcggcgagatcgccgtgcgagttatccgtgccgcgaaggatgccggcatcgcttccgtagccgtgtacgccgagcccgacgctgacgcaccgttcgtggagctcgccgacgaagcgttcgccctcggtggagcgacggcagcggagtcctacctggacatggacaagattttgaaggctgcggccgacgccggggcagacgcgatccacccgggctacggattcctctcagaaaacgctgagttcgcccagaaagtgatcgacgccgggctgacgtggattggcccctcgccggaatcgatcgccgcgctcggcgacaaggttacggcccgccggatcgcggagcgcgccgatgcgccgatggctccgggcaccaaggagccggtcgccgacgcagacgaggtcgttgcctttgccgacgagcacggcctgcccatcgcgattaaagccgcgttcggcggcggcggccgcggtatgaaggttgcctacacccgcgaggaaatccccgaactgttcgagtccgcgactcgcgaggccaccgctgcgttcggccgcggcgagtgcttcgtcgagcggtacttggacaaggcccgccacgtcgaagctcaggtgctggccgaccagcacggcaacgtggtggttgtgggcacgcgcgactgctcgttgcagcgccgttttcagaagctcgtggaggaagctcccgcaccgttcctcaccgatgagcagcgcgagcgcattcacaccagcgcgaagaccatctgcaaggaggccggctactacggcgccggcacggtggagtacctggtcggctcggacgggttgatctcgttcctcgaggtcaacacccgcctccaggtggagcaccccgtcaccgaggtcaccgccggcatcgacctcgtgcgcgaacagttccgcatcgccgcgggcgaaaccttgcggctgaccgaggaccccgcaccgcgcggccacgcgttcgagttccgcatcaacggcgagaacgcggcgcagaacttcatgccggcgcccggcaccatcaccaagtacgccgagccgtccggcccgggcgtgcgggtggattccggagtgcgcgccggttccgttgtcggcggtcagttcgactcgatgctggcaaagctgatcgtttcaggagaaacgcgcgcggaggcaattgagcgcgcccgccgcgcgcttggcgagtacaccgtcgaaggccttcccactgtcatcccgttccatcaggcggtgctgaacgacccggcctttatcggcaccgacaaggggttcgacgtctacacccgctggatcgaggaggagtgggacaacacgctcaactcccccgccgacgctgagcccgatgagaacgcggcggacgagaagcgcacctacgctgtggaggtcaacggtcgccgcatcgagatcgcgcttcccagctccctcgtgtttggcgcggggcgcaagaagcccgctaaacgacgcagcgccggcgccaaaaccgccatctcaggcgatgccgtcgcctcccccatgcagggcacggtgatcaaggtcaacgtggccgagagcgaagacgtcgccgagggcgacgtgctgctcgtgctcgaggcgatgaaaatggagaacccggttaaggcccacaagtctggccgcgtgaccgcgctggcagtcgagcccggcgcgcaggtgaacaaagcagccgtgctgatggagctgaaggactagaacccggccgcctgcgcgataaacggcgccgccacaaccacgatcgagagcacggcgatcgtaataagcgtgacgcgccggatgtccgcaccgtcgttgctcacattttgcgtctgcgcgccacccgcgggcacgacaactggcgtgcgcacctgaatggtggctggccggtgctcgccgtagtgcttggcaatgagctccatctcttggtcggaggtcgggccttggacgtctcgagcaactgaggccctcagcgcgcggtactccccgcccggtgtgtagacgatattctgcccggtgaacacaccaaggaatccgtctcggccctcaatccacacgggcgatccggagtcgcctgcgactgcgccggtgtcctcccagtagatgttgccgccgagcgtcccaatcaggttcgagcaggtagtcgacccgctcgccgctccgtgaaaacagatgcggtcgcccggtcgcagatcggcgatatcggcggcagtgtcgcctgtgtaccggttgtagccgtggaggggccggtcgaactcgactcggccccagtcgctgccggtgccgggtgcgacgtagtttgccgaaggtttaaagcggccgatgttgtgccattggccgccgacctgtacggcgacccggtcgttgctcctgccgcagtgcgcggcggtgtaaccgacctgctcgctttcggtcttgtcgatgaagccgagcgtgcattgggagttggagccgacccggattgtcttgccctgagtcacgccgactatttgggcgttcgcagccggagccgcgccaattgccatcaccgcggccacggcaaccgccaccggaacctgtctcatggtggctcagcctacagccaccatctgcgcagcctcaagcaaagccaataggatgtggttatgcctgagttcaccttccgacacgccacagaatcagaccgcacgtaccttcagcgcttgaacttcctcgccgacgtcttcggcgacgagactgcagagattggacctgaagagcgcgagggcatcgcgggttacgtcgacgactgggaccccgagcgcgacggcggcatcattgccttcgacgagtggcgcacacctgctggtggcgtgtggctgcggtactgggcgcagcctgacgatggccacgcaaacttcggtgccgacatccccgagatcgcgatcgcagtggaacagcgtttcgccggcaaccgcctcgctgcgcaacttcttgaggaggcagcggcgctcgcgcgggagaagggctcaccgaagctcgcgttgtgggtggatccggacaatgcccgggcgcgccaccgctacgagaagttcgggttcaaagacgtggacggccaccccgacaccatggtgtttgacctctaaatagccccagacagcaaaaaagcaactgccccgccgcgaactgcggcggggcatggcggttagttgatcaccacaaccaagtcgccgccctccaccttggtggcttgctgcagcgcgacgcgctcgaccgtgccgtccttggtggcggagatggaagcctccatcttcatcgcctcgatggttgcgacttggtcgccggccttgacctcgtcgcccggcttgacggtcacgttcaccacgccggcgaacggggcggccacgtggcccgggttggaggtgtcggccttctccacctcggcgacagtggactcggcgttgttgtcgcgcacccacatcgggcgcacctggccgttgacggtcaggatgacctggcgcatgcccttttcgtccggctcgcccacagcatcgaggcggaccaccagcggcggggtgttgtcgtcgatctcgccgtagtagatcatcgtctcctcgccctcttcgaggccgtagaagaacgtcttgtcgccgagctggtccgtcacaccgtaggtgcggcggtgctcgaggaactcgtcgtactgcttcgggaagagcagcttgtccagcgcgatgcggcgggtctcgtggtcctcgctttcgaggtccggcgcgagttcctccggcacctccacggtgtggtcgacctcggcgcggtcttcaagcgccttctcgcgcagaagcggccagccgcccggaggcgtgcccagctcaccctgcaggaagccgatcacggactccgggatgtcgtacttgcgcgggttgtcggcgaactcgtacgggtcgacaccggcgccaaccaagtgcagcgccaaatcaccgacgaccttggacgacggggtcaccttggtcgggcggccgaggatgtcgttcaccgccgcgtagtagtcttcgatgagctcgaagcggtcctccaaaccgagtgccttggcctgtgtgcgcaggttggacagctggccgcccggaatctcgtgcttgtacacgcggccggttgggccggggataccggactcgaacggcgcgtaaacctggcgcacagcttcccagtacggctccatgtcggagacagcctgcagggagatgccggtgtcgcggtcggtgtcggcgaacgccgcgacgagcgcggacatggacggctgcgaggtggtgccggccagcggggcggaggcgacgtcgaccacgtcggcgcccgcgtacgctgccgccaggtaagttgccagctggccgcctgcggtgtcgtgggtgtggacgtgaaccggcaggtcgaagcgctcgcgcagcgcggtgaccagcttggtcgctgcggcggggcgcagcaggccggccatgtccttgatcgccagcacgtgagcgccggcttccacgatttcctcggcgaggttgaggtaatagtccagcgtgtagaggtcctcagccgggtcgagcaggttgcccgagtaggccatcgcaacctcggcgacggtggtgttggtctcgagcacggcgtcgatcgccgggcgcatctggtccacgtcgttcagggcgtcgaagatgcggaaaatatcgatgcccgaggtcgcagcctcctgcacaaaggcgcgggtgaccgtgtccgggtacggggtgtagccgacggtgttgcggccgcgcaggagcatctggatgttcacgttcggcatcacctcgcggatctcgtcgaggcgcatccacggcgactcgtggaggaagcgcatgcccacgtcgaaggtggcgccgccccacgcctccacagaggtcagctgcggagtgaggtagccgacgtgcttggccgccgccacaagcgtgttggtgcgcacgcgcgtggcgaggagcgactggtgcgcgtcgcggaacgtggtctcggtgacaccgagggcggtctgattgcgcagcttctccgcccacttcttcgggccgagctcgagcaagtcgtcgcgcgagccgcgcggcaggtcgccgtaatcggccttcggcagcttcttcgacggctggatcgtggtcgggcgggcgccgttcggcttgttcacggtgacgtcagccaggtaattcaggatcttgcccgcgtcgtccttcgcggcgggtgcctcgagaaggtgcgggtggtccgcgatgaagccggtgttgacgcgctcgtggcggaactcctcctccgacagcagcgcgcggaggaagccgatgttggtggaaacgccgtctaccgcgaactcgttgagcgcgcgcagggcacggtcgatggcgacctggaagttccggccgcggcaggtcattttcaccagaagggaatcgaagttcggggtaatcggggtgccgacagcgaccgagccgtcgaggcgcacgccggcgccgcccggggagcggtatccggtgatcgtgccggagtcgggacggaaaccgttcttcgggtcttcggtggtgatgcggcactgcagcgcagcgccgttgacctcgatgaggtcctgggtgaggtggatgtcctccagcttggcgccagccgcgatgtacatctggttcttcacgatgtcgatgccggtgacttcctcagtcacggtgtgctcgacctgcacgcgcgggttcatctcaatgaagacgtggttgccgttctcgtcaaccaggaactcgactgtgcccgcgccctcgtagttgatctccttgcagaagttcaccgcgtcctggcagatgcgctggcgctgctcctcggtgatgtgttgagccggggcaatctccacgaccttctggtggcggcgctgcacggagcagtcgcgttcgaagaggtggacgacgttgccgtacgagtcggccatgatctgcacctcgatgtgctgcggcttgatcacagcgcgctcgatgtagacgttcgggtcgccgaacgcggcctcagcctcgcgggacgcctcggcggagagcttctcaacgtcctcgatcttctcgatgaagcgcatgccgcggccgccgccgccagccacagctttcacgaagacagggaactcgaactccttggcgtactccgccagctgcttcgggtcgctggagggctcggagtccttcagcgtcggcagcccggcgcgctcggcggcgtgcactgcggccgctttatcgccggtcagctcgagggtctcggcggtagggccgatgaacttgatgccttcctcagcgcagcggcgtgccagctccgcacgctcggagaggaaaccgtaaccggggtagacggcgtccgcgccggtcttcttggcggcgcggatgatttcttcgacgtccaggtaagccttgaccggctgaccttcgataccgatctggactgcctcgtccgcgaacgggcggtggaacgagttgcggtcttcgcgggggtagacggcaacggttttggcaccggtctcgaacgctgcgcggaacgctcgcaccgcgatctcgccgcggttcgctaccaggattttcttgaaagacggcaggtcgttcagcgggaggttatccgggttcatattgttcctttctcaaggaaggacgagggtcatagaacaccatcagtttaatacaggtcacatcattcgttgtgtgggtgggggtgggaaaacgcgggcgtcgacaagcaacagcccgcgtttcgggggtggaaccctagcgctcgatgtggcgctcctccgggccgttgtacgctgacagcgggcggatgagcgagttgttctcgaactgctcaatgatgtgggcggtccacccggtgatgcggctcatcacaaacagcggggtgaaaaactcgatgtcgaagccgagaatgtaatacgccgggcccgacgggaagtcgaggttcgggcggatgttgatcgaggtgttctcgtacatggtcttcgccatgatgtcgtacatctcaacccacttctgggagtccttctccgggtgctcggcggcgagcttcttaaacgcggcctccatggtcggcacgcgcgagtcgcccttcttgtacacgcggtggccgaagcccatgacaagctccttgttcttcagcttgtccaggcaccactcctccgccttggcggggtcgccgatctcctccatgtggtgcatgacaaactcgttggcgccgccgtgcagcgggcccttcagagcgccgatagcgccggtgatggcggaccagccgtcagacatggtcgacgcgatggtgcgggcggtgaacgtggaggcgttaaacgagtgctccgcgtagaggatcatggtcttctcaaacgcctcgatgtcagacggaatgttcgccggggacttctcgtcgtcgccgaagaccatccagaggaagttctcggagaagcccttctccttggaaggcgcgatgtactccttgccctggcggcggcggatgtccgtcgccacaatggtcggtagcttggccaaaagctggcggccgatggagcgcaagtggtctgcgtccggcgtgaacttctccggatcgtgggtgcccaggtaggacaccgcggtgcgcagcacgtccatcgggtggcaatccgtcgggaggaagttgatgatctggatcaactcctcgtcgatgtcgcggttggccatgcagccgctgcggaactccgccatctgctcctcgttcggcagctcgccgtgccacagcaggtacgcaacctcttcgaacgtgcagtgctcggccagttcctggaccgggtagccgcggtagagcagcgagttggtctccgggttgaccttcgacacggcggtgtagtcggcaacaacgccgttgaggcccttgcggatgtcttgatcagtcatttctggttcactcctttggaatcgaacaaggtcgagctagttgaaggtcgagctgtaggtgtctttggaataggtgaaaacggactggtcgaactggttgtactggtcgtacttcaccagctcgtagagccgtgaacggtgctgcatcttgtccagccacggcttttgggtgccggtttcggcgatgtcgcgcagcatcgcctcggtctgccccatcgcgatgcggaaggtggtcaccggccagatcaccgcgttgtagccgagcgcttccaggcgcggcgcggggatcaggtcggttttgccgaactcggtcatgttggcgagcagtggcgtgtcgacggcagcgcggaacttcgcaaaatcttcttccgaatacaacgcctcggtgaagataagatccgcacccgcgtcggcatacgccttggcgcgctcaatggcctcgtcgatgccctcgatgccggctgcgtcggtgcgcgcgcagataacaaacgcgtcgtcgtggcgctcccgcaccgctgcggtgatgcggcgcaccatcacatcgcggggcacgacctctttgccgtcgaggtggccgcagcgtttcgggttcacctggtcttccaggtggagtgccgcaagaccggcggcttcaaactcggcgagggttcgcgccgccgacatcggctcgccgaatcccgtgtcggcgtcgatgagcaccggcaggttggtggcccgggcgatctgcccgccccgcgcggcgacctcggtcagcgtggtcaacccgatgtccggcaggcctaagtcgttcgccatcaccgcaccggagacgtacacgccttcgaaggcgccgatgtcctcgatcaggcgggcggtgagcgggttaaacgcgccgggcagtttggtgatcgtctcactgttcagcgagtccctcaagttctgtctgcgctcgtggggcgtggattcgggtgtgaacattagaagatgcctccggggatctgcggtgcttcggcgcgagcggcgtcattgacggcgatgttcagttcgctgagatcggtcaggttttccaggtcctggactgtggtaaggaaacgctcttgctcctcggggtccacgacgccgctcgcaagcgtgcggaacttggcaatgtagttctcccgcacgaacgggcgagcgccgagcgggtgggcgtcagcgacggctatctcgtcctcaatcacgctgccgtcggtgaaggtgattacggcgcgggcgccgaacgccttctcgtccgggtcgctcgagtggtagcggcgggtccattccggatcctcaaccgtggagatcttgtgccacaacgcaacggtctccgggcggccggcgcgctccggggtgtaggagtcgacgtggtgccaggcgccgtcttcgagtgcgacggcgaacatgtacatgatcgagtggtcgagggtctcgcgggaggcggtcgggtccatcttctgcgggtcgttcgcgcccgtgccgatcacgtagtgggtgtggtgggaggtgtgcagaacgattgagtcgatctccgcggtggtcttgccggcgccggcgatcgtctgcttcatgcggcgggccaggtcgatcggcgcctgcgcctggtactcggcggagtgctccttggtgtaggtgtccaagatcgcgcgcttgccttcgccaggtgcaggcagggggacggtgtaggtgcggtccggggagtgcagcatccaggcgatcacgccgtcctcgccctcccagatcggggctggggcaccctcaccacgcattgcgcggtcgacagcctcgatggccatctttccggcgaacgcgggcgcagacgccttccacgaggaaattaggcccttgcgcgactggcgcgttgcggtggtcgtgtgcagcgcctggccgacggcctggtagatcgaatccacgtccagctcgagcatggtgccgataccggcagccgccgaagggccaaggtgggcgacgtggtcgatcttgaactggtgcagggagatgcccttgaccaggttcacctgaatctcgtagccggtggcgatgccgcggatcaacgccttgccgtcgaggcctttgtgctgggccaccgcgaggatcggggggatgttgtcgccggggtgggagtactcggcggccaagaaggtgtcgtggtagtcgagctcgcgcaccgcggtgccgttggcgaaggcggcccactcggcggagtatgcgccgtcgataccgaagacctgggcgccgccgctggcggccgggtgcgcctgcgccatcacgcgggcggtggtcacaggtcggcgggcgtaagaggcaaccgcaacggaggcgttgtcgatgatgcggttgatgatcatctccttggtgtcctccggcacctcgacggggtcggcagcgacctgggcgatcttgtaggcgaggtgctcctcaaccgggaaatcctcggcggatttgcgtgtgcgtacttcatggtcgatcatgcggctcgctccttttcagcaagggatgggtgctgcacgtcatagtaagaagcaaagtgtgtttcagatcatgttcgctcttgcgaatctttgtgtcgtgaatacagcgagtatgtaaactttgtaaaccacaaggtagacacacgttttcacggacggagcaggatgtcgaagctgtacgcgggggcgcgaatccacacactgcgcgaggcccaggggctcacccaggtggacatggcgaagaaactgggcgtctcagccagctatctcaaccagcttgaaaacgaccagcgccccctcaccgtcacggtgctgttgcagctcagccgggtgttcgggctggacgcgtcgtacttctcgcccgattcgcagcagcgcaccgtcggcgagctggcggagctgctccccggtgtcgacgagcacgagatcgccgatttcgcggtgcgcttcccccgcatcgccgacgccgtgcgcgacatcccagccctgattgaccccgcggcgcgcaacccgcacgccaccgtccgagacttcttccaagacaacaacaactacttcgacgacctcgacaccgccgcggaggcgttcgcgctgcaggcgccgtcgcgccagcttcggctcacccgcctcgccgcggcgttcgaccgggacctcggatacaccgtccgcttcaaccactacgacgcaggcccccgctccgcgcgcagcgccgaagcgcgtgagcttcggctccgcaccgggctcaccgaggcgcagcagtgtttcgagctcgcgtaccactacgggttgataggacacagcttgcttatcgacgcccacctcaaccccatcaccgacccggcggcagcaaacctcggccgccacggcctggcccagtacttcgccgccgcggtgaccatgccctacggcgaaatccttgccgcggccgaggaaacgcgctacgacatcgacatgatcgccgcgcgcttcggcaccggcttcgagtccacctgccagcgcttgggcaccctgcagcggccgaatgcgcgggcagtgcctttcgcgttcgtgcgcaccgaccgcgccggcaacatttccaagcggcagtccaccaccgcgttccacttctcccagcgcggcggcacctgcccgctgtgggtggtgcaccgcgcgtttgagacaccgaaccgcgtcacccgccaagtagcggtcatgccggacgggcgcacctacctgtgggtggcgcgcatggtgcagggacctgcggccgagttcggctcaccgaggcaggagaacgcggtcgcgctcggttgcgacaccgcgcacgccgaccggttggtctacgccgacgggttggacctctcccctgcttccgcaacccccatcgggcccgggtgcgagacgtgcccgcgcgagcagtgcccgcagcggtcgtttccggctaatccaggtcagagtgcgcgatgaggcgccgcgcagcttccgtcaccgagccggacagtgacgggtaaaccgccatcgagtccgccagctggcggacagtgaggttgtttgccaccgcgatggtgatcgagtggatcagctccgaggcggtcggggcgacgatcacgccgccgaggacctggcccgaacccttgcgggcgaagatcttcacaaaaccgtgctgcagcgagcgcatcttcgcgcgggcgtttgtggccagcggcagcttgtagatgtcggcttcgacttcgccgtcgcggatctgctgctcggtgacgccgacagcggcgatctccgggcgggtaaagacggcgttgcccaccgtcttcaaccggatcggcacgacaccctcgccgagcgcgtggtcgacggcgatgcgcccctgctgcgccgcgaccgacgccaggggcatgaggtcggtgcagtcgcccgcggcgtagataccggcgacgttcgtgcgcgacacgcggtcgacgtgaatgtggcccgacggggtcgtctccacgccagccgcctcaaggttgaggtcggcggtgttggggatggaaccaatggacatcatcacgtgcgagccgcgaatctcgcggccgtcggtggtgcgcacgatgactccgtcgccggtgttctccacgctctccacgcgcgcgtccttctccaggtgcacgccgaggccctcgagcacggtctccaacacatcggcggcgtccgcgtcgtcgtgcgggaggatgcggtcgcgggaggcaaccatggtgacctcaacgccgagctcggcgtacgcggagacgaactcggcgccggtcacgccggagccgacgacgatgaggtgcgtcggcatctcgatcaggtcgtacatctggcgccagttcaagatgcggtcgccgtccggctccgcgcccttgagcacgcgcggcgacgcgccggtgcacaccagcaccatgtcgcagtccagccgctcctcttcgccgttggccagctcggcgacaacgcggtgggtggtgtgccccagctgctccgaggagaagcgggcgcggccgttaagcacgcgcaccccggcgcgctctagctgcgcgtggatgtcgcgggactgctcggaagcgagcgcgaccacgcggttgttcaaggcgctgattgccaggcgagcttcacccagctcgtggttcaagcccatcgcgtcggcgcggcgcaggtcggttttgatgttcgcgccggcaatgaagctcttggaaggcacgacgtctttgcggatcgcggagccgcccgcgccctggttctccaccaaggtgatgtccgcgccgtactttgaggcaacgagcgccgcctcgtagccgcccgggccgccgcccatgatcacaatcttcttcgacaccagcactctccttaaaagcttgagggcaaacgttgggggcaaaatcgccagctagtctaccggcacattctcagctccgcccttgcaggtggccgagtagtagtgctccgccacggcgccgaaaaggcggacgccgacgccgacggcgcgctcgtcgacaagcaaattgccctggtgcaggtccggctttgcgccttggccgttccacactccgaggcgcaccatcgtgcccggcacttgctccaggtaccaggagaaatcctcgccgccggaagactgcggcgcggtgacaatcgcgtgcggatccttcgaccggccggccgctaccgcgatcgccgttgccgcgtcgtcgttgagtaccggcggcacgccgcggacgtagtccaggtggtacgtgcagcccgtgggggcgatgatcaggtcgattaagtcggtcagaatcccctcgagctcgcgccacgtgccaatgtcggcggttcgaaccgtgccgtcgaggatgccttgcttcggaatcgcgttcgcggcgtcgcccgcctccacgtgcccaaaaactaggacagtgccggtgcgcgggtcaacgcggcgcgagagcagagcaggcagctgggtaaccaccgcgccgagcgcgtagaccacgtccgccgacatgtgcgggcgcgcggtgtggccgcccgggccctccacgcgcaaccggagcacgtcagacgccgaggtgatggcgccagcgcgcaccccaatctggcccacccgcaatttcggttctgcgtgcagcgcgaaaatcgcggacacgccgctcagcccgccccactcgatgacatccagcgcgccgccgcccatcacttcttcagcaggttggaagatgcaccgcaccgggacggaaaggtccgccgtcgacagcgcgcaggcgagggccaaaaccacggttgcgtggacgtcgtgcccgcacgcatgcgaaacaccggggtgaacggatgcgaactctaagccggtctgctccggcacgcgcagcgcgtcgatgtcagcccggaacgcgatgcgctctccttgcgccgggccgatatccacgtagcaaccggtccccgggaaccgcaccgcctcgagtccgtgctcggcgaggacgtcgacgatgaagtcggtggtcgctatctcctcgttggacagctccgggtgcgagtggatgtgtcggcgccagccgatcaccgcgtcctcatgctttgcgaaccacgcatccacatgcgccgagatcgatgctgcgaccgcctctgtcaccgaagtgctcctccttcaccgaaccgcaccaccccgtaaaagttccagtcagttactttacgctaggccagaaacctgtcgacgccgtgcggtgcgccgcacttgagataggcgtcggcgaaacgcgcagtatccgtcggcgcagccggccagttgacggtcaccgcaacgtcgtcgccggagggtacaacgcacagcttttcgacgaccaccccagcccccggcagtagcgccgctggcgggacgtacagcgctcctgccaggcgatatattgtgctgatggttggatcggccgcgcgcgagccgttgtagtcgttgcgttccaaattcgacacgagcgatctcgacacgccggcgatttccgccagccgcacctgcgtgagcccgcgcatctgccgcaacattttcactcgctgacccaacgttaaggcgtagctcgcccaatacgactgcggcaacaattccgacatcggatttctcccccaagtaccccaccaaagttgttgtgaagcagcttattacaggctaagaaaccgcgccagggatgcgcaggcgaagtgtttagagatcgatgttgcgcggaccgtagaggcggtcgcccgcgtcaccgaggcccggcacgatgtacgcatcggcgttgagttccgggtcgatggtcgccgtgaccagccgcaccgggccgccgtgcgcctcaagcctgtccacgccgggctgcgcgctgaccatgcagacgcaggtgatgtcgtccgcgccgcgttccaccagaaggtcgatcgcgtggatcaaggacccgccggtggccagcatcgggtcgacgaggaacaccggctggccggacaggtcgtgcggcagcgcctcaaggtagggcaccggctcgtgtgtgttctcgttgcgggccatgccgatgaagccgacctgcgcgtccggaatcattgacaaagcgggatcgaccatgccgagtcctgcgcggatgatggggacgacgatcgggggcgttttcaagcgggagcccttggccgtgccaaccggggtcgcggtatcgaacgtttccacctcgaggtcgcggctggcctcgtagatcagcatggcgccgaggtctgccagggcggcgcggaaggccgcgttgttgctgcgctcatcgcgcatgatggtcaggcgggacgccgccagcgggtggttcacaacggtgatgtgcatacgaccatggtaggaagtttcgcgcctgggggaaccgtcacccgccgctgggcgtctaatacccatggaaactttcgccctggatgctcacgccgtcttcgcccacaccgactcgctgcgcgcggatgcgggcgcactcacacccctgccccacgtccctgtcccaagcggctttcccttcgaggtgttccacgccgcgtaccgcaccgccatcgatgcggctgagcggcgggcgcagcaagtgcgcgacgaagcgcgccggatagccgcgaacatggagacgaccgtgtacgcagccgacagcgtcgacggtgccacaagcgccgggttgggggcactgctgtgacgctctcgcctgtgttttctgccctgggcagccacatcctcgacccggtttcagtcgggttgaagatcctcgcgcacaagccggacctcatcccgaccatgccccgctaccgcacacccgggttcgacgatttcgctccgctcgccgccgtggtcggcgcggacccggcgcgccacatggcgatggtgcagggcttgcgggactaccgaggcgagattagcgacgctgtggccgccgcgtcgctgttagttgcttcgacggcctcgaagatgacggcgatcgccattgacacgatggataaggggtcgcgggcgctcgccttggggagcgtgctcggccccgtcggtgctggcattgcggcagcggtggtgatgcaagatggagtgcaaaaagcgtgcaacgagctggaggcgctgcaccgcgaactcggtgtgttgaaagacaagctcgaactcgccaccgcggccttgctcgcagttgcggtaccgggtggttccgcaggcgccagcgccgcgtcggagacgctgcgcggtttcgtgggatccgctcctgccccagccgtaacccctagcgcggccgcaccgcccaaggtgagcccttcggcagtgccgtcccgcacccagccggcgtcggtggaggtggtgcacgcgccgccgacggtggacccgatgggccagtcgggctcaagcgcggggccgacaccggctgcccaagccgcggtcgccgccgccaaatcccaaatcggcaccccgtacgtgtggggcggcgcggcgccgggcgggttcgactgctcggggcttacgtcgtgggcgtacaggcaggccggtgtagagattccgcgcactgccgcggcgcagacggtaggcaggcaggtctcctacaacgagctgttgccgggagacctggtgttgtggaccgggcacgccgcgatgtacgtgggcgacggcatgatggttgaggctggtagcccggtgcaaatgaacccggtgcgcacgagcaacatggggatgggattccaagggttctggaggcccaccgggtaaactttccgcccatgagcacgcgagcgattctccccgtcaaactggccctaaccgagggcgacttctacaccctctgggcgccaacctggaaggagaagggctccgagtggcaggccttcttgggcgacgacgaatccgtgctggtcttccgctcccccgaggagctgctcgcgtttttgaactcaaccccgcgccacgacttgagcgaccaccccaagtgggcgcagttccagtcccagggcgaggcccgcgtggtgcccaacgacaagcagtactacgacatcgttggcgcgccagatttccttgccggccgcccgagccacgagaacgtctcttcgctgtcgcgcgtatttcagatctcccgctcgctggcagatgttgccagcgccgagcaggcacaaatcttcttcgcctcgcactcgatcctgaacaacgtcacccgcggctccgaccactactccggcgagaacggcctcgacgaatggtccggcgtggggcgggtcgtgctgaagaactgggagtcggtcgtgcactccctcgaccgcgccgtccgcgtagtggagactgaccagctcgacccgcaagcggttgcggcggcagcggcctctatcgccgcggccgcggaagcaaacgagcgcgcccagcaggaacgccaagacgcggaggccgcgcgcactgcggcgcaggacccgtacgacgcctccgactggggccgcgctggcatcgacccggtgaagatcaccatccagggcaagacggtctacacgctgcgtacctacctcggcaccgcgccggtgttcttgggcaagtacggcgagattttcaccttccccaccccaaagcacctcggccgctggattctagaaaacgacgaccacgatctcgcgtcggtgtcgacctggcaggatgtgatgaacaccgcgcacgcgggcgagctgaaggtggaggtccacccggacaactcctactccttcagcggactgaccgatgacattgcgaaaagcgttgacgccgtggacacccagcagatgggcaaggcgtacgagctgctggcagacgcagccgactgggccaaggacgactcgctgaactccttccttttggccaacccgcgcatgcaggactacctcgcgtacatgctcggctcgaccgaggctgccggctacgtgccgtccccgccgtttacggacaaggcccaggcgtgggcggagatggaagagcagctgatcaagcgcttctccaagttctagacccagcgcccgaaggtgccgccgaaacgtggcacctttacaatttcgacctatgtcagtggaccaggtcgacccgctcatcagctctatctaccgctggatggatgtctcgggcgtgttgctgatgggcatcatcggcggcacgctcgcccgccagcgggggtacgacatcgttgggttcttcttcatcgcgatgctctcggcgctcggagggggcatgcttcgcgacgtcctgatcaaccaaggcaccgtcgccgcgatgagccagccggaatacttgatcctcgcgttcaccggcgccctcatcgccagattcacttacttcaaaggccgcgcctgggagtttttgcagtcgcacggtgatgcactggtctccgcgctgtgggcttctaccggtgcatcgaaggcgatccagtacggccttcctacacttcccaccatcatgatgggtgtgttcaccgccaccggcggcggcatgatccgcgacgtggtgatgggccgcgagccgtcggtcttcggcggcaaccaacccaccgtgatcccggcagtggcatgcgcggtgattaccttgatcggcaacgcgaccggatatttggccgtggcgatggtcgttggccccgtggtcagcttcgtcatgttcctctttggctactacggcaactggcgcatcagtcaagatccagagttcgcaccggtgaacgcgactgcgacccaggtcgcccacttggccaagaaggccgagcacaagtcgcgcgccgtagcacgcgagctcgagccgaagaccgtccggtcgtggcgccacaagcagatggaaaaggcgctgcagcgccgcatcgaggccgaaatccgcaagggcaagcggccggtggacgcgcgcaacgacgcggacgagttcctcaacgagttcaccaaccagttccccgccatcgacgcggagatcatcgccgctgcggccgcggaggagctggttgaggaaggcctgttcgacggcgtgggcgtggacttcgccggcgactcctacgacgacgcgccgcagcccgacccggccgagaccgaggcggtgaacgccgacatgctagatatcattcttgccgacgaggccttaaccgacgagctcatcgaccgccttgtcacccgctacaaccaggaagacgagtagatgaaaagagcggcgggggcgttgatggtggcgtcgataagcctgtgcttgagtcctctagcccaagcgaccaccgcaaccacgacgacgaccgaatggttgcccccgagccgcgagcacgcgccggacaccgatgcctgcccgcaggccacctggccgccggaaccggtttccacctccgagcgcgcggcgagctcccccaccccgctggccgcgacctacgacgggccgtgcggcatcaccgcggccgacggctacaacgtgccggaggaggtggtcgcttccgcgtggctggtggcagatctggacaccggcgacgtggttgcgatgaaagacccgcacgggcgctaccggcccgccagcatcattaaggtgctgctcgcccttgtggtgattgaggagcttccgcttgacgacgcggtggatgtctccaccgaatcagcaaatcaggagggatccgcagctgggattggcgcaggcggccagtacaccgtccgcgatctgctctacgggctgatcttaaactccggcaacgactgcgcgcacgcgctcgcccaaaagctcggcggcgatgaggtggcgctgagcaaggtcaacgccttggccgcggagctcggtatgaccgatacccgggcagcgtcctattcgggcctcgacgccgccggcatgtccacctccgcgtgggacatggggctggcctaccgcgaggcgtttaccaacccggtcttcgctgagatcgccgacacggagtcttacgacttccccggcttcgacgagctacccgggttcaagctctggaacgacaaccacctgtacctgtacgacccggacggcatcggcggcaagaccggctacaccgacgacgcgaaccacacgttcgtcggcgcggtcgaccacgacggacgccggctgctggccgtcgtgctggacaccacagcgtgggaccacggcgcgtggcagcaagcgcaaatgctcctccacgccgcgtacccgatctcgcccgcggcgtcggtggcaaacctgaacgcccccgcggcggagccgagtcccgagcccagccccacaaccacgccggctccggtgaccgaggagccggaaaaagaaaccgcaaccggcccacgggagacgtggctgccggttgcgattgttgccggtgtcgcggtgttggccgccttagcggcctggctcagcaggcggctcggcgggctcgggcgccgctagttgcgggtgagcagtgaggcgatgccaacgccgatcgcgccgagcgccgcgccgacacccacagctgcaccggtgttggtgtgctgcgaggcagctgcaccggcgcgcacgttgatcacggcgggctccggtgcatcggccggggcagccttgagcgactcctcggtggtggcggtccacgccgcgacgtagagcaccacgcgccagatcaggtacagcactaccatcagcgcgatgatcgggccgaaaatcgcaccggccgggttgccggtggcggagctgacaatcacggtcgcgaactgcttgatcagctcgaacgcaacggcgccgagcagcgcgcccttcaggcccgacttcactggtacgtcggtgcgcggcatgtagatcatcatccaaaccatgacgatgaagttggccaagacacccacggcaagaccaaccagccagaccacgaagcgggaaccggggaagtcgcccaggccgaagtgcgccattagctgggtagtccacccggaagtgccgactgcggtgacaccgaacgcgacaacgaacaagatgatgagcacgatgaggccaagcaggtcccagagcttcttcatcacaaagttcccgccttcgttcgcatcgatgccccacattgcggaaatgccgacgcgtaggtggttcatccagttcaaaccggaccacaaggtggtgagcaaaccaacaccggcaaccgcgccacgctgatcgatcgcagtttgcaccagctcattgaccttgtcgcccacttccccttcaaggttctgggtgatctggtcctggatctcctgcatcagctcaggccgggcgttgaggaagaaaccgagtccggcgaacatcagcatcagcagggggaacagcgccaacaccgagaagtaggtgatgccggctgcgaactggttgccgccctcggaaccgaagcgttcctgcatgcgcatcaagtggccgacagccggtgccttctgcttcagctcgtcggccgcgccctttttctgcttcttcgtggcgcgctcaatgccgtggtcgtcggtgtatgcctttcgaggcgaggtagaagttgccatcggcgtcccttcccgttcactgtgcctcttcgaggccctacgtatgccggagttacatcgtagagcaccggcggcgcctagcgcttgggggcgagaaaaccaaccttgccgtagacgtcttcaagcaacggctccgcaacctcgcgggcgcgctccgcgccacgggcaagaatcgcttcgagctcgccgcggtcgctcatcagctcgtcgtaacgagcgcgcagcggggtggtgaacgcctcgagcgcttccgccgtgtccaccttgagctgcccgtagccttgcccctcgtaccctgcgacgatgtcgtcgatcggcgtgcccgtcagcgccgactggatcaccaggaggttggacacaccgggtttgttctccttgtcgtaggcaatcacgccgtcggcgtccgtcaccgcggagcgaatgcgcttggcggatgtcttcggctcatcgagcaggttgataatgcccttcgggttcgcacccgacttgctcatctttgcggtcggctcctgcaggtcgtagatcttcgccgcgccttcggggatgaacccgtcgggcaccacgaacgtctcgccatacttcgcgttgaagcgctctgccaggttgcgggtgagctcgaggtgctgacgctggtcctcccccaccggcacaagctgcggggagtagagcaagatgtcggcggccatgagcatcgggtacgtgaacaagcccaccgaggtgcggtcctggccctgcttggcgcttttatccttgaactgcgtcatgcggctcgcctcaccgaacccggtcaggcactgcaggatccaggtcagctcggcgtgcgccgggacgtgcgactgcacgaacagcgtcgacttgtccgggtcgatgcccagggcgatcagctgcgcgcagccggcgatggtgcggtttcgcagctcctccgggtcctgctccacggtgatggcgtgcagatccgggatgaagtagaacgcgtcgtagttgtcctgcaggtcaatccactgcttcagcgcaccaaggtagttgccgaggtgataggaatccgccgtgggttgaatgccggagaggacgcgctgctttgtcatgcgcatcagtctatccatggacatcacatccaagctcactagtatttcagcacatggggtgccaccagtttcggaagcctgggatgcttcaaaaggcaagttcaagcgagcgcacatctcagctcccctagaaaacggcgcttggtcacgatgaggttaacgacattccctgaactagtaattcaatctaggatggtcgatgaaagagccggaagggaggaacaatgccaactccgacacactcatctcgggccactcaaaggagcaccggacatcgcccgtcacgcggccaaatcgcggcggcgaagctcatggtcaagcgcgagcaggaaggtaagggccgcgtcgagattactccgaagatccgcgaactcgccgctttcgagctttcgtagacccttaaccccattccaggccttcacttccgagtgacggcctggttttttcattgacacgaacgccccaccagttctatagttacccacatgagtggtaaacccatataccaagcgattgcggacgagctccgcgacatgatcggtgccggcaccctggcaccgggcgaccgcgtgccgtccaccaacgagctctccgcctaccactctgtgaaccccaccacctcggccaaagcgctcaccgagctgttcaacgagggcctgctggaaaagcgtcgcggcctcggcatgttcgtgctggattcggcgcgggagcaggtgttaagcactcgtcgtgaagcgtttgcccgggatttcgttgaaccctttgtccacgccgccgaccagctcggattcactacggaagaactgaccgacatgattgccaaggagcgcaaccgatgaacctgacccccggtttttacgccctggtcgggccgaatgccgcaggcaaaacctactacctccattcgctgatgggcccgcacgctgcattcgtccccgcgggtgcggatgcaaagttcgcgggcaccacggtgggcgatcatctgcgcgccgcccgcaccgcccgccccatgtcgcgggtggatttccccgacgcgcgcatcaagaacctttccgtaggtcagcgccgactgctcaccatcgaggtcgcgctggccacgggcgcagagcttttgcttctcgacgaaccctttgacggcatcgacgtcgctacgcgcaaacaggtccgccaacgcctcatcgattatttggcggaaagcccggaacgcaccgtgattatggcgtcgcaccggccggaggacttcgcgggcctggccacgcacgtgattcaggtgttcggccgtgaggtctcgcgcccggtggcgctggatgacgcgcgtctgtgcttccccacggtcacgggccccaccgccgagatagaggagctggccgctcgcttccccgtcgccgaattgtccagcctcggcccgacaacgcgcgccacgttcgccgaacccctccgcgatgaggagtgccacctgcccatttcttacccggacgacgccgaactgattgacctcatggccaccgaaaggaccgcacgatgaaactcttcctcagccccttcaaaccggcgatctacttgggcgggttcgtgctgttgtgcctggtcgctcccctcggccgcctcgctttcggcgacgggggcctgtggaccatggcgagcgccgccgctctgtgcctgttcttcgcggccggcgcagcgaattggccagcgttgaatcagctcggggccagcttcaaccgctggatgaactcggcggtgttgacggcgctggtggcggcggttgtgctcgcgccgctaacggccgcatccgcggtgtaccaccaagcgcacagtccgtattacttgtggtacgacccgttcatcatcaccaacggcgagccgatgctctggatcgacggtaacggcgagccctacctcgtcgaaggggcggcgcaagacgcatcctcggccgcgctgaccctgctgttccacttcgtcatctttctcacgatcgcgctggtcggcctcgcagtcggtcttgcaaaagacactcgcatgctgtggctactgatgggcgcgctgttcatcggcagcttcgtcggtgtcttagtcggtgtggtaacggaagatccgttcgctccgttccacaccacctcctacatcattgccgtcacgctcggtgcaagcatcgtgctggcggcgtgtgcgattgtgttcgcccgcacgcgtagctttgtgcgatgagtgggcgcgcacagccctagaccgcaattcccggtggcggctacgtttcttggtatgactgacgttgtcaaaattaacgctcgatgctctggtctcggaatataagtttcagactcgctcccagggggtgagagcagcaatccgggcgctccagcgcgaatccctagctcgtgcttatgattcctgcttcagcgatcccacgtggaaagccgaagctgaacaatgggatgtcgtatccggagatggactcgcagatgctcaggggtgaaatttatctggtggactttgagccgaccgttggtcacgaagccaataaaacctggccagcagtaatagtcagcaacgatctcgccaaccagagcgcggccatccacggaggcgtagtgacggcggtgccgattacttcgaacaccaccaacgtctacccctttcagacgctgctcgatgctgacgaaacgggcctccggctggactcgaaaactcaaccggagcaaatcagagcggtttccgtgcaccggcttagccggcgcatcgcacaactctcccatcagcaaatatctgagcttgattgggcccttcggatccagttggacctttaactgtgaacaggcttggtcctaccgctccagccactccgagcgcagcagcccgtggcgggagcagcacgcctcccacgccatggggctgattttcaccaccatgcggcggccgcacagggggcaaatgcgcggtgcgtcgtaggggcgcgccggatcgagggggagctggatttcgccgctgagcacggcgtcggccagctccgtcgaatcggggacgcgcattaaagggacttcagcgtgtcgtacagcgcaccgtggccggagttctgcttctggcccaccggggtgatggagaggttcaggttggaatccatcacgcggtcaaccgcgtcgcggtccttctccattgggcggccgaaggtagtcaggtagttgccgccgataatcgcgttggcgccgccgaggaggccctgctcggtgccgtcgtccccaagcgcgagctcggtgccgccggcgaagcgcagctgggtcgacggcatggctaggcggaacgcggcgactgcgcgcagcgcctcgccctgcgggaccaacgggcggtccgcgaacggggtgcccgggcgcggatcgaggaagttcatcggcacctcgtgcggcgtaatctcagccagctgggctgcgaactccgcgcgctgttccagggtctcgccgaggccgatgatgccgccgcagcaggtctccatgccttccgcgagcacgtgctcgagggtgtccttgcgctcctgccaggtgtgggtggtgaccacgttcgggaagaaagacctcgcggtttcaaagttgtggttgtagcgcatcacgcccatctgggcgaggcggtgcgcctgctcgcgggtgaggatgcccagggacgcggaaatggagatatccacttcctcggtgatggcggtgacagcctcggccacctggtccagcagctcgtcggtcgggcctttcaccgcggccacgatgcagaactcgctcgcgcccatcttctcggattgcttcgcggcctccaccagctcggcgatgttcagcgtcacggcgcgcaccggcgactcaaacaggccggactgggagcagaagctgcagtcctccgggcagccgccggtcttcagcgagatgatgccctcaagtgacacgtccacgccgcagtgcttgatgcgcacctggtgggcgaggtccagcagttcctggaggcggtcgtcctcaatctgcagcacctgcaggatttcgtcctggttcaggccctcgccgcgctcgaggcatttctcgcgggcaatgtcgaggatgtctttggtttcaactggtgcagtcatgggtactcctgaacgccgttcaacaacagggaatgtgtggcagtgtagcgccttagttgaacgatgttcaggaattggctcccgcagttactattccctccgccccgacttagctctacaccctgtgcgtatgaacagcaggtcggtaaagattaaaaagtctgtgtcgggaacgtaccgcactagtcggaccgtggctgggcgagctggggcacgggcaggtaaggaagcgcgcgatgtgcgaacgcgccgcctcgtgatcaccccacccacggagcccgccagtttcagtgtcgacgacatggccgacggcgaactcagttccgaagaaattctggccgcactgcggagcgattagcaactggaagctatggtcgcctggtactttgacacgtccgccgccctgaaactgctgctgagggaggccgagtctccgcagttggttgcagcgacacgaaacatgcatgaccgagttgcgacgtgcggcgcagcgcgaaaagaatctcacccagcagctcgtctccaacctgctgcggaagtttcacgtcgttcagatcgaccgacctgttttcaaccaagccggattacttccgggccggcatctgagatccctggatgccctacacgtcgcgactgccttggatatgcaggcggacaccctcattgcctacgacaagcgcatgttgaaggcagctaacgaagccgggctgcagatactatcccctggcgcttagcggtactcgaccaacagcggggcgtggtcggaccaccgctcctccaccgtgggagccttatccacccacgcactttgggcacgctcgagcatgttcgcggtggcggcctgcacgtcgatgcgccacccagcgttgttattgaaggcttggccgcggaacgtccaccacgtgtagccggcgtcgtccgggtttaaccggcgggccacatcgaaccagttcgggttgtcgcaggcgcagcgccccggcgcgtcggaggcgtaatcgacagcgcccgcccagcccggtgcggacttcagttcgaggtcttgcgcttcctcgtccgggaaggcaccgaagacagcgtccatgaaggcgcgctcgtgcggcaggaaaccggacttcttgtggttcgtcttccagttcttcagatcttcgcggcggtggcagatgttccaatcgccgccgatgaccatgtccgggtactcggccgaccactgttccagtagtggttcgaaggcatcgaggaagcggtacttctcgtcctgtttctccgtcccggcggatcctgaggggaggtagagggaggcgatctgggtggcgtcgtcaagcgaagccctgatgaacctccctgcatcctcgaagcctgtaatccccacctcaacccgtgagagcgggagcttcgacaggatgccgacgcctgcgcgacccttcgctgccgccggcgcgacctcgaggtgccagccctgctcgagcgcgggggcgagcgctgcggcggcctccgcttccgtggcgcggacctcctgcatcagcaccacatctgcgggggtctgttcgagccaggcgagcattcccgggttgacctcgttgcgcactttggtggcggcgcggatgccgttgacgttgacgctggcgatggtcagactcatgagtttcgaccctacaggcgggaccaagccggtacgcttgagggttgaagtctgaacaaaacaaaggagctatatgtctaagatcatttggacccgcaccgacgaggcaccgctgctcgccacgtactcgctgaagccgatcgtggaggcgttcgcgtcccaggcgggcatcgacgtggaaaccgccgacatttcgcttgccggtcgcatcctcgcgcagttcccggaccgcttgaccgacgagcagcacattgacgacgctctcgcgcagctgggcgagctggccaagacgccggaggccaacatcatcaagctgccgaacatctccgcttcgctcgtgcagctgaagaaggctatcgctgagctgcaggccgccggcttcgacatccccgattacgaggatgcgcaggagaagtacgacgcggtgaagggctccgccgtgaacccggtgctgcgcgagggcaactccgaccgccgcgccccggaggccgtcaagaacttcaccaagaagcacccgcactccatgggtgcatggtctgatgactccaagaccaacgtggcgaccatggacgctggcgatttccgtcacaacgagaagtccgtgatcatgccggcagccgacgagctgaccatcgcgctggttcaggccgacggcgacgagacggtgctgaaggacgggctcaaggtgcaggagggcgaggtgatcgacgccacctacatgtccgcgcgcgccctcgacgcgttcctgctgggcgccgtgaaccgcgcgaaagaggagggcgtgcttttctccgcgcacctgaaggcgaccatgatgaaggtctccgaccccatcatcttcggccacgtggtgcgcgcgtacttcaaggacgtctacgacaagtacggcgaggagctcatcgcagccggcctcgacggcgagaatggcctcggcgcgattctcgacggcctgtccgagctggaaaacggcgaggagatccgcgccgcgttcacgcaggcgcttgaagacggcccggatctggcgatggtgaactcttcaaagggcatcaccaacctccacgtgccgtccgacgtgatcattgacgcgtccatgccggcgatgatccgcacctccggccacatgtggaacgccgaggaccaagagcaggacaccctggcaaccatcccggattcctcctacgccggcgtgtaccaggccgttatcgatgattgccgcgctaacggtgcattcgatccgaccaccatgggcaccgtgccgaacgttggcctcatggcacagaaggccgaggagtacggttcccacgacaagaccttcaagatcccagccgccggtaccgtcgaggtccgcaactccgcaggcgatgtcctgctctcccacgaggtcgaggagggcgacatctggcgcgccacccagaccaaggacgccccgatccaggactgggtcaagctcgccgtgaaccgcgcacgcctgtccggcatgaagaccatcttctggctggatgaggagcgcgcccacgaccgcaacctgatctccctggtggagaagtacctgggcgaccacgacaccgaaggcctggacatttccatccagtccccggtcgaggccacaaagacctccatcgagcgcatccgccgcggcgaggacaccatctccgtcaccggcaacgtgctgcgcgactacaacacggacctcttcccgatcctcgagctgggcacgtccgcgaagatgctctccgtggtcccgctgatggctggcggcggcctgttcgagaccggcgccggcggctccgcgccgaagcacgtccagcaggttgaagaggagaaccacctacgctgggactccctcggcgagtacctcgcactggcagagtccttccgccacgagctgaaccagaacggcaacgccaaggccggcgtgctgggcgacgccctcgaccgcgctaccgagacgctgctcaacgagggtaagtccccgtcgcgcaaggtcggcgagatcgacgaccgcggttcccacttctggctcgcgacctactgggcagaggagctggcgaagcagaccgaggacgccgagctggctgagaagttcgcgccggtcgccgaggagctgcgcgccaacgcggagcagatcgacgccgagctgttgaacgcacagggcggcgccgcagacctgggcggctactactggccggacgaggagaagacctccgcggtcatgcgtccgtccgagaccttcaacaagatcatcgacggtttgaaggcgtaagtttccgctgcggcatcgcgttcaccgcatggagccgcgaggcggggtgcaggtgccccgcctcggggctttttgttctgggcggggtggcgcggcagcacagtggatcgccctccaaacccgcacttctagacacccgattggcgtccaccacaaagtgctcttcacctcatcaacgaacgagcgagggctccggcgaatgtcttcgggcgtgtaacgaagaaagtagtacccctcgttgctgagacgtttctgccgcagaaattcagcttggcggacgcgttccgcatcggggtccttgtacttgacgttgccgtctatctcgatgacgagccagccgtcgataagcaggtcgacgcggtaccccctgacttccacttgggcctcagtacccaagatccccgcggcgatcagcagcgctcggggtaggactcgtactgcgagtctgacaacgcagttgcgtggcgcaaccactctcgcgctgtcttgatgtttttgcgccgacccattgtttcaagttccgcggccaccatcccggtaggccgtgcattcgcgcggcggagcgccccagcaggactgcagcgttgctctccatagcggccgctttctcctccacgtagcggcgttcgtgatactgcagcccctgccactcgcgcgccgggaagaacgtcaccacgccgacttgcacgacgtcgcccagtttcggcccgcggtgcgtgtgtttgcgctgatcgacgatgagcgaactcagttccgacttccgttggtcccaatcaacagccatagctatcagacgccaccactcccccactggttccgtctggaaaatttattcaaccaaaacggcaggccatctccccataacagacagctcggttcagtatcggtgccgcagcaactagatttttcacccatggcccaccttgcagcagagggcgagctcgccacgatcagcatcggggatcttgtcaccgaagccggcgtccgcatacccaatgtggagatcgcgtaccgccgctggggagcgcgcaaaggggacctgaacggcaagaacaacattctgctggtggagcatgcgctcaccggcgactcgaacgccgccgagtggtggtgcgaggcggtcggccccggtaaggcgctggacaccgacaagtggtgcgtgatctgcaccaacgtgctcggctcctgctacggctcgacgggacccgcgagcgaacacccagacggcggcgcgtgggggtcgcgcttccccgcagtttccatccgcgacatggtccgggctgagcaggcgttcataaccaagctcgggatcggtcgcgtccacgccgtcatcggcggctccatgggcggcgcgcgcaccctggagtggacgctgctctaccccgaccaggttgacttcgcgctcgtcctcgccgtgtcggcgcgcgccagcgcgtggcagatcggcatccagtccgcccagatcacctcaattacccaagacccggcgtggcagggcggagactacttcggtaccggccgctcccccgacgcaggactcgctgccgcgcgccgcatcgcccacctgacctaccgcggcgagctggagatcgacgagcggttcggcacctccgcgcaaccgggagagaacccgctcggggcctaccgtgacgatgcgcagcgcttctcggtgcagtcgtacctcgcgcaccaggggaagaagctcaccgagcgattcgacgccgcgtgctacgtcaccctcaccgaagcgctcaaccgccacgacgtcggccgcggacgcggcgggctgaacaaagcgctggcgagctccatggtgcccaccatggtcgttggtgtggacacagatattctttacccctaccaccagcaggaacacatctcccgcaatctgggaaacctcctcgcgatggcaaagctgtcatcccccgtcgggcacgatgcgtttttggtggaggcgcgccagatggacaggattctgcgaaacttcatcgcgctgacaggagacacgccgtctgcgcacgacctcgcggttgcccgcggcgcctacgacatctagctcctactgcacctgcgcggcgccgcgcgactgccaccagcggatcagcacaagcaccacagtggaggtgccgacgccgatgagcgtcatcgccattgcctcggcgcggtggccctgctcaaactggttcatgatccacggcgcaagcaggttgatgcgggtcgggcggatcagcgacgacatcaccagttcgcggatgccgacgaagaacgcgagcaaccagccagcgaaaatgcccggtgcgagcatcggcagcgtaatgcgccagaacgactgcccgcgggtcgcgcccgcgacagccgcggcctcagaaagcgtaggcgacatcgacgccgcggacgtcttgatgttctgcaccgccataggcacgaagagcacggtaaatgccatcaccaagatgaactgagtgccgtacggcgtaaacggcagacgcggcgagttccacagcaggatgaaaccgatggcgagcacgatgccgggcacggtgtccggcgcgacggccaaaaagtcgctgagcttcgcgggcagcgaggtgcgccgcatggtcagcacagtgacggccagcgccaaaatcactgcggtcgtagcaccgatcgcgccaaggatgatcgagcgggtcagcgcctcctgacccgagggcatggacagcacgatcccgaagtagtcgaaggtgaggttgtccagtgttggcggcttcgaccgcaggatcgtcatcgcggcaagcgtgatcgaaatgtacggaatcgccacggtgaggatgaacaccaccgcggtgaacatccacgccagcaccatcccagcgcgcgagacccgcaacgacaccggccgagagacgcgtccgccgcttgcaaggccgccgcgccctgcccactgctgaatagcccaggcggtcacaccgagggcaaagagcacgcttgacgacgccgccgcttgcgaaaagttcagcggatcaatcgtcacatcctggtagatcgacgacacgaggacttggtaaccgatcgcgttgccgagcgtaaccggggtgccgaactcgcccgcggctttgatgaaaacgatcagcgcgccgagcgagtacgggccgagcaccatcggggcgacaactcgggtgaactgctgccagcggctggcgccggcgacctgcgccatctcgagctgtgaggcggggatggaggcgagtgcgttgcgcagaatcaaatacaggaaggggaacagctccgccgccataacgaagcccattccccacacggagttgacggcggagcgcacagcggagccagcggtctcccccagcagcatgtcggcaacaccgcgcaggcgcgtgaaatccatccacgccagcgccgcagcgaacggcggggtcatgaacgggatcatgaccatcacctcgacccagcccgccttgcgcatgggcgtccatgcgcggaagaaggcgagcggcgcggcgaagagagtcgagaagaacacgacgaggacggaaagccacaccgtgttgccgatgatgcggagcatctccgggcgcagcagcgtgtccagtgcggagtcctcaccccggtagccggtcaccgctgtcaccagcacggagaacagcggtgccgctactagaatgagcaagatgaccagcaccaggtagagcccggcgttgggcttcgctttcgtcctcatgagcgcggtgtcctacttacttcaggtagcgatccgcgaactgctcgcggatgttcttggactccttggagatcgcggaccagtcgtcggagatctgcttgatgtccttcagcgccgggccgttcttcggctcgacgttcttgttcgccgggatcatgttcttggacgcagagatctgctgcgcttcctcggagaacatgaagtcgacgaacgccttagcggcatccatgttgtcggtggtcttcatgatcatgaccgggcgcggggtgacggtggtgccggaggacgggatgacaacctcgagcggctcgcccttgccctgtgcggagtaggccgagtagtcaacgccaccgaagacgatgcccttcgagccggaggtgaccatatcgagggccgggccgttagcaccctggacgatcatgccgttgtcgaagagcttgtcaaacatctcccaggtcttctcctcgccccactcggacaccatcgcggcaagcaaatcggccgcggtgccggactcgcgcgggtccggcatgatgacctggtccttgtacttcgggtcggtcaggtcctcccagtcggtcgggatgtcggagacaacgtcggtgttggcaacgagggcgagagcggagccgtcacggccgtggaaagtgtcgtcggaggcgttccagtcagcgttggcgtccgcaatgttctccggcgcgtacgcctcgagtgcgccagactcggcctgcttggaggcagcgttccaggatgcgaggtagacgacgtcggcctgcgggttagcctcttcagccttgatcttggccgtgatgtcgccggtggtgccggcgaagacgttgacggtgacgccggtgcggtcctggaaagcctccacaagcgcgtcggtcaggccctgcgggttcgccgagtagtagtcgatggagccggagaggccctcaggtgccttccactccgcggcggtagcgttcgagtcagctgcgccgctggtcggggtggcggtgtcgttcgactcgacggagccgcaggccgcgagggtgagcgcggcggacaggccgagaacggccgaagcaaacttcttcatgacaatccttcttctggtcaaacaggggaaacaatcaacgggcgttgacggtcaggagaacctggtcgccgcggcccaggcggtgccgggtgtaggcgagccaaggctcgtccgcgccgggaacagtgcaccggatgtcgtagcgaccgccggtgtagtggctctccaccacctcgccgacgatggagtccgccggaaggggctccggcggctgcccatcgagcggggtcacctgcacatcttccggccggttcgccggaagacggtcgtgcgtgttggtcacgccgacaaagccggcaacgaacgcgtcggccggatggtcgtacatctccaccgggtccgcaaactggcggacgttgccggcgttcatgaccgcgacacggtccgacatggccagcgcttcggcctggtcgtgggtcacgtagatcacggtgaggttcaactcgtaggcgagtttggtcagctccgagcggatctgggttcggagggcggcgtcgagggcggacaacggctcgtccataagcaaaagctccgggtcggacaccagcgcacgcgcgatggccacacgctgctgctggccgccggaaagctggttcgggcgctgctgcgctttcgagctgatgccgaccatgtccatcgcgcgggcgacgcgcgcctcacgctcggacttagccaccttctggctgccggtggtcagcgggaactcgacgttcttggccacagtcatgtgcggccacagcgcaaggtcctggaacaccatggacaggttgcgtttgttcacgggaacattgacggaggggccgaaaacttcccttccggcgaactcgatcacaccagcgtccggggtttcgaggcccgcgatgcagcgaagcagcgtcgacttgccgcagccggacgggccgaggatggagacgaactcgcctttcttgatatccagcgatgtctcgtgcagaccggtgccgtccgcaaactcgcgccgcacgccgcgcagggagacttggttcgtaccttccaaaatcactcggggcatgataacggtcaatagtaatatgtcaattactttaaagttacgactcgatgaactttcctacgacccgagcgcgtcgacggaatacgcgagccacatcatcgcggcacctagcgcggaggcgaacacggcatcgaaacgccgagagcgtacggcgacgagcccaatttcgcgggagtcacaggtcaggcgcatgagcgcgagccacaccatcgacgcgccgagggtaaatgtggcgcggcgccagtgttcagtggccgcgaacacgccggaggcaagcaccccgaccacaagcagcacccacatcgcccgctgcgcccatctgggcagcggggaggccgcgttgccgcggtcgtgcgggttgtccagggtcggatgcgtcacggttgttactgcgcagcctggcgctcggcgctctccacaatgttgcgcacaaggaacgtgcgggtcattgggcccacgccgcccgggttcggggagacccagccggccttctcccacacatccgggtgcaggtcgcccacggttttgccgtcgacgcgggaaacgccgacgtcgagaagcgcggcgccctccttgatcatgtccgcggtgatcatgtgcggcttgccggcggcggcgatgatcacgtccgcgcggcgcgtttccgcggccaggtctttcgtgccggtgtggcacagcacggtggtggcgttgacgccgcgggaggtgagcatgagcgaaatcggccggcccacggtcacgccgcggccgatgacgcacacgatcgcgccgttcaactccacaccgaagcgttgcagcagcttgatcgagccgttcggggtgcacggcagcggcgccggctcattgagcaccagcttgcccaggttcaccgggtgcagaccgtcggcgtccttatctgggtcgatcagctcgaggacgcggttttcattgaggtgcttcggcaggggcagctgcacgatgtatccggtgacggctgggtcgttgttcagtgcgtcgataagctgctccagctcctcctgcgtcgtatcctccggcagctccttttgaatcgaagcaatgccaagctcctcgcagtccttgtgcttcatgcgcacgtagttctggctggcggggtccgagccgacgagcaccgtggcaagccccggggtgatgccgcgctccttgagcgcggcgacgcgttccttgagatcagcgaagatctcctcgcggtaaagttttccgtccagtttgatcgcagtcacgccctcgattctagacttaacccccgtgcgccccctgaacatcatcttcgacaaccccgtcatccccggaaacaccggcaacgctatccgcctcgccgcgaacacgggcgccgtgctgcacttggttgagccgctcggcttcaacttcgacgacaagcacgtaaaacgtgcgggcctggattaccacgatctggcggacgtgcagatccataagtacctcgatgcgtgcctggctgcgctgccggacgcgcgcgtgttcgcgttcaccacgcaagccaccacgttttaccaggatgtggcgtacgagtggggcgacgcgctgctcttcggcactgagccgaccgggctgccggaggagcactcgcaccacccgcgcgtgaccgaccggctgcgcatcccgatggtcgcgggacgccgctcgatgaacctgaccaactcagcgtcggtcgcggtgttcgaggcgtggcgccagcttggtttcgcaggcgggatctaaccgaagcgcttgtcccaacgctgctggtagaacggcggaaggatgttcagctcccacatcttgcgggcaagctggtcgtcgcccatccagccggcgaacgcctcacccatggtgaaaccgtgcgacggggcaggcttggccgcgatcacgtcacctgcccggaccaccccctcccgaatgacgcggaagtaggcgccgcagtcccccgcctcggtgaagcggcgcacccacgcgcgctcgcccatccactgcgcgaatgtgcggcacggggtgcgcggcacgctgacttccagttccgcttccccgatctggaagcgctggttgatcaccgcgtccgcccacacaatgcccgaggtggtgaggttctcgccgaacgcaccgttcggcagctcgcggctgagctcgcgcccccactggtcaagcagctcgcgtgagtaggcgtagaccgctttctgctggccgccgtggtgcttggtgtcgccgatgtggtcgcctgcgataccggagccgtcgccgtagtccggtcccggaatgatcacgtcgatcttttccgccgggatcttgttgatgccgctttgccgcttcagcccgcccggatccgggacggggcgcgcaatgttggtggagagcacggtgggggtcgctggggaggtcacgctggccatgcgtgtcaggctaccggcaaccgctaacggaaatcgcgcgagccgcgggagagccagtcgcccattgccagcgagcgcttagcgcgatatagtcaagaacactaagccggattttgccggcacattggcaacggccctcgtctttgtgacgggggctgtcctcattcaaggggggacctttccaacgcctcgagtatccaccggtgccgtgatccagtcgggtgttccgccattgcggaggttccacgaggaaaacccattatcaatggtgtttctgagctcaacctcaacaaccccggtagtccgtaacaccactgccgcaaggtatgtgttccagaggtagagctttgcagcaagcacctctccccctattcctgccagctgctcgtagttttcccgcagtggtcctggcaaggactgcagtagcacccctgccgtcactgaatccacgggatttgtcgatagttccaccgtgccccctgttccatcccctgacagaactccccttgtaaatgccttgaatcttaacggaaatcgcgcgagccgcgggagagccagtcgcccattgccagcgcctccaacctgtcagccaccacactgacggcgcccgaggcgttctgcacgatcccgcgcaccaccatcgccttcgacgtgcgcgcaaccaccttctgccggttccaaagccccaccgagatcaccacgttcaccagccccgtttcatcctccatcccgagaaatgtcacgcctccggcggtggcggggtgctggcggtgagtgaccacaccggcgacacgcacacgagtgccgtccgcaacgtgggcaagttcgctagcgcgcagaaccccctcggcagtgaggcggctgcgcagcatctccaccggcatagtgccgggtgtgacaccggtggcggcgacgtccgcagccatcagctcgaacgcgttcatgccaggcagcgcgggcgcgctgatcgccgacatgcccggcagcatgccttcccgctccgtggcggcgatacccgcctgccacatcgcttgtctgcggtccacgccgaagcagtcgagcgcgcctgcgcgggcgagcgcctcgacgtgctccacggtgaggtccgcccggcgcgcgaggtccgggatgcctctaaacggctgggcggcctcgatgcggtctgcggcggcatcgcccaacccccggatgaggttcaagcccacacgaatggtcccgccgctgcggtcgccgcctaggcagcgcgcctcgcgccccgactcgttcacgtcgacaggcagcacgcgcacgccgtggcgccgcgcgtcctggatcaacgactgcggcgagtaaaaccccatcggttgagcccgcagcagccccacgcagaactgcgccgggtagtagaacttgaaccaggcggagaagtacaccagcgaagcgaaggactgggaatgcgactccggaaaaccgtaggcggcgaacgccacgatcttctgccacagccggtccgccacctccgcctcgatccggttggtggaccagcagccgtcgaagaagcgctgcttgagcgcctccatcttctccggggagcgcttcgagcccatggcgcggcgcaccccgtcggcctctcggccggaaaaacccgcggcgtcgacgcagatctgcatcagctgctcctggaacagcgggatgcccaacgtcttgcccagcgacttctcaagcaccgggtggtcgtaggtgaccggttccaacccgtcgcggcggcgcaggtacgggtggacggacccgccttggataggtcccgggcggatcagcgccacctccacgacgaggtcgaaaaagcagcgtggtttcagccgcggcagcgtgcccatctgcgcgcgggattccacctggaacacgccgacggaatcggcgcgggaaagcatggagtacacgtgggcgtcgtcaagcgggagctcccacaggcgcacttcgcggccggtggtgtccaaaaccaagtccatcatgtggtgcagcgcctcgagcatgccgaggcccagcagatcgaacttgaccaagcccgcggaggcgcagtcgtctttgtcccactgcaccaccgagcggtcctccatgcgcgcccactccgtgggcaccacgtccgcgatcgggcgatcacagatcaccatgccgccggagtggatgcccaagtggcgcggctggccgcggaactgctcggcgagctcggcgacgggaacaggcgggtccgcgatccccttcgaccaactgtcggcggcgccctgggcgtacccgagcgcccgcgccgcgtcgcggacagcgcctttcgtgcggtacgtgatcacgttggccacttgggcggcgttgtcgcgcccgtagcgggtgtagacgtactggatgacctcttcgcggcgaccggattcaatgtccaagtcgatgtcgggcgggccgtcgcggtcgggagagagaaatcgctcaaatagaaggcccgcctcgatcggttccacgctggtgatgccgagcgcgaagcagactgcggagttggccgccgaaccgcggccctggcacaggatgttcttgcggcggcagaagtcgacgaggtcgtggacgataaggaagtagccggggaagttcagctcctcgatcaccatcagctcatactcgatttgtttcttcgcccgcgcacgcacatccagcgtccgggaagcgtagcggacctgagcgctagacagcgtgagcaggcgcaaaaagctcatctcgtcgtgcccctcgggcgtggggtacgccggcagctccggggcgaccaggtcgagcgtgaacgcgcattgcgaggcgagctcggcggcgtaggccaccttctcctcgcacccgggaacaagtcgcagcagctggtccgcggagcgcaaccagttcgcccccatcgggtgcagctcgccgtgggcctggtcaagggactcgcggcgcgccagcgcgcgcttggcggcggcaagcctcgccgcgtcgcgggtggcggcagcggggacggcggtgacgatcgccgggatgtgaacgaagcggtctagtgattcgtgccgatccgcgtcttccggcagcatcgagacctcgtattcgcgcacgacgttctcgcccccgaaggcatcgatcacgcggtcgaaatcgtccgcccactgccatcccgcgagcgcgacgcacgctcctcccagccgctcgccgataagctccagcggcgggtacgcaactttgcctttctcgcgggtggccatgtgcgcgtccgccatcaaatgcgacaggcggcggtagccctccggaccgcgggcgatgacgggcagaatgcggggctcctcctcgctgccgagtgtcagctccgcgccgaagactgtggcgatgccgcactcggcggcggcctcggcgaacttcaccgccccgtagaacccgtcgcggtccaggatggccagggcagataaacccagttccgcggcgcgggccacgaggtcttcaggttcgctcgccccgccgaggaagctgtaggaggacacggcgtgcagctccgcgaacgggcgcgcggcggcgcgcggggcggcagccgggcgagatggaagcagcccctccggggcaccggtgtgcgcggccggctgcggcgcagggcctggccggcccgacaggatacgctccaaacgggaccacgaaagcggctcgcccccgttgaatctcatgcttcccacgatagcagtgttcgaaactgtgttccaacgcttgcagcgaccggcgaagctccccacaaacgcccgaatagactaagcggtacggacggtgatagattctgcaaccgtaggtttttgcaccccccttgaaaagaaagcaagaggatccaacgtcatgcgcacttcccgcatcaccgcggcgctcgcagccgccaccatcgccgcgaccagcctggtcgcctgctccaacgagtccaactccaccgacgcgaccgacgcagccgctgagggcaacactgtcgtccgcatcggcaccaccgacgcagaccagcaggcgtggagcgtgttctccgacctcgccgaggagaacggcatcaccctcgacatcgtgcagttctccgactacccgccggtcaacgaggctctcgcgcagggcgagctggacctgaacaagttccagcacatcctctacctggctaagtacaacgccaactccggcaacgacctgaaggtcgtcggctccaccgagatctacccgctcgcgctgttctggaaggaccacgactccctcgacggcattgagggtaccgaggtcgcgatcccgaacgacgactccaaccagggccgcgcgatcaacgtgctggttcaggccggcctggtcaccctgaaggacggcgccgacgcgctcgcgccgaccccggctgacatcgactcggctgcctcgaaggtttctgtggtgccggttgacgcatctcagaccccgtccgcctacaaggagggccgcccggccatcatcaacaactcctggctggaccgcgccggcatcgagccaagcgaagctatcttccaggacgacccgggttcggagcagggcgagccgtacatcaacgtcttcgcgtcccgcgcggaagacgttgacaacccgacctacgtcaagctcgccgagctgtggcacgacgcagccgtcagcgaggccgtgcagaaggattcccgcggcaccgctgtcgaggttgagcgtccggcagacgagctgaacgacatcctcgaccgcctcgagcagaacgaaaagtaaatggctacaaccggcacccggattgaattccaggacgtcagcaaggtcttccgctccggcggccgcgaggtcgtcgcagttgacggcgtcacattaaccgtcgagcccggggagatcctcggcgtcatcggatactcgggtgccggtaagtcgacactcgtgcgcttgatcaacgggcttgatcaggcaacctcggggcagttgcttttagacggcactaacgtcgtcggccgctccgaaaaagaactccgcggcatccgccgcaacatcggcatgatcttccagcagttcaacctgctgacctcgcgcaccgccgccggcaacgtggagtacccgctgcagttggcgggcgcgggcaaggccgagcgcaaggcgcgcgttgcagagctgctcgacttcgtcggcctgtcggagcgcggggacaactaccccgagcagctctccggcggccagaagcagcgcgtcggcatcgcccgcgctctcgcgacgaacccgtcgcttttgcttgccgacgaagccacctccgcactcgaccccgaaaccaccgaagaggtgctcgcgcttctccgccgtgtcaacgaggagctcggcatcaccatcgtggtgatcacccacgagatggacgtgatccgctccatcgccgacaaggtcgccgtgatggaaaacggccgcgtggtggagtacggctccgtctacgaggtgttctcgcacccgcagactcacgtggcgaagcgcttcgtctcgaccagcctgcgcaacacaccgaacgaggtggaggcgcgcgagcttttggacgcagcgcccggccgcctcttcaccgtggatctcaaggagaactccggcttcttcggcgccgccgagaccgcccgcgcgaagggggtcaccgtgcagccggttcacgccggcatcgccaccttgcagcagcactcgttcggcaagatgacggtgcgcctcaacggcgacgacgcggcgatcaacgagttcctgtccacgctgcagctcaccaccgacatcgaggagatcacccgatgacgagcaacatcaacgaattcatcctcgcggagccgaactgggaccgcctcggccccacctttgtttctgcgatcggggacacgctgtggatggtggcgatcaccatggtcgtcggaggcttcttcggcctgctcctcggcatcttcctctacaccacccgcccgggcggcatcttgcagaaccgcgcggtgtacacgctgatcaatgtggccgtgaacttcttccggccaatcccgttcatcatcatgatcgcaatgctctaccccatcaccctggcggtggtgggtaccacgatcggccgctcggccgccacgttcgtgatgtgcttctcagcgacgttcaccgtcgcgcgcattgtggagcaaaaccttgtcgccatcgaccccggcgtgatcgaggcagcccgctccatgggcgcaggcccgtggacgatcatccgcacggtgatcctgccggaggccctcggcccgctgattctgggatacacgttcatcttcatcgccgtgatcgacatgtccgcgatggcgggctacatcggcggcggcggcttgggcgacttcgcgatcgtgtacggctaccgccagttcgaaccgcaggtgacgtgggctgcggtcatcgtgatcgtggtcgtggtccagctggcgcagttcctgggcaactggctgtcgaagaaggtcatgcgccgctaggtacgcttgatcagcgtgaagattgcggcattcgacttcgacggcaccctgctccacagccgcggcgacggcacccacagcttcaacgcggaagacttagaggccatccgcgcgtggcgggaggcgggccacctcgccgtcgccgccaccggtcgctcacgctccgcgctcaccttcggcatcggggacgccgacctcacctacgactaccgggtgctttccaacggcgcctcggccaccaccggcgacgatgacgagctcatctacgcctaccccattgacccggacatcctgcgcgccgcggttgctgagttcaagaacactgccgacgtcgctgtcttcggcaccacggtcgggcccatcgacggcgcgtttgttttgaacaccccgcgggtctcggcgttcaccggccacttcacccgtctgaccacggacgacatcgaccaccacacctttgccgtggtgccgatctgggtgccggagaacgaggcgctgcgcgcgaacgtggtgcgctgggcccagcggttcgacaacgtcaccgtcgcgcagaaccaggactacgtggacattatggctgccggccgcagcaagggcacgggcatcctcgaactgttgcgcacgctcggcgcgcggcgcgaggacgtggagctctactccttcggcgactcgtggaacgacctgtccatgcacgatgccgcggacatttcgcacagcttcccgcattcgcccgcggacgtccaggctgcgacggaccacgtcatcgacgcggtcgcggacgcgctcctccgctacatctaaacgcgcaagttaaacgcgctcgactgcgtccaccacccacgcctgaccggtcttcggttgcttgccacaggagtcgacgacaccgccgatgtcgcgaagactgagcgccacctcgtacgcggcgccggtggccgtgtcggtgactcgcacgttggagcggttggtggtgattgtgggggcgtcgacaagcagctgctccatgccaacctgcgcaccgccgcgcgacagctctgccgctaccgcgatttccgctgcctgcgccggtgccgaaagggtgccgcggccgcggttgccgggcacgaagtacagccccgcctcggcgtgctcgagcaacgcacgggctgcctgctcgttcatcctcccgtaactgaacgcccacggcatcagcagcattgtcggcgcgaacctgtggcccttgatgtgcgaggtctcccacaccatgtcgtcgctgcgctgcaactgccggaccagcgggcggcccttgatcgcgcagcactggtcgcgcttggcgtgggtgcacaccaacagcaggggctttgttcttaccgacgcccccctattcttccccggacccgataaatccagatccaaaaccgcctccggcccgtcgacgtggaggacctcggttacaccctggtcggcgaagacgaggtagacgtggtggtcctggatgagccggcgctcgcgtgttgcgtggcgaatcaacaaaaacgtggcgtggtttgcctccacgtggtccttgatccgggcagacaactcaggtcccaaggtgtcgccgtcgagcacgtcgcggctccaggcatccggccactcgaagaggacgtaggtggatcctggtttggcggtgccgggcagcggctcgacctcgacatctgagcaatgcatgcccttcactctaactacttaacgtttcggtaaccattgccccgaacacccctcttgagttttgccgcccaacgcggccgagttagcgtgaattttgtgttttttcttcccccgtcggcccaagatgccgcgcgccgcgcagctggggtggctgcagcggccgccgcgctgtggcttggggtggcgggctgcgggcaagtgcccgcggtcggcgacggttctaggagcgctccgcttagccaacctgcggtgatggccggggttggcccgcaccacactgggtctgccacatccaccaccggcacggcggtgctcagacccctcggctcggccaacccgtcgccaaagacgcagcgcccctcggagccggcgcagctcgcagtagctggtgtccgcgtgggcaaccacgaaggtttcgaccgcgtggtggtagatctcgccggcgacggcgacccaggctggttcgtcgactacaccccgacgccgctgcaggccacgatcggccgcccgcttccggtcagcggcaccgcgtttttgagcatcaacgtcgacggcactgtgtaccccggcgaactcggcttggacgagaccggtgtcgagcgcttgagcccgacgagcaacatcgtcgacgttgccagcggcggcacctacgccggccgcagccagatcgtggtgggcttgcgcgccgaggcgccctactccgtgcaggtgctcgaagacccgaagcgcttggttatcgacatcgtccaaggctagcgccgggctggtgctaatagacggcctccacacgccaactccgcctcgaccacacaagcaaccaccccgacaccggaccgtctgatcccccgagccggcccacgacctgcagccgcgccaccctgttgcggcgctctggggccgcccaccagccctcgtcgacgggccagggccccgcccacccggtgaccagatacttcttgtcgccccacttcagcgcatagggatcagcggatagtaacgcctcagcggtgacttggacggcggctgcatcggcgctgatcaacgtaatgccggaggcggggtggtcgatgcccccgccgaggcgcgccggcagcggcgccgggaccgcaccgggccacgactgctcggaaacctccggtggcacctcaccaaacggaaccatccggacgcgttccgcgacaccgcggccgcctacgaggcggggctgcaccaccgcgtcgatgcccagttgggactgcacccgctcaacgcagcggcgcgcgccgtctgaagacgcaccgtccgaccacagctcccctaccgactccggctcagcgagctccagcggctccaggatgagcgaagtgatagcgcctgcgccgccgccggtgagccagccgccgagctgccagcgcacccggtccgctgtgcccgattcgctcaacgcctcgcgcgtgcgccacacccgctcaacgcggtcgccgctttccagttccgcggtgatctttagccgcaggcagttacggccagcgtccttgaggcgctggtgcaaactcgccgccagcgcgcgggcggcgaaggcagccgcgtcgacacgctcgatcgggtcttccggggtgatcgccaccgcgaggtcggccaccggcaactccggggccacccggcggtccggcgcggccgcggcgatccggtgaagatgcatgccgctagcgccgaaccgtgtggtcatcgcggctggtggaatcgctgcgatgtctccgagagtggcgacaccaagctggctcagcgtgcgcaccgtgtccgcgtctgcgccgagagcaacctccgcggtgagcgccctgaccgggtgctggctgaggaacgccgccgactcccctggcggcacgatgtgtgatgtgcgcgcagcgatgacggcggtagcgatctcgtcggcggccccggcgaaggcgtcgatgccgcggcgcgacgccgcatcaataagcatctcgagcgcgcggtcctcgctgccgtgaaaacgggccgccgcctcgagatccgcgaccacgaggcccgggcgcagcacctcgacggacgcggcgacgtcgtccaaactggcgccgagggaggcgaacatgcgcccgtcgcggtccgggttgtcctcgatgacagtgagttcgggagcagcggcttgcgcgttgcgcacccgcatgccgcggcgaatcccgagcgcgcgggcggcgcgcgagcacaccttgatgcggtgctggctggcgatggcgacgggttcttcaatctcatcgtccaactcaagcttcgccgcctgcaccggccaatccggaaaccacagcgcagcgacgcgcaccctacatcaccacctgcagtttcggacgatccagttgctgctgctgcgccggggcgcgccccagggtgacggtcgcgctcgctgggcgggcacccttctgctcggctcgcacacgcagctcaatgccgcggatgcggcccgtcccacggccgataccgtgaaaatcagcgatcgcgccctcgagggacagcgccggcgagggcacgcggacgttgactgccatgagcgcggcgttgcctttgcgcacacgggcgagcaggggccgcgcgcgcaccggggtgagctcgagcgcggtgcgcgagcgcaggaccaccaagtcgagcccctccgccagcacgccagcaaccgcgagatcctcgatgcccggatcggggacagcgataacgcgttcaagcccgtcgcggtctacgcccgcgtacgacagctccggccaccccaccacgccggcgtgcccgccggctgcggtgacttggtcaatgacctccaccaccagcgacggcgtgtcactgcagtggctcacggcttgcctaggcagcccgccgttcggcagcacgtgcgagagcggtcctggcacagcgaggacctcggcatcctctacaaccgggcgggggacctccccgccgagctgcgccatcttcgcccttaactgggcaatctgctcagcacgactaggctgcgctgcagcttcttgcacccccgcggcctccccggggggcgccgcgagtgctcgaatagacgttccactcacgccgttcagtatgcaccgcgcccccaacacagacaaccacaaaggtcgaacacattttctaaaccgaaacgtagtctctcttttattcgcccagctgttccgcggtaacgtacctacacgtgaacccgctttccgcatccgatgcccgcaaccgcgtcacgccgattccgactcctgcacccgtgcggcttgttggctcagcgggcgcagctgggtcggtcgcaatcatggtgtcgcagcttgccactggcgcgaaactagtgatcgcactggcgtgcgtggcggcggccctgacaataacgctggcgcacccataccgaaagcggatgcgggagtatgcggatgtgagaagagtggacaggaggccgtcgataagcatgctgcttccgctgatgctgtggtggctactgctgatgctggcgccgctggccggctggcctgcgtggggtgccgtaacctgcttcatcgttctcttcggcgcggcgtgggtgctgttcccccacgtggacggatcgcgccgcctggcctacgcggactagaaagcgcggagggaaatctactcgaaaccgtttcgagtagatgaaaaactgcagctcaaactagaaacattcgtttcgagtagatttcgagtagctgtttcgagcacttgtttcgaactcaccgccgacctgatgttgggtacgtagggaacaatgaagccatggaaaacagcggcagcagaagcggctttcaagccgagctggacaggatgtgggaaacgcgcccgccgcgcatcccgaaggatcagggcggcaaggcactgataggcggcgtgtgcgagggtatcggcgcgcgctacaagctggatccggtgctggtccggctggtgtttgtcgcactgagccttgctggcggcggcggcatttttctgtacctgctgtgctggctcaacatgccccgcttcggcatggtggtcagccccggcaaggcgattacggcgcagagttccacgctcacggagatggaaaagcgcgaacgctccaccggttgggcgctcattgtcgggctggtgatcttccttccctccgcgaccaccggcgagggtctcagatcactgttggtcatggcggcggttgcgttcactgcttggtacttggcctacaaacgcgcgccagagccgccggccggccttctgccgccgaaacagagcgcaagcaccacccgcgctctgccgaacccccacccgttccagctcgacccgagcgtccggcggccctacgacgtgcagccggtgcaaccgccgcacaccgcgcaacctccgcacccgtacgcgcagccgccgcggcaaccggacccgcaaccggcagcgccgcacgcagacgaaccgaccccgttgtttgatttcacgcacctgacccctccgcaggggtatccgcaccctgctgtcggccgcgccactcccccggcgtgggatccgctcggcaccgcccccgaactgtggcacttgcccgatcccgcggccgcggacgcctccccggcaccgcagactcaagcgcctacggcgcacgaccgcggctcgaagcgccgctggctgtggctgcccgtcggcctcgcagggctcggcatcgcgggtgcggtgatcgcggcggggccgaacgtcagccgctactccttcggagcgggtccgaactgggcaaccggcgacatcaccctcacctacgacgacgtcgaagcgatcccggacctgcaccgtctcgccggggacatcaccttggacctgcgggagttggagccgttggactcgcccgcgacgatcgagatcggcaactacttcggcaacatcgacatcctgctgccggagaacgtgccggtagacactcgttgcgaggtgggctccggctctgccttgtgcccgagcaacaccgtaaacgagcgcgccgacgggcaacttctgaccatcgacgcgcgccagtacatgggcacggtgaccgctcattaaatccgcacacatcgccatcgtcggtgccggcccccgcggcatctcgatcacagaacgcattgccgcctacctgcgctcccaccccacagatgcaccgttcacactccacgtgatcgacgacgcacagatcggcgccggccgcgtgtgggacacccgccaaatccgaacgctgtgcatgaacactctcgccggcgcagtcacgctgttcgctgagcccggagcgaccgtcacggcccccgtgctcgagggcccgaccatgtacgaatggatccagttgctgcgcggcgaggtcggaggcatcagcgacgcgaagcgcgcgccgtttgttgccatcactccggatgtcccagcggagttcgcagacgagatcgccgccacccgccccgagtccaacccgtcccgcgcgctctacggcgagtacctgcgctgggtgtggcgcgtggcaaaagcagcgcttcccgcaaacgccgcggtggttgagcacaacgctcgggtggtcggcatcaggcaggctcgaggcctcgatgagctgctgcttgacgacgccacgttgatcccctcttccgccaccgccctggcaaccgggtgggtgctccccgtcctgccggaggttgcgggcgcgagggaggcaggcgccgggttcacctacgtcaccgccaacaaccccgtcgagcaggacatcgcggcgcttcgccccggcgaacgcgtcctcgtgcgcggtttgggcatgggatttttcgacctcatggcccttgccaccgttgaccgcggcggccgtttcatccctgacaactccaaagctgccggggtgcgctacgagccttcaggggaagagccgcacctgattgccacttccgggcgcggctacccgtacctgccgaaatcggagtaccgctcgcttccgccgaaagcgaacttggtgcggttgcacgccgcgatgacagcggccgatcagtcgggggagcctgtgtccttcggccgcgacctgtggccggccctcgcgcgtgacgcatacagcgagttttaccgcaccgtcgccgagaagcacccgcaggcgctgcgcatttcactctacgaggtgctcgccatcatcgacactgtcgacttggtcactcccgccacgacacagagcatcctcccagtggcgagcgcgctgacggccgcgcttgtaggtgtgatcgacgccgacagcattgagccgttcgacatgacgcgctggattgacccgctcgcaggcaccgcttccgcgacaacggatgagctgggcgcgctgatcgtagccggcatggcgcgtgatatctcggaagcggaggccgcgtgggattcgccgctcaaggcggggttgtgggcgatctccgcgggccgcaagccggttgccatcgcgacggagaacggccgaggcgcacccgaacacgcgctgtcgcagtacatggcgttcggccagatggtgggcagcggccctccgctgttccgtacccgagagctgctcgccctgcacgaggcgggcttggtcacgttcctcggaccgcagcctactgtccgcgtcgagaacggggcggtcgtggccacgagcggtgagcgcaccgcccgggcctccgcgctggccgacgccttcctccccggcccagatctccgccgcgccgccgacccgctcacggcagcactcgttgcaagcggccgcgtgcgcccgttcgcgcccagcggcacccccaccgcagcgccggagaccgacgacgccacccgccgcgcggtgcaccccgacggctcactcgatcaacgcctccacatagttggcatccccaccggcgaacagtgggcggacaccaccatctcccccatgcccggcaccgacccgctcatgctccaagagacagataaggccgcccgctcgttactacgagcagccggcctgatcggttaagcgctacagcgcgcagcgcgttactcccactcgatggtggcgggcggcttcgacgtcacgtcgaggaccacgcggttgacatccgctacctcgttggtgatgcgggtggagataacctccagcgtctcgtacggcacgcggacccagtccgcggtcatcgcgtcctcggaggcgaccgggcgcagcacaatcgggtggccgtaggtgcggccgtcgccctgcacgccgacggagcgcacgtccgcgagcagcacaaccgggcactgccagatctgctcgtcgagtccagcctttgtcagctcctcgcgggcaatcgcgtcagccgcgcgcagggtgtcgaggcgctcctcggtgacctcaccgatgatgcggatgcccaggcccgggcccgggaacggctggcggttcacgatgacctcgggcaagccgagctcgcggccaacggcgcgaacctcgtccttgaacagcaggcgcaacggctcaacgagcgtgaactccacgtcgtccggcagaccgccaacgttgtggtggctcttgatattcgccgtgccggtacctccgccggactcaaccacgtcggggtagagcgtgccctgcaccaagaaatcgacgtcctggtccgacagcacatccgccactgcgcgctcgaaggagcgaatgaactcggcgccgatcgctttgcgcttcgcttctggctcggtcaccccggcgagcttgtccagaaacgcggcgcgctcgtccacagtcaccagtttcgcgccggtcgccgcgacgaagtcggtctcgacttgctcgcgctcgccctggcgcagcagaccgtggtccacgaacacgcaggtgagacggtcaccaattgcgcgctggacaatcgcggccgccacagcggagtcgacaccgccggacagtccgcagatcgcgcgaccttcaccgacctgctcgcgcacctgctcgatgagctggtcggcgatgttagatgcggtccagttctgctccacaccggcgatctcggtgaggaagcgagtcagcacctgctggccgtgaggagagtgcagcacctctgggtggtactgcacacccgcgaacttgcgctcgaagttctcgaacgcagcgaccggcgctcccggcgtagacgcggtgacggtgaagccctccggcgcctcagtaacggaatcaccgtgcgacatccacaccgggtgagactcggacaggccgttgtgcagcacgccgcccgtgacggtcatctgggtgcggccgtactcgcgcgcgccggtctcggcgacggtgccgccgagcgcccgcgtcatcagctggaagccgtagcaaatgccgaagatcggcaaatccagctcgaaaatcgccgggtcgaggtgcggggctccgtcggcgtacacggacgacgggccgccggagagcacgagcgcaaccgggtctttcgctttcagctcgtcggcggtgatggtggagggcaccacctccgagtacacgttcgcctcgcgcacgcggcgggcgatcaactgggcgtactgggcgccgaaatcaacgactaaaacggggcgggtttgcggagtagtcacggtgacaaatgataaccgatcgcgctacctccgcgaacacccgaaccctagagccttgggcgcaccgccagctgcaccttctgaaagctcttgacagtggtgtagccgcatttcgccatcgtccggcgcagcgcaccgaccaagttcaggttgccccatgggtcactggacgggccgttgagcaccacctcgagcgggaacttggggtggtcgaaatcaggcatgacagccccgcgcgggttgcgcgggtgcgcggcctgggcctcccagtacacgccgcccgcggcggcctcttcggcgcgcgccaaggggaggccgaccatgactgcgtcggcgccgcacgccaaagaaacggcgatctcgttggcgttatacacctccgagtcggcgatgacatgcacgtagcggccctctgtctcgtcgaggtagtcgcggcgcgcagccgcgacatccgcaatagcggtggcgataggaagccccatgttctgcgggccgaaactcattccggagccgacaatgacacccgccacgcctgcgcgcatcaggtgtgtcgcggtggcgtagtcgaacacgccgccagcaatgaccgggacctcgagcgaaccgacgaactccttcaggttgagcgactctccgcccttttgcacgtgctcggcggaaaccagcgcgccttggatgaagaggatctcggcaccagcggcgatcaccacgggagcaagttcgcgcgcgttctgcggactcacgcgcaccgcgacagtgacaccggagtcgcggacctggcggatgcgctcccaaagcaggtcatggtcgagttccgcggcgtgcagcttttgcagcacctccgtagcttgcgtatcaaccccgtcggggtttgccacggcgaccacctgagcaatcgccgcatcgaggtctgcgtggcggccccacagcccctcggcatcaatcaccccgagcgcgccctgcttgcccatctcgatgacaaactcggggctggctagcgcatccgttgggtgggacacgatcggcacgtcgaagatgtaggcgtcaacgtgccacgtggtgtccacgtcttgcgaggaacgggtgcggcgggtggggaccagcgatacgtcggaaagcgaataggccctccgggcctcgcggccaataccgatttctactgtttcgcgcatgctgctcctagccgcggtagttcggcgcttcgaccgtctgcgtgatgtcgtgcgggtggctctcacgcaagcccgccgccgtgatctggacgaactgcttcgtctgcagctcctccaccgacgcggagccggtgtagcccatcgctgcgcgtaagccgcccacgatctggtgggtgatcgcgtcgatctcaccgcggtagggcacgcgaccctcaataccctccggcacgagcttgtcctcggtggcaacgtcagcctggaagtagcggtccttggagaaggaacgcttttcgcccgtcaggccgcggccctgcatcgcgcccatggaacccatgccgcggtagcgcttgtactgcttgccgcccacgaccacgatctcgcccggagcctcggcggtgccggcgagcatcgagccgagcatgacagaggacgcaccggctgcgatggccttggccacgtcgccggagtgctgcataccgccgtcggcgataaccgggataccagccttcttcgccggcacggacgcctcaagaatcgcggtgatctgcggggcaccgacacccgccacaacgcgggtggtgcagatggagccggggccgataccgaccttgatggcgtcagcgccagcgtcgatcatggcctgcgcagcgctgcgggtggccaggttgccgccgatgacgtcgacgcggtcaccgaagtccttcttcacgcgggagaccatctcaagcacgcggttgttgtgcgcgtgtgcggagtcgaccaccagcgcgttcacgccagcctcaaccagcatcccggcgcgctcgtatgcgtcctcgccggtgcccacgcccgcggcgaccatcaggcggccctcggcgtccttagaggcgttcgggtactgctcgctcttgacaaagtccttcaccgtgatcaggccggcgagggtgccgttgtccgaaacgatcggcagcttctccaccttgttggcggacagaagggacagggcctcctccttgctcacgccctccttggccacgaccagcggcattggggtcatcacctcagcgaccttgcggtcgaagtccggctcaaagcgcatgtcacggttggtgatgatgccaaccaaacggccgccctcatcaaccaccgggaggccggaaatgcggaagcgagcgcacagcacgtcaacgtcgcgcagcgtcatctccggtgttgcggtgaccgggtcggtgaccatgccggactcggagcgcttcacaatgtcgacctgctccgcctgctcctgcgcgctcaggttgcggtgcagcacgccgatacctccctggcgtgccatggcaattgccatgcgggactcggtgaccgtgtccatcgccgcagacgcgatcgggatgcgcagcgaaatgttgcgggtgaactgggttgcggtggagacctcggacgggacaatgtgcgactccgccggaagcagcagcacatcgtcgaacgtcaagccacgcaacgccaccttctccgggtcgtcgcctccggtgagaactcgctcagttgccatgtgttcctctcctgacagttacggcttttgcacataatattacgcacctcccacacacggcctaacgccggtgaaagcccagcacagctgcgttcggagcgaaggaggcggggcgaggattccgtgtttgcgcgggtgactagagttgggccttgtgagttacgacgacatgatgcccctcgacccgttcgcggacgacccgaacgatccggcatcgttcatcgaggacgacgaggtcgccgagccgctctccgagcaagagcgcgcagaggtaatccaggacctgggctacgtgcgcgactgcatgcgccggctgcgcccgcgaggcatccagggcattttcttccagtgcgaagactgcgagcagctgcactactacgactgggaaatcatggagcagaacatgctcgcgtccctgcgcggcgagctgccgccggtgcacgagccgggcgccgacccgaacgtcgatgcgtacgtgccgtgggagtacgccatgggcttcctcgacgggctggacgcccgctagcccctaccccctagccccccctgtgcaccggcgctcaccgcgccggtacgacttgcggcgccacctcgtcaacaccagcgccgtagctcgactgggtgttgacctgcggggactgcttcggcaccacctgaggcacctgcccttcaccctgtggcgcgctggtttgcaccttcggcgaggactgcccaggctggggcgcctgagacgactggcggctgttctggctcgcctgcccctggtttgtcggagactgcggctgcgccggctgactctgctgcgctgacggcgcaggctgctgcggctgggtgggctgggcaggttgcgccggctgcggcgcctggtgcgagctcggcgcgggctgggccgccgacgggttcgccggcgcggccggttcctgttgcgccggcttgtctggctgcgccggacgctcctgctccggcgaaacagtcaccgtcacggtcaccgtcgccggccgctccccgtcacgtgccgcatcatcatctgcgctgccctcaccagggcccgggaccgggttcatcgactccaccagccggttcgcctgctgcagcagctgggcaaggtagtcggaatcgcccgcttggctcgccacttcgatctctttgagggtggacgccagctccaccgcggcagcgcggtcgccgaagactgcggtagaagcgccccacaacggggagcccggggttgcgttgtacagcgccgcgcccgatccggcgatcagggctgaggctgctgcagcgccgataaacccggcagcccacggattcatcctcgtgcgcttggggcttgttgcttgccgacgccccgccgcctcccccatcccgcccacaccagtctgggcgcgtttcgtgcgctgctccgcaagcgagatcggctccgcaggttccggctcgaccgcgtcaaccgagggctcttccggcatcggccgctcgatgtctcgtttcatggccagcaaaagtcccgcgagcggatcggccccgtgcgtggggtcctccccgcgtgcgagcgcgtcgagcagcgcatcggtgccgtctaccggcgcgaactgcgtggtcgcgtcttcttcgtggtgctcatcggcgcgccgtgtcatctcactggtcctgttcttcgatcatcgtgcgcagcttcgcaatcgcgcggtgctgagccacccgcaccgcgcccggggttgaacccacggcctcggctgtttcttccgcagaaaggcccacaaacacccgcaggataatgatgtcgcgcgccttatcacctagttcatcgagtaaaccctcaatttggttacgcgcatccacgtcaatggcgtaagcctcgggggtaacccccgtgtccaccgtgtccggcacctcttccgtgggggtgagcttgtcgcggaacagagcccgatgcgcgtcggcgaccttgttgaacgcgatgccgtacacgaacgccatgaacggtttgcccatgttttggtacttgtgaattgaggtggccactgccaggcacacttcttgcgcgacgtcttccgcggtcggagttcgcccgccaccgatgcgcgcgcgggtgtagcgcagcacgttggggtggatgaggcggataacccgctgtagagccttcgcgtcgccgccggcggcgaggggcacaagccgggcgagctcgtcttcggtgtccggttgcggcacggcgctccttcctcttgtgcatcacgcctcaacgcgtcagttggtcagcgtacaactgcccgcccccgcaccacaggttcaggggctaggttccgcaggctatgaacttttaggctgaaattcacccacgcttaaccttgagcaaattcccagcttaaagcgtcgtttttcccagggtcaagagtgtttaaagcttcacgttaccgcacggttacccgccgttcacccgggcagagaacactacttttccggcactacttgaggcacacaataaggagctagacgacaatgtccctgccgcacttgcttcccggaccgaacgccgatttttgggattggcagctgcatagcgcttgccgcggtgaagcgtcagagatcttctaccacccggacggcgagcgcggcagggctcgcacgcaacgcgagaaccgcgccaaggcgatctgctaccagtgcccggtgctttcccagtgtcgcgaacacgccctgcgcgtggctgagccgtacggcatctggggcggaatgagcgagtccgagcgccaggcggcgctgcgcggcgcacgcggcggtgtgaaggtggccgcagcgtccgccaagtaggtccaaggcttagcgacgcaagccccaacaccaagtgaaggccctgcccccgttttacggggccagggccttcgcgttgccgtacgacggcgagcgcggcagttagtgggcgtgggcgtggccgtgctcggcctcgtcctcttcctccggcttcgtcaccacggatgcctccgtagtcagcaccatgcgggccacggatgcggcgttgaccactgcggagtgggtcaccttcaccgggtcgatgatgccctgctcgatcaggttgccgtactccaaggtggcggcgttgaagccttcgccgttgcccacctcagcgatcttggacacgacaaccgcgccgtcgagaccggcgttttctgcgatccagtacgccggcttggtcagcgcgcgcgacaccgccagaacaccggtgcgctgctcgccctcgaaaccgtcggcgtaggtctccagctccttcgcaatctgcacgagcgcggagccgccgccggcgatgatgccttcctgggccgcggcgcgcgcggcgttgatggcgtcctcgacgcgcaacttgcgctcgttcatctcggtttcggtggccgcgccgacgcggatcaccgcgacgccgccggagagcttcgccaagcgctcctccatcttttcgcggtcccacgtcgaatccgtggtctcgatgtcgcggcgcagctggttgcggcgctcctccaccgcctcggcggagccggcaccgtcgacgatgacggtgtcgtccttcgtcaccgtcacgcgacgcgcggaacccaagtgctccaaggtggcgtccttcaagttcacgccaacctcggggtcgatcaccgtggcgttggtgaccactgcgaggtcgtccatgaacgcggtgcggcgctcgccgaagtacggggacttcacagcgacgaccttaatggtcttacgcagggtgttcaccaccagcgtctgcaacggctcgccctcaacgtcctccgcgatgatgagcagcggcaccgactcggttgccacctgctccagaagcgggaggaagtccggcagcgaggagatcttgttgcggacgaggagaacgcgcgcgtcgtcaagcaccgcctggcctgcgtccggatccgttacgaagtacggcgacaagaagcccttgtcaaaggagatgccctcggtcagctccacgtaggactcgatggactgggattcctcgacggtgagcacaccgtccttgcccaccttgtccatcgcgccggcgaccatctcgccgatttccgggtcgcgggaggacacggtggccacgttcgcgatctcgttggacgaggacacttcggtagcgcgcgctttgagctcctcgaccgtcttttctgccgctgcggcgatgccgcggttcagctcgatcgggttcgcgcccgccgcaacgttgcgcagcccctcggccaccatcgcctgcgcgagcagggttgcggtggtggtgccgtcgccggcaatgtcgttggtcttcacggcgacagacttcaccagctgcgcaccgagattctcgaacgggtcctcgaggtcgatgtcgcgggcgatggtcacgccgtcgttggtgacggtcgggccgccccagctcttggacagcacgacgttgcggccgcgcgggccaagcgtgaccttcaccgcgtcggcgagcgtgtcgacgccgcgctggataccctcgcgggcctcctggtcgaatgcgatcagttttgccatgagtggcgtctcgcccccttgttacttctcgatgacagcgagcaggtcgcgggcggagagcagcaggtattcctcgccgttgtacttcagctcggtgccgccgtacttggcgaagatgacggtgtcaccctccttgacatccatcgcaacgcgtgcgccgttgtcgtccagacgacccgggcccacagcgatgaccacagcctcctgcggcttctcagcggcggagtccgggataaccaggccggaagcggtggtggtctcagcctcggcgatctgcacgagcaccttgtcgtcgagcgggcggatgttgacgtttgccatgatcagtagctgacctttcgtcttgtcaatgtgagcgtttggaatgttcttgcggtaaatcccatgtcgcgcagccgtcgtcgcgggtgaacaactgtgctcgagacaacccgtttagcactctacccacgagagtgctaactgacaaccgccgtttccacctcaagcgaggtgtccgtgccagtgcccaacgacgacggggacgccccctccgcgatcagctgcgccgccagcgccgcgatcatgacgccgttgtccgtgcacaggccgaaccgcggcacgcgcagctcgatgccccgctcggcgcaacgcttcgccgccagctccctcagccgcgagttcgccgccacaccgccgccgagcagcagcgtcgccgcgccggtatcttcgcaggccagcacagctttcatcgtcagcacgtcgcacacagcctcctggaacgaagcgcacacgtccggcacggaaatttcggcgccctcacgctcggccgcctcaacgtagcgcgcgaccgcggtcttgacgccggagaaggagaagttgtagcggtgctcgccgcgcatgtcctcggcgcgggtcaaggcgcgggggaacgtcacggttggctgcccgagggcagcttgcttatcgacgaccggtcctcctgggtaccccaaccccagaagcctcgcgactttgtcgtaggcctctcccgctgcgtcgtcaagtgtggagcccaactcgcgcatcggtttgccgaccgcctcaacctcaagcagctgcgtgtgcccgccggaaaccaaaagcgccaccgcgtgctcgagctctgcctcgccctccaagttcgccaccgcgacgtggccgccgaggtggttgacaccgtagaacggtacaccccacgccgccgcgtacgccttcgcggcgctggcgccgaccagcagcgcgccggcgagtccgggtccaaccgtcgccgccaccgcgtccggcttttcgatcccggcctgctcaagcgccgccgccatcacctgcggcatcgcctcgaggtgggcacgggaggcaatttcgggcacgacgccgccgtagcgcgcgtgctgctccatggacgaggcgacctggtcggcgaggatctccacctcaccgccgccgccaaggcgcacgatacccacccctgtctcgtcgcaggaggattcaatacccagaatgatcattcagttctaccccttcggctgtgacgctcgcgctgcatggagtacgcatctgcgccggacggctgatagtagcccttgcgcgtgccgaccacgaaaaacccgtagctttcgtagagccggatagccggcgcgttgtcggtgcgcacctccaaaaacaccggcccgtccaaaaggtccgcagtgtgcatcagctggtccatgagcgctctgccgatgccgcggccctggaaattacgcgcaacgccgatggtgtgcacctcgaactccgggtcggttttcggtcccagcattgccagtcccgcgtagccgacgaggtgcttgtcgtcgaaagcgccgacgtagaaggtgtgcggcgcggcaatctcgtgcgcgatcgcctcctgcgaccaagggccttcgccggcaaaaagttgggattcgattgcggcggccgacggtgcgtcggcaagcaccagctccctgaacatcatttcggcggagtggcgtccgggcggcgcaagtagagcggcactagcggggcgggcgccgcgtcgaagtctgccgccttgaccaggccctcagcgcgcggcgcgacgtaggtgacctcaccagcttgcaccgtgagtttgtctcgcagcggctcaggcacgctgagcacgtcgaccttgtgaacgggcaccgcgcccggcgcgcacacgtccgggccggcgacgcgctccccgccgacgtagtgagcccagtacacttcgcggcggcgcgcgtccgtcaccaccaaggtgttgcctttgccggccagctccgccacagcgtcgtgggtgaccacaccgtgcacggggatcccgagcgcttgcgcaaacgctgatgcggaagccataccgacccgcaacccggtgaacgggcccggcccgcaccccacgacgaccgcgcccagatcgcggtacgccgcgcccgcttcggccatgaggctctccaccgccggcacgagccgttcgttgtgcgcccgtgtggtttccaccgattcggccagcacgcggccggaatctgcgtctgccagaccgacaatgagatcggtcgtggcggtatcaacggccagaacgagcattattggcggatacccagttcccagtggccgtcagcgaagtagaacggcatcccagcctgcagcgggtaggtttccgcgtgcggggtggtgcaaatatcgatctgcttcaggtcgacctggtcgagggcgaccggagcgtcgacgtccggcgggagcagcaccacgtagccgctgtcgccctcgaggtccgggctctccgccagggcgaaggcctcgagcttggcgtcgatgagctcctgcggctcgttcgggcagaggaaggtgtaacccgcgtactcgttcgcgtcgtacaccagttccgggctgaccagctgcgccacgacagcgccgccgcttggctgcacgtcacgcagtgtggtggacagcgagtttgtcggcgcgacgacggtctggccgggagcggctgcggggcgcgacagcgggatcgcgatgagaccgacgagggcgacaatccacgccacggcagcgaggatgacccaggtgcgctgggtgttggagagtttcagcatggtgccaagcctacaacccgccgccacgtgcggcgcaccaggtaataatgcgcccctccgaactcgggtcctcgcgcaccattgattcccggtcgatagtgaccagcagatattccgccgcgatctgctccaccagccccccgccccattcagcgaccaccactgctgattcgagttcggtgtccaggtcaagcgcgtcgagctctcccaggggatcgccggacgacccctcgcccagcagccggtacgcgtccacatggatgagcgctgggccgccgtcgagggagcggtgctcccgcgcaatcacgaacgtcgggctagtcaccctgcccttgacccccatgccgtctgcgatgccttgggtaagcgtcgtcttgcccgcgccgagagggccgtcgaggatcaccacgtcgccagcctcaagcgcggcgcccagctcgcggccgagctctctggtttccgccgcctgctcgcacacgcgcctgccttgttcaggaaacgccgttttcatcgctactcctgtactgccgctgggtgcgccccttcggcgcacagacgatttcgtagttgatggtgccgactcgctcagccagctcggtggcggacatgccgccttcgccgaagagcactgcctcgtcgccgctgtgcacacccgcctcgttctgcccgagccagatcaccagctgatccatgcacacgcgtccgacgaccgggtagcgcaccccaccgaccgcgacctccaggtgcggctgccacgcgcggcttaccccgtcggcgtagccggcagcgacgaccgcggtgtagccgtcttcgggcgcgcgccacgtcaacccgtagctgaccggatcgtcagcgctgaccggcttgacggcgaggatgctcgccacccacgacatggcctcgcgcagcccgtggtcgtcgccggggaccggttctagcccgtaaaggctcaagccgggtcggacctgctgaaagtggaggtcggggcgcgtccacaccgccgccgagttagcgaggtggttgcaaaccgggttcagccccgcggcgacggcgcgctcaagggcgcgggtgaagcgctcgcattggagggaggtgtagggctccgcgggcgcgtccgcgaaggcgaggtggctcatgagtcccttcaccgcaatgcggccgtcgcgctctgcggcggcggcgagggcgaagacgacgtcccactgcgactcgtcgaacccggagcggtgcatgccggtgtccactttgaggtaggtggtgggggtaaacggggcgtcgataagcatctgcaaatgctctctcgtcggggcgaccagctcgatgtcctcgggcaactcctggcccgggtcccacagccaagaaatgaccggcagatccgtcactgcccgcactgcgcgcgcctcagcgagggtggtcaccccgaacgcgtccgccccgttcgctgccatcaccggcaccgcgcgttcgacgccgtggttgtacgcatctgctttgaccacgcacacgagccgagcctgccccacctgccgcttcaacacacgggtgttgtgggcgatagcatccaaatcgatgcgggcggtcaaactcatgggcctacgttacagcaggtgcaccgcgcccagcacgatcagcaaggccgacaccgcccacgtcgccgccagcgaaaccgtcgacgggtgccgccgggcccactcgagcgtgcggcccgcagcggaatcaggcaccgctctcacccacgccaccagcagagcgcacagcgttggcagcgacagcgcgatcgtggcgtacagcggaatggttccgtagcgggtggcggcatcgaccccggcggtggacagcagagcgaggccgccgtaaaacggcaccgaggtcgccgactggatcacgccgagggcaaaacccgtaaagactgtggtcgcggagggggttttgagcggagccatgattttgttcacgagcgcgctgttgtcgccgccgcacagcgcgagaagggccgtggcgacgcccgtggctatcagcacgatgccgaacacaggcccgtccacgaaccgttggaccgccggaccgaggccgtcgaacaccgcgagcatcacaagcgcgagtccagcgacgccgagccagtctccggcaaccagcagcgcagtgatcgcgccgtagccgcctttgccccggggggcgacgatgccgacggcaacgatcaccgcaatgagcagcaggttgatcgagtcaatgaacgcaagtgagagtgccccaagcaccccagccaccctagcgcaaacaaacccgtggccacacaccgaatcaagtagagttggctgtgtgtctgcgaatttgaagcaactttctgacttgtcgaagcgcggcccctaccgtgtgctcgagggcgacctcggttacaccggtctgccgggcaaggtgtacgcgccggccgagggcaaagaccttcctggcgtggcgttcggccacgactggcgccggggcatcggcgcctacaccgagacgctccgccacttggccagctggggcatcgttgttgccgcgccggacaccgagaccggattgaacccggaccaccgcggcttcgcggctgatctcgagacggcgctgcaggtgcttggcgccgtgcggatgggcaacggcaacatcaccgtctcccccggcaagctcggtgtggccggccacggcatgggcggtggggccgcggtgctgaccgccgtcgacaacgccaaggtgaaggcggttgccccgctcttccccgcgaacgtggctccctccgcggttgaggcggcgcgcaacatctttatccccggcatgatcgtgggctcgggcgaagattccaactccctgttcaactcgggaaacccggcgaagctggcctacaactgggccggggacgtgtcctaccgcgccgtgaagaagggggcgcagcaggatttctctgaggacggcatcgggtggcgcgtgcttggcatcggcgcttccaaccgcggtgtgcaggccaccacacgtggcctgctcaccggcttcctgctgcaccagctcgccggcgaaaagaagtacgccgcgttctctgatccggaggcctccggcaagaacatcgactccctgacgggcgatgccctcgcagaggcagccggcctcacccgcgacgacgcgaagttttcccttttctagcgcgccgccttagcggggcgtttcccacggtggactccccggcccctcgcgccgcagcacggactgcacttgaccctgggccgcctggttgcggtcgcggcggcgcggcatgccgtactcacctcgcgggataggcatcggaggccgctgcgggtgcagctcgcgtgaaaccgcgtactgctgggctgtcacctccatcttcttctgcgtgtcgcgcaggatcgcctcgaaatcctccagccgcttcgcggtgcgccgctggtagcgctcggcgaactccataaaatccattaccaatcccccagtttcttactcccccaggccgcgcttggttccggcgcggcaggctgcggtccgctcggaccattggatgtggagctcggtgtcgcaattgagcttcccccggtgccgctgctctgcgctgcgggcaccgtatgcatcatggcagatttttccttgggcggcacgggctcaggaactttatctagctcaggagggggtgcggcgacattgtcgcactccttttcctcaggagtgggtgcgggtgcgggtgaaggcacggggtcgccaccaccggtcgatgtgcagcactcgcaggcgcagtgcgcttgggcggcctcatagagcgagtacgcgaggaatccgaccccgccgagcaccgcaaccgcgcccaggcggccgagtggcgtgccaatcagccgggcggggtcggattcgcccgcagctgacggcagagtcatggtttcggcaacggtgcaggtgaccgtttccagcccagcgttctgctcgccgggcacctcgtagtcgaactcgaccttcggctgcttcggctgctgcggctgagccgaatcggaggctgcggtcgcgggcgagctctcagctgtgcggcaacgccgcgctgtcggtgttgcgccgggctgctgccgcgcggcgggaggacggtcaccagccctcaccccgtccaacactggcgatgcagaaccagccgcggaaggtgcggccggggctggagctggtgccgcagcggttggcggcgcagacgccggagtggtgggcactgcaccggccgaggcagtcgaggaggaagcggtggcaccgaccggcttcacgtcttccggcgtgtggcttaccgccgttgtttctgcagctgccgtccccggcgcggctggattgccagctggagcggtacccaccccgcctggtttacgtttgggagcatcgtctgcgcaggcgcaatcgcattcgtaattgacgggtgccgccggctgctcgtcggctgcgtcatcaatgttgtcggcgatctcttcgaggcactgctcgaccgcatcgttgtggtcggaaaccgccgcgcgggcggcgtgcaacgccttgatgaccaactctgcggccatggagccgagctttggaaacgggaacgctcccacaagttgcaggaggcgtttggcggtgtcgaggaagagttcaacggccttcgccgccgctgcgcggattgtttcaatgcacgcgcagcattggtcgatgcggtccgccacgcgcttgcgcttctggaagtgccgctcttccttcttcgcgtcgaggcgttcgcgcaagctgataccttcacggtcgaaccacgacctagatgactcagcctgcggcaagtaccccggccgggcgttcacagcgcggcgcgcgccgttgattccccgcgctactgcgcggaaagcgtccaagttcaacccagtcgagcgggccagcagcgtgcggatgtcgccggcgagagatcgagcctgcgaacgctgcgccggggtaactcccggtgtggcgtccatcaacgataacgtcgcgtgcacctgagcgttgatcgtgagcgtccacgggtcttgggatgcgctgttgattgtggtggtgaccatctaccagttcaccccgttcaacgatgccgaggcagcgtcgtcgtgatcggtcacatcgtcgaccagggacaggatgctctcccagttcgccgaccgggtcgaaaggtacgcaagcgaggtgtcgtgcaatctgtctagcgccccgacgatgcgggtgccttgggcgctgaaccccgccccgaaatcggtggttgccacctctacacgctcgtgttgcagccggctaacctcgtcctcgtacgacgctatggccgcgccgtagagcgtgcgcagctcatctgtgtcgagctgcgggccttgttgtgcttccaaagccttcccccttcttaaaacccggccgcgtacgcagccgggtgcgaaacagttgccacgtattcagactccgcttttgcggtgccggttccatggcgggggaaaatcttggcggaggcgctgactctaactggctacaccgcagcgacaaccgcagcgaggcggcctgcaaccttgcgcgcctgctcctcgttcgccgcttcgaccatgacgcggaacagcggctcggtgccggagggccgcagcagcacacggccggattccccgagctcggtctcggcgtcgctgatcgcgctctgcacctcggcagcgtccatgatcttcgacttgtcggacaccgggacgttgatcagcacctgcggcagcacctgcatgactgtcgccagctctttgagcgaagcgccggtctccttcatccgcgccatcagcgacagaccggtcagcgttccgtcgccggtggtggcgtgcgccgggatgacgacgtggcccgactgctcgccgcccagcgagtagtcgccgcggccgagctcctcgagcacgtaccggtctcctactgcggtctccttgagctcgatgcctcgctcgcgcatcgcaatcttcagccccaggttgctcatcacggtcgctaccagggtgttgtcgtacagcgcgttgcgctcctgcatgccggtggccagaatcgccatgatctggtcgccgtcgacgatgttgccctcggcatcgacggccaaacagcggtccgcgtcgccgtcgtgcgccagcccgatgtccgcgccgtgctctaccaccgccgcctggatctgttccatgtgggtggaacccgagccgtcgttgatgttgaacgcgttgggtttgtcgaagatggtgacgacctctgcgccggcggccgcgtacgcctttggcgcgacctcgaacgccgcaccgttagcgcagtccacgacgactttgatcccgttcagatccgccggcacagcctccttcaggtgtgcgaggtagcgctcttgggcgtcgggcgcctcctcgataatgcggccgataccggtgccggtcggaccagtgtcgtccagctgggcgatagctgtctcgatctcgtcttcgatctcgtcgggaagcttcttgcctccggcggagaagaacttgatgccgttgtccggcatcgggttgtgcgacgcggagatcatcacgccgatgtcggcgccgtaatcgtccgtgaggaacgcaagcccgggcgttggtatgacgccgacacgcaagacatcgacgcccttcgacgccatgccagcagccatcgcagcagccagcatctcgccggagacgcgcggatctcggccgatcagcgcggtcggccggcggctgccggagggccggtccttggtcagcacggttgccgcagcggcaccgagcttcatggctaggggcgcggtcaaggcctcgttggccaagccgcgaacgccgtcagttccaaaaagtcgagtcataaattccattatgcacccgccggaaacggccgctttacccgccggtggattatttgaaaacaaaaatgccgccacttcaaccggagtggcggcattcgttgcgcgtgcggccgcagcgcagaacgcaagcggtttaacgcttggagtactgcggtgcgcgacgtgccttgtgcagaccagccttcttgcgctccactgcacgggcgtcacgggtgagcaggccagccttcttcagggtcgggcgctcagccgggttgtagacgttgagtgcgcgggcgatggcgaggcgcagtgcaccggcctggccggtcgggccgccaccggagatgttggccttgatgttgaactggccctcgcgctcgagcagggtcagcggctgcaggatgtcctgctggtgcagcttgttcgggaagtagtcctcgaacgcgcggccgttgacggtgatgacaccctcgccctcggtgacggtcacgcgggcgatagcgcgcttgcggcggccgacggtctggatcgggccctcgtgcagctgcaccggctcaaccgcgtcgccttcagcctcgtcgacctcgggagcgatcgcgtcaccgatggtgtagttgaactcctcggtcgcggccgtcgcggcatcgatgtcgatgtcctcagcggtgtaggcgtcctctgcgtagttgttcggctcggtcattactgtgccacctgcttaaactcgtaggtttccggcttctgggcggcgtacgggtgctcgtcgccgacgaagacgtgaagcttcttgatggactcgcgggaaagcttgttgtgcggcatcatgcccttcacagcttcctcgatcacgcgatccggacgctcgtccagcgcgcggcccagggtcatggacttcagaccacccgggtaaccggagtggcggtagcgcatctcacgctcgcgcttgttggaggagatgtggaccttgtcggcgttgatcacgatgacgtggtcgccggtgtcgacgttcggtgcgaactgcggcttgtgcttaccgcgcaggatgtctgcgacggtggaagcaagcttgcccagcaccacgtcggttgcgtcgacgacataccacttacgggtgatgtcaccgctcttcgggtggtaagtagacatgcatgactcctttaaagtctgtctagatggctgccggccagaatcggtgcgcagtctgtcccgccggcggccggtggagacccggcggaagacatgcgaaacgcacaggtgttacaccctacggcaggctcacacaggaaacaaaacccgcccgcgccgctctgtttcaagcggcgcgggcgggcatcgcgctgttactcccccatttgctgttcggcgcgccggggcttacccccagctgttcgcggccgcggtgttgacggccatcatctggttgttgccctcgtccacagtggcggcgatctggttcaggatgcggttgaggtcttccgccgcctggtcccactttgcctggtgggcgcgatagctcgccgcggcctcgccctcccaggtgtcggtcatcggcttgatcatgtctttgaggtcgagcaactggccgttgatgcgggttgcggaggagcggatgtcttgggcggtgttagaaatctgggcgaagttgtacttgatctgcatgggttcttccttgaaagtgtgtcgtcgtgggcggcgtcggcgctacagcgcgagacccggggtagcggccaagcggtcgatgttttcggtggtggtcacatcggtgttctcgtagtgcttcgcgttgtcccggatgttgccggaaatgtcggacagcgcctccgttaaccggcgctgggcgtcgtcgtagcggaccattagctggtcaaagctctgctgggcgcggccctcccaggagctgcgcacggattgtgcaacttcctggatgcggtcgatttcgcggttgacgtcggcgttgactgcgtccgcgcggtccgcggtcgagcgcatcacgtcggcttcggtcttgaattggctcatggtgtttccccctcgaggtgtcaggtaagaacagccgatagcggtgaactgttcacatagttggactcacaaaacacgcttccggttccatcggttctcaagaaattttcggctccggggaaaactccgccgactccatcgccatccggcaagtggccgactgcacctttgtcggcgcagtgcgcgtgtggcaggcgataaagatctggtggttgccctccggccaggtcttccagagcacctcggagccgtcgccgggcatttcgcggtaggtcagcacctgcccgtcggcgcgcaccaactcggtttcatcgtccgcgtcaatttctgcgagcacctgatccgccatcgcctgggcgggcaggttgtagagctcctccacagctatgtgcagccgaaaatcggggtcaagcccggtcgcgcgccagttcccgccgacgtcgccggcagtgaacccgtgcggcagctccacgcgcaccccggcttcctccaagaacacggtttccggttcagggggcagttgcttatcgacgcccccttcatcccccttctccacaacctcagtcgcagtctcctccggttcctcgatctccatgggtccctcgggctccgcggcagccatgaaccagcgagccaggatcaccgtcgcgctcgcgaccagcgccaccacgaccgctaccgcagcagcaaccaccaccgtcgagcgctgcggctcctcccactcctcgacgccctcttcttcgtccgccggcaccttcgggtcgtcgtcggggacttccggcagctccgcggtagtgagcgcgatgtcgtactcccccagcgccgcttcaatgcgctcgaggcggcttcgagacgcgctgacgtgcacgtgcgcaccctcgggatgcggcccgaagacgttccgcacaaacaccgcgatctcgtgctccgagggcgcgtcgaagcggtggaggttcgcggctcccgtgaacacggtcgaggtatccgtcaccgtgatccggagctggggtggtgcctcggcgctcacaggcttccgccttcctcgtacggcgcggcgacttggactgcgccgacagtttcgccgcgctgcaccagggttgcgcgccccggcgccaggggtttgggcctaaccccgaagacgctgccttcgtcccggttgccgtccattaccaaaacgtctgggtagatgtcggtcagcgcgcccaagaacccgccgtagagtgcccttgatatgccgctgagcttccgggcgcagacgatgtggagaccaatgtcgcgggcgtgcgggacgagctcggcgacgtcgcggagcacagcgtcgttgaccaggtccatgtcgtcgatgacgaggtagatttcggggccctgccaccagctgcgctgggccagttcctgcggggagatgccggcgccgggaaggcgcgcgctgagtgtgtgaacgagcgccttcaccgcatcttcgatggatgtcggcgacgcgccgtaggctgcgaccatcgtgtcgtccgcgcgcccgaggtgggcgcggcgcgggtcgaggatgaccatgcgcgcggcctcgcgcggcatggcctggatagcggtgaccgcggcggcgatgaaggtggacttgccgcagccgcttgcgccggtggcgacgacgtggccggaggtgctccacagcggctcaaggcggggtccgccgacgcctaacgggattgagggggtggtggcggcgtcgataagcaactgcactggtgcgtgcgccggcaggaccttcagcgctggcacccgcacctgccccgcggtgacctgcgaaatgtgggcgaaatcctcggcgaccgtgcgcgcgaccagcatgactttgccttccggtgtgagcccgatgcccggcctggcgggcaacgtggtttgcgcttggcggtcgatcatcgaatccatcgcttcggtgagtttaagctcccaccgcgtggcgatcagatcgcggacgttgctgcgcaccgcggaccagcgctgcgtggtgatcaccagatgcacgccggccgcaggaccttcggacgcgattcgggtgagcgggtcgcgcaagtcttccagtttggagtcagctgcgagcagcgcgtgccagccgtcgatgagcagtagcgtgtggcgcgcgtgaccgggatcggggttgtccagcacggcggtgatttcatccaccacgcgccgcaccttctcctcgtcgccccttgccgcggtgccggccacgtgcggcagaacctcgatctggtcgagcccaccggcgccagcgtcgatggcgtagatcgcgacctggtcggtggtgtgcgtgagcgccacggaggcggcgagcgtgaggagcaactccgacttgccggtctgcggcgcgccggcgatcgcggcgtggccgccggaagctgcgagatcgagcagcagcatgtcttggcgctggtggtagggctcatctaccaaccccattggcacgcgcaggaacccgaagtccccgtcgccggggcgcacactagacagcgccagctgctcgggcaggggcggcagccacacctggtgcgcgcgcattccggcgaacgcggcgagcgcccgggtgcgctccaccacggcgtccaccaccgtggtggaggtgtcggtctcaataacctcggtcaccgcccgcgcggcgtcgagggcttcctcagcctcatcccaaccggtgaactcgtgcacgaacaccgggttcgcgccggcgcgcccggccaccttgcgccgcaccggacccgagacgtagaccgcgcggaacctggtgagcccgtcggcgcccgccttgaggtagccggagccgggctcgcccggcagctcgtaggcgtccggcacaccgagcacctggcgcgattccgccgccgaaaaggtcttgaggccgatgcggtatgacaagtgcgaatccaggccgcggagtttgccctcctccagccgctgcgacgcgagcagcaggtggacacccagcgaccggcccagccggccgatcgccacgaaaaggtcggcgaagtgcgggtgctgcgtgagaagctcagaaaactcgtcgaccaccacgaacagcgcgggcagcgggtcgagcggcgcgccggcaaggcgggcgtgggtgtagtcggtgatgttggcgaagttgcccgccttgcgcagcagctcctgcctgcggtgcatctcccccgacaacgcgtcgtacatccgctccaccagcaccgcttcgtcctccaggttcgtgatcaccgccgacgtgtgcggcagcccctcgcagccgaggaaggttgcgccgcctttgaagtcgacgaggacaaggttcagctcgtccggcgagtgggtggcggccagggcgacgaccagcgagcgaagcaattccgacttacccgagcccgtcgcgccgatgcagaggccgtgcgggccggaaccgccgtgagcggcctccttcaaatcgatgaacaccgcttggccgtccggtgtcgtgccgatcggcacggtgagccgttggcgcgtgccctcgcggcccggccacatcgccgccacgtcagccgcgtcgacgcgggcgtggccgccggttgcctccaggcggtccaggccgagcatggcaagcacgtcggcgccggcctcaccgcttgcggcgtcggggcggcggtagaaggcgagccgccgggccacgaggagggcctcggcgccggtgaaggcgtcgacgtcgccgagtaattccggaccgcgcgcggtcaacacagtcaccgagtcgtcgcagacgaggtgaagcgcgtcctcgtcgacgaagaagtcggggtcggggtgcaccgtgatagtgcagtcggcggtggcgagtggggggttgaaggtggcgtcgacaagcatcaagctccactgcgcctcctgcggcgtccgtgcgtgcggcagccactttgtccaattgaagcccgaggatgcggcgtcgatgccgacgagctccgggccgtggaaaaacgccagttggcaaacgatggaacgcgccacgtcgtgggcccgcgggccggccaaggtgacagagcggaacgcagcgagctggaccacgatcggcatgccgtgcaccgcgctgaccgcggcgacggtgcggcgcagactgaccgcgcacaccgggtcgaggtcctccgtcgagccggggtcatccacctcgaccggcgtgtgcaaggcggtggctcccgtgccgacgcgcacctgcagcgcctgcgccgactgcgcaccgcgctcccacacccgctgagtggagactgccatcgctagctcggccggcttcgggtgcaggtagttgaaatgcgcccgctgcatgtccgcgcctgcgcgggcgcgtttcgccaacgcgtcgaggtgccgcaggtagacccggcgggtctcgtcgatgtcgctcttgccctcgcccgggttgaacaggccaatcagcccgatcagcatcatgagcgggaagatcagcatcatcgggctcatctggcggccagaggccaccatcagcgccatcaccgcgccgaccgcggcgaccatgatgacgggaatgagcaccctgatcagcgcgatgggctgatctttctgcactcccggcaccgcttcggcgcgaagcgagccggttggcagcggcggcgcgccgtcttccggcgcgacgtgaatcggagcgatgaccgggttgtggtcgaggccgagcatgcgtgaagttccccctgtactcccgcggacgccggttccccctcttttggatccggacccccaatccgcgatgcaggcaaagtatagggctgtcttcaagctcctgcaggacgcggctgattcgcccaccggtggacgggcttaggctcctacggcatacttgagcccgtccacgcgcgggcaaacgggggttccgcgcttttcacatgggggaaatcatggttgcctcgtcaacccatcacgttgtccgtgtcaccgttcgcatcagcgcggctgacgtccaccgcgacatcgacgtcacgctgccgacatcgtccgcgctcgccgaagtgttgcccgaactcgcgcgcatcatcgacattccgcacatcccgcgcccgtggcaggcggccaccgccgcaggggcgccgctggacatgtacgctccgctgcacaagcttcggcttgtcgacggctccatcatctcgctgacccccgccgagccgccctcgccgccggtggtccgcgacgccacagaatcactcaccgccgccgctgccgccgcgcacgacgcccgcggcctcgacaccgcggcgggcatcgcgggctgcgccggcatcgcgctcgtcctcatcccgcacgcaggtctcgccgccgcgctcgcggccgcggcgttggcgctggcgctgcttgcacggctgcgcagctcgcagccgctcttcttccccgttccgccgttgtgcgcggcggctgccggcgcgtgggtcgcagggccgcgcgccgagtgggtatccggcaccgaccccgccgttggcgcggccgcggccgccatcacctgcgccgccgcagccgccgctgggtccgcggcgcgtctttcgggccccgccgcaaccacgttccacctcgcgaccagcaccattgccgccatcggcgcgctgggcgcgtggttgcccgcctccctcgccccggcggccatgacagtgctagccagcgtcaccgctgtgacggcaactccaggcttggccagccgcgccgcggggttgaagatcccccggatccccaccgctggcgaggagctgacgcattccgacggttaccagctcgacgtggacgcgcgcagcgcgagcgcagtggcggtcgccgacgcactctccgccgcggcggccgcgtgtgcggctccggctcttgcgtgggcctctcttaccggcggcacctggccgatcgcgctgtgcctggctaccgccggcgcccttgggctgcacgccctgcgccaccactacccggtttcgcgcgccgcgctgactatcgcggcgctcgcggcgctggccggggtggtcgttgccaccgccggcgggggcaccgctgaaacggtgctcgccgctgccgtggccgccgccgttgctaccgcgcccctgtgggcaccccacctgcccgagctggagccaaccacggtggcctggtttgaacgcgccgaagccgccgccatcatcgcgctcatcccggttgccgtgcagatgaccgggctgttcgcgctcatccgggggctgtaatgaaacgcaccatcgccaccgccctcgccctggcggcaacagcgaccgcgttcatccccgccgcccgcgcccaggactacgcctgcgccgcacctgcgcacgcgccgtttgccggcgccccagatcttcaaccgctgcgccagttcgccaccggcgccggtgtcgccgtggccgtcatcgacaccggggtagcaccttcacccgaactgccgcacctgcgcgccgggcaagattttgtggatcccgcttcccccgacccgcttttcgattgcgacagccacggcaccgttgtcgcaggcatcatcgcagggcaaacaatcggggtggcgcccggcgcgtccgtgatctcgatccggcagacctctgcccactaccgcagccgcgacgagaccgagttcgccggttcacttgccacgctcgccgcagcaatccacaacgcgcttgaccagggtgcgcgggtgatcaacatctccgtcgtctcgtgtcttccgccggaggtcgcgccgcgcgtggacctcgccgtggtcgaggaggcgctcgccagggcagaaacacagggcgcggtggtcatcgccgcagccggtaacgcctccgacacctgtggccaagggttcaccgtggtgccggcccacttccccaccgtcatcgcggtcggcgcccgcgccgacgcgcacacggtggcaagctactccatcagcgcgcccggccctgaagtttctgccgacggggcggtaccactagccctcgcctccgacggcagcggctgggcggcgggcacccgcggtgcgcgcggtgaagtcgccccgtacgtgggaaccagctttgcggccccgcgcgtcgccggcgcggtggcgctactgcttgagcgctacccccgtttaagtccctcccaggtcagggagctggtctatgccgcggctgaaccccgaggcggggcgctcgacgcgggcaggctaattagccacctcccgccggacgacgtccccgcgtcggacccgatcgtgatcttgccggcggcaggcgcggcctcgagcgctccggggaaatggtgggtggcgctgccgctggccgcgctggttgccgcggcctcgttagtacgccgccgttagcgccgactgccggttcagcggctcaccttccggaagcaacgagacgatgctccacgccgcctcatcgacgcgctgcacgccgatgatctctaacgtcttctcgtcgggcactgggtggcgcagcccgcttgtcgcgaccacgtggtagccgaaaccggaatcgatgcccacggctcctgcggcgagcccggcgaagtgggtggccaccgacgacccggacagttcgaccgccccgtccacagccccaccgtccggcgcgtcctcagccagcgccgctgcgccgccctcgggtccggcgcagattgcgcgcgccgctgggtcgagccactcgggtacccgcgcgggcaggcgtaagacgattggcggatcgagatcggggtagttggcgattgccgggggatcaacctccgtgacctgggctgaagcactggtgagcaggtgcgcttgggtgggtgtgatgggttgcacgtgggcgtcaataagcaaccatgctccctcggctgttgtgagcaccgctggtgcggggtgaggcagcgcgtagggcggcagctcgcggactgcgacgaagacctgggtgggcggtgtccagcggggtgtggcggcgtcgatacccagcccgcgccgcagaatccgcccctctggtgtggtcggcggcggcagcagcgcgcggccctgagcggtgaccacccactcgcggttgtcggcggctgcgaggacagcctcgttctcgcccagcggcggcggggcctcgcccgcaatcacgctgacggtgtcgcctgaagtgcacaccgaccaatcctcgtggtcggagtcggccggcgcgaagacgttgggtgccgtggcgatcccgacggggacgccgcggcccatcgccagcagcgcctcgtcgcctactcgggcaggctccgctggcgcaccagcgaccagccgcgccgaggtcaggttggtgactgggtgcgcggtgtcgtcgacgcgcacgtacagtgccccgtcggctccgcgcagaatcggcgcgccgcccggatccgggttcggggccatccacgcgaacagccccatcaccccggagatcagaagcgccgcgacggtgccgaagatcatggcgcggcgccgcgaggcgagcggatcgtggatcatccggacgtcgccgaagatgagcccgtgctcgacccggcggcgcataaacttgtgtccggaaacttgagtttttgttgttggcagcacgcgcgccatgtgtccccctcccccgagaatcgggttcgaggataccgcgcgggagcggcgcgcgcagggtaccgccgctgccgcgggcgttctgtctacccgctggcagcagtagttcccgccgcctcgagctcgaacagctcatccgagccgttcgcgagggcgtctttgcgcatgtcggcgagctcggcgctggtgaacgcctcgttgacagcgaagatcgccaccgtacccttgcggtagacgggcgtcatccccttcgacgcccataggcctaggttggcttccttgttcgtgcgctgcccgtcccagaaggactgggggctgaccatgtaaaagcgaatgttcattttctccacggcctcgtcggccggattgtcggccgaggcgcgcccgcgcagcccttctccgatgaaatcggggtgccagaacgtggtgtcgaaggcagcgccgcgtcccgcgttgggccagaggtagtggcgcgatgcggtgggcacgccgctgaacgcgtagagccaggagtgcccgtcagacgggtcgccgatggtgaggccctcgtaagcttccgggcggctggcgagccacgtgaatgcggcaatgtcgtcttggctaaccatgcgcccgtcgttgcggggggcggtgaagatgtgctcgttggcgccatcaagcgatgcccgagcggagggaaccgcaaccgcggtaagtcctgccgcaactaccaccgatgctgcggcggtcacccgcaccccggtcgggttttcacggcgcgcggcgagcggggcgagggtgaccagcctcaccatggcggcgagcgcgaccgctgccgaggcgaccaggcacatcaccacggggatgatgaggcggtgcggcgtgttgtagtgcagactgctgatctgccacaaggcgtcgcctacccagccgtcgagcggtgcggtcgagttcacggtggtcaaaaggcacaccgcgtaaaacaggctcggccagatctggccgcgccaaacgagcatcactactgccccgatgagtccgagccagagcagcggcatcgggtcgaagtccgggaaaaactcctccacgtggcgcgtcagcagaaagaaggaggattcccacgcgtcggtgtcgttgagcgcctcttgcgccacccacccggagacctcgctcgcctgcttcgagcctgcgagcacctgcggaaggtacacgacggaggcgccgacggcaggcagcgcaagccaaagggtgtccgacaaccggctgcgctccgggcggacaagcagtgacgtgagccacgccaaggcgaccgcgaccacgaccacgctcaccgcagacggatgcacgcagagcaagcccaaaaacccgagcgccgcggccaacgctgaaacgtggtcgcgcggcacggtcaggaacagccagatgacgatgccggtcagcgacattgcgaactggtacggccacatgccgacgtattccgcaatccacaacacatgcggcacaccagcaacacccacggcggcaaacgcggcagcgatctgagcggtcaggccccgcgagcgcaaaaacgctagcaccaggcaggccatggtcagcggcagcgcgatccccgacagcacgacctgggcgatgttcagagctgggatcggatccagcccggcggcctcgccaaagagggcggcgccggcgtggtagcccgaagggtagagctgcaccgcctgcgtctcgatgttctgcagctcacccatgcgcgttggcgacgcgacgcccgtatccatgatgaagcgcaccgcgttggcgtgccactgcgaatcccaaccctggaccacgttgtagacgccgttgggcgcgcgttggagccagtgaaggcggtccgctgtgcacaaccacgcgcctgcggcaacgccggcggcgggcagcatccaagccgggtcgagggggcggcgctcacgagtgcgcgctatggcgaagcgccacacagcggccgcgccgagggcgagtgccaggctcaccccgtacgtccacaggttgaacggcgcagaagtcaaaccccacatccacgcgctcatgccgatcacgccaaaggtgaccggcagcgccgcagccgcggcagcgggcgcgcgcatgccggacaccagcgcgatcaggaacccgggcagcaggaagaacgcgatcgcgaaccacagggcggctgtgcttgccatcgttcctcctttctcccggaagcattctagctacaagctgcggcggtcccgcgtcacctccgcgcgggccgcgagatcttcgtctttggggtaggtcacgccagttagtgtgagtccgcacgcgggggcgaggcgaagggtgggctcgcgggcgtcggcaagcaatagccccctcgcccactccgggtcctgcttgccctcccccacagtcaggcacgcggccgtaagcgcgcgcaccatgttccagcagaacgcgtcggcggtgatgtgcgccaagtagagctcgggctcgctctcgcttgacgcgtccccccaccgaaacgcctgcacttcgcggatggtggtggcgtgctcgcgaggtttgcaaaacgccgcgaagttgttgagccccaccatgtagccggcagcttgctgcatgcgctcgatgtccacgggctttccccaaacagccgtgtcgcgggcgcgggtgggcagcgcgcccgctgggtgggtggtgacgcggtaggtgtacgagcgggtcagtgcggcgaaccgcgcatcgaactgcgggggcacttgccgtacgccgaagacacggacatcggttgggagcagttttgctaatcgacgcaccaacctccccgcatccccatcaatcgatcgctggcgcaacgtctcctcggggacgtccgcgtgggccacctgcgccgaggcgtgcacacccgcgtcagtgcgtccggcgaccgtgagcgaaacgggcgcgcggagcaccagcgaaagcgcgtcctcaataactgcctgcacggtgcgcagctcgcccttctggcgtgcccacccgtggaagtcggtgccgtcgtaggcgatatcgaagcgcagccggatcgtgtcagtggggtccatcggtgcaacagcgtagcagcgcagcacacacaaaaaagtgccccaccacaatcgtggcggggcacccggggcgcgatacgcgcttgcagagggggtttcaggaccctacttctgctgctcctgctccggggtctccggctcagcagcctgggcctcgacagcagcctcgtcggcggcctcagcctggacagcctcaacctgctcggtctcgaccgaatctgcggtctcctcgaccggagcggtggtctcctcgacctcaaccggagctgcggcctcctcgcgggcggctgcagcgcgcgcggtgcgggtagccgcgttggacacggtctcctcggtcaccagggagatgtgcaccatcggcgcgttgtcgccggcgcggttctccagcttgatggagcgggtgtaaccgccatcgcggccctcgaacagcggagccaggttgtcgaacaggtgcgcaacgacagccttgttcggcagctcagcagccacagcgcgacggtcagccagcgagccgtgcttcgccttggtgatcagcttctcagcgtaggggcgaagcatcttcgccttcgcctcggtggtcttgatagcgccgtgctcgaagagggattgcgccaagttctgcaggatgtgctcctggtgcttggcggaccctccgagacgggcacccttcttaggggtaggcatgaataactcctcgtgtgcgtgaaatgagcgctagctcaaagatgaatgttctactcggcgtcgtccgcggcggtgtcgacgtagtcaccggtctccgcgtcgtacccctcgatctgggtgggatcgaaatcttccggagcgtccttcaaagtcaggccgaggttcgcgagcttgatcttcacctcgttgatggacttctggccgaagttgcggatgtccagcagatcgctctcggtgtactcggcgagctcaccgacagtggagatctcctggcgcttcaggcagttgtaggagcgcacggagaagttcaggtcttcgatcggcaggttgtaggccgcgatgtactccgtctcctgcggggatgggccgatctcgatgccttctgccatcgtgttcagctcgcgggccagcccgaacagctccacaagggtggaaccggcggaagccagcgcgtcgcgggcggacatggagttcttggtctccacgtcgatgatcagcttgtcaaagtcggtgcgctgctcgacacgggtcgcctcaactttgtaagcgacgcgggtcaccggcgagtagatctggtcgaccgggatgcggccggcctcgccgccggagttcggcatagccgggacgtagccgcggccgcgctcgacaacaagctccatctccaggcgggcctgctcgttcagagacgcgatgtgcagatccgggttgtggatctccacgccggccggcggctcgatggagcctgccgtaacctcgcccggcccctcgacgttaaggtacatgaccaccggctcgtcggagtcggaggacagcaccatgtctttgacgttgaggacgatctcggacacgttctccttgaccccgttaatcgtggtgaactcgtggaggacaccgtcgatcttgatcgacgtcacggccgcgcccggaatggacgacagcagcgtgcggcgcagggagttgcccaaggtgtaaccgaaaccgggctcgagcggctcaatgatgaacttcgagcggttggtgtcgatgtactcctcggtcagttgcgggcgctgagagatgagcatgaacttctccttaatcggcaaccactatttgatgccggtaggaacggatgtggggtagaaaaatgcttacttcgagtagagctcgacgatgagctgctcctgcagcggcacgtcgatctgagcgcgctcgggcagctggtgcacgaggatgcgcagggtgtccggaacgacctgcagccaggccggaaccacggaatcgagcaggttgtcctgggcctcctcgaaccacagcatcgaacgcgacttgtcgcgcacatcgatgatgtcgtactgggtgaccttgaaggacggaacgtcgacagccttgccgttcacggtgaagtgaccgtgggagacaagctggcgagcctggcggcgggtgcgagccaggcctgcgcggtagacaacgttgtccaagcgggactcaagcagaaccagaaggttgtcgccggtcttgcccgggaggcggttggcctcctcatagtagcggcggaactgcttctccatcacgccgtaggtgaagcgggccttctgcttctcctgcagctggagcaggtactcagattccttgatgcgggcgcggccagcctgccccggagggtaggggcggcgctcgaaggacatgtcgccgccgacgaggtcgacgcggaggcgacgggacttacgggtagcagggccagtgtaacgagccatgataagttacctcttttcctttcagccttaaacgcgacgacgcttcggcggacggcagccgttgaacggctgcggcgtcacgtcggagatcgaggacacctccaggccagcagcctggagcgaacggatagcggtctcgcggccggagcccggacccttaacaaaaacgtcgaccttcttcatgccgtgctccatcgccttgcgggcggcgttctcggcagccatctgcgcggcgaacggcgtggacttgcgggagcccttgaagccgacgtggccggaggatgcccaggagatcacagcaccggacgggtccgtgatggacacgatggtgttgttgaaggtggacttgatgtaagcgtggccggcggccacattcttctttacgacgcggcgtccacgacgcgcgccagcacgagtcttcggtggcatgtgttacttcttctttcctgcgatggtcttcttcgggcccttgcgggtacgcgcgttggtcttggtgcgctggccgcgaaccggcaggccgcggcggtgacgcagaccctggtaggagccgatctcaatcttgcggcggatgtcagcctgcacctcgcggcgcagatcgccctccacggtgtaggaggactcgatcgcgtcgcgcagagctgcgagctggtcgtcggagaggttgtccgtgcgcaggtcgggagaaatgccggtcttctcgagcagttccttggctcgggtcgggccgatgccgtagatgtaggtcagtgcgatctccatgcgcttgttgcgcggcagatcaacaccagcaagacgtgccatgaggtcacgttcctttcgggttgttacggtggtttgctccctacccgtccacgccaagcaacgctttgtccggaccgtgccggaggatgggttgtggtttcgcgcggctctggccaccgtggccggaggtagacgagctgtgactcacgcgggcgcgctttgtttgcacgtagtccccgccgcaccgctctgggtaaggaggcgaatgcttatttacttgtagcggtaggtgatacgcccgcggtccaggtcatacggggaaagctccacgatgacgcggtcctctgggaggatgcggatgtagtgctggcgcatcttgccactgatgtgggcgagaacctcgtgcccgttgtccaattcgactcggaacatagcgttcttcaagggctcgacgatgcggccctcaacttcgattgcgccttcttttgccatacactccacttcctaaagcaccggcgtttgcgctggtactcgacgtattttcctgactgctacgcggtgcggaccggtcggcgtgtgcgatctggtctacaccaacgttcgactatagtgcctcacctgcgaaaagcgaaaccgcccacctcggttgcgagatgagcgggagcagtgttgcgaggagcagattctagtagacgtacaccttgtcgccgatctgcagatcgttgaagtacttctgcgcatccttggagtacatgcggatgcagccgtgcgagaggatgttcgggtcgccctcgtggaacgcgatgccgttgttggtgaagtaggtcgcgtacggcatcggggccatgttgaagatgtagctcacttcgtccttgaccttgcggttgacgtagtgggtgcccttcggcgtgtcgtaacccgggcggcccgggccgatgaagacggcgccgtagtacacctggccgtccttctgcagccaggagcggcggccgttgatgtcgatgcaggcctttgcgtccttcgggcaggacccgtagtcgaagcccgggcgcgcctcagccacgggagccggagctggagccggtgccggggctggcttgggtgccggcttcggtgtgcgctccgcgatcaggcccgggaacagcgcctcgacaatcttgtcgatgccctccttagcctgagccggcacctgcgggccgaagaccgcaagcgagtcagcttgccggcgcagcgagttgcgcaggttccacgcgttgtcgcgggaggctttgtcgcgggaagagctcagctccgagaactttttgttggcgtcgttcaggaacgaatccgcggtgacgccggcggaagaggagagcggtgccagcgccgggagcgcggctgcgggctgtgcgaacgcggtggcggcgatgcctgcggtggccaaaagcgcggcggcgcggcgggaaatcttcagcatgaagcgaaagtatagcctgtcaatcgcgcggggtgaggatgcgaggcccctgtgaagtcgctgccacggtgtgctcccagtgggcggccggggagccgtcggcggtgacgacggtccaatcgtcgtcttcaaccacggagtcggtctcgccgccgagtatgagcatcggctcgatcgcaagcacggaaccttcctggatcagcggccccctgttcggccgcccctcgttagccaggaacgggtcctcgtgcatggtgcgtccaatgccgtggccgccgtagccgtcgaggatgccgagcgcgactccaaaccgctcctcggcagctcgagtcgcccgctctagggcgtgggagacatccgtgagtttgttgcccggcaccatcgccttcagcccttcggcgagcacccactcagtcgcgcggttcagcttttccgcgtccggcgccaactccccgattccgaacgaccaagcggagtcccccacccagccgttcagcgtggctccgcagtcgatggagataaggtcgccgtcggcaagcacaatgcttttcgacggaatgccgtgtaccacaaccgaattcaccgaagcacagatggacccggggaagccctggtaccccaaaaacgtgggcgtggcgccgtggtcccggatcaccgtctctgccacagtgtccagatcgagcgtggtcgctcccggcttcgcggcggcgcggacttctttcagcgcggcgccgacgatgcgacctgccgcctccatcgcgtcgagctcctcgggcgtcttcgcggcgatgcgccgtttgcggaatgccatggcggttctccttttcgcggggtggatagtgaaacgcaaaaagccggtgcgagcaccggccaaaacgcgcgagtttatgcggggcttacttacccagcgactgcagcgtgcgggcgttgatctcgtcgacatcgccgacagcatcaaccgagatgatggcgtcgccgtagtggtcgatcaacggcgcagtctcatcgcggtacacgccgagacgggtgcggatcgtgtcttcgttgtcgtcggcgcggccgcgggcaagcatgcgctcaaccacgacgtcttcgtccacgacgaagttcaaaacgccgtccagcgcttcaccgcggttgttcagcagctccgtgaggatctctgcctgctcaaccgtgcgcgggaacccgtccaacaggaagccgtccttggcgtcgtcttggttcaggcggtcctccaccatgcgggcggtcacgtcggtcgggactagcttgcctgcgtcgatgtagctcttcgcctcgacacccagcggggtgccctcgccgatgttggcgcggaaaaggtcgccggtggagatgtgcggaacgccgagtttttccgagagaatcgcggcctgggtgcccttgcctgctccgggagggccgagaagtacgagacgcattatcgcagaagtccttcgtagttagattgcagaagctgagattcgatttgcttgacggtagtcagggcgaccgaaaccataatcaggattgccgtgccgccgaagccgctcatgccgttcgcgccggtgccggcaacacccgcgtccatcgccaggttcggaagcaccgcgatcgccgcaaggtaaatcgcgccaacgaacaacaggcggttcatgacgaagccgaggtactcggcggtggcgcggcccgggcggatacccgggatgaacccgccgtacttcttcatgttgtccgcctgctccaccgggtcgtactggatggagacgtagaagtaggcgaagaagataatcagcacgacgtaggtcaggatgtactgccacgaacccgggttctgcagccacgccatgacgttgttcatccaccagttgtccggctgcgcggtctggttcatggtgacgatctgggtgatcagcaccggcacatacatcagcgaggaggcgaagatcaccgggatcacgccggcctggttgaccttcagcggcaggtacgtggaggagccgccgtactggcggcggcccaccatgcgcttggcgtactgcaccgggatgcggcgctggccctgctcgatgaagatgatgccgaccacgagggcgatgacggcggccagcacgaggaagaaggtgaccgggccggagttctgccagatggtgacaccctcaatcgggatacgggtggcgatacccgcaaaaatgagcagggacatgccgttgcccacgcccttctcggtaatgatctcgcccagccacatgatcaggatcgcgcccgaagtcatgacgataatcatcatgatcagggtccacgcgctgcggtcctcgacgagcaccggcaccccgcggccgagcagctgctcgcggtcggcgagggccacaatgccggcagactgcagcagcgccagcgccaccgtgaggtagcgcgtgtactgcgtcatcttggcctgcccggcctggccttccttcttcagctcctcgaacttcggaatcaccaccgtaagcagctgcacgataatggaggcggtgatgtatggcatgatgccgatcgcgaaaatcgacagctgcagcagcgcgccaccggagaacaacccgatgatggagaacatcgaggcctgatcgccctgcgagatgtcttggaggcgctggttaatcagcgcgtagtcaacacccggggtggggatttgagcaccgacgcggtacaggatcatcagcgcgagggtgatgaggatcttcttgcgaagatccggatccctgaacgcctgagcaattgcggacacaaagcctcctggcttccgccgcgaacacggcagaagagtatggacagtattccaaatgagtcaccccacctgccgaaaggcaggcgaacgctcacccgtacatattggaccccactactctagcagctcacccggcaaagactaagcccgcttgagcttcgcggctcgcaccccaacgcacgatcgcaggccccgcacccgaaagaagttaactccgccacaatcggtgcaaattgtccaactttagtttgagctgacctactctctattcgtactacctaacgtttgcattcgaagtctctatgtaaacggggacgatgaagggaccacgatggacacaattgagcagtctgggcagactgcgactaggcctacgcgcaacgtcagccgaagaagtttcctgcggtggtccgcactggcaggcggcaccaccgctgtggccgcggcggcgggcaacctctttcacggcgtaccgggcgtgggggtaagcaacgctgcggaagcctcgggctcttccagcattttctggtccgcctgcacggtcaactgcggttcgcgctgcccgctgcgcctgcaagttgacgacggcgctgtaacccgggtgctcgccgacgacgccggcggcgacgagatcggctcacagcagatccgcgcctgcgtccgcggccgctccatccgccaccgcatttacaacccggacaggttgaaaacgccgctgaaacgcaaacccggcactaaacgcggcgacggggagtgggtggagatttcctgggaccaggcgctcgacgaaatcgcggacaagatgaaagacttgctcgccgagtacggcaacgaatcgatctacttggcgtatgggacaggcacgattggcgcgactgtcgcgaggtcgtggccgcccgcggaaaccccgttcgctcggttcatgaacctgatcggcgggtacctgaaccactacgccgactattccaccgcgcagatcaccgccgcatacccctaccattacggctcgtgggtcacgtcgaactccttcgacgatgttaagcattccaagctgcaggtcatgttcggcaacaacccgcttgagacccgcatgtccggcggcggcgaaacgtttgtcacccagcaggtgaagagaaaacacggtgtgaagacaatcatcgtcgacccgcgctactccgaaaccgcagtcggcttaggtgatgagtgggtgcccatccgccctggtaccgacgccgcgttcgtcgccggtatcgcccacgtcctcatcgaggaaaatctccacgaccaagagttcttggacacctactgcctcggcttcgacgaggagcacatgccggacggcgcgccggtaaacgcgtcgtaccgctcctacatcgagggcaagggccccgacggcgtggaaaagacccccgagtgggcggcgaagatctgcggcgtgcccgcccagaggatccgccagcttgcccgagaaatgggcaccgctaaaccaaccgcggtcactcaggggtggggcccgcaacgccacgccaacggcgagaaccaggcccgcgcagtgttcaccttggccgcgctgctcggccagatcggcattccgggcggcggcaccggcgcccgcgaaggatccgcctccctgccaatgacctaccccttcaacacccagtacgaaaacccggtggagacctcaatctctgttgcgatgtggccgcaggccgtcgaccatggccgggagatgacagccacaaaggacggcgtccgcggcaaggacaagctcgacgtgccgatcaagatgatctggagctacgccggcaacaccaacacgaaccagcacgcggacgtcaaccgcaccattgagctgctccgcgacgattccaaggcagagctgatcgtggtcagcgacatccagatgacggtctccgcccgctacgccgactacatcctgcccgactgctccaccgccgagcaaaccgacctaattcagcagggctcggccggcaacttggagtacaccattctcgcctcgcaagcgatcgacccgctttacaactgcaggcccatctacgacgtcgttgcggacctcgccgaccgcttcggcgtgaaggacaagttcaccgaggggcgcacccaggaggagtgggtgcgatacacactcgacgagtcccgcaaggacatcccggagctgccgacgtacgagaagctgaaagagatgggcgtgtggcgccgcgagggccaatcggtcatcgcgttagaggacttccgaaaggaccctaacgccaacccgctcgagacgccgagcggcaaaatcgaaattttctcctccgagctgcacaagatcgcaagcgagtgggagttcgacgacgctcaaaccggcgaccggatcaccgccctgcccgagtacgtcgagacctgggagggcgcggaggccgccgcggccagcgacacgtacccgctgcagctgatcggacaccacaccaagggccgcacgcactcctcgtacgggaacgtggattggcttcgagatgacgcgcacccgcaggtgctctggatcaaccctgtcgacgccaaggagcggggcatccgcaacgacgatgcggtgttcgcctacaacgaccgcggtcgtatccgctctatcgcgcgcgtcaccccgcgcatcgccccgggtgtgatctcggtgccgcaagggtcgtggttcaacccgaaggacggcggcgtcgacgtcggcgcgtcggtgaacacgctcaccagctggcacccctccccattggcgaaaggcaacgcccagcacaccgccatctgccaggtcgagaaggcctaagcacccgcgcaataagaagaaggattgtgatcaacaatgtctgataccagcaaggataggctgaatcagcgcctcggtttctacttcgaccagagcctgtgcaacgggtgtaaggcgtgccagatcgcgtgcaaggacaagcacgacacaccgatcggtgtgaactggcgccgcgtggtggagtactccggtggcgattggaacaccgcggacgggacgctgaccaccaatacgttcacctactacacctcgatctcgtgcaaccactgcgacaacccgatctgcgcgcaggtctgccccaccaccgccatgcacgtcggggaagacggcgtggtggccgtggaccctgagaagtgcatcggctgccggtactgcgagtgggcgtgcccctactccgcaccccagttcaatgtggacaagggtgtgatgaccaagtgcgatctctgcgccgactaccgctcagagggcaaagacccggcgtgcgtctcggcttgcccgtcccgcgccctggattggggcccgatcgatcagctgcgcgccgagcacggcgacgccgccggcattgccccgctgcccaaccccgcgttgaccaaaccgcgcctgagcatcaccccgcacaaggatgccaagcggtgggatgcctacaacgccggcgagatcaccaaccacggggagatctagcgacatgaacatgcatgagtggccgttgaccttcttcaccacgtttggccaaatggccgtcggcgcctttgtggtgctcggcgtcatcaccgtcgccggccgcgccaagtactcccgcaacgccatcgacaggatttgtgtgccggcactctacgccatcggcccgatcatgatcgcgggattcttcctcgccttcttccacctcggcaaccccgcgaacgcgctgaacgtcatgcgaaacatcgggtcttccggcctcacgcaggagctggtcgcgggcagtgttttcgcggtgctgggcttcctcttcgctgcgtgccagttcttcgacaagggctcagttgctttccgacgcacccttgcactcctcacagccgcagtcggcatcgtctttatcgcgacaatggcccggctgtacatgctgccaaccgtgccggcgtggaatcactggacgacgccggcagcgttctacctttcgggcgcggtcaccggactgctctctattgcggtggcgttgatctcctacaactggctcgaagactcagccctgataaagcggctcatcccctcggcccgcaacgaggaccaaacgccggagcagaaagcggaagtctggcggctcattagcgactgtctgcggtggatcggcatcgcgctcgtggtggtcgtgccgctgatcttcttggtgatggtgttcaactactcccgccccgagggccccaacccagcggagttcgagttcaacaccactgcctttgttgtccgcatcgtgtttctcttgaccggcgccttcatcgtcggcctcctgctcgccgtaagcggccggaaacaacggcccaccgcatccacgcttgcttggatcatcgtggcttacgtcatggtggttgtcgccgagctggccgggcggttcatgttctacggcgcgatggacagggtgggcatttagtggacacggaacacgcgcagcgtctgagcctcgcagctgacatagtcggccagctttttctcgacgaaccttcgccagagatgctgcaagcgctcaccaaccctgacctgttggcggactggccgctccaggacgcgtcctcgcgggcagccgctacctcgctcatcgagcgcgcggaatgcggccgcccggacaccgttgaggacctcaaacgcgaccacctctacctcttcataggggccggaacaccactcgcccagccgtacgagtcgccttacttctctcccgacggcctcgtgctcgatggcgcagctgcggaggttgaggcggcgtacaaagccgtcggcttcaacgcgacgaagcagtggggcaacctcccgccggaccaccttggtttggagctgcggtgtatcgctcacgtcgcagggatggccgcgggcgccgcgtcggtcgatgagcgcgagcgtcttgtgggcttcctccggtcgtttaccgcctcgcaccctgcaaggttcgcagatcaggtgctcgacggcgtacaacagcacgcggcaaccggcgtgtaccaggctcttcctagtttgacccgcggcgtcctgcacgccgcccttcgcatccgctgatccaggcaaacaaaaacggcccgctttccgatggtgtttcggaaagcgggccgcctgcttagcccgtgcggggtctaggcctcggtctgatcggaatcgatcaccgtggagccgccctgcagcgggtcggagtcgaggacgccgcgggcaccctcggtggcctcagccgccggggtcgcgtcgccggccgcggaagcaaccgggccctcaacgttcttcgcggcgcgcgggcggaactcctccgtggtggtggagccgccggcagcctcgatcttctctactgcggacttcgagaacttggtggcggtcacgtcgagcttgacgttgatgtcgccgttgcccagaaccttcaccggctccttagcgcggaccaggccagccgcaacaatgtcggcgatggcgatggtgccgccctgcgggaacgcctcggccaagtcggaaacgttgaccacctggtactcgatgcggttcgggttcttgaagcccttcagcttcggcagacgcatgtgcagcggcatctggccaccctcgaaagcagcggaaacctgcttacgagccttggtgcccttcgtaccgcggccagcggtcttacccttggaggcctcaccgcggccgacgcgggtcttagccttgttggcacccggagccggacgcaggtcgtggagcttaatgatgtcagccatgtgctatctactcccctgctacttcttcaacggtgaccaagtggcgcaccgccaggatctggccgcgggtagcggcgttgtccttcttcacaacagactggccaatcttgcgcagacccagagcctccaggttcttgcgggtgaccggcttctcgcccaccttgccgtggtgcaacgtaatcttcagtgccattgttctttacgcctcctgacctgcgcgtgcgcgcagcatacgggcgggagcgacttcctcgacggacttgccgcgcttagcagcaacttcctcggggcggacgagctccttcagagctgcgacagtcgcctgaaccacgttcagcgcgttgtcggagccgagggacttcgccaggatgtcctgaacacccgcgcactcgagcaccgggcgcactgcgccgccggcgatcacaccggtaccgggagcagccgggcggagcataacgatgcccgcggcttcctctgcctgcaccgggtgcgggatggtgccgccgatcatcgggacgcggaagaagttcttgcgagcttcctcagcacccttctgaatagcagccggaacttccttcgccttgccgtagccaacgccgaccatgccctggccgtcgcctaccaccacgagcgcggtgaaggacatgttgcggccgcccttaacggtcttcgcaacgcggttgatggtgatgacgcgctcaatgtacttgtcgcggtcatcgttctggttgcggcggtcgtcgcggtcgcggcggccgcggccgccacgctccccgcgctcgccgcggttgttgttgttctggtcgtcggcggagcgcccgccgtcacgccgttcacgttcggccattacgcgatccttccgttgatggtgttaattgcggtgatcattaaaacttcagaccaccttcacgagctgcgtcagccagcgccgcaacgcggccgtggtacttgtagccgccgcggtcgaagacgatggcgtcgatgccagcttccttcgcgcgctcagcgaccagcttgcccacctgggctgccttgtccttcttgtcgccctccatgtcacggatggacggctccatcgacgacgcggagaccagggtgtggcctgcaaggtcgtcgatgacctggacgtggatgtgacgcgaggtgcggtgcacgacaagacgcggggtctccggcgtaccgcgcagggtcttgcggatgcggtagtggcggcgtgcgcgagcctcgcggcggcgggacgagatgtccttgccaaccggggtgcgcttcgcgtttgcagtgttctctgcggtgttgctcatgattacttacccgtctttccgaccttgcggcggatctgctcaccctcgtagcggatgcccttacccttgtacgggtcatccttgcgaaggcggcggatgttcgctgcaatctggccaacctgctgcttgtcgatgccctcgatcgagaacttggtattgccgtcgacggagaacttgatgccctccggcgcggtgatcaggatcgggtgcgagtagccgagggagaactcgaggtcctggcccttctgctgcacacggtaaccaacaccgaagatttccatgttgatcttgtagccctcggtcacgccgacaacgaggttgttgaccagcgagcgggacagaccgtgcagagcgcggttgttgcggtggtcgtctggacgggacaccacgatttcgttgtcctcgacggaggcggtgatcggctccggcagatccagggtcagggtgcccttcgggcccttcacctcgacgtgctggccgtcgatcttcgtctcaacgccgttcgggatggcaataggtgccttacctacacgcgacattgttaatccaacctccctttaccagacgtaagcgaggacttccccgcctacgcccttctcttgtgcctggcggtcggtcagcaggccgtacgacgtggagatgatcgccacgccaaggccgccgagcacctgcggcaggtcgttggacttcgcgtacacgcgcagacccggcttggacacgcggcgcagaccagcgatggaagcctcgcgggtcgggccgtacttgaggtcgagggtcagcgtcttgccaaccttctcgtcctcaaccttgtagtcgttgatgtagccttcctgcttcagaatctcggcgatgttcaccttgatcttcgacgaaggcatggacacgttgtcgtgctgcgcgtgcgacgcgttgcgcacgcgggacagcatgtccgcaatcggatcagtcatggtcataagagaccgtttccctttctcgttgcggttccctaacccacctgacccgtatagataaggtcgcgttctccgtgtggtctgtcgggggctacttcacgctccccacgctcagtaacgtggggcgctcgccgcctcccttgcacgcggtccgcatttcggcggggggcctgcaacaaagttggatggtgtaaaaaacttctcggacataagtccgacggtctaagctacctgctccgccacacgataagcaaatcccctgccgcgccctaacacggcagcgccgggcgtgcttggacgcgggtctgtccgatgtcggtcatgctgcccgcgtcttggccctggaagaaggcggcgggatcaagcgagcgcttgctagcccgcgctgcgccaatcgctagcccatggtccactgcgtattcgtcgcgggcggtttgggcggccgacagatcgccgacaagcaccagcccgtacccctcgttcgacgaggcgacggtctcctccgcggcttggaggcgctcggcgatgcggtgcgcgaaccccgccataaacgaccggcggctcaccacaagtgaatcgaactcgctctccttttgcagtccgcgggccttggccatcatcaccggcaacagtagcgagtacagcatgtccacccgctccagatgcctccccaggccgaagatggtggcctccttaaccctggtcgaacacgaagcgctccggtgaaaacccgtgcagtggagcgcgccagcaatagcgtgaagcagacgcgactgcatgtcggtgtaactaccgctgaatgtgtacgtcttgtacgtcgggcggtcgccctcgtcgagcgctgtgaggtcgcgttcgtcgaacccgtacgtagccatgagcgtgaacgccttgtcgtagaacgagtcgccctcgggcgttccctgccgatcggccgcctggttgagcagtttttgcaccttctctttgattttgtcgatgttttgcaaggtaatcccctcttttcgttgttggtgtcacagttatatcccgctgccccaacacggccaagggcataccgcgcgagcctgtggaatttgcctcggtgcccctgtggacaacccgcgttcactacagtgaagtgccatggctgagaacaagagcgacacatcactgaccacgacccaccgatggctcaccgctgtggcggaagagctcggcatcgacccggagctcgtgcgcggcctcgtcggcgacatcctcgacctcacggcggcagtggcccacaacgggccgtcgcgcccagccgcgcccaccaccgccttcgtcgtcgggctcgcagctggcgcaggggccggcgacgccgctacagtgcgcgacatggttgcgcgggtagaggagatgctgtcgacgtatgagcagaattaaccgccgcttcgcggtcaccaaggtcacccggggacagggcgacagcgcggggcggttctacaccgacactcgcgcggacaccgtgacggtggaagagccgctagaaatccgcgcgggcggagacacgctgacgaccacgatgcgcacgcccggccacgacatcgagctcgcccacggctggctttacgcagaggggttaatcaagcgcgccgaggacgtcaccactgcccgatactgcgcaggctcgcagaaccccgagggcaccaacacctacaacctgctcgacatcgaccttgctgcgaccgcaaagccggtcaccccggagttcatcaggctcacccccaccactagcgcgtgcggagtgtgcgggacgcagtcgatcagcgagatcctgcacaagacgcatcagcccatcgagcccgtcaagctcaacccggacttggtgatgcgcctgccggacctgctcgccgccgagcagcagcagttccgcaagaccggcggcattcacgcagcgggcgccttcgacctggacggcaacgcagtggttgtcagagaagatatcgggcgccacaacgccgcggacaaggtgatcgggcatttgcttctgggcggcagcctccccgcctccgacctcatcctggtgatgagctcgcgcgcctcattcgaactggtgcagaaggcggccatggctggattcccggcgctggtggccgtgtcggcggcgtcgtcgttggcagttgagctcgcccgcgaggcgggtatggcgctggccggcttcacccggcccgaccgtttcaacttgtacgccggcgaacttgcgtagggtcgaatgcatgactgcacgcgaagtgtcccccgggtaccaagcgccgttctaccccgctgtccagcacgtggagtaggcgctcgaacccgagaccgccgagcacgtcttccttcgcgcggccgcgctcaacggctgccgcgtgtgcacgaccacgcaccgccgcaactcgcgcgtcgcgggctttagcgaggagaagatcaccgcgatcgagaactggaccgagcacaaggaccagttcgacgacaaagaaactgcgctgctcgagttcaccgacgcagtgaccaagctcgaagaccgcgaggaagcgatctctgatgagctttgggcgcggatggaaacactacggcgccgaaggcacccgcaatgtgctcgtcgccatcatcacgatcaacgtgtacaaccgcttcggcatcgccgcgcagatggacccggcgagtgtgaaggacgccagcgagttcgacctcgcgcagtaaccgcccggcagccaaaacccgcacctcccagtctcgggagatgcgggttcacctcgtgcaacgtggtctcgggtcagtccttgtacaccgtcttggtgttgttcagccaggcgtagacggcgccgatgccgaggccgccgccgatgaagttgcccagccacaccatcagccagttcaggccgacggcgccgaaggtgaagttctccggctgcgggtcggcgaacagggtcatggtcatgagcgagaagttggcaatgatgtgctcgaggcccaggcccacgaaaatcgcgatgatcggcacgatggcgaagaacttggacacaatctccttggactgcagcgccatcacgatggccatattgaccacgaagttcgccaggaccgcctcgatgaacgcgccccacgcggacttgtccaccttgccttccgagatggtggcgatgaggtgggtgttatccattgagcccagcttcgccgactggctcaggatggcggcgacgatgaacgcgccgacgaggttgcacagcgtggctgcgaccacgaaccagatggtcttgccccacgactggttgcctttggcggaggcccaggagccgaacatcatgtcgcccgtggcaagttcgccgttcagcacgacgatggcgaagaggccaaatccgaagagcagcgcgaaaacgacgctgccgagccccggcgcgagcttctccaccgcgttgcccgcgacacctgcgaacgcggtggcgacggtgaggtaaatgccggcgaggacggcgcggccggcgaaacgaccgaagtcgttgtcgaggagctcaacctttttggctgcgcccttatcaagtgtttctgcgagagacatgtgacagaccttacaccccacccagaaaacgccgaagcccccggtcccgctttcaacgggtgccagggggcgtcggcaagcatcaagcccttaggcctgctgcatcttgccgtccttgtcagcgaacgggaagccgaggtggcgcaggagcgcgcggccctcgtcgtcgttggtggcggtggtcacgagcgtgatgtccatgccgcgcacgcgatcgatcttgtcgatgtcgatctcgtagaacatggtctgctcggacaggccgaacgtgtagttgccgttaccatcgaactgcttgtcgttcaggccgcggaagtcgcggatacgcggcagcgcaacggtgagcaggcggtccaggaactcccacatgcggtcgccgcgcagggtcaccttcgcgccgatcggcatgccctcgcggagcttgaagttcgcgatggacttcttcgcgcggcgcagctgcggcttctgaccggtgatcgcggtgaggtcctcgagagcgccgttgatcaccttggagtcgcgggcagcgtcaccgacgcccatgttgaccacgatcttggtcaggcccgggatctgcatgacgttgtcgtagttgaactcgtcgttcagcttggtgcggatctcgtcctggtagcgggtcttcaggcgcggggtgtaggtcgaaacagtctgggttgcttcagtcattgttagatgtccttcccgttcgacttggccacgcggaccttcttgccgtcctcgtcgaagcggtagccaacgcgggtcggcttgccgtcggagtccaggatcatcacgtttgagacgtggatcggggcctcctgggtcacgatgccgccggactcggcgccacgctcgttgtaggagttcgcgacgtgcttcttgatgcggttgacgccctcgaccaggaccttgtcacgctgcgggtaggccgcgatgaccttgccctgggcgcccttgtccttgccggcgatgacctgcaccatatcgcccttcttgatcttcatgggttagatcacctccggtgcgagagacacaatcttcatgaacttcttgtcgcgaagctcgcgagcaaccgggccgaaaatgcgggtgccgcgcggctcggtgtcgttcttaatcagcacagctgcgttctcgtcgaaggagatgtaggagccgtccgggcgacgggtctccttcttcgcgcgcacaacgacggcgcgcacgacttcgccttccttcacgttgccgcccggggcggcttccttcacggtggcgacgatggtgtcgccgataccggcaaagcgcttcacagatccaccgaggacgcggatgcacaggatctcacgtgcacccgtgttgtcggcgaccttcaggcgcgattcttgctgaatcacttgtggtctcctgacctgggtcaatgtgcgccagatttccgtcctgaacgcacgtggtcaaagtattgcttgaagcctattgcttatcgacgaaccccgttcgctcgttcctcgcgcacgagggggagcacaacgtggtcgaagggtctcgggcgatccactcggaaacgcgcgtcacgcccgaccagcgcaagacaactggaacagttaatcacgccagctagcgaacctcaaattcccgtctcgcttcttggtgatacctgtaataaattgaaaatgtgagtttctttgaagctgcccccaaaatcatttccaacaagttggctctgtttgggcaagagccggcccgcttcgccactcgagcaatcctagcgggcgtctacctcggcatcatgaccgcgttcgcggcctccaccgcgcagttgctcgacgagtacgcgcccggctggggcaagtacgcgttcggcgccatcttcgcctccacgctgtatatcatcatcgtcctacaaggcgagctcgccaccggtgacatgatgttcatgacctacgggtccatacacaaactgaccgccttctggcgaggcgttctcctggtcctgttcgtcaccttcttcaacctcgtcggcgccgtagtcatcgcttggctcatctcgcggaccaccatcggccagcacgtcgaagcggacagcttcctccacgggctcctcgtggccaaactgcagaaatcctccgccaccttgtttgtcgaggcgatcctggccaacatggtggtcaacatcgccttcatgctggccacccaggccggcaaggactacagcgccaagctgtggggcgtcatcttgattattccgtcgttcgcgaccatgagctacgagcactccatcgcgaacttcatcctcaccaccctcggcggcttcaccctcggccccgacgcgatcgagggcttcaccgcttggaacgtgattcgaaactggtccgttgtgtggctgggcaacttcgtcggcggcggcctgatcatgggtggcctttacggatggctgaacctgacgaagaccgactataaggactagctgctcccttacgcttgcctgcggcgtgcgcgctcgacatcaaccttttcgagctcgtgcgccgctttttctgtccgcgtgccgcgacaccgctgggctcgcatcgcgacgcgggctggcgtgtctggaaagatggtcggcgtgaatactccagcagttcagccatctgcacagccgaccgcgtcccccgcgggcaacgacccgctcgatgcggtccgcaccctgcgcgacacgctggcggcaaccacgctcgcgcccgacgtggctgcggacgccaacgccgtggtcaaccagctggacgactacatcctgccgcgcctggctaatctcgacgcgccacttttagccgtcatcggcggctccaccggatccggcaagtccaccctggtcaacgcgcttttgcgagagcgcgtctccaaccccggcgtcatccgccccaccacccgccaaccggtgctcgtggccaacccggcagacgcggagtggttcaactcccctcgcgtgctgcctggtctcacccgctcccacggcgcgggcaacgaacagtcgaccgcgcttcgcatcgtggagacgcaaagcatcccgcaggggctttcgcttctcgacgcaccggatttcgattccatcgacgaccgcaaccgcgcgctcgcttcccagctgctcgccgctgccgatttgtggatcttcgtcaccactccggcgcgctacgccgaccagctcgtgtggaatttcttgaacgacgcggccggccgcggcatcgaggtcctggtggtgctgaaccgcctcgacgaggtcgcccagaagaccgtgccgcaggacctgcgccgcatgatggacgaggccggcctgacaggcgccaccgttttcacggtgccgttcgtggccgacctgggcaaagatgcagcagccgcagacgagttcttggacgctgcgctggtcagccccttacgcgactacctgcagcgcttggcggaggattcagccgcccgccgcgcggtcgccggcaagacggtcgcgggcgcgctcgagggcgcgctagaccgggtatccgccatcacggagagccgccagcgccgcgaggacttcgccaaccagctcgacgaatccatcttcgagctgtacaagtccgcgcaccgccacatcattgacgcgacctccgacggcaagatgctgcgcgccgaggtcatggaccgctggcaggacgtcgtcggcacatccgacgtgatcaggggttttgagcggtggttttcgcagacggtggacaaggtcggcagctttttctccggtgaaccggcgccgatccgcgaggtggagaccgagctcgagtccggcctgcacgccgtgatcgtggacgcggccgacaccgccgcctcccgggcctgggcgcacgtcggcgccgtcgcaccggagctgcgccagcacgccgatccgtctcttgcgcgcgcgagcgaggacatcaacgcccgcgcggcgcagctgatccgcgactggcagtccggcattgtcgagcacattcaggagaccgccggcgagaagcgccagcgcgcccgcgtcatgtcgctgggcctgaacgtggccacggtagcgctgatgctcatggtcttctccaccaccgcgggtctgacaggtgtggaggtcggcatcgcgggcggctcagctgtggttggccagaagctgctcgagacaatctttggagaggacaccgtccgccgcatggcctcagacgcgcgccgcgacctcgacatgcgcctcgacgacctgctgcgcgaggagcgcgagcgctacttctcgctcactgaccccctactccagggcgcatccgcggaaaccatccgtcaggcggcggatggggctcgaggggccgtcgataagcggttcccgggtgtgctcacaccgctgcccgcacctgctgccaaccctcctgcggtacgcgaggacgtccaggcgagctttgaaagcggcacgctgcgcggcctgttcgaccagctgcgcggcacgttcgggcaggagcgaaactaatgggcatcttttctgcgaagcccaccctcggcgagcggctaaacgcgctggatgaggccgccgacattgccgcgccgtacctgccccaggtggaggttcaccagctcaagcgcgtcgcgacgtctggcgccgaacgccgcgcgctgtccgccgagcacaccgtggtgggcttcttcggcgcaaccggctccggcaaaacaagcctctttaacgcggtcgtcggcgaggacttgggcaaggctgcggcgaggcgccccaccacgtcctccccgctcgccgccgtctggcacccggagggctccgaggaactcctggactggttgggagttgaggaccgccgcaaccgcgagggcgatttcgccccgcacgctggccccatcatcctgctcgacctgcccgatttcgactcggtcgaactgtcgaaccgcgagatcgccacgcgcctcgccggccaggtggacgtgctggtgtgggtgtccgacccggagaagtacgccgactccgttatccacgaacagttcattcgaccgcacgccggccacgccgcggtaacgcttgcggtgctgaacaaagccgacctgctccacccgctcgaccggccgacggttgctggcagctacaaggagcttttgcttgccgacggcctgtcaaacatcaccgtcatccccacctcaacccgcagcggcgacgggatcgacgacctgcgcggcgcaatcgcgaaggtggcgaaagcccacaacgcccagtccgcccgcatcgaggccgacatcaaggccgcgacccgcgagttcctccccgcccgcgaggccggcgccgtggacaaacatgcgaagaaacagctcgacgctgtgctttcgcaggccgccggcgcagaccgcatcgccgacaccacggctgcggcctaccgcaagcgcctgcgcgagcgcaccggctggctgctgacatcctggatcacccgtttcaggcccgaccccttgaagcggctgggcttgcgcgaagaggccgacgaggtcggcgtgcaccgcacctccatgccggagcttgacgccgcgtccaaggcggtggctaacaaaggactgcgcgactactcccacgccgctgctgagggactgccccacgcgttttccgccgctatcgccgaccgcaccgaagacatctcccaggcgctgccctcggagctggaccgctcgatcgcacgcacgcagctgcccgcggagccgtcgaagggctggtcgatcctcactgtcttccaatggctcgcgctcgtcgcggcacttatcggcgtcatctggtacctcgtggtggcgttcgtgcccggtgtgctcaccccgctcgtgggcgataacctcgtcccgcaggtcgagggctggccggtgccgacgctgttgatcatggccggactgctcatcgggttggtaatcggcctgattacctccgtcttcggcggggtgatcggcggtaacgtgcgccgacgcacccgcgcagcaatacagaaagaggtggcggccacctcgcagaccaccgtcgtcgaaccgctgcaggcgatccgcaacgactacgaccacttcgccaaccgcatcaccaccgccgccaagtaggtacgttggggtggcatgacaacgcgaatccccaacgtgctttccatcgccggcaccgacccaacaggcggcgccggcattcaggctgatttgaagtcgatctccgtcgcaggcgggttcggcatgtgcgtggtcacctcactcgtcgcgcagaacacccagggcgtgcgcgaaatccacaccccgccgcaggagttccttcaggcccagctcgctgccgtgttcgacgacgtccaggtcgacgcggtcaaggtgggcatgcttggcgacgccgccaccacaaacacagtctccgagttcctgaagggccagggcgtgcccgtcgtggtggtcgacccggtgatggtggcgacctccggcgaccgcctcctcacccaggacgcggaagaggcgcttcgccagtttgtgaaggatcacgccaccgtggtcacgccgaacatcccagagttggcggtgctgacgaataacgctgaggctgaaagcttcgaagaagcgctcgagcagggccgcgactacgcccgcgcgaccggcgtggcggtgctggtaaagggtgggcatttgagcggcgacgccgcatccaacgcgctggtccagcccgacgggaccacggacgtcgccgaggtaccccgcgtggacaccaagaacacccacggcacggggtgttcgctgtcctcagcgctggcagcgcgcctgctgctggattcggaccccgctgccgcgcttgcctggacctcgacctggctgcacgaggcgatcgcctcagccgacgagctcaacgtgggcaaaggccacggacccgtgcaccacttccaccggctctaccgcttggcggacggggtctaagccgcccctactcgtagcgcagcgcctcgatggggcgcatgcgcgcggctcggctggccgggtaccagccgaagaagagcccgatcgcgagcgagaacagcagcgcgatcagtacggcgcttaccggtggcagcgccatactgcccatcgccgaggtgccggccatacccaccgcggtacccagcagcaccccgatgacgccgccgagcaggcagatcatcatggcctctgtcacgaactgggtgcgcaccgcccggcgggtggcgcccagcgccattctcacgccgatctcccgggtgcgctcggtgacggacaccagcatgatgttcatcacgccgatgccgccgaccaaaagcgagatgccgccgatagccgagatgacgaggctgatcatggacatcgtctggttgacttgatcaatttcggacttggtgtcgagcaccttcgcctcgaaatccgcgtcgtctgcgtacgcctgctccgcccacgtggtgacgtcttgggacacgctgtccgtgccctctggggtgagcgcgcggatctgcatcatggagaaaccctggacggggtcgctagcaagccgggcttgcgctgtgtacggcacgtagatcagcgcgtcctccggaacgtaaaccagcggcgaggacttcgcagcccgcccgtaggcgccaaccacctggaagctggcgtagcgcccgccgacctcgacgtcgagattcgcgccgacggccgaatcggggtccccgttgaaatacttctccacgacttccggggagataacggcgaccgcccgatcagcggcgatgtcgtcgtcggtgaacactcgcccggcggtcagggtgtggttctggacctcgatgtagtccgcgttgacgaactcgactccagccttgccctcgttcagcccccgggtgacgcgggcggtctcgcggccggcgtcgagcgcaatgccttggatttgcggaccaatgtaaccgcggagttggtccaccatctcgggcgtgatgagcgattcctccggaacttcctcgtagtaccaggtgtctgcgtcttgctcggtttggcgagctttgacttgcacgttaacgtcgttcagcccgaactgctcaaagtcgtccaagagctgctgctgcattcccttaccaagcgacataatcgccaccactgccgcgatgccgataatcacgccgagaagtgtcagcaccgagcgcagcttgttggcccgcaggctcgtgcttgcaagcctgagcgcctcgcggggattcactcctgctcgccgccgttatcaagcagcgcgacccgggtgcccaccctgtcgcggtagtcccccggcgacttcaccacgcgcgtgccctcgggcaaacctttaacctcggcctcgaggtcggtgacgagtccgagggtgacgtcagcgctcgcgacgtcgtactcctcctcggagccgtcgactggggtgagcacgatgacggagtaggagccgttgttgtcgataaccgcctcgcggggcacggttagcgtctccttcgccgtgccagtggtgatctgcaccttcgcggtgccgccgatgcggagcccctccgtgtcgccggtgacttcgatggtgacggggaactccggccgcgccggggcttggccgccctcgggcccgcccggggctggcgccgcaacagaggaaatgtcggtgaccttgccgcggtactgtttcatcccgctgctcggagtagtgaaggtgacctcgttgcccaccgtgatcttgcccgagtcaacctcgttcacgttcgcggtaaggatgagccggttcgggtctgcgacggtgacaaggtgccccgccgacggttgaccgcgctgcgcgatgacctcggtgaccaccccgttcatcggggagcggacctcgccggaggcgacatcgacgcgcagctggctctgccccacctcggcagcagcctgggacgcgctcaggctgcgctgcgcctggtccacgctggaggcggtggctgccagctcctgctgcaccgacaggcgcgtgacctcgagagcgatatcggcgttgttcttcgactggaacgcctgggaaaccgcgcgctgcttcgcctccaaatcggcgtcgactgcctggagggaggcatcgtaggcgcgctgcgcggcgtccagctcgcgctgggcgccggtgtagcgctcatccgcctcgaggatgccgatgacggggcccatctggtcgatctgcgaggtcagcgccgagaccacgttgttgacgttcgcgcgcaccgaatccaacccggcaagcgtgacgttgcggcgggccgcgtcgaccgcgttcgcctgctgcacgatgtcggggtccatgccggactcgtggagttgcttttggtggttgaaggtggccaacgcgtcgtcgtaaagcagctgagcctcgcgctgcgccgcctcggcttgcgtgatgcggctgttgagcccgcggttcagcgcctcctgctgctgccccagctcctgctgggcgcgctggagctcgttctgcgacgccacgtccgacgtcatctgctgcgcccgctgggcatcgagctcgcgctgcgcgctcgaggtgtcgacccgcgcgacgatctggccctcctgcaccggctggccgacgcggacgtcgatagccgtgacgggacctgtcagtgtggtggtcagcgcgaccacctccaccgaaccgatgttggcgctcgccgacacctttgaaaccacgtccttcggcgccagctgcaccgtgtccgatgcgggcacggccccggtgccgtccccgcaggcagcaaggagaagcgccgcgagaaccggcgcgctacgagcagcgagctttcgagttttcacgcagttaggatagcaaagctaccggcgctactcgacggtcacagacttagccaagttgcgcggctggtcgacgttgaggcccttcgcctccgccaccgcgcaggcgaagacctgcagcggcaccgtcgccagcagcggctgcagcaggcccgctgattcagggatgcggatgatgtggttggcgaactggaccacgtcctcgtcgccctcctccgcaatgacgatggtgacggcgccgcgggcgcgcacctcctggatgttggagacaaccttggcgtgcaggttgttgcgggacagcttcgacgggacgatgacgaagaccggctgcccctcctccacaagcgcgatcgggccgtgcttgagctcgcctgcggcgaagccctccgcgtgcatgtaggccacttccttcagcttcagcgcgccctccagggcgaccgggaagccgacgtggcggccgaggaagagcaccgacttggcgtccgccagctcgtcgcccagctcgcgcacctcgcctgcgcggtccagcacctgctggatcttgtccggcatttcctgcagctgcgccacaatgcggcggatctcatcggcgtacttgttgccgcgcacctgcgccaggtacagggcgagcaggtacgccgcaacaatctgggagatgaacgccttcgtcgacgccacggcgatctcggggccggcgtaggtgtagagcacggcatccgcctcgcgcggaatggaggcgcccacggtgttgcagatcgcgattaccttcgccccctgctcgcgcgcgtggcgcacagccatgagcgtgtccatcgtctcgccggactgggaaaccgccacgaccaaagtctgctcgttgacaatcgggtcgcggtagcggaactcgtgcgcgagctccacctccgtcgggatgcgacaccagtgctcgattgcgtagcgggccacctggccagcgtaggctgcggtgccgcatgccacgatgatgatcttgttcaccgagcgcagcaccgactcatcaatgcgcagctcgtcgagggtgagcgcgccggtgtcgtcgaaacggccgtagagcgtgtcgcgcacagcagcgggctggtcgtgaatctccttctccatgaaggagttgtagccgcccttctcggcggctgtgatgtcccactcgacgcggaatgccttgccttcagcagcctccccgtcgaaggtgatgatgtcatagccgtccgccgtgacggtgacaatctggccgttgtccatctcgaccgcgtcgcgggtgtactcgatgaagccggaaacgtccgagctcaggaagttttcgccctcgccggtgccgatcaccagcggcgagttccagcgcgccgccacaattttgtcgggttggtccgcgtggatcgccagcagggtgaacgcgccctcgaggcgctgcgcggtcagctgcatcgcctttgtcaggtccgcgcctgcttctgcgttgtagatgtccagcagcagcgtcgccgcaacctcggtgtccgtctcagaggcgaaggcgtagcccttgcccgcaagctccgccttcagcgcggcgaagttctcgatgatgccgttgtgcaccaccgccagcttgttgccgccgacgacgtgcgggtgcgcgttctcgtccgttgggccgccgtgggtggcccaacgggtgtggccgatgcccaggctggaagtgtccagcgggttgtccgcgatttcggcctctaggtcggcgactttgcccgccttcttccggcactcgatggtgccgttcgccgcgatggcgacaccggctgagtcgtagccccggtactccaacctgcgcagcccatcaatgatcacgttcttggcgtcgcgctgcgcattcgcagcgacatatccgacgattccacacatgggaaaaacgctacacgcgatcacccacgtgggtagaaaataggtacgctcaggtgctttcttcgatgccggcgatgtcccgggcggcctgtttggcaaagggcgccacacccatcaacgtcgccgaaccttcgccgttccagttgccgtagccaacaaggtgcagattgtccaccacaggttcgcgaccgcgaacgaggtgacggaacgggccgagggctggccggaagccagtgcaccagatcaggtggtcgtgatcaagctcatccaggttgtggaacatgggcgtggcggtgagctggtgggaatcgcggagctcacggagacgaggaagcgcgacaatgtccccgagatccggcccagcaatgccgcccaggatctgtcggcggctgcggaggaaaaggtctcgtccgtcgacgtcatcaggcatccagcgaggctcaccccgcgtgaaccacgtgacctccgcagtgccaatgaggtccccggcgatctgcgcacccgagttcgcaccgccaaccaccgcgacctttgcgccgcggaacggttcaggcccagggtaggtgaccgtgtgccactgacgcccgcggaacgtgccgggatagtggggcacaaaaggcgcggaccaagtgcccgtcgcggcgacaagatggtttgcagtgaattgaccggcgcacgtatccaagcggaacaccccgctgtcgtgttccacgtctcggacatcgaccgggcgtcgaacgggcaggtcgtatctgcgttcgtagcgttcgaggtaatcgacgacgtggctcgccggcggataccccgggtgcggcggcataggccagccgggcaggttagaaaatcctgcggccgaaaacagcgtgagcgaaggccacgcatgcaaccacgccccgcctggggcttcttggttgtccaagacgaggaagtccaccccaaggcggcgcaggtaataggcggtggctaggccggattgaccaccaccaacgatgatggcggtatggtgctcagccaacgaaacccaccactttcggcatgcgcggtagcgccgccatgaccttgggcaggtgattcatgacggcgagtctagtcagttgcccataggtacggcgaaacccgcctcggccctggagttgggctgggcgggttgacgcttgcgtcgataagcggtgcttgcttaacgagccttctcgatgatctcgacgagacggaagtgcttgtccttggacagcgggcgggtctcctcgatgcggacgagatcgccgatgccggcggagttggtctcgtcgtgcgccttcacgcgcgtggtggtacggacgatcttgccgtacagcgggtgggacttgcggtcctcaacctcaaccacgatcgtcttgtccatcttgtcggacacgacgtagccgcggcgacgcttctgcaggcccttctccttcggcttcgcctcagtgtgcttcgggcccttgccagtgttgttctcagtcacgtttgcctcagtcatggttatgcctcagctcctgcagactcgggtacaacggacaggccgagctcgcgctcgcgcagcacggtgtagatgcgtgcgatgtcgcgcttcacggtggagatgcggcggttgttggtcaactgacccgtcgcgagctggaagcgcaggttgaacagctcttccttcgcctcggacaggcgggtgcgcagctcatcgtcgttgagctcgcggaattcggatgcgggggtaccggtagccattagaactggtcctccttcttgatcacgcgggtcttgcacggcagcttcgcgccagcgcggcgcagagcctccatagcagtctcctcgttcgggtaggacatctcgaagaggatgcggcccggcttcacgttggccacccacttctcaaccgggcccttaccggaacccatacgcacgccgagcggcttctgggtcagcggacggtccgggaagatgttgatccagaccttaccgccgcgcttgacgtggcggttgatcgcgatacgagcggactcgatctggcggttggtgatgtaggccggctcgagagcctgcaggccgtagtcaccgaagttgatctggttgccgcccttggacacgccggaacggcccggacggtgctgacggcggtacttcacgcgcttaggaataagcatgtttagccctcctgcttctgctcggcgcgctgctggcggcgctggccaccgcggcgcgggcggcgatcgcggtcgccgcggccaccgcgctcgttcttcggtgcgttgagctcagactcacgaacgccaccgacgacatcgcccttgtagatccacaccttgacgccgatgacgccgaaggtggtgtgtgcctctgccgtgccgtagtcgatctccgcacgaagggtgtgcaggggcacgcggccttcgtggtagcgctcgacacgggacatctcagcgccgcccagacggccagaggtcatcaccttgatgcccttgacctgcgggttgcgcatcgcggactggatagccttgcgcatcgcgcggcggaacgccacacggttgacaagctgctcagcgatcgactgcgcgaccagggtcgcgttggcgtcgacgttcttgacctcgatgatgttgagggcgaccatcttgccggtgagcttctccagctcgcggcggatgcggtcagcctcagcgccgcggcggccaatcacaatgcccggtcgggcggtgtgaatgtccacgcggacgcggtcgcgggtgcgctcgatgacaacatcggcgataccggcgcgctcgaggttcttctccaggtactcccggatcttgatgtcctcagcaacgtagtcggcgtagttcttgtcggcgtaccagtgggacttccaatcggaagtgatacccaggcgcaggccgtgggggtggattttctgacccattagttcgcctcttccttggactcgacgacaacagtgatgtgggaggtgcgcttccggatctggaatgcgcggccctgtgcgcgcggctggtagcggcgcatggtcgggccctcgttggcgtagcactctgcgataaccagggtgcgcggatccaggccgaagttgttctcggcgttggccgctgcggacgcgacgaccttggcaaccggcttagcggcgtcctgcggcgcgtacttcagaattgcgagggcctcggacacggacttcccgcggacgagagccagcacgcggcgggccttcatcggggtagtgcgcacgaacttggccgtcgcggatgcagtggtgatggtctcagccattgcttatcgacgtcccttcgtttccttgacgtgacccttgaaggtcttggtgggtgcaaactcgccgagcttgtggccgaccatggactcgtctacgaacaccggcacgtgcttgcgtccgtcgtggacagcaaaggtgtggccgatgaaatcggggagaatggtcgagcggcgagaccaggtcttgatgacctgcttggtgccggcctcgttctgagcgtccaccttgttgaggaggtgctcatcgacgaacgggcccttcttcaggctgcgtggcatgtagtcttacctcctcttagcgcttcttcgtgcgacggcggcgcacgatcatgttgttcgagtaacggttcgggttgcgggtgcggccttccttctggccccacggcgaaaccgggtggcgaccaccggaggtcttaccctcaccaccaccgtgcgggtggtcaaccgggttcataaccacaccacgcacggtcgggcgccagcccttccagcgcatgcggccggccttaccccagcggatgttgatctggtcggcgttaccgacctcaccaacggttgcgcggcagcggatgtccacgcggcggatctcggaggacggcatacgcagcactgcgtaggagccttccttacccagaagctggatggacgtacctgcggaacgggcgagcttggcgcctgcgcccggcttcagctccacgcagtggatggtggtacccgtcgggatgttgcgcagcggcaggttgttgccaaccttgatgtcggcgttcggaccggactcgatcacggtgccctgggtcagacccttcggcgcaatgatgtagcgcttctcaccgtcgtagtagtgcagcagcgcaatgttggcggtgcggttcgggtcgtactcgatgtgagcgacctttgccagcacgccgtccttgtcggaacggcggaagtcgatcacgcggtagcgacgcttgtggccgccgccgcggtggcgggtggtgatgtggccgtgagagttgcggccacccttcttcgggagcgggcgcagcagggacttctccggagtcgagcgagtgatttcctcgaactcggaaacagagctgttgcggcgacccggggttgtcggcttgtacttgcgaatagccatagtgtgtccttttctatcggtatcttcgtgatacgagagccacggtcttagaccgttgcgccgccgaagatgtcgatggagtcgctgccctcgcggagagtgacgtaggcgcgcttggtgtccttgcgcttaccgaaaccggtgcgggagcgcttgcgcttgccctcgcggttcgcggtgttcaccgaagcaacgtcgacgccaaagatctcttccacggcaatcttgatctgggtcttgttcgcagacgggttcacgaaaaacgtgtacgtgttctgctccatcagcgcgtaggtcttctcagagagaaccggggcgatgatgatgtcgcgagcgttggcgatcttagccatttacttctcctcctccgtagcgccggctgcagctgcgagctcgttgccgcggttgatgaaggtgtgcagtgcctcgaccgtaaacacgacgtcgtcagcgttgagcacgtcgtaggtgttcagcatgttcggagagatgatgtggacgcccggcagattccgtgcggaaagacgggagttgacatcctcgctgccggtaaccagcagaacggacttacggtcggtcaggcgctcgatgaaggcgcgggcggactttgtcgacggggtctggcccgggacaaggtcctccacaacgtggatgcgaccgttgcgtgcgcggtcggtcagtgcgcctgcgagagctgccttgatcatcttcttgggggtgcgctgcgcgtaggaacgcggctgcggaccgtgaacggtgccaccgccggtgaagtgcggcgcgcggatcgaaccctggcgggcgcgaccggtgcccttctggcggaacggcttcttgccaccgccgcggacctggccgcgggtcttggtggcgtgggtgccctggcgggctgccgcgagctgcgcgataacaacctggtgcatcagcgcaatcgaagcctcgcggtcaaaaaactctgccggaagctcaacggtgccgttggtagctccctcagcggtgtggacgtcgagcgtcaagttcgtcatgcgtgagcaccgcccttcactgcggtcttgacggtaacaaggctgcccttcgggcccgggatagcgcccttgatcaggatcaggttgttgtcgccgtcgatgcgttggatcttcaagttctgggtagtaacgcggttaccgcccatgcggccagccatgcgcttgcccttgaacacgcggcccggggtagcgcaggcgccgatgccgccgacgcggcggtgcgatgcctggttaccgtgggcagcaccctggccggcgaagccgtggcgcttcatggcgccggcgtagcccttgcccttggtggtgccgacgacgtcgacgtaggtgtcgccgtcgaagatggtcgcgttgaactcctggccgacctcgtactcggaggtgtcgtccatacggatttcagccacgtagcggcgcgggttcacgccagcctttttgaagtggccagcctgcggcttcttcgccttacggggatcgatgtcgccgtaagcgatctggatggcggagtagccatcggtctctggggtacggatctgggtgaccacgcacggaccagcttggacgacggtaaccgggataactcggttgtcctcgtcgaagatctgggtcatgccgatcttcttgcccagaatccctttctggttgtcagacatttttgttctcctgcttactggatgttcacgtcaacgctggccggaaggtcgatgcgcataagcgcgtcgacggtcttcggcgtcggatcgagaatatcgatgaggcgcttgtgggtgcgcatctcgaagtgctcgcgagaatccttgtacttgtgcggagaacgaatgacggcgtacacgttcttttcagtgggcaacggcaccggtccaacgacgcgggcacccgtgcgggtgaccgtctcaacgatcttcttcgcggatgcgtcgatcgcttcgtggtcgtaggccttgagcctgatgcggatcttctgtcccgccacgcttacctcttcctcgcatccccacattcccgttacttgccttgagtaaagctcgtattcggaattggtggggttgtagcttgtagtttctctataacgttgtccgggctgggcccttggctcaacgccagtgtcgttcaatgactgccatgacactgccggaaagatggggcgaacggcgcaaaactgcgcgtacgtgccattgctttccccgtcccttaatagataaggaataggtgtcagactcggaagggtgcgtgacctttcgcgtactgccgctgtttatttgccatgtcccaccccggtgggtgtgtcatggtcgcttcaccatcgccggtgcgtgcgcacgggccatgtcaaagcaacctgcgtatttaaacacacggcacaaagtaaatgcaatttccgcttgccgacgccccgcgcaacaccaaacccatttccttaaaagcaggtaggcttgccatgtacgtatctccctttgaaaggacccatcatggcccagaacaccccggctaactccacctccaccgagactacggcggccgcgaacactgccgccgctaccccggccgcttccaccacttcggctgttgagccggagcaggttcgcccgcgcaacgagaacctggagaccgagcacggcaccacggttatcgacgacaacgttgtgggcaagatcgccggcatcgccgcccgcgaggtgtccggcgtgcacaacctcggcggcggtgcagcccgcatgtggggtgctgtccgcgagtccttcacgtcctccaccaacgtgcagcagggtgtcaacgtcgctgtccaggacggccatgtgaacgtcgctgtcgccatcatcgcagaatacggcgttgctattcacgagctggccaacgccatccgcgagaacatcaccgtcgccgtcacccgcatgaccggcctgatcgtcgaccgtgtcgacgtcaccgtccacgacgttcacctgccggagcaggagaccgccgcgccccaggaacagtacgacgagccggtgaactaccaggcagctaacccggctctgggccagtagttatggcacaggccaccgttacccgcgaaacggcccacgcagcgcgcgatgccgcgctaggcgtggacggtgtggcgggcctcgacgggggtcgcgtcggcgaagtcgctctcctgcttcccggagagcgcgttgagggtctgaagcacgcgcaacgcggcgacgcgggaaccggcatcgaggcgcacattgtcttcgacgtcagttccggcagggacatcgagtctgtcgccggtgacgtgcgaaacgcgattcttgccaacacggacttcacgttcgtcgacgtcgttgtcgccgacgctgttgacggcgcgtcctcgtccgactaaccggaagacacttcaaccggaaacactggtgttttaacatggatatctttgcgaacaagacggctctcggcgtgcttatcggcgttatcgtcgcgttcttcgtcaccttcggcggagccctcgggctgctgtggctgctgctcttctccgtcatcggcggcgttgtcggcgcccagctcgacgggcgcgttgatttggcccgcgctgtgagcacgacctccggcagaggccgaggctaatggacgagtcgttttaccacatcagcgaaaaggcggtggagcgcgtcgccgagctggcggcgctgaccgtacccggcgtgcaccacctcgacgcgcagctcgccggcatcgctgggcgcaagtacccgcgcgttaacgtgcgcttggacttggcctcctccattgctgcggtcgatgccgaaatcgcgacgacataccctgcgccggtcgcggcgatcaccgacgctgtgcgcgccacgatcatcgcccacatccgagccctgtgcggcctcgatgtgtcccgcgtcaaggtcaccgtcgcccatgtggaaagcgacccgcagcagggccgcgtcacatgggacgacgtggcgagccacaccgctgagccagaaccggacgcaatccgcgtgtccccgtcccgcgtcacctctcctgtgacgaaggagcgcgaagaactgacgccgatcgaggtcgcggcctcgtgggaggaaatgcgcgaagttaccgtcccggcgccgcccgaggtcgagcacgtcgaagtgcccgcggaaccagaggtggatcacgtggcaacccccgaaccgggctacgtacgaacctccggtttcgtcggccctgcccgcgaactcgaggagatttcggtgcccccagagcgcgaggttcgcgtcccactgccgacccgcccgcaggagctggcagcaattcacgtccactcgacggacgttcacggggtggacgtgccggaacctcgcccgctcgtgcccgcccgcgcgcggccgaggccggcgctcgcacctgtgtatgcgcaccagacgcgggtcgagccggtttccttgccgctgcgcaagcccctgaagcaggtgctggtagaccgcccgccgatggtggaggtgtcgattccgccagcgccgaagctgcgccacgtcgcccctcccccaccacagcaggtgctccggcctgttgcaccggcgccgcagcccctgaagcagatcacgatccgaccggtggagaagtactatgaccgcacccgttagagaacgcgcggcggaacagccccgccccctcggaccgcaccctggcggcgagccgcgagcgaacccagctgcccgatggatcaccgttgtggtcgggcttgcgttcctcgcgcttgcgggccttttggctcgggaactgtggtttgtataccaagacgagcctttcacctcgtgggtgcagcccgtgctcgacttcttagctaaccacgtggtcgacgctgtggctgtgaccgtgggaatcatcatctcgctgatcggcctgtggctcatcattgcctcgttcgtaccgcgcaagcgcacccacgtccgcgtcaattccaccgcatccgtctggatgcgcccggtcgacatcgcccggaaggccacgtctaccgcccgcgctgagacgggcggggaaacgatccgctctaaggcagaccggaagaagctgaccgttgacgtgcctgaagacggcacgggaacagcgcaggagcgcgtcgcagcagcactcaacggcgaattttaccgactgcagaccccaccggcggtcacggtgaagaccactgcaccggtgcagccgaaccaggccgctaacacccaggaggtggcacgatgaccaagggcctcgcattcttcgaccgtttcgtgacgtttctcatcggcctccttctactggttgctggcctactgcccgccgcgttgtattgggatatcccttacgtcagcgactggctcaaccagttcgaccgctccgcaattgcggcggtcaccgaccagagttggtacaactccgcgttgattatctccgcgctcctgctgttcctgctcggactctggttcatcctcgccaacgtgcgcagccgggcgttctccaaccgcgagatcaccccggctgacccggcgcacggagagactgtcatcaatgttcagcggctgagcgacgcagcttgcgctgccctttccagcgaggaagctatcgccaaggcagactgccgcgtggcgatggtcggccagcgcccgaccgcgacattcacggtcaccgcggaacccgagtaccagctcgaggaagcaattcaggcgatcgagcgagcaaacgaggacttccgtatcgccaaccacacgatggagatcgatgccgtgtggaagctgcatctggaccgcgtagcggcctagacctctagtagccagactgccgcaaccggccccagccggcgagttttaccgccgcccgctggggccacttccatttccccgcccggtaccaccgcaacagcgcgccacgggataatctcgagttcggtctcgcgccccgcggtcgtccacatacgaagccgctggcctagcacggcccggcttccatcctcgaagagaataagccacctagccgaacccacttctgtctgctcgagaaacgcagttcccggtgcacgcgcggcgtcaatcaccgtcatcaactcgacaacccccatccggtgctccgtcccctcctcgtcggtgatgacgaggggcctcccagggccagctgggcgcaggcccgagtacctccacagcccgggcatccggcgggggtcgtcgccgctgcgggcaatgaccgtgccgccggacagcgtgacggtcatacgcggtgacgacgtagcgatcaccgtcggagaggccggcgccgctgtgatgagggcggggtggcgggaggacacctcatcgagaagcatcaaaagctcctcttcagtcgagccccaggacaaccccttcgtctgcagcatgccgatgaatgccgggagcgagagatcgggctggccctcccaagcgtcttggagagcgcttatgagccgcgggatccgggtggggtctgatccttgcacgcagcaaagtgtactggaccccagaaacgcgaaaagccgcaccccgtggcgggatgcggctcttcttagctaactaactggtgctagccaagtctcgaattagtcgaggatcttggtaacacggccagcgccgacggtgcgggagccctcgcggatggcgaagcgcaggccctcgtccatagcgaccggctggatgagctcaacggacatctcaacgttgtcgcccggcataaccatctcggtgccctccggcagcttcacaacgccggtcacgtcggtggtgcggaagtagaactgcggacggtagttgtcgaagaacggggtgtggcggccgccctcgtccttggacaggacgtagacagaaccctcgaacttggtgtgcggggtgtaagcgcccggcttgataacgacctggccacgctcaacgtcctcgcgcttcagaccgcggagcagcagagctgcgttgtcgccggcctcagcggtgtcgaggagcttgttgaacatctcgatggaggtaacggtggtcttctgggacttctcgcggataccgatgatctcgacctcatcgttgaggttgaggacaccgcgctccacacgaccggtaaccacggtaccgcggccggaaatggtgaagatgtcctcgatcggcatcaggaagtcgcggtcggtctcgcggaccgggtccggaatggaatcgtcgcaagcctgcatgagctcaacgatagagtcgacccacttctgctcgccctcgagagccttcagagcggaaatgtgaacgatcggagcttcctcgtcgtagtcctgctcagccagaagctcgcggacctccatctcgacgagctcgatgatctcctcgtcgtcaaccatgtcgcacttgttcagcgcaacgaggatgtacggaacgcccacctggcgagcgagcagcacgtgctcgcgggtctgcggcatcgggccgtcggtagcagcgaccacgaggatcgcgccgtccatctgagcagcgccggtgatcatgttcttgatgtagtcggcgtggcccggggcgtcaacgtgtgcgtagtggcgcttcggggtgttgtactccacgtgggagatgttgatggtaatgccgcgctcgcgctcctccggagccttgtcgatggcggcgtagtcgaacgccttgttctcctccgggtactggttagccagcacggtggtgatggcagccgtggtggtggtcttgccgtggtcgacgtgaccgatggtgccaatgttgacgtgcggcttcgtacgctcgaactttgcctttgccacttgttgtcctcctggacttcatggtggctacgaccttcgcagccacgtggtttacatttgccttgctccacggcccactcgcgcaggacgccaagcaacgaccatttcacaatgtgccagttacatgatcctagattctgaatgaccgttttacaaaccggccgatccgtatcaaacccggacctacctagtgggtaacggccggctcaaaccccggcgatctgcttcgatcgcagggtctcagcgagccgctacccaccaggtgatgcactcctccccctcgttcgacccgccgccctggctagcggcgacgggccgtcaggaaaggatgcgggaggcgctgcccggcttagttgccgttgcgctcgtcgatgatctcctgtgcgacgctctgcggaacctcagcgtaggagtcgaacaccatggagaagttcgcgcggccagcggtggacgaacgcaggtcgccgatgtagccgaacatctcggacagcggcaccttcgcgcgcacaaccttggcgcccgagcggtcctccatcgcgtacacctggccacggcgggagctgatgtcgccgttgacggtacccatgtactcctcaggggtgacaacctcgacggccatgaccggctcgagcagaaccggcttcgccttcgccacagcttccttcagaacctgggagccagcgagcttgaaggccatttcagaggagtcgacgtcgtggtacgcgccgtcctcgagggtcgccttaatgttcaccagcgggaagccggccaggaagccgtactgcatcgcgtcctggatacccgcgtcaaccgacgggatgtactccttcggcacgcggccaccggtgacggcgttctcgaacttgtaggttgcggactcgccctcctccagctccgacggctccgggttgtacggctcgatggtgacgatgaccttcgcgaactggccggaaccaccggtctgcttcttgtgggtgtagtcgaggctctcgaccttcttgcgaatggtctcgcggtacgcaacctgcggggaaccgatgttcgcctcaaccttgaactcacgcttcatgcggtccacgagcacgtcgaggtgcagctcgcccatgccgccgataacggtctggccggtctcctcgtcgagcttgacggtgaaggtcgggtcctcttcggcgagcttctggatagcggtgcccagcttctcctggtcagccttggtcttcggctcgatggccacctggataaccgggtccgggaagtccatggactcgaggatgatcgggtgatccgggttgcacagggtgtcacccgtggtggtctccttcaaaccgatgaacgcgtagatgttgccggcgtcagcgtgctcaaccgggttctccttgttcgcgtgcatctggaagagcttgcccacgcgctctttcttgctcttggtggagttgagcatctgctcgcccgggatagcctggccggagtagacgcgcacgtaggtgagcttgccgaagaacgggtgcacagcgatcttgaacgccagtgcggagaacggctcctcaacagacggcttgcgggtgagctcctcgctgccgtccacagaggtgccgtgcacctcgccgatgtccagcgggctcggcaggtagtcaacgacagcgttcaggatcggctcgatgcccttgttgcggtacgcggtgccgcagaagaccgggtagacctcggagttaaccgtcatcttgcggatggcagccttgatctcctcgacggtgagctcctcgccgccgaagtacttctccatgagctcctcatcggactcggcgacggtctcgagcagcttctcgcggtactcctcagcctgctcctgaagctcagccgggatctcctggatctgcggcggggtaccggtctcaaccttgcccggccacaggtacgccttcatctcgacgaggtcgacgacgccgtcgaagttgtcctctgcgccaatcgggatctgcataaccaacggcttcgcgccgagacggtcgacgatggtgccgacggtgtagaagaagtccgcgccgagcttatccatcttgttgacgaagcagatacgcggaacgtcgtacttcgcagcctgacgccacacctgctcggactgcggctcaacgccttccttaccgtcaaagacggcgacagcgccatcgagcacgcggagggagcgctccacctcaacggtgaagtccacgtggcccggggtgtcgatgatgttgatctggttgttgttccagaagcaggtcaccgcggcggacgtaatggtgatgccgcgctccttttcctgctccatccagtcggtggttgcgccaccgtcgtgggtctcgccaaccttgcggttgatacccgtgtagaacaggatgcgctcggtggtggtcgtcttaccagcatcgatgtgggccatgatgccgatgttgcgaaccttgttcaggtccttaagcacttcttgtgccacgtttattaccccaacttgttagttgtcgacaccgccgcgccgcgatacttctgcgacgccgaagcgtctatagcggatattttccttgttcgattattccattacttcgcgaaagtagcactgggagacccccgcttacgcgccacatagcaacgacccggtgacaatcatcgatatttcgaccacggcataagccgcgggctgattgtccaccgggtcggtgcgcattgacgcaattgcgaaaatggctctactactaccagcggtagtgcgcgaaggcgcggttggcctccgccatcttgtgggtgtcctcgcggcgcttcaccgatgcgccgagaccgttggacgcatccagaatctcgttggcgagacgctcggtcatggagttctcgcgacgctggcgggtgaaggtgaccatccagcgcagagccagcgtgttggagcggcccggctcaactttgaccggaacctggtaggtggcgccaccgacgcggcgggagcggacctcgagatccgggcggatgttgcccagagccttctccagggtgccgaccgggtcagtaccggtcttctcgcggcacatctcgagtgcgccgtagacgatgcgctctgccgtggacttcttgccgtcgatgaggaccttgttcaccagctgggtgaccagctcggagttgtaaaccggatccttgactacgggacgctcaggtgctttttgcttacgcattgtttacttatcccttcttcgcgccgtaacgggagcgagcctgcttgcggtccttgacaccctgggtatccagtgcgccgcggatgatcttgtaacgcacacccggcaggtccttcacacgaccaccgcgcacgagcaccatggagtgctcctgcaggttgtggccctcgcccgggatgtaagcggaaacctcaacaccggaggtcaggcgcacacgggcgaccttacgcagcgcggagttcggcttcttcggggtggtggtgtacacacgggtgcacacgccgcggcgctgcggggagcccttgagggcggccgtagcaacctcggtcttcttgtccttgcggcccttgcggaccagctgctgaatagtaggcattcacgctctttcgtggttacgcgaccgcccaagcttggctatacatgcaaaaataggggctcttttccggggccctgccgttttgcatgaactaccgtgtgagcgggtcgcatggagttcaataacttccactccgcgggtattcgcgggggaaacctcgataaaggtacaccacgtggcgcaaagagcacaagttgcttatcgacgcccaccccagcccaactggcctgcggcgccggcctcgacaacctgctccttcgaccaggtccacggcaggtagttgtccaccagggattgggaggacgccgcgaacatcaccgccaccgctatgggggccgtcgcccaccaggtccatctcataggtcgatcccttgtggcaccggggagtttgtccagcggtatttcaaagaccatcgtgcactcggtgcggacgcctgggtaggtcacctcgcacgcacgaagcccaggatcgactgaatcgaacagggtgccgtcttccgcctggattcgcccgcggagcaccgtggtggcctccggggtgaatccgaaattcatctgcactcagctcgcgtgcgagggcacaccgttgagcttttcggacacagtcacgcgagcgctgtcgaatgtgcccagtttcggggcagcgctgccgtattcgtacggcgcgtacaccaggtcctcggccttcggcagctggccgcggatgaacactcccaagctgatgagggcgagggaggctgcgacagcggcaacgcggcggcttggagcgctcatttgagggtcacctccgcagtgcgttcgccgagaagccagcgcatctccggcacctcggcgaacatgtaaccttccggctcggcctcctcgaatccgccgcttatacccgtcacaccgacgagggcgagcagcgccgcaatagtcgcgcttgggcgactttccgctcacgcctggatattaagcctgagcacggcgtctgtgcgcgggctccggttaatctgggctcatgaccacaccgaatgctccccgcaagcgggccagcaacaccgagcgtgagcgcatttcgcaattgcttgacgacgcccacgtcgacggccagctcagcctcaccgaattcgacgaccgcaccaaggcactgtgggccgccacctacgccgacgaactgcctgcgttagttgcggacctcacccccgtggaacacggcagcgggaccctcgagcccatcagctcccagcccggcggctccgccctctccttttccatcatgggcgagtccgtgaagaagggacgttggcacgtcgccccgacacacacctccatcacagtcatgggaggcaacgacctcgacctcaggaacgcgacactgtccgcacacgaaacggtgattaacgcgtttgcggtgatgggcggcatcgacatcatcgtccccgacgacgtccgggtgatcgacgacggcatcggtgtcttgggcggctttgagcgtcgcgacgacccctcgtccagcacctctcacgatcacctgcccagcgacgcgccggtggttcgagtccgcggcctggcgcttatgggcggcgtcgacatcatccgcgcggcacgcgacgcccacatcagctagcgctgaaccgctagtgctgagccggggcagcccgtcggatgagtgcgcggatgtggttggaggtgtcgtcgtcaagcgaaagcactgcgtagctcgtgggccacatggagccgtcgtcgagctgcgcggcggcgagcgcgcggtcctcctccggcatcgcgtcgatcaactcttgtgggaaacacgtcgccccgccgtctccgttttgccaacgcccttaggtccgtctaacgccaccgcggccacatggggaaggagctcgtcgagttcggcgtcgacggtgcggtctaaataggtcatgagctgcatcgtaacaccactaatcgaccatttgcagacgtcctactcgtccatttgcaggcgtcctactcgtccatttgcagacgccgtaccaagttggggccggggtccgtcgaaaagcaaaaagcccggccccgaaaccgggaccgggccagcagacctagctagatgccagaagtgctaggccgccttagatctggtcgaaaccgtactcgtccagcgggacggaggcgccggtgaactcgccgtagccttcgtcgccgtagatggagtcgccgaagctcggaatcgagtacgccgcagagcgggccgcctcggtcggcttgacctgaatgttgcggtagcgggagatgccggtaccagccgggatcaacttaccgatgatcacgttctccttcaggccgatcagcttgtcggagcgcttgttgatcgcggcatcggtcagcacgcgggtggtctcctggaaggaggccgccgacagccaggactcggttgccagggaggccttggtgatacccatgatctcggagcgcatctccgccggctcgccgccgtcggcaaccgctgccgcgttgacctggcgtgcctcggagaggtccaccagagtacccggcaggaactcggtggtacccgagtcgatgacggtgccgcggcgcagcatctggcggatgatgatctcgatgtgcttgtcgtgaatcgacacaccctgggtgcggtacacggcctgcacctcgttgatcaggtgcttctccacaccgcggcggccgagcacctcgagcacgtcgtgcgggtcggcggcgccgcgcataaggcgctcgccaacctcaacgtggtcgccctcgcgcagggtgcgctcgatgtaggcgtccgggttggactccatcgggcggcgcacctgggccaggccctggcgcttcgacagcttctcgtagaccacgtcgtccgagtcgtcgtccgggtggatcgtcagcgtccagaagttgccctcgtcctccagtgtgaccgtgccggccacggaggcgatcggggcgcggttcttcggcacgcgggcctcgaacagctcctggacacgcggcagaccaccggtaatgtcgccgccgacaccaccctggtggaaggtacgcatggtcagctgggtacccggctcaccaatggactgcgccgcgacgatgccgacagcctcgccgatgtccaccagctggccagacgccatggacttgccgtagcacttcgcgcacacgccggtcggggtctggcaggtcagcacggagcggacctttgcctcggtaacgccggccgcgacgagcgcgtcgatgcgctcctcggacagttcggtgccggcctcgagaatgacgttgccgtctgcgtccttcgcgtccgccgcgagcacgcggccggacacggaggtctcgaccaggtcgtggcggtggaaggagccagcggtctcctcggccaccggcaccttgacaccctggtgggtgccgcagtcgtcctcgcggacgatgacgtcctgcgccacgtcgaccagacgacgcgtcaggtaaccggagtctgcggtacgaagcgcggtatcggccaggcccttacgggaaccgtgggagttgttgaagtactccatcacgctcagaccctcacggaaggaggtcttgatcgggcgggtaatgtactcgccgcgcgagttcacaaccatgcccttcataccggccagggtccagatctggcgcatgttaccggcagcaccggacttcacgatcatcggaatcgggttgtcgtccgggtagagatcctccacagcctgacccaccttgttggtggcgtcctgccacagctcgaccaggcggtcgtagcggttctcctccgtcagcgcgcccttctcccagaacttgcgctcgatctcctcggcctcgcgctcgtactcctcgagcacctctaccttgttcggaagcaccagcacgtctgacatggagatggtcacgccggagcgggtcgcccagtagaaaccggcgtccttcatcttgtccagcacctgggcaacggtgatcatcgggtacttctcaaccatggactggatgatgtcgccgagcagcaccttgccggaaccgccgcccttgcgcaccatcgcgccttcctggtacgggaagttgaacggcagaagctcgttgaacatgatgcggccgagcgtggtgtccatcatccaggcctggcccttggtccagccctccgggaactgctcctgctcgatctccggggtcgggcgcaggtggtcgatgcgcaccttgatcggagcctgcaggccgagcacgccgcggtcgtaggccatgatggcctcgcggtaggaggagtaaacgccctgctccggaccgttctcgtcggccggggcgtacgcgccctcgccgccgatctcctgcgggcccttcaccatggtgaggaagtacaggccggtgaccatgtccaggcgcggcattgccagcggcttgcccgacgccggagacagaatgttgttcgaggacagcatgaggatgcgggcctcggcctgcgcctctgcagacagcggcaggtgaactgccatctggtcgccgtcgaagtcggcgttgaaggcctcgcaggccagcgggtgcagctggatagccttaccctcgaccaacttcggctcgaacgcctggatgccgaggcggtgcagcgtcggtgcgcggttgagcagcaccgggtgctccgcaatcgcctcttcgagcacgtcccacacctcagggtgctggcgctccaccttacgcttcgcgctcttgatgttctgcgcgtagtcgttgtcaaccaagcgcttcatcacgaacggcttgaacagctcgagcgccatcagcttcggcagaccgcactcgtgcagcttgagctgcggaccgacaataatcacggaacggccagagtaatccacgcgcttacccagcaggttctggcggaagcggccctgcttgcccttgagcaggtcggacagggacttcagcgggcggctgcccgggccggtgaccggacggcctcggcggccgttgtcgaacagcgcgtccacagactcctgcagcatgcgcttctcgttgttcacgatgatctcgggcgcgccgaggtcgatcatgcgcttcaggcggttgttgcggttgatcacgcggcggtacaggtcgttcaggtccgacgtggcgaagcggccgccgtcgagctgcaccatcgggcgcagctccggcgggatcaccgggatcgcgtcgaggatcatgccggccgggtcgttgccggagcgctggaacgcagcgacaaccttcaggcgcttcagggcgcggatcttcttctggcccttgccctcggcgatgatgccgcgcagctcctcggcctcagcgtcgagatcgaagttgcggatcagggtctggatagcctcggcgcccatgccgccggtgaagtagtcctcgtagcggtcgacgagctcctcgtacaggttctcgtcgataaccatctgcttcggggcgagcttggtgaaggtggtccagatttcgtccagacgctccacctcgcgctcgccggcctcgcggatgtgagtcatctccttgtccgcggcgttctgcaccttcttgcgggcagcagcggtcgcgccggcggcctcgagctcagcgaggtcctcctccagcttctgcgcgcgctccgcgatctccgcgttggcgtccgcctcaacttccttcttctccatgagcatctctgcttccagggtggagaggtcgttgtggcgggcctcatcatccacggaggtgatgatgttggctgcgaagtagataatgcgctcgaggtccttcggcgccaagtcaagcaggtaacccaagcgcgacggcacgcccttgaagtaccagatgtgggtaaccggagcggccagctcaatgtggcccatgcgctcgcggcgcaccttggacttggtcacctcgacgccgcagcgctcgcagatgatgcccttgtaacgcacgcgcttgtacttgccgcaggcgcactcccagtcgcgggtcgggccgaaaatgcgctcgcagaacaggccgtccttctccggcttcaaggtgcggtagttaatggtctccggcttcttaacctcgccgtgggaccagcgacggatgtcgtcggcggtggccaggccgatgcgaagctcgtcgaagaggtttacgtcaaacacgtaatggttccttatcttcttggtggttgctgttcgttcacgggtgcgtcggcaagcagctgcttatcgacgcccccttgtcctagccctatgccgtatccgcagccgcgccctcgtcgcgggacaggttaatgcccagcgaggaaccggcctggtcgaactcgtcatcgtcgccgtcgagctccatcggcgtgccgtcggtggagagcacctccacgttcaggcacagcgactgcagctccttgagcaacaccttgaacgactccgggatgcccggatccgggatgttgtcgcccttcacaatggcctcgtacaccttcacgcggccgaccacgtcgtccgacttaatggtgagcagctcctgcagggtgtaggcggcgccgtacgcctgcattgcccacacctccatctcgccgaaacgctggccgccgaactgggccttaccgcccagcggctgctgcgtaatcatggagtacgggccagtggagcgggcgtggatcttctcgtccaccaggtggtgcagcttcagcatgtacatgtaaccgaccgagatcgggtacttgtacggctcgccggagcggccgtcgaacagcatcgtcttgccgttctcgtccaccatcacttcgccgtcgcggttcggcttggtgttagccaaaaggcccgcgatctcgtcgttggtcgcgccgtcgaacaccggggtggccgtcagcgagtcagccggcacgtcgtagaggtgctccggcagggtctcgagcagcttggcgttcttcgggtcgtccgggttcacggtccagccagccttggccagccagcccaggtgcacctcgaggacctggccgatgttcatacggcgcggcacaccgtgggtgttcagaatgatgtccaccggggtgccgtccgccatgaacggcatgtcctcctgcgggagaatcttgcccacaacacccttgttgccgtggcggccggccatcttgtcgccgtcctggatcttgcgcttctgcgcgacgtaaacgcggatcatctcgttgacgcccgggctcaaatcgtcgtcgtcctcgcgggagaagcggcgcaccgcgatgaccttgccggtctcaccgtgcggcaccttcagggaggtgtcgcgcacctcgcgggccttctcgccgaagatggcgcgcagcaggcgctcctccggggtcagctcggtctcgcccttcggggtgaccttgcccacgaggatgtcgccgtcgcgcacgtccgcgccgatgcggatgatgccgcgctcgtcgaggtccttgagcacctcctcagagacgttcggaatctcgcgggtgatctcctcggcgcccagcttggtgtcgcgggcgtcgatctcgtgctcctcgatgtgcacggaggtgaggatatcctcctccaccacgcgctggttgaggatgatcgcgtcctcgtagttgtggccttcccacggcatgaacgcaacgagcaggttgcggccgagcgccatctcgccgttcttcgtgcccggaccgtcagcgataacctggccggcctcaacacgctcgccctggctcacgatcggggtctggttgtagcaggtgccctggttcgtgcgctcgaaggtgcgcagcatgtaggtctcgtgcgtgccgtcgtcggcggcaacggtgatgaagtcgccggtgacgttctcgatcacgccgcccttgctggtaatcacggtgtcgcccgcgtcgtacgcggcgcgctgctccataccggtggcgacgtaggcggcctcagcacgcagcagcggcacagcctgcttctgcatgttcgcgcccatgagcgcgcggttcgcgtcgtcgtgctcgaggaacggaatcatcgccgttgccacggacaccatctggcgcggggaaatgtcgaggtagtcgacgcccttggggccgacaacaccgatgtcgccgtccttcaggcggacctcgatgcgctcgccggtgaggttgttgtccttgtccatcggcgtcgccgcctgcgcgatggcgtaacggtcttcttcgtccgcggtgaggtagtcgatctggtcggtaagctgaccgtcgacgaccttctggtacggagtctcgatgaagccgaacgggttgacgcgggcgtaggaggccagcgcgccaatcagaccaatgttcgggccctcaggggtctcgatcgggcacatgcggccgtagtgcgacgggtgcacgtcgcgaacctcgataccggcgcgctcacgggacagaccacccgggccgagcgcggagaggcggcgcttgtgggtcaggccagacagggagttgttctggtccataaactgggacagctgcgaggtgccgaagaactcgcggatcgccgcggaaaccgggcgcacgttgatcagtgacgtcggggtgatcgactccgcgtcctgggtggtcatgcgctcgcgcacaacgcgctccatgcgggaaaggcccacgcggacctggttctggaccagctcgccgacggtgcgcaggcggcggttgccgaagtggtcgatgtcgtccgtgttaatcgggatcatctcgccgttcggcgccttcatctcgttctcgcctgcgtgcaggcggacgaggtactcgagcgtggtggcgatgtcttcctcggtgagcgtcatcagaccctcgtggtcgccgccgaggcccagcttgcggttgaccttgtagcggccgacgcgcgcgaggtcgtagcgcttcggcttgaagaaggcgttctccagcaaggactgcgcgaggtcgcgcgtcggctgctcgcccgggcgctgcttgcggtagatctccagcagcgcctcgtcggtgttggcgacaccgtcggattccagggtggccatcatgatctcggagaagccgaagcgctccgtgatctgctcggtggtccagccgagcgccttcaacagcaccgtcaccggctggcggcgcttgcggtcgatgcgcacgccgacggtgtcgcgcttgtccacgtcgaactccagccacgcaccgcgcgacgggatgaccttcaccgagtgcagcggacgctcggtggacttgtcaatcgtctcgtcgaagtagacgcccggggaacgcaccagctgggagacgacgacacgctcggtgccgttgacgatgaacgtgcccttgtccgtcatcagcgggaagtctccgatgaagacggtctgggacttgatctcctgcgtgtcgttgttgatgaactccgccgtcacgtacagcggtgcggagtagttgatgtccttgtccttcgcctcttcgatcgtgtacttcacgtcttcgaagcgcggctccgacaggctcaggctcatgttgcccgagtagtcctggatcggggagatctcctcgagaatgtcctcgaggccgctggtcaccttcgcggtctcgccgcggagttcctgctcgcgttcgcgccactccggcgtgccgacgagccacgcgaaggaatcaagctgcacatcgagaaggcccgggacggtgatgggctctgcaattttcgcgaacgagtagcgttcgggtgccccggggatttcagccatattcatggtctggtctgagactgccaagttgggtccttccagcaccttgggcggaggccgcagcaatctgctctggcatacaggttggcgacgtttccgctggttaagttagcatttggtctgcttcggaagacccgccccagagatagcaaaatcaccttgtcaaatcggttttcccaaaccgctcgagcaaggtttgcgcgcacactggagacggcttccagcgcaaagagacagcctatactacacaggcgcgcttgtaaagcactcagccggcagcctaccaccactaccggcgcgcgcgggaaaaccgcaccgcaagaaatgcgccgagggcggtcagcagcgcaccgagggcggcgacgatgcgcgcgatcgtatgtgcgcgcgacgcgggcgcgacacccgaaacggcctggacgagctcggtgacctgcgccgtgtccatctccgcgtcgtacatcacaatgttctcgatgccgcggccggctgcgtcgccgtaaaagtcgtcgaccttctcgttgatgccgaccacgaggccggaaatgcggtccacgagcagctcgcgctcggcggagtggaagtagaaggcgcgctgcggctcgccctccgggcctgggaggtaggtggtgtttcgcgcgtcggcgtagagctgggcgacgttcaccggcgcgatgacctggcggaagcggtacacggtgcggcccgcgatctcctcctcgcccacgaattccgccggtgccgaggtgcgaagggtggggtcgaacacgtcgtaggcgcgctgttctacgtttgcggggaaggtgagccacggggcgtcgataagcacctgctccgcgggcatacccataacaagctgcacctccgccgggtcgcgcacctcggcggtctcgcggtcgagggcgaacgaccaggtggatgcggtgatcaagttatcgaagtcggtgccggccttgcctgcgcgcagcgtgtcgccgacgcgcacggcggcggtgtcctcgtcggaggggttgcggatttccatgtgcagctggcgcgtgaccggcgcgggctggccctgacgtttgccgttgtcgtccgtcagggtccaggtggcctcgccgagggagaggggcaggcgtgcgttggccagaagcaacctcggagcaacgagcccgccgaccagcagcgcaacgccgaggccgacgagcagtgcctgaaaagcgcgggaacggtgcatggtgcgctaccttaccgcaggatatcgcggccccacttcagcgcggcggccaaggagtcggcgaaaacgtcccgaggcaggtcgttggccatcaggttcatgcggcgggtgcgcgtgacgttgcgcggctctgtgtacttcgtcatgccgtgctccccgtgccggcggcccgcgccagactgcttgaacccgcccatcggcgcgtccatcgcgctccacgctggcgcgtacccctcgttgatgttcaccgttccgctctcaagctgggatgctaatcgacgccccgtcatcctccccgcccacaccgacgcgttgagcccgtactccgagtcgttcgccttcgtcaccgcctcgtcgagggagtcgacgacctcgatgtagaccaccggcccgaagacctcctcggtgtagaggtcagcgtcggtgggcacgttcgtgagcaccgtcggctcgaagaacgccgggccgatgcggtggccaccggtcagcgctgtggcacccttggcaagcgcgtcgctaacaaacgcctcgatcttgtcggtgtgcgcctccgagatctgcgcacccatgtcgatgtcccaatccttgcccgcccccaccgtcatctgatccacgcggtcgacgaaccgcgggatgaactcgccggctatgtccctgtgcacgtacatccgctcgatggagatgcacagctggcccgagttggcgaagcaggcaagccacgcgccctcgaccgcgcgatcgagcggcgcgtccggggcgatgatcatggggttcttcccgccgagctccatcgagtagtcgatcagccgctctgccgcctgttgggccagctcttttccggtcttggtcgagccggtgaacatgaggaagtcgcagcgcttaatgatcgcctgccccacctcgctccccggcccggtgaccacctggaacaggtccctcggcaggcccgctttgtagaggagctcggcacccttcaacgcggacaacggagtctgcgagtccggcttgagcaccaccgcgttgccggcgagcagggccgggatcgcgtcgctgatcgcgagcgcaagcgggtagttgaacggcgcaatgatccccaccacgcccttcggcgggcgctgctcgtgcgtcacggttaagaagggcattggcacttgccgacgcctcgttctcacatacccgcgcccatgatgtgcgtaataccgactggtcaacgctacatccatcacttcctcgagcgcactcaggcggttcttgccgttctcgtcttggatctggtccatcaactcatcccggttgtcgatgaccaggttgtggaaccgcaacatgatcctcttgcggtggcgatagctcgtctgcgcccacgcctcctgcgcgcgccgcgctttggtgaacgcccgctcgacgtcgtcttcggtctgtttcgggacccggccgatcacctcgccggtggcggggttggtgacgtcgatgtgctgcgttcgtttcatgccgcccagcctaggcggtgcgtgggcggcgccgcggtggcgctttggtggcgctcgggcggcgccgtggcggtgatagcgggtaactcggtcagcggtggaacgcgacctgcggaaatgcagattgcggctggagttacccgctatcaccgagagccggccgcagccaaggacaacgaacctgtggataactcgcgccgcccgagcccgagttatccacagttccagcaaccgccgttcccctctgtcgtttcatctgccatcatcccgggtatggatcgggggaaacaggacgaacttgtcggaatgctgttgaagctgcggcgcgatggcacggctgtcgacggctcgggggccgcggggtccggcaccgtggtgctcggcctatccacgaaatacggtgtcgcctaccacgacttcgctggcctgcgctcgtacgagcggaagtggctgtgctgcctcgccgtcgcgaagtcaatgcggaaagcggcgttggcgggcagatccgccgcccggatccacggcatgtgggtgatcggggaccaaactggggctgcggaaagggtggagttggtgttgggggcggggagggtgccgtcgaaaagccaatggcccaaggggtgtacctatctcgagcagcgcggaaggaaaccgacgatcgtggagcatgcgacggtgcgcgtgacggatccgctgtcgaccgcgttcgatattgcgctgcaccacgggttccgcgaggggctggtcgccatggattggatcttgcaccaccacacgacgcgtgaggtcgtcgaggcggaactggagagattcgggccgacgcgcaacatcgacacgctgcggaaggttgtccagcacgccatcccgaactcgatgtcgccgtacgagtcgtacgccagggcattgcttatcgacgccaacatggacggttgggtcgccaacgccaaggtcggcgagttcttcatcgacctgctgcgccgccgcctcggcatcgaaatcgatggcggcgtgaagtacgacggcgagacctacaaaccgctggatgaaacgctgcttgctgagcggaacagggagaagaagatccagaacaagggcattatcctctatcgcgtttccccggaggtactgctgcgtcgcgaggaggagttcctcgccgaggtggagcgcctgcaggtgattgccgacgcgatggggccgctcccgccggatatctagcgtcgtaggcgcggcccctggctcccccgccgcgagttgatagcgggtaactcggtcagcggcggaacgcgacctgcggaaatgcagatcgcggccggagttacccgctatcaccgcacactgggcactacccccggcaacgcaaaaccccggcaacgcaaaaccccggccccgcaccgtatctaggtgcaggaaccggggtgagtggtcgcggggtgatatcacccctaggcgactacttgagggtgacggtagcgccagcctcttccagcttggtcttggcagcctctgcgtcgtccttgtttgcgccctcgaggatggccttcggagcaccctcgaccatttccttggcgtccttcaggccgaggcccggaaccagctcgcggacaaccttgatcacgccgatcttcttgtcgccagcggactcgagcacgacgtcgaactcgtccttctcctcagcagccggagcgtcgccgcccgcagcacccggagcagctgcaactgcaaccggagcagcagcggtcacgtcgaagacctcctcgaattccttcaggaactcggagagctcgatgagggtcatttccttgaactgctcaatgagctcgtccttggtgagcttagccattgtggcttcctttctttgacctcgtgtgaggtcgtttcatggggtgtgtagttgttggtggacgtttgcggtttacgccgcgtcgtcctgcttgtcctgcagtgcggcaacaagtcgtgccgtcttgg

SEQ ID NO: 6 - DNA, 223168 bp, Corynebacterium cassirii
  source 1..223168: mol_type = genomic DNA
gccaggatcaaactctccacaaaaacatttcagtaaaagaaaccgagccgtgaaaagcccaaacccaaccaaaacaaaaccacccaacaaaaaacgttggactggcaatcctttgaaaaaacgttggtcatgtatccgacgaggaaaaaccacaaccaacaaaaaatagtgaaaccatcacacgtcccaccgtccaacagcaccacccaaagaaaaagcagcactgccaccggcacacaccacaacaaaaatcatggcgcacacgcacaacaatcacaccaaacaaaaaagtattggcacactatcgagttctcaaacaacacacgcacacctgacagctgcgatttcgcttctgtcaaaagcggcttgaaaaacattaccgagagtaacgaatcatgtcaactcgttgactttctgcagttgttccgactgccgaagcagtgggctaaacattagccacacgcttcgaatgaatgcaaactgcgctgctcaaacggcatttctgagatatcggtaccgactcacacgcgttttacgcccgcgaagttcttcttgccgcggcgcagaacgagccacgtgccgtgaaggaaaccctcgtcgctaggcacccagtcctcggattccacgcgctggttgttcacgtacacaccgccctccctgatcgaacggcgggcagcgcccttcgagtcggcgaggccagcaccaacgaccaggtcgacgatctgtggcacgtcgcctgcagacacttcgaacacctcggtctcggacacggcggacgcaagggtcttctcgtctagctcggccaggtccgctttgccaaacagcgcctccgcagccagctcagctgccttgcgggcatcttctccgtgaaccaaatccgtcatctcctgcgcaagacggcgctgggcttcacgcttgaagggtcgctcttcaacttcctgcgctaggcggtcgagctcctcctgatccaggaacgtaaaccagcggaggtagcggaccacgtcggcgtcagcggtgttcaaaaagtactggtaccacgtgtacgggctggtcatttccgggtccagccaaagagagccgccaccggtggatttgccaaacttcttgccttcggaatcggtcacgagcggcacggtcagcgcatgcacggaagcgccgtccatgcggcggttaaggtcgacacctgccacgaggttgccccactggtcgccgccgccaatttgcagcacgcagtcgtactcgcggtggagctgcacgaagtcgttcgcctgcaggagcatgtaggagaactcggtgtacgagattccgtcggactccaaccggcgcttgaccgtctcgcgaccgagcattgtcgaaatggaaaagtgcttgcccaggtcgcgcaggaactcgatcacgccgagcttgctggtccagtccgcgttgttcaccagaagtgcggcgttgtccccctcgaaggagacgaagcgggacaactgcccggagattcggtcggcccagtccgcaacggtgtcggcggagttgagggttcgttcgccgacgtctcgcgggtcgccgatcatgccggtggcgccgccggcgagcacgatcgggcggtggccagccatctggaagcggcgcagcatcagcagcggcaccaagtggccagcgtgcagcgacggtccggtcgggtcgaagccgcagtacaaggtgatgggcgattgcgcggcgccgcggagcgcgtctaagtcggttgactggttgatcaggccgcgccaagcgatttcgtcgacgatgttctggggggaagacatgaaaaaagaacgctccttcttacgcgtggtgggcggggtggggctgcgcttcgtcgataagcagcaccggaatgcccccatctatccggtacgcgacaccgagccgctcgttgatcaacagctgctcatcttcgctatatcgcagcggacctttgtcctgcgggcagaccagaatgtcgagcaaacgcggatcgagactcatagggctaatcgtacctgcccgcgatctcctcgccgccgtcgaggccgggcagggcgccgagttggttgcggaggaatttcgcctgcgaatccatcgcacgcaagttgtcgtccacaatgccctgcttgatccggccgacggcgctggtgagggtggaaagcgaatcggtcaccactgccacggcgcgcgggtcctggcgctgcggggctgcaaggtaggtctgtgtgacctccgggtagtacaccttcaccacgtcccacatcgtctgacggtgctcgggcgtgggtgtgagatggtcccactcccccagcacgaagcggacgttgctttccagctcctgcgcctggcggaccacggcggccggtgcggcggcctgccgcagctgggctgcggtccggttcagcgcgtcgtcgagaagtgtgggcgtcggcgtcgtggcggacggaagcgctcgctgcttcggcggcggggtgagcacggccccggcaccgtacgcggcgatggccgcgaccggccagagcggcccgaaattgaacgcgatgtggaggaccaccactaggatggccacgaggaggccgacttggttctttcgcgacaataggtagttggttgccttactggaatccacggatctccttgaatgccgaagccagatcgccgttcatggcgtcgaacaccgcgccaccggtcagctcggcgagctgttccatttcggacgcgttcgagttgccgtacaggatgataaagaccggaacacggcgcagctccgccggtagttcgcggtacgccctgctgaactcgtcaaagttttcgcccatgttcgcctggccgtcgccaagaagcacgatggaggggatgccgtcggaggtgtcggtcgcggcgagcgccgccaacagcgccgggtagagtgcggtcccgccgccggcggcgaggctgtcgacgtacccgttcagctgcgccgcggagtcgggggtcgcccggtcgaagaccacggtgagcggttcgttggggacatcgtcgaaggaccacagggtcacggtctcgcggtcccgaagcgagacgtcgccggtgagggtggacgcggtgccgtcgataagcgaatgcatgatctgcttcagtgaagctagccgcgttccctccatcgaaccggaaacgtcgagcacaaacgtggtggtgccaggtttgcggtactggttgttgtaggcgtagagcaggtcgtcgacgaccccctggttcgcggggaacggcagctcaatgacctgctgacctgcgatttccgcaggcacgctggcaacctgagcgacggggcggcggtaagtgttcgcgacgtcgtcttggtgctccaagagccagtcggcgagcgcgcggacgcgatcccctgcctccggcgacgccggatttgcgagggtagataaggggtaatcggcggagatgacgccgtcgctcggcacgatgacctcgatcggctggccgtccgcgcgcagctggtgcagcgtcgcctcgtagttcacgatggcgtccgcgcgcgacgggtccgccacgaacgcgtcggccaaccagccggaggaaccagagaccagcgactgggcctgaaacaacccctccagcgtggtgcttacccgctccaaatccgcgggactaatcgcctcgccagtgtcagcaaccgccgtggcgacagacacgagcgccgagaatcccgagttagacgacgacgggtcggtcataccgaagcggaactcgcccgattcagcggcggcggcgaagtccgcccatgtcggctggttcgcgtcccaaccgaggcgcttcgcagcttcatcccaaacgccaaaagcaacggggctagtggcgattttcgtctcgtctgcaagcttgcccgacgcaccgatgaggttcacgtaccggttcgttgcaaaccacgtggcgtcgactgcaccatcgaaatcgccgcgggcgagcgactgcgagttgtccagcgtgccgccggggaactgcatctcaattgagaatcccagttcgtttgcagcttgctgcaccaagtcttggatgtctttcagctcagtcgccgcgacaatggtcagatccgaggcgcttccggggccccctgacgaactcgaggtggtttcagtcgagcacgcggccacggccaccgttgccagcagcgcagtgatcagcgcccaaagtttcttcactgctcttcctcctccttcttcagcggcggggcgatcgagccgtagcgcgtgccgacgccgtcgattagctgttccaagcggtcgtagttcggcgcgtcgatggagttgacgtaatcggacggcgcgggaaggccgcgcttttccatttcggtggccagcgacccctggtttgcgggccggaacccgtggcgcgcggcgagctgttgcagctgcggatcgttggtgagcaagcgcccgagttctttaccttcctccgtcaccccaacaatgccgtggttcgccagcacggtcgggctcagctgcaacaacaccatgtcgtcgcggattcgcgaggtgtcgctcatcaactcaccgaggtactgcgcctcatacaccatcaccatgggtgcggcgccgatgccttggcttaagtactccgcaaacggtccggaagacgaggactcggagtacccctgaccggtgaagaatggcgcgatctccccgaccaagtactgcgtgtcttctgcacggtccgggtcgcgctgctgaaactcccaagccaggagggacaagtacatcgccgcagaattagacgtgcggatatccgtggaacggatctgcaccgtgcgcggcgacgggaatgcgtcggaaaagtcgcgccaacgagcacccgagcgggcgaggtcgacgtagcgcgccatatccatcacataggcaccgttgtcctcggtcaccacgccctgctcctgcagaatgtccgcgatcgtcttccagctggccaccgccatcggcgagaagaacgggtactccacggagtagcccgacccctgctcgcggactttctgcgccgcgggcgctgatgacgggaacacgaaatcttcagcggcaatgtcggtgcccgttgcaatctggcgggagccggcggtggtgacgtgcacctcgtaccccaactccgccagccgggccgctacgtccgggtcctcgaagtaggcgcgcttctcagagccaatgacgccgtgcacctgggtgagaccgccgtccgccttttcggagcccgggaaaccggtcgacccgttgcggccaaggacaacggcggcgataaccaccgcagtaagtaaagtcccaagcgcgatcgacactatccgtctcccgcgcttgggactttgcgtgctcgtcgcactgctcggaacgctcatacgcacatcgtagagcgcgccggacgccggtgctgcctattcggggcgcaccggagtagccgcccactgccggtagccggcgcttgcagctgcgacgcgctcgcgctgctcctcaacgcgcaccttggcggtgccgccgcgggtggtgcgcgacgctaccgccccgtcgatggtgagcacctcacggacctcagggagcagtcgcttatcgacgcccgcgagctcctcatcactgagctcatcaaggccaaccccccgagactcggcgatgcgcacgcaggcgcctgaagcctcgtgcgcctcgcggaacggcacgccctggcgcaccatccactccgccaagtcggtagccagggtgtaaccagcgggcgcgagctcgcgcatgcggtcttcgtggaagacaagcgtggacaccagcccggtgaaggcgggaagaacaatgctcagctggctgacggagtcgaccagcggctccttgtcctcctgcaggtcgcggttgtacgccagcggctgcgccttcagcgtggctagcaggccggttaggttgccgatcaagcgtccagacttgccgcgcgccagctccgcgacgtcggggttcttcttctgcggcatgatcgacgacccggtcgaccacgcgtcgtgcagcgtaacgtagccgaactccggggtagaccacgcaatgatctcttccgcgaagcgtgacaggtccaccgcgatctgagcgagcacgtacgccgcctcggcggcgaagtcgcgcgacgccgtgccgtcgagcgagttgtcggcagctgaatcgaagcccagctcctctgcgatcgcctcgggatcgagtgcgagcgaggacccggcgagcgcgcccgagccgtacggcgacaccgccaggcgcttgtccaggtcctggatgcgctcgaggtcgcgcagcagtggctgcgcgtgagcgagcagcgagtgcgcgagcaggatcggctgagctgcctggaagtgcgttttgcccggcataatcgcgtccgggtgcgccttcgcctgctccacaatcgcgtcgatcaggtcagccacctcctgcgcgatatcgcggattgcgtcgcgcagccacatgcggaacatcgccgcgacctggtcgttgcgggaacggccggcgcgcaggcggccgcccacttccggcccgacacggtcgatcaggccccgctccatggcgccgtgcacgtcctcatccgtcggcagcggaccaaacgatccgtcggcgacgtcggcgccgagctggtcgaggccggtcagcatggtgtgcaggtcggcgtcgctaagcaaccctgccctgttgagcactttggcgtgagccttggaagcgagcacgtcgtagggcgctaacacccagtcgaagtgcgtggacacgctgagggcgaacatcgcctcggaggggccgccggagaatcggccgccccacagcgcaccctcgttggtcttgtgctgctgcataccgggcctacttctgcgcgccagcttcgcggtcgcgcttgttcgcgatctgggagctcaggccgtgcaggcgcacaaagcccttggccagggtctggtcgaaggtgtcgcccgtgtcgtaggtggccaggttgaagtcgtagagcgagtggttggagcggcggccgttaaccgtcgccttgccagcgtgcagcaccatgcggatgtcgccggtgacgtgctcctgggtcgactcgatgaacgcgtcgagggagcgcttcagcgggccgaaccacaggccgtcgtagacctcctcggaccagcgcgcgtcaatgaggcgcttgtagcgggccaactcgcgctcgacggtgacgtcctccagcgccttgtgcgcggtgatcagggcgaccgcgcccggtgcctcgtagacctcgcgggacttgatgcccaccaggcggtcctccaccatgtccaagcggccgatgccctgcgcaccggcgcggcggttcatctcctcgatcgcctggagcacggtgacctggcggccgtcgatagccaccggcttaccgccctcgaaggagatgatgacctcgtccggagcgttgcccaaggagggatcctccgtgtacgagtacaggtccttggtgggcgggttccacaggtcctccaggaaaccggtctcaacggcgcggccccagacgttctggtcgatagagaacgggctggcggcggactgctcgatcggcaggtccttgccttccgcgtactcaatggccttgtcgcgggtccaggcgtagtcgcgcgccggggcgatgatctccaggtccgggtcctggtttaagaaaccgacctcgaaacgcacctggtcgttgcccttaccggtgcacccgtgagccacgtgggtgccgccgaactggtggccggcctcgacgaggtgcttcacaatcagcgggcgcgagatggccgagacgagcgggtactcgccctggtacatgccgttggccttaatggtgggcaggcagtactcctcggcgaactcgtctttcgcgtccacgacgatggactcgactgcgccgcagtccagcgcgcgctggcgcacagactccatgtcctcgccgccctggccgaggtcgagagaaacggcgatcacttcaccgccggtcatctccgccaggtacgggatagccacggaggtgtcaaggccgccggagtacgccagaacgacgcggttggtcatggaaattgctccttgtagatgagtagaagttgcggttagttaggttacccgcggtcgctctcgcgtttgcggggggagctggcaaagagttgatctgccagatccttgccggtgaagggttcgcgggccaggacgaagatggtgtcgtcacctgcgatgcagccggcgacttggtcgaggcccacccggtcgatgtagctggccaggtactgcgctgccccaggcggggtgcgcagcaccgcggtggagtacgagtggtccaccgacaccaccagctcttcaatcatccggccgagcttttcgcgcgggccggtctggatgtcgtgcgaggtctcggccacggcgccgacggtgtagtaggcaccgctgccgtccatcgggcgcaccttgcgcgcccccagttcatccaagtcgcgtgacagcgtggcctgggtgatgtcgatgccctcggccaaaagtaggtcagagagctgcacctgcgaagcaacacgggtggcggcgaggatttcgaggattcgcgcttggcgcgcggtgcgcgacaccggctgcgtcatggctggtgctccagaagccaagtcagcagcgccttctgggcgtggaggcggttctccgcctcgtcgaagacgcgcgatgccgggccgtcgatgacctcggcggtcacctcgttgccgcggtacgcgggcaggcagtgaaggaagatcgctccgtccgcggccgcatccatcgtcgcctgcgaaacctggtacggcaggaacggcgtgcggcggtccttgccgtcgctttccatccccatcgacacccacgtatccgtgatcaccacatctgccccgtcgacggcgccgacgtcgctggtgacctcgatcttcgcaccagtctcctcggcgcggcggcgggcgcggtcgacgaactcggtgcgcggcaggaagccctcagggccgatgacggtgatgtccatgcctgcggtggcgaagccgatgaggtagctgttcgccatgttgttgtcgccgtcgcccaagtacacggcgcgcttgcccgaaaggccagctgcgccctcctccgggcagaggttctcgatgatcgtttgcagatccgcaaggatctggcacgggtggaggtcgtccgagagcgcgttgacgattgggacagtggccgtttccgccatgtccagcaggttctggtgggcgtaggtgcgccacacgatcgcggagacgtaccggctcagtaccgctgcggtgtcttggtaggtctcccccttgcccatctgggagttgccggtttccgtcacaatcgcgtggccgcctagctgcgcgatgcccgtgtcgaaggagaaacgcgtgcgcgtcgacgttttgtcgaacagcacggcgacggactgcggcccttccagcggacggtacttgtacgggtcgcgcttcatctccgccgcgagcgcaagcacctccgcctgctccgcaggcgagaggtcgtcgtcggcgagaaagtgccgtggggtgtggtgtgccatcagttctcgttctccgtgttttccgtcttctctttcgcttccgcaatcaccgcttcgacacgcgcggcggcttcgctcagctcctcgtccgcaatcaccagcggcggggtgaaccgcagcacgttgggcttaggtgcgttgacaatcaccccgtgctcgtacccgagtgcttgggcttttgctgcccagtcgccgtcaaggactgcgcccagcatcaggccgcgcccgcggacctccttcactccctcgatggccgcaacgcgcgacgcgaacgcctcgcccttgcggcgcacctcggccaagaaggcctcgtccatggtgtccagcacgacctcggccgcggcgcaggaaacggggttgccgccaaaggtggtgccgtgcatgccaggggtgaacctcgccgcgacctcgccggtggcgatcaccgcgccgatcggcatgccggcgccaagacccttcgccatggtcaccacgtctgggcgcaccccaggggcaagatcgtgctcaaacgcgaagaaggtgccggtgcggccgacgccggtttgcacctcgtcggtgataaggaggatgccgtgggcgtcggcaagctgccgaagctcttgcaaaaagccctcgggcgcgggcaccacacccgtttcaccctggatcggctcgaggaagatcgccgcgacatcctcggggtcgatctcgacgagcttgcgcacgtagtcgatgtcgccgtaggggtagaactccacgccgccggcgaccggctggaagggcttgcgtttcgacggctgcccggtcagcgcgagcgaacccattgtgcggccgtggaagccgttggctgcagcgaggatccgcgagcgcccagtcaagcgggcaagcttgaacgctgcttcgttggcctcggcaccggagttgcagaagaacacgcgggcgtcggggtcgccgaagcgctcgatcagttgagttgccacgttcaccgccggccgggaggcgaagatattggacacgtgcgcgagctgcgagacctgcgcgctcaccgcctccaccaccgccgggtgcgcgtaaccgagggagttgaccgcaatgccggcgagcaggtcgaggtactcgcggccgtcctcgtccgtgaccgtcgacccggtaccggagaccagcgccacggtcggggttccgtagttgcccatcaacgcggcttgccagccgctgacaatctcgctcattcgttgtcgtccttccgaaagactgtgccttctgggtactccgccgcgtcgtagacgtccggcagcaccattgtgccaatgccgcccatggtgagaagctccagcaaaaccgagtgcgcgatccggccgtcgatgacgtgcgccgccttcgtgccgccgcgcaccgctgtcagacacgcctccattttcgggatcatccccgaatccagtgacggcatcatcttctccagctcgcccacggtgatcttggacaacagcgaatcccggtcgggccagtcggtgtagaggccctccacgttggtcagcaccacgaggcgctccgcaccgatcgccgcggcgagcgcgccggcagcctcgtcggcgttgatgttgtacacgttgccgtcgtcccccggcgcaatgccggagaccaccgggatgcgcccggcctcaatgatgtccatcaccgcggacgggtcgacgtgggtaatcgtgcccaccagcccgatgtcccgcagctcaccgtcgacctccaccaggcggcgctcggcggtgaacagccccgcgtcttcgcccgaggtgccgaccgcgtacgggccgtgggagttgattttgcctaggaggtcgcggcccacctggccgaagagcaccatgcgcgccacgtctaggatctccggggtggtcacgcggaagccgcccacgaactcgcccccgtcgagccccaagcgctgcatcatcgcgctgatctgcggcccgccgccgtgcacgacgaccggtttcgcgccgacggtgcgcaagaaaaccatgtcggcggcgaaggcgtttttcagctcctcgtcgatcatcgcgttgccgccgtacttcaccacgacgattttgtcgcggtagtgctgcagccagggcagcgcctcggccagcacatgggcgcgcgcctcgttgctcaaccgctcgctgtgggggtaggtcatcgcagtcgctccttttctcttacgtgctgtacgcggagttgatctccacgtatgagtggcttaagtcggttgtgcgcaccgtggccacgcccggcccgccagtacctaaatccacttcgacgtcgatgtccacacccgacaggtcgacctcgcgcgcacccggcgcaccggtggacgccacgcacacgggctgaccgttgaagctgaccgaaatgttgtcggggtccatctccgcatccgccatgccgacggcagccagcgtgcggccccagttcgggtcggagccgaacatggcgcacttgaacaggttgtcgcgcccaatcgtgcgcgcggcgttgagcgcctgcgcgttgtcgcccgtcccgcgcacggtgatgctcacgcgcttcgtcacgccctcggcgtccgcctgcatcttcccggccagttcctgacacacggtgaggatcgcatcgtccacctcgtcctgcgcgggggcgacaccgctggcgcctgacgccatcacgatcacggtgtcgttcgtcgaggtcgacccgtcaatgtccagcgtgtcaaaggtcacggcggccgccttgcgcaaggctgcgtcgagggcttggctgcttaccgacgcatccgtcaccaccacagccagcatcgtcgccaacgacggcgcgagcatgcccacgcccttgcccatcgcgccgaccgaccagccgtcgcgctgcacaaacgcttccttcgccacggtgtccgtggtcagaatcgcctccgcggccgcgcgcccgttgtcgccgagcgaccccgccaccgcagcgataccggcgcgcaccttctccatcggcagcagctcgccgatcaatccggtggagcacaccgctacatcgttcggctcaagggcaagatgcttggcgacgcccacctgcatctcccccgcatcctcatccccctgcttaccgttgcacgcgttcgcgttgccagagttgatcagcaccgctttcagctgcccgtcgcgcaccgcctcacggctcactttcaccggcgaggccgtcacgcggttgcgggtgaacaccgcggccgcgttgaactccggcccctcgttgaccacgagcgccatgtccggcttgccggagggcttgatgccggccgtggtcgcggcagcgacaaagcctgcgggggtggacaccgaaccgtcaaccattgtttcctctcccattacgtttcgccttctctggtctagggcgcgacagcctggcgcggcaaccctgcggtctcgtccaaccccagcgcgatattcatgcactgcacggccgcacccgcggtccccttgaccaggttgtcgatcgccgaggtcacgagcagcacacccgcgtcctcgtccacctcgacctggacgtggcacatgttggagccgaccacgttctgcgtctgcggctgcaccccctcgggcagcacccacacgaacggttcgtcggcgtaaaactcctcgtacgctgcgcgcacgctcgcggcgtcgacgccgctgtgcagcggtgcggtgatcgtggtgaggatgccgcggggtagcggcgcaagcaccggtgtgaagctcacggtgatcggtgcgtcggtggcctcagcgacgttctgcttgatctccggggtgtgccggtgcgcgccagcggtgctgtaggccttcagcgagcccatggtctctgcacccagcatcgccaccgaggccttcttccccgccccggacacgccggtcacagacacaatccgcaggtccggcttggcgacgcccgcctgcaccgccgggtacgccgctagcgtggcaccggttgggaaacacccaggcaccgcaacgcgtttcgcttttgcaatgtcctcgcggtggcccggcatttccgggatgccgtacggccacgagcctgcgtgctgagagccgtagtagcgctgccacgcggcgggatccttcaggcggaagtccgccgcgcaatccaacaccagcgtgtcatccggcagctggttcgcgatctccgcggagaacccgtgcggcaggccgaggaacaccacgtcgtgggccgcaagcttttccgcggtcgtggcctcgatgacccggccggccagctgcggcaggtgcgacaacacctgcgccgccggttcacccgcggtcgaattgccggtcagagccccgatctccatctcgccggagacgtaatccgggtgaccgagcagcagccggaggatctcaccgccggcgtaccctgtggcgccggcaacagcgacggtgtaactcatgcaaacgaacctagtactttatgcattggttcgcaatttataccgagccgctgcgacctagatgccgcgcaccgccgctccgtgctcggcctcggcggccttggcggcgcgcaggcgcgcctccgacgcctcgtcctcggtcaatgtcttgtccacggcgcggaacaccagggcaaacgccagggacttcttgtcggggccgagctgatcggactcgtagacgtcgaaaagcgaaacgctctcgagcagctcccctgccgaggcctcgatggtgcgccgcaccgcctcggccggcacgtgcttatccaccacaagcgcgatgtcctggttgaccgccgggaacgcggagagtaccggcgcgggcagcgtctccgtaagcggcagcgcggtcagatcgatctccgtggcgcaggtgcgctccggcaggtcgagggcctcgaggacctgcgggtgcagctcacccgcgtagccgacgacggtgccgcccaccttcagcgctgcgcagcgtcccgggtgccacggcagctgctgcgcagcctcaacctcgagcgcaacacccgcggccgccgcgaccacctgcgcggactggatcgcgtcggcccaggtgtaggcgcggcccttccccagcgggccgtcgagctcgctgtggccgacagctacggtcgccgcgtgcaggtgctgatccggcagcgactcgatcagctcggtaatcgtcgcctcatccgggcgctcggcaacgctcggcagcggcgaggagtcgccgcgcttcacagcggtttgcgccaccgagaagatctgcaggtcgtggcggccgcgggccacgttgcggcccacagcctcgagcatcgacgggagcagggtcgtgcccagcacgccgtagtcggcgtcgagcgggttttgcaccttcaccacgttgcggcgcggatcgtcggcatccaggccccacgtgtcgaacgtggtgttcttgataaacggcgtcggaatgatctcggcgtagccggagtacgccagcgcgtgcgtcacagcgcggcggcgtttctgcagcggcgacagcccgcgcccgcccaccggggtcggcaggatggacgggatcgcgtcgagcccttccagccgcacgatctcctcaacgagctcaacgggaacggtgaggtctccgcgccacgtcggcggggtgaccttcagtgtgtcgtcgtcggcttccacctcgcagccgacctcacgcaggcgctgctcgaccgtctccgcggtgtactcaacgcccgtgatttccgacggccgcgccgcccgcatcgcaatcggctctcgcgccggcacctcgccgaccagcgtgcgccccgcctccacggtgccgcccgcgatctcggcgagcaaggcgcaggcaatgtcgagcgagacctcaacaatcgccgggtccacgccgcgctcgaagcggcgcgacgcctcggaggacagcttgtggtggcgggccgtcttcgccacggtgagttcgtcccacgtggccgcctcgaagtaaacgttggtggtctcatccgaaatctcggaggtggtgccgcccatcacaccggcgagcgactggatgccgttgtcgtcggcaataacgacgtcggtagcggtcagcgtgcgcttgacgtgatcgagcgtttcaaaagtctcgcccgcttcggcgttgcgcacgtgcagaccaccggcgatcttgtccgcgtcgaacgcgtgcatcggctggccggtcaggagcatgacgtagttggtcacgtcggtcgccgcgttgaccgagcggatgccagacagcattagctctcgctgcatccagaacggcgcgggcgctgccgggtcaatgccggcaaccttgcgcacgccgaagcgcttcgccttggtcgactcgtcgacgttcacctcgagcacgtcacctgccggggccggcacgccggagacgtcaataccggcgacggacgggtcttccgccacgtcggtgtagcgcaggttaaacgcggaggcgatctcgcgggccaggccgcgggccgacagcgcgtacccgcggtccggcgtgacgttgacgtcgaagaccgtatcgtcgctgccgagaatctctcgggcgtcggtgccgggggtcgcggtgccgtcggcaagcgtaataatgccctcgctcttcgcggtgagaccgagctccgccgcggacgccatcatgccgttggagatgtggtcgtaggtctcgcgcgcggcgatctcgaaccctccggggagtaccgcaccgggcagggacacaaccacaaggtcgccctcagcgaagttgcgggcgccgcagataatgccctgcggctcaccggtgccgttggcctggccgacatccacctggcagtagcggatcggcttcttgaacccggtcagctcctcgatctcgaggacgcggccgatcaccagcggcccttggatctccggcagcggctggtagccctccgtttcaaagccgacgcgcacgaagcctgcgtcgagctcttcgtcgctcacagtccagccctcgttgcccgcgttttgcagcagggaggtaatccacttcttcgaaatcagcattattgttgctccttacgcctgcacgccgaacgggatagtgaaacggacgtcgccctcaaccatgtcgcgcatgtccgtcagaccgttgcggaactgcaacgtgcgctcaagacccatgccgaacgcgaaaccggtgtagacctccgggtccacgcccacggcgcgcaagacgttggggttgaccatgccgcaaccgccccactcgatccagcccgcgccgcccttcttgttggggaaccacacgtccacctcggccgacggctcggtgaacgggaagtagttggtgcgcatgcgggtcttcgtctccgggccgaagagggtcttggccaggtggtcgagcgtgccgcgcagatgcgccatggtcagtcccttgtccacagcgaggccctcaacctggtggaacaccggggtgtgggtggcgtccagttcgtcggtgcggaatacccggcccgggcaggcgatgtagatcggcacgtcgcgctcgagcatggtgcgcacctgcaccggcgaagtgtgggtgcgcatgacctgcttggagccctcctcgccgatgtagaacgtgtcctgcagcgtgcgggccgggtggtccgggatgaagttcagcgcgtcgaagttgaagtactcggcctccacctcggggccctcggcgacctcccaccccatgccgatgaagatgtcggcgatctgctcgctcagcgtcgtgatcgggtgcatgccgccggcctggctgcgtgcggtgggcagagtgacgtcgaccgtctcagccttcagctgctgctcccggtactcagcctcgcgcacctggcgaagttgcgcgtactgcttctcggccttgccgcgggccatgttgacgaagcgcccggcgtccttgcgctggtccttcggcagggtgccgagcgagcgacgcgcgagcgagatcggggacttctcccccaggtgctcgcggtgcgcctcctccagcgcgggcagatccggtgctgcctcgaaggctgcgatcgcctcatcagcagcccggttcagggcttcctctgtcagttcaatctgtgggttttcggagctcactgctcgcccgcacctttccttcacggctgggtttcaaagggtttcaaaacgcagacaagcatacctgcgggggctacgccgtcccgcgacgaggacacgttctcggcgccagcgatgcggtactctgtcggctgacgactcaggagcagcgcgggaggtggcgacatgcagctaaacgccggagcagagcttgtaaacgttctcgaggaaaccggtagcttcccagaattttcggtgcccgcccgcgaactggacgatgcgcgggtgccgtttcagtcctgctagctcccctttaccagctgctgtctcgatgggtcataggtgtagtcgacgatctcacccgacataattagctcgatcgcccggttgatcacgtctagcggaacaaggaaccattcgttggcggcaaccgacccaccggcctcgtccacaatcgcagcatccaaccgtacagctgcaaaaagtcggtgtagcaggtgctcaagcgcggacgggcggagactatacactcggtaaatcgcgaccttctctacgggggccataaggtatgtagggctcttctctgcaccccgaatgcgcttgtccaccggcgtggtggagaagccaatcttgtacaagtccttcagcccccgaatatcggggtgatcgctcttcgaccgaaggacgtagataaacccagtatgcagatccgcgtcgccaatctcggcggcagtgaaaccggtacgagtgatggcaaaaccgccctgctcccccatccgcgccccgaacgactgtcggtacatggctgactcggtgccattttcaaaaatgacacgcaagcgctctttgcgttcttccttgtgcttgaggctcaccatctcggattctcggacttcggcgataaatgccatcagtcctctgaggatgaaaaaggccccaggcactaccgtctgtgcacccttaaactctgtcattgcgcaagttccatccgcaagttcagcatgcttctgtttgaacaacggctcgaacttgtcgaaatcttcacagcggcggcgcagttcccgctcagattcttttggcttatcccgcttcggcagcgacgaggtgtcgaagatacctccagcatccccgagcagatcgagggcgtcggagcttaacagatcatcaaccgagatgggagcgtcctgcacctcaagcaacccatgctcatcaatgtcgcttagagcttcggtcttagtcttgcttgcacggatacccacaagccgagctccgaattttcgctcagagatgttcatggtttccggatccggttcgcgcccctgcgcggacacaaactcgttgacttccaggaaagcacgccgcaaacgatccgtttcggtgaccggcagtggtttctccggcatgtcaaggagaccatcctcatccgccgctataagggcatccaactttgcgaggaacgcttcttcagccattactcatccccttcctggttctctgcgcgagatttcaactcagatttccgttcgttgaccactttccgcatcactagcagcgcctctgccaactgcttctcttccgggttgtcagaacgccggtcaggttcgcggccttccattttcatccatgcctgcaccttggggaacagctccatcgcctcttccgccgtcatctcaatccgggtggtcgcaattgcgtcctgaataagcgacagcaaactgggtgtcactgacttggataggatctcgaaagcccgctggaacgggttaatggagtcgatgaggttgatactcagctcatcgacgttgatgaactgattcgccatctgaatgaaccgtttgtccccaacctccttcacctcgccggtcttgacaaccgaatccacgactactcgctggcgaacttcctcaacttcgtcatcgctgaggtctgggtactgctctcggataattttgggaatgaggactttgttcgtggtctccgggtccaccttgcccaccgccgctcgtgcgaaggtggggtcttgcaaaatcgtcgcctttagatcgttgaggtccgtgtccacaatctgctttacccggggtgtggacggctctttaaacccgtcgatcttcaccgtgtttccctcggacttgtcatccggatcatgcttgggtttgaactcgaagttttgggccagcacctgttccatgagcaacgacgcggtgatggccttgagcatgttattcaccgagatggtgacctcgctctgcaccgcatccggctctgccagcaagtttgtgaactgcgcgtgcgatttgccctcgctgtcgcgcgtgacccgcccgatgatctggatgatctccgtcagggaggaacggtagccgatggtcagggcgtgctcggcgaacggccagtcgaagccttcctttgccatgcccagcgcgatgatgatgtctaccgcgtcctggtccttcgaggccacatccaccaggtagttcagggtgcgggcgcgggccttctggtcagtgtcgtccactaggtcagcgatgcggagcgtttcaccattgtcgtggcgccgcaccacgatgatgccggtgtcctcttcctcttcaatcaccacgccgattgaatcgatgatggcgccgacctcctcgattttgtccttggtggattcgccggagttcacgttcgggatgtgcaggatggttttcttgtctaagtcgagcacttcgcccaccgcgtcggtgtagcgtccctggtagaagtggtgcccgatgcccagggacttcagatgctggtacccgttcaactggtcgtagtagttgaacgtgacgggcgtgaacttcgcttcgtcttccggcagaagcacgggcaccgtgtcgccgcggaagtaggaaccagtcatggccacgatgtgggcgtcggagccgttcatcacttcccgcagcaggtagccgaggcggctgttgtccaggtcggcggagacatggtggaactcatcgatagccagcaccgtgccgttgaatgcatcgggtgtaagtttctcgaatgcgaaacgtagcgtagcgtgcgtgcacacaagcaccgcatctggcccctcaaggaagcggatgaactgcgctaccttgctcgtgctgctgcccggcgtgcacaggttattttcgggtttaatttcccagtcagcgtaaaaaccgtgggagcgcagatcggtcggagcaaacgaaccgccgatggaacgctccggcaccgccacaatcaccttcctacgaccttgataaaaaagcttgtccagcgcaacgaacatcaacgcgcgggatttgcccgacgccggcggcgccttaatcaagaggtattgcgccgcgcgctgttcgtacacgcgacgctgcatttcgcgcatccccagtccgtctgtgctcaccgaggtccccgcctgcgcgtactccacgcgaatgacgctgtccttcacgttctttcggttcatcgtggccatgagttcactccatttcgtcgttccgcttttgacgctgcccattgtcgcaggcccctcggacaccactcggcagagttagcacacacgttcccactcgctactttctcgcggttttcctcgagcgcttcgcaggcttcgccgcctcttcagcggcgatcatttcctcgtacagtgcgaacaggtccgccagtcgctcctcatccgaggtatatggcttcgtcgagtacagcgaatccaccaattcatcattcgcttcatgggcctcccgcaggtttcgcggcattgagtcccggtcatacacctccgccaacgttcgctcgcagtggtactctcgcacatccaaaatccgcaaggccgtctcgttcaatcgagccttcttcttctcgacgccctccggcaccggaaagttgttatatacaatcgtgttcgaatacctgaagtccgttttcatcttcccgccaaccgcccgaacccaggccatgtgcatttgggaggtgaggagggcaaagagccacggctccgcgtcgtagacggcaaaagcagcattcgagataactgtatttggccccagatatcccatcggaatatacgcgcggagctcggaggagacgctgggcacgatgatggaatccgttggtttataggcaatctgcacaaaacggtgaggttgagaggcgtattttgccgtgctcggagctttactctcggaccgttcccttgcaacccggtccaacctgcgcgaaatttctggaatgcgtcgcgcatcttcgatctgggaatcctcaatccaaagacagtaacgatcttcaccgttgatgtattcgctcgctccggtgtagcgcttgataaatggttccgctacaggagtttcatcgaggagtctccgcgcatcctgcgctgtgagatcgagtgggccccggggcatgcttccgaagaccatgggtgggaagacgcgagctaacggggtgtttcgacggcccatgaaaaccgaggctgcatccgccaaataaccattgatgttaccgacctgattttttatcccatcggtgtacaggaacttcggtgcatcgctcttcgcccgcaggccgatcaccacaacggtgacgccagcattccccttcgcattgttttcccatttgaaggaggtataagcaaacccgatttcaacccccatgtcgaagataatggggaacatcaatccaacatgctcaccctgcacgacggagttggtagagaccagcgctagctgcgcaacggtgccggcgatgtactccgcacctttgatgaaccacaacgcgatgtagtcgagattcttactgtacggccggtcgccgaagacgtacccgtaatccgccttctgctccgcggtctgcttcttggagcctgcgtacggcgggttcgagatcaggtagatctcctcttccccgttgttcgggcaaacttggttccagcccatgcgggtggcgttgccggcgtggatttggccggtctccttcagtgggataagcggaatggccaccttgaactgctgctcgaattcgcggttcatctggtgcttcgcaatccacagcgacaggatggccacctcgacggcgaagtcatcgatctcgattccgtagaagttctcgatactgatgcgggatttgtcgaagagcggttgtgcttttgccagctccgcctgccgttgcaggatcgcgtgctcaaggcggcgcagctctttgtatgcaatgactaggaagttgccggaaccgcaggcggggtcgaacaccttgatcgccgcgatgcgatcaagcaagcgcgccagcttggtggagctgttgtaggccgagtcaaactcgtcgcgaagctcgtcaagaaacagcggctcgatcgtcttcaaaatgtttggcaccgacgtgtagtgctgacccaggttcgaacgctgtcctggatccacgatcgcctggaacatcgaaccgaatatgtccggattgatgtcttgccacttcagcgtgcccagatcaatgagcgcctcacgggcctttgcactgaagcggggcactgtcagatgcgcgtcggagcggaaaagccggccgttgacgtaagggaactccaccagataggcgggctttttcgccggagcaggctcgtccagggctgcaaacagttcgcgcaggaatgtgtcggtatcggagccatcgccaagcgtctgcgaagccaccgcgttcgtgaattgattatcgccgaaaatgcctgtgtcctcggcgaagaaacagaacaacagtcgggtaaagaacacattgaggccgtggcgggaggtgtcggcagccatcatgtcggggttggcagaggcgagctcgtcgaaaagcttgcccatgcgctccgccgccttcacatcggcgtgcgattcagacgtgtactgcgttttctccatgcccgcccatgggaggaagaaagtgaagtgttggtcgatctgacggatggggaacgtgcggttctccgtcgtcttcgtgtcgaacgccagtacatcttcgtagtccgtcacgataatgaaccgcggactgtacttcaccaccgtcggcgcggtgcgaagccgctccagctcttccaggagaccaccgtccacctcgctgaaatacacgacgttcttttgtgctatttcatgggtcgggtcatctgcgacgttgagacttccattgcgcaggcgcgtgacgttgcccttcgaccgtccaaaggcgagaagaagatcgaagataaactcccggtcatactcaacctggtttgctaggtgtgcgacccgtttttcgatcgcctttaggttcagccgtgccatgcggaagagtgtaagcgggcaccgctctatatagggatgacgacccggaaatcgaccgtctcgagtacgtcgacagagagcggacacgcacgggtggaggttacttgcctgctagctctgcgaggcgaaccagatcgtcctcacccagttttgtttggcgcgcgcactccgcgattagcgttctccgagcgctttggccgattcccagaggcagatactcgcggcggttgcgaggttgagcgactcggcgttgccctgaattggaatggaaacgcggtagtcggcggtttcgagcaggtcctcgggcaggccgtgggcctcgttgccgaagagccacgccgtgggctggcgcagggcatcgccgggctgggccaggttgaggtcgccgtgcattgttgtggcgaacgtcgataagcctgctgccctgagctcccctatcacgcggttgatgtcccggtcgcgggcaaccgggatgtggaagagcgagcctgcggtggagcgaaccaccttgggcgactccgggtcgaccgtgtcgccggcgaagatgaccgcgtcggcccccagcgcgtccgcaatgcggatgatcgtgcccgcgttgcctgggtcgttcgtctccacgcacacggcgacggtgcccggcttacccttcagaatggatcccaccgaccacagcaccggcctacagacggcgaaaatgcccgtgtgcgacaccgtgtcggcgaggtggtcggcggctttgtcggtgatcgggtggatgtagacgtccatgtagcgcgcggtggtcaccacttcggcgaaacgctccgcggcggtctcggtgacgaaaaggtccgtcgccgcacccgtggcggtcgcggcctcgacggaattctccccctccacaagaaacgccttcgctttcttgcggccggcagcgcgcttgagcttcgccgcgttcaccacccgcggggtgcgctcggtgtagggctgggtgaaatccaaagtcatggcacacagcctacgtcggcgccgcgatacgcttgcagccgtgatgagatccttgcgcgcagacgctgcttcaagacgcgccgcgatcgtcggtaccgctgtagtgctcgccgcggttgcggcggtgagcctggcgactattgccggcggcgttggtgacgggatcgtcagcggcactgtgattttccctttggctgctgccgcggttttaggtgcggcgtacttctcccctgtcgcgggggccgtcggttacggcgtcttgctgcagttcgccgcggcgcacgcagcgtaccgcggcccgctcatcgtggccgggtcgatcctgttggtcgcgctcctcgggctacgtgcgcggccgcgagcgagcatccctttagcgctgctgacttggtacttactccagacgcacctgacggccggggtggtcgttccggacgacctggccaccgccgtattcctcctgctactgctcgcggctgcgtgggccagcggcaccgcgctgcgcaacgcaatgaaggttcgcagcgaggcgtatgcgcgttataagcagcagcttgacgacgaacgcgagcgcaccgtcaaggccctgcacgggtcagtcgcggcgtcgttgacctccgtggtcttacgcagcgaggcgctagccatggccggcaacgcggaggacgcagcttcagcgcagctgatcgccgaggacgcccgccgcgcgatgcacgaggttcgggagctcatccggttcatgcgctccgacgacgcgttggcggttctcgctcccgctgaggtgaccccgtttgcctccctccaggagctcaccgaggtgctgcgaagccacggcttcaccgtgatcgagtcggggctggaacccgcggtgttcaagggcgcgtctctgccccacgccgcggaggtctgccgcgagatgcagacgaacctgctgaagtacgccgacccgagtcggccggtcattgtcgcggccgtggcggacgacggcgccgtcaccgtagcggtgcagaacatgatcgctccgcggcagcgcaacgtccacatgacaacgggcatcgggttggaggacatcgaggcgctggtggcggccgacggcggctcgttctcgtctggcttcgagggtgacacgtggcgctacgagctgcgaattccgaatgcaccaaagtagcctccccgggtgggtactttcgttcccccttcgcgcgcctcattgcgactgccggctgcaaaggcggataatgagggccagctagtttcgcgtcaccagaacgaaaggacccgttcccatgcgcacccgtgtatcgcaaaccccgaagcgcgtcgccgcagctgccttggctgccgcagcactcaccgcgatcgctccggtttccgccgcccaggccgaggttgctgaggttgctgaggttgctgaggagaaggtcatcaccaccttcgcatccggcgcagtcggcgacaccttcgaatgcggcggcatcatcggccgcctctggtgcaagtaaaccaagcggggctttaagcggtgagcaacgaacgcatccgggtgtttcttgtcgacgacgacccactcgtccgcgacgtcctcacccgctacctgctaactgcgggagacatcgatgtcgtgggcagcgcctccaacggcgccgaggccctcgacctcatcgacccggatcaagtagacctcgtgctctccgacgtctacatgcccaagatgggcggagccacgcttctccaccacctcagccagcggccgaacacgccggcgtttctcgccatcacatcgctagagaacgacaaggcgatgctggacatcctcgcccacggcggccgcggctacatcctgaaaagccaaccgccggacgaaatcgttctctccgtgcgacaggcggtcaccggcggcaccgtggtctcccccgccgccatgaacaatctggtccgctaccttgcgccgcacgacgccgaagcatccgctccgattgccggcaacgagcgttcctacccagcggggatcaccgccgccgagcgcagcgtgctcgacctgctgtgcgagggcctcagcaacgccgacatcgccaagcgtctcaactactcggagtcgaccgtgaagaagcacgtgtcgaacctgctcagcctgtacgacgtgacctcgcgcctcgatttggtggtgacggtgctcagcggccgccggtaggtggcttggtcgccggtgggtggccggtgggccgccagcggatcgcagtccgtcgctggcgagtcgtgctgatagcgggtaacttccgcccgggccgacgtttccgcaggtcgcaaaatggcctcttccgagttacccgctatcaccgatcggcacgcgccggtaagccgccggccggtgcccatcggcagccggtccgccgccggtaggctgccagtgggttgcgctgatagcgggtaacttccgcccgggtcgacgtttccgcaggtcgcgaccaagccatctctgagttacccgctatcaccgatcgccacccaggcgtcccaagccagcaaaaagtccccgccgccgcaaagtaagcggcagcggggacttgctcgtagaacgaggcgttcttacgcagcgttcacgggagcgttgacgtcctccgggagggcgttcttcgcaacctcgcacagggcggagaacgcagcaaagtcgttcacagccagctcggcgaggatcttgcggtcaacctcgacctcagcaagcttcaggccgtggatgaggcggttgtaggtgatgtcgttcatgcgagcggcagcgttgatgcgctggatccacagcttgcggaactcgctcttgcgcttgcggcgatcgcggtaggcgtaggtctcggagtggacccactgctccttggccttgcggtacaggcgggagcgctggccgcggtagcccttcgcggacttgaggatcgcgcggcgcttcttcttggcgttaactgaacgcttgacacgtgccatgagttcttacttccttgtctttcttcgtcgtggtagtgaatcaggcagtgcttaggacatgccgaggaggcgcttggtgcgcttgacgtcagccgcagcgacgtccgtggtgccggacagcttgcggcggcgcttggaggaaagcttctcgttgaggtggcgcttgccggcctgctcgcgacgcagcttgccgttaccgttaaccttgatgcgcttcgcggtgcccttgtgggtcttctgcttcattgtgaaagcccttcagaatcgttgacgtgctacttcttgcccttgcgagcaggtgcgaaaaccatggtcatgttgcggccgtcctgcttcggacgggcctcgaccaccgcgagatccccaatgtcgtctgcaagacgctcgaggagacggaagccgagctccgggcgcgactgctcgcggccgcggaacatgatcgtgactttgaccttgttgcccttctctaggaagcgctcaacattggccttcttcgtctgatagtcgtgctcatcgatcttcggccggaacttctgttccttgaccacagtctgctgctggttcttgcgggcctcgcgggccttctgatcctgctcgtacttgaacttgccgtagtccatgatcttgcacacggggggcttggcgttcggcgccacctcgaccaggtcgagatcggcgtcgtacgccagtttgcgggcgtcgtcagtgcggacgatacccacctgctcgccggacgggccgacgagacgaacttccgggacacggatacgttcgttgatccgagcttcagcgctgatgagaacactcctataaacgaggaaaacaatgtcagttgctaccggtgctaccgggccacgcgccgagccctccctaagaaaaaacccgctggaaccgtttgggttcagcgggagttcgtcagcagatcagatcgcgcatgcgcaatcctctcgtaccgtttacccgtagccaactctaaccggcggcgtggggtgggaagaactccacttgtggcccgcacacctagaaaaggtgcactgggcggtagtgctggtaaaagtaccacgccccaccgcccatctccaaattggcgcgcacagcgccacgacggccgcgcggttaagcctcggcgaggatgtccttcaggaactggccggtgaaggacgcgtcgacctttgcaacgtcctcaggggtacccttcgccacaacggttccgccgcccgagccgccctcggggcccatgtcgatgatccagtccgcgctcttgatcacgtcgaggttgtgctcgatcaccagcaccgtgttgcccttgtccacaaggccgttgagcaccagcatcagcttgcggatgtcctcgaagtgcaggccggtcgtcggctcgtcgaggatgtagatggtgcgtccgttggaccgcttctgcagctccgccgcgagtttcacgcgctgggcctcgccgccggagagcgtggttgcggactggccgaggcgcacgtaacccagacccacgtccaccagcgtctgcaggtaacggtggatggacgtgatcggctcgaagaactcggccgcctcagagatcggcatgtcgagcacctcggcgatgttcttgcccttgtagcgcacctcgagcgtctcgcggttgtagcgcgcgccgtggcacacctcgcagggcacgtacacgtccggcaggaagttcatctcgatcttgatggtgccgtcgccgcggcacgcctcgcagcggccgcctttaacgttgaaggagaagcggccggccttgtagccacgcaccttcgcctcctgcgtctccgcgaaaaggttgcggattttgtcgaacacgccggtgtacgtcgccgggttcgagcgcggggtgcgcccaatcggcgactggtccacctgcaccagtttgtccaggtgctcgagcccctcaaccttcttcacgcgccccggtacctggcgggcgccgttgagttggttctgcagggtcttcgccaggatctggttgaccagggtggacttgccggaaccggaaacgccggtgaccgcgaccaacacacccagcggaatctccacgctgacgttgtcgaggttgttttcgcgcgcgccgacgactttgagcttgcggtccttgtccacggctcggcgttccgacggcacctcgatcttcttgcgcccagacaggtagtcgcccgtgagcgagtctttcgccttctcaatccccttcggcgcgccttggtagaccacctcgccgccgtactcgccggcgcgcgggccgatgtcgatcagccaatccgcctcgcggatcgtgtcctcgtcgtgctcgaccaccacgagcgtgttgcccaggtcgcgcagcttcttcaaggtcttgatcaggcgctggttgtcgcgctggtgcaggccgatcgacggctcatccagcacgtagagcacacctgcgaggccggaaccgatctgggtcgccagacggatgcgctgggcttcgccgcccgagagcgtgccggctgagcgggcgagggtgaggtagttcaggccgacgtcgataagaaagtgcaacctcgcctgaatctcccgcagcacggcacctgcgatcatttcctgcctgtagcccagcaccaggttgtccaggtactcggaggcgtcctcaatcgacagttcggtcaggcctgcaatggatttctcgccgtgcgtcgtggaatcgagcctcaccgcgaggatctccggcttcaggcgtgcgcccttgcacgtcggacacggcacttcgcgggtgtaggccagcagacgttccttctgtgcgtcggaatccgcctgctccatcttgcgctcgaggtatccgatcacaccctcgtaggcggcggtgtaggagcgctgccggccgtagcggttcttgtaccgcacgttgacctgggtggacgagccgtgcaccaagtgcttctgctgcgtcttggtcagggagctgaacggcgcgtgcgcgtcgaagccctcttccttcgccaacgcctcgatgagctttacaaagtaggccttgttcgggctggagttccagatctggaaagcatctaccgcgggcgcgtccgggtccgggataacaaggtcgatgtcgacctccttgcgcacgcctaagccgtcgcaggccgggcaggcgccgaacggcgagttgaaggagaacgcccgcggctcgtactcctccacgtccagcttgtgtccgttcgggcaggccatcttctccgagaagatctgcacccggtccgggtcatccgcgtccaggtcgacgaagtcgaagcccaccagaccgtccgccagcttgagcgccgtttccaccgaatccgtcaggcgctgcttctggctcgccttcacggtcagacggtccaccacaacgtcgatagtgtgcttgacctgcttctccagcttcggcgggtccgacagctggtacgtctcaccatcgacggtgacgcgggcgtaaccctgggcggcgaggtcttggaacaggtcggcgaactcacccttgcgcttgcgcaccaccggcgcgagcacctggaacttcgttcgctcctccatctggaggatctggtcgacgatctgctgcggcgtctgccgctcgatcaccgcgtcgcacaccgggcagtgcggggtgccggcgcgcgcgtagagtagacgcaggtaatcgtagatctcggtgatcgtgccaaccgtggagcgcgggttgcggttcgtcgacttctggtcgatcgagaccgcgggactcaacccgtcgatgtaatccacgtccggcttgtccatctggccgaggaacatgcgcgcgtacgacgacagcgattcgacgtagcggcgctggccctcggcgaagatggtgtcgaacgccagcgaggacttaccggagccggacaggccggtgaagactgacatcttgtcgcgcggcagctcgatgtcgatgcctttgagattgtgttggcgcgcaccgcgcacagtcagccgttcagccacagaagtgatcgtcctttcgcctcgaacccccatcaacctaccaactgcccacacacgcctgctattcctcgccgctagggttggatgcatggaaaatgccttgacgctgcaccacgtttcggtctccgacatggacaacaactgctaccttctggcatccagggggcaggggctgctaatcgacgcagccgataacgccccagcccttttcgcgctcgcagacgaggccggggtcaccatcaccgatgtgctgaccacccaccgccaccgcgaccatgtccgcgcgctaccgtccgtgctcgaggcgacaaaagcaacccactgggcgccgtacctggagtcgccggcgcttcccgcccccgtcgaccacgaactcaacgacggcgactacctcgagtttgccgggcagcgcctgtctgttgcgatcctgcgcggccacacccctggcggcgcctgcacagcagcggtgattgacggcgaaacgcacctgttcgtcggagactcgctgttccccggcggtctgggcaaaacctcctccgagggcgacttcgtacgactgtttaaagacgtcaaggaaaaaatcttcgaccgcttcgacgatgacaccgtgatccatcccggccacggcgcctccaccaccgtcggcgctgagcgccctcaccttgatgaatggtgggagcgccgctggtagtcgccaaaccccgcctcgctggcggcgaatgttgtctacagtgggttgtataactgcatcatttcaacgtagaaggattggttagatcatgattcgcaagatcgcgcgaccaatgctcgcatcggtgttcatcatcgatggcgtgcagaccgtgcttaacccggcaagcgccaaggagagcgccgacagcgtgctcaagcagctgcgcgccgctaccccccgccagtaccgcgccttcctgccgaaggacccggagactgcggcacagatcgctggcggtgtgaaggccggcgccgcgtcgctcttcgccctcggcaaggctcctcgcacggccgcggcgctgcttaccgccacctccgccgcctcgttggtgggacgcaacgcgttctgggagaccagcgacgctgacgagaaggcccgccgcaaggcaggcgcgctgaccgacctcgccctcaccggcggcgtcctgctcgcctccgtggacaccgcgggcaagccggacatgaagtggcgcgcgcagaacgccgcgaaggtcgcccgcaagaacgtgcagcaggcgctgccgacccagtccgaggccgagaaggccttgaacaaggcgggcaactggttctccgacgccaccgaccaggtcggcgactacatcgacgacaacaagggcgactggaagaaggcggcccacaaggctggcgacgcggcgcaggacctcttcggtgacgcgcgcaagcagacgtccaagttcctttccaacgccggcgactggctcgacgacgcgaccggcgaggtcgaggacaagtaccaggacctcaagccgagcaaggtccaacagtacaaagcgaagcgcaaggtcaacaactttgtgggcgacgcgcagaactgggccgaggacgcatgggacgacgtgaccccgtccgcgctgcagaagttcaaggccaagcgcaaggtgaactccgttgtggatgacctgcagtcctccctcgacgatctcaccccgtctggcctggacaagttccgcgcaaagcgcaaggtgagcaagaaggcctccaagctgcaggaccgcgcgcaggatgccgtggacgacctgcagaccgcgtgggacaacctcgacgcctccccgagctggtggcagaagcgcaagtggaaaaagaaggctaacaaggctgaaaagcaggcgaagaagcttgtgaagaaggcgcagaagaagctgggctagcccaagcttcggccccgggaaccggaataatccggcccccggggccgtttttctctttatgcgtgactacgagcagaagcagttggccgaggagcaggcgcatgtcgacgtcctgttccagcacttgggcgccgaagttgacgccgcccgcgccaagctcgccgaggtgcaggccgacgtggaccccgacaacccggactccgatgcgcttgtccgccgcgaaaccgagtaccacgcgctaaacgcaaaactggaccaactcggcatcgctgaggtgggccttgtcttcggccgggtggacgtgcacgacgacacccccgagaaccccgtagcggggcgcaccgacctcgaccgccgctacgttggccgcttgggtttgagcgaccgggcagatcactaccgcacgctgttgctcgactggcgcgcccccggtgcgcgtccctactacctggccaccacggcgcaccccgagggagtggagacccgccgcaacatccggatgcggggccgaacggtgacggcggtcgacgacgaggtgctctccggcgaaggcgcgcctacggaatccgacggcgcgggcgtcggttcggaggccgcgctgcgccgcgccatgaacgcggcgcgcaccggccacatgcgctcaatcgtcgagaccatccagcgcgagcaggacgagattatccgcgacccaacccgcggcgtgatggtagtgcagggcggtcccggcaccggcaagaccgcggtcgcgctgcaccgtgttgcctacctgctctacacctggcgcgagcagctctcgcgcaccggtgtgctcatcatcggccccaacgacaccttcctcgactacatctcccgcgtgctgccggagctcggtgagacgggcgtagtgctcaccaccatcgccgatcttgtgcccggtttcaccccggaagcgctcgcatcgaacgaacctttcgcagcgcgcgaggtgaagggctctgaggaaatggcggtgattttgaagcgcgctgtgcaggcgtacgagacggttccgaaggagccggttgcattgcttatcgacggggtgccggtctccgccactccagccatggtcaaagcggcccgcacccgcgcgcgtcgctcgcgcaaaccccacaacgccgcccgggcccacttcgcggaggagctgacgagccagatcgccgcggcgctggcgcaccgcatcggcgaggacccgctcggtggggagaacctgctttccgcggcggacgtggaccagctgcacgacgacttagcggagcacccgcaggtgggttcgctgatcaacgctcacttccccaccctcgcgcccgccgacgtcctcgatgcgctgttgaccagccgcgaagccatcgccgacgccgctggggattacgacgagtacacccaagatgcgctctaccgcgagccgggttcgccgttcacgccggcagacgcggcgctggttgatgagctcgctgtcctcatcggcacggacgacgccgagaaggaacgccgccgcgaggaggaggaatggcgcgcacaggtcgctgaggctgaggacgcgctggacatcctcgcgtcgtcggaagccaccgacaacgacgacgaccagttcgaagccgagatcctctccgcggccgacgtcattgacgcggagaccctggcaaggcgccaacatgtgcgcgatacccgttccacggcccagcgcgccgcggaagaccgggcgtgggcgtacggccacgtgatcgtggacgaggctcaggagctctcgccgatggagtggcgcatggtgttccggcgctgcccctctcggtggatgacgctggtcggcgacactgctcagacctcggcgccggccggcacggacgactgggaggcgacgttggagccgtttgtgggagggcggttccgtatgcacgagttgacggtgaactaccgcaccccggcagaaatcatggcgtacgcggatgaggtgttggtgcgggctgggggcgacaaggcggagcagacaagcatccgctccggcgccccagtcgcccactacccgcacggcaccgacccagacgaggtccgggccccgctggacgagcgctcgtgcgccgtgatcgacgcgggcaacgtcgggctgatgaagggcctcgagtttgaccacgtcatcgtggtcgagccgcgcaaaatagtagaggcctcgccacaggggtggcaagacctctacgtcgccgtcacccgggccacgcagaccctgtcggtgatcggggaactgtaactagctactcggtgaccgtgtggacgatcatcacgtcgcagtcggactggcgggcgacatctgccggcaccgacccgagaagacggccggtcagggagttgatgccgcggttgcccacaacgagcagctcagcgttgttgtcgttcacaattgccatgagcgcctcaaccggggtgcccgggcgggttgcggtctgcacgtccttcgcaccgtgggagcgggcgtgctcagccgcagcctccaggttcttcagcgcctggtcgtcgccgaggatggttacggaatcctggcgcagcgccttggaggcgtcctcctcagacttgtagtaggcggtgccgataaccagggtggcgtcgaacgccacggccatcttggcggcgcgctcaacagcgaggagagaggacttggagccgtcggagccgacgacgatggtgttgtagtagttgcccatggtctaaagtgtaacccttcagcatcagctacgtgcttcggcccgagtgtccaccaacatcacatccacgcgggccttcaccgccacgttgcccggcaccgtgccgaaaacacggccggcgagcgagtgcatgcccttgttgcccacgacgaggagatcggcaccgatctcggccacggcctcgatgagcacgttcgcgggcttaccggcccgggagatcagctccacctccccggcctgctcctcctcggccaccgcctcggcgcgcgccaggatctcctgggactcggtttcggtgatggtgttggcgccggtcagctccgcgttcgtggagttgagcaccgatccggatgccgagtagtgcgcgcaaagaatggtcagctttgcgccgtacacgcgggccaggctggccgcggcacgtaccgccgccatggagcgcggcgtgccgtcggtgccgaccgcgactgaggaatacgaatgcatgctcgttatcgtccttgcatttctcgtaccgctagttaccagtctctttcataccacgcagttccttgcgcagatcggcgatttcatcgcgcaggcggccggcgagctcaaatttgagttcgcgggcggcttcgcccatttgctttgtcaggtcgtcgataagcacctgaagctcatccgacgccatcgctgacacgtccgggcggtccgcaaccgccgcatcggagctcaagcttggcgacgcagcgtccccttcaccgttctcgtacacctggtccaggatgtccgcgatcgccttgcgcagcggttgggggtcaatgccgtgctcgttgttgtaggcgatctgcttctcgcggcggcgctccgtctcgtcgatcgcctcctgcatggactcggtgatctggtcggcgtacatgatgacctcgccggagacgtttcgggcggcgcggccgatggtctggatcagcgacttggtggagcgcaggaagccctctttgtcggcgtccaagatggccacgaggctgacctcgggcaggtcgagaccctcgcgcagcaagttgatgccgacgagcacgtcgtactcgccgagccgcagctggcgcaaaagctccacgcgctgcagggtgtcgatgtcggagtgcaggtagcgaaccttgatgccgttgtccagcaggtagtcggtgaggtcctcggccatgcgcttggtcagggtagtcaccaacacgcgttcgtccttggcggtgcgtgcgcggatttcgtggatcaggtcgtcgatctgccccttggtcggcttcacggtcaccttcgggtccaccaggccggtcgggcggatgacctgctcgacgaactcgccgcctgaagcctcgagctcgtagtcgcccggggtggccgacatatagacggtctgccccacgcgcgcttcgaactcatcgaaggtcagcggacggttatccaccgcgctgggcaggcggaagccgaactcgaccaggttccgtttgcgcgacatgtcgccttcgaacatgccgccgatctgcggcacggtgacgtgggactcgtcgatgatggtgaggaagtcctccgggaagtagtcaatcagcgtggccggcgccgagcccgcggggcggccgtccatgtggcgggagtagttctcgatgccggagcagaagcccacctgctgaatcatctccaagtcgtactcggtgcgcatgcgcaggcgctgcgcctccagcagcttgcccttgctctccagctcctccaaccggtccgcgagctcgagcttgatgtcctcgatagcgcgctccatgcggtcgtccgtggccacgtagtgggtggccgggaagatgcgcacctcgtcttcctcgctgatcacgtcgcctgtgagcgggtggatgtagtagagcgagtcgatctcgtcgccgaagaactccacgcgcaccgccacctcttcgtaggcggggatgatatcgacggtgtcgcctttgacgcggaaggtgccgcgcttgaagtcgatgtcgttgcgctcgtactgcacgtccaccagaaggcgcaggaagcggtcgcgctccacctcctccccgacgcgcagcacaatggagcggtcgaggtaggactgcggggtgcctaagccgtagatgcacgacaccgaggcgacgacgaccacgtcgcggcgcgacagcagcgcggacgtcgcggagtggcggaggcgctccacgtcgtcgttgatcgacgagtccttctcaatgtaggtgtctgtctgcgcgatgtaggcctcgggttggtagtagtcgtagtacgacacgaagtactccaccgcgttgttgggcaacagttgccgcagctcgttcgccagctgcgcggccagcgtcttgttcggcgccatcactagcgtgggccgctgctgctgctcaatcagccacgcggcggttgccgacttaccggtaccggttgcacccataagcacgacgtcttcctcgccgcgccgaaggcgggcatccagctccttaatcgctgccggctggtcgccggagggctcgtactcggagatgacctcaaaacgcttttcgcgacgctcgatctcgccgacggggcggaactccgattgcgcgaggacggggtgttcagcagcaaaagccatgctggcaagcatacgcccagcacaatcccagcgacgaacactgaagatgaggctcccgtcgccattccacatcccccattgggattcaaccagtgctgcgagaagggacgtatccctgcagttcagcccgccggagtaccgtaggtagtatgttcgagaccttgcagaacctgatggccccggcttctgtgatcttcgtggtggcgatcatgttctccaccggcctttcgctcaaggtcgatgatttgaagaagaccctcgtgggatggcagttcttcgttcgcctcctgctggtgaattttctcgtggtccccggcaccatgctgttgttcgtccagctggctaaggtcgcacacccctactccaccggcatgctcatccacgcgtgtgtggccggggcgcccctgattatggcgctcacgcagctgagtaagaacccggtcgcgctcggcgctaccatccagctggtgcttatggtcgccaccgtggtcatcatgccgctgctgctacccgcggtgctgggtatcgaggacgtttcttcaagtgcgttaatcgaacccctgctgttgcagatggtgtttccgctcgcaatcggcatggttgtgtttaatgtggcaccgacgctgactgccaagatccgcccgctggtgcgtaccctggccaacgcagtcatgatgttctttctcgtcctgtctgtggtcgccttcggaccctacttcggcgatctacagttgtggaagggcgtgttggtgggcatgctcgccctcaccgtggcgttttacgtcggttacggcaccggcttggacggcggcggcgcgaagtctcagctgggtgccctgggcactgcgcagcgcaacacagccgcgggcgtgatcagcgcgatggcgttcgacgagccgctggtgttcatcaccttcgtgttcatcaacagcttcatgatgttcgtgctcatggccttcgcgaagcgcttcggcgcaggcaagacgatgccgctgctctccgcgttgttggaccagcgtccggttgccgcacaggagcagtaggaatcctcccggccgtccctgcgctaggacgcgtacttccgggtggctgcgagccagtcctccagctcaccggtatcggcccacaggtcgtagagctcggactcaccggggcgcgttgctttcgctgcgtggcggcggatccaccgccggtcatccaaactgaaggggaagtccaacgcgtgtgcgacagcttggttcgggacgtggccgttgagtaccgcggccagtgcaatcacggattccgcctcgtcggcacccaagggcccgcgaccgcattcaaaccggaactggtccatgcgaaacgtgccgtccgccagggcgacgacagcttccgtagctgggtcgttgtcgaacggacccgtatcccaagttcccatggcggagtaggttaaaccgcagaggttaacgcccggtaaatttcgttggtctagaacaaatactttaggttccaattatctcaacaagtcgctctacttggggcgcgagttgggatttcggaccgttgttgtcgatgacgaagtcggcagcggcgcggcgggtagcgtcgtcaagctggcgggcgatgcgcgcccgagcgtcgtcctcatcaaggccgcgcgaggagacgagacggcgcacgcgttcctcagcatcgacatcgacaaccacggtgaggtccatgtcgttgtgcagaccctgctccaccagcagcggcatatcgtaaacggcaaccttgtccccccgtgcctcagctgccgcaaattgacgctcggcatcagcacgaattgcggggtgggtaatggcgttgagcttctccgtctctccctcggaagcgaacgcgcggcgggctaaccctgcccggtccaaggtgccgtcctcgcggatgaggtccgcgccgaacgtcgccgccacctcgccgagcaccggtgaaccgggcttcatgatctcgcgcgcgatcttgtccgcatccacgatggtgtagccggtctcccccagcatcgccgccaccgtcgacttgccgctgccgataccgcctgtgagcccgatgcgtttcataggacccaaacgtagcaaaacggcccgctgccaaccgtggagttcagcaacgggccgtcgccaagcaagccagcctaaggcgggctaaaggttagttgccggccagcttctcgcgcagagcagcgagctgctcgtcagaagcaagggaaccaccctcaacctcggaaccgtctgccgccggagcgccggcaccggtctcggaggtgtagttggtctcggaggagtagttcgagtcgttgccgccctgctccgcagcctcagctgcggcagcgcggtggcgctcgatctgcgcggtgtgcgcggtgtggcgacgctctgcctcggcgtagcgtgcctcccactcctggcgagcctcctcgaagccctccatccactcgttggtctctgggtcgaagccctccgggaagatgtagttgccctgctcgtcgtaggagtcggccatgccgtaacgcgacgggtcgaactcctcggtgtagtcctcgtctgcctgcttgagcgacagagagatgcggcggcgctcaaggtcgatgtcgatgaccttgaccatgacctcttcgccgacaccgacaacctggtccggcacctcaacgtggcgctgagccagctcggagatgtggacgaggccctcgatgccctcctcgacgcggacgaacgcgccgaacgggacgagcttggtgaccttgcccgggacgatctggcccacagcgtgggtgcgggcgaagacgcgccacggatcctcctgggtcgccttcagcgacagggagacgcgctcgcggtcgagatcgacgtcgagcacctcgacggtgacctcgtcgcccacggtgacaacctcggacgggtggtcgatgtgcttccaggacagctcggacacgtggaccaggccgtcaacaccgccaaggtcgacgaaggcgccgaagttgacgatggaggacacgacacccttacgcacctggcccttctgcagctggtgcaggaagtcggagcggaccgcggactgggtctcctccaggtaagcgcggcgggagagaacaacgttgttgcggtgcttgtccagctcaatgatcttggcctcgagctcctggccgatgtacggatccaggtcgcggacgcggcgcatctcgaccagcgatgccggcaggaagccgcgcaggccgatgtcgaggatgaggccacccttgaccacctcgatgaccgtaccggtaaccggctggtcgttagcttgcagctcctcgatggtgccccaagcgcgctcgtactgcgcacgcttcttggacagcaggaggcggccttccttgtcctctttggtcaggacgagagcgtcgatctcgtcgccaacctcgacgacctcatccgggtcgacgtcgtgcttgatggacagctcgcgggtcgggataacgccctcggtcttgtaaccgatgtcgagcagcacctcgtcgtggtcaaccttgaccacggtgccggtgacgatgtcgccatcgttgaagtacttgatggtcgcgtcaactgcggcgaggaattcctcagggccaccgatgtcgttgatagcaacctggggtgcgttggaagtgcgcatatgtatatgtgctccgaaaataggagatcgaaatgtgtaggggcatatctctcggcggcaccgtgaaggcgcgcaacacggtggggctacgatctcacgacaagagtggtagggccctcctattacggccgccgccaccccgtcgcattgatacgcccgcataacagtagtgactttgaccagctgaagcaaataaacatgagtgcagaaacgcaggccaaccgccgccattgggacgcagacgctacgcgctaccacgccgagcatccggagtacctgagcgggttttactggtgcccggaaatgctcagcgaaaaggaagcgcagttgcttggtgacgttcgcggcagatccatcctcgaaatcggctgcggatccgccccctgcagcgcatggcttgcggagcatgccgcggacgagaacacatttgtgaccggcttcgacatctccggcgctatgctcgcgcgccgccccggtaccgcggctgagctcccccttgtccaggcagacgtgctggccatcccctaccgcggcggcgttttcgacaccgcgttctccgccttcggcgccctgccgttcgtggccgacctcgacgcggcactcgctgagattgcccgggtgctcaaacccggcggccgtttcgttttctcagtcacccaccccatgcggtgggtgtttcccgacgaccccgaggcgctgcacgccgagatcagttacttcgagcgcgcctatgtggaggtcgacgacaacggccgcttgagctacgcggagttccaccgcaccttcggcgactgggtgcgcgcccttcgcagcgccggcttcgagctggaggacgtgctcgagcccgagtggccggagggcttagcaaccacgtgggggcaatggtcgagaaagcgcggcgagctgttcccgggcaccgcgatcttcatctgccggctccggtagacaagcctgtagaacctgttaagttcgtagacagccgtacaggtgagcggcatggagggataactgaatagctcgcggggcgggtgccggtggtgaccaccgcggcacccgccccgtttcattgtctttccggctagtgcgccgcctcgtcccagttcgtgccctcgccggcggaaacttcgagcgggacgagcagctcaatggcgccgtccatttcgcgctcgacgatctcgcggaccgcgtccagctcgcccggggcgacttcgaccaccaattcgtcgtggacctgcagtaacactcgcgaggtgtagccgtccaaggcggcgtcgacacgcagcatcgccaccttgatgatgtcggcggctgtgccttggatcggtgcgttcaacgcggcgcgctcagcgttctcgcgcgcgagccggttatcggaggtgagctcgggcaggtagcggcggcgcccgaaaatcgtggaagtgtagccgtcgcggcgggcctgctccaccacctcatctaggtagcgtttcacaccgccgaagcgctggaaataggcctccataatttgttttgcctcccctgccgggatgcccagctggttagacaggccgtacgcggacagcccgtacaccaagccgtagctcatggctttgacgcgacggcgcagttccggggtgacctggtcgatcggtacttcgaagactcgcgagcccacgaagttgtgcaggtcctcccccgccttgtacgcctcgatcaagcccgcgtcctggcttaaatgggccatgacacgcatctcgatctgggagtagtcggcggtgagcaggcagtcgtagttcttacccacggtaaatgcggagcggatcctccgcccggcctccgtgcgcacggggatgttctgcaggttcggctccgcggagcttaggcggcctgtcgacgccaccgtctggttgaaggtggtgtgaatgcgcccgtccggctgaatcgtcttaatcagcccctcgatggtggacttcatcttctggtactcgcggtgcgcgagcaggtggtccaggaacgggtgcgggtgcttctcagccagagcctcgatctcgccggctgcggtggagtagccggttttggtcttcttcgtcttcggcaggtcgagtttgtcgaagaggaccacggagagctgcttggggctggagaggttgagggtgggctcgtcgacaagctgccgcgcttcctgctccaccgcggcgaccttgtccgtgtagtcgcgcagcagctcgtcgagcacgtcctggtccacggcgatgccggcgtcctccatctcggcgagcacgctggtcagcgggatttccaggtcagcgtagagctcgaaggagtcgatggcgctgagttgggcggacagttcggcggcgagttcgaggacggccgaggcggcgtcgtgaagcgccgtgctccgcagctgcttctgcaaatgccgctggtagacgtcctccagcgcgtaggtgcgctggcccgggcgcaacaggtaagcggcaaccgccgtgtcgtgcgcaatgccgcgcagcgtgatgtcgcggccgcgcagcatgtggtaggcggccttcgcgtcgtgcaggaatttgggtgagtcggactcggcccagcgcttcagcgccgcgtcctcctccggggacaggtcggctgcgtcgcgctggagggcttttcgctgcttatcgacgatagcgatcccctccacatcccccctcccaggagcaacagtgcccgtgaggtacacggccacaccttcgccctcgcgggccgcaagccactcgtcgagggggatatcttccacgaccacgtctggcaacgcgacggtgtcggccgaggcggtgtcggcaggcgcgccggtggtctccaccaccgcaaggacgcgctcgcgcaggttcacgccgaactccagatcgtcgaaggcgcgggccacctcggccacgtctgccggcttgagctgcagatcgttaggcccgaccggaagttcaacgtcggtgaccatctgcgtgagctggcggttcatcttcacctgctcgatgcggtcgcggaagttctgacccgccacacccttcacgttctcggcgccagcgatcagtgcgtcgagcgagccgtgctccacaatccacttcgcggccgtcttctcccccaccttcggaatgcccggcaggttgtccgacgggtcgccgcgcagcgccgcgaagtccgggtactgcgccggtgtgagcccgtacttgttctccacctcttcgggcgtaaagcgggtcatcgtggacaccccgcgggtcgggtacatcagcgtggtgtgctcgtccaccagctggatgtagtcgcggtcgccgctaaccagaacgatctcgaaatcgccctcggcgcgggcctcggtgaccaaggtggccacgatgtcgtcggcctcgaagttctccttcgacagggtggcgatgccgagggtggcaagcgtctcctcaatgattggcacctggcccttgaactcgggcggtgccgcggagcgctgcgctttgtactcgggaaactgctcggtgcggaacgtctgccggccgacgtcgaacgcgaccgccatgtgggtgggctcctcatccgccacgatgttggccagcatggacagaaagccgtacaccgcgtttgtgtgctgcccaccggaggtggagaaattctccgcgggtagtgcgtagaaggcgcggaaggccatggagtggccgtcgataagcagaaggcgtttcacggcctccaagctacccggccaagctgcgccggactacgggcgggtgggggccggcgggtagtggccgccgaagcctgcgtacggtgccggcgcgggttgagccggcgcgggtcggggcgctgtgtctactgccgctgcgcgcaggccaatgcctgcgatggcagcgccggcgacggaggcgacgagccagacgatagcgccggcggtgtacctactccagagctggttctcggactgcagggcgcagacgaagaaccacacgaactcccacccgtacgcggtagccgcggtcacccacgccgcgcgccagcgcttcgtggcgccgagcactgccgctgcgacgacaagcgtgaggaacccgtagaaggtgagcgtgtaaaaaccatcgttcatgacctcgacgaaccacgcgatcggggcacgggtaaatgccgccaagagcaccgccagcactgcgctcgcacccatgagcgaccaatgcttgccctgcggtgccgggttcggcgaccacagcgcaacagccgtgccggcgcgcttggctcggacgagctccgcgatgctgagcgcagcgccggcgaggccaagcgccatccataaccaggtccccgcgcccaccgcagcgtcacgcgccccgtattggtcaactctttgttgcagggagacatcgtcaaagtagatcttgaccggaaacgaggcgagatggactgcccagaagaactgagtgagtgcggcaatcagggcgatcaccggggttgcccaccagccacgggcgcgatgggcgagtgcaacggtaaggacaaggcttaggagcacgaccaccgcggcgatcggcaacacgatccactggtttacaaactcgccacgaagcagcagcgaggtgtcgaagccggtgtgagtctcgccgtcggatgacctgactgttcggtggccaaggagcgtgcgcacctcgacgatgctccacgcacccaaggtcgcgctggtcttgtacgcctgcagaaacgaggtgacgagggacagcgcggccaccaccgccatgccgatcgggaacacccgcagcagctggttcgtcttaacggtttgcgcaggcgcgcctggcccgacgggcggcggcggaggggcgccctgcgggccgaaggccggctggtaggactgctgcggatgggagggcgggctccaaggattgtgcgtcacggtaatttccttcgttgctctctcgcctaactgcctgcgcttgtacgaccaccgttatacattaggcaggaaaataccagccagagtgtagggaaattttaatgattttcatcctgctcgccgtcgccgcgatcgtggccgtcggctatttcatttttaaggaggtgcacgcagcttccgcgattttcgcggtgggtgtcctgctcctcatcatcgcggccgccaccggccggatcgagtactcgtcggcgaagattgagccgagcggcaacgcgttctacgacgagcttttgatcattgagtcgctgttcaagtcccggtactcgggtaccggtatggcgatcatggtgctgttcgggttcgtgggctacatgcgccacatcggcgccgacgccaagaccgttgtggcgctttccaaaccgctgcgcaagttcaacggctcctactggctggtgcccatcggtttcctcgttggcaccctgctctcactcgtcgtcccatctgccgctgccctatcgctgctcttggtcgcaacgttaatgccagcgctcatcgcagctggcctgtcgccgctgacggtgggcgcgatcatcgtgacgtcctccaccattgccccctccccgctcgaagctggtctgatccagggcgcgtcgctggtggacatgaccgtcaccgagttcgtgttcggcaacgtggctaaagcaaccattcccgcactggtcatcgtggcgttcacccacatgtggtggcagcgccgctgcgacattaaggacgcagcgaagatgcaggctgaggttggcgctggtgttggcgcgggcaacggttccgccggcaccggcgccgaggtgacagccgcggacgccgcggaaatgcaggaatccgaatccgaccggcgcgtgcgcgaggccgtcgagcgagccgagggcctgcccggcttctacgccatcctcccgctgctgccgctcatcctgatcatcgtgtccgcgattctcaatcgcatgggcgtgatctcgttcgaggcggagatcctcccagtgaccgtggtctccctcatggtgaccatggtgatcgaggcgatcaggcttcacgacataaactacgccgtggactcgctgaaggaattcttcgcggggctcggcgaggccgctgcgggcgtggtcgccctcatcgtggccgctgccatcctggtcgagggcattacccagatgggtgtcatcgacggcctgaccaccatcgcccagcgctcttccggcgccgcggtgctgatggtcatcatcttcgtcgcagccaccggcctcatggcgctgctcaccggctccggcgtggctccgtacttcgctttctccgagatggtgccgggcctggcagcccagacttcgatccacgctccgcagatgctcacctcgatctggtcagcgtcgaatctcatgcggcagggctcgcctgtcaacgcggcggtgatcatcgtctccggcgcgctcgacgtgaaccctgttgaactggtgcgtcgcacgctggtgccgatgctcgtcggcacgatcgcttccgtcgtcttcgctttcatcttcatcgcgtagcgtggctacgaaaccgctggtgggcacgcgattcaacgatgcgcccaccctgcgctacactttgaaatcacgccgctgacgcttgaacgcgagctttcacgcggcgcggatgccccagtagcccaattggcagaggcaacggattcaaaacccgtccagtgtgagttcgagtctcacctggggcacacatgacagacttacggggatcttggaaaactcgctctagattctcgcgaccgcgccggctgtgtgcgtctgaattcagtacggtcgcaaggacgaaacgtaaagacactcattttagggaaagttgtcgatttaccaacgacagcttagatgcacttagcacgcactagccgtgtttcttgttccaccgataccggcggaagtaaaagatcggcaaaataaggacgtagtaaacgcctagtgtaaatatgactgggatcagcagttcatctaggttgaaattgctccagaatgagctgtttgcgctggggtgctgggtgccggattcctcgttgacgggaaataccacgtacatggcgattgccccgagaggcacaatgacgaaactctgccaccatggcggaacccatggcgccccattttcgtctctggcggcgagcgcccctccgaaacccatttcaaacctagatcccatccccagaacctccttagctgatgtgcatctgtacacttctcgacttcgggttcgtctgcactacggttttgggtctcaacgaggatgcccgtggaacttagtctacgactggaccgtaatgccgttggttaaagaattcttcgaaatcccgaagaaccccgctcacccgcctcgacgagaggcttggtgggcggggttctctgctgtgtgacggctacttgctcgtgcgagtgagcaccatcatctgcttgttgtcgtcggtcggctggagcgtcagcgtctcgccgttgaactggccctcgaacgcgaggtcttggccggtcttcacgtcggcgagcttgatcttctttccgccgtctttggactggcagcgggcgtcgtccgtgttgccggcgttatcggtgaacgaccagcggcacttgttgcccagctccagggtggcggtgccctcttttgcaccggtgtcgatgttggtgacatcgccggtatacgtgcccgccgtcgagctgccgcaagcggtgaggccgacggcggtcaggaccgttgctgctacgagtgctgtctttttcaactctgtcctcctgttgagcaaagtaagaatgtccttaaatcgttgtgctgctgacaatagcgcgccgtcgtaaagcaggactatcccccgtgaccggattcgcggccgtcgagataaaaacgttatcatctgcggtatgcgcaaaaccttggctactggcgtcaccgcctctcttctcctctcgggtgcccttgtcgcaccgaccgcgtctgcacagaccgcccagccggcaggcaccggcgcgaacagctctatcgaaagctcgagttcagctgacaacgccggcgagaagaagctgggctcgtcgcgggatgagacgaagaatgttccggaggcgccgtcgataggcaagcgctccgacgccctcgatttcctggacgccgacccgtacggcgaccccctctacatcgacccggagaagaacccgctgaagaaggtctccagctccgaaatgttcacggactggaccaaggacatgccggagggcaccggcaaggatgtcgtccagggttgggcggctggctcatccattccggacaccgcgaacccaatcgaactgtggaagcaggaagtccagggcctgggcatgatgtcgtccggtcttgccaccggcgacttcgcgcaaagctcccgcggttctagccaggcaacttcggtgattatcccggtgctggttggcagcctggtgattggccaactcattgagttggtgatgcgcggcctgcggatggcgggtattgaggtcccggccctgaccttctagcggttaggtgggcagtccccctctacataactgggcgcagctacttcggtggctgcgccttttttcgttacgtccccacccacaagggcccgaatcggcgctcttccccctgagggtttattatgcactgcggtgtatgtttttctttccgacgtgatttttggtgacggatgcgatttttaggcaacaacccgaggcgcgcagcggcgctgatacccgccgcggcgttgccgctggcactggcggggtgcgtgaccaaccacgagggtggaaaccccgacggttgggaagcgatcgtccctgagaccgtgcctgagatcgcggcgatggtcccggccgaggttgctgcagacggggcgttctccatgggcacgaacccacccttcgcaccgttcgagttcaaggattccgacggcaacttaatcggcctcgagctggacttgggccgtgcgctcgcgggcgtgatcgggctggagtaccgcccgcaggaaatggacttcgccatgattctgccggccgtgcaagccggcagtctggatgctggcatgtcgggctttaccgacaacgaggaacgccgccagacctttgacttcgtcaactttctctacgcgggcatccagtgggcgaagcagccggacgcagatatcgaccccgctaacccgtgcggcttgactgtcgctgtccagcgcaccactgtctcggacaccgacgacgtccgcccgaagagcgaggagtgcgtcgcccgcggcgaagacccgatcacggtcctggcgttcgacacctctgacaacgcggcgctcgctgcgctggtcggccgcgccgacgcgctgagcgccgactcccccgtgacggcgtgggcagtgcagcgttccgacgggcgcatggagctcgtcggcgacatgttcgacgccgcgccctacggcatcgccgtgccgaaggattctggcctagctcctgcgctggctgccgccatgcagcacctaatagacaccggcgactacaaccgcattctcgcccagtggggcgtggatagcggccacctcgagcaagcgatgatcaacgaagagccgtacgcacagcaaccagaagggcaacgataaccatgagcaatcgcgtgacaccgcgaaaccgccgggaggctcccgcgcgtcccgagcgtattgaggccaaaccgctgcgccaccccggacggtgggtcctcgccgctatcttggtggcgcttttcatctggttcgtcgtcggtgcagcccgaaacgaggcgtacgggtgggacacctacttccagtacctctttgacacgcgaatcgcccgcgccgcgctgcacaccatcgcgatcacggtcctcgcgatggtgatcggcgtcgtcggcggcgtgatcctcgccgtgatgcgcatgagcccgaacccggtgtttaagtcaatcgcgtggctgttcctctgggtcttccgaggtactccggtctacgtccagctcatgttctggggcctgatcggcgcgatctacgattcgatcaatctagggttcgcccagatctcgctggagccgttcacctcttcggcgttcatgctcgccgtggtgggcttgggtctcaacgaggccgcctacatggctgagatcgttcgctccggcgtgtcctcggtgcccgagggccagatcgaggcgtcgaaggcgctcggcatgggctggggccagaccatgcggcgcacagtgctcccccaggcgatgcgcatcattatcccgccgaccggcaacgagttcatctcgctcttaaagacctcttcgctcgtggtggctatcccctattcccttgagctctacggccgctccatggatatcgcggccgcgttgttcgagccggttccgctgctgcttgtggcggcgacgtggtacctggcaatcacctcgattttgatggtcggccagttctacctggagaagtacttcgaccgcggcgcgtcgcgccaactcacctcccgtcagctggcgagcctcgcggacgcggagggcaccatccccaaaaacgtccagatcatcgacgccccggaaaagaaaggccgttaacgccatgacaatcaagcacacccccatggtgcaggccgtggatgtctggaagtccttcggcaacttggacgtgctcaagggcatcaacttggaagtgatgccgggcaccgtaacgtgcatcatcggcccgtccggctccggtaaatcgacgtttctgcgctgcgtgaaccacctggagcaggtcacagccggtcgcctctacgtcgacggggagctcatcggctaccgcgagcgcgacggcgtgctctacgagatgagcgagaaggacgccgcgaagcagcgtcgcgatatcggcatggtgttccagaacttcaacctgttcggccaccgcaccgtactcgacaacatcatcgaggctcccgtccacgtcaagggccaaaacaccgccgaggcgaaggctcgcgcgatggagctgctcgccatggtcggtttggagacgaaagcagacgcgtacccgatccagctttcgggtggccagcagcagcgcgtcgccatcgcgcgcgcggttgcgatggacccgaagctgatgcttttcgacgagccaacctccgccctcgaccccgaactcgtcggcgaagtgctccgtgtgatgcgcgcactggccgacgagggcatgacaatgatcgtggtgacccacgagatggcgttcgcgcgtgaagtcgccgacaacgtgattttcatggccgacggccagatcgtcgaggcaggtcccgcggacgaggtcctcgagcgaccgaaggaggagcgcacgcaggccttcctgtccaccctgttctaggcggtcagcaggccggttataccgcgtacaagcgcggtgagaccaccgaacgccgccaaccccaaagccacgcggtaggccgcggccacgggcactttggtggcaactcgagcaccagcaacgattccggccaccatggccgcggacgcggctccccaagttgcggacgcaactgctgcgaggtccgcggcgcccgtggcctcctttatcccgaacgacaacgccccgctgaccagaaagatcggctgcagcgtcgcggcgtagatcgatttcggccagcgcgctgcttgcgcgtagaccgtgatggcggggcccgcgacgccggcgagcgtgttcatgaaacccccgaccgccccggcaaacgccgctggccacgttccctcaatcgggggaacgtagcgtttacctaatgtgaccacgctcaacgcggccaacaacagcacgcccaccactacaagcagcacgtcaggcgacaccgcccggatgagaaaagcacccggcaccgcacccaaaatcaggcaggcggcaatgggtgcgacgcggcgccagtccacgttagcgcgcattgcgattgtgttggacgtcgcgttaatggtggccagcacgttgaccaacatgacgccttggacaggccccatgagcacagagagtgcaggagcggcaatgagccccagccccatcccggtgacgcgttgcaacgcggccccggaaaagacagcgagaaccaccccggcaattatggcggccgacatggctacttcagtttctcagcaatggcgcggtgcaccgcctcaggtaccaatcctgtgatgtcgccgccgtacttggccacctccttggtcagggaggaggagatgtagccgtacttctcgtctgtgagcagaaagtaggtgtccaccccgcttaaccgccggttcatctgcgccatgggcagctcgtactcgtaatccagcgcagaacgcagccccttcaccagcgcggtgacgtggtgcgcggtggtgtaatccactaacaacccgccccagctgtccacccgcacgcccgggatatcggcggtgacggtgcggatgagctcgacgcgctcgtcaatcgtgaacaggcccgatgttttcgtcgggttgccggtcacaagcacgatgacctcgtcgaagtggcgcgaggcgcgggtgacaatgtccaagtggccgttcgtgatcgggtcgaacgagccggggcacacagcggtggtcatctactcctccttagcttccgggtcttcgtagacggccatgtccatgcgggcgatgccgtacaggcgcttcttcaacttctgcccggttggggtgaattccggcggccaagcggtttcggggctttcgcggtggcgctcgatgacgacaacggccccgtcgacaagcaacggcttcagcgcctccaccatctctgcgactgcctcgtcggcgaggtcgtagggcgggtccgcgagcaccatcgaaaagtgcttgcgcggtgcgcgggcgacgtacgtggacgccttcaccggctcgacggtcacgtccgggtgccccaccacggacacgttgtgctcgatgatctgcacagcgtgcgggtcgttctccaccagcacgaccgactccgcgccgcgggacgctgcctctaggcccagcgcgccggaacccgcgaagaggtccagcacccgttggccggggaagccgaagcgcacttggagggaggaaaacaggccctcgcgggcgcggtccgacgtcgggcgcgtgccctccggcggcaccttgatcttgcggcctctggcttcgcccgagatgatgcgggtcatcgacatggccccgctcctttctgctgcacagtgtgtgctctaactcttatccaaatactcgaagtcttccgccacaaacgtcgccgttgcggcgcgcgcgaactccaaattatccgcgacgatgtttgccgcgtcgtcgtaggcccgtttcaccagatcgaaatcgtcgaccaagttcacaagctttagcgtgcgggtgatacccgattgcatcgtgcccagcacgtcgccttcgcggcggttgagcaggtcgagctccgcgagcgcgaacccgtcgttggtcttcgcaacttgcgcgacgcgctcgaaggcggggctgccctccggcgcgagcgtgtggaaaaggcacagcgactcgttgccgccgcggcccacgcgcccgcgcagctggtgcagctgggaaatgccgaagtgctccgactcccggaccatcatgaccgtcgcgttcggcacgtcgacaccgacctcgatcaccgtggtggaaaccagcacgtcgatctgaccggcggcgaagtcgctcatcacgtcgtctttctctacgcccttcatttggccgtggagcagggctacctcgaggtcgcgcagcggaccggcttgcagcgcggcggcggtctcgagcacacccccttccccgtcgatgcgtgggcagacgatgtaggcctggtggccggccgcgacgtcctcgcggatcttttcccacgcccgctcgacccagcgctcgagccactgcggcacgacggccgacttaatcggcttgcgcccgcccggcaactctttcagcgtggagactgaaaggtcgccgaacacggtgatcgcgatggtgcgaggaatcggcgtcgccgtcatcaccagcaggtgtggagtgagctcaccagccttggcgcgcagctggtcgcgctgctccaccccgaagcggtgctgctcgtcgacgacgaccatgccgaggttgaagaactcgaccccgtcctggatcagggcgtgggtaccaaccacaatgtcggcttccccggtgacgatcttcaacagcgcgtcctgcttcgccgcagctggcatggagccggtcagcgccaccaccttgaccggcacaccggcagccatcagcgtgctggtcagcgaccgggcgtgctgcatgaccaggacttcggtcggtgccagaaacgcgcactgcgcgccgttgtccacggcctgcaacatggcgagcagcgacacgatggtcttgcccgaacccacctcgccctggagcaggcggttcatcggctgtgtgagcgagatgtctgccgagatgtcggtcaacacgctggattggccccgggtgagcgggtacggcaagcgcttgagcagcaggtcctggtcgccgccctccttgcgcggcagcggcggcgcgctgcggtgcgacgcgtccgctcggcgcacccccatcgcgagcgcgacagacagcgcctcgtcgtactttaggcgcgcgagcgccgcttctggcccgtccgggcccggctcgtggatctggtgcacggcggcgttgagtggcaggtacccgatgggcgtgaacccgagcggctcttcaaccggcggcagcgattgaagcaccatgtggatcgcgcccatgatggtccacgtgctgacgtttttcgtcgccgggtagagcggcagccactcgcggccggagaggatctcttccaactccccgaagtgggacaattgacgaagggagccggtggcctgggtcggcccgtcgagaagcacaaaatccgggtgctgcaactggggccggtcgtggtacacggagaacttgccggtgaacatcgcgcgccggcctggtttgagcacccgcctcgcgtactcggagccgaagaacgtggcggcaaaagtgacgttgccgtcgtcgataccaattttgtagatgggccgcttggggtttttccggttggtgatcagctgctctgagaccacggtgccgatgagggtgacggtgtcgccctcttccaggccctcgatacccgagctcgtgccgtagtgcaggtaccggcgggggtagtagcgcaacaggtccccgcacgtgatgatgtcgaggtgcttggcaatggcgcgcgcctgcttctggggaatcaccaggttcagcgggcgggtgtcctcgaagccgagcatggcgctactccaccccgatctcagcaaccgcgccgagtttgtctgccgggaatgcgaacacgtcgacgccgaggcggtccggcaactgcgccagcgcagcctcttccacggcttccgggtcgaagaagatggtgacctgctcgccgccgtgagacaagaatcgctggcaggtggtggtgatggcgtctgttggttcgtcggcgatcaacaccagctcaccgcgggtggtcaccactatgtcgcccctcgccaccgcgccgccctggatcagccccgcgcgcggcgcccggtgcgcaacggcggtgcgcatctcgcttgcggcctcggccatggcgaacgcggcggtagccaagggctggctcggatcgtgcacactcagtgccgctaaaccggagaccagacgcacggtgggcagcagggtgacggattgctcgaacgcccgcgcggccttttccaccgcggccaactgccgctggtcgagcagcccgttcggcagcaagacaacctcgctggcgtcagaccggcggatggcggcaagcaggtccgccacgacgttgtcgcccggcgctaccggttccgcaccagcctcgcggtacagctgggtgagagacccgggaggcgtgatggccaagatgaggcgctcgggcatggcagtgacgggcgtggagggaaggacttccaggcgcagctgcgagacctcgccagcggcgaaggagcgctcgatgacgcgccccgcgtccgtggagtggatgtgcaccttagcttccgtctcgtccacgcgggcgacgatcaggctgtcgcccaaccccgccagctcagcttccagcgcgtcgacgtcgccgttgaacatgaacatgacttcgaggttgccggtagcgccgtggctctcgccggcgtaaccagcaaccccacccaccggcggcgcggcctcatgctccgcggcgcttttcacaggcgcagcatcgacttcctcagtaagcgcttcgaggagcaccacaagccccatgccgccagcgtccacgacgccggccttgcgcagcgcttcgagctgggacggtgtgttggccaaggcggtgcgggcagcctccgtagccgcgagcgcgacgccttcgatgctggactcgctcccgtccccggcatccgccacctcctgggctgcggcgacggcggcggcgcgcagcacggtaatcacagtgccctccaccgggtcggcgatcgccttgtccacgaaccgcaccgccgccgccaaggagtcggcgataacggcgccacccggcgcgtcatcggccatggattgggccacgccgcgcatgacctgggagagcaccacgcccgagttgccgcgcgcgccttttacggcgccgacggcgagcgcttcggcgacttggcggggatcagcggctgcgggcaggcgctccgcttccgcgacggccgacgccatggtgtgggccatgttcgaacccgtgtccgaatcgggcacggggaacacgttgagtttgttgatctcgactctccggcggttcagctcgtcgcttgcgcggcgggcccacgacatcagccgtgcgccgtcgaatcgggatgggtgcgccatgggggcttagtttacaacgaccaatcgacaggctttgcgccttgggcttgaaggtgcgcgttcgcacgagagaacgggcgcgagccgaagaacccccgcgaggcgcttaagggcgacgggtggggcgaggcgatcactggcgtgtccccaaggaacttggccgcggtttgcgcgtccctgccccacaggatcgccaccagcggctggtcgcgttcggccagcccccgaatcgccgcctcggtgatctcttcccaccccttgccgcggtgagagcccggctcgccggggtggacggtaagcacccggttcagcaggaggatgccctggctcgcccaggaggaaaggtcgccgtcgacgcgcggcgggatgccgaggtcgtcgtttaactccttgtaaatgttcaccaaggagcgcggggcggccaccccgggttgggtggaaaaggcgagacccatcgggtgcccgggtgtcgggtacgggtcttggccgaggatgagcacgcgcacctcgtcgaacggctgctggaaggcgcgcaggatgtcgtcacctcggggcaggtaggcgtcttgcgcgcggaggaagtcgcccattaggtgcacttgcttttcgacgcccccgagcacccccatccacgatgcatgcactggcagactcatgcgaagctctcccatcctgcggtgtgggtgggcggcgtggcgtcgacaagcacctgtgcccctttcactactttgccgatggagcggaacccgaccggggctaagccgtcgcaagtgccgatgagcgtgtggtcctcgccgccggtgagcacccactcccaggggtcggtaccgagcagctcgccggcggcgacgaggagcgcatcgggggcgatcgccaccgaggacaggtcgatgccgacgccggagcaggacgccatggtggtcaggtcgcggacgaggccgtccgagttgtcggtcatggcggtcgcgccggcggcgcgggccactacaccgcggcccggagtgatctcggggacttggtgagcgttgaccagcggttcgagtgacggcgggatctccttgccggacttaagcagcgcgagcccagcggccgagtagccaatgcggccgtgggcgaccaccctttgcccgggtcgggcgcgcgagagggtgagcgcgtcgaggttgccgccgagcgagccgatggcggcgagcgagatcaccagctcatcccccgacgtgacgtcgccgccgacgagctcggaggaccacgcttccgccatggtgcccacgccgcgggccaactcctccaccaccgaaagcggcgtcgagggcggcgcggagaccgcgagcagcgctgccacaggggtcgcgcccatcgcctcgatgtcggcgaagttctgcaccacagccttctggccgacgtggaagggtgtggtggtctccgggctgaagtggcggccggcgaccagcatgtcggtcgccgccaccacgcgcgagttcggggcggagcgggtcagcaccgcagcgtcgtcgccgttgaccgtagacggggctgccgcgacgatcgccttgatgacgtcgccttcaccaacctcgcccagggttgggccggcggagggaaagccggtgtgaatcacgttgtaacaaggcctttcactagactatgccgccatgagctcgactgttaaggacgaattccagattaaccggactttgctctccatcatcctcgccctcgctctcgggctcgtcgccgcggtgcttttcggcgcgcgctacaccttcaacacggtcgcccagcaaccggtggccatgccggagcttccctcgtcgcaggccgattccgccgagtgcgccgcgctgatcgattcgctgccggcgaaggtcgcgggacataagcgcgccgagctcgcccagcccgccccggcgggcgcggccgcgtggcagtcgtcgtccaccgaccgggtgacgctgcgctgcggagtcgacctgccgctgcagtacaccgcgctggcgttgaccgaagaggcgggaggcaccgagtggctgcgcgtcgacgacccggcgagcgagctcagcacgtggtttacggtgaaccgctcccccgtcgctgccgtcaccgccgagcgctccggccgcgccccagtcggcgacattgacgcctctcccctcccgctcacggatctggctccggcgccggcacctctgtcgcagctcgccgctggcgacgctgcggcatgcggcccgcttgaagattcggtgccgcaggagatcgcggagggctttccgcttgtcgacgccccccagccccacaccctcgcatggcaatcatccggcaaccagacggtggtgctgcgctgcggcgtggcggatcctgcgaactacgcgccgggcgcccagcttgtgcaggtcaacgacataacctggttcgaagacgacgcggacgcggccgccaccacctactacgccttggggcgcgaggcggtggttgccgcgtcgatcccgctgaccggctccaacgagatcatcacgaacgtaagcgaccttattgccggcgcgatccccgctcgagcgcagtcgtaaccagagtgcgcaaaagctccgggtagctcaggccgcttgcctgccacacctgcgggtacatcgaaattgaggtgaagccgggcatggtgttgacctcgttgagcaccgggccgccggcggtgaggaagaagtccacgcgcgcaagcgaagcgcagttcaacgcctgaaacgcggtaaccgcgagctgctgcagtttctcggtggtcgcctctccgtagggcgcggggatggtggcggtgacctcgtcgtccaagtacttcgtctcgaacccgtagaagccctccgccgagtcctcggtgccgttcaaccgcgccggtaccgacgcctccacacgcccgtccgggtactcgagcacgccgacctcgacctcgtcgccgtgcagtgcgccttcaacgagcactttggtgtcctctgcgaacgcgagctcaagcgcgggttccagctcctcccaggtatccaccttggatacgccgatggaagatccgccgttcgccggcttcacaaagacaggcaaccccaggcgatcgcggtcggtatcgctgagcgtctccccggcgcgcaggatggcgccgggcgcgaccgcgatcccctcggcctccactagcttcttcgtgtactccttgtccatcccgcaggccgacgcgagcacgcccgggcccacgtacggcacgccggaaagctcgaagaggccctggatagtgccgtcctcgccatatttgccgtggaggacggggaagacgacgtccacttcggccaccacctcgccggtggctgggtcggtgaaggtgccgcgggttgaagggtgcgtcgacaagcaaactgcccttccaccggtgacttccggcagctcgcggccctgaaccgggtcgagcgaaccctcgacccaagttccgtcgcgcgtgataccaaccgggaagacctcgaacgcgtcgcgcggcagctcggccataatcgcgccggcggaaatgcaggaaatcgagtgctcggtggactgcccaccataaataacagcgatgcggatcacgtggcgatcctacccggcgctactccgacttcttgcttcggcccatcagcgccgcgatcgcgtcggagaccttcagctccgcgtggcacaccgcgtgcacggcctgggtaatcggcagttccacaccctcgcgctggccgagctggaagatgcttgccgacgaaatcacgccctccgcaacctgccccttcgtcgcagccttggcctcctccatggtggcgccggcgcccagcgcgtggccgaacgtgcggtttcgcgacagcggcgaggagcacgtggcgaccaagtcgccgagccccgcgaggccagcgaacgtgcgctggtcggcgcccagcacgaggcccaggcgggtgatctccgccagcccgcgggtgatcagcgtggcgatggtgttctctcccagcccctggccagcagccatgccgcacgccagcgcgatgacgttcttcgtcgcgccgccaatctcgcagcccaccacgtcggcgttggtgtacgggcgcaggtagctcgttgcgcacgccgcctgcaccagtttcgcgcggttctcgttctcgcaggcgatcactgtggccgccggttgctcttcggcgatctcgcgcgagaggttcggcccggacagcacggcaatccggtccgtgtttgcgccggtgacttccgcgatgatctcgctcatgcgcatgtgcgtgccggtctcaatgcccttggagatgctgagcagcgtcgcgtcgcccgggatgtgcggtgcccactgggtgaggttgccgcgcatcgtctggctgggcacgccgaacacggcgatcgcggcgccgtcgagggcctttttgaaatcggccgtcggggtgatcgcttgcggcagctccacaccctcgaggtagtcggggttctgccgcgtttcggcgatcgtcttggcaagctcttcccggcgcgcccagagttgcaccgagttgcctgcgtccgcaaacaccttggccagcgtggtgccccacgaaccggcacccatgactgccacgttgaccacgattcgcacccgccttgcttgcttctgacgccatgaaaatgcttctacagaaactaacatctgccagctcgcgaggccggttggcggggcgggtaggcggggttaataggcggggccggatgcagcgcgcgcaagggtaggacacaatagaacctatggctgaacattccccggaccccaccacaatgcacgagcaggacaaagaccgcgcgggggaaatgtttatcaccggccggcaccaggagatccccgtcaagccggacaaggagttctcccgcaccacgctcgccgccggcgctgttttgtggcgcggcgacctgacgcacccggactccctcgaggtggcctgcatccaccggccgcactacgacgactggtcgctagccaagggcaaactcgacccgggcgagtcgctggtcgccgccgccgtgcgcgaggtgcaggaagaaaccggctacgacatccgcctgggcaaactcatcggcaaaactgtctacccggtcaagggcagcaccaaggtggtctactactggacgggcgaggtcacaggcggcgacttcaccccgaacgacgaggtggacgagatccgctggctgcccatcgcagaggcgaaggcgctgatgagctacgacctcgaccgcgaggtcttggccaaggcagagaagcgtttccgcacccccgcagacgcgcgcatcctgctcgtgcgccacgcccgggcccacgagcgcgagaagtggtccggcgacgacaacctgcgcccgctggacaagaagggccgccgccagtccgagatgctggttccgctgctcgcgcccttccaccccgagcgcatctactcggcgcagccgcagcgttgccaagcaaccgtggccccgctggccgacgagctgaacttggaggtggaggttgaagcactgcttgacgacgctgcgtggcactccaccatggtccaatccaaacaggccatctcggagatcatctcccgcggcggcgtcagtgtggtgtgcgcccaaggtgaggccatcccccagatcgtggcgtggctgtcgtctcaaggcacactcccgatcgacaccgacatcgccgcgaagaaggggtctacctgggcgctgagcttcagaaacggccagctcaccggcgccgactacatccccaccgccctgccagtgcagtagctctggacctactactgacgtaccaagagaaaggatcatgcgcatggccgacaccacggctttggcaccaatcacccaagaacgcgtcgaggcgcaactcgacgcgttcgacctgaagtacttccgcggcgaggacggcaacacccgcaccgcgttccccggtctcgtgtgctttttcgatttcaccgacgccggctgcaagatttcgagccgctggctcggtaccgccgccacgcccgaggacattgaaaccctgcgcgaaacggccaacgtgctcaaccgcatcatccccctggtgcgcacccacccgattttgcgctcggacgacaccgcaatcgcggtcattgaggcgccactgttctccaccgtgggcgtgaccgacgagcagctgaaacagatgcttgaatattacttctcctccgcccaccacgtgatggccgaactcaagcaggccctgccgcacatcgacgactccctgaccgaaagcaaggcgtaaacgttatgactactgcgaacacccccgccaactccccagatcttcaaccgctctccctggagcgcgtcgcggctacgttcgacgagctcggctggaagtacgaccttcatccagagacgcaggctctccgcactgggttctccggtatcggcatggagatcaagttcctcgccccgaccgtgagcattgtcagcaccgtcgccgtcgacgtcatcaccgccgaccgctataaggacgttctcacctgggtcgagaactacaaccagcacagcgacttcccctccgcgtccgccttcgaggacacccagcgcaacctcgccgccctcggcgccactttcgctttgcccggctactgggactacaccgacgagcaattccaagcgcacctcacctccggtatccagggtgttgtgaactgcgcccgcgagttcctcggccacttcgccccggacgttctgcagcacctcgattccgccaacgccggcgcgggcaccggcgaagcgtaggcagctgcagcggttgcggctccggctgctgtagaggtggcggttgctggccgcttcggccgatacagctcaaggtcaccacaaactgttgctgacaaagtggcgcttccaaagtgttgtttgcacatggtcattaactgagtacgcaccccctaggcaggccgccactactcgactaatgaccatctgcaagcaacactttggagatgaccatctggccagccccgcgatggccccgcaacagcccaatcagctgtgaaagaagtgatgcgtgggacaaggttctgccgcgcataatcgtcggcgattcgaaactgccctagcgagatcgccagccgccgcactttcccctgccgcaaaccgttgcttgcaaagggttgcttgcacatggttatcaaccgagaagacaccccctaggcaggccgccactactcgactaatgaccatctgcaagcaacactttggagacgaccatctggccaggctgcggcgacccggcagcagcccggtcgagcgttgcaaaagtgatgcgtgggacaagattctgccgcgcataaccacctcatcctcaagtagacggtcttatgcgcggcagaatctcgacgtaagaggcggcgcgggcgcccagcttgactagagatcgaccgccggcttgaaactggggcgggatgcctcgaaggactcgatggcggcttcgtcgcggagcgttaggccgatgtcgtcgagaccttccataagccgccagcgggtgtattcatcgatctcgaaggtgtaggtgttctcgccgacggtgacggtctgatcttcgagggacacggtcgcttcgaggcctggctgctgctcaagctgcttccaaatgagctcgatgtccgattcggtcatgatgccggcgaggaaaccggccttgccggagttgccgcggaagatgtcggcgaagcgggggctgaacacagcgcggaagccatagtccatgagtgcccagacggcgtgctcgcgggaagacccggtaccgaagtcttcgccggcgaacagcacggaaccgttgcggtacgcatcctggttcagaacgaagtccgcttcgttctccctccagttcgagaacagcccgtcctcgaaaccggtacgcgagacgcgcttgaggtagcgggcgggaatgatctggtcggtgtccacgtttgttcgggtcagcggcacgccgacgccggtgtgggtggtgaatttctccatgggtgtctccttacttacaggtcggcacttacaggtcggcggggccggcgaggtggccggtgacggcggtagctgcggccaccagcggagacaccaagtgggtgcgtccgcccgggccttggcgtccctcgaagttgcggtttgacgtcgacgcggagcgctcccccggcgctagctggtccgggttcatgcccaggcacatggagcagccggcggtgcgccactcggcgccgaactcttcgaagatcttgtccaggccctcttcctccgcctgctgcttgaccatcgtggagctcggcacaacgagcatgcgggtaccgtcggcaatgcgtcggccgcgcaccacgtcggcggcggcgcggaggtcctcgatgcgggcgttggtgcaggagccgaggaagacagtatcgatggcgatgtcgcgaagcggggtacccggcttgaggtccatgtacttcagcgccttctcggcggcctgcttggcggcgtcgtcaccgaagctctccggatctgggacgttctcgccgagcggtaaaccctgtcctgggttggttccccaggtgacgaacggggtcagcgcggaaccgtcgatctcgacgacagtgtcgaaggtcgcaccctcatcggtcggcagcgtcttccagtacgccaccgcgtcgtcccagtcctgacccttcggcgcgaactcccggcccttgacgtactcgaaggtcttctcgtccggggcgaccattccggcgcgggcgccggcctcaatcgacatgttgcagatcgtcatgcgcgcttccatggagagtttctcgatagcttcgccgcggtactcgatgatgtggccctggccgccgccggtgccgatcttggcgatgatcgccaaaatcaaatctttcgccgtcacgccctcggcgagctcgcccgagacctcaaccgccatcgtcttgaacggcttgagcgacagcgtctgcgtcgccatcacgtgctcaacctcggaggtgccgatacccatcgcgatggaaccgaacgcgccgtgggtcgaggtgtgggagtcgccgcacacaatcgtcatgccaggctgggtgatgccgagttgtggcccgacagtgtgcacgatgccttggcggatgtcgcccatcgggtacaggcgcacgccgaactcttcgcagttcttgcgaagcgtggccacctgggtccgcgaggtgggctcggcgatctccaagaggttgccggatgcgatgccctcggtggggacgttgtggtcttccgtcgctaagtgcagctccgggtggcgcagcgtgcgaccagccacgcgcaggccgtcgaacgcctggggcgaggtcacctcgtgcagcagctggaagtcgatgtaaattagatcgggctgaccgttctcacccttggtcacaacgtggtcgcgccacactttctccgccagcgtcaacggcttctcggccatcgcgtcctcctcaaacgtccaaaattccagcatgcggaatgctagtatccatcgtgtgagacagtatagcgaagactcgggcatcaaagttcttgaccgctcggtagcgatcgtgcgatccgtagcgtcgggcgacaagtccctggcagccttgagcgaagacaccggcttgccgcgcgcgactacccaccgcatcgccaccgcgctggaaatccaccacattctctcgcgcacggagcagggatcctggaccatcgggcccgcgctggcccacttcaccgcgggtaccccgccgcagctgctcaccgccgcgggaccagtaatgcgcgagctcgttgaaacgacgggcgaatccgcccagctttacgaactcacgggcgacacccgcacctgtattgccgccgaggagcccgaaagcggactgcacaacgtggtgccggttggctcccagctcactctgtcagcgggctcagccgcccgcgtcttcgcggcgcatttgcttatcgacgcccccttcaacccatccgacctcgaacaagtcagagccgacggctacgcagaatccgtcgcagaacgagaagtggggctcgcgtccgtgtccgcgccggtgttccagccggacggcgcgctcgtggcggtgctgtcgatttccggtccggcggaacggctcaagccctcccccgccgagcgctggggcaaggagctgcttgcggcgaaggtgcggttggaggagtcgctgtaggcgtcgcgccggtcgatcgcgtcgagctcgccttgcggccacaccacgttcttggccagcggaatctggtgcgacgcgctctccaggatgtgcatgaagtagcccgccgcgttggggatggccacgatgtcgccggctgcgaccccctttgggaagcggatcttgcgccgcaggatgatctcgtcctcgatgcagtacgcacccaccaggaacgcctcgaccggttccccgtccgaggtgcgtttcaccagcaccggatcggtaaggtagtcgtccgaggtggtgcggcactgtgtacggttcatctctagaccgaccaggggcaggccgtccgagcgggtcttcacaaacgcgacgcgggcgaggatgacaccgcagccgtccagaagcgagcgccctggttctaggtgcagtcggagaccgcgttcgcgtaatccgtctgcgataccgtcggcaagcacttgctccagccattccccacgcgtcggctcctgccagtacgggtaggtgttggtgagcggatccgccttccacgtgaaggcctctgcgtaaccggcgcgctgggcggcaatagctgcttggtagtcgtcccactggcacttgtgctcgaggtagcgcatgggaactcccccgccgatgtcgatgaactggggggcgtggcctgaggcggtgagggcgtcgacaagctgcatgcactcgcgcagcgccgcagagcggtctgcggccgcgtacccgtgaaggtgggcatggagaccaacgatgctcacgcttgccgacggctcgctgagatgcccaacccaatcctccagccgctcgccgaaccgggtaggcggcatggtctctggatcgggcgccagacgcggggcgacgcgggcggtcaacccggacgcctcggcgagttcgcggatgcggtcgtactcagcgcggttatcggccgaaatgactacaccgttgtcgatggccaactgcagcaggcggtccggcttgatggcggcggagaggataatgcggtctcccggcacgttgtggtcgagcacttggcgcagctcgttctcgctggcgacgtcgacgccgttgccggtgtcgcgcgccgtgtcggcgaaaacaaggcccttattggccttccgcgcgtagaacactttggtctccacaccgaaacgctcacccgcttccaccaactcgtcgatgttggcctgcattgggcccgggttcaggacgttgacggggctgccgtagcgctcaatcagcgcgtggcaggcatccgggtccgcgagcagttcttgcgaccactcgaaatgtttcggttggagtggcgggagcccgtggacgcgatccggtttctccatcgctgcggcgctgacgcggtcagcccagcggtcgatgacgtcgtgcttggtgcgcttcagggtgtcgtggccgaggatcaggctttcgttcatccgcccggccgcggcgatgtgccgctggcccacgagcgtgccgtcgcgctcgacgtgcagggcgttggtgtcggcatagcgcttgccgacgcccgcctccaccacattgcccaccagcgtgccctcgaccacgccgggcgggggcaggactgcgtcgatgatcacggtcgcgccgacctcccctgccagcgtgcggaggtcgtcgtttccgcgggccaggagctcggtgcggattcggccggcatcgagaagttgtaggaggatctccgctgactccggcggcgggccgaaggcgacgcgctccatcgtccgggtgaacgcatcgaagtccttgccgcccagcgactcgcggccgccgaacgaggcgcgctcaatcagcgcgtcgtaggtgtcacggaaggccacctgcgcggccagcgccggcgtccacggttgttcgccccgggacgcagcgagtgatgcgcgcagttctgccaccgcgtcgccggtgaaatcctcgccggcgagaacgctgcggatgtcctgcgcgtccccgtctccaccggtgatgcggaggatctcgagcgcgcagtcgaggaggatgtcctcaagctcgctcaggttgcggcacccgaggatcgcctgcgacgccgcgtcgatgcggggctgcgcccgctttttcgcatccccgtcaagataagccttgacctccatgaagcggccggagcgggtgaccgggtagaaaactttcgcttcggcgtacttcaccacgtcaataaacgtcagggccgctccccgcaccagtacgatgtcgtcctcgctgacaacgtcgaggttcgatgccgggtacgccggggccacaaccctgcagccgcccacggattcgtatgccagcgaacccggccaatcgtgcgcgtggccggtgacgataagaacttcgtcgaagcgttcccccgccacgtcaaccccgtccgcggtgggcgagatctcctccacccgctcgatgcggtgcgtcacgcggcagcgcagcggcaggtgctcctcgagggcgcgccaggaggcggccaagtgctcgccaacatgcgcgcgactaggaaagtcgccttccagctgatcctcggggtcgaagggacccagctgcgttgccacaatcgtcttgggcgcgttcaagatccacgctcgcggcacggaaaccccgaacgcccctggcgctgacgcctcgggaagcggccggtcgttgaacacggtcagatgaattgctgccccgcgctgccgggctcgctccatcagtgcttccgccgcccacagcccgcgcggtcccgcgccgatgatcgctaccttcatactgcgcctccaatctgctccgcaacccactcgtcgttgtacaccgtgtccaaatacgcccggccgtcgtcgtggaagatggcgacaatctcgcgcgcggcaccctcatcgatgagctgggccacagctgcggcaacagcgccgcctgatgcccctggcacaaaccctgtggtgcgtgccaacccccgtgccgagcgcaccgcatccgacgcaggcacccgaatgacgcggtctggaacgacgtccttcgacaactcggtcaccacgcctgcgccgtagccggggaggatgcggtcgccgcgggtgccgtcgaaaagcacggagccctcagcgtcaaccgcgacgacggtcgtgtcgtaaccgtgctcgcggatgtgcttcaagcagccgccgacggtgccggttgtgctcacagccacggcgagcaactccggggcgtggccaagttgctccacgatctccgccatcgtgccttgatcgtgggcgtcgaacgctgcgcggttggagtactggtctaggttcaccgccccgatctcctccttcagctgcgccacgaggttgcggcgcgcggtgagccagtcgcccgtttcggggtcaggctgctccaccgggtgcagcaccgccccgagggcagcgatcatcgacagcgtcgcccggttggtgcgggggtcaactacgcagtgaaactcccaaccgcccgcgaccgcctcccgcgcgagcgcaatgccgaggttgccgctggaggactcgaccgcaaccgcgcccgggtgaagcagccccttcgcggtcgcgtcggccaccatcgcccgcgccgagcggtccttcgcgctgccgccggggttgaaagactcgagcttcccccacacctggctttcgccgccctcctggaaaccgcgggaaagatcgacgagcggggtgccgccgatcgcgccgaggatgcctggcgcggcagcggttgaaggtagattcatgcgttccagcttatgcgctagagcgcctcgagctccgccacccgcttctgaagctccacaaccagcgggttccccggcagccgctcggaggcgacgttgctcacagcgcggtaccaccactgctggcgctcctttccggagttgaaccgcgcccagatgtcctccccgattgcctggtggtccgccaggatggacagcaagttgtgcagcttgtccgccgcggagatcagcacactgccgtcgtcggaggcccgcaggtgctccaggtacgcgtccgcgcgggactgccaatcgggcagcaaggaatccttcgtcacaccgccaacgagttccacgacccgggggccgaaatctgcttccatctcctcggccgaatactcctccggcacgtcctccagaatgtcgtggaagagcgccgcgatgagcacgtcctcgtcgtccgtgacttcggagaccaagtgcatgacgccgaagatgtgcgagatgtagggaatgtcggtgcccttgcgcacgtggccccggtgcgcccacgcagcggtattgatggcgcgaatgaggcgcggcgacgcggtgaattctttgttgaagctcgtggtgtttgtcatggctcgtatgttacgtccccacctctacacgccagcttcacgtgacgaacatatgttcgaacgaataagcgaaacaaaacctccagctcgttgttgaaccggaggttttgccttgtaccccgtacgggatttgaacccgtgttaccgccgtgagagggcgacgtcctaggccgctagacgaacggggcgcgctcgcttgcttgcgactccacaacaatatggcacgcgcgccgcctccaacaaatcgccaggccaacagcatttctcgacgagaacctttagaagaaaacggtgtactcgcgctccataaacgcgccgctgccggtgcgcgcgtcccagcacgtcaccccgacctcttccacagcacagaccatctcgccgaagtacaccacgtcgccgtacggcacgacctccggcaccagcgtgtcggtttcaccgaacgcgccctcgaagtatgccggaacgtcgcccttcgccagcgcctccccgtttacgacgtcgatggcccacttcgccatgccgttcggcaacgtgcccatcgcgtggttctcgttgtacgacagcaccccgcagtacatcgaccgcgcatccgcaccgtcatcccacatctcgcagccgatgttgccgctcggcgcggtgaacaccccgacgtcgccgtactgcgtgtgcttgaccgtcgcaacggggcgcgcctccggcggcaccggtcctcccgcacccggatacgcagccggtgcgcgagcgggcggctccggcgccgcctgctcgcgcgagggctcctcactcgccggctcctcgctctccggcgaggcagacaccaccacggtcgaggtctcggtttcgaccagcgcaggcgtttgctcgccggcacaccccgccaaagccagcggaaccgccaaaaacaccgccgacgcacaattcttcaggttcgcagctatgcctccttgtacaccagcggcgacgttaccgtcagcgcgacccggtcccccacctcgggtttcggcgtcagccccagccgcgcacggaactccacgccactcgcctccagcgtcacggagtacgagttcacctcgtagagcacggaagtcacggccgcatccaaggagctagtgcttgtcgacgcccccgtccccaccatctccggcaacaccgcgaccaccacgctctcaccatcgcgaagctcgtcatctgcctgcacgtcggcgacgggccaggacattcctagcgacgccacctcgactagaccttggcgcacgacgccgtcgagcaacgtggcgtcggcgataaacgacgctacccacgccgtcgctgggcgggtcacgatcgcttcgggggtgtcgagttgttcgaggcggccgtcgtgaagcactgcaatccggtcggcaattgcgatggcctccttgcggtcgtgggtgacatgcactgtggtgaggttggactggcgggtcagcgtcaccaactcgcggcgaagcgagtcgcgcagtggctcgtcgagggcggaaagcgcctcgtctaaaagcagcacctccggctccgcaacaatcgcccgcgcgagcgccacgcgctggcgctgcccaccggagagcgtcgcgggccggcgcttgccgtatccctcaaggccaactgttgcaagggttcgctcgacgcgctgcttttcctccgcgcgcttcacgccggctcggcgcagcgggtaagcgacgttgtcggcgacgctcatgtgcggccagacggcgtgctgctggaacaccatgcccatgtgccgcttctccggcggggtgttggacacgtctgtgccgccgagctcgatcgagcctgctgatggctcgatgaaccctgcgatggtgcgcagcagcgtcgtcttgcccgaaccggacggtccgacgagtgcgacgaactcgccgctcgggatcgccaggttgatgtcctctaagccaacggtgccgccggggaacaccactttcaggccgctgaccacaatgtcgctcatgatcgcctttcttccttacgcgttcttgccggggtttcgcacggttaacgccagcgccgcgataccgatcaccgcgaacatcagggcgagtgcggacgcctggttatagttgcctgactgctgcaggttaaacagctgcacaccaatggtggtggtgccgggcgcgaccaagaggatggatacagtcagctcgcgcactgcggtcaccgccacaaggaccgcgccggagaacaccgcgggcagcgccatccggccgctggtgtcccacacggcgcgcaaccggcccgcaccggagatttgcgcggcctcctccaccgccgccgggatcttcgccagcggcgcgcgcaccgcctgcagcaccatggccgtaaacgcgcagacgtaggcggcgagaatgatccagcgggtgttgtacatgccggtgtagcggccgacgatcacccagccgacgccgatgatcaaccccggtagcgccgacggcaggagcgtgatcaaactgagcgccgtgttcgaccgcgccctggtgcgcgttaccaaaataccgatcatccagcccaggacgccgcacgctagcgctgccccaagtgcgagcgtgacagagttgccgaacccctcgcgcacgcgcggattggccagggtgcgctggaagttgtccaacgagatattctccatcgtgaacggcacaccgggcgccggtagcagcgcgcggtaggtcaagccgagcagcggtccaagcgtcagcgctagtgccagcacccaggcaaccacggacacgggccacttggccgagccgagtgagagtttcatggtgccgccgccggagacggtcgacgtggcgcgccgcgacaccgcgtagtcagcgaccacagccccgattccgaggatcatcagcaccgcgccgactgtcgacaccacttgcagcgggttggccaccgtccccgattccataaaccggtagaccatggtggcaagcgtttcgaaccgcacaggcgagccaaggatcgagggaataccgaaatctgccaggttggatactgccgtcagggtaaacgcgctcagtagcgccgggcccagcagcggaatggtgacggtcttcagcaccgtgccgctgcccgccccgctcacgcgcgccgccagctccagatcggatggaatggagcgcaacgccgcggacacgatgacgtacaccaccgggtacgaatgcaaaaccatcaggaagatgatgccgtcggcgccgtagatgtcccagatggggcggccgaagaccgcgttgagtccctggttgcgcccgaacagctgcagccacgagatcgccccgacgaacggcggcacaagcagcggggacagcaggaacaaccgcagcgcggtcgcgccggccacgtcggtgcgctcaagcaggatcgcaatcgtcccgcccacaacgacagcgccgacggacgacagcagcgtggtgtagacggagttccacgtcgccttgcccaggccctgctcaaccagcaccggaaactggttgcccccgagcgccagcgacaccaccatggcgagcggggcaagaaacatcgccgcggcaatcagccataccccaatgcgggcgaggccgatacccggcgagaatcgtttggtcacgcgtgaacctagttcatcgcgttctggaagaagtccaccgagcgctggcggtccttggtcagggtctccaggtcggtgctcatcagcgcgatgtcgctgagcttcggcgcgtcgcccggggtgccgacagactcgatcaccggcaggtagttctgctcgacggcgatcttctgggccttctcagacaggatgaagttgatgtagcgctgcgcggcgtccttgtgctccgaatccttgaacacggcgatcggctcggtgatgtacggcgagccttcggtggcgtaaacctccttgatcggggagcccttcgctgcgaggtcgcgcaccaggtagtcgacgacgacgcccaccgggtggccgccagaagcgatctcctgggaggtcgggccgttggatgcggcgatcatcgggtggtttgcgccgaggtcggtcacccacgcctcgccgagtttgtcgtcgttcatccacacagtcgcgttgaaggcggctgcaccggagacggccgggtccggcatgacgatcttgtccatgtacttctcgtcggtgaggtcagcccacgacgccggagcgtcagcctggtcgacgacgtcggtgttgtaggcgataacggtcgggatcaggcgggtgcccacatagaacccgtccgggtcaaccacttcctcgaggacatcgccggtctcgacgctgtcgaactcgctcaaaaggtcgtcgctcttaaaaccctcgaacgtcggggcatcggccgcccagatcaggtcagcctcgaccttgccggaggtgcgctcagcctcgatgcgggccttcagatcgccagtgccggcgcggtacacctggacctcgacgtccgggttctcctcctggaacgcgcggttgatctcgtcgaccttctcctccggctcggaggtgtagagggtcagcacagtcttctctccggaggcggcggcggtggtcgcgccgtcgttggccgcagtcgtcgcggagttgtctgcggacggctcggagcaccccaccagcgtgagcgcggcggtgccgaagattgcggcggcagagagggacttgttgaggaagctcatgggggtctccttgcgtcaggtgaactaaggctcagccaaaagtaacaccgttgccccgcacgcgcgcgccgagcagggggcgagctgacgaaaagaaaaaacctccgggcttctgcgtggagcagatgcgccggaggcttgttgtaccccgtacgggatttgaacccgtgttaccgccgtgagagggcgacgtcctaggccgctagacgaacggggcaaaggaccaagatcaacgtttcgatcttgtcgctggcctaccaggactcgaacctagaatgacggtaccagaaaccgtagtgttgccaattacaccataggccattcgttttccagcgacttgcgctcgctgaacaacgttgaacactataaccacagaccgcaaacacgaccaaatcgccagctcaaaggacaattcggccgagtcacaacggtgtgattacccggcgattattccgccgcgaacggggtctgctcacgagccgaacgaaggcgggccagggtcgagtcgcgtccgagcagctccatggactcgaacagcggcggagagaccgcctctccggagatgccgacgcgcagtgcgccgaaagcgacgcgcggcttcagcccgaggtcggtgatcagcgcctggttgagcgccgcctcgatagcttcggtcttccactcgtcctcgctgatcgcttcgagcgcggcgataccagcatcgagtggggcaaccgccgcttccttcaggtttttcttcgcggccttgtcgtctaggacgaggtcttcgtcggcggtcacgaggaacttcagtagcccgtaggcgtcggaaagcaccttgatgcgcgtttgcaccaggtccgctgcgaccgcgaacttctcatccgggtagtcggccgggaaatcggtgtattcggtcaggtacgcgcgcagccggttcttgaagtcctccggctcaagcaggcggatgtggtcggcgttgattgcctccagcttcttctggtcgaaccgggccgggttgcccagcacgtcggagacgtcaaaggcgccgacgaactcctcgacgctgaagatgtccttatccgcagacagcgaccatcccagcagcgcgaggtagttgatcatgccctccgggatgatgccgttgtcgcggtggttgaacaggttcgattccgggtcgcgcttggacaacttcttgttgccctgccccatcacgaacggcaggtggccgaactccggggtgaagtccgcgacgccaatgcgcttgagtgcctcgtacagcgccatctggcgcggggtggacgaaagcaggtcctcgccgcggagcacgtgggtgatgcccatcagcgcgtcgtcgacagggttgaccagtgtgtagagcggcgcgccgttcgagcgggcaaccacgtagtccggctgcgtttcggacttgaaggtcacctcgccacggaccaggtcgttccaggtccagtcctgctccggcatgcgcagacgccacaccggcttgcggccctccgcctcgaacgcggcgatctgctcgtcgcttaagtcccggtcgtagttgtcgtaacccagctgcggatcgcggccggcggccttgtgccgctccgccacttcctcgttcgtcgagtacgccgggtacacctcgcccgcctcaatcagcttgttcaggacatctttgtagatgtccatgcgctgcgactggcggtacggctcgtgcgggccgccagtgacaacgccctcgtcccaggtcattccgagccagttcagcgagtcgatgatcgcctggtacgagtcctcggagtcgcgcgcggcgtcggtgtcctcgatgcggaaaacaaacgttcccccgctgtggcgggcctgcgcccagttgaacagggctgtgcggaccatgccgacgtggggggtgccggttggtgaggggcagaatcgaacgcgcattgttccagcttgagtcatagccttgatgctacaggccgggaaatgcgcggcaacgacccgctacttcgagtggcgggaaaggaacgcccacatctcgtctgccgccgacggcgagtaccaccagaagtggttcgagccgtggacctggatcacctcgacgcccttggcgcagccgcgggcagaaacccgcgtggcgttgctgcccaccggcgcgcggtcgacggcgccggcgcagcggttgcggcgctcgtacgacacgaacatctccggcaccgggatcacgcgctggcctcggcggatggtgccgtagtacggggtgagcccgtcgctcatgccgtggatggccatgaacgcgaccggaatgttctggcaccccatgttcaccggcgcatagtaagcaccggatacgcccgcgacacccgcaaagaggtccgccatgtggcacgcggagaccgcagccatgccgccgccggtggacatgccggtggcgtagatgcggcggcggtcgatgttgtagtagcgctgtacgtcatcgatcatggcccgcacaaacgcgatgtcttggcccgggccggtcgccgcggtcggcgagccctcccaagaggcgccgattgcgcgagggtacacgatgattgcgtcgcggccgacggaggattcgcgcaggcgggagtagttgcggaagttttcggtggagtcctggtacgccgagtagccgaccatcaccggggtcgggtttgccgggttgtagttgcgcgggacccagatcaggtagctgcgaccggcggcccagatctcgccgttgcttccgttggcaacgggagcaggtgcttgttgacgccacgggccaacctgagccggcgcggggatgggagccggcgctggagcacccggcagggaggaaccagccggcagagagtcattcgccatctggacaaacttgttccactctgccgtagcttggccaattgctgcgttggcatcgcgggcgatctgcgacgacaagtcctgcgcctgcgcgggggccacggtaccggacacaagagcaatggccgtggcgacgcgcgcgagtgcgcgtgtaaatcgagcgttcaagagcgggtacccttccccagcaacagtcacaggaataacacacgtaacagtactgcagcgctcagcgagcaacaaccggaagcacacgcctgcgacaccgcaccgcaagttacactgattcaccgtgtcacccgccccccagtccgcttctgcaccggcccgccccgactccgctcccgatttcctgctctcgcggcaatcgggatcggtgcgcacacagggcagctcagcgacgtttaacaaggtcgaggatgcggtcgaagcgctgcgccaaggcgacgcagcaatgattgtgggagcgctaccgttcgagcaggcctgctccgcggcgctcacagtcccgcagcgggtcatcgccgaagccggcgcgctgacgccgcacccctactacacgcacggaccggggtcgctgctttccgcttcaatcgcgggcttcgacccctcgccggcggagcacctgcgccgggttgaagccgcggtgtcgaccatccgccgctcgtcgctggacaaggttgtcctcgcccgcgccgtggacatcgccttcgatcccccagtcgacccccgcctggtcgcggcgcgcttgatcgagctctcggcggcgcgcgacggtttcatcgccgatctcacgcccgccgggcgacgcggtcacttcctcgtcggctcctccccggaggtgctggtaaaacggcagggcaaccgcgtcacctcgttcccgctggccgggtcggcagcgcgtgtgaccggcgacccccaagccgacctcgctgccggcactgccctttcgcagtcggcgaaggatttggacgagcacgcctttgtggtcgaccacatccgcgcgcgcctcgccccgttgtgcaccgagctggccgtgccccaggcaccgatgctgaccaagaccaacgaaatgtggcacctcgccacaccgatcgagggcacgctgaaagatcccgcccccagcgcgctcgaactcgcgtcgctgctctaccccaccccagccgtgtgcggtacacctgtgtccgcggccgaggcgctgatcaccactgcggaatcggaacgtggcttctacgcgggcgcagtgggctacaccagcgccgacggcgacggcgaatacatggtggcgatccgctgcgccgaggttgacggcgagggccgaaccgcccgcgcgtgggctggcggcggcctcaccgccgattccgatcccgagtccgagctggaggaaacctcggccaagctccgcactatgctgcgcgcactcgggctgtagcgcccaagctctacagtctgcctaggcggattcgaccgggttgcccagcttgccgatgcccgggatctcaacctcgatgaaatcgcccggcaccatcttcgcggttcccgcgggcgagccggtggccatgacgtcgcccggcagcatggtgaaggactgcgtgacccactccaccatctggcctatgttcagaatcatctggttcgaattcgagtcctgcttggtctcggtcacaccgtcgtgggtgaggtgggccttgatcggcaggtcggagaagtcgaacttgtccagatccgtctcaatccacgggccgagcggaccaaaggtgtcaatgcccttggcgcgggcccactggccgtcggcgaactgcaggtcgcgcgaggagacgtcgttgatgatggtcacgccgcgcaccaccgagcgccattcttcagccttgacgtttttgcagggcacgccgaagacgacggccagttcgccctcgaactccacgccggtggcgaagtccgggatgcggatcggcgccccagggccaacaactgcggtcgacggtttgatgaagattgtcggcggcaggtgctcggcggactccttgaacacttcggcgacgtggtcggcgtagttgcggccgactgcgacgatcttgctcggcagggtcggcgcgagcagcctcacgtcttcaagcttgtactctttgccggtgtactcggggtccgtgaacggggtgccagcgatcgctttcgcgctcacgccctcgtcatcgatcaccgcgaacgtcatcccgtctggtgttgcaattcgtccaaaacgcatggttcaaaagcatacagacttgtacgtggcgcgagtcacgttttctcagcgcttgtttgccgtcagagcgaggtagagctcggcgcacgcgatcgcgtcagtcagcgcgttgtggttgcggtacgcgggcaggttgtagcgctggcgcacgcgcgcgagccgcaggtcttcgccccgcgggtacgtgcccatccgctccatgtggcgccgctccatctccatcgtgtccagcacctcgttcgccccccacttcttcttcaccccccactggtcccggtaaagctgggtgatgaacccggtttccatctgggcgaagtgggcaagcaggcggtggccgccaagtgccgcgtcgaggcgctccaaaaccagcgagtggtccacgccgaggcgcgccacgtcgtcgtcggtgaccccgtggatcacggccgattctccgatgcgcacgccagaaagaatgtggtactcggcttgcgacaggtcgatgactctgccgcgcacgggcacccagccgatggagacgagcgcgtcgcggcccggtttgagccctgtcgtttcgacgtcgacggagaggaggggtgcgtcgtcaagcaagcccttgcccttgaaaaacccgagcacgtcacaccgcccgtgtcgggtacttgttggccaggccgttttgcatggacttgatcacgccgaacgcgtcgcgaagcgcggccttgtcccgctccggcagctgcttcgggtcgatgtggtaattcggcgcctcacctgcgcgaacttgcgcggcctggtggcgcatcgcggcgtcggaaaggtacgtgtaggcgtcgagcaggtccgccgcccccttctccgacaccgtcgacccggccgccgcgcgcagtctcgcgtcagtctctacctcgtccacgcccgcggtcagcgcgtagagccgcgccatctgcaccaccgccgccgtgccgccgcgcttgatgtcgagcgttgccgcgtactcgccgctgcgctccaccacgaacccgcggaagatgccgatcggcggctcgcggaaggtagccagcgccgcgaggtgcgtgtgcaggcgcttcgaaccgcgggccgaggaaagcgccgccttgcgtatgccgtcggccatctcgcgccacccctcgccagcgccggcgaccgcccggaagtcgaagaacacctgcgcgtgcagcagcgcgttcgggtccggcgcggtcacccagccgtggaacgccgccgcccactgcgacgccgtcatccgccacgcagggttcgacgccatcatctcgcccgggcacagcgcctgccccgcgtgcgcgagaccctggcagataaactggccaagatgtgcgaagtattcgccgtgcgtgtccgggtcaaaggaatccgccagcaccagcgcgttgtcctggtcggacgcgggacccatctcggacctggcctgcgacccaacagcgacaaaggcaaagggaacgggaggggcaccaagcttgtcgacgcccacctcaaccaacctccgcgccacagcatccgcaatcgcggtgagcaaccgctgcgcctccgccgcggacgcgccgcgctcgaagaaccgcaccgccaccgccaccgcccgctggtacgctccggcgagctcgtcgtagctggcccgccccacatccgcggcgaggtagatcgggtccgtctgcaacagccgcatgaagtcggaggagctgataacaccggtgatggcgtcgtcgcttctcaccggcaggtggtggatgcccgcctcgctcatcgcaagcacagcctcgaagacgagcgcgccaccgtcgatagtgagcacaggtgtcgtcatcacctccgacaccgggcggtccgggtccacccgccgcgccaccacgcgtgcgcgcagatcgcggtcggtgaggatgccaagctcctctcccccgtcgacaaccaggcacgagacgcagctgtcctccatcaactgggcggctgcggcaatcgccgtgtcgggcccgcaggtcacgagcgcccgcgccgccgcaacatcgctgaccggtgtgcgcagcacgtcggccgagcccaggtcctccacctcttgcgcggcggctcgaacccggcgcgacgccgtctggaagaagcggtgcatgtccgggtgcgcggcgagcagctcgtcgaacgcctgccgcggcaggatcatcaggacgctgtcttccaccgcctgcatgaggtagcgcgactcgggctcgcccacgagtgtggagtagccgaagttgagtccttcgccgcgcctgtccagcagcgtgttgttgtcgcccacgatgtccacggcgccggagcggatgatgtagagcgagtcgttgcgctcgcctggtgacacgacggcgtcgccgcgccgaacgtaggtgatgcccatcttggccggcagggcgcgcagcgtgtcgtcgggcaggtgggtgaacggctcatgcgcggcgatgaaccggtagacctcgtcgagttcgactgacatgggccaacactagcgcgccagagccaggcgcaaccgggtttttggaagacagcccgctactggtagctgacgaaccaggggcgcgggttaaccgtgttgtaggtctcctccggcgtaaaggttggggtgtcctcgtcgatgaagttcttccacgccatgtagtagttcgggtcgaggccctcgcgcagcacgttccaggtgtcgaacttctgctccggcacaccgtggccgtcggcgtggagtacccacgcgagttcgggctggccggtgcggatgttttcccggtccgggtacatggcaagttggaactggtggaggatcagcagcttctggggcaggttgttgtcgcgcacgagacccgcgagccagtccgcgaccacgttaatctcctcggcggtggcagagccgatgcgtgacaacggcgcctcaccggggttgagcttccactccgcgtccagggcgaggcccacgttgggccgcttcagcaggtcctcatacatcttcgcctgctccaggaagcttccctggcccggctgcaagtccagcacggcgtagccgcccgcctcaagaatcgcgtcgacgtacgggacgatgtcctccaccggggtttcgttggagtagttgccgtcgtcgccggggtactccgaagcgaccgtgacaatgacctcgaaggctgggatgaccggctggtcgtccagcggcgcgtaccaggaggcgtactgcttggccagctccgcggcctgcgccgggtcctgctcccccatcacgccgagttctgggccgtaggggtggccgtagagggcgaccatgcgccgacccgggaagacgagaccgccgccgccgggcagctcgccgttgccggccagcgctactcgcgactggtagttctcgttcgagccccactgccgcccgagggcgatggtgtcctgcgaggtgacagtctgaatgctctcgtgagtgtcccgcgggtctgcgacgcgcaacacatcgacgtctgcgccggcggccttagcagtggcgaccgcaccgcgcgacgacaccgccgtggcaaacaccgggggcagcacgagatcgaccgggttggcagcttcctgcgcggcgatcgccgcgatgtcgcccgccgggtccgcgctttccaccgtgccggcggcctcgatctcctcgaggtagtcctcgtccgcggcaggcagctcgatgacgcgcgacgcgcctaagcgctccacctctgcgtcgaccacctcttccgcgcccgactgcttgaccagcatcggggcaccgagcgagatagcgaccgcagccgcctgcatttgggtgtcgcggtccggcgccgagaccactaccgtctcggctgtatcgaagaaccgctgcgagacctccgcaccggtgccgtccgggtcctggatgacctcggagccgtccattggaagacgcttctcttcgtccctcgccgcaccagcgtcggcgccgccaatgccttgcccggacgagcaggccgtgagcccgccggcgagcaccagcgaagtggacgtgaggatagcgattgcggtgcgggagaaagccatgcgctcgaatctatcgcagcgcggctgcgatccggtcaccgacttccaccgtgcggaccgccgagccgccgcgtgaggcgacgtcgtcctcgacagcctgctcgatacgcgccgcgttgtcctcgtcgtcgaggaagcgaagcatcatcgcaaccgacaaaatcatggcggtcggatccgcgatgccctggccggcaatgtccggcgcggagccgtgcaccggctcaaacattgacggcgtctcgcgcacggcgttgatgttgcccgagcacgcttggcccacgccgcccgccacggcaccggcgaggtcggtcaggatgtcgccgaacaggttgtcggtgacgatcacgtcgtagcgcgctgggtcttgcaccatgtagatcgtcgcggcgtcgatgtggttgtagtcgacctcaacctctgggaactcggccacgacctcgtcaaccacgcgctgccacagcccgcccgcgttgaccagcacgttggtcttgtgcaccagcgtgaccttcttgcggcgcgtcatggccagctcgaaggcgtagcgcaccacgcgctcgacaccgtggtaggtgttctgcgacacctcggaggcaacctcgtggggcgtgccctggcgcaacgtgccgccgttgccggcgtagagaccctcggtgccctcgcggaccacgacgaagtcgatgtcgcccgggtttgccagcgggctcgtcgacgtcggatagagcctcgacggtcgcaagttcacgtagtggtcgagcttgaagcgcagcggcagcagcagaccgcgctcgagcacgccagccggcacacgctccgggtcgccgacggcaccgagaagaatggcgtcgtgctccttcaggctggcgaggtcagcgtcggtgagcaactccccgttcttcaggtagcggcgcgcgccgaggtcgtactccgtggtctccacgtcgtcgcggacggtgtggaggaccttcaggccctcggccatgacttcggtgccgatgccgtcgccggcgatcactgcgattttcattaaatgagacgcctttcctactggatggaatcgttaggtgtgccttgagggtagcagtaaacccccagccgccctgccaaatgaggacgaaactgggggccggttcggtacttcgaactagtccaggtcgatttggaccgactgcgcgtcaatggactccgcgatcgagcgctcgagctcctcaggcacctcggactccacgcgcaggatcagggtcgcgccgccgcccttggtggtctgggtgagcgcggcggcctcgatgttaatgccagcgtcgccaagcttggagcccaccttgcccagcgcacccggggtgtcggtgtagcggaagaagaggttgcggccctcagcccgcatgtccacgccgcggccgttgatgcgcacgatcttctccacgccctccaggcccgtcaaagcgccggtcactgtggaggtttcgccgcctgcgccaaccacctggacctcgagggcgctgcggtgcgcgcgcgcctcggtctcggtcgcggtggagtagctcaatccccgggcttcggcgatcgaaggcgcgttaacgaaggtcaccgggtccgagacgatgcccgagaacaggccgcggacggcggacaggcccagggtttcgacgtcctcggtggacagctccccgcgggcggtcaccttgagcgccaccggcgcgtcgtcaagcagggtgcccgcaagaaggccgagcttgcgggaaagctccagccagcgggccacctcctcgccgacgcgacccccggtgacattgacggcgtcggcgacgaactcgccggccagcgccttgagcacagagtcggcaacatcggtgccggcgcggtcctgcgcctccaccgtggacgcgcccaggtgcggggtcaccacgacttcctcgagaccaaacagcggcgagtcggtgcacggctcggttgagaacacgtcgaagcctgcgccgcggatgcggccggccttgatcgcgtcggcgagcgcctgctcgtccaccagaccgccgcgggcggcgttgatgatgatctggccctgcttggccttggagagcagctcggcgtcgaacatgccggcggtctccttcgtcttcggcaggtggatggtaacgaagtcggcgcgcgccatgaggtcagtcagctccaccagctcaacgcccagctgggcggcgcgggccgggttggcgtacgggtcgtaggcgatgatcgtggtctcgaacgcgctgaggcgctgcgcgaacagctggccgatgtggccgaaacccacgatgccgatcgtcttgccgtagatctccacgcccttgaacgcggaacgcttccactcgccgtcgcgcagcgtcttgtccgcggccgggatttggcgggcggtggacagcagcagcgcaatcgcgtgctcgcaggcggagtggatgttcgacgtcggagcgttggccaccatcacgccgcgttcggtggcggcgtcaatgtcgacgttgtccaagccaacgccagcgcggccgatgatcttcagcttcggcgcggcctcgatcacttcgcggtcgacggtagtcgcggagcggaccaaaagcgcgtcagcctccggcactgcggcgagcagctcctcgcggttcgggccgtcaacccagcgcacctccacggtatctccgagagcctcgacggtggattgggcgagtttgtcggcgatcaggacaacgggtttagccacggggacactcctgcaattacgtaaaaggaacagttaccccgatacattagtgcgctggcgttggccccgccccgtcgtcaagcaaataagattcttccgcctgcataatctccgctcgtagcttgtcgtccggaccgaactgcgccccgagcgcaacaagcgggaggtccgccagccccgccatcgcgaacagcgtctcctctgacgcccgcgggtcgggatcgtccaccacaaccacgtcggcgccgaagctgcgcgcgttggcgacggacgcaatcgaactttccgcagtcgcgacgaccgcgggggccatttgcgcgtcacggcgcgacatgatgggaaacggcttcgcctctgcccccttcatcaccgccggctcggcccacgtagcccgcagccaggtcggatcgcgcgggtcgagggccgcaacctcggcgacagcgtccgcggggtccgacaccgggcgctggttaaaccgcacggccatcatcacccccagcgctgcggggccgcctggatcgcggtagacccgcacgcgcccggaggtgcgcgcgagcgagacgtcgccgacggtcagcacggtgtgggtgcgcagcctttccacctcctgcgagatctcctggtgccgcgccgggtcgtacacaatcatcggagcgtgcgcagcaacagcaatcgaggcagcccgcagctgcgcttcaacggtggcgtcgctgacaaccagcgtttcggagttgctgaagaacaggcgcagcgacgcaacgccttgcgtgtcgtcgaccacgacgggccgctcctcgaagcgctcggccacgtggcgggattcgttggtggcgattgcgcgctccagcgggttgagctcccgcgtctcggcgcagcttgtgagcgcggcaagcgccgccagcgccatcaagcaggaagcggcgcgcctactcgccatcctgctcctctggcgcgctatcccggatgaccggcttgtccatcgcgtattcgatcagggagatgaaacggcggcgtcgataagcaacaaagccctcccagtccgaagtaaccaggtctgcaggtgagatctcgtgaccctcgatgacctggtcaaactccgcgtcgtcgagcagcgatttcgactgcagcctgggcaggtagcgcttcggctcgttattctcgatgaccgcctcggtgcgctgccccatcggcgtgcggttgagcacgcttcgggcgacgtccggatccgcgccgatgctggcgcaaaacaccggcgggaacacggtgtgaaagcgcggctgcagctcagcggccgtgtccttgtcaaaacgcttgccggtgcgccaatcccgcgcgccgcgggccatcaacaacgcgaagaggccgcggtagacgccgctttcctccgtggcggaaaggaggcgctcctcgttgaactgcgcatcggcaacggtgcgcggcatggtgtcagtctcccccagcacccacggcgtgacctgctcaacgtcgagtgccgcgcggatcgtcggcgagtgcgccccgtagagctcgccgaacacgccagaccagaaccagcggtgaaggcggtcgcgcgagtcggtgttgtccagcgcgcctgggtgctcggccagccgggccaggatcgtggccaacggaacaatttgcgacgcgtagggaacctgctccgcggtgagaatcgcgcggtcggcgagaaaatcagcagcctgctcgaaagcgtgcgcgagctcgtcggcgtgggcgcggtactcctccaaggaaatggtgaggatgtcgccgcggtggccggttgcctggccgtggcggctggagatcagcatggcaagggcgcggagaaactcgacgcggccaatacggtcgagcgccgggtgctggcgcaaacgggcttccacaccggaccagtgctctgccagcacgaaatgctcgtcctgcgtggcgaacatcgtggtgagcagatcaaagacgtccatctgcacgccagcggaattcgcgtgggcgaaaatctggcccaccccgacctgcgaggtggcgcgctcaacgcggatcaccggaatgtcgtaggccggcagcgtgcgcatcacgccgttttggaagatcttcaccgcctcgcgcatctcggcgcagtccgtgcccgcggccatgtcgatgagcaggtcgctaccctcgcgccacaacagctgggagacgggcaccacgccgtagcggagcatgtcctcccgggaggtgataccgctgtcgatctccgggccgaagtgggagcggacgttgccctccaggtcaaccgcgaagacggactccaccggcatcgggtcggaagcgacagctgcgcgcacgtccacgaaaaagcggcgctcaatccgctcgccgcggtaatcaacggtagggatagtgccgtcgccggtgaacgcgtggaagagggaggtcagtcgctgctgcccgtccaaaagcagaagccccgggtgggtgccgtgcgcgtcgataccggtaagcgggcgcggccggaaacgcaccggcgagttgcgcgtgtccaacgcgagaaacgatccgaccgggtagccgcgcagcacggacgtgatcagcgtgcggatccgatcgacgtcccagatgtactcacgctggaaatccggcagctgcaactcgccgcgttccgcgcgcgcgaacagatcaatcagtgaataactcggcgtggtaaaccccatgcctcaaactgtagaacacatccccaacacgagctggctagcaaatcctctcgtggcccacgtgctctgggcgttccagctggatggtggagtggtcgacaccgaggttgcggagcgcgtgctgcgcgtcgtccaacagcccgccggcatctgcggcgtcggacacgacgaggtgcaccgtggccagcacatgggaaccgtcgagcgaccacaggtgcagatcgtggacaccgactaccccgtcaagggcgcgaagcgccggctccaccctctcaacgtcgaaaccgtgaggcacctgttcaaggagcactttggcggagttgcttaaaagctgccacgcccgcgggatcaccagcaccgcaatcacaagcgacgccaccacatccgctgcccgaaaaccagtaacgcgaatgaccacagcggcggcgataaccgccaccgacccaagcatgtccaccaccacgtgcaggaatgcgccctcgacattcactgacgcttcccggtggcgcgagaggatcaacgccgacagcgcgttcgccaaaagtccgatgaccgcgataaccagcatcgtggacgcgtcgacatccgccggcgctttcaaccgccgcagcgcctcaataacaatgaagaccgaaatcacaatgactgtcaccgcgttcacaagcgccgctagcacctcgatgcggcggtagccgtaggttgcttgggcagttgcttgccgacgccccgccatcaccgctaccaccgcaatgatcaaccccgccgcgtcggaaagcatgtgcattgcgtcggccatcagcgccatagaaccggagagccaaccgccgaccagctcggcgacaaacaccacgccggtgacggcgagcgcggctgacagcgcgcgcagcggcgtggattggctggggccgtggtggtgatggtgacctgtactcatggcaacagagtatacggcggaatgatcactattgaaaaagatttgaaaataacccttcggtccgtatcgccccacgagctgggaaaacaagcggggcgcgcagcaaaaggtcggcgtgcctcgttctcaattctcaaagttttgctaccgtggtttaccgaaggctaggttccagctcgcggctggctcctaatcagaattatttattacgaaaggaagctagtcaatgactacccctaacccgaacgatccgacccgcaacatcgacccgaagaacgtcgacccgaagaacgtcgacccgaacctctcccacgagtcgacctcccgccgcgtcgagaccaccccgaccaccgagcgcgtcaccacccagcgcaccacctctacctccggctccaccgctgtgaccccggaggagaacaacaacggcggcggctggtggaagtggctgatcggcatcctcgttgccctgctgctgctgtggctgctgtggagcctgttctccgacaacgacggcgacaccgacaccacctcctccaccaccactgctgcgaccgaggttgtcgacgagaccaccaccgtcgagtccggtgttgagaccgtctccccgaccgctgcggacgagaccctgaccgagaccaccgttgtcgacgtcaccgacaccgtcgcgccggcgaccaactaacagctagcgcctcttcgcaggcgcggcgctttccccgctacggtttcggccgtggcggggatttttttgcgcgccccactctcggtgatagcgggtaactccgcagcagccggtgagcgacctgcggaaacgctagatccgcaccgagttacccgctatcaccgtccgacatcaacaccatttgtacccagacagacgaaaatcccgccggccacgtggccggcgggatcagcgttgagcgagctacttacgcggtctcatcgagcgggttcttgacccagctcatcatgtcgcgcagctcagcgcccgtcttctcgatcgggtgctgggagatctcggcgcgcaggccctcgagctcggtgttgccgttctcgacgttgttgaccaagcgccgggtgaaggtgccgtcctggatgtccttcaggatctcgcgcatgcggtctttggcgctctcgtcgatcacgcgcggaccggagaggtagccgccgaactccgccgtgtcggagacggagtagttcatgttcgcgatgccgccttcgtagatgaggtcgacgatcagcttcatctcgtgcaggcactcgaagtacgccatctccggctcgtagccagcctcgaccagcacctcgaagccgttggtgatgaggtactccaggccgccgcaaagcacagcctgctcgccgaacaggtcggtgacggtctcagcctcgaaagtggtcgggatgacgccagcgcgggcgccgccgattgccgccgcgtatgacagcgccaggtcacggccgttgccctgcgggtcctgctcgactgcgatcagacacggaacgcccttgccgtcggcgaaggtgcggcggaccaggtggcccggacccttcggcgcgaccatggcaaccgtgacgccctcggccggctcgatgagcttgaagtggatgttcaggccgtggccgaagaacagtgcgtcgccgtccttcaggttcggctcgatgtcgttcttgaagatctcagcctgggaggtgtccggagcgagcagcataatgacgtcggcccatgcggcagcgtcggcgttggacttaacctcgaagccggcttccttcgccttggccgcggacttggagccctcgcggagaccaacgacgacgtcgacgccggactcgcgcaggttctgcgcgtgggcgtggccctgggagccgtaaccgatgattgcgaccttcttgccctggatgatggacaggtctgcgtcgttgtcgtacagcacttcaattgccatgagtggaacactcacctttcctatatattgggacgcttgtttcacattatgacacacccgcggtgtgccgggatgcaatagctcgtttttggctagttgtttttcctcgacggcgccatggtcttcgagccgcggttgagcgcgacctggccagagcggaccatctcgcggatgccgtaggtctcgatgacatccaagaacgcgcgcagcttctccggcgtgccggttgcctcgaacacgatggagtccggggacacatcgaccacgcgggcgcggaaaatgttcgcggtctccaccacctgcgcccggttctggctgttggcgttgaccttgactaggagcagggaacgggcgatggtggcgtcgtcgtcaagcctgagcaccttgatcacctgaaccaacttgttcagctgtttggtgatctgctcgatggcatactccgaggcgtcgaccacgatcgtgaggcggttgattccctcggcctcggttttcgcggagaccagagagaccaggttgtagccgcggcgcgtgaacagcgcggtcacgcgggtgataatgccgtcgacgtcctggacgagcaccgacaggatattgcgggtgtgttcgtcttcgtgagccattagttcgtctccttgatgtcgtcgatggtctcgctgatagcctccggagtttcgccggcggattcctccatgtcgaagaacgggcgcataccgagcgcgtactgcatatcggagttcgacgcgccggccgcgatcatcggccacacctgcgcgtcctcgcccacgatgaactcgaccacaaccgggcggtcgttgatctcccgggccttctcaatggcgggcgcgacgtcttctttcttggtcacgcggaaggcgactgcacccagcgcctcgctgagctgcacgaagtcgggcacgtaagccgtctccccgccgagcttggtgtgggagtaggtgccctcgtagaacaaggtctgccactggcgcaccatgcccaggttgccgttgttgatcagcgcgaccttgaaggggaagccctccatcgcggcggtggtcagctcctggttggtcatctggaagcaaccgtcgccgtcgacggcccacacttccttatccgggcacgcggccttggcgccgagcgcggccggaatggcgtagcccatcgtgcccaggccgccggagttcaaccagtggcgcggacggtcgaagtcgatgaactgcgccgaccacatctggtgctggcccacgccggcgacgtacacagcttccggtcctgcgatggacgacaaggtctcaatgacgtactgcggggagagcttgccgtcggactgctcgtcgtagccgcgggggaagcgctccttcagctcaccgaggcgcgcaatccacgcgtcgatctccggcgccgcgttgcgggacgagtcgcggaacgcgtcggtcaactggctcaacacgcgcttcgcgtcgccgacgatcggcacgtccacttcccggatcttgcccacttcggccgggtcgatatcggcgtggatggtcttcgcctccggggcgaaggttgaagtgtcgccggtgacgcgatcgtcgaaacgcgtgccgatggcgatcagcaggtcggattcctgcagcgcaccgaccgccggaaccgaaccgtgcatacccggcatacccatgtacagcgggtggtgctgagggaacgcgccaagcgccatcaaggtggtcaccacggggatgccggtgatctcggcgaactccagaagctctgcgtgcgcctcggcctttactacaccgccgccgatgtagagcacggggcgcttcgcctccgagatcatcttcgccgcctgcgcaatctggcggttgtgcggcttggcgttgggtttgtagcccggcaggtccaccaccggcggccactggaactcgatctccgcggcctggacatctttcggaatgtccaccaggaccggtcccgggcgacccgtggaagccaagtggaacgcggcgtagagcgcgcgcgggatatcctcgggggccgtcaccatgaggttgtgtttggtgatcggcatcgtgatgccgcggatatctgcttcctggaaggcgtcggtgccgatcagcggggagccgacctggccggtgatcgcgaccagaggaacagagtcgaggtacgcgtcagccagtgccgtgaccaggttcgtcgcgccgggacctgaggtggccaggcacacacccacttttccggaggcgacggcgtagccttcagcggcgtggcccgcgccctgctcgtggcggacgaggacgtggcgcagcgaggtcgcgcgggaaagcgcgtcgtagagcgggagcaccgcgcctcccggaaggccgaaaataatgtcgactccgagctcctccaaactgcggactacggcgtcggcgccggtgaggatttcgggctgcgcttgactgggtgaatcgtcgagcgcagtcgagggctttggtgaggctgccacgatgcaaagctccttactaggttccttcaggtttaaaaagacggcgatctcaaaaacaaaagcccccgagcgagctgtgtgctctcgagggcgcttgttgtgttgcggttagcgtgagttgcaacccgctacggcaagcgccgcaccggaattactactactgctagctgcgaagagatcatgcggctgatcatacacaaatcacagctgcgcacgcggcaaaagaactagaattttatgcactatgccttttgcgtacatcttcgagcaggcgtggcggtggctcgccgacaccggcatcaacctgctgattcttttgctcctcgctctgctcgtcccccgcgctggccggttcgcgaaccgctttttcgcgcggcacgtgaacaagtcctacgaccaagacgagagcaaaagccagctggcggtcaccggcgtggtggtctacatcgtccagctgatcgcgttcttcctcatcttcattttcctgctgcagcaaatcggcttctcgctcgcgggcgcggcgatcccggctaccgtggtctcggccgcgatcggtttcggcgcgcagaacatcatcgcggatttcctcgccgggttcttcatcctcaccgagaagcagtacggggtcggagaccacgtcacatttcaaggcaacgggcttgacgtaagcggagacgtcagccagatcaccatgcgcgcaaccaccatccgcaccatcaaccaggccaccgtcaccattccgaactccgcggcgcgcatctacatcaaccagtcgaactactgggtcaacgcgctcgtggtaatcccggtgccgttgctcggctcgcagtcggcggagcacgcgatcgagcgctccgagcgcgccgcccgccgcgctatcgcgcgcgccgacatccacccgagcgtcaccggcgaactgcaagtccacccggccgtcgaggtcaacccgccgtcagccgccggactgccgtggaccgtggacatgcggttcatggttcgcgtcgagccgctgagccagtggatggtcgagcgcgccatccgcgtggcagtcctcgacgagttctgggaggagtacggcagcgcgccagagcttttcccgcttgccgacgccgcgccttcctcccccacccccgaccaggagactcaccctccgaccgagcgcatggcgccaatcgctccccgcgccgcgataccgtccaccccgaccccagatcccacgcccgcgcccgcctccccaccgagcaccgccgtcgaggacgcggtccccaacaccgtgttcaacgggctgatgcgcgagagcaccatgtggctcctcgtcgttttcgccgtcacagtcctcgtccgcggcctcaccctcaccccgggcacggacagcgacgcgaacgccggcgtgcttgccccgccgcagcgcagcacggagataacctcccctgccgaggacaccgccggccccgcaactacgagcccgagcatcccgccgagcgagtctcacgctcccaccaccgagcccagccctaccccggagtccgagcccgcgacgccggaacctacgacgccggagcaggaatcccccgagacatctgcgcagccagagggcgaaccttcacgtgaatccgtggtttcgaccgccccgctgcgcggcatcctagattgaaccagcgtgttgcacgttggctagcatgacaaacatgaatgaggccaaacacgtctttcgcccatcccgcgaacacgtcatcgcgatcgtgatgatgatcggcatcgcgcttatcggcgtcatgtgggcgccaaagtacctggggtgggtgctggtccttttggccctccccatcgcttgggtctacaccgcctccaccacagtggatgaccgcggcatcgcaatgaaatacttgttccgcaagaacgcccgcgtgacctgggacgatctggccggcgtgtcgtttgtgggagcaaaggctctcgccaccacgaaggcgggtacggagtacccaatgcctggcgtaacattcaactcactcccagagctctccgctgcgtcgaacgggcgcatcaccgacgtgatcaccgaagcagcggaagccgccgacgggaagtacgaaatcatcgacaaagagggctacagcgtcttgctcgacgaagacgagtacaacgcgtacctcgaaaaacacccggatacgccgggccctcggccccgcaaaggagaaaccaagtgattccgctccgctcacgagtaaccaccgtcggacgccaggcagcgggtgcccgcgcgctgtggcgcgcaaccggcactgaggagaaccagttcggtaaaccgatcgtggcaatcgtgaactcctacacgcagttcgtccccggccacgtgcacttgaagcacgtcggcgagatcgtcgccgacgcggtccgcgcggcaggcggcgtgccgaaggagttcaacactatcgctgtcgacgacgggatcgcgatgggccactccggcatgctctactccctgcccagccgcgagatcatctcggactcggtggagtacatgtgcaacgcccacacggtggacgccatggtgtgcatctccaactgcgacaagatcaccccgggcatgctcaacgcagccatgcgcctgaacatcccggccgtgttcgtctccggtggcccgatggaggcgggtaaggcgattaacgcaggcggcgtggtcaagccgaagtcggaccttatcgatgcgatcgccctgtccgccaacgatgcggtgaccgacgcagagctcgacgagattgccaacagcgcgtgcccgacctgtggctcctgctccggcatgttcacggcgaactccatgaactgcctgaccgaggccctggggttgtccctgcccggcaacggcaccacgcttgccacccacaccgcgcggcgcgccctgttcgagcaggcgggctctcgcatcgtcgagctgtgcgagcgttactacggccagggcgacgagtcggtcctgccgcgttccatcgctaccgagcacgcgttccgcaacgcgatggccctggatatggcgatgggcggatccaccaacacgatcctccacatcctcgcggcggcgcaggagggcgaagtggacttcgacctcgccgacatcgacgaactctcccaccgcatcccttgcctgtccaaggttgcgccgaacggcgaagcccacgtcgaggacgtgcaccgcgccggcggcatccccgcaatcctcggcgagctgcgcaggggcgggctgcttcacgacgacgtccacaccgtcgcctacgactccctcgacgcgtggctctccgactgggacatccgctccgagaacccgctggacgaggcggtggagctgtaccacgccgcccccggcggtcagcgcaccaccgagccgttcagccagtccgctcgctgggaaagcctggacaccgacgccgccaacggcgtaatccacgacgtcgagcaccccatcacctccgacggcgggctcgtggtgctgcgcggcaacctggctcccgacggggcgatcctgaagaccgccggcgtggaggaaggtctctgggagttctccggccccgcacgcgtggtggattcgcaggagcaagcggtgtccatgatcctcgcccgcgaggtgctcgagggcgaggtcgtggtcatccgctacgaaggtcccgccggcggcccaggcatgcaggagatgctgcaccccacctcgttcctcaagggagccggactgggtaagaagtgcgcgctgatcaccgacggccgcttctccggcggcacctcgggcctgtccatcggccacatctcccccgaggcggcccacggcggtctcatcggccttgtccaggacggcgacattatctccatctcggtggccaaccgcgagctgaagctcgacgtcgacgacgaagtgttggcgcagcgccgcgcagagatggaggccagcgacaacccgtggacgccgaaccgcgtccgcgaggtgtcgaaggcgctgaaggcctacgcaaaaatggcgaccagcgccgacaagggcgctgtccgccaggttgattaaaaagggcgtgcgacctagaccacgaacgggttgacgtcggtggcgaaccaccagatcaacccggccgccgcgaggccgacgatcagccagatccagctagacgccagcgggcggcgcgcccaagagcggccgttgtccacgccgtacaggcccggtccggtgaactgaagcgtcagcgcgatgccgacaaggatccacggcagccagacgcttgcatcccacgcgagcacgttccacccgttcgctgaatcgaccaccgcgtgcagcgctgcgaacgcggtgaccgccaccgctaccgcggcggcgaccggggtgatcaggcccaagacgatgaacacgcccgcggcgagctcaagcgtgggcaccatgatggccatgccgttgccgaacgggtagttcgcgtatgcgctttccagccccgcgataccttcggacccgccgagacggaagaacgtgcgcagcgacgaaatgatcaggtacgcgccgaagcacaggcgcagaagcagcaacccaaagtcgatggtgccgcggccaactggggcgatttcctcgacaaccggctcagaggccacggagacctcctcgtagacggggtcggccggcgggatgtacaccggctcgcgctccagcgccaccgtttccgccggcgacgcagccggcgtaaccgtcgtggagacggtctcggtggtgacggtgtcgcccgccggggcggcgaactcctcggtgggtttgtagtcgggcacgttgtcgtaagcaaagtcgtctggggtcacgtcgcgcgtgttgtcttgagccatgtgtccaacgtatgcgaccctgctggtttgcttgggaaggtcttcggcgtgcctgcccaccaaggctggcgatggcctgtttccacgcctatcgcaccacaccgaatcctaaagggcggataccggatggcggatatgcattcgggaagcggcacatccgcccttcgatatccgcccccactcgcccctggcgcccgcgcctcccgaacaggtgggtttggccagaacgatgccaaacgtcttgggacgtagcggtcacccgctatacatgcgcgaaacaggccctgttatattctttcacccatgcaccggtttcgttggctagatacgcatgatgccgaaatttggggcaccgtgtgggagtttgtaacttgggtgcccgccgatctcgacgagcacctgaagagcacggagcggatggctctgacggactacctaaccttgctgtcgatcgcgcgggctgaggatcaccacatcacgatgtcgaacctcgcccacgcgacccgcatgtctccctcccgcctgtcccacgtgatggaccggctggaggaccgcggtctcgccacccgcacgcgcagcgagcaagaccgccgctcctctatcgcctcgctgacgcccgacggtgttgagttcatggtccgagttacccccgccgtggtcacccacatgcgcggaacgatttttgaaacggtgacggaagaagagctggatcagctcaacgccatcatgaagaagatcatgaagtaactttccccggtttcgcctctcggtgtgctttgttaacatctcttggctactttcacaccgatccgaaaggtttcacccatggggaaaacgctcaaggtcgccttggcgttagttggcttgttggtgggcgcgggattcgcctcaggccaagagacgattcagtactttctcgcgttcggctactggggcatcgttggtgccgtggtggcgggcctgatcatcatcttcgttggttcggcgattttccagctgggcagctactacctcgccgacgaccacagcgcggtgttcaacaacgtttcacgcccctgggtgtcgaagtacatggacatcgccaccatgttcaccctgttctccatcgggttcgtgatgatcgccggcgcgggctcgaacctggagcagcagttcggtttttccacatgggtgggcgcggcgatcatgaccgtcgtgctctttctgtccgggttcttgaacgttgaccgcctcaccgacgtcatctccttccttactcccctgctgatcatttgcgtcatcggcgcgttccttgtcacgatcgtgaacatgccggacaacattgccggcctcaacgagctagcgatgcagaacgtcaacgcgtcgggcaccttcgataactggttcgtcaccgcggtgaactacgccacgctcgtgatcatcatgggtgtgtccatgatgctggtgatcgccggctctcagctcaacccgcgcgaggctggcatgggcggcctgctcggcggcatcatcttctccgtcatgctgctgatcttggtgttcgtgctcttcttcaacatggagtacatcttcggcgccgacctgccgctgctcatggtgttcgacaacatgcacccggcagtgggtaccgcggtgtccatcgtgatctacatgatgatttacaacaccgcggtcggcatgttctacgcaatggcccgccgcctgacccacaagaacccgcagcgcttccgcccggtgttcttcaccgtggtcaccatcggcttcggactctcgtttatcgggttcgccgacctggttggctgggtctacccgctactgggctacctcggcctcatcctcaccattgtgatgggtgttgcgtggttccgcgaccgcggcaagattaaggacgagacgcagcgccgcgagcgcctggcagagctcgccgaaaccgcgctcgacccggaatcggacgacctcacccgcgctgagcgccgcgaggtggagaccttgacggctgattccaacgtctccgacacggagctgtggcaatcggtgcaggaggaagttgcggctgatctccacgccgacgattcctctcagttcaacctcgacgacgtgccggccctgaacccggattcggacgagtacaacggcgcgccggaatcgcgcggcgagaagatcgactggcaggcctacggcgagatgtacgagacgggcagttttccggccgtcgctccgaaggagaccaagtagggcgaagtaggtccggacggtttcgaagccgtcggcaatcgccgcggactacgtggcccttggtgtcttcgcgctgatggcgcgggcggcgcacacggtcacccgcaaagtgttgcttccagagtgttgcttccagatggtcattaaccgagtacccgtgccgatcccgatttcggcaacggcggttaatgaccttttggtagtcaccatgtgaggggtgctgctggtgtggcggaattctgccgcgcataatcgcgcgctgatggcgcgggcggcgcaaacagtcacccgcaaagtgttgcttccagagtgttgcttccagatggtcattaaccgagtacccgtgccgatcccgatttcggcaacggcggttaatgaccttttggtagtcaccatgtgacgggtgtgtctggtgttgcgaaattatgccgcgcataatcgcggaccattctgccgcgcataatcccgtcgatgatcccaaacagcccccgccacacatctcatcgtgcggcgggggcggtggtttttggtcgctaggaaagcttcttcgcgatcagctggttgacctggcccgggtcagccttgccctgggtcgccttcatcacggcgccgacgatcgcgccggtgaccttcttgttgccggccttgtacttctccacgatgtcggggttggcggcgagcgcctcgtcgacggccttctcgatggcgctgtcgtcgcgcacgacctcgagcccgcgggccgcgaccacctcgtctacgctgccctcgccggcgatcacgccgtccatagcctggcggccgagcttcgtggtgagcttgccttccttcaccagctcgaccacgcgcgcgacgtcggccggggtcacgccgagggcgtccagatccttgcccgcctcgttagccttgccgttgatgtaggacacccaccaggcgcgcgcctcatctggcgtggtgcccgcctcgacagtgtcgacgatcaggtcgagcgcgccagcgttgaccaggtcgcggaactccttctccggcagctgccactcctcctggatgcgggcgcggcgcacccacggcagctccggcagggtggcgcggatttcctcgacccactcgggtttcgcaatcaccggtgggagatccgggtcgttgaagtagcggtagtcgctcgcctcctccttcggacggcccttggaggtggtgccgtccttctcctggtagtggcgggtctcctggaccacttccccgccgtccgtcaggacggccgcttgacgctgcatttcgaagcgcacggcctgctcgacagatttcagcgagttgatgttcttggtctcggtgcgggtgccgaattcctcctggccgatgggccggagagacacgttggcgtcgcaacgcatcgagccctggtccatgcgcgcatcagatacgccgagcgccttgaccaactcgcgcagcgcgccgacgtacgccttcgcgacctcgggtgcgcgctcgccggcgccgatgatcggcttcgtcacgatctcaatcagcgggatgcctgcgcggttgcagtccaccagcgaggcagtcgcgcccgtaatgcggccagaggccgaccccaggtgggtgagcttgccggtgtcttcctccatgtgggctcgctcgatctcgacgcgccactcggtgccgtcctcgaggacgacatccaggtagccgtcgtacgcaatcggctcgtcgtactgcgagatctggtagttcttcggctggtccgggtagaagtagttcttgcgggcgaagcgggaagactcggcgatcttgcagttcagcgccagaccgatcttgatggcccactccacacctttggcattcaccacgggtagtgcgcccggcaggcccagagaaaccgggtcaatattggagttcggctcggcgccgaagtgggcggaggacgtggagaacatcttcgtctccgtggccagctcgacgtgcacctcgagacccatcaccgggtcgtacttttccagtacctcgtcgtaatccatcaggtcgtacgcagtcatgagtgacagtctaatcaccgggccgactcggtcgatgctcgccggtccttggacctaaagatcatcgccagcaccgcgccggagaggttgtgccacacggagaacacggctgccggcagcgccgcaagcggggtcatgtgggtcgccgcgagggtcgcggccatgccggagttctgcataccaacttcgatagaagtcgtgcggcaggcctgctccggttggcctgtggccttgcccgtgaagtagcccaccaggtagccgagcgcgttgtgcagcaccaccgccaggagcacgatgaggcccgcctgcaccagtttctcgcgcgagccgtagaccacgttggccacgatcatcgaaatcgcgatgacagagatccacggaaggaaaggcaagatggcgtcgacaagcttgggcgccacgaggcggatgacaaggccaagggtgaccgggacgaggaccatcttcacaatcgaggtggccatggcggccgccgagaccggcatgtgttggcccgcgagccacagcgtgagaagcggtgtgaagatcggggccaaaagcgttgacacggacgtcatagcgacagacagggcgacgtcgccgcgggcgaggtagctcaccacgttcgaggaggtgccgcccggcgcgcagccgacgaggatgacgccggcggcgatttccggcggcaggcgcaggacccaggtcagcaccacggcgattagcggcatgatgacgaactgcgccacgacgccgatgagcacgggcagcgggcgcttgaccacttcggcgaagtcgctgaccttcagcgtgagccccataccgaacatcacgatgccgagcagccacgtcgtccacccggagattggttccacgacagctggggcgaagtagcccaaaaggccgcccgcgatgaccaaaagcgggaagccgagggtggccatgaacgcggagcggtcctccgcagattggtcagtatttcgctgtacgttatccatagtgcgggatagtactcccactatatggactatctgcatacggcctcccacacctcgcggtaactggcagcgagcgtgtccacggtttcgtgggcgttgagcccggaagggttgcccaccacccagacaggcacgcctgcgatcccttctgtttggcggcctttgcccgcacgcggacgttggaacgcggtgcgaaacgcgccgatgccggcgatcatgagtccctctgggcggtacgtggccaccttgtcggtgagttccttgcccccggcgatcagctcgtcgcggctgagctcgctcgccttcgcggtgtagcggttgacgatgttggtgaagcccaagccctgcgcggcaagcatgacgttgtcggcgtcggtgaggccgtcgcgggcgtcgacaagatagggcgtgatgccggctgtgtgcagcgcgggccagaacctgttgccggggtacgcgaacggcgcatccaccgcttccgagcgccctccggggttaatgccgacgatccacagcgtcgaatgagcaagattccggtcgtgcatctagccgaacatactgcgggcagtgcggtaccgctccggcgggacctgcttgaggtgcgccactgcgctctcgagcggcacgaggtcgatgttctcgccgtgcagagcgacgcacgtatcgaacttgcgctcgtgggcggcgcgggcagcgtgcaccccgtagcgggtggccagcacgcggtcgtacgccgtgggcgtgccgccgcgctggatgtggccaagcactgtggtgcgcacgtcgtagcctaggcgctgtttgatctcgtcggcgatgatctggcccataccggtgaaggtcttgtgcccgaactcgtcctcctcacccaggccagcgtccatcgtgccctccttcggcaccgcgccttcggcgacgacaatgatgccgtatttctcccccatctggaaacggcgctccatcgccttgcaaatttcctcgatgtcgaagggttcttcggggatcacggtgtagtgcgcgccgccggccatacccgcgtgcagcgcgatccagccgacgtggcggcccatcacctccacaatcaggatgcggttgtgggattccgctgtggtgtggaggcggtcgatcgcgtcggtcgcgacagagactgctgtgtcgaaaccgaaggtgtagtcggtcgccgcaacgtcgttgtcaatggtcttcggcacaccgaccacggggatgccgttgtcggcaagccacttcgcacccttgagcgtgccctcgccgccgatggcgatcagcgcgtcgacgcctgcgtcatccaaattcgccttgatctggtcgatgcccgctttaaacttgtccgggtgcaggcggccggtgcccaagatggtgccgccgcgcagcagaatagagtcgatgtaggcgtcgtcgtacaggtcgatcctgcggtcctccatcaggccgacccacccgtcgaggtagccgacgaccgtggagccgtactccgaattggccgtgcgaacgatgccgcggatcacagcgttaagccccgggcaatcgccgccggaagtcaaggtggcaagtcgcatgccttaagcctagcgcgcttaaacgcggggcttcaggcttatcgacgccaccgcccccaccaccatcgccgccatcggcacccccagcgcccacgacgccgtcgccgcaacctcgcccgaggcgagcaccgcgcccacaagcgccaccccgaccacgctgcccacctgccgggcggtgttgtacagcccggaagccgcgcccgtgtggtactccgcaacaccgcgcatggtcaccgccgcgttcggcgcccacacgaacgccccgccaacgcccaacagcgacgtcacggcggtaaaccaccacaccgaaactcccgcgcgcatcagcaggatcgccagcgccaagccggctgcgcacacggcgaagcccgcggcgcagagcttgcccgggtcgcggcggtcagtcagataccccgccaccggggtgagcacgagggcaaacaccgacattggggcagctactgccccagaagcggtcggcgacgcccccgccaccgtctgcaaccagtacatcaacgggatgaacatcgacgccacgctcagccccatcatggccacgccgagcgcgccgagcgcgaacgagcggtcgcgcatcagctccagcggcaggaagccgttgtcggtgccgtttctggcggagagcacaagcaaccccagcagcagcgcgccgagcagcaccgacatccacagctggaagtggatgccgtagaccgcgcaccccaacccgccgaaagaaagcagcacgggcaacagcgtgacccgctcaccgcttctgggcagcgccggcaagaaaaccaccccggcaacgagcgccgccgcaccgagcccggcttgcacgaaaaacgccgcgcgccagcccgaggcttccgcgactgccccgccgataacaggaccgatcagcgacgccaccgagccgatgacaccccacgcggcaaacgctcggccctgcttcgtctcgtcgaacacgcgcgggatgagcccgaacgcctggggcaggaacaccgcggcgccgaagccctgcaggccgcgcgccgccaccagcgagccgaaagaccacgacgcgccggcgaagatcagcgcggcgacgtagatggcaaggccgatgagaaagacgcgacgctgaccgtaggcgtcgcccagcttgccggtggccggcatcggcgcgacggtgcacagcaggtagatgctggtcagccacactgccccgccgacttcgaacgggagcagcggggtgatcacgggcatgaaaccctggtcaatgaggacaagaaaataccccgcagcaagggctgcgagggtattccaggggttaacggccggcttcaaacgccgcacccacgcggtaaagccgcgcgtcctcgaacgccggggcaatcagctgcagaccgaccggcagcccagtgtcgcccgcctcgccagcgggcagggacatgcccggcaagccggcgaggttcagcggcagcgtgaacaggtcgaagttgtacatcgccaacgggtcgtccaccttctcgccgagcttgaacgcggtggtcggcaccgcggggcccgcgatgacgtcgaccttttcgaaggccttttggaaatcctgggcgatcagcgtgcggacacgctgcgcctgcaggtagtacgcgtcgtagtagcccaccgacagcgcgtaggtgcccaggatgatgcggcgcttgacctcgggcccaaagccctcgccgcgggtgagcgccatgacctcctcggcagagtgcgcaccgtcgtcgccgacgcgctggccgtagcgcatgccgtcgaagcgggcaaggttcgagctcacctcggaggtctggatgaggtagtaggcccccatcacgtcctcgaagctcgggcaatccacctcgacgatttcagcaccttggcgctgaagctgagcaaacgcgttgtcgatgatctcgttcacgccgtcctgagtaccaggacggtcgaactgcttgacgcggccgaccttgacgcccttcaagtcgcccttcgcaccctcgcgggcagcgtcggcgagcgcgggcacatcgcggtccacgctcgtggcgtcgaactcgtcgtggccggcgatgatctcgtgcaaaagggcagtgtccaatacattgttcgcgcacgggccgacctggtccagcgaggacgcgcacgccacgacgccgtagcgcgacacgccgccgtacgtcggcttcacaccgacagtgccagtcagcgacgccggctggcggatcgagccaccggtgtcggtgccgattccaagtggcgcctcgccggcagcgagcgcggccgcggtgccgccgcccgagccgcccggcacgcgggtggtgtcgtgcgggttcttcgtcggcttgtaggcggagttttccgtcgacgagcccatggcgaactcgtccaagttggtcttgcccagaatcgggatgccggcctcgcgcagcttggttaccacggtcgcgtcgtatgggctcatatagccctcgagcatcttggacgcagcggtggtcggcgcgtcggtggtgaccaggagatctttcagcgccagcggcacgcccgcgagcgcggacgccggctcgccgccgcttttgacctgctcgtcgaccttgtccgccgccgtcagcgcctcttcggcaccgacgtaaaggaacgcgccgatctcgccgtcgacctctccaatgcggtcgaggaacgcttgcgtgacctcgcgggaggtgacctcaccggcctggatcatggcggcgagctcgtgcgccggcttcgaaaccaagccgtcttgcggaatggtgtactgcgacattgttctagtctccctctcccagaatctgcggaaccacgaagcggttctcctcaactgccggcgcctggtccagcgcctcggcctgcgtcagggttttcttctccacgtcttcgcgcatgccggcctcgatcgagtgcgggtggctcataggcgtcacaccctcggtgtcgacgctttgcaccttcgacactgcgtccacgatggtgtcgagctgcttcgcaatgtcgtcgagttcatcgtctttgagcgcgatgcgcgcaagtttcgcgatgcgcgagacctcgtcgcgggaaatctcagccaatgtgcttccttttctgttcaagggttggcggtgaaaacgcctccatcttacgtgccgcccccacacgccaagtcaaaacctcttggtgcgggttgctataaatatggccatgtcctatctcatccgcgtttcgcttccagacacccctggcagcctcggcgagctcgccgtggcgttcggtctggtcgacgcgaacatccagtccgtggacattgtgcagacgggcacggacggccacgtcaccgacgacatcgtggtgtcgctgccgaccgggacgatggtggatgccgtggtgaccgccgccgcctccgttgacggcgttgaagtggactcggtgcgcccgttcactgggcgcgtcgaccgacgcggtcaagtgcaaatgcttgcccgcatcgcgaaccagtcgaccaacatcgaggccgcgatggccgagttggtcgaggtcgtgccgcggacgatgacctcgtcgtgggcggtggcgcttcgcaacaccgacgcaggacttgtgcgcgtcgccgcttctcaggcagcgccgggcgacgacggcaccagcccgcacatgctggacgtggatggcccccgcatcctcttccccgagacggacacctggatgccggacgcgtggtcgttgctggacacagcgctggcgatcaccccgctgcagggcaccgacctcgtgctcgtcgtcggccgcatcggcggcccggactttttagcgtctgaggtctcccagatcggcgacctcggcgccattatcggcgcgatcctacgctagcgcgccgagcgcttcgggtcctgcttccagcagcgccacaaactgctcttcgttgagaatcggccggccgagctcctctgctttcgctgccttggagccggcgttctcgccgacgacaacgtaatccgttttcttcgacacgctgccggcggccttcccgccgcgcgacaggatcgcctctttcacctcgtcgcggctaaacccgtccagcgtgcccgtgacgaccacggtgaggcctgcgagggtctgcggcaggtcctccccgccagcgtcctccatcgtcacgccggcctctgcccacttgcgaacgatctcacggtgccaatcgacttcgaaccaggccttgaacgattcggcaatgatctggcccactccgtcggtttcggcgaggtcggacaagggtgcgtcgataagcgcctgcatcgacttgtaccgcgcggcgagcgcgcgggccgctgtgggtccgacgtggcggatggacagggcgaccagcacccgccacagctccgcgtccttggctttctcgaggttgtccaaaagcttcttgcccgcggcgctgatctggccgtccttgcgggtgtaggcgttggatttctccaggtcgttttcggtgaggtcgaacaggcagccttcgtcttcgagcacgcccgaggtaatcaggtcgtgggcgcccttctcgccgagcgcctcgatatcgaaggcgccgcgggaggcgagatactccagccgcgcgccgagctgggccgggcacgagcgggtgttggggcagcgccagtcggcgtcgccctctttcgcaggcgcgagcgtggtgccgcacaccgggcaggcttgagggaagacgaactcgcgctcggtgccgtcgcgcagatccgcaaccgggcccacgacctccgggatgatctcgccggctttgcgcaccaccaccgtgtcgccgatgagcacgcccttgcgcttgacctcgtgctggttgtgcagcgtggccatggacaccgtcgagcccgagacgaacaccggctcaagcacggcgaacggggttgcgcggccagtgcggccgatggagacggcgatgtctttgagcttggtggtcacctcctccggcgggtacttgtaggcgatcgcccagcggggcgcgcgcgaggtcgcgccgagtgcgcgctgcgcgtcgatggggtcgaccttgaccacaaggccgtccatctcatggatggcgtcgtggcggtgatccgcccagtacgcgacgtctttctgcacctccgcggccgttaccgcccgcttggtgtactcggagaccggcagaccccacgccgccagctgctcgtacgcctcgtgctgggtcttcggcgcaaaaccctcgcgcgcgccgatgccgtggcagatcatgcggagcttgcgctttttgacgtcctccgggttcttctggcgcagcccgcccgcggcggcgttgcgggggttagcgaacggcttgccgccttcggcgatgcgcagctcgttgagctcggggaaatcctcgggtcggatgaacacctcgccgcggatttccaccagcgcgggcgcctcgccctcaagctcgtgcgggatgtcctcgatcaccttggcgttgtcggtgatgtcctcgcccacgcggccgtcgccgcgcgtcgcagcccgggtgagtttcccgttctcgtacaccaggtcgatcgacaggccgtcgatcttcagctcggtcaggtacggccccggggtcttgtccagccactcctgcatctcgtcgggcgagaacacgttgtcgaggctcatcatccgctcgaggtgggtgacgtcggcgaagacggtggaagcaaccggcgcaccgacctgcttcgtcggcgactccggcaccgcaaactccgggtgcgcttcctcgaacgcttcaaggcggcggtacaacgtgtcgaactcagcgtccgagatgacgggctgcccgttgtagtacaggtcgcggtggtggcggacctcctcagcgagctcgtcccactggcggtggaggtcctgctgctcgggcgcgttgtcagtcatagcgccccagtctaggctcccctacttctcgtagagcgcgaagacgcgggaggtaatgctcggcgcgcccttaatgttcgcggggccgaccacaacgacggcgccggtggcgggcacctggtccaggttggtcatgacttcgacctggtagatgtcctgctcgaggatgtaaagctcgccgtagaggaaaccctcgcgcgcggccgtcacaccggcgtcggtgtcgagcgtctcgtggccgatggcggccacaccgcgctgctccacgaggaacttcagcgcgtcgagagaccagcctggagtgtgctgaacgccgtcgtcgtccaggttgcggaacgccgccgggtcctcccagcgggcgtgccagttgctcgagaacgccacgaagctgcccgcgggaatctcgccgtgctcggcctcaaacgcttcgatcgcctcgacggtgacctcatagtcagggtccgccgcgacctcgtcctcgaggtggaggacgaaaagcggcaggatcagttcgtcggcgccgatggcgtcgacaagccgcttgccctcggcgaagtggcccggcgcgtcgatgtgtgtgccgtacggcgtggcaagggtgtactccttcgcccagaagcggtcctgctcgatggtgttcacggtgcgctcgcgcatcggctcgaacgccgggaaacgcgggatgtcctcgtgcacctggtgggtcaggtcgacgcgggtggcggcgagcactcggctttggaaatcgttcacgttggaattggtcatacccttgaatatcggacatcccgcgcgctgacagcaaccgttgtattcaccgcgcccggccgtgttggggcgctcgttagaatgatccgcatggctaccccagcaggcttcgacgcgtcccggatgctctccttcgacctggaaaccacctcggcgaacccgcaggaggcgcgcatcgtgacctctgcgctggtgcgtatcgacgggcgcgaggtcaccgcgaacgaaacactcgcggaccccggcgtggaaatccctgcggaggcggcgaaggtgcacgggatcagcaccgagaaggcgcgggcggagggccgcccgcacgacgaggtgctgcgcgagacggttgagacgatcaagcggggctgggaggacgggctgacgctcgtcgtgttcaacgccccctacgatctcacggtgctgcgaaccctcaccggcgatttcactgtgacaggaccggtgtacgacccgcttttgatcgaccggacgaaagaccgcttccgcaaaggctcgcgccgcttgagcgacatgtgccagttctacggagtgcgcatcgacaacgcgcacgaggcgacctccgacgccatggctgccgcgcgcattgcgtggaagcaggtgcgccagtggccggagctgacggagatggatgcgggcgcgctcatggagtaccaggcggtgcagcactacatgctgcaggaggagcgccgcgaatacctgaccaaacagggcaaggacgcgtcgcgctgctcgacgagctggccgatgatcggttagcgcagcgcggcagccatctcccgcgccgtacggaagttgcgcgcggtttcgagcagcgtctcgccggcgtccgcgtaggtgtcgatggtggcggtgccggggtcgatctgcagctcgtcgaaaagttggagtacctcgcgcggcggggtgaccgggatggcgaggcgcgccccgcggtcgagcaatcctgcgagggcgtccttgttctctttgaggcttgtggtttgccacggtgcgtcgataagcagcggcgcgttgagcaggaactccccgtaacccgcgtaggcctcctctggctctggcaccgccgcgatgcgctcgtactccgccgcgcccgccaacgcgcccttcacgacgtcggcgagcagcggctcgtcgagttggaggacggttggggcaattcgcttttcgacgtccccccgatgctccccaaccgccccctcgagcgcatcctgcagatcgcgcaccgcgccttggtcggtgatcatgcggtggccgttcggcatctcgatcgcggcggcgagcgtccacggccccaccagctggaccttcacgcgatcgaccttgcccgcccacaactcctcgaggacgtccaagtcgcgcgccatgttgtcttgcagtccgcgtttgcgcgcagccacccgccacccgcgcgggccccggtcaaccgggatgtccagaagcgccgccgtgcggccgatggcgtcgaagccgatcccgcgggcgggcaactgcgggatgtgcggcagcggcaactcagagagcaccacgtcggcggccttcaccaggtcggtgcccggcatcgggccgagtccaaaaacgaggggggtatccacgccggtcatgctacgcggtggcgcagatggtgcccgagccgagcacaacgtcgccgcggccgtccggatccggcaggtagagcacggcagcctggccgcgggccacgccctccagcggttcgtggagggtgagcgtcatgcggtcgccctcgatctcggcgcggcatgccacgaccccgccgtgcgcgcgaatctgcacgttggcctcgaactcgccggtcatcttcgggtggagcaccttgaggcggtcagcagaaatctcgtggaccttcaacgcttcgcgcggtcccacagtcacggtgccggtctgggcgtcgacgtcggtgacgtaacgcggcttgccgtcggcggcgggtacgcggatgttgaggcccttgcgctggccaatcgtgtactggaacgcgccgtcgtgcgctttcagctcgttaccctcggtgtctttgatcatccccgggcgcatgccgatggagcggccgaggaaggcctgcgtattgccgtcagggatgaagcagatgtcgtaggaatccggcttgctggcggtggaaaacccgtgccgcgcagcttcctcccggatctgcggcttctccgtgtcgccgaccgggaagatgcagcggtctagctcgtcgcgggtgagcacaccgaggacgtacgactggtccttcagcgggtcggcgctgcggcgcaggttgccgtcatcgtcgatgatggcgtagtgaccggttgcgatcgcgtcgaaaccgagcgtcaccgcgcggtccaacagcgccgcaaacttgatcttttcgttgcagcgcaggcaggggttgggggtctcgccgtgctcgtacgaccacacgaaatcgtcgatgacttcttccttgaacttgtcggagaagtcccacacataaaacgggatacccagtttgtcgcagactcggcgcgcgtccgccgaatcttccagcgagcagcacccgcgggcggactcgcgggtctgctgcgcgtccttgctcagcgcgaggtggacgccgacgacgtcgtgtccggcctcaaccaggcgcgcggcggcgacggaggagtcgactcccccgctcatggccgctagtactcgcatgtcgcggcagtgtagtcccgtgaaggcgaaaggtgaaacgtccggctgcaccgcagctgctgaccgcagcgaatcaactggccttcaaggctctcccccctagacggataccctcctggggtattatcgtaagaagcaacctcgctccaatgaggagtgttgattttcggtgccgcgaccccgccgcggccaaaccgatcagaaacaggaactggaccggaagaaaggaacccactgtgagcgacaagcacacccactccagcgccggaaccggtgagcacgccggccaccacgcccacgcacaacgtcacgagagcagtacccacgaggcccatgccggtcacggcaatggcgggcacaccggccacggaggacacggaggccacggagaccacggccacacaggtcatagtgatcacgtcggccagtttcgccgcctcttttggatcatgctgcttctcgcggtcccggttgtcgggttcaacgccacattcgcccacctcatcggttaccagctgccagacgcagaatgggcccggtgggtctcaccgcttctcggtaccgtggtgtacttctggggaggctggccgttcctcacgggcgctgtctcggagatccgttcccgcaaacctggcatgatgctgctgatctcactggcaatcacggtcgcgttcatcgcctcctggggtgcgtcgctgcgcttcctagatagcgagctggatttctggtgggaattggcgctactggtggtcatcatgctgttggggcactggattgaaatgcgctccctcgcccagaccacctcggctctggactcgctcgccgcacttctgcccgacgaggccgaaaagatcgacggcgacgaagttgtaaaggtcaccccggcggatcttgaggtcggcgatgtcgtaatcgttcggcctggagcttccgtacctgccgacggcacaatcgtcgacggcagcgccagcatggacgaatcgatggtcactggcgagtcgaaaacggtgcgccgcggtgaaggcgagcacgtggtcgctggcaccatcgcgacagactcgggcctgcgcatcaaggtcacagccacgggtggcgacaccgcgttggccggcattcaaaagctcgtcaccgatgcgcaagaatcgtcatcgcgggcgcagcgcctcgcagacaaggccgccgcgtggttgttctggttcaccctcggcgccgccattctgaccgccgtggtctggaccgtcgtcggcatgccaaacgacgccgtggtgcgcaccattacggtgctcgtcatcgcctgccctcacgccctaggcctcgcaatcccgctggtcgtctcgattgcgactgagcgcgccgcccgcggcggggtgctgatcaaggatcggctcgcactcgaatccatgcgcaccgtcgacgcagtactgttcgacaagaccggcactctcaccaagggcgaacccaccgtcaccgcgatcgacaccgccggcgggcgtgataaagaagacgtgcttgcccttgcggcggccgccgaggcagacagcgagcacccgctcgcacgcgccatcaccggggctgctcaggcccgtggcgtagccgtcccgcaggcaatcgacttttcttcgtccccagcagtgggcgtgaaggcaactgttgacggtgaggtaatcgaggtcggcggcccctacctgcttgagcagcattccgccgaagagctccccattgcagacgagtggcgaaaggagggcgcgatcattctccacgtcctcgccgacggcgaagtgatcggagcactccggcttgccgacgagatccgtcccgagtcccgcgacgccgtcgacgcactgcactctgcgggcgcccaggtcgtcatgatcaccggcgatgcgcaggccgtcgcggacaccgtcgccaaggacctgggcattgaccgggtcttcgcgggtgtgcgtcccgagcacaaggccgcgaaagtcaaggaactgcaaggcgagggccacaaggtcgccatggtcggcgacggcgtcaacgacgcccccgcgctggcccaggccgatgtcggcatcgcgatcggtgccggcacagacgtggcgatcggctcggcgggcgtcgtcctggcaagctccgacccgcgatcggtgctttcggtcatcgagctctcccgtgcgacctaccggaagatgaagcagaacctgtggtgggcggccggctacaacctgctgtccgttccgctggctgccggtatcctcgccccaatcgggttcgtgatgccgatgagcgtcggcgcaatcctgatgtcggcctcgaccgtcgtcgtcgccctcaatgcgcagctgctccgccgcctcgacctcaccccacagagcagcaccgaccgtatgctcaaccgatccaagtgacccgacaccgctcacaccactcaggaggcccatgatgaacgaccacggctacatcagcgagaaagaccgttacctcgctcggctcaaacgtatcgaggggcagacccgcggtattcaccgcatgatcgacgaaaacgcctactgcattgacatcctcacccagatcagtgcggttaacgcggcgctgaagggcgtagcactgggtttgctggatgatcatttgaggcactgcgttgccggtgcgatcagcgatggacaagacgctgacgccaaaatcaaagaggcgtccgacgctattgcgcgactagtgaaatcctaggggcacctgtcgcagcaattcggattcccccccttctgcgcccggaaacacgaggagcgactgggcggcctctgcggcctaccctgcgcagtgccgacgcccgcctcgagtaccctcaccagccatggtcgcaaaaagcgagttttacgagatcgacaccggcgtcgccgaggtgctgcgcgagcccgacggttccatggtgctgctcgtcaacggcgtgcccagctcacacatcgtgcccgacgatccgacgcggttggacttcgagtacatgcggtggatcgccgactttctggatgaagcctaccccgatgaggcgaaagcgaagtcgcggttgacgcacctcgggggcgcggcgtgcacgctgccgcggtatttcgcccaccagtggcccgggtcgagaagcaccgtggtggagatcgactcggagctggcgatgcttgcgcgcgagctgtttcacgtgccgcgcgcaccggctgtgaagatccgggttggcgacgcccgcgaggtcgccgacggcttcaagccagccacgcgcgacgtgatgatccgggacgtgttctcgtcggcgacgactccgcgcagtctgacgacggtggagttttatggacgggtgagggcgtcgttaagcgagctcggcttgtatgtggcgaactgcggcgcgcacgcggacctgaaggaggcaaaagaagagctcgcggggatgtgcgaggtgtggccacacgtcgcagcgatcgcggacccgccgatgctgaaaggccgccgttacggcaacatcgtgctcatcggttcgaaccggccccttgaggcgagcccggagctgacccgcaacctactcatgggggcggtgccggcgcagttcaaggacgaggcgtggtgccgcgcgcttgcgaccacaccgcgctacgacgcgtagcgcgaggcgttgtcgaggaggatcaacaggtcgcctacttggtacttgccgccgagcatcttcgcaagatcctgcaggggtagctggtcgttgtccgccagctgctggactaagttggcgatgttgcgcgcgtcgttgatgttgaacccggcgcggtcagccgccttggtcagctcagccacgccgagcgcaccgccagccagcgccaagatagccaggacaagcttggtgttgtcctgctcaagcaccttcagctcgccggactcggggacttggaaggtttcgagcacgccgccgcccgcgctcaggttgcccgcggtgaactggttgaactggcccatggtgccgttgtagaggttcatgtccactggggtggcgatgccggggatgcgcccggattcgctgcgctgccagaacgtgagcttgtcccatccgccgacggggcgtggcggctggttctggtacgcggccagccacagcgggtagtccgtgaacgcgttggtgttgttcatgtgctcgtaccagaagtagcggtaggtgtagagcatcgggcgcttgccggtgaggcgctcagtctcggtgagaaagatcttggtccacgccgcgagttgaagcggggttttgccctcggcgacctcgaggtccagcacgggcggcagggtcaacgccgggccattgttgaccaccgacgcgaagtagcgggcttgggtcagcgggtcctcggcggggcgagcgtagtggtaggcgccgacgctcatgccggcgttcgcggcctcgcgcgcgtcttcgtcgtagaagacgttcttccagccctcgccctcactggctttaatgaaggcgaactgctgcagaccgggccccgacaccgtcttccagtcgatggtgcggccgcccggtcgttggtggccagcgacgtcgacgccggagacgagcccgggcagcggcaacgcgtccgccggcgccgcgggggcggcaacggtcagtgtgagcgcgagcgctggtgccaccaaggcggccaggactgaacggggcctgcggaagacatgcatggcgaaaactctaactcacgcgcaccccaccaacaccgcctgacacgccagcccccgccgccacattgattcacatgcgtcacatggcgccggcggcgcgggctttctccacaacctccgggagcacggcgaggaatgcgcgcacgtcgtcgtcggtggttgtgcggccgagggtgacgcgcagcgcccccatcgcctcgtggtcggtgtaccccatcacctccagaacgtggctgatgcgcaccacaccgctggcgcaggccgagccggctgaggcctcgaagccctgctggtcgagcagcatgaccatcgcgtcggcgttcgcgccggggaacatgaagtgggcgtggccgtccagcgcgggctgctgggtggtgacgatgacgtcgtcgatggcggcgcgcacaccgtgaacgaggttgcttctcagcgcgctcacacgagcgttcaccttctccatctcagcgacggcctctgcaagcgctgcagcggtcgccgcggcggccgctacgtccactgtgccggagcggatgccccgctcttggccgccgccgacgatgagcggctgcggtgccggggagcgcttggccaacagcaggccggcaccgcgggggccgccgaacttgtgggcgctggcagccagcgtggtagcgccgagcgcgtggaagtcgaccgggatcttgcccaccacctgcacggcgtcgacgtggaagggtgtgccggcggccgcggcgcgctgcgcggcctctttcaccggctgcaccgcacccgtctcgttgttcgcccacatcagcgaggcaaccgcggcaggggcgtcgagcggggtcaattcctggacgtgcccgtcacgcccgacctcgagccaatcgacctcggcgccgtcctggtgaacaagtgcgttcaccgcctcggtcaccgccgggtgctcgacggtggaagtcacaacgcgggcaggacgcccagcagcaacggaggcgcggaagagcccgcgcacagcgatgttgtctgcctcggtgcccgatccagtgaacaccacctcgaccgggtccgcgcccagaagcgctgcgatctgctcccgggcctcctgcagcacggcgttggcgcggcggccggaggagtactggctgccaggatttactgcggccgcatgctcggcccaggcatccacagcgcactggcgcatcggggtggtggcggcgtgatcaaggtaggtcatagccccctattctaacgcttggcgggggccgcaaatgtgggcgacggcggcgtcgccgatgcgcgcgatgaccaccgtcatcgggagcgtgcccttcagcttcagcttggcgcgtagctggtcggggtcgacgttgacgccgcgcacgaggatctccgcgctgcccgcgccgcgcgccgtaagcgctgccttcaacttcttcagcggcactgcctcgtagaactcgaacccggtgtagccctgtgggatcgtcgcccccgtgcaaaacgcgatgtgctcgtcgagcatggtcaggccgtggcgcgtcgcccagtggttcaccagcccggcgcgcaccaccgccccgtcgggttcgacgatgaagcgcccgggcgggcccgccggcgcggtgtcgggctcgtcggaggtagcgcgttcttgaaaactgtcgcgaagcaccaccgcctcgcggccgcgcccgaagcccggggtgtacaggcacgcctctttcaccccgccgtcgacggagacgacgctgacgaggccgtcccaccctgagtagtcgatgcccggcgcgcatttgacggccagttctcggccgcggtgagctgcgacaaggtctggcagcggtggcaaaagctttgcggggtcggtgatgcggcgcccgcctgagcgccgggccgggtcggcgaccactgcgccgaccgccgaggaggtgaccggggttaaggcgtcggcctgggtcagccacgcgccggggcccaagttgtggcgcgccatggcgaggcggggcatgtctatgtcggagcccagccactgcaggccgagagtcgaaaacgcaggcgcctcggacccgatggagcaggtgacgtcgtggacgaggtcgaccccggcagcggcgatgcggtgagcgcgcacatcggcgacagcgcggggcgtggcttgttgggcggcgtcggcgtcggtaagccaatgctcggggaacttgcccgcgctcgcgcgccgcgcgacaacgagcacgctgaccgcgcgggcatagtcgccaaactcgcgctcgagcaccgcgcggtcggcgaacaccgttttcttagcaagcgccagcgaaggtgagaccgcggcgatgcgctcggcgttcgccgcgagaaactccacctcggcgagggtgtagctcactgtggcctcccgatgcgctctttcgggcggcggtggaagaactcttctagccgctcgtcgtcgactgggtcgccgtagatgggcacgatcgcgcgcccctcggctgcacgaagcgcctcatccacggtgtcgaagcgggacagctccaccaggtgcagccaggttgcgggggcgaagcgcacaagaccagcgcgccacccgtcgatcaacaggccgggcgggaaccagttcgcgtcgtcggcctcgcccgtgtcgccgtcgggctcctgcccagttggcgtggcagctaggaaggaaaaggtgtcgaaccagttgccgcgctcagactgccccacccagcgcgagtagggcttgagcagatcggcgcacaccagcaagtcgttgtcttggagtacgtcggtcaaggacaactggtgggattcgagggcgaggcggtgggagtggaacacggaggcgtcgtcaagcagcgtgcccttttgatccaccgcgaggaagatgcccgactcctcaaacaactccctgacggcggcgaacagcaaggcgtgcgccttgtacttggtcagcccgagctggcgggcgagcgagatcgcagagcggccggtccacaagtcgccgtcgtcccaggaacggcccgggaagtcgcgcgtgtccacgccgccaccggggaacaccgtcactccggggtagttgagcatgctcagcacgcgctcctgcatccacacctcgagaccgttcgtgccgtcgcgcatgagcaccacggtcgcggcgagcctggcgccgctgaagcctgtggtctcggagacgtcgatggcgtcgccggcgtccgccgatacggcgcctgtcgtgcgcgacttcacctcacccctcctcacctgctgctacttggcccggtgggctcccccgcgcttcttccgcgcgcggcgcgcgaagtagcggccgtcgtcgtaggtgacctcgatgggctggtggtaggccttggtgacgttctcggaagtcaacacgtcctcaatcaggccctgcgcgaccacctcgccctcatccagcagcatggcgtgggtgaagccgtacgggatctcctctaagtggtgggtgatcataacaatcgccggcgcgtccgggtcgagcgccaactcgcccaggtaggtgatcaggtcctcgcggccgccgaggtccatgccggcagctggctcatccagaatcagcagctcagggttggtcatcacggcgcgggcgaccatgacgcgcttgcgctcgccgtcggacaatgtcgcccacgtccggtcgatcaggtgcatcgcgccgacttgctcaagcacgtcgatggcctgctcgtagtccatctcgtcgtactcctcgcgccagcgccccatgatggcgtaaccggcggagaccaccaggtcgcccaccttctcagatcccggcacgcgctgggccagcgcagacgaggtcagcccgattgcggagcgcaggtcgcgcatgtcggtcttgcccacctgctcccccagcacaaacgcggtgccggaggtggggaactcctgcgctgcggccatgcggatcagcgtggtcttgccggcgccgttggggccgacgatcacccagcgctcgtcgagctccacctgccagttcacagggcccacgagcgtgttgccgccgcggacgaaggagacgtcgcggaaatcaatgagcaggtctgggtctgtcatctcgttcacctttcccattgtggactatttcgcgcgccaagtggggcgcgacgtgaccaacgcgctacgaattcaccatgtcgcaagcacgggccttggctacgctgggcatgaacgtgggacacctatcccccacacccgccacaccttttcaagcgcgagaggacgcagaatcaatggttgcacgcttcggcatcgacgacgtcaggccccaagtctccgggcgcacactgcccgcgaaggccgtggtgggtgaggtcgtgcccgtctccgccctggtgtggcgggagggccacgacgccatcggcgcaacactgaccctttcctccccttccggcgaggagatcctggtgccgatgcagcaggaggtctaccgccccgattacgtccacgccattttcgcgcccgaggagcagggcctgtggcgcttccgcgtcgacgcgtggagcgacgtcatggccacctggcgcaacgccgtgtcgaaaaagctcgccgcaggccagacggaagctgagatggccaacgacatcgcgcacggcatccagctgttcaccgaggccgcgcagcaggtcccggcgacccacaggcagcaggtggagcgcgctggagcactgcttgccgacgccgcgctgcccctgcccacccgcatcgacgcctgccttgaccccgtagtcaccgacatcctcacccaccacccgctgcgcgagctcatttcgcacggaccgatctgcgacattctcgtcgagcgccgcgccgcgctggtgaactcctggtacgaactgttcccccgctccaccggcggcgtggacgacaacggcgagccggtccacggcacgtgggcgacgaccgcgaaggcgctcgaccgcgtcgcggccatgggattcgacaccgtctacttccccccgatccaccccatcggcgaggtgaaccgcaaggggcgcaacaacaccctgacgccggaggccaccgacgtgggctcgccgtgggcgatcggctcttccgccggcggccacgacgcgttccacccctcgctcggcggtgaggacgagttcctcgacatgatggaccacgccgacgagctcggccttgagatcgcgctcgacttcgcactccaggccgcccccgaccacccttgggcagccgcgcacccggatttcttcaccgtgctcgccgacggcaccatcgcctacgccgagaacccgccgaagaagtaccaggacatctacccgatcaacttcgacaacaccccggacgccgtctacgacgagatctaccgcgtgatcatgtactgggtggatctgggcatcaccacgttccgcgtggataacccgcacaccaaaccggtcaacttctggcactggctaatttccaaggtccacgagaccgacccggacgtgatcttcctcgccgaggcgttcacccgcccgccgcgcatgtacggcctgtctaaggccggcttcagccagtcctacacccacttcacctggaagaccacgaaggaggagctcaccgattttgcgcagctgcttgtcgacgtcgccgatatctcccgccccaacctcttcgtcaacaccccggacatcctgcacgagtttcttcagaagggcggccccgcggcgttcgcgctgcgcgcggcgctcgccgcgacgctgagccccttgtggggcgtctactccggctacgagctctacgagcacgagccggtggcagagggcagcgaggagtacctcgattccgagaagtaccagctgcgcccgcgcgacttcgatgccgcgcttgcccgcggagagtcgctggagccgtatctgacgctgctcaaccgcatccgccgcgaaaacccggcgctgcagcagctgcgcaacatccacttccacgacattggcaacgacaagctcatcgcctactccaaggtcgacgctgtgaccggcaacgccgtgctcgtggtggtgaacctggacccgtactacacccaggacggcatgctgcacctaaacgtcgccgaactggggttgaacccgggcgagtcgttcgaggtgcacgatcttgtcaccggcgagcgttacacctggggcgcggacaactacgtccgcctcgccccgcaggtcaacgtcgcgcacatttttcagcttccggatgtctccccggagcgtcgtcaagcacttgctttccggcgcatctccgatcacgactaccgcccatagaacctaaaggacccgacatttccatgacttcgccagatccctcttacctgatcccggaggccgaccgggcccgcttgacccaatgcaagcaccacgcgccgcacgatttctacggctggcacccggccgccggcggctccgtggtccgcacccgccagctgggcgcggaaagcgttgccctgctcgtacacggcgacgaggtagcgatgcagccgatcggcgacgacatctgggtcgcaggcctcgacgacgacgcagcctctgattaccgcctgaagatcacctacccgggcgcggagccgcacgtggtcgccgacccgtacaacttcctgcccacgcttggcgagttcgacctccacctgatctccgagggccgccacgagcgcctctgggaggtcttaggcgccaacgagcacaagtacaccactgcgctcggcgaggtcgccggcacctccttcgcagtctgggcaccaaacgcgcagggcgttgccgtcgtcggcgagttctgcgggtggaacccgaaccagtacccgatgcgctccctcggcgcctccggcgtgtgggagatcttcatcccgggccttggcgccggcacccagtacaagtttgccgtccaaaccgcttccggcgagcgcgtggacaaggccgacccgctggccaaacagaccctgtgcccgccggagaccgtctccgtggtcgccggcgcctcgacgtacgagtggggcgacgaggactggatgcgcgagcgggttggcatcgacgcggcgaacgcgccgatgagcgtctacgagtgccacatcggctcgtggaaggagggctccaactacgccacgatgcgcgaagagctggtcccctacctggtggaaaacgggttcacccacgtggagttcctcccggttgccgagcaccccttcggcgggtcctggggctaccagatctccggctactacgcaccgaccgcgcgctggggcaccccagacgatttccgggcgctggtcgatgccctccacgccagcggcatcggcgtgatcgtcgactgggtgccggcccacttccccaaagacgcgtgggcgctggctcgtttcgacggcaccgcgctctacgagcaccccgattggcgccgcggcgagcagaaggactggggcacctacgtcttcgacttcggccgcaacgaggtgcgcaacttcctcgtcgccaacgcgctgtactggttcgaggagttccacttggacggcctgcgcgtcgacgcggtggcctccatgctctacctcgactactcccgcgagcccggtgagtggctgcccaaccagtacggtgggcgcgagcactgggatgccgtccagttcctccaggagatgaacgccaccgtccagcgcacccaccccggtgtggtcacgatcgctgaggagtccaccgcgtggccgggcgtgaccgcccagaccgaagccgacggcctcgggttcaacctaaagtggaacatgggctggatgaacgacacgctggagtacttctccctcgacccgatccaccgctcctaccaccacaacgagatcacgttctcgctggtgtacgcgttcagcgaaaagtacgtgctgccgtttagccacgacgaggtcgtgcacggcaagggatcgctctgggagcgcatgcccggcaacgactggaacaaggcggcaggccttcgcgccctctacggctacatgttctcccacccaggcaagcagctgatgttcatggggtgcgagtggggccagaccaccgagtgggacgaggcgcactcgatcaactgggacaacgtcggcgagggttggggccacgagtaccaccacggcatccgccgcctcgtgcgcgacctgaatttcgtctaccgcgacaccgcggcgctgtactcccaagacaactcgccgatgggcttccagtggctgaagggcgacgacgcggagcacaacctgctcgcctacgtccgctggggcgcggacgccacgccgcttttggcagtggtcaacctctccggcgccaccttgcaggattatcgcctcggtgcgcccgaggccggcgaatgggagctggtcatcaacaccgaccaggccatctatggcggcgccggcaacgagatcgcgcagtcggttgccacggaatcgacagcgtgggacaacttcgagcagtccctctcactgacggtgccggcacttagcgtgcagtggtaccagctgcgccgctaaaacagcgcgctggcgagctgggtccgcgcggcgatcacgcgcggatccgacggctcgaagagctcgaagagctccagaaggcgtgcctttgcttcggggtgggccttcacgagcgggatgaggcgggagaacgcggcctcagggtcacctgcgacgacctcggcgtcggcggcgtcgagttgcttctccacgtcgtctggatccgcctgagcctccgcgatcgggtcggtggtccgattattcgggtcaagccgcttcagcacggtgacggtgttcttggcttgggtgatttggggatcgttgggggcgtcggaaagcatggcgtcaaagaccgctactgccgcatcgaagttgcctgccgcaaactcttgctccgcctgctcccaacggggatcttccggcgcgtcagcctcctcggcaggggcctcatcaccgagtccctcgagctgcgggccgatgttggtcaccagcgcctcgagccactggctgagctggtcgcgcggctgatcgccctcgaaattggtgacagggcgccccgctgcaagcgcgatcaccgtcggcaacgcgcgcacgccaagtgcctgcgccatctgcgggtgcgcgtccgcgtcgaggtacgcgacctgaaatccccgctgcccggcagcaagctctgtaagagtctccttgagccgggtcgattcacctgaacgggcggtgccgatcatgagcaccactgggatctgcgcggagcgctcgaacgccttggcctcgatgtcgtgctcagagacctcaataaacggctcgaactgaccgctagcgagttctcgacgcgcttccgcctgctgcgccaacgcgcccaagtcgactgccccgcctgtgaacgattggttgaactgtgccatggtggcgctccttacttgtcaaagtgcttctctagcgatgccattttctggtgcagcatgtcagtatggcctggccggatgtccgccttaatcacaagcgagacccgaggagaaacggcctctactgcctcggtggcacgcttgatcacgtccatcacctcgtcccactcgccctcaacggtagtaaacatcgacgttgtctcgtgcggaagaccagactcgcggaccacgcgcacggcacgcgagaccgcctccgacatctccgcgttggggttgttggtgacaaccggtgccaccgaaaacgctgcaatcatgccgcccagcctactcaccggcgctgccagcagtgcttgtgccaatggcgccggtcgtccacgccgcggccggaatccttcggccacgcaaccacgtgcgcgacaccgggcggaatgttctggttacaacctgggcagatgtagaacttggcggcagctccagacccgatctggcggacgcagaacacctcgccgttggtccagctgggcccctccatttcttgggtaccgatgaacgttgagccgtcgcgcggcaggatgtaggcgggccgcggtgtggtgcggcggtttttccgtggcatgtcccaaatgtttctttagaagagtcgcagttcgttggattcgatgccgcgcagctcaccgtagtccagggtgacgcagcgaaaaccccggtcctctgccagcgtgcgcgcctgcggcttaatctcttgggcggcgaagacacccgcgaccgggtgcagcagctcgtcacggttgagcagctccacgtagcgggtgagttgctcgacaccgtcgatgccgccgcggcgcttcacctccacagccaccgtcgcacccgtcgcgtcgcgggcgagaatgtcgacgggaccaattgccgtcgggtactcgcggcgaatcagggtgtagcccgtgccgagcgtggtgatgtgctcggccagaagctcttgcaggtgggcctcgacgccgtctttgaccaagccgggatcggtgccgaggtcgtggctttcgtcggcaagcacctgctccaccgtgatccgcaactgctcgcccttcgggttctccacgatccagacctgctcgcctgtgtcctccccctcgaggtcgaccactgattcctcgcgcatggtgcacggcggcgtcatccagttgagcggtttataggcccggtcgtctgcgtgaatggagaccgagccgtcggctttgatcaggatcagacgcgtcgctagcggcaggtgggcgtccaacctgccaacgtaatcaacggaacagcgggcaataacgagacgcatgagtagcgattgtacttactggccccgctgagcccgctcggcgagctcgttcatgtccgcgcgctgggtgcgggaatccggcgcagactccacccacgaaatcagcgccatctcggcgcggcggtcccccgcaaactcaaaatcaccctgcggcccagtgagcagcagcacgccttcaacgccgggcataaacccctgctcctcctcagtgagctcgcggatgccgttgaaggtgacttggcgcctatccagcgaatagtcgtagttgaacgacaaggagcgcagcttgtaaaaccgcgcctcctcccccgcgtagcgcagcacaccgtgacgccagccgtgagcaccgtctgcgggcagcatccggatgatgccttgcacgcctgagttgcggacattggtgaagcgccaccccccggcgatggcaaccagtgtggcgacgagcagcaggagacacagaacgatttccacccgcaccactcctctcaatgacacccgctagctctagagccgtttctattcatcctagtccgcaaacccgcgggataaaaggcaaaacaccctcctggcgaacagtcaccaggagggtgttttcgaaagtgaagagcgccgtctacctaccggcgcggcgaaccgcggcgagctcggcctgcgagcgcgcctgcgtggtcgtgtcttcgtcggtcaggccggtctcggctgcggccgagtcaacctcgtcggcgaagattgcgtaatcggccaacaccgtgacgcgatcgccttgcacggagaagaacccaccctgcacagctgcgacgaggcggtccccgtccactggcttgatggtcacgaccccgttgtcgcgcaactgcgccagcagcggctcgtgaccgggcaggatgccgatctcaccttcggtggtctgggcagtgacgatgtttgcctggccctgccagagcagtcggtcaaccgagaccagttgagcggtaagttcagccatcgtttacccctttacgcttcctgcagcttcttgtacgcggcctcgacatcgtcgagaccaccaaggttgctgaaggcctgctccgggtagtggtcgaactcgccgctagccagcttgtcgaacgcgtcgatggtctcctccagcggcacgtacgagccctcgtcgccggtgaacttcttcgcaacgaagaagttctggccgaggaaacgctggatcttacgcgcgcgctgcacggtgatcttgtcttcctcgcttagctcgtccataccaaggatggcgatgatgtcctgcagctccttgttcttctgcagaataccgatcaccttctgagcaaccgcgtagtggcgctcgccgacgatgcccggctcaaggatgcgcgaggtcgaggtcagcgggtccacagccgggtagatacccttcgaggcgatggaacgggacagctcggtggtcgcgtcgaggtgggcgaaggtggtcgccggagccgggtcggtgtagtcgtccgccggcacgtagacggcctgcagcgaggtaatcgaacggcccttggtcgaggtaatgcgctcctggagcacacccatctcgtccgccagcgtcggctggtaacccacggcggaaggcatgcgacccagaagggtcgacacctcggaaccggcctgggtgaaacggaagatgttgtcgatgaacagcagcacgtcctggttctgcacatcgcggaagtactccgccatggtcaggccggacagggccacgcgcatacgaacccctggcggctcatccatctggccgaagacaagcgcggtatcaggcagcacgcccatgtcctccatctcgaggaacaggtcggtgccctcacgggtgcgctcgcccacgccggcgaagacggaggtaccggagaactcacgcgcgatacgggtgatcatctcctggatgaggacggtcttgcccacaccagcaccaccgaacaggccgatcttgccgcccttcacgtacggggtgagcaggtcgatgaccttaatgccggtctcgaggatctcggtcttaccctcgaggtccttgaacgccggtggctcgcggtggatcgaccaccgctcaccatcctggccgaccgatgggtcgtccaagcactggccgagcgcgttgaacacgtggcccttgacctggtcgccgaccggcaccgagattgggttaccggagtccttcacctgcgcgccgcggacgaggccgtcggtcggcgccatggcgatggtgcgcacgaggttgtcgcccaggaactgggcaacctcgaggatgatgtcgcgggacatgctctcgaggtcgatgtggacctcgagagcgttgtagagcgcgggcagctcgccgcgtgggaactccacgtcgacgacggcgccgatgacgcgcacgactcggccgttctcagaaccgcgcgggttctgagtgttctcgacacgaccttcggtgcgagcctcagccgcgggctcagcctgcaacgcggcctcgcccggcgtctcgtcgcgctcatcaaagttgagagcagtagtcatgatttagtcactttcctcactaccggacagcgcgccggcgccgccgataatctcggtgatttcctgggtgatttttgcctggcgggcctggttcgcctcacgagagaggttgttggccagctcggtggcgttatcggtcgcgttcttcatggcggtacgacgagacgcagattcggcggccgacgcctccaagaagatggagtacagcgagcgcgacacgtacacgggcagcagctcatccatgagcgtatccgggtccggctcgaactccatgtccggagccacgccgtcggcgggcgccagcatgctctcgttctcgtacttgaactcttcaagcacgggctcgatcggcagaagctggtggacgcgtgcctcctgcgtcagcatcgagacaaactccgtgtacacgacgtgcacctggtcgaagccgcggacggcctcgccctcggttgcgttgacgccctcgcgccacgcggtggtgccttcggagccagccaagaagccgtcgacgacgaaacggcggacgtcgtgggttccgtcccaagacggcttctgggaccaaccggtccaagcgccagcgacatccataccgcggaacttgtagtgcgacacacccttgttgcctgtgacgaggcgaacaacctcgtagcctgcgtcggtgagcatgcgctcaagctctgcggctttcttcagcacgttgtggttgtagccgccggccataccgcggtcagaagtgaccacgaggattgctgcgacccgaccgttctcacgctcgtggagcatggggtggtcgagggaactcgcagccgcgaggcgttccatgacgttcttcagctcgtcggcgtacggtttcgccgcctcgacgcgctgctgggccttggtgatctgcgaggtcgcgatcagttcctgggccttggtgatcttcttcgtggagttgacggacctaattcggtcgcgccattcgcgaagcgttgccatggtatttcctcccttcctttatgtagtagtcctcgagcacgtgcgtgctacttggagcggctgacgttgagcttgttcttcgaaacctgcgaggggtccagcggctgggcctccggctcgcgcacaatgcgctcgccggcagaggtctggaaggtgcgggcgaactgctcgttaacgcgcaggatagcctcctgggaagcctcgtcgagggcgttgcccccggcgatctgctcgtagacctccggcgcggttgcgcggatctggtcctgcagctcgaactcgtagcggcggacgtcttcaaccggaacgacatcgaagacaccctggttcgcggcccagatcgaaacgatctggaactcaacaggctgcggtgagttctcggactgcttcagcagctcaacgagacgctggccacgctcgagctgcttcttcgaagctgcgtcgaggtcggaagcgaacgccgcgaaggactcgaggtcgcggtaggcggcgaggtcgagacgcaggttacctgcgaccttcttcatgcccttggtctgtgcggcaccacccacgcgggacacggaaatacccacgtcgatagccgggcgcacgccctggttgaagaggtcggattgcaggaagacctggccgtccgtaatggaaatgacgttggtcggaatgaacgcgcccacgtcgttcgccttggtctcgatgatcggcagagccgtcagggagccagcgccaaggtcgtcgttgagcttggccgcgcgctccagcaggcgggagtgcaggtagaaaacgtcgcccgggtatgcctcgcggcccggcggacggcggagcagcagcgaaatcgcgcggtacgcctcagcctgcttggtcagatcatcgtaaataaccaggacgtgcttgccctggtacatccagtgctggccgagcgccgcaccggtgaacggcgcgagccacttgaagcctgcggagtcggaggccggagctgccacgatggtggtgtactccagagcacctgcgtcttccagggtctggcgcacaccggcgatggtggagcccttctggccgactgcaacgtagatgcagcggacctgcttggacgggtcgccggtctcccagaacgccttctggttcaggattgtgtcgatgcagaccgcggtcttaccggtcttgcggtcaccaatgatcagctggcgctggccgcggccgatcggggtcatggcgtcaatcgccttcagaccggtctgcatgggctcctcgaccggctggcggtcaagcacacctgcggcctgaagctcgagggcgcgctcttcgttcgcctcgatcgggccgaggccgtcgatcggctggcccagggggttaattacgcggccgaggaagttctcgccgaccggtacggacaggacctcgccggtcctcttgacattgtcgccttcttgaagggtctcgaagttacccagaaccacgacaccaatcttgtcggtctcaaggttctgcgcgacgccgatgacgccatttgggaactcgagcagctcgttcgtcatgcaacctggcagcccggaaacctgggcaataccatctgcagccgaagtcaccacgccgacctcctcacgggaggcctccgcggagtagctcgaggtgtagttcgctatcgcgctacggatctcatcggaggagatcgtcagctccgccatgttcttcctgctctcggtagtttcttccagcatgtgtacttagtaaagggtcatgttcgctgcgaggtcggtgcgcagccgcgtcagcttgccgcgggcggaaccgtcaatttcctcgtcgccgactcggacgatcatcccaccgaggaggctggggtcaacctcggagtggatggccatctcgcgaccgtaaatgttctcaagcttttgtgcgagggcttcgcgctgagaggaggtgagctcctccgctgcgacgacgcgcgcaacggccttgccacgcaggccagccacgtcctcggcgagtgccgccaagtcgtccaccgggttctgcacaggacgcccgatcacctgaagcgcgagcgcctcggtaaacatggacaccttgccgtaaatcacgctggccagaagaccacgcttttgtgctgcagtagcgttgtggtcggagagcagctgtacgagctccttctccttctccagcaggacggacagctcgtaaagctcgtcctcaacctgctcgagctggccctgttcgtctgcgccgcgcatgagggcgcgccggccaagtgcaaccaagcctgcacggaactcacgcggggtcgaccactcctgggccgcagcgtcaacgaggatctgcttcgtcggctcggccaccttcgggccgaagacgtcgctgatgatgccctcgcgctgcgccgcctcgagagacgggtccgcaactgcgacgcgcagagaacggctggcgtcgagctggtccacgatgaggaacagctcggtgccgacctgcgctgctacggctacggcgttgtcggagttgcggatcagctcatcgagctgaccttccacgtgcgcctgtgcttcgcgactagctgccttcatatcgcctacttcctcatcgacacgtggtcgagctcagagaggaagtcatcgatcgtgttggagcggcgggtagattccgaaagctccatgccaagcagacgctcggcgaggttgatcgagttctggcccatctcattgcgcagctcagagacaacctgctcacgggatgcgagcagctgctgctctccagcctcgagaatgcggcgggactcttcctcggcgcgggcacgagcctcagcctcaatctccttgccgcgtgcgcgcgcggcctcgcggatctcagctgcctcggcacgggcctcagcaagttcagcgttgttcttctccagggcagccttagcttccttttgggcgatttcagcacgctcgatgccgcccttgatccggtcctcgcgctccgtcagcacttcctggaacttcggaatgacgtacttccagaagagcaggaacacaatgaggaatacaacgagcgaccagaccacgtcgtacggtgccggcaggaggagcgacggggtcgattccagcggcatcgtctcggagcccgccgcagcgtcagcggccacgatgaatgcgttgacgttagtcatagggtgctcctgatctaaaaggggttacggggtttgaaaaaacgcgcgtgtgcttttagaacaggaagccggcaacgaagccgatcagggcgagggcctcaacgaaggcgatacccaggatcatggtggtacggagctgaccagccatctccggctggcgagccatgccctcgacggtcttgccaacgagcatgccgatgccgatgctggcgccgatcgtgcccagagcgtagccaatggtgccgaaaccgttgtaggtgttgatggtggtcacggtgtcggttgcctgagcaaggatgatctcgttcatgtgaaagtcgtttcctttctaggtgcgctacggctggggtgttggtttatgccgcagcgcaaatgacaatgtttggggtattcagtttggccggtaggtaagcgctttgttagtgcgcatctgcgtgcagcgacagctcgatatacaccgccgttagaagggcgaagatgtacgcctgcaggaagatgatgagcaactcgtacagggtgaacagaatcgctgcgatcagggtcaggccgctcacagccgtccatgcattcagctgccagaacaagaagttcgtggcggagtaaagcaggacgagaatgatgtggcccgccaggaagttcgccataagacgaagtgccagggtgattgggcgcagaataaaggtcgagaaaatctcgatgggcaccaccaggaagtggagtgccgggggcagccccggaatcacaaccgagtgcttgaagtatgcggcgccgtagcgttgcacacccgcgtagatcatcgtgatgtaggccccaaccgccagcactaacggcataccgatgcgcgaattaggcgaaatattgagccccgggatgatcgtggcggcgttcatgaacaagactgtgaaaaagatggtagcgatcaccggaaggaaccgctttccgtccttcttgcccaaaacgtcctcggcgatatgcacgcggacaaagtccacgcccatttcggcgaagttttgcagccccttgggaaccagttgcggcttcctaaaggcgataacaaagagaagcaccaagatcgccgccacaaacaggcggacgagcatgatgcgatccagcgcgaaccaaccaccagcgaagtcctcgccgatgaactggccgaacgtgtgccccgggaaaaattctggaccaagttcaggggcgtggaacgtccccttcatggctaacgttgtaacgctcagcgttctctcccgttctcgggccgcatccgtgtggaatgcggtgcgatggacgtcttcaagaagactgcctccgcggcggactccgtcgcacatctgctaccgcgggacagggggtggaccatagagcaagggcagacccttcctcgaagtaaacccagcggatagcctaacaggttgatcacggttttcccgtgtcaggggcccctagcaacaccccacctcgccccccttgcactatccggggccgatagagctgcgtacagctagtttccaccgccttgttaactcgatcacaggcgcggttacggcgtggtcagaggcgcgatccaaattgcggccacaggggtagggaaaccagagcgtcgtcaagcaaaaagctctatttcggcgtgatgtacaccgtgcgagcggtgacgattgcccaggtctctgctgcgacggcgaccacaactgctgcgacagtggtgaccgcgagcgccgttgggtcgtagaagctgtagctgcgcagccaatgaaggatgagtcctagcaccaccattttcaccacccagccgccgagaaccaccgcgatcatcacggacggggaagaattcgaggtggccagcgccgacagagcagtggccagcacggccccaccgccgatggctacccccatgattacgccccaaatccccggaaggtcacgcgcgaccccccacgccacgagcgacgccgccgcgagcgcaaccagcgccaaaccgccgaacttcagcgcgcgggtgagcgggctgcgaggatcctcgaactcagccgagtcacggacggtgaagtctggggatgccatgggccacgatcctacacggagcgctaccgctgcccaggagcggagatcttgcctttcgccagtggcaccaaggtggccacaaacgccagcgccagggcgatgacggtaaaggccgccgcgtaccgggtgggcacgatactaaagctcaccgcgccgaaggcgacggccgagacccacatgtagagcaccagcacggtgcgccggtgcgtgtgacccatgcggagcagacggtggtgaaggtgacccgcgtccgcctcccagggccgctggccgcgggcgaggcggcgcaccacagcccacaccaaatcaacaacgggcagcgcaatcgccgcgatcacgacgatgatcgggctgatcagcgcgacgatatcggcggcgccgtaaagcgacatgttgatcttgccggacgcggaaacgctcgcggccgaaagtagcagcccaatcaacatcgcaccagagtcccccatgaaaatccgcgcgggctcgaagttgtgcggcaaaaaccccgcgcacacgcccacaagcgcggcgcagatgatcgcgggcgggtacgcggaaaccgccccgccttggtcgtgcaggacggtgagagcaaacagcaaaatcgccgacccggcgatcatgccgaggcctgcggcgaggccgtcgataccgtcgacgaagttcaccgcgttgatgagcatcacggtaaacaacgcgcttaagacaaccccctggacttgatccaggatcaacgtcgtgcccccacccacgggaacgtagaaaaccgtgaagacaatgccgagcagtgccatcagcacggcggcgaccacctggcccgccagtttcgccagtgcgccgagctcgtagaggtcatcgatcacgcccaccagcacgatggcaaacgcgccggcgaccaccgcggtcatctccggcgtcaccggggcgaacccccgggtgagcgccggcagctgctgcgcgaggaacaccgcggcgacgaacccggtgaacatggccaccccgcccgcggacggggtcggctgcgtgtgaacgtcgcgctggcgaatctccgccacgcggccggtgcgcaccaacagcgagcggaccaggcccgtggccaagaacgtgatcgcggcggcgaccaagagcacgagaccgagctcccgcagcggcacgccggctccgttcatttacttcctccgcatcgaggccgggtcgacgtcgaggacgttaccgatttgctcggcgctgatcgccccctcgcgcaggatgacggggcggccggaggaaatgtccacgatggtggacggctcgccgatcgcggcgtctcccccatccaggtagacgggcaccttggagccgaactgctgccgcgcgtcgccgatgttcaacgccggcgggtggccggagatgttcgccgaggacaccgccatgggcccaacctgctgcaggagctcgatcgcgagcggctggttcggcatgcgcagaagcaccgtgccgcgcgtgtcgcccaagttccacggcaagctgggcgcctccggcacgacgatggacagcccgcccggccaaaacgcctcgaccagcgtcttcgccgtgtcggagaactcgcgcaccaatccttggatggtgctccaggacccgacgaggaccggcaccggcatgtctgggccgcgcattttcgtggccagcagtttttcaactgctgcattgttgaacgcgtcggcgccgatgccgtaaacggtgtcggtcggcatgacgaccaagtcgcctgcgcgaagcgcgtctaccgcggcggcgagcccgtctgcgcgggactcctgtgtcaaacagtcgtaggtggttgcgggcatatgggtagcttactcgctaccacgaagcggctccgacccgtcaggtcttgcatcgcctgaacgtcggtgaaacccccgtctgccttcaggcactcctgcacgagttcggacgtggagtcgtcgtgctcaatgccgatgcggcccccgggtttgagcagccgcttggcgacgggcacgagcccgcgaatcgcctccatcccgtcagcacccgaaaacaccgcctcgtgcgggtcgaagtacacctccgggtcgaggtcgggcgtctcgggcacgtacggcgggttcgcgacaatcacgtccacagtgccgctgagctcggtcaaaagctccgggtcggtcatgtcccccttgtggaactcgaccccttcgccgttgcggcgggcgtaggcaagagcttgttcttgcttgtcgacgcccaccacacgcgccgcaggaacccggcttttgaggtacacggccaaggcgccggacccggtgcctaagtcgatggcggttggggggtttgaggtggcgtcggcaagcaactgtgccccccattcggccagcacctcggtttccgggcggggcacgaacacccctgggcccaccgaaagctcgtgcggaccgaactgcgccgtgccggtgatgtgctgcagcggctcgcgggtagcgcggcgggcgattgccgcagcgtagtcgctctcgaaaccgtcgtagggttcagtgaaacgcaccatgagcggcgcaacgccgagcagcgacgcggcaatctcgcgcgcgtccacctcgggagaggcaacgccggcgccagcgagctcgcgtacggcgtcggcgatgaggctactcagcttcaagtcgctcctggcgctcgtggtcctgcagcgcagtgatcaaatcatccatgttgccgtcgaggacggaatccaggttgttggacttgtagttgatgcggtggtccgagatgcggttctcaggccagttgtaggtgcggatgcgctccgagcggtccatggtacggacctgggaggcgcggccctctgcctctgcagcctcagccttctcgcgctccagctggtccaggcgggcctggagcacctgcatcgcgcgagcgcggttctgaatctgggagcgttcgttctggcaggtcaccacaatcccggtgggcaggtgcgtgatgcgcacggccgagtcagtcgtgttcacgccctgaccgcccttgccggaggagcggtagacatccacgcggagatccttctcgtcgatgttgacgctttcaatctcgtccgcttccgggaagacgtagacgccagccgcagacgtctggatgcggccctgcgactcggtcacggggatgcgctgcacgcggtgcaccccgccctcgaatttcagcttcgaccacgccccgtcgcgcgacgggtttttggacttcaccgcaaccgtcatgtctttgacgccgccgaggtcggactcggcaacgtcgagcacctcccaggtcaaggcgtgcttttcgcagtacttctggtacatgcgagccagatcgcctgcgaacagcgcggcctcctcgccgccggcgccggctttgagctccatgatcacgtcgtcgccgtcgtgctcgtcgcgcggcgccagaaggtccgccagctcctcctccaggcgaacgatctcgccctcgaggcgctgcgcctcgtcggcgaactccttgtcctcgctcgccatctcgagcgccgcctcgcggtcctctcgggcctggttcagctggtcgttgaccttgataatgggctgcagctcggcgtagcgcttggacagcttgcggaactggtcttggtccgcggcgacatccgggtcgcccatctgcgcctggatgccctcgtactcggacacgtagtcatcaacaagcgatacgttttgtgccattagacgtaatcctcctcagtctggtccgcggccatcggcgcggacttggcaacgcccatgaggaactcgccgttggtcttggtcttcttcagctgcttgatcagcatgtcaatcgactgctgcggatccagcgcggagaggatgcggcgcagcttgtgcatcacgcgcgcctcctccgggctcatgagcagctcgtccttgcgggtgccggacgggttgacgtccacggccgggaagacgcggcgctccgcaatcttgcggtccagcttgagctcggcgttgccggttcccttgaactcctcgaagatcaccgtgtcgccggcggagccggtctccaccatcgcggtggcaatgatggtcaaggagccgccttcttcgatgttgcgggcggcgcccaggaaccgcttcggcgggtacagggcgttagagtccacgccgccggagaggatgcgtccggatgccggcgaggagttgttgtacgcgcggcccaggcgggtaatcgagtcgagcagcacaacgacgtcctgacccatctcgactaagcgcttggcgcgctcgatggcgagctcggccaccgcggtgtgttctgacggcgggcggtcgaaggtggaggcgatgacctcgccgcgcacgctgcgctgcatgtcggtgacttcctccgggcgctcgtccaccagcacgaccatgaggtagcactccgggttgttggtggcgatcgcgttggcgatgttttgcaggatcgtcgtcttaccggccttcggcggggagacgatcagcgcgcgctggcccttaccaatcggcatcaccaagtcgataacgcgggtggtgaggatgttcggctctgtctccagacgcaggcgcttgttggggtaaagcggggtgagcttgtggaactccttgcgcgccttcgcttcctccggggtcagaccgttgacggaatcaacgcgcaccaattggttgtagcgctggcggttgcggccgttgccgtgcgagtggccctggccgttcgcacgcacctggccgatgaccgcgtcgccggagcgcaggccgttttgacgcaccagtttgttgttcacgaacacgtccgcttggttctggcggtagccggtggtgcggataaacgcggtgttgttgtccacaatgtcgacgatgccggcgacttcctgcagctcttccggctcgaagctctggttgttgttgtcgttgtggttgttgtcgcggttctgtccgccgtcccggctatcccggttgttgcggttgcggttgcggcggccgcgccggccccggcggccgttgccgtcgttgttgtcgtcgcggttgtggttgttgtcgcggtggttgttgccgcgctcgccgcgatcgctgcgctcgccgcggtcttcacgctcgtcgtcgcgctgcgctgcgtcgtgtttcggggcgtcctgcttcggctcgttgttctggttgttgttgtccgcttccgcctcttcattctggcgggcgcggttgcggcgcgctcggcgcgcggcggagcgggactcgccgcgctgctcgtcgccgccctcctgcgcctcggtcgcggccggtgcctgagcagcttcggtggtctcagcggcgccggtggtctcagccgcctcagcggcgcgcttcgcctttgccggcacctggccggtggtgatcgcctcgatcagctcccccttgcggagggcagaaacgcctttcagcccacgctctgacgcgattttgcggagctcgggcagcttcatcgaagccagatcttggtttgcagccgtattaccttctgcggtcacggatgtcctttcgtcgctaagccagatgcccttgtgcgggaggtggaatgtcccgcggccgtgccggcagctttcgtctattgatatgtcgcgcgtgcccctcgaccgctcgcgcgggcgacaccggcggcgcgaaaccaccttggcacttgttgtgaggggcggatccggcctcgccaatgtgtccaacttcgctaggcggaggttgacgcctgggccgcggagcgcgggccgcaggcgaaatgcagagatccggaagctgagtatagcgcacgggccttatatccatattcgagcggtgttggcgcgtcacgctagagttggccacatgctttcttctatgcaggaggtgccgttttccgtctcccggatcttggagttcggcgccaccgcgcacgggcaaacgaagtgcacgacctggcgcgggagtgccgcggaggagacgacgttttccgctatcgctgcccgggccgcggcgttcgcgaacgccctgcatgaggatctggggatcgacagcgaccagcgcgtggccacgatgctctacaactgctcggagcatatcgaggtgatgttcgccgtcgcgtcgaaaggcgcggtgttcaccccgctgaacgtgcagctgatggaggaccagatcgcctacatcatcaaccactccgaggcgcaagtcatcgtcgcagacccgcgcctggcagagaagctgggacgcgtgcttgaaacctgcccgctggtggaaacggtggccttcatcggcctcgaaccggtggacgagctggcgaaggcgctgcccgaggccacagatgtccgcagctacgaaaagctgctggacggcaggtccaccgtctacccctggcccgagctgccggaaaccaccgccgccgcgctggtctactccaccgccaccaccggcgctccgaagggcgtggcgtactcgcaccgctcgctgtggctcgaggcgatgagcctgcgcgccactgattcgctggccgtcacgcacggcgagtcgtttctgtgctgcatccccgtctaccacgtcctgagctggggcgtgccgctcgcggcgtttatttcgggcgcgccgttggtcctgccggattcggatgtgtcggcgccgacgctggccaaactgatcgccgcgacccacccgcgcgtggcgcacggcgtgccgacgttgtggattcagctcatggtgcactacctgcacaacccaccggagcgcatgagtctccaggagatttatgtcggcggctctcccgccccgcccgggctgatcaaggtgtgggaggagcgctacggcgtggacgtggtgcacgtgtggggcatgaccgagacctccaccgtaggcacggtcgcgcggccgccgtcgggcgcggccggcgaggcccgctgggcctaccgcatctcccagggccgcttcgcgccgtggcttgagtaccgcgtggtcaacgacgggcgagtgatggcatccaacgacctcacccagggcgagatccaggtccgcggcaacctggtggcgaaaagttattaccactccccgacccaggaagaggggcgcatcgcctccgagttccgcggcgagacgatcacggacgagcaggagcacttcaccggcgacggctggctgcgcaccggcgatgtcggcaccgtgacccacgacgggttcatgacgctctacgaccgcgcccgcgacgtcatccggtccggcggggagtggatctactccgcgcaggtggagaacctgatcatggagtcggacatggtggtcgagtgcgctgtcatcggcatcccggacaagaagtggggcgagcgcccgctggccgtaaccaagctgctggagggcacggaacccaccgccgaaaccgcggctgcgctccgcgatagcctcgcagacgtgctgccgcgctggatggcgccggagtactgggcgttcgtgcgctcgattgacaagacgtcggtcggcaaattcgacaagaaggatctgcgcaagcacctgcggcgcggcgagtacgacattattgccctgcccggccccggcagccgggacgcgaagtagaagccctaacatggcaggcaccatggcgcgttctttacctttgaccctcgacgaccagtacggccggaccgcccgggatctgcgggtgagcctgacggaccgctgcaacctgcgctgcacctactgcatgccggccgcgggtttggcgtggctgcccaccgagcaaaccctcactgacgccgaaaccgtccggctgatccggctcgcggtggagtcgctcggcatccgccaagtgcgctttaccggcggtgagccgctgttgcgcaagtcgctcgaagagatcgttgcagcgacgaagcagttgcttaccgacgaaaacgtggcccccaccaccgcgctgaccaccaacgcgctcggtcttgcgcgccgcgcccacgccctgaaggacgcggggctggaccgcatcaacgtctcgctggacaccaccagcccggatctctacgcgaaactgacccggcgcgcccgcatcgacgacgtcttcgccggcatccaggccgcccaggacgcgggcttggcgccgatcaaagtcaacgcggtggtcatgcccggcgtcaacgaggacggcatcgaggacttggtggacttcgcactcgacaattcactgcagctgcgctttatcgagcagatgccgcttgggccccgcgagcactggaaacgcggcgatatggtgacagcgcagcagatcctcgaccggctttcgacgcgcttcacgctcacccccgccgaagagccgcgcggcgccgcgcccgccgcgttgtgggacatcaccgacggtgcgcgccaaggcaagctcggcatcatcgcctcggtcacccaccctttctgcggggcgtgcgaccgcacccgcttaaccaccgacggttcggtgcgctcctgcttgttctccacccaggctgacgaggtctcgctgcgcgacgcgatgcgcgcaggtgcgaccgacgcgcagctcgccgacctctgggcgcaggccatgtgggcgaaaaagccgggccacggtatcgacgagccgggctttttaaagcccgagcgcctcatgagcgaaattgggggctagatgcgcaccatcgcaggtcacactgaggtagtcctcgcgctagcttcgccgaggcgagagagcagattgcttgtcgacgctaccggccacatcctcgccgcccccgcaaccagccggctgagcattcccccgttcgacaactccgcgatggacggcttcatcgcccacgacgccgatttgggcggcgaaggcccgtggacgctgccggttgccggcgacatccccgcaggcgcgcagccggtagactgcccgccgggtgcggcggtgcgcgtgatgaccggcgccgcggtgccgcgcggcggcgatctggtggtcatccccgtggagcaaaccgatgtggcagccgggcccgtgccgctgccggagacggtgacgatccacgcccgcacccccggcagaagccacatccgccgcgccggcggtgatatcgcccccggcgacgtggtggccgaggccggcaccgtgtgcgacgcggctactgtggccgcccttgtttcggccggggtgcgcgaggtggaggtgttcgctcgcccaacggttgcggtcatcaccaccggcgacgagctggtcagctggccggacacgcccgaaggcgcgacaatcccgaactcgaacttgcccatgctcgcacgcatcgcgaaggacgccggcgccgccagcgtcgtggagctacacgccggcgaccgcgcgggcggcgagcacgatttccgccgcgttctcgagcgcgccgcgagccagtacgacgtggtcgtcacctccggcggcgtctcggcaggcgcgtacgacgttgtcaaagaggtcaccgctggtgccaccatgtggttcggacacgtggcgcagcgccccggcgggccgcagggcgttggttcctggggcagcacaccgcttgtgtgcttgccgggcaacccggtggccgcgttcgtctcggcgcatctatacctgtggccgctcgtccgcgcggcggccggtcacacgacagggcttcgtctcaacgagcgggcgcatataagggcgcgcatcggagacggcttcccccagccccaccccgagctcgagcgcgtggtgccggtgacggtgaccttcggtccagagggcgcgcgagcggctgcgttttctgcccgcgcgggctcgcacatggtcggctccctggccggggtgaacggctttgcggttctgccagcgggggcgcgcggcgccgagcccgcgccagaagcggacgtgtggctcacccgcctctagctgccgtagggtcaaacccatggaatttacgcacttgaactccgacggcgccgcctacatggtggacgtgaccgcaaagcagcccactgtgcgccaagccaccgcgcaaggcgaagtggcgtgctcgccagaggtgatggaggcgcttcgcagcggcaccgtgccgaaaggcgacgtgctcgctgtggcccgcgtcgcgggtatcgcggcagccaagcgcgtgcctgagctgctcccgcttgcccacaccatcggcgtgcacggctgcgaagtgaacatcagcttggaagacgaccacgtgtttattgaagcgaccgtgcgcaccgccgaccgcaccggtgtggagatggaagcgctgaccagcgcgagcgtcgcggccctttcgatcatcgacatggtcaagggcgtggaccgctccgcctacatccgacggatggggatcacggcgaaatcgggtgggcgctccggcgactggtcgcgcgagctgccgggggcgtaagcgcgtggtggagtgcggtgtcatcgtgctggccggggggcgttccagccggatgggcgcggacaaggcgcaggtgcacgtcaacggggtgcggctggtggatgcgcttctcgcctccctgccggcggagatgccgcgcgtcgtggtctcccccttcgatctcggttttgaaacggtgagcgaggacccgccgtttggcggccccgtcgccggcatcgccgccggggcgaaggcgcttgcgaccccgctagttgcggtgctggcggtcgatgcccctgattcggtgcggcttgtgccccagctcatcgaggctgtgacaacgcccgacgattcgggggcgctgccggatgttgcggtggtgatggacgacgaggggcacctgcagccgctgtgtggggtgtggcgggcggcgtcgttaagcactgcccttgaagcggtgaacccgcgcgacgcgccggcgaaggcgctgctgcgggctgcgggaagcgtggtgacggtgcgcggcgacggttccgaacgcgactacgacaccccggatcaactggctgagctgggagagatcgagctgcggtaggcgcgcgtgctaggttgaaccggtgatgaaacccgcccgaatcgccgccgcgctcatctgcacaagcgttgcgggcgcctgcggcgctcccgccggcggcgacgggctggtggtgctcggcgccgcgtcgacgcgcgtgatcaacggggagcttgaggcgcttgccgacaccccgctcaccttcatcaacgccggctccgccgcgctggtgcagcagctcgccgacggcgcgccgggcggcgtcctcatcaccgcagacaagaagaacatggacgacgcggagaacgcgggtcttgtgaacgaccctcgcgaggttgcccacaacactatggtgatcgctgtcccagccggcaacccggcggggatcgaaagcgccgcggacgtggcgcgcgagggcgtcaacctcgtgctgtgcgacgaaaacgtgccgtgcggcgccgtcgcccgcacgctgctcgacgcaaacgggatcaccgtgaaacccgcgtcacgcgagcacaacgtgaccgacacgctgggcaaggtcacctccggcgaggccgacgcggcggttgtctaccgcaccgacgccatcgccgctggcgaggccgtggagaccgtcgagatccctttcgccgaggaccaccccaattccctctatgcggcggtcgtttccgcgagcacccgcccggacgaggcggctgccctcgtggcgctacttaccagcgcgccgatggcagccgtgtggcaggaccacggcttcacccccgccgcggacgcggcgaagtagtttgccaatgggcacgcggcgcgggcagagcccagcggtgatactgctgggcttcatcgccttgaccgtgattgtgctgccggtcgccgccctcggcacccgcgtgccgtggggagagctcggacagattgccgccgcaacggagacccgcgagcttttgggggtgacacttacttctgctgtccttgccaccgcgatcagtgttcttttgggcacgccgctggcactgttgctgcagcgcatgcggcgcggcgcgcacctcgcccgcgcactagtgttgttgccgctggccatgccgccggtggtggcgggtctggcgctgtcggcgtttatcgggcggcgcggcatcgcggcaccgctgctcgacgccgtcggcgcgcacttcgcgttcgcgtttccgggcgtggtcgccgcccacgtctacgtcgcgctgccgttcgtggtgatcaccttagattcggcgcttcgacagctcgacccggaaatcaccaactcagcggccgcggtcggcatcggcgagcgaaccatcatcagccgcatcgtgctgccggcgatcgcgccatctttggccacggcggcaggtctggccttcgcccgctcgctcggtgagttcggcaccaccctcactttcgccggctccatgcccggggttacccgcacgatgccgctcgggatctacctcgcccgcgaaatcgaccaggacgtcgcttacgggctcgcggctatcctgatcacgctcgccgttgccgcgctcgccctcgctgccctaccgaggctgttccgccggccggcaccgacgccccgcgtgcgagcgaccggggtaatcgatgtcgcgaggcttcgggaactgacgcgaccgcgcgccaccggcgcagttgcgggttttcccaccggcgccaccaccgcgctcatcgggccgaacggcgccggcaaaaccacgctcctgcgctcgcttgcggggccgggcgttgtcttgctcacgcaaaaccccggcctgccgcccacgtcgacgccgctgaaggccatcgcgatggtcacccaagactccgcggcagcgcgcgagctgcttgccgcggctggcttgcgcgagctcgcccacgtccccgtgccgtccctctccggcggccaagccgcgcaggtggcgctcgtgcgcgcgctcgctgcgaagccgagctcactgcttttagacgagccgcttgccgccatcgacgccgccgcagcgggaagctggcgcgagctcttacgagccgcctccggcgaccggaccaccgtgttcgtgacccacagcggcgcggaacttttccagctcgccgaccacgtcgcggtcatggagcgcggcgaggtggtcagccttgcccccgcggacgcggagcgcgacctgccggcgacggcgttctccgcccagctgcagggcctcgcccgcgtcgagggcaccgcgcaggctgctaccgcggctggcggcgaggccatcatcgaaagcgaggctggacaactgcgcgggcacgcggcggcagcgttggcgccggggcaagccgcggtcgcagtctacgacctggccgatccggagaacgtccgcatccacccggcgcgctaacggtgttcgcgcctatccgccggcgaacggcgggagcacgtcgacgcgctcggccccttcaagtggggtgtcgggggcggcgcggtggccgtcgacaagaaagctgcagcgcgcaaggatcggacctagctcggggtggcgctcggcagcgtcagcaagcacctgctcgagcgttgcctgcgtgtccgcctcttcttccgcgacaccagcggcggcgcgagcggccgcgaagtagtgaatacgcatacgactacagtagcccccatgcctgtgagcccagaagcgcacctcaacgcggtgcaagagctagtcacagcccacgcgccgaacccgcgcacgcagcgggtccttgccgccgacgcgctcggccgggtactcgcccgcgacctcgtggcaaatggcgacatgccgccgttcgacaactcccaaatggacggctacgccctcccccgcgccggggccgcggtatgggaggtcggccccaccgttgcagccggcgcggaccctgacgcgatctatccggacgggctgggggctaaggcggcgccggtaatgacgggggcgaaactgccccgcggcaccgcagccgtagtgccggtcgaggcgtgcgagccggccgagttcgtcggcactggcgataccgtgacggtccccgactgcgcgccgggccagttcatgcgccgcgcgggctccgacgtcgccgcgggcgacgtgatcgcgccggccggcacgctggtgaccccggttgtggctggggtgctggcgtcgcagtgcgtcgaggaggtggaggtgcgcgcccgccgccgcatcatcatcgtcaccggcggcaaggaggtcggcggcgcgggcgcggcgcagatcccggatacgaacacgccgatgctggaggcgctggccgcgcgccacggcatcgaggtcgccgcaaccattcgcaccgatgacgatccggaggcgctggctggggaggttgaacggggcgtcgacaagcatgctcccgatgccatcgtgacctccggcggcattagccacggcaagttcgaggtggtccggcaggtctttgctgacgggtggtacggccacgtcgcgcagcagcccggcggcccgcagggacgaagcgtctttcgcggcgtgcccgtggtgagcctgcccggcaacccggtgtccacgctggtcagcttccggctttttgtcgccccggtgctcgggcaggcagacgagccagtgtgggcacccgtctcggaagccatcacgggcttggaaggccgcgagcagttcctgcgcggccggatcacccacggccgcgcgacccctatgggcggcgcgggctcgcacctgctcaaccaagccgccgaggcgacgtgcttgatccgcgtccctgccggcaccgagcttgccgaaggcgacctcgccctcatctacccgttgtaaggtgatacgtaatgaatactgcacgagtcattgtcgcttccacccgcgccgccgcgggcacctacgaggacaaatcaggcccggttgccgtcgagtttttgcgccgcatgggcctcgacaccccagaggcgacggtggtgccggacgccgagatcggccgcgctgtgcgcgaggcgctggcgacccagccggcggtgctcatcacctccggcggcacggggctgacccccgacgacctcacggtgaagactatcgcgccgcttttggataaggagctgcccggcatcacgcaggagttcttccgccgcggcctggccagcaccccgaccgcgatcctctccggcgcggtggcgggtctggccgggcgcacgttcgtgatggcgcttcccggctcccccggcggggtgaaggacggctgcgcggtgctcgagccggtgctgccccacatcctcgagctcaccggcggcgaccacgcgtcccacccgcccgcggacccggactacgtggctgagcagacgggcgtggtcgttgacacggtgctccaggacagcccgctggaggacctcgccgcgcgcgccaccgagacgacgctgaccaaggcgatgggcgcgctggtgcgcttcgacggcatcgtgcgcgaccacgacggcggcgagcgcgtcgcagccctgtcgtacgagtcgcacccgagcgccgctgacgagctgcgccgcgtgtgcgaggaggtggcagcagagcaccccgtgcgcatcttcgccgcccaccgcaccggcgaagtcccgatcggcgagctcgcgttcctcgtcctcgccgcctccgcgcaccgcggcgacgcgttcgccgcctgccagagcgtcgcggaccgggtcaaggccgaggtgccgatctggaaggagcagacgcttgtcgacggcacgtcccactgggtcggcatcaatggataggtacgcgcgccaggtcgcactcatcggcgacgacgcccaagccgccatccgaggcgcccgcgccggcatcatcggcgcaggagggctcggctcacccgcggcgctctacctcgcggcggcaggtatgagcatggtgcttatcgacgacgacgtcacctccaccaccaacctccaccggcaaatcctccattccacccccgccgtgggcactccgaaggtggagtcggcggcgcgtcgcctccacgatctgaacccggacgcccaggtcgagaccgtgaagacccggctgacgtgggacaacgcgcttgacatcctgtctggctgcgacgtgatcctggacgggtccgacaacttcgccacccgccacattgcctcccacgccgctgcgcgcctcggcatcccccacgtgtggggttcgatcctgggctacgaagcgcagatcagcgtgttccacgcttcccgcggccccgtctacgaagacctcttccctgccccgccgccgcccgggtcggtgccatcgtgctcccaagccggagtgctcggccccttggtcggcgtcgccggttccgcaatggcgatggaggcaattaagctcgtcacaggcctcggcacgccgctgatcggccgcgtggcctactacgactcgctcgccgcgtcgtgggagcacatcccgctcgcggccgacccagcagtaacggaaaaggtgctgaccagtgctccgccgacgggtccagccgaggtggcgctgaatgacatcaccccggcgaccacggtgatcgatgtgcgcgaaccgcacgagttcgccgccggccacctgcccggctccatcaatgtcccgcttggcgagatcctcgccggcgccacccccgacgagctcgaaaacggcggcgtgatcgtgtgcgcggcgggcgtgcgctcggcgcaggccgtcgccgcgctggaggcgcgggggctgaccgggctggccagcctccgcggcggtctacacgggtagcgccgcgcagaacactaaacccgggtcagctcagcggtggcggggcctgcaatctccaggttcagcacgcgcaggccggactcgcgggcctcatcgagcagcgcgggcgcgatctcgccggtggtgagcaccatagcggtcggccccgcgccggagaggaacgcggcgtggccgcggttgcgcaggcggttgacccactccgccgtcaccggcaacacgtcggcgcggtacggctggtggagacggtcgcgggtaccttcccacagaagctccgggtgggactgcagggccgcggtcatcaccgcagtgcgcgagacgttgaagcgcgcatcgctgtgggtgacgtggctcggcagcacggcgcgcactgccgtggtcgaggcgtgaaagtccggcacgagcgcaaccgcgcggattgaggagtccaccgggatgcgcacggcgcggtactgcggcttggactggccgtcgaccgggatgtcggtccagctcaccactgccccgcccagcacggacgcgccggcgttgtcggggtggccctcaaactccgacgacagttgcaccactgtcttctggtccagcggggagccggcaagcgtgttcgcggcgaccacgccggcgaccgccgcagctgccgaagatcccagcccgcgcgactgcgggatcgagttgtggcacaccacgcgaagacccggggcagcaacgtccgaggccttcaagccggagcggatcgccttgaccacgaggtgggagttgtcgcgtggcagctcgtcggcgccctcgccgaagatttccacttgcaagccggattgggtgacttccacctcaacggtgtcgtagacgccgaccgcgaggccgagcgtgtcgaagccggggcccaagttcgcggtggacgcaggcaccgtgacggtggcttttagcccaacttcaagatcgattgccatggtgtctcctcgttgcggctctagtcgtgcaggcgcagcacggagttcaccgcgcaaacgtcgtcgtgggtcttcagcttctccacaatcccgcgcaggttgcgctcgctggccctgtgcgtgaccacgatcaggtgcgccccgtcggcagattcctcctggcgcacagcggcgagcgagacctctgcgtcggcgaagtggcgcgccaagtccgcgagcacacccacgcggtcgttgaccgtcatgttgatgtggtagcgggtctccacgtcgtcgaaaccgacgaccgggtagttcgcgtaggggttctccgcaggcgcgcgaccgccgtggatcttgttgcgggcggcaccgaccaagtcgcccagcacggcggaggcggtcggcgcgccgccggcgccgttgccgtagaacatcaggcggccagccgcttccgcctcgacgaaaatagcgttgtagctcttgtccaccgtggcaagcgggtgctcgttcggcaccagggtcgggtgcacgcgggcgttgacggcgcgggtggtgccgtcttcgttcaccacccgctcgcagatggcgaggagcttgatcgtctggttcgccttctttgcggcggcgatgtcttcggcggtaatggagctgatgccctcgcagtagacgtcgtcgaaggtcacgcgggtgtggaagcccatggacgcgaggatcgcggccttggaggcggcgtcgtggccctccacgtcggcggtcggatcagcctcggcgtagcccaagcgcgtcgcctcggcgagcgcgtcctcgtaggaggcgccggtggacgccatcgcgtccaggatgaagttggtggtgccgttgacaatgccggcgatgcgctgcacctggtcaccggcaagcgagcggcgcagcatgcccacgactgggatcgcggcggcgacggcggcctcgtagtagaggtccacgcctgcctcgttcgcggcgtcggcgagctcggagccgtgggcggcgaccagcgctttgttcgcggtgacgacggacttgccggcgcgaagcgccttgagcaccagctcgcgcgggtagtcgatgccgccgatcagctcgacgacaacgtcgacgtcgtcgcggtcgatgagggatagcgcgtcgtcggtaagcacgagcccctgaacctcgggggcgtccttgtgcttctccacgttggagacagccacgccgcggacctcgatcggcccgccgatgcggttttccaggttggaggaaaactcgccgatgaggcgcagtacctcggtacccacggtgcccttgcccaaaatggcgacgccgactggttcgccgacgcccttgccggggtagttgccgttgctctcagcagctgtcatggggtctcctcctgatttttgtgacgcgtcgcggcgtgcgacaacgccatagtgtaccgcttagtctatttcgtggctggttagtattcgcgggccataatgtcgtccaccgtctcccggcgcaccatcggggtgacgcgtccgccgcggacggacacgactgcggggcggccgaaggagttgtagttggacgccatcgagtagcagtaggcgccggtagccgcgagcgcgatgaggtcgcccggggcaatatcgtcgggccacttcgcgtcctggacaaggatgtcaccggactcgcagtgggagccgacgaggcgggtggcggtgggctccccttcggtgaagcggttgaccactcgcgtgtcgtacagcgccccgtaaagcgacgggcggatgttgtcgctcatgccaccgtcgatggcgatgtaacgcctcgtggtggtgtaggacgtgtccacatccttgatcacgcctgcagtgtagacggtgactgcagcaggtcccgcgatcgcgcggcccggctccaccaccacggtgggagcggcgatacccagctcgtcggcagcttcctgcaccgcggccagcaggtcgcgggccactgcctccacgtccaggggctcctcccccggcatgtaggcgatgccgtagccgccgcctaagtcgaggtagccgagcgcgactccgcactcgcggaagatgcgggcgtagagcgccagcacgcgctcggcggcgagcttgaagccttccgcgtcgaacacctgtgagccgacgtggcagtgcaggccggtcagctccagccactcggagttgatggcggtgacggccgcgtcgtaggccgcgccagaggccatagagataccgaacttctggtcctcgtggctggtggcgatgaactcgtgggtgtgggcgtccacgccgggcttgacgcggacgaacacgtcctgcttgaccccggcttcgcgcgctacggcctccagctggcgcagctcttggtgggagtcaatcaccacgtggccgacgtgtgcgtcgacgcacaggcgcagaaaggcgtcggacttgttgttgccgtggacggtgatgcgctccggcggaaagtcggcggcgagcgcgatgcgcagctcgttctcgctggctacgtcgagggcgaggccttcttcgtccacccagcgcgcaatgcggcgcgtcagcatcgccttggacgcgtagtgcacgttggcaggcgcgcgaaacgcccgcgccatgtcgcggcagcgggagcggaagtcgtcctcgtcgatcaccatgacgggcgtgccgtactcctcggcgatctctgtcagcgggaccccagcgatggtgaccacgccgtcttcctcgcgcttggcgccgcgcggccacacgtgcgcgggcaggtcgttgaacccagcggtgtcgtcgccgaacggggtggagatgaaaacagtcatctacatccgctccggtgcgctgacacccagaaggtgcagggcgttggcgagcacctggcgggtagcctgtgcgagcgcgaggcgcgccgagtgaatcggctgcggcgcttcgccagccttcggcagaatctggcacgcgtcgtagaacttgtggaatgcgctagccaaatcttccgcgtagcgggccacgcggtgcggctcgcgcagctcggcggcggccttcaccacggccgggaactccccgagcgtgcgaatcaggtcgccctccttctcgtgctcgagcaggccgaagtcgacatccaacccgcccgcggaacgcgcgacgctgacgcccgcgtcggctgcgcggcggtcgatcgagcacaggcgcgcgtggccgtactgcacgtaataaacggggttgtcagaggactgcgtggtccacaggtccaagtcgatgtccagggaagagtcgaccgaggagcgcaccagcgcgtagcgggcgccgtcaacaccgatcgcgtccacaaggtcgtcgagcgtgatcacggtgccggcgcgcttggacatcttcaccgcctgcccgtcgcgcaccaggttcaccagctggccgatgagcacctcgacggcggccgggtcgtagcccagcgcctgggcggcggcgcgcaggcgggcaatgtagccgtggtggtccgcgcccagcatgtagatcgccagcgtgtggccgcggtcaaacttgtcggccacgtaggcgatatcgccggcgatgtaagccgcgttgccgtcggacttgatcaccacgcggtccttgtcgtcgccgaagtcggtggagcgcagccaccacgcaccctcggcctcgtacaggttaccgttgtctttcagcgtctggatcgcgcggtccaccgcaccggactcgaacagggagttctcgtggaaatatacgtcgaaatcgacgccgaactcgtgcagcgactccttgatctgcgcaaacatcatctccacgccctcggcgcggaagcgctcctgcacctcttcttctgtcccggaaagagcttcaggatacttctcgacgaccgcgcccgcgatctcagcgatatacgcccctccgtacccgtcttcgggagtcggctcccccttcgccgccgctaccagcgagcgggcgaagcggtcgatctgcccgccgtggtcgttgaagtagtactcgcgggtcacgtccgccccggaagcctcgagcacgcggccgagcgagtcgcccaccgcggcccagcgggtgccacccaaatgaatcggacccgtcgggttggcggagacgaactcgaggttgatcttctccccgttcaaaagctcggagcggccataggcctcgcccgcctcgaggatctgcgcaaccagctggccctgcgcgtcagctgcgagacggaggttgatgaaccccgggcccgcgatgtctgcggaggcgatggctgggttgttcaacagtgcgtcgacaagcagctgccccaactcgcgcgggttcatgcccgccttcttcgccacctgcagcgcgatgttcgtggcgtaatccccgtgctcggggttgcgggggcgctcgacggtgacctcctccgggagcacggaggtgtcaaggtcgcgcgcgctgagcacgtcgaatgtgagctgccggatggtggcggcgaggtctgctggcgtcatgggggccaagtctacgtcaccccatcgctacccccgtgcgccagtccttccaaattttcgctttcaagtgacataattcgccgtgtcatttttttgtgatctcccgcaactttttgaggagcctctatgaaccaattccaggttgtaaccgacgcgatcggcggcagcgtcggcctgtcggctctggtctcaaccctgccactgctgaccttcttcatcatgctgctgggcttcaaggcccgcgcgcacacctccggcgccgtcgcgctggtcgtggccatcctggtcgcgatcctgggcttcaacatgcccaccaccatggccctgtcgtccgcgctgcgcggcggcctattcggcctcttccccatcgtctgggtgatcctcacggcgatctggttctaccaaatcaccgtggcctccggccgcttcgaggacctgcgcctggtctttgacaagatgggcaacggcgacgtgcgcatccaggcaatgctcatcgcgttctgcttcggcggcctgcttgaggcactcgccggcttcggtgcgccggtggccattaccgccaccatgatcctggcgctgggcatcccgccgctcaaggcggccaccatcgtgctgatcgccaacaccgcgcctgtggccttcggcgccgtggccatcccgattaccaccgctggtgaggtcggcggccgcaccgtcgagcagaccgagaacatcgccgccatcgtcggccaccagaccccgctgctcgcgttcttcgtgccgttcatcatcgcgtggcttattgacggctggcgcggtgtgaaagagaccgcacctgcggcgttcaccatcggcctgaccttcggtatcgcacagtggtggacctccaaccacttcgcctaccagctcaccgacgtcgtggcctgcatcgtggcgcttggcgccgcgttcatcctgctgcgtttctggtccccgcgcggcgtcaccgaactgcgccagcgcctcaacctgccggcccagccggaggaggaagtccacctgccgggcaaccgcgtcttcatggcgcttttgccctacgccgtagtcgtcatcgtcttcggcctagccaacctcggcagcaccctgccgaagtggctcagcagcttcaagatcagcttcccgtggcccggtattgagaccggcacgctgctgaacgcagctggcgacgaggtcacgaccgactactcgttcgcgtacctgaacaacccgggcaccctgctggtgatctccggtctgatcgtggcggtcatctacatgatcttcaacgagaacggccgctaccgcctcacctggggccaggtgggcaaggagttcaccgacaccgcctaccgcatgcgctggtccgcgctgaccatcgtgttggtgctctcgctcgcgtacgtgatgaactactcgggccagaccgtgaccatcggcgagttcttcgccaacctcggaggcgcgttcgcgttcttcgccccggtgctgggctgggtcggcgtggccgtgaccggctccgacacctccgccaacgccctgttcgccaacctccaggtcaccgccgcgaaccagctgggtctgaacccggacctgatgctggccgccaacaccaccggtggcgtggtgggcaagatgatctccccgcagtcgcttgccattgccgctaccgcggtaaacatggagggcaaggagtccgagatcttcaagaaggtcgtcggctggtccttcggcttcctcgtcgcggtgtgcgtgatcgtctacctgcagaccggtattttgagcggtcttgcgccgattgttgaataagcgagtaagatcacacctgttccaaggtgccccgctcaccctctgggcgagtggggctttttgcgttcacccttgttttcaatctgtttaaggagccaacatgcgagtagcactgttttctacttgtatcggcgacgccctgttccccgacgcgcacaaggccaccgcgctggtgctgtcccgtctcggctacgaagtggtgttcccggaatctcagacctgctgcggccagatgcacgtcaacaccggctaccaggagcaggcaatgccgatcgttgagacctacgtcgacaccttctccgacccgtccatcgattacgttgtcgtcccctccggctcctgcaccggcgccgtgcgcgagcagcacgtgcagctcgctgagcgattcgggagcaaggcgcttgttgacggggcgaagcaaacctccaagaaaaccctcgacctgtccgagttcatcgttgacgtggccggcacctacgacgtgggcgcgttcttcccgcaccgcgtgacctaccactcctcatgccactcgcttcgcttcatcaaggtcggcgagcgcccgaaggagctcctgcgccacgtcgagggcctcgagctggtagacctgccgaactccgaggagtgctgcggcttcggcggcaccttctccgtgaagatgccggaggtttcctccgcgatggtctccgacaagacccgccacatcaaggagaccaacgcggagtacgtcaccgccggcgactcctcctgcctgatgaacatcgctggcgcgatgagccgccaacactccggcatccgcgccgtccacatggccgagatcctcgcctccaccaaggagcacccgtggacgcctgagtccgccgcgtactcgaaggagaaaatgctgtgaaagttgcacttggcaaaccgcaaatgccgccgcacgccgtcggcccgaaccacctgcgcggcaccgagaagtttcagaaggccgcgcacaccgagctggacaacgtaaccaagcgccgcaacctgaactacgccaccaccaccatccgcgtgaagcgccagaaggcggttgaggagctggatgactggcaggatctgcgcaacaccggctccgccgttaagcaggacgtcattgcgcgcctgccggagctgctcgaggagttcgagcgcaacgtgaccgcccgcggcggccacgtccactgggcgcgcgactcccgcgaggccaacgacatcatcgctcgcctggttgaggagaccggcgagaaagaagtggtcaagatcaagtcgatggccacccaggagatcgcgctgaacgaggagctggaaaagcgcggcatccacgcccaggagaccgacctggctgagctcatcgtgcagctgggcgaagacttcccgtcccacatcctggtgccggcgatccaccgcaaccgcgccgagatccgcgacatcttcgtggacaagatgccgaacacggacgactcgctgacggccgaccccgaggaactggctgacgcttctcgcgctttcctgcgcgagcagttcatgaaggcgaaagttgccatctctggtgtgaacttcggcatcgccgagaccggcaccgtctccatcgtggagtccgagggcaacggccgcatgtgcctgaccatgccggagacgttgatctccgtcatgggtattgagaagctgctcccgaagttcgatgacctgggcgtgttcatgcagctgctcccgcgctcctccaccgcggagcgcatgaacccgtacacctccctgtggacgggcgttactgagggcgacggcccgcagaacttccacatcgtgctgctggacaacggccgcaccgccgccatgtccaacgagatcggccgcgaggcgatgaagtgcatccgctgctccgcctgcctgaacgtctgcccggtgtacgagcgcgccggcggccactcctacggctccgcttacccgggcccgatcggcgccatcctcaccccgcagctgaccggcatcgactccgcagacgacccgaacagctccctgccgttcgcgtcctccctgtgcggtcgctgcaacgaggtctgcccggtgaagatcccgatcaccgacatccttttggagctgcgctaccagaaggcgaagaacgagccgacccgctgggagcaggctgggttcgccggcatcggcttcctgtggggccacccgaaggtgtggaaccgcgccgtgcgcatggtcgcgctcggccgcgtcctcggcggctttaacggcgaaatcgagaccatgccgccgccgatctccggctggacggagtaccgcgacgtggctgtgccgccgaagaagtccttccgccagtggtgggacaccgaggaggcccaggagctgctcgccaacgcacgcaaggaaggcatccccagccgcgagggccacgccgatatcgaagagttcatggatacgccggaggagttcaagtaatcatgacgacgaaaatttcttccaacgcgtcccacggtaccttcggtgacgacgagcgccgcaacgccgatgctaagaaagaaatgctgcgccgcatcaaggacgcgcagcagctggccaacactccgaagcacgtcgatgtcccacgcgagtacaacaccagctctgacaagagcccggaggagctgcgcgagatcctgatcgaccgtctggtggactacaaggcctccgtggtggagaccaccgaggagaacctggctaaggacatcgccaaggcgatcgaggaccgcggctgggacgaggttgtctacgcccccggcctggacgagaagctcttcgagcacgtcaagggcagcgtccgcgccgacgacccgtccaaggatccgcgcgacctcggcgacgtggttgccgtgaccgactcgcacgtttcctgcgcggtcagcggcaccatcgtgctgcaggccgatgatgtctgcggccgccgcgccctgtccctcgtcccggaccaccacgtgtgcatcgtccgcccggagaccgtggtctacggcgtgccggagatgttcgaccgcatggacccgtacaagccgaacacgctgatctccggcggttccgcaacttccgacatcgagctcgtgcgtgtcgagggcgtccacggcccgcgcgacctggtcgtgatggtgctgagctagacagacaaaacggccagccacgtccctttgcggatcgtgactggccgttttgctgtcattgtttcccgtgccacgctttcgcgcgcagaagtaagtatggcggatcaaccgtcgagcacaatgggcctgccctgtgtgtttctcacgtattgggtgccagcgtgctggaatctacgcaatttcggtgccggcgcacgtcggtgctagtcttggtcagtcggagatttactccggtgatgtcttcgtagctcagtggattagagcatcggtttccggtaccgaaggtcgcaggttcgaatcctgtcggggacacagtgtgaagtctcgagacatcgttcctacggtgtctcgagatttttcgttttggggttgcccgggggttgggcgagttcgttgtgggatcggttgtagtagatgcggtcttcggtgagtgtgtaggacgcgatttgttccccggtggtggtgattttgatgtcgacgtggttatcgacgatgaccattgtgatgggttctccgccccagcgtctcccgatgtagaggcgtcggagttggccgcgccagcgcagtgttgctttaccgttgttgccgactttgtcggtgcgtaggcgaaagtcttcggtggtcttgatgaggggtggtgcggcttttggcagtgcggtgtatgcctcgagcggtgtggcttggccgagtgctctgtgggggcgtgttcggttgtagtagtcgatgatttcgtcaatgtcgttgttgagtctttcgatgcttgtggcagggggtaaagcggcgagtgcgagtttgagtgtttggtggaagcgttctacttttccctgggtttgggggtggtagggtttgccgtttttctgctgtatgcccaggtcgaggaggagttgttcgaagccgtttcgtgatgggttggttctatcgccgctggtagtgaaggctcgtccgttgtctgtgagggtggattgcgggtagccgttggtttcagcggcgtggatgaaactgtcgatgacgtttcctaccgtggcgttgctaaatgctttgcagtagaggacgtagcgggagtggtcgtcgaggattgtcaggattgcgacacgccggtggcctgcgatagaccagtcgctgtagtccatttgccaggtttcgttgggttggtcggcttcgaacctaatccatgagctgcgtgggcgtttttaaggctggggtgtgacgtagccgttgttggaaagtatgcgatggattgttgatgcagctggcggcgggtccacgccttcttgttggaggtgccagcggatggtgtgagcgccggcgtctgtgccgcggctggtgagtgtttctcgcagttcgatgattcgtttaacaacggtgtcgtcggtggcgcgggggttggtgtgtgggcgtttggatttgggttcaagggcggggaaaccaccttcgttgtatcgcttttgcagtgtgcgtacccagcgagtggagacgttgaagtgtgctgctgtttcggcctggttcatgccggtgatgagcatggtttcgatgatgattcgcgggcttggcttctttttgttctccattggttaagcatggaggaacgatgtctcgagacagctgattgcgggaccccggggcacttctgtcgaggagactgcccaccggtacggtgtatcgagacatgtacacaggaaaggccggaacagtgtcacgagacatgcggaacgatgtcaccgaaccagacactgtcggggacacaatatgaagtcacgcagggggtttcacgaaactgttccaatcttttcacgaaaccccgcgccagccgaaagaaaacggccgcgaacacaaaagtgacccgctccgttcgttcggaggggtcatttttctttgtctgaacgccgttcctgcacgggttatagcgcggattgtttatgagcgcggaccgagccacggaagagtttccgtactcatctggtggcgcggtttttgcagcgcttcatagcggtcttgttgctgtgatcacgcaggactggctgcgggtagttgttggggtctgaaccgagaggggtgcgcccggtcggggccgtttggaacactgctgctccgtcagagcccgaaggctccgccactgacgaggatcacgatgccgaggccgatgagaacgatgggaaagaggatgtcctcaaagcgttcgagcacttccgcgatcggggggcgggtggcgacgaactttgccagggccaccaggaccgcaacgagcgcgaggaagataacacagtaggcgactactgtgagaggttccacgctgaggaatacaggggtgtagacgccgatgttgtcgccgccattggcaaaagtgacgcctgcgactgtccaaacgccgaccttcttgccggcaaccttggcctcgtcgtcatcgtcgtcatcgtctccgcgccaggcctcccatgcggcccagaggccgaggcccagagggatgagaccaaagtatgggatggctgccgggggcaggaatgctccggcaccgatggtcacaaggatcgcggcgacgaggatgccggcaaatccgaggtactggccggccagaatacgggcggtggtgccgctctggcctgcccctcgcgcgaagaaaagggagagcacgatgatgtcgtcgatgttggtaactgcgaacaggcctatcgcctgcaagaccgtggtgagcattacgcgccctccccagctacgtcgcatccgggaaccgagcaggcgggatcgatgcacggggcatcttcgtctactgccaaggtggcatcgaccaatgtagtcagcgcctgcgccaggtgcggatcggcgatctcatatcgcgtccgacgcccctcgggctcggagacgacaatcccacaatcgcgcaagcatgccaggtgattggacacgttcgagcgtgtcaggtccagatctcgggacagttccgccgggtaagcgggatggtcgagcagggtcaagatgatccgggatcgagtggggtcggccagtgcacgacccaggcggttcatcacgtcgagacgcgaagcaatagtcagcatgcactgaactatacagcgagcactgaactagtcaagttccgggtagcggtacagctgtgtgtgctgctcaagagacagtggaagtagcagagatggcagagattccggcaaagttgcgaaaacagcaccgccagcctggacaccggtaacgaagagcgcgacggtcacgtgcgcagcgacgacttcttcgccgtcgagcagttcccggagatgacgtttacctccaccagcttcgacgttgacgcttccggcaacggctcggtgaccggcgacctcaccatcaagggcaccacccgcccggtgaccttcgaggttgaaaccttcggcgttgaggaggacccattcggcaacacccgcatcggcttcgaggcgaagaccacgatcaaccgcaccgacttcggcatcgacttccaggcaccgctgaactccggcggcatgctcgtcggtgagaaggtgggtatcgagatcgagggctcgggtattaagcagtaaagggggcgtcgctaagcaaagccccttataacggcggatccgctattcgcgaacctgccgttaattttgtctgcgcgcgtcgatgtccgccacaacctcctctgggcgctcggcggaggcaaggtacgtcgtggtgcgggtatcgatctgcaccgtcggcccaccgacgatataggccgtggcgtttccgacggcgcgcgggcctgccccctcgatgagaccggtgtccgggccgacctgaacgctggtgatagtgctgaggtttaccgagtgggagaagcccagcaccgacatagtgaccgcctcgtcggacaccgtgattgtggtgcgcattgcaacgcaagcaaccgtaaggccgacgagggcgagggcgaagatgaccgctgcgggattcgagtcgaccaacatcggagccagcgcagcggtaaccgctagtgccgcagctaccgccagccacaggatcgggccgttcagtcggcgcgtgtacacggactcggacatgccggacagcgtaggcgcgccgcgggaaccgtgcaaagctgttgatacttttgtggcatgcacatgccgccaatcggactcatcgctctgcagggaatcggtgttgttgtttttgtgctcatcgcgtgggtgctaacgcagcgacggatgggatttccgtggtctgccatcgggtggggcgcgctgtcgttcccgctgtcgcagattgctcgactcgccgtgattacaccgctgaacgtgctgtgggcccagatcctctcccccggtgcggcggcgacggcgacggtggccacgatgttgatcagctcgggcttgtttgaggagacaacccgctgggtcgtgttgcggttctggacgaagagcacccgcgcgtggcgcgaaggcgttgggttcgggttgggccacggcggcatcgaggccatcttgatcatcgcgggcacggcgctgacgaacgcggtcctgatgatgaactcggatgcgattgtagaaagcgtggccaagtccggcgacccggccgccgctggagcgatcggtcaacagatcgatacgcttaagcagctgacgtttacagacatcggactgagttggtacgagcgtgtgcttgcggtggttgtgcacgtcgcgttcacgctgatcgtgcttcgcgcggtgcgcgagcgcaggtggcagctgtggctgctcgccgtcgtcgcgcacatcgcgttcaacgcggtggtggtggtcgtcggcgcaccagcgggtgcgttggcggtgtacgcgatcatgacggtcgtcgcagccgttgcactgtggactgtagccttcggcccgctgtcgcgccgcgcagtggaaggcgcgggggctagagcccgttaaaactcagccgggatgacgatccaagacacgacgtaggcgaggaaacccggcaggaacccggcgagcgcgagcaggacgaagacgatgcgcacaagcgtcgggtcgacgttcaagtactcggcgaagccgccacacacgccggcgatgaccttgtcggtcatggagcgggtcagccggcgcggcggctgcgggttgttgtacatggggtacggagaagacatcagatacaccctttcgatgagactctagctgtcgttttccatcctattgtccaccgcgagtactgcgtcgacgaatttctgcacatgggcgcgatcggtgctggtagtcggtgcaaaaatcagtcggcgcactgtctcgacgtggttcggcacagcgtcctcgaggcgttccagcccctccgctgtgagcgccactgtgacaccgcgggcgtcgttggcacagctccccttcaccacaagaccgcgcctttccatgcgagtcacctggtgcgaaccgcgcgagcgatcccaattcaattgcgcgcataagtcccgcaagcgcatgcactggccctcagcctccgacagctggaccagcaccgcgtactcggccgaggtgagatcgaagtcggtgcgcagctcctcgtcgatttccctgctgactttcagggccgcctcgatgagtccacgccagaggcgttgttcctcctcactgagccattgtggttcgtttgccactgctcccctcctgtttatttctgccaagttactgccaattcattggaaagatcaattttcggtttgttgacgcgtccattatttactacagtcttacatcaatgcatccccctccaaggcattgcatgtacagagtttgagcccggcaccgccccctccagggtgccgggctcaaacgcttccttcgggttacgcgctcgcggtgggcgccttcagttccgctatggcatagcgccgcgccgcgttgacgcggtcgaacctgctggggaaacaggtcaacacgatcacctgggcgttttgcccaacttggtcgaagagcaggttcatgcggctcagccggtctgggtccgtggccccaagcgcgtcgtccaccacaaccggaaccggcgacgtcgaccccgtgcccgtgaccaggtcggcgatggcgaaacgggtcaggatcgccagctgctccttcgtgccgccggagagctccgacaatggcaccgtcgtgccgtcgaccgtgcgctcggtaatctccagcgaatcgccgaagttgaagtccacgctggagccgtagatgacgcgggcgtggttgcgcagggcctcgttgaacggcgcggtgtagcgggcgcgggcggcgtcgcggtgagccaccatcgtctcccggagaaggcgggcggcttcggcgcggcgggtggtgcgttggagatcggtttcggccttgtctagctccgcctcggcacggtctgccttttctgcggcgccagcggcgaggtcgatgcggccagcgagctcgcggatccggttctccgcgtcggacttgcgctgtttcaggttttcgacgcgggtagtggccccgttaagcaagcgctcggcgagctccgggtcggccgcagcggaacgcgctgcgaggtcgtcgtggaccttcttcgcctccaccatctcggcgcgcacggtctcgagcgccgccttcatcgcgtcgcgcgggtgcttctcctccgccgcgtcgagctccgcctgggccgcgtcgcgctccgcgtccttcgtctccgagcgggtctcaagcacagtgagctcgtttgcggccttgcggtcagcgtacggtttcaccgccgcgtcagcgttgtccacttcgcgctccgcatccgcgagggcggtttcagcttcgcgcagcgcttgctcggtgtcggctggggtcagttccgccaccgcgccatcgtcgagacccaactcttcggcgagctcggccaccgtcgactgcagagccgcgcgctcggcgcgaagggtttctaggtcgctgcccccgagcaggtccgcgcggcgctgcttcgcggccttgaacgcggtggcgtgctctttgtgctcgtcgcgggcggttcgggcggcggcgatggaggggtatccggtggcgtcgataagcgaatcgagcttttcctccgccttgcgcactgcctcgcgggggtcctcggacccctgcgccgcgcggtacaccactgtgtagtcccccagcaccacctcggtgccctcgaagaccccgatggataccgtcccgtcgacctcgcgctgcttaccgtcaaccttgatgctttggccggtggcgcagatgtccagcttcgcggctgcggcgtcgagcaatcgccgctggagcgcgacatcgctttcagcttcctcgagtgcccggatgtctttgtcggtgacctcccggcgcggggtcttctccagcaggtcggtgtaggtcttgtcggcctcctcgacgcgctcgatgagctcgtctttggcgcgcagatcgtgtgccgcgcgcgcgaggtcgcgccgtttgccggcggttctcgcggtactgcgcgcatctgccgcgccggctttcgcttcctcgcgcgcctgggtgagatttgttagcttctccgcctcctgctcagcggcctcgcgggcgggagcaagctttgcgcgaatgtcgcccgcttccttggtaagggtctgtacccgctgggtgagctgctcgcgcaatgcaaggtcttcctcagcgcgctcaagcgccgcggcagcgcgggtaaattcctcgcgcgatcgttgcgcctgctcaccgagttcgcgggcctgtacagcctcggcctcgcgcgcagccgcctcttcaagcgcctcgggcatctcggcatcggcgtttcggatctcctcctcgcggcgggcgacctcgtcgacataggtcgaaagctccgccacctcgcggcgagcgcggtcgtgcgcggccttcgcctcttcgaccgcagtgaacttggcggcgtaggacgccttctccttcgccttcgcacccgcggtgaagtacttggcgtactcctcctcgaccgcggccatcaggtcagtgtcctctacggcgaccgcctcgcccccggagcggtcctgcagcgcagcggcgatcgagggaatgccggcggcttgaatacccgggtcgagctggccctggcgaaggaacaggttctgggcgagctcgcggtccatgtgctcgctcaagatgcgctcaagctggtcgtcggcttccctgcccgtgtaagtcttgcgctgcggcgccgtgatctcgaggactgattcggggcttttcagccactgtttgcgaatggtgaaggaggtctcgcccaccgtcgcgctgagcgtgacagcgggagtgacgtcgcggccgaccggcgagacggctttgatctcctttttcttcgccgagctgcgctcgcgtaggacgaggtcgaccgcgtccaatatggtggacttgcctgcctcgttgtcgccgtggatgacaatgacgccggtgtctggcaagtcgcggagtacaaggtgttcgatgccgcggaagttttcgatttcgaggctgtgaatgcgcattcttacttctcctctttgctcacgcggaacaacaggttgacggcgtcgcgggcttggctgtcgttggcgccgccatctgcgcccgaggcaagtgaaaccagctcgcgcatcgcttctttggcgtagccggtcagcgggaggttctctagctcctcgtcgctgggttcgaggtgcagattcatcagccgctcgcgggggtacagggcggcgaagatcggctccaactcccccaggcgccgctcaagatctgcggtggcctcgagcccgagcgtcccggagagcgcgtacttgatcacggtgcgggatttgtcggggtaagcctccaaggtttcgataacgcggtcgacatcgccggcgtccgcaacgtcgaagtggagggcatcgaacgtccactggccggtggccaccggcttcacatcgacggtgctcgtcgtcccggttttgtccacgctgactacaagcacgttgccggaatctgtctcgccgccggccaccccgggggtgagatcgtggtagtcagtcgtctccggcgagcccgagaaccacacccggccgcttgctcccaactgctgcgttgagtgggtgtccccgagcgcgacgtaatcgatggtgccgtccgccagcttttcctctaaccccaggaggtcgatcagcgccgggttcgcgtccgccccgtagccctccacttggccgtggcccacaaggatgcggatgcgctcgctcggcgctagatcgcgcaccgacttggcgcacaggtcctcggaggcgtgcttggtcattagcggcgcgccgacgacatccactccgtccgcgacctcgaccgggccgcaggaatcgagcaccgcgaccccctcgatgccctcggtgctgcggaagatcgagtcggccaccagcgggtcgtggttgccgggcagcaggtagaccggcacgggaagtttgcgcagcgcctccagcgcgcggcccaaggtcgcgagctcgagcgcgttgtgctcgaacacgtcgcccgcaacgacaatgaactgcgcgccgtgctctgtagccacctcccccaagcgctctactgcgcgcagccgcgcatcgtcgaaacgggattgggcttcgggcggcaagaactttcttgtcatcccgatctgcaggtcggaggtgtggatgaaggtggtgtgcgtcatgccttaaccaataccaggccaccccaacacgcccgcgccctcgtcgaacacagaggctaaaggatggctcgcctgcggataacgatttgcgcgagttgaccgacccctgtagctcccacggatttgactagacaacatacctggggaaacgggcctgaaaagcgcccgtttttccttgggagctacaccccggtccggactgaaacgcgcactcgaccacgaacttgaaccggcccctgcagctcatccccaccccggctgccctgtagctcccaatgatttgactagacacctcacctggggaaacaggcctgaaaagcgcccgtttctccttgggagctacaccctgggccggactgaaacgcacactgaaaccgaccgctgtagcccattcgcaccccggcaaccctgtacgcgctagtcgtcttcttcgaccagcgtgtcgtacaggtcttcgatgtcggcgaccgcgttgagcaggtcgatgttggtaaacgacacgctttccaacgcgcggcgcagaaggtcggtgtcggaatcgtcgatcatgggggcgatcttggggttcggcaggtcgggcatgtcccggcccgaccagaagtattcggatccggcttcggcgttggctttggcgatggtgtacgccccgtcgcgaagcgatgcctccaccgcatccatcgccatgttgcggatggcgaacacggtggccggctgctggttgatgcgccgggccgccgcgacggcgacggcgacggcgtgcttgcacacatcagcagggtcggggcagtcgcagaagaaacggaactcctccggggcggccccgaggaagacgtccagcacctcgtcagggaactcgcccttctctgcccgctcaagcccgccaggcgttgccgccatcgcactcatcgcctgcttcagctcttcctgcgtgcgtaccggaaggatgaaaccggcgtagaacggttcgttctggctgcccgccacgcttgcgtccatggagttcggccgcacccgaagctcggtgacgtgacctttctcagcgtagtcgcggccccgcttcacgcgccccgcgtctgtgcggcgaagcgcggcattgagcaccaccatcgcggcgtgggagagctggtccgcaggctctgacaccgtgggtgaacccgtctcctccggggagctcacgcgccggcgcgcgccaaagttggcgtagatgacgttgtcttcgctcggcctattcacggtgccccctgaaactaatgagcttggccaggtcatcggcgtcgagctcggtgatccagccctcgccctccccgaccacggcgccggcgaggtgcatcttgccgtcaagcacttcctggatgcgctcctccatcgtgccgcgggtgatcatcttgtacaccgtgacatccttctgctggccgatgcggaaagcgcggtccgtcgcctggttctccaccgcagggttccaccagcggtccatgtgcaccacaatcgacgccgcggtgaggttcaaccccgtgccgccagctttcagcgacagcagcatcgcgggaggaccgtccggggattgaaagcgctccaccatcgcgtcgcgggcatttttgcccaccccgccgtgcaggaacgggatctgctcaccgagccgctcgctcaagtacggctggaggatgtcgccgaacgccttgtactgggtgaagatcagcacgcgctggccggtctccgcggcctggtcgaggatctcaaccagtttctccaccttgcccgagcggtggcgccccttgatggtgaccggggagccgtcgccgagaaagtgcgccgggtggttgcagatctgcttgatgcgggtgatcatcgacaaaacgagcccgcgccgcgccatgccctcgcggcgcgccagctcgcgccccatctcctcggtcagcgcggtgtagagcgcgccctgctccgccgtcatgtccaccccgatgacgtgctcggccttatccggcaggtcgtccacgatcgcctggtccgttttcaggcggcgcaagataaacggcgcggtgaggcgctgcagccgctgccccatttcctcgctcagcgcgtcgtcgccgcgctcgatgaccttggcaaagtggttgcggaaaaaggcttgcgagccgagcatgccagggttcacgaaatcgagcaggctgcgcagctccgccagcttgttttcgatcggggtgccggtgagcgcaatgcgctggcgcgccggcaggcgccgcacgcttttcgccgcctgcgtgccagcgtttttgatggcctgggcctcgtccaccaccacgtggtcccactggatcgccgagaggtcggcggagtccctgctcaccacgccgtaggaagtgatgaccaggtccgcctggctcgcggctgcgacgagttccgccccgcgcaggcgcccgttgccgtggtgcaccacaaccttcatgcttggcacgaacttctgcgcctcgcgggcccagttgcccaccaccgacgtcggcgcgatgacaatggacggccccgctttccgccccgcgtctgcctcgaccgcgaggagcgcgaggagttggagggttttgcctaaccccatatcgtcggcaagcactgcccccaagttgttcctggacatgaaatacagccagtccacccctcgccgctggtactcgcgcagcaccgcttgaacggtgggcgggatgtcaacgcgctcgggcgccgggcggtccgtgccgccgagcagggagttgtaccaggtcgcgccggtgatctcgaccggcggttccaagcccgcctccgccgaggactcgagcgcgagctggcgcagctcggacgcggacaccgtgccgccgagctcctctttctccgcctccttcatctcctcgcgcagcttggccgcgtgcgccgcgagttcctcagcgtcgccgctacccgctgccttcgccatcgcggcaagccgctcggccgcctccacgcgctgagtcagctcctcaagactcgatttgtgcagctcgcgcatgtagcgctcggtgcgggcgagcccggccttatccgccagcacccactcgccgcggagcttcactaggccggacttggagttgaccagctcccgcatctcctcgtcggtaagttccatgtcgccgacggagacgcgccagtcgtactgcatgagcgtgtcgaagcccaggtggcgcacagtggatgtgtcgtacgggttctgctcgcgggtgacgtgcagtttcgcgcgtgtctccgcagtggtccacgccttcggcagcatgacggcgaagcccacggcgcgcagcctggatgcgcccgcgcggacaaactccgcgatctcgtcggcggttaagtagatgtcccagtccccgtcgtcggggccgccctgcacccccagcgggtgcgggtggcgggctggatccaccaggtcggtcgcggcgaccgcgcgggcgagctcgctgcgcaggcgctgcgccgtctgcccgtcgtagtcgtgctggcgcaccgggcgcggcgcgtcggtgccggagcgcacctgcacgcgcaccggccacacgttggcgtttgcgctttccccgccaccgccctcgccgtcctccagcggcgcgtccgcgatgaacaccagctgcaggttgacagcggcgatcgagccgttccagtcccccatccgccgcgacagaagcgcgctgccgcggcgcagcggggcgccagtgagcagcgagttgatgaagtcgtgccggccgtacgggcgcgcatccagggcggtgccggcgtcgcgcagccgctcggtggcaatccagtggaccagcgtcttggccatgtcctcgctcaacgtggggttgttcgcaaccagcaccccgggcgcggccgcgaccatggacgcgagccaaccgcgctccgccacgccggtgccgagctgccactgtgcgtaccagagcgcgtccttcagcggcacctggatagtcacgcgcccggcgcgcacgaagcggtcgaggccgcggaacatctgcacgagccaacgcaggtccggcgcgagcgccccgctctcctccggcgccagcttggccaggccggataagagcagcaccgtgtcttcaggcgtcagcgccgccgtgggcgccaccagctccacggggcggcccttgggtgtttgcaaccggatctggttgcggtggcggaacttgttgccgtctatcagctcgtgcaccaccggcggaaacgtctctggcccaaccttgtccatggtgacaatgcggtggccttcgacctgctcaacccacatgttgaggccggactccggcaaccagagtccgtggagcaggaattgaggcatacccactgttataacaccctcctcaaacacggccgtgagcgttcatttaatgaagtacgatgtcatccacatcacacttttagtgagaaggaggaaacatgtcagacaatttttggctggtgctcgccatcgtcttgtacttcggcgcgatggttgccatcggcttctactcgtggatgaagacgagtaagtacgacgactacgtgctcgccgaccgcggcctaagcccgtttgtcgccgcgctgtccgctggcgcgtcggacatgtcggggtggctgctcatgggtctgcccggcgccctgtacgtctcgggcatgagcgagctgtggatcgtcatcggcctgttcatcggcacctgggcaaactggaagtgggttgcgccgcgtctgcgcgcgtacaccgaggtctccaacaactcgatcacgctgcccagcttctttgaaaaccgcacccgcgattcttcgcgtgtcctgcgcgttacggctgcgctgatcatcatcttcttcttcacgttctacgtttcctccggcatggtctccggcggccgctactacgagtccaccttcggcggggattacgtcaccggcatgctcattgtcggctcgattacagtgctttacaccttcttcggcggcttcctcgccgtgagctacaccgacgtggtgcagggcatcttgatgttcgcggctcttatgatcgttccgatcatggcgctgatcgccgtggataacccgggcgacatcttctcctacgccacctccaacccgtacggcccgtggccggagggtaacccggactacttcaacgtggtcgccggcgtctcggtagcaaccatcatcggtaacttggcgtggggcctgggctacttcggccagccgcacattgtcacccgcttcatggcgctgcgctcccccgctgaggcgcgggcaggccgtcgcaccggcatgatctgggtcgctttttgctacgttggcgcgatcttcaccgcgctagcagccaccatctacttcggcaccaccaccgacttcgtcacggaccgcgaaggattcgagaccgtgttcctggatctcgcgcgcctgatgttccacccgctgattgccggcatcattctcacagccgtcctgggcgcgatcatgtccacgatgtcctcgcagctgttgatcacgtcctcggccctgatcgaggacctctaccgcatcttcaagaaggagccgagccagggcgctctactcttcttgtcgcgcaccatggtcgttgccatcgctgtcatcgcaatgttgatggcgtttaacccgtccgacaccatcctcggcctcgtcggcttcgcgtgggcgggcttcggcgccgcattcggcccggtggtactcgcctcgctgtactggcgccgcctgaccgcccctggcgcgatcgcaggcatgatcgtcggcgccgtgaccgtcttcgtctggggcacgttctacggcgacatcatctacgagatcgtcccgggcgtcattctggccaccctcgcgatggtcgtcgtctcgctgatgacccagccgaagccgggtgttgaagcggagttcgatcgcgcggttgccgtcaccgattacgcccttgcccaccccgaggtcagcttcgccgacgcgctgcggaaccaggagggcgcaaagggcgtctaagaagggtgtgcgacgctaccttctcatcctgaccgctctcacagcactcaccgtgccgttccccacggggcagctgcttgtcgacgcccccttacaaccccgcttcaccaccaccggataccagcgccaacaggcgttcggaccggggtgggcagtgggccccaacggttgcgacagccgccaaaccgccatggccgccgcgtggtccacgccgtgcaccgtcgcctaccgcgactgggacgtcggccccatccgcgacccctacaccggcgacaatctcctcccgatagacgtggagatcgaccacatctacccgctctccgcggcctgggacatgggcgcccacgcctggccgcaagagatgcgcctcgccttcgccaacgacccgctgaacctcaccgtcacgtcgtcgcgggccaaccagtccaagtccgacgcgctgcccggcgagtggatgccgccggaccgcttagcccgctgcgcctactcccggcgtatttcggcggtggcatcgaagtacaacctgccgttcacacgggaagatcagcgcgctatgcggcgctcgtgcggagggtttcagggtctcatttcccgcagatccctgtagtgttgggcgtcatgaacacatttttcgtcttcctgcacgtcgctgcagcgatcgttctgctcggtcccgtggtggtttcctcttcaatgttcccggcagaagcctccaaggcgcgcgccggcggcgaagagtccaccggtcacgcatcggtgctgcacaagatcacccgcaactatggcctcctctccctgctcgccccgctgctcggcggcgtggtcatggccatggactgggaggtgcacaagtccaactacctgctgcacaccgccatcgtgctttccgtcatcgcgtgggcgatcctgctcggcatggtgatcccgcaacagcgcaagattatgggctccctcggcgcgcttgagccggccgacgcagctcctggcgacgtcaccgagaacttcgagaaggccaaggctaaggcagcagccggcgccggcatcttcaacctgctctggttcctcaccctgatcctgatgttcgtccctgccccggacacctggtaaaccgcctgcgcgaagaccaagaaagtgcccgccctcgttcattgagggtgggcacttcccgtttgggcagttgctgatagcgggtaactccgcaaggccgtcacgacgacctgcggaaacgcgaaccaggccgcgagttatccgctatcaccgtccggcgcggcgctagtcgcggtcccggttccggaacccaccgccgcggccaccgcggtcgcggtcccggcccccgcggtacccgccgcggtcgcggtcgccccggtagccgccgcggccgccccggtcgcgcggcggcgcaccgtggtcgcgctggatgttgatcagctgaccggagatgcgggtgtcgctcaggcggtcgagcacggactggtcgaggttcttcggcagctcaaccagagtgaagtcgccaccgatggtgatgcggccgaagtccttggagctcagcccgccctcgttagccagggcgccgacgatggcacccgggcggacgtgctggcgcttgcccacatccaggcggtaggtgtcgaagctgccgcggtcaccgcgatcgaagcggtcgtcccggtcgcgaccgcggcggtcgtcgcggtcgaaacggtcgcggccccggcggtcctcgcggtcgaaacgatcgcggtcgcggcggtcgcgcttgtccttcggcggctccttcatcaggaactcgtcgccggcctgggcctgggtggccagtgctgcggcgacatcgtccatcgggacgttgttggccgcggagtactcgcgcaccatcgacttgaacacgtccaagtcggaggcctccaaggacgcggtgatggaatccatgaacttcgccttgcggctttcgttgacctcgtcgaccgtcggcaggtccatttcctcgatcgtcgcgttggtcacgcgctcgatggagcgcagcatccggcgctcgcgcggggtgacgaagaggatggcctcgccgctgcgcccagcgcggccggtgcggccgatgcggtggacgtaagactccgtgtcgttcgggatgtcgtagttcaaaacgtggctgatgcgctccacatcgaggccgcgggcggcgacgtcggtggcgaccaggatgtcgaggcggccgtcgcggagctgatccaccgtgcgctcgcgctggttctgagcgatgtcgccgttgatagcggcggcggagaaaccgcgggcgcgcagcttctcggcgatctcctcggtctcgttcttcgtgcgcacgaacacgatcatggcctcgaactcggtaacctcgaggatgcgcgtcatcgcgtcgagcttgttgcggtgcgcggtgaacaggtagcgctgggtgatgttggtgttggtgcgggtctcgctcttgaccgtcacctcgaccgggtcgttgaggtactgcttggaaatgcggcggatcgcacccggcatcgtcgccgagaaaagagcaacctgcttgtcctccggggtgtcctcgaggatgcgctcgacatcttcctggaagcccatgttcagcatctcgtcggcctcatcaagcaccaagaagcgcaggttggagatgtccagcgagcccttctccaggtggtcgatcactcggcccggggtgccgacgatcacctgcgcgccgcggcgcaggccagaaagctggatgccgtaggcctggccgccgtaaatcggcagaatgtggatgccgcccaggtgatcggcgaacgactggaaagagtccgacacctgcagcgcgagctcgcgcgtcggcgcaagcaccagcgcctgcgggtagcgctccttcgggtcgatctgtgacagcaccggcagcgcgaacgccgcggtcttgcccgtaccggtctgcgcgaggccgacaacgtcgcggccctgcatcagcagcgggatggtctgcgcctggatcggcgacggctgctcgaaaccgacgcgcttgacggcgtcgacgaccgtgcccggcaagccgaggccgtcgaagccgttgtcttcggccggctcctcggcaggctccccagccccagccggctcttctgtctcgattacctcttcgagggtgacaatgccctcggcgttggctgcgtcgtccgcagcgccggtctcctcagaaacccccgcatccctggtgtcgttttctgcggctgcgtcagcagtggccgcgacatcctgcgggttatcctgattttccgacaagttcatgtccggcttattctcgccgccggtggcgttttcggaaatgctcattgttcgcccaccttacgccgttgacccgttaatctgctatttgtgatttttctgcgctcctcgaaactcctcgccacgctcgcctgctccgcgctgctcgcgagctgcggtgtgccgctgttcggccaggctggttctggggtggacaagggtgcgtcggcaagcagtgcccccgacttactcgacacggccgaaaccgacgaaccgtacgtcgacgtcgacccgaatctgtttatcgagggctcgggcgccaccgtcgcgggcacaccggaatccggtgtttccgggtgctacctgatcgacaagactcccgaggacccgcggctgagcgcgctcgttgtgtgccaggcacgctttcgctatcccaccccggatatcgagttcgacggaggctggcccaacccgccgttcgccaacgtcgtctccttcgatttcgacgcggagaaattcgaaacggggatgtcgccgggttcgcaagggttcatgtccccgccgcgcgcgctcgagccgggtgagcgcgtcaccatttacggcacgacgatctaccacttgcgcgacggcgggttccgcgccgagcgcgccggcgaaggctacgaggtgcacagcggggtgatccagcacgactgggattcgaccgaccgcgtcgcgcagtccaaggagccggtggacaagggcaccgtctgcggccgcgtctactcgctggataacaaggaccggcttgtcgtcgccgccgaggacggcaccatctgccccgccgccatggacgcgatggacggctacatcacggcgctgcgggagggagatagcagcatccagggcaacgccgcgctgtgggagtcgccggagaactggggctgctccggccgctacttcttcgacggcgaggagtacgtcggcgccaacggcaagctcagctgcagcgcgggcgggttgaacggcagcgcggcgggtgacggcagcggttccgtcgtcgcggttgaaccggacgatttgccccgcctgtagcccttggctcacgtaatctcgtgggcatgtcgtttcttccccggcccgcggtaatcgccgccgcttcgtgcgccgtgctgcttggcgccaccgcctgcgcaggtggccaggacgcggtcccggaaccgacgatcgacgccgcacctgcagcgacccgctccgcagagacgtcagcgaccaccgcgacgtcagcgaccaccgagaccaccgcggacgccccgaagatgctcgagcgcagcgccaacgagttcgaggtcccaggcgcctaccacgagatgtacgccgtcgcgctcaaggaggacgacgcgacctgcgtgtacaaacccggcaactatttcggctgcgaggtgaatttccagggcgtgctcccgcccgacgagcagccgtacgagttcaccagcggccccgtcgattacgtgggctttttagacgacaagttctacacctccgtcctcgtcggcggcggcgacggcccgggggtgtaccacccgctgaaccccggcgagttcgtcgagatcggtaacgtgacgtttacccgcaaccacgacgcctcggtgcgggtgacgacgggtagccactggttcgagatcgacgcggacggccagtacagctccgacagcttcgacccggccgcgggcggcgcatcgacgcaggaggtcgccgcaggcccggccacgtgcgagacgttcgactactccgggcgtttgttcgttgtcgaagcaactgatgcgagtctatgcgccgctggctcccaggccgcgcagggcatgacgcgcgagccaagctccctgccgcgcgagtacgagattgacggcatctcgttcacgtgcgaggacaagggcggcgagcggtcggtctgcaccgcgtccaccggcggccgcgtcgaggcccaaccggcctaaacctgcgccgtaggattgccccatggccatcctccgcacccgcccgctgctcctcgccgccctcgcatgcgccgcactcaccgcctgcggcacggacgcgcaggagcaggcgcttgacgacgcccccaccacctcctcccaaaccccctcccctgcaaacacgcacacctcggaagccccaacccccaccgagaccacgggcaccagcgaggccacggaaaccaccgagcccaccgaggccaccgccgcgccaactaccgcgtccttcgacgccgcccccgcgcccgcagtggagcgcgaccccgccgacttcaccgaggcggagccaaccgacccgttcgccgcgtacgcgatcacgctctcccccggcaacacgtgcgtctactacgcaggtggcggctacttctcctgcgacctcgcgctggcaggtgccctgccgcctctggacccggactacggagcacccgccggccagcacccggacgtcatcatgtggggcgacgaccgcggtttcgccgtcacccactccaccggcggcggcgagggcgcgccggaagctgcccagctcttccccggccagaaagtcaccgccggggattacaccttccagcatttccaagacggcaccatgcgcgttgagcgggccgggcactggttcgaggtctcaccccaaggtcagtactcctcggatcgcttcaccccttaagctcatcgtatgaattccgccccttcggcgcccgcacgaggcctgacacaccgtcacatccacttcatcgcactcggctccgccatcggcacgggcttgttctacggctctgccggcgcgatccaggcggcgggtccctcggtgctgctggtctacctgctcggcggggcggtcgtgtacttcatgcttcgcgcgctcggcgagatgagcgtgcgccacccggtgcgcggctcgttcgccgtgtactgccgcgagcacctgggcggcttgggcggctacatcaccggctggatgttcgccttcgagatgatgatcgtgtgtttggctgacctcactgcgatcggcatctacatgaagttctggttccccgacaccgcgtcgtgggtgtggatcgcggtgacactgctcgtcatcggcgcggcgaacctggccagtgtgcgctggttcggagaactcgagttcgcgttcacgctgatcaaggtcgccgcggtggtggcgatgatcgtcggcggcgcggcgattctcaccttcggactcggtgagaaccccgcgatgaccggcatcgacaacctgtggaacgacggcggcttcttccccaacggcggccaaggcatgatcgccgcgttcatcctcgtgctcttcgccttcggcggcaccgagatcattggtgtcgccggcaccgaggcagacgacccggaccaggcgatcccgaaagccgtcaacaccgtgccgctgcgtatcctgcttttctacgtgctcgccatcctggtgattttgatgctgaacccgtggcgcaccatcaccggcgacgagtcgccgttcgtgcagatcttctccacgctcggcgtctcctgggcagcggggctactcaacctcgtcgtgatcaccgcggcgctctccgcgatcaacgcagacctcttcggtaccgggcgcgtgctcaccggcttggccaaggagggtctcgcgccgcgcgccatggcgaagacagtgcgcgacatccccgtcatgaccacagtctcgctactcatcgtgctggttgtgggagtggcgctcaacgcggcgttccccaacgtctttgaaaccatcgcggcactggccaccttcgccaccgtgtttgtatggttgatgattctgctcgcccacatcgcgtctaggcgccgcatgacgcccacgcaagttcaggcgctgcgcttcccggtgccgttttggccctacgggcagtggttctcggtggcgtttatcctcttcactttcggcatcatggcgtggctgccgcagtaccacttggcgctcgcggtcggcatcgggttcctgctggtcatgacggttttgtactttgtaacggggcgtccgcaagcaactgcccaagcgcacaccgcctacgaccgcaagtagccgcgctcagataccaccattgtggaacaatgggcggtgtcaacagcagcagatgctaaaaggagcgcttgacaatgaccgccgcacaaaaccagtcccaggtcacccccggcacgaaggtcgtcctcatcggcgcgggcgccgtgggtatcgcctacgcctacgcgattttgaaccagggtctcaccgaccacctggcgattatcgacctcaacgaggaactcacctggggccaggtcgaagacctctcccactccgtgccgtttagcggcaacaacatcaaggtttccgtcggcacctacgccgactgcaaggacgcagccctcatcgtcaactgcgccggcgtcgcgcagcgcgagggcgagacccgcctcgacctggtcgcccgcaacgtcaagatcttcgactccatcaactccgaggtcatggccaacggcttcaacggcatctacgtcgtggccaccaacccagtcgacgtgctcacctacgttacctacaagcagaccggcctgccgtccaaccaggtcatcggctccggcaccgtgctggacaccgcccgctggcgccacaacctgggcaagcacttcaacatcgccccgtcggcggttcacagctacatcatcggcgagcacggcgactccgagctcgcggtgtactcctctagccacatcgccggtgtaccgatgaccagccttttggacaaggaagcggagcaggacccggagatccacgccaagatcgaggacatgttcgtgcgaacccgcgacgccgcgtacgacatcatcaaggccaagggcaacacctccttcggcatcggctccgcgctggctcgcatcaccaaggcgatcctgcgcaacgaggacgtggccctgccggtctccgcgtatcttcaaggcgagtacgcgctcgacgacatctacatcggcaccccgaccgtgctcaaccgcaacggcgtgcgcaacgtggttgagctgcgccttgccgaggacgagtacgagcagttcgcttcctccgccaagacgcttcgcgaggtcaacgagtccaccgggctgaccaactaaggggcatttgcttaacgacgcagcgggggttgcgtcgctaaactgtcgctcatgccgaaagtaatcgacgtcgtagctgccgcaattgtgcgggatggacgcgtccttgccgcccagcggggaccgggcatgaccatggcggggttatgggagttccccggcggcaagattgagccgggtgaaacccctgaggaatcgctcgctcgtgaaatcgctgaggaacttggcgccgacatcactgttcggaatcacatcgtcaccactgatcacccgtacgatttcgcgacggtccgtttggcaacgtactactgcaacctgctcgccggcacaccggtggcttcagagcacgccgagctgcgctggctcaccgctacggagatgcacgaattagactgggcaccggctgacattgaagcggtgcacctcatcgcccgggacctcgccgcgtgaacagatcactcgagggattaagacgtgatctcgagttcggtttcatcgatcgcacagtagctgccgaacgtatagaaaatccgtctctgatcgctaatgatcgggcgaacagcatgttcggcatgcttcggtccgaactctccagtgcggacagcttcatattttccgttgcgttcatttcgactggaggcattggcacgatcctggaagaactggccaaattcaaaggccagggcactatcatcacgagtactctgaacgacttcaacgagcctgcagcgtttcgtgagcttctgaagttcgaccacatcgattcgtacgtcatcgagggcccacaccacgcaaaggggtacatcttcgaccacgatgaccatgtcaccgcgattgtcggcagctcgaacctcacgcgaagcgcgttgctgtccaaccaggaatggaacctccacttctccacccatcaagacggtgatattgctgttcagttgaagcaggcggtgcacaatcacctcgcccgcgcggtgccgcttaccgaggattggattgaacggtacgagcaggcccgctcaactcgcgccttcgtcgtccgcgataaccaaccaatcttggtctcaccgggtggcgagcgcatcgaaccgaacaagatgcaacacgaagctcttgggagtttgcgcgaagttgttgactctggcgccaaacgagcgctcataatctctgccacgggaacaggtaaaacaatcttggcggccctcgccgcaagagagatgaaccctggccgaattctcttcctagttcaccgagaacagatcctgcgcaaagccgctgacgcattcgcgcgagtgctggaaattgacccctcggatattggcttcttcgtgggcacgcagcgcgatatcgacgcgcgggtggtgttctctacagttcagaccctctcgcggccggagaatttgtttaacatttcccccacccacttcgacatggtcattgtggacgaggtacaccgctcgggtggcgagacgtaccagcgaattctcaaccatttcgatccgggattcaccctcgggctcactgcaacgccagaacgatccgacaggttcaacgttttcgagctcttcgattacaacgtcccttatgaaatccgtcttgagggcgcgctcgaaaaccacatgttggtccccttcgattactacggtgtcacagactatgaatcagccaggggttcaatcggcgactcggctggcatcgatctactgacctcgcccgagcgtgtggactacatcgcccagactctcgagacgtactcctttgcccagggcacgaagggcctgatcttctgcagccgcatcgaggaagccgataggctatcccagctgctgaatcagaaggccgttcacggaaaactactgcgaaccgtcgcattgaagggcgagcactcgacggcggaaagagaagccgcaattcgtcgactggaagacggcgagctggattacatcctgtctgtcgatattttcaacgaaggcgtcgatgtgccggcggtcaacgtcgtcgttttgctccgaagcaccgagtcatcgatcatatttacccagcagctgggccgtggcctacgcaaagcggacggcaagaagtcgctccgcgtgatcgacttcatcggtaattacgccaacaactacctcatccctatcgcactcaccggcggcaacccgggcgataaagatcgcctccgcgacaacatgcgtcgaaagagacgcgagccgattgctggttcctcgacagtgagtttcgacgaggtcgccacccagcgagtcctggagtctttacagaaagcgcgcatctccgataggcgtgtaaagcgcggcgagatcgaacggctccggagccgtttaaatgtcattccacgattggctgacttcctaacgtttgaaacgctcgacccgtttgtgctcgctgcaaccgacaaacaagcccgcaactactgggcgctactcaaggcgtttaatttcgtcgaatcgggcccgagccaagcggaagatggcttcctctctatgctcagcgtggaattgctcaacggcaagcgcccacaagaactgctactgctccgcgaacttcttcgccgcggtccgaacgcccagctatccacgagcgaattcgctgaggtctgtcacgagtggtcaccattgatccaaaccggcgaacccacattgacctcggtcgaacgagttctcaatcttaagtggagtatcgacgccgcagcagcacgctatggtggtcaacctcttgttctgcgcgctgacgacagcttcaagctgggttcggcgttcgcggcgctgtactacgcctaccaacccgatcatcctgatcgcgctgaaagctttcgtttccacgtcgacgacgtgatcgaaaccggcctccgtacgaatgcactgcgatacggccggagtgacaccttcgtgccgcaacaaacctactcacgaaaagacgcttcccgactgctcaactggagcaataaccgggagtccaccatctacgggtacagcattgacgcagcgactaagacatgccccatctttgtcacgtaccacaaggacgctgatgtcgcggcgaacatccgatatgaagacgagctcatcgacccatcgacgatgcgctggttctcccggcacggcaagacgctaaagagccgcgaactccaggcaatgttcagcggcgaagtggacctctaccttttcgtaaaacgcgaggatgctgatggctctgacttctactacctgggcagggtggacgcggaggacccccagcaaaccaccatgcgcggcgataaggggaaagacctcgacgtcgtgaccaccatgctcaagatccgggtgccgatcgaccaatccatgttcaacgtgctcaccgcgagcaaactcgcgccgcgcggttaatcagcgaagcagccacgacgcgtcaacacgggcgaaggcccccacctccccggcgaacgaggcgtcgtgacacgtcattacgacagctttacctgttgaaagcccatcggcgatgagggcacgagccacccctctgcccgaagagtccaagccgacgtccggttcgtcgagaagcacgagctgcctcccctgcgagaacacctgtgcgagctgcgccaaacgcaggtgcgccgcagggagatcgagcgggtgctcatccggatccagtttcacccccagctcggttaatcgcttaagcgcagcttcgtcccccacgaaccctgcggtggttacctccgagacctgatctgcagcgcgctgtagcgcgagggaaacactcactccatgggtgtcctccaacccagggttgccgtccaaaccagcgagtgcgcgcaacaacgtagtcttcccggcgccgttgtctcctcgcagccatagaacctcgcctggcttaagcgcgagatggatcggccctgcggtgaagatcggctcggtgctcttgcggggctgccaccacttccgcttctgctctccgcgggttgcaaccacctcgccgaggtcgatcatcggcatttcggatggcgcaacaggtggtgggaggcggactggttcagcggcaactggaggtcccaactctccgcggacaagtgaaaaatgcccctctcccttggtggaaaggacaactgtgcgagacggcagtgcgtcgaggagcttctggatgcgagcggcggactcggggtcgaggccggcgaacgggtcgtcaagcacgagggtctcgggttcaaggactgcgacgcatgcgatcgcgagacggcgggtctgcccgcctgaaagggtggtgggatcgtgctctgcgaggtcggtaagaccagccgcatcgaggattgcgtcgacgcggcgttgcatctctaagcgaggtacgccgcgctgctcgaggccaatggccgcttcctcaaccaccgtggtgcgcaagtacgtgacgtgcgcgatcgggtcttggcccaccacagcggcgttcggccacgtgtcgtggatctggttggcaagcgtgctcaagcccgagccggaagcgccggtgacggtgacttgtttgtgcgattgaagcgcctcttcgagcggactcagatccacacgaccaccaccaagcaggccaagggcacgaggatccggatcgcgcgctggaacgcggaatcatggaccgggcgcagcaccgttcgcggtccgtcaatgccgtagcctgcggtttcaagcgcccttccccggttcgcggcgagcgtgagcagctctgccagcaccggcatgatgacgtgaggtacgacagttttgatagtcaccgggcgcgctttgagacggttcgcgtcgcggaccacccgcacccgcgcagctgcctgcgggaacagttgcagggtggcaccggtgatgtaggacaaacggttgccgtagcggcgtacctgcagcgtcttcgccaagtccgggactcggacaaacaccccggctgcgaggatgcacgccatgagcgcggtgaaacggagtgctagctcgccggctacagcgaggccgtcagcggtaatgagtggcgcgaagcgctcctcgccgtatggagcgtggataagcaccattgacagggctacggggaacgccaaggcggtgaccgctgcgatgagtgccaagtttcgtgtcttcgccgtgccggccatcagcgcgatgacaagcaccgccgccgacactgcggggcggttagcccccatgaccacgatccagccggagacgcccacggcgagcgcggtcaaggggttgagcatcggttagacctgttgcgtaccctgctgcgcacccggcgcgaacgcgctgacggtacgcttcggcagcgccttgaccgtgaagaacgcgatcaacatgacgatgaccttgtccaccgggtcggagatgaacgcctgcgtggtcaccgacgcgatcaaggacgcgcccatttcgcggaacaggctgacgagtgcgccggtgcccacgcccgcggtgccgccgtagacgaacgccgcaaccggtgcggccaccatgccgccgattacgccaaggagcaggccgtagagcaccacggtgccgacgtttttgaacgcgttgagcttgtgaatgaacacgccggagaggtagccgatcagtgccgcgccggccgcgaacggcagcgcggccgggttgaggaggccccacaccaggttgttcagcgcgccggtggtcatgccggcgatcgggcccgccagcgccgcgaccagcacggtaccgatggagtcgaggtagagcggcaaaccgatggagccgacgatctcgcccaccacggagttgatgatcatggcaatcgggatcaaaccgagggtgcgcgccggcaggaccgggacggtagcgatgagcaggaggatcgtgccgaggccatagccaacgagagtgatcacgccctgggtcgagccagtgacggtgtcccagtcggttggtcggacaaggacgaggtagagccaggtcgctgcgatgatggcggcgccggcaatgacgagtccgcggcgcgcaggcgtccagacggctggttgtgacatgggtgtgccttccgaagaggatgagggtacgagcggatgccgccgccgcacctatgtcacctcggtgcgggagcaatcgccggggagtttagcagctcttagccgcaattaatcgtcagcctcgctgtggtagccggccgcgagagcggcgtcgcccgcagcgaactgcgcgtgcaccttgcacgcgcgctcgaattccgcccacgctttctccacgtcgcagccggtcagcacgttcgcgttcggcgcgttgtcccagatccccttcacatccgcggacacggcgccgcgcatcagctcggagtctgcttccacctggaggtatgcagggcaagttgtcgaagggatccgttcgagagcaatcagcaccgtcagcaggtcgtggatttgggcgccgtatccctcccccacgtcttcgtggaattcgaagtagaagcgggtgatgtcgcgcagaggctcagcgatcgcctgagagcccaacaacgcgacgatgcggtcgaggcgctccggggccagccacatctgctccgtgacattcaagggacacagcgtaattgttgtcccggcttcggcagcggctgcgaagatgtcgttggccgcgtgcgggtccacccagaagttccactccgcgttcggcgtcgtgttgcccgggtagtgcaccgcgccgcccatcaccgtgatatggcgcagctcggcgaaatgccgcgggtgcatctgcgcgaacgcggcgaggttggttgcaggcccggtgacaatcaggtggaggtcttcggtgccgcgctcgatggcgtcgatccacagcgcgtcgaagtcgcgctcaacgtggcgctcgggcgcggtgacgtaacccaggcccgtttcgccgtgtgtctccggggtggtggtcagcggcaacgccagcggtgcgtcgcagcccgcggcgagcgggatcgtgcgcaagccgcactgggacagcaaatacgcggcgttgcgggcgcactgctcggcgccgacattgccggcggaggtggtcacgcactcaatctgcacctcacgggcgtggttcaacgcggcgaggtaaatcagcgcgaacgtatcgtcgatgcccgggtcgcagtccaaaatgacacgtttcaccgcatcgtctccttacctatcgtgatccagatcgccagcgagatcgccgcaatcgccgagcacaacccgaacgccacgctgaagccggcggcttgggcgataaagccgagcacgatcggggcaagaatctggccgaagtcctgcgtcatttggtacgtggacagcaccttgccgccggagcggtcgttgccgatgatgtctgcaagcgacgcctgaactgccgggctcatcagcccgccacccatgcccgcgagcgccgagaagatcaccagcggccagaacgacgtggcgagccccagaacgccggtgaaaatgccggtgacggtgagtccggtgatgatgagcggacggcgcccgtgggcgtcggcaagcctgcccgaaaactgcagtgcgatggccatacctgcggcgaacgctgtcagcgcaaggccggatgctgccgcaccgtgctcgaacaccgccgcggcgaacagcggcaggatggcaacgcgcgcacccatgttgacgaagccgttggaaaacgccgcgctgagcagcgccttgtacgaggggtgctgccaggcggtctgcagtcgcatcggcgccttggccggcggcagcggctgcgcgtgcttcgggtcgtgcgtgagcacccacaccagaaacgccgcgcaaccgaccacaatgccgtagatggcaaacggcgcacggtggccgaggaaggacagtgccgcgccgacaatcgggccgacaatgttgcccaggagaaacgcggtggcgtacagtgcgttcgcccgcccacggatgctcggatgcgtcacccgcacaatcagcgcttgcgcggacagggtgaacatagtggagccgaatccggccagaaaacgcagggcgagaatgtgccagtaggcctgcgcgaacgcgacaaagaaggtggccgcggcgacgatagacagtcccgtcaggtagacgggacgggagccaagcttgtcgacgagcacgccagcccccggagcgcccaaaagccgcgccagcgcaaacaccgaaatcaccgcaccagcggcggccatggagacgttgaagcttgccgcgaactgcggcagcacaggcgcgatgaagccgtagccaagcgcgatgagaaacgccgcgctcaccagcacccaaatggtgcgcgggatagtgggctgattcgtttgaatagaggggttcgacatatcgctgtttagcgtagcctggctggcaaatcgccaccgatttcgaacttgtgttctacttttcgaacggctgtgtcgcacctgcgttctaaagttcgggccatgttcaacaccaacgtcaccccagtcactaccgtcagcacccccgtcgccctcgcggacgagatcacccagcgcttccccacccacctcgacgcgctcaccgcgatcatgcaccacccgcgctcgctctcgcgtccgaccgcgtcctggcgcccgccgctgaagacgctgccccgcttcgccggcggaggcgaactcaacgccgcggtaacgcgcaggcgcgtcggcccaaaggcgaaggcccgcatactcggctacggagaaacgcaggtgcccgcctacctcattgagctgcggctgagcgacccgtcggggctgcccgccgaccgccgcctcaccgaggcgtgggtccgcgcgctcgtcccagaagatgccatcggcgcggtccatgagctgccgtctgcccgagccgccacatacgtgtggcttgtggacggccacttcaaccccatcgcctccccgtcctccatgttcgaggggctgacggcggcgtaaacgcgggatgcggcgctagatctcgtcctcggtgtcgaccgcctggtccgggtcaatcccggtcgcctcatcgtcgtcggcgaagctgtcgtcgtcctcgtcatcgtcgtcgtcctcgtcgtcggcgccgaagatgtcgtagacgtccggctcgtcgaagtcgtcctcgacgggcaaaagctgcgcctcccactcctcggcttggtcggcggcgagggagaggacgtcgaaaagccgatcgaagtccgtgaacgacccgaggtcgagcacctccgcctcgccgatggcctcgtcgtggatagcctcgaagaggcgcaggcggtcttcctcggtgagctcggcgtcgccgtcggactcccacagctcgccgatcgcgtcgtcgaccacgtcgtcgatgttgtccgggtacaccacgaacttcacctcggccttcggcgtgccgccaacgacctggagagtgacctgcagctccgcgttctcccccacctcggcgcgcaccagatccgggttcaccgtgtcgtgcaggaactcgagatcgccgatgcgctcatcggtgccgtcgagcaggtcgcccaacaccgtgaccatctggtccgtcgccatgtggtcggccaccgcgcgcaccgcgtcctcgaccgagaacaccaccgcgaccaggatggactcgaactcgtcgtcgtcctcgtccacgtcggccgccgcaatatagacgttggccgcgggaaggtgcgggtcaatctcgacgaactggatctccacgtccgccgtgatcgggacaaacatggtctcatcgtgcacgcgtgactcaatgccgtcgcggtccagcgcgccggcgatgtcctcgaaaaagctcataggggaacatgcctttcctacaaggtgtatccacgttcgggattcgggcctgccccagcctagccgtcaatgccgcgcagcgtgcgcaaacgcgcgtgcgcagcgggcgcgcgctactggtcgtcgtccaccacggagtccggcgtatccgggtccggtgagtgcctgccccactcgcgcatatcgaagctctcccacgcgcggcgtttctcagccttcgggtccagctccacggaaaactccctgtcgatcaccgcggtcgcccgccccggctcgtcctcgttgcggaagccgtactgcggccagtcgtcccccgggaaaccgttgtggaaaaacgatccccagtggtactgcatgatgctgctgacttggtcgaacgcttccttcgacccgaagcggtcgattttcgacgcccgcgtggtgttcggatccccaaacaccgcaaccaagtccgatgtgtgcacggcgccgagacctaaacgccgcattgtctccgaggcgtagtcgaagcggtacatccacgtcggcgccacgcgtcgatgcgcggtggcgagcatcaccgacggcgcccagaaaatggcatccgcgatgagctcagcgaagtccgcgcgcccgccaacgtcgcggtacgcatgaatcacgccgcgggcgttatcggggtcgtagacgttgagcgcgcggcgcgcggcgcgctggcgctgcttcaccgtctggtacatcgtcttggcaaagctcgcctcgtcagcgttcgtgccgatcaaaagcggcaccggcgcctgctcgccggcttcgaacacgtcgatcgggtgctctggaagcgtcaccccgtcgacggtgggcatgaaagccgtgttgaactgcaccagctctttgccgttcatcagcatctgctgccccgtgcgcacgaggtcctcggcactggctgcgcgcaggtcgtcgatggtggagagttgggacatgcccatgccgtcgataagcctgtgcacccacatcgccgactgcacgcttgagtgcacactggcgctcggcggactttgcgccacggcccggtggaacagcccccgcgcccccggcgcgcacatcaggtggatcaccgcggcgccgccagcagattcacccatgatggtcaccctgcccgggtcgccgccgaaggccgcgatgttgtcctggatccatttcagcgagaggatctgatcgtggatcgccgggttggacacgcagtcagacccgagcgtgtgcagatcgaggtaccccagcacgcccaggcggaagttcaccgagacgtagacaacgtcggtcacctcggcaagcacgtggccgcgcagcaccttctcgttgctcgcgccggtgacgaaggtgccgccgtggtagtagaccaccaccggcagctcctcgtcggtgttcgggcgcacgatgtcgagggtgaggcagtcctcggtgccaaccaccgagtcgttccacccgaagttgccctgcagcgcgggcggggcgaagcgcgagccgtcgcgcacgccgctccacggctgcgccggcgacggcgcgcggaacctgttcggccccgacaccccactaccgtagggaacgccgcgccacgtgcgcacaccggtcctgttgtggacgatgccgcgcacagtgccaccggtggttgacacatcgagcgagaaatcgtctgacatggctcctaggttagcccctcgaatggcccgcggatcggcccttcgatcggccctgaatctgtcgggcctgctcgcgcgcggggcagctaaactgtccagcatgttcggacgcagcaagaaggccacaaaggccgattcggagccgaagcgggatctgcgcccccgcgatggccgtgacaacagcgacaacagcgacaccgcctctcctgaagacatcatcgcgtcgctgaagacggcggacgcgcgccgccttgaagaagacgcgggcccgctgggcaaggcgttcatcagcgccgtcgacgccgcggtgcacctgcagtccggcaccattcgcgcgtacgtgaactggctgcgccgccagaacccagaggcctcgccgcaggagctgcaggagatcatggcagcgcacttccggaagacggctgccaccaccggcgcgggcgcaggtgcggcggctgcgatcccgggcgttggcctgatcaccggaggcgccgccatcgccggcgaatccgtcctctttttggacctcgctgcgttctacaccgtggcctctgcgtacctgcgcgggttggacatcaaggaccgcgaccgccggcgcaccgtcgtgctcgcaacgctgaccggcgcgcagggcgtggcgatcgtggacacgatcctcggcggcggcaaggccgacctgccgtcgaagcacaccctggcacgcttctccggcccgggcctgcaggaagcgaacgacatcctgagccgattcgccatgaagtcgctgaacaagcggatgcgcaggagctggttaggcaaactcctgccgctgggcattggcgcgttcgcggggcgctccgccaaccgcaagctcgccgacgcggtgctcaacaacgttgcggaaagcctcgggccagctccaagccagttcaccgagccgctgccggagaagggcgcaggcgacaaggacgagcgcgaggccgaggccaagctcagcgccaacccgcgcgagttcgccgcctggattgtgcagctgttcacaagcgccaagcgcgacagcaacgccaagcgcgacaagtaaatggcgtcaaacgccaaccccggccgtaacctgctctaccgatcccttcgcgctaaccgcggcccggccatcgccgcgttcacggcggcgggcctaagcgccgtgttccaaaccgcggtgccggcgctaacaggccgcgccatcgacatcgccgccggcaacgcgcaaggaagcatccaccgcatcgcgtgggcgatggtggccattgcgctggcctccttcgccgtcaacttcctgcgccgcttcacgtccggccggctggcgtcgaactcgcagcactggctgcgcgtggaactgcttcgcaccatgcaccgcctcgacgggccgggccaggacaacatcgccgcgggccagatcgtctcgcgctcgattacagatctcaaccagttccacatggtgctcgccagctcgccgatgctgttcacccgcgcactgcagctcaccaccacactcgtggtgatgttcgcgatggacgtgccgctgaccctcatggcactggcgttgatgccgctgatcctcttcgaggccaaccgctcgcgccgcgcgctctacgccgcgacctgggtgaaccagcaggccgcggcagatctcacacagcacgtcgaggagacggtctccggcgtgcgcgtggtcaaagcgttcggccaggaagagcgcgagatcgatcgcctcgaccagctcggccgcgagctctacgcggtgaagatgcgcacggcgaagctcaccgcccgcttccagccggtgctcgcgcagctgccgaaggtcgcgcttgtgatcaccatcgtcgccggcgggctcaccgccatccgcggcgatatcaccgtcggccagttcgtcgcgttcactggttacctcaccgcgatgaccacgcagctcgaggcgctgacccgccagtacgtgcgcatgcagatgggcatgagctcggtcgaccggctggaggaggtcctagctctcgcgccgacgaccgcccgcaaagcacccatcgcgccggccgcgcccaccggcatccgcttcgacaacgtcagcttcgaaaccaacggccacctagtcctcgaccgcgtgacgctcaccgtcgcacccggcgaacaagtcgccgtcgtcggcccgcccggcgcgggcaagtccatggcggtgcagctcgccggcgggttctacgagccgggcgaagggagcatttcgcttgtcgacgcccacctcaaccccaccccctacccccatctcacccacgccgacatccgctcgcgagtcacctgcgtcttcgacgaagcgttcctcttctccgcgtccgtgttcgacaacatcgccctcggcgcgcagcaccgtagcggcgcgcaagcgcttgacggcgccgcgctcgacgccgcggtgagagaagctgcccgccttgcccgcgccgacgagttcatcgagcggctgccaaacggctacgacaccgaagtcggtgagcgcggactgaccctttccggcggccagcgccagcgcatcgcgctcgcccgcgcgctcatggccaagccggcagtcttagtcctcgacgacgccacctccgccatcgacgccgaaaacgaagcgctgatcctggccaacctgcgcagccacttggacggcgtcaccgtcatcgcggtcgcgcaccgccagtccaccgtcgaccacgccgaccgcgtcgtcgtcatggaccagggccgcgtcgtcgcagacggtccgcgcgaggaggttgcgcgcacggaggtgtaccggggtgtgatggttgaggggggcgtcggcaagcagcagcccttgagcgaactgtggcccgacgtgcctgcacccccgccgcccgccagcgccacacctgagcttctgcagcgggtcgagcgcctgcccgcggcgcgcgaaacccctgccctgagcgaggcggcccttgcgcgcctgcgcgagccgaaccgcgacttccgcgtgcgcagcctgttcaaagccgtgcgctggctcattgccgccaccgtggtactgctggtcgtcggtgtggcggcggacctggcgtttcccacgctaatccgcgcgtcgatcgacggcggcatcgagccgcgcgactccggctacctcgtgcgcgtcggcgccgcggcgctggttgtcgtcatcgtcgcgtgggccgccgacgcactgatgaccgtgctctcctcgcgcgccggcgagcgcctgctctatcgcctgcggctgcgctcctacgcccacctgcagcacctgggcctgagttacttcgagtcccgcctatccggcaagatcatcacacgcatgaccacggacatcgacacgctgtcgtcgtttctgcagactgggcttgcgcaggcgatcgtggctgtcggcagcctcgcgggtgtgagcgcgatgctggttgccacggacctttcgttgaccctcatcgcgcttgcggccgtgcccgtgatcgtcgcggcaaccgtggtgttccgctcgttttccaagcgcttctacaccgaggcgcgccggcaagtttcggctgtcaacgggcagttcgccgagcagatcggcgggatccgcgtcacgcagatgcaccgcggggaggcccacgccgaggcgcgcttcgccgcagagtcggaccactaccggcgcctgcgcatgcgcaccgtgaccgcgatgggcctctacttccccggcatgcaggcgatcagccaaatcatgaccgcggtggtcattttcatcggcgcgggccgcgtggccgacggcacgctgtctgtcggcgtgctcgtcgcgttcacgatgtacctaagccagctctacggcccgatccagcagctcggccagatcttcgactcctggcagcaagccaccgtcagcttcgagcgcatcaccgacctgctcgctgaacgcaccaccgtccccgacctcggcaccgcacccggcgccgctcaggccgcgcggggggagctttcgcttgtcgacgccaccttttcctaccaccccgaccacccacccgtcctcaagtcgttggacctcacattcgcccccggtgagaccgtcgcattggtcgggccgaccggcgcgggaaaatccaccgtggtgaagctgctcgcccgcttctacgacccgaccaccggcgttgtcaccgcctccggcgcggatatcgcgtcgtttcctctggttgggtggcgccgggcgcttgcgcaggtgccacaggagtcctacctgttcgagggcaccgtggcggacaacatcgcctacggcgcgcccggggccagccgctccgagatcgagacagccgtggagcgcatcggcgcgctcggcatcatcgccgcgatccccggcggcttcaacgcgcgcgtcggcgggcgcgggcggggcttaagctccggccagcgccagatcatcgcgcttgcccgcgccgagatgctcgtccccgacgtgatgcttttagacgaagccaccgccaccctcgaccccgcaaccgaactggccgtgcttaacgccgccgaccgcgcgacctccggccgcacgtccgtcatcgtggcacaccgcctcgccactgccgcgcgcgccgaccgcgtcgtggtcatcgacgacgggcgtatcgtggaatccggcacgcacgccgaactggtgaaagaagggggccggtatgcacgaatgtgggcggtccaccgataatgggggtaccgaccccgtcgtgaccgaaaacacggttccacggcgctaccatcggcttgaagtctacgaaagaccctgcaaacttacttgttaaaggaaggcgatcactgccgtgagcagcgaaaacacatttgggcagaacagctggctggtcgacgaaatgtaccagcagttccaaaaagaccccaattctgttgacgaggagtggcgcacgctcttcgaagacaacggtgcgccgaagacagccaagggcaccccgaccgttaccccttccgatcccggcgcaagccagccgaagaccgacccggacgtagcgcgcaccaccgcggcgccgagccaggacggccgcgagaccaaggtcgacttggctgcggagcagaccaagaaggacgctacggttttgccgaagccgcgcaagtcgccgctggaccgtattaaggacgtccacgtcgagccgggcgagacccagctcaagggcgcatttaaggcgatcgcgaagaacatgaacgagtcgctggaagtccccacggccaccaccgtgcgcgacatgccggtcaagctcatgtttgagaaccgctcgctgatcaacgaccacctgaagcgcacccgcggcggcaagatttcgttcacccacatcatcggctacgccatcgtccaggccaccaagctgcacccggacatgaacaagagctaccgcgaagaggagaagaagtctttcgcggtgcagccggagcacattaacttaggcctggccattgacctgccgggcaaggacggctcccgctccctggtcgtcgccgcgatcaaggagtgcgagaccctttcctttagccagttcgtcgaggcctacgaggacattgtggagcgcgcccgcattggcaagctcaccatggacgatttctccggcgtgaccatccagctgaccaacccgggcggcatcggcacgcgccactccatcccgcgcctgaccaagggccaaggcacgatcgtcggcgtcggcgcgatggattacccggctgagttcgccggcgcctccgaggaccgcctggccgagctcggcgtgggcaagctggtcaccctgacctccacttacgaccaccgcgtgatccagggcgcagagtccggcgagttcctgcgggacatctcgcagctgcttatcgacgacgcgttttgggacgacatcttcgagtcgttggagatcccgtactcgccactgcgctgggcccaggacctgccgaacacgggcatcaacaaagacacccgcgtgatgcagctgatccactcctaccgcgcccgcggccacctcatcgccgacaccaacccgctgcgctggcaccagccgggcctgccgaagccggactcgcgcgacctgctgctcgagtcccacggcctgacgctttgggacctggaccgcaccttccacgtcggcggcttcggtggcaaggagaccatgacgctgcgcgaggtgctctcccgcctgcgctccgcctacaccctgcacgtcggcgccgagtacgcgcacgtgatggaccgcgacgagcgcgagtggctgcgcgaccgcatggaggccggcatgcccaagccgaccaacgcggagcagaagtacatcctgcagaagctcaacgccgccgaagcgttcgagaacttcctgcagacgaagtacctgggccagaagcgcttctcactcgagggcgccgagaccctgatcccgctcatggacgcggcgatcgacaccgccgccggccagggcctcgacgaggtcgtcatcggcatgccgcaccgcggccgcctgaacgtgctgttcaacatcgtgggcaagccggtcgcgacgatcttcaacgagttcgagggcaacttcaaggccgcccagcagggcggctccggcgacgtgaagtaccacctgggcttcgagggcgagcacatccagatgttcggcgacggcgagatcaaggtctcgctggccgccaacccgtcccacctcgaggccgtcgacccggtgctggtcggtatggcgcgcgcgaagaccgacctactcaaggccagcgagggccgcgaggactacccggttatgccgatcatgctgcacggcgacgcctccttcgctggcctcggcatcgtccaggagaccctgaacctgtctcgcctgccgggctactccgtcggcggcacgatccacgtgatcgtgaacaaccagatcgggttcaccaccaccccggattccggccgctcctccttctacgccaccgacctggccaagggcttcgactgcccggtgttccacgtcaacggcgacgacccggaggcagcagcgtgggttgcccagctcgcaaccgagtaccgccgcgagtttggcaaggacgtcttcatcgacctgatctgctaccgcctgcgcggccacaacgaggccgacgacccgacggtgacgcagccggtgatgtacgaccgcatcgagtcccacccgtccgtgcgcacccgctacaccaacgacctggtgggccgcggtgacatctcccaggaagacgcggagaaggcggcgcaggacttccacgaccagctcgacgcggtcttctccgacgtcaagtcgtctgaggacaagccgagcgagcagaccggcatcacggactcccaggagctcacccgcggcctcgacacctcgatctccgaggacgagttcaagcgcctcgcggctacctacgccgacctgccggaggacttcacgccgaacaagcgcctgaagaacgtgctgaagaaccgcggcaactcgttcgaggccggcaacatcgactggggctggggcgagctcatcgccttcggctcgctggcggagcagggcaagttcgtccgcctcgccggcgaggattcgcagcgcggcaccttcacgcagcgccacgcggtgctctacaacccggacaacggcgaagcgttcaacccgctcgaccacaacgccaccgaggccggcaacgagggccgcttcgaggtctacaactccgcactcaccgagtacgcgggcttgggcttcgagtacggctacaccatcgccaaccacgacgcggtggtggcctgggaggcgcagttcggcgacttcgccaacggcgcgcagaccatcatcgacgagtacatctcctccggcgagaccaagtggggcgagctgtccagcctcatcatgctgctgccccacggctacgagggccagggcccagaccactcgtccgcccgcatcgagcgctacctgcagctcgtcgcggagggctccatgaccatcgcgcagccgtcgacgccggcgaaccacttccacctgctgcgtcgtcaagcactcggcgagatgaagcgcccgctggtcgtcttcacgccgaagtcgatgctgcgcaacaaggccgccgtgtcccagccggccgacttcatcgagaccaccaagttcgagtccgtcatcgacgacccgaacttcatccagaccggcaacaagaaggtcgacggcgcggacctggacaaggtcgagacgatccttttgtgctccggcaaggtctactacgagctggcgaagcgcaaggagaaggacggccgcgacgacgtcgccatcgtgcgcgttgagatgctgcacccgatcccgttcaaccgcttgaaggacgcgttcgcgaactacccgaacgcgaagcagatccgcttcgtgcaggacgagccggccaaccagggcccgtggccgttctacaacgagcacctccgcaacctcatcccggacatgccggagatggttcgcgtctcccgccgcgcccagtccaccaccgcaaccggtgtggcgaaggtgcaccagcaggaggagcaggcgcttatcgacgaggcgtttgccaactagcccgccctacacgggcggctgctccgggtcgatcgagaccacagcaccgcctgcgggccctggcgcgatgccggcgtactcgagcagccagtcggccacggcgacgtcggcaggcaccccctgccccaccttctcggccgattcggcgatgtcttcggtcgccatcatgcgggtgatgaagttgatgcgctggatggtgccgcggtcgaacttgccattgcggaagacagggatgatgttctgcacgagccgctcgccgtcggtgtagccgcaaccctgcgccggggagggatcgaccgttcgcatggtggcgggcagcgtgcccacggccgcgtcgtacgtcgccaccgacagctcctcgccctccataccgcttgccgctagttccgcagccgcggccgagtcgtacgtttcaagcaccgcgcctgtgcacgtgaccacgagatcgaccggctctgcgcgcaagatctctagcgggtcgagcgcctcggcgccgccgaagctggacacgccggcggcgtagcccatggcgtcgaagatctggctgtagatctcccccaacaccacctgctcctcggagcttgcgtcgatgccgatcaccacaggtatcggctcgtcggcgcaggacgccacgcttgccgacgccgccacaacgcccaaccccccaagaagccgcctacgcgccatcggcaggacgcggatcacccgccggggcacttatagacgcaatcaagtcgcgggcctgaggcgccgcgtccggctcgcacagcacgtcgtagtggcccgccacgatggaggtcgccgacgcgaagtcgcgcttgcctccggagaacccgtacgcgatcgccgcgaagatgatgccgaagatcgcgccgatcagaagggcccacaggaaaatggaccagccggtgcccggctcggcgaatagcgtaaaaatcaggccgatgaacaggcccatccacgcgccagacagcgcaccgccgccgagcaccttgccccaggtcagccggccggtgatgttctcgacctgcataaggtcgacgccgacgatggtgagcttctccacggggaagttgcggtccgacagcccgtcgacagccgcctgcgcttcaagataggtgttgaaactgccgaccggccatccggagggcactgctttgacgttgggtttagtcatggtccctcactatacttacccagtgatatgactacttcgaaccacatcacgcgcgaggccgtctacgaggcactttcgcgcgtcgaggacccggaaattggcaagccgatcacggagctgggcatggtcgagtcagtgaccatcaccggcgcggacgtacacgtgggggtctacctcaccatcgccggttgcccgatgcgcgacaccatcgagcgcaacacccgcgccgtgctggaggagctcgacggcgtgggcagcgtcggcgtcaccatgcacacaatgagcgacgagcagcgccgcgccctgtcggagaagctgcgcgccgagcagccgagcaccgcaatccccttcgccgacccggacacccgcacccgcatctacgcggtggcgtccggcaagggcggcgtgggcaagtcgtcgatgacggtgaacctcgccgtagcactcgccgagcagggcctgagcgtgggcattgtcgacgccgacatatacggccactccatcccggggctgatgggttccgccgacaagggcccgactgtcgtggacgacatgatcatgccgccgatcacccacggcgtgcgccacatttcaattggccagtttgtggagggcaacgcgcccgttgtgtggcgcggcccgatgctcacgcgcgcgatccagcagttcctcggcgacgtctactggggcgatctggacgtgctcttcatggacttgccgccgggcaccggcgacgtggcgatcacggtcgcgcagctcgtcccgaacgcggagctaatcatcgtcaccaccccgcaagccgccgccgcggaagtcgccgagcgcgccggcaccatctcccagcagacggagcagaaggtcgcgggcgtgatcgagaacatgtcggggctcatgcttgacgacggcaccgttcaccacatcttcggccaaggcggaggccagcgcgtcgcggagcgtctgactcaactcacggacagcgacgtggcactcctcggctccgtccctttggacccgaagcttcgggagcacggcgacgacggcacccctgtggtcatttccgagcccgactcccccgccgcggccgagatccgccgcattgcgagcacgctgaaggtgcgccgcgactcccttgccggcaagagcctcaacccgcaggttaagtaacatcctcccaggagaagccgccccgccgcttctcctccggcgccgccggtttcggcccggccttcggcgccggccgcggccccgaattcacgcgcggttcctcgtccgcctccgcgagcacgcggcgcgggtcgaagctgccgaggtagtcctcgtcgccctcgaacaacagcgatgacaccgcccgcttcggccccatcgccgcgtagcgcgacacagtgtcgagcggctttttgaactcgtcgaactcctccagctcgccgttgagctccttcttcgcgttcgcgatggccttgcgggcggcgtagatggccgcgcgcacgtcctcaatcacgctggggagccgctccgggccgatgacgatcagcccgatcacgaggacgagaaaaaattcgccccatccgaaactggaaaacaccgttcctaccctactcgcggcccagcagcgcccgaagcgcctgctccgctttttcccgcttgccggcggccgcctccccgctctcggcgccgccgcactccgccttcgtcagccccgacaacttggccaccagcgagctcggcgcgcgcacgtcctcgccgcacgagccgcgcacgcgctcagacgcgccgcgctgggtggcgacctcgtcttggcattcggggcattgggcgaggtgttgctgggcccgtcgataagcagccgtgctcagctcgttgtccacgtacgccgccaccgcctccgggcttaggtggtcggtggacgaaaagtgccggtgtcccgtcatcgggaacggatcaactcccgcgcggcgacatccacctgcgcttgcgcctccagcgacgcgcgcagctgcgtgcggccgcggtggatgcgcgagcgcaccgtgcccattttcaccccgagcgtgtcggcgatttcctcgtagctcatgccgacgacgtcgcacagcaccaccgcgacgcggaagtcgggcgccagctcgtccagcgcgtgctgcagcgcggggtccaagttggtggccgtgtacgcctgctccggcgtcatcgcggtgcccggcacccgctcgtagtcctccggcagctcctccatccggatcttggagcggtggcgcaccatgtccagaaacaggttcgtggtgatgcggtgcagccagccctcgaacgtgcccggctggtagcgcttcaggttgcggaagacgcgcatgaacgtctcctgcgtcaagtcctcagcgtcgtgctggttgccggagaggcggaacgcgagccggtagacgctgtcggcgtgctcggcgacgagctccgcccacgacggcatctccccgcaccccgcgtcgaaggcggctgtgcccgtcaactcaccagcgtcgtccatgcgcagcattctatccgactatgctttcagggtgtgagtgatgagatgacgtcgtacatccttgaggcactgcttgacgacgcagcgctggaacacgcctacgtcgaaggggaagaaaacggggtgcgcgggccgtcgccgatcgtcggttcccttttgaccaccctggcaaccggcgcgtcgcaaggcgcggtggccgtaacccccgccgccggcgtcgtgggcctgcacatcctgcgcggcctgccggagaaggcgacgctgacctgcatcgagccggaggcggcgctgcaaagcggcgcgaaagaggcgttcaagctcgccggccactcgccctcgcgcacgcgtttcctcaccgcgcagccggcgagcgtgatgagccgcctcgccgcggagacctaccagctgatctacctcgacgtctccccgcgcgagcttgtcgccatcatggacgaagcttggccgctgctcacgcgcggcggcacgctggtcatcgccgattcgcttctcgacggcacgatcgccgaccccacccgccgcgaccgtgaaaccgaggccgcccgccaggccgacgcgcacgcggacgcgcttgcgcaagacggcgccagcgtggtcacccgcctgccgctcgacggcgggctgaccctgattacgaagcgttagaccacttcgttcttgcccacgaccactaccccgccgtcggagacggtgtagcgggagcggtcgcgctcgtggtcgacgccgatgatctcgccgtcggagacgtagacgttcttgtccaaaatggcgtggcgcaccaccgcgccgcgcccgatgcgcacacccggcagcagcaccgagccttccacggtcgcgccctcttccacgcgaacgtcagttgaaagcaccgagttgcgcaccgtggcgcccgagacgatggaaccggacgccaccatcgactcctgcgcaataccgccgagcacgaacttcgccggcggcaggttcgagtcctccgtggagtggatcggccacgccttgttgtagaggttgaacaccgggtgcgaggagatgaggtccatgtgggcctcgtagaaggagtcgatggtgccgacgtcgcgccagtagcccttgtcgcgttcggtcgcgcccgggacctcgttcgtggaaaagtcgtagacgtgcgcctggcccttcgacacgaagtacgggatgatgtcgccgcccatgtcgtgagccgagtcgtcgttttgctcgtcttcgaggagtgctttgattaacgcttccgtcgaaaagcaataattgcccatcgacgcgtaggtggtgtccgggtcgtccggcgtgcccggcgggtcggcgggcttttccaaaaactccgtgatcgagccgtcgccgtccgcctggatgcagccgaacgccgacgcctccgtgcgcggcacgcgaatgcccgccaccgtggcgtccttgcccgaagcgatgtggtcctccaccatctgcgacgggtccatgcggtagacgtggtccgcgccgaagacgagaacgtaatccggcatgtcgtcgtagatcaggttcagcgactgcacaatcgcgtccgccgaaccggagtaccagcgcttgccgcggcgctgttgcgccggaaccgaggcgatgtactgcggcgtcggaccggaaacgttccaggccgtggccacgtggcggtcgagcgagtgcgacttgtactgcgtcagcaccgcaatgcgcatgtagcccgcgttgaccaggttggagaggacgaaatctatgaggcggtaattaccgccgaacgggaccgcaggtttcgcgcggtccgcggtgagggggaacaagcgcttcccctcaccgccagcgagaacgatggcgaggactcgaggctggctcttcatggccccaagcgtagggaatccggcccgtttgcgcagcacattcagcaggtccatgcactagtctgcggaaattattaagctcggcgggcatgaaagtcggaatgctgaccaaggagtatccgccggagatctacggcggtgccggcgtccacgtcaccgagctgacgcgcttcatgcgcgacattgtcaacgtcgacgtgcactgcatgggcgcgccccgcgacgaggcgcacgtgtacgtgcacggcgtggatcccgagctggcggatgcgaacggcgcgttgaagacgctgtccaccggcctgcgcatggccaacgcagcttccggtctcgacgtggtgcactcccacacctggtactccggcctcggcggccacctcgccggcctgctgcacgacatcccgcacgtagtcaccgcccactcgcttgaaccggaccgcccgtggaagcgcgagcagctcggcggcggctacgacgtgtcgtcctggagcgagcgcaacgcgatggaaaacgccgacgccgtcatcgccgtctcctccggcatgaaagacgcgattttgcgcgcttaccccgccatcgaccccggcaaggtgcacgtcgtgctcaacggcatcgaccccgagaagtggcacccggagaagggcacgataactgacgagctcggcgtcgacacctcccgccccatcgcgagcttcgtcgggcgcatcacgcgccaaaagggcgtgccgcacctgctgaaggcggcgcagcagttcgacgaggacattcagctcatcttgtgcgcgggtgcgccggacacgccggagatcgccaaagagaccagcgacttagtggcgcagttgcgcgctgagcgcgacggcgtgttctgggtcgaagagatgctgccgtcggagaagatccgcgaggtctatgccgcctccgacgtgttcgtctgcccgtcgatctacgaaccgctgggcattgtgaacctcgaagcgatggcgtgcggcaccgccgtggtcgcctcgcgcgtcggcggcatccccgaggtggttgtcgacggcgagaccggcacgctggtcgactacaacgagaacgacgcggccggtttcgagcgcggcatcgccgacgccgtcaacgccatcgccgccgaccgcgacgcggccgagcgcatgggcaaagccggccgcgaacgcgcggtcgccgacttctcgtgggccaccatcgccgaacaaaccgtcgacatttacaaaacgctgatttaggacgctgcttacatgactaccttcagaccagaactccacatcaccgcggaagaaggcatcctcgaaggacccgccggcgtggttcgcctcggagaggagaacaaccgcgtttggcacatgttttaccagtaccgccccacgcctgacgccgcgagccggtggggccacaacatgagcgaggacgacccgttcagctggtacgagtgcaacgacgcgatcatcccggccggcggcgagcgccacgtgcgcgccggcgcggtggtgtgcggcaccgagagcgacggcggggtggacatctacttcacctccaacacagacgcgggcaacacgattcagctcgcgcgcgtggacgacgtgaacggactttgcgccgatctggacgccgacggtgctgatgtttccgctgccgtgaagcgcctcggccaagtggtcgacgccaccggcgagttcgacaacctccgctctccctgcgtgttccccggctggtccagcgccgccgaccgcgattccggccacgagggctggggtatgctggctgtctccggctccacggacgccccgcagccggtggtattgagttcgggcgacggcagggcttggcttatcgacggcccgttgaacttcaacggcgaccccggcatcgaactcgacgcctccgtggtcgccccgcgtttggtccgcctgcgcgacgaagtcgacggcgagatttacgacgtcctgttcatcaccgtcgagcgcgacggcaaggacgtggcgagctacatcatcggcaagctggaaggcaacacgttcaccgttgtcacgccgagccagctcttcgaccacggccacgacttcacccgcccgcgcaacacgaactacccccgcatcgccgaggaggagctgaagcgctacgagcgcgcgtacatctacggcttcatgacgaactcgggccgcgccggcgacccgaccgccgagccaaactgggcgtccgagggctgggcgaacacgctcaccctgccgcgccgcgtgaccctgcagcacggccacctctaccaagtgccggcgccgggcctgcctgaggcggtcgacgccgcggagcgcgccctgatgtggaccgggctgtgcaccatccccgcaggttccgaggtcgtcgccgaggtgctcgacgccagcggcgagcccgccgcgcgcatctcccaccacggcgagcgcattgagctggaccgcttcgacggcgatccgaagcaggccgcgcttcacgacgaagacgaggacaacatcaccatcatcgtcgacggctccaccctcgaggtgtacgccggcggcggcagcgttgtcatgtcctcgcgcttctggcccgcgggcggcgcaagcgggatccgcgtgcgcaccagcggcagcgccgagatcttcagcgagtggcggcgcggccacaccgcgctggggatctaatgccgcgcacgggaacgcggcgtagcagggcgatcgcagccgccgctgccgcgtcggccctcctcgctgcgtgtggcggcgagcccgcccccaccacctccgc

SEQ ID NO: 7 - DNA, 196859 bp, Corynebacterium cassirii
  source 1..196859: mol_type = genomic DNA
gtggggtagaaggcgtcggggcgggcgtcgataagcaaacgaagctctgcttcgtcgagctgcgcaagtgcttgggcaaaagacatttccagcaatcctacgtgcgttttgtttcccggcgtgagataatgctgcgtatggctaaagatgcagcgaagatcggccgcgcgaacccggcatggcccacccacgttcccggtaatggtcacccggtgaccgaaatctccaacaagctcactggcgcgaacagcccgttcggcaacgagcttgtcctgccgctgccggcagaccaggtcgggtacgtccacccgaccacgcgcatcaaccggtaagcattatcggtagcaaaaaggaccggctccccgctgcggggagccggtcctttttgccgcgcgcgtttcagccgttctaacgcaacgcggcgatcgcgctctggacgtcgccggtgagtgcggcgtcgatcagcgtctggttcgccaggtagaagccgttgtagtcgtggcggttcgcggcgtagttgtcgtgaacgaactgcggcacggcgaagcctgcgtctttcacagcctgggtgagttggttgtacagctcgtcaacggccagatcggacttggagctcgttgccggagccgcgggagcggccggtgctgcaggagccggggccggggccgctgcctggtggtcgcggttggtcggcgccgagttcaggccgtagcgcgcggagcaagccggccatgcgccccagccctggccggcgagggtgcgctcagcgacgatgatctgctgctcgcgggtggccaggtttgcggtcggggcgaactggccgccgccgtaggcgagccaggtgccatatgagaactgaaggccgccgtagtagccgttgccggtgttgatggcccagttgccgccggactcgcactgcgcgagcttgtcccagtcggaatccggggcggcggaggcctgcggggcggcgatgccggtgagcgctgcaacggccgcggtgcccgcgagcgtcttcttggtcaccgaggaggtctgcttggagtggcgtcccatggagatgttccttcgtatcgacttcggttgacgtttgcggcaagcctaacggtttataacgattcagtcacgctgcggatacgatacgaacgatatgacacgtccgcgaagagtgtttgtgctggttacgcgcgattcaacatgtagatgtgaactgcaccacaggtagtgcgatctgggtgcgttgcgggcaggagtatgctgaagcctttaattagaggaggtttcgccatgccagttggaaaagtcaagtggtacgacgcggaaaagggcttcggtttcgcgtccaaccccggggatgaggacgtctttatcggtcgcaacgtgttgccggagggcgttgacgaactcgtcgccggccagcgcgtcgagttcgacttcgccgccggccgccgcggcccgcaagcgctgcgcctgaaggtgctggagaccccgaagcgccgccccatccaccagcgcaagccggaggagctgggcagcatgcttgccgacgtaatgacgctcatcgagacgcagattcagccggcgctgaccgcgggccgttacccggaccgcaaggaatcccgccaggtggcggagatccttcgcgcggtggcgaaggagctcgacgcttaaaaagccagcacctagaacccgaccgaccacgtcgcgatcacggggatttcctccccggacgcgtcgtggtcgattgctagcgctgaaacctctgcgaccacgaggcgggcaccggactcggtgaccgcctctacgtcgtgttcggaggcttcgcccgaggtgtagacggtttcgttgttggcggcggggtcgtcgtaaatcgccagcatccgccagctggagttggctatttcagcagggacggaaacgtgcaccgccgcttcgtcgagctccatgctcggcggctggccgccggggcactcctcgtccagttcgcagacggtgtacggctcgacctcgagcgtcttcccagccgaggtgacctcgacgcgcagctcgcgaaccggggtgccggggcgcgagttctgccactccagaaacgcgtacaaacccgcgaccagcagcagtgccgcgatcacgatcgcgatgacgggcttcacactcttcgctccagcaggacgtgccatgggtgcgcagtctagtcggccgcctcgaaggtgacgcggtacaggtcgggccagcgcttgccggttatgtagaactgcgcggggtccgacgtgccgggaatgtgggcgatgccgttgagcacgttgttcgggtccgctgcggcgttgttgggcacgccggaggcgtcgatgaccgcggtgacctcgcccgtcgacgcgtcgatgcggacgatgtcggtcgtggtgaagatgtttgcgtagacgtcgccgcccacgcactccagctcgttgagtccgtcgacaggcgcgccgccgcgggtgacggtgaagcgctcccgctcctgaagcgtcacggggtccatgcgtcgcagctctgcggagccgtccgagaagatgacctcgtcggcgtcttcgcggaagcagatgccccagccctcgccttcgtaccccgcgcgcgaaatctcctcgagggtgaccgggtcgcgcagcaccgctacctggtcttgccaggtgagttggatgaggtgggcgtcggcaagcgtaatgccctccccgaagtgtgtcgggtcgagtggcgcggaagcgacctcctcaccttcgacggtgcggcggtacacccgagactgcccctcccagccggtgccgacgacgatggtgccgtcgggcgcgacctccaaaccttgggtgaagctggtgtcgtcgaaatccaggcgctcgtgcaccacggcggtcagcgcttcgggcgcagcatcagctgagcagccggcggaaagcagcgaggaacacacggcgagcgacccaacgaggcggcagtgtttgaccatggccaccatcttgcatcagccaattctgcgttgcgcataatgggggagtgagacaaaccagacgccaacgcacctcctccggctctccgcttcttaccccagaggcagtggagaccgcccgcggcgcgctcgcggacgttgccgacgacggccaaatcggcgatcacatcggggtgacgggcttaagcgccaacgtggccacccaccgcttcgaggcgcacctgcccggctacaccggctgggagtggaacgcggtgctggcatgcgcgaccgggtcggacagcgtcaccatcaacgaggtcgccctggtgccggccaccggagcgctcgaggcgccggagtgggtgccgtactccgagcgcgtgcgcccaggcgacctaggtcccggggacttcattgagcttttgcctgacgacgtccgcgtgacccaagattcattctcccgccacgccatcactttccccggcagggagacgaagtattacctgactgagcaggggctcgccgacgcggagaagcgctggcgcactggcgactacggtcccaacagcgagttcgcggagaaggcggcgctgcactgccgaagctgcgcgttctacatcccgatgggggagccggtgggcgacaacttcggcgtgtgcacgaacatgtactccgcggacggtcatgtcgtggccgcgtcctacggctgcggcgcccactcagacaccgtcgtcaacgactagcgggtgctacacccgctccgcgagcagcttgcgcgtctcgttcacctcgcggtgggagggcaagccgccgcggtcgaacaggaggcgcgccgggcggggcgtgccgtactcgagccacgtctccaccagtcgaacgccgtagacggggtcgatcacccacacttcgttatcgcgcagttcccccacaacgaacccgcgaggctcctccacgatgtccgcgccgcggctggcgaggatgtcgaggaccgatgcaagcgctaccgagcgcggcgagtgcgggtgggtggagacccggacagcaccccgctcgatcaccgcaagcgggtgcatgattgcggaaaggatgctgcccgcggcgtcgataagcaagccctcctgcgccggcagcgcggcgagcgtgctctgctgccagccgtaatccggaccggtgcgggtgggctgggtgcgctcgtccgcaaccggctccgcggccacggtgatttccaccggcgcaggggccagcgggcgcagcgcgagcgaggcggtgccgccggtaatctccagcacgccgcggcgggtgcccgccacatctgccagctggatgcgcaggcgctgcagctctttctggctcacacctagatcgcgcagcgcgcgagcgtaccgcggcgcgtcgatcaccctgccctctgccactacgaaattgaaaacgtccacgcttactacggttgccccaaatgcgcctgaattggaaaaaatggttgcggagtgcaagtctatgtcagtcattagccagcgaaatcctatggccttcccatgagtacgaagggttgcacacttcccgtgactacgaaacacgaaccggcgcacaagccggcggcaggcggtctcgaccggtttttccacatctctgagcgcggctccaccgtcggccgcgaggtccgcggcggcgtggtcacgttcttcgccatggcctacatcattctgctgaacccgctgatcctgggcacgagtccggaccgcgacggcgtggtgctcggcatcccgcaggtcgctgccgtcacggcgctcgtggcaggtgtgatgtgcatcctcttcggcgtggttgcgaagtacccgttcggcatcgcgacgggcctcggcatcaacaccctggtggcggtgaccctggtcgggcagcagggcctgacctggcccgaggcgatggggctggtggttatcgacggcctgattatctgcctgctcgccgtcaccggcttccgcaccgcggtgttcaacgccatcccgaactccatgaaggtggccatgagcgtgggcatcggcatgttcatcgcgatgatcggtctggtggacgcgggcttcgtgcgccgcgtgccggacgccgcgatgaccaccgtgccggtgcagctcggcttcgagggttctatcgcttcctggccgacgctggtcttcgttatcggccttgccatctgcggcttcatggtggtgcgcaacgtccccggcggcctgttcatcggcatcgtggtcaccaccgtcatcgccatgatcgtcgaagcgctcaccggcgcaggttcctcggcggacgacccgcacggctggtcgctggccgtgccgcgcctgccggagtccttcggcggtgtgccggacctgtcgctggtgggcaaggtcgatctggtcggcgcgtttgtcaacgccggtgccgtcgccgcctcgctcatggtgttcacgctcgtgctcgccaacttcttcgacgcgatgggcaccatgactgcgctcggtcgccaggcggaacttgcggacgagcagggcaacctgccggacatgaagcgcgccctggtggtcgagggcttcggcgcggttgccggcggtttcgcctccagctcctccaacaccgtgtacgtcgactcttccgcgggtatcgccgacggcgcccgcaccggtctggccaacgtggtcaccggcgtgttgttcctgctcgcgatgttcttcaccccgctctacgaaatcgtgccgatcgaggctgcggcacccgtgctggtggttgtcggcgcgctgatgatgatgcaggtcggcggcatcgagtgggacaagttccacgtggcgctgccggcgtttctcaccattgcggtgatgccgttcacttactccatcgctaacggcatcggcgtcggtttcatcgcgttcacgctgatggcgctgttctctggcaaggcgaaggagattcactggatcatgtggctgatctccgcgctgttcatcgtctacttcgcgcaaggcccgctgctggcggcattgagctaatgcttatcgacgaccccttcaacccccttctcgacgacatccggaacctgaagcgttccgacgccgagaaggggctcgtcattgccgagggaccgcttgtggccggccgcctcgtggaatcgcgttttccgcttcgtgccgtctacgggttcggcgggcgcttagccgcgttcctggaagaacatggtgacgagctttcccgccgcggcgtgccggtgtacgagaccccgcgcgaggtgatgggtgccgccgcaggctacgacctgcaccgcgggctgctcgcatcggcggaccgcccagagccgttgacggtgcctgaggtgatcggcggtgcgcgttcactcgtcatcctcgaaggcgttggcgaccacgagaacatcggctcgatcttccgcaacgccgccgggatgggcgtcgacggcgtgctgttcggcgcgtccaccgcggatccgctgtaccgccgcagcgtgcgcgtgtccatgggccacgtcctgcgcaccccgttcgcccacttggagggcaccacgaccacttggcagcgctcgcttacgcagctgcaagatgcgggcttccacgtcgttgcgctcaccccgtcccacgacgcggtgccgctcaagcaggcgtgcgcggggcgcgagaagatcgccttcctcgtcggcgccgagggcccgggactgactgagcacgcgatgcgcgcagctgacgtgcgggctcagatcccgatggcgccgggcacagattcgctcaacgtcgccacctcggcggcgatcgcgttctacgagttcatgcgctagcggtcggagtggcgaatccgctcctggattgcccgcttcgcctcagccaggcggcagcgtatgtcgcgcccgaggcggcgcgcggcagcgactgacgcatccgcaagctcggcaaactcgttgccgtcttcggccggcggcgtgacgtcgtagtcgtcgtagtcgttgtctttttctgcgaagcgcgcggcgacttcgctcaccgtcttggttttcggcttctccggcggcgcaatcttcggctctgggcggccgtcgaccgcgtagccgaccacgtggacgtctggtccggcgccgcggtgctccagatccaccccgacccagctgcgctgcgcctcatgcatcaggtccttcggctcgaaaggcagcgtgatgccgccgagctgctccgctttctcgccggcccaatagaccgcttcgaagggctcgggcaaaccgatgtcttccagcacccgctgacgcgtcgcagtcaaggagcggcgaaggtcgtcgccgacgtagtgggcgaagcccgcgtagtccgtgtcggctccctcggcgaagaggtaggtgtcggccgccggcagcgcgccgcggaggtactcaacagtctccgtgagcttgtcggagtcctcgacgaacgtctggaccaccgcaacccccgggtagccggcgatgtagaactcgtctctgcccggcttggaggagcggtttaaggggaactcgccgattggggtgatgggccacgctgggttgatctgcgccagcagcttgcggccgaacccgcggtccgccttcggctcggcctcgagcacctcgcgcgggttggctgcggtgataaaccagaacgtcacaactgccgggtagcccatggttagctccttggacgcttctgcgtggtgcgcacaccgagcaggacgtcctcccagtgcggggtaacagccttgcggcggcgcttctgcggttgttcggcctcgtcagggtgctgcaggaactcgccttcgagcgcctccggctcgtcgtcctccacggcggtcagcgagcgcaccggctggacgaagtcggggtctgtcaggtcggcagcgacggcgtcgcgcgcctccgtggtcgctcccgcgcccatctggcgcttgaacgaccacgtcgcttcgttatcggtgaggcctgcttgccagcgaaggtggacgacccatgtgtcgccgggttcgcgggtggcgtcccacgtagcgtcgacaagcgaatgccccctagccgcgaacgctgaggcgaggatctcaaacagggtgagcttggccgggccgccgtcgcggattgggtgggactgcttggcggcttcggcgatctgggagcgttccagcagcaccgggtgcgcgtagggctcgacgcggcttgcggcgacccccatttcctcggcgagctcggtgacagtcgcgccggcgcggatgcgggcttgaatctcgctgggccgcatcgacagcgccgtggcgaagagcggatccggctcgggcagcgtccgctcgacctcggcgggtgcttccgcctcagacgcctcagcggaggcctcgtcgaccgtctcggcggcttcggccagctcggccggttccgcaggctccgtcaacaccgccgggacctgcgggatctcggtgcgtgcgagctggtagcggacaccgtcagcgtcgtgcagtacaaaaaactgctccgttgactcctcttcactgagatatagctcgcgcataatggcctagcttaacccagggcagcgctaatttttcgcaccgacgccctgctcgagcagcgcgtcgatcgcgtgggtgagcgtttcgatgtccgcggtgtcgatcgaggggaacatgccgatgcgcagctggttgcggcccagcttgcggtacggctccacgtctaggatgccgttgtggcgcagcgccttggccagctcggcggcgtcgatctcgtcgtcgaagtcgatggtgccgaccacgagtgagcgcgcggcggggtcggtcacaaacggggtggcgtgctcgtgcgactcggcccaggagtacagcgcgttggcgttagcggtggtgcgcttgaccatgccctcgaggccgccctcggcgttcatccactgcacttggttcgccagcatgagcagcggcgccacggccggagtgttgtaggtctggttcttgcgcgagttgtccacggcggtttgcaggtccaagaatgccgggatgaagcggccggacgccttgacctttgcaatgcgctcgatggccgcagggctcatcgcagcgagccagatgccgccgtcggaggcgaagcacttctgcggggagaagtagtaaacgtcgacctcggtcatatcgacggggaggccgccggcgccggaggtggcgtcgataagcaccagcccctcggtgtcgggccgcacgaccggcaccatggcgccggtcgaggtttcgttgtgcgcccacgcgaccacgtcagctgccgtgccgtccaggtcgctcgggctgggggcggtgccaggctcggccttgaccacttgcggctcctccagccacggcgcctgcgcggacgccttggcgaacttgcccgagaactcgccgaagctcaaatgtgccgactgcttttcgatgagtccgaacgttgcggcgtcccagaacgccgttgcgcctccgagggagaggatgatctcgtagccctcgggcaggttgaagaactggctgaggccgtcgcgcacttcgccaaccaggttcttcaccgccggctggcggtgcgacgtgccgatgatatcggcgcccttggcgatggcgtcgagctgctcggggcgaaccttcgacgggccgcagccgaagcggccgtcagcgggaatgagatcggcagggagggtggggtagacgctcatcgagtggtcttgtccttcgctcggttgaaattgcagtaggtcgcataatataccggttggttcctctgggcggggcgggaaagcgatatctattcgccgccgcagaatgtggccggatgctgtttgcgcgaaccctgtcgtccgcatcacaggcggtgctactatggcacatggaaaatgtccgggttgtcatttcaactatctcgttcctgcaggttactgcggttacgggtaagtctggcaagacggattgtgatcacacgtggaaaggcacacagtggcttctgagaatgaaaacaaggcagtactgcactacccgggcggcgagtacgagatggacatcatgcgcgccaccgagggcaacgacggcgtcgtgctgggcaaattccttggcgagacaggcctggtcaccttcgacccgggctacgtctccaccggctcgaccgagtcgaagatcacctacatcgacggcgacgagggcattctgcgctaccgcggctacgacatcgcggacctggcagagaaggccaccttcaacgaggtgtcctacctgctgatcaacggcgagctgccaacggtggaggagctcgactccttcaacagcgagctgcgccaccacaccctcttggacgaggacttcaaggcagcgttcaacattttcccgcgcaacgcgcacccgatggccgtgctcgcgtcctcggtgaacattctctcggcgtactaccaggaccagctcaacccgctcgacgaggagcagctggacaaggcgaccgtgcgcctgatggcaaaggtgccgatgctggccgcgtacgcctaccgtgcgtcgcgcggtaagccgtacatgtacccggacaactcgctcaacccgcgtgagaacttcatgcgcatgatgttcggttacccgaccgaggactacgagatcgacccgatcctcaccaacgcgctggacaagctcctcatcctgcacgccgaccacgagcagaactgctccacctccaccgtgcgcatgatcgcgtcggcgcaggccaacatgtttgttgccatcgccggtggcatcaacgcccttgcgggcccgctgcacggcggcgcaaaccaggccgtgctcgagatgctcgaggacatcaagaacaaccacgacggcgacgccaccgacttcatgaatcgcgtgaagaacaaggagaagggcgtccgcctgatgggcttcggccaccgcgtgtacaagaactacgacccgcgcgctgccattgtgaaggagaccgcgcacgaggtgctcgagcacctcggtggcgacgagctgttggatctcgcgatgaagctcgaggagatcgcgctgaacgacgagtacttcatccagcgcaagctgtacccgaacgtggacttctacaccggcctgatttaccgcgcgatgggcttcccgacggacttcttcaccgtcctgttcgccatcggccgcctgccgggctggatcgcccagtaccgcgagcagctggagatgaactccaagatcaaccgcccgcgccagatctacaccggctacgagcagcgcccgttcgtgccgaaggaccagcgctagccgcgcgcttatagcgtgtaagaagcgctgacagcgcgataaccgccggttcacggcattcccctataattttggggaagtccgtgtcggcggtttttctatgccgccgagtcaacgaacaaggagaaattgagcaatggaaaagcccatcattgaggtaccgcaggaaccggcgccgatggatcttgtcatcgaggatctggtggtcggcgacggcgcagaggctgtcgcaggcgggcacgtcaaggtggagtacctcggagtcacctacgactccggcaacgagttcgactccacctgggaccgcggcgaggccgcagagttcccgcttgctggcctgatcgagggctggcaggaaggcatccccggcatgcgcgtcggcggccgccgcaagctcaccatcccgccggagaaggcgtacggccccgccggcggcggccacccgctcgccggccgcacgctggtctttgtcatcgacctgctcgaagcgaactagggagcacttatgcgagtccccgtgaccaccctgaacgacgggtacgacttccccctcctcggccttggcacgtacaagcttcaaggtgacgaggtggaaaaggtggttcgcaccgcgatcgagctgggctaccgccacatcgacaccgccaaggtctacgacaacgaggtcgaagttggcaaggcgatcaacgccgccattgcggcaggcgacgtgacacgcgaggagctgttcatcaccaccaagctgtggaacgacgaccagtcccgcgctgcggaggcgtaccaggagtctctgaaacgtctggatctggatttcatcgacctctacctggtgcactggccggtgccgcagcaggggacctacgtccaggcgttcgagcagatcgtgcagcttcagggcatgggccagctgcagtcggtgggtgtggcgaacttctacgaggagcttttggacgagcttgcggctgccacaggtgtgaccccggtgctgaaccaggtggagctgcacgctgggttcacccagcccgagttgcgccagtatcacgccgaccacgacatcgtgacggaagcgtgggcaccgctcgcgcgcggcgagaatttcgacgcgcccgagatcgtcgcggtggctgaccgccacggcaagactccggcgcaggtcgtgctcgcgtacctgcttcagatggggtgctcggtggtgccgaagacctccaacccgcagcgtctggttgagaacatcggcgcgctcgaggtcgaactcaccgacgaggatatcgccacgctcgaccaggtgcagggaggcaggatgtcgggggatcctcggacgttcccgaactaagtcattgaggcgtttgcgcctcgcggaaggaaacagggcagttgcttggcgacgtgccctgtttttctattgccccatccgattatcaacgcgtcgggggtgaggtagtacctattaatgtgccagttcagggcgggtgacgggggtaacaatccgggcttcgcaaagccccaaacgccgaacgctgctgccgcttgtgtgttgtaggttacattttgcttcaagcgttgcagatccaacaggattctcgcgcagtgattgacttcttcgacttagaaaggatgagcctgtggccggatcaacagccatcacgggccgccgcgaacccacgcctgaggaattcgtggcgatgcagcaaagccccgaattccaagaactacgtggcaccttccgcggtttcacgtttcccgtgatgatcggcgctttcatctggtacgtgtgctacgtggtcgtcgccacgttcgcaccaggattcatgggccggcccttttggggcctcaacgtcggcctctggttaggcctggcgcagttcatcaccaccttcgctatcacgtggatctacgtgaagtgggcgaacaagaacatcgagccgcgtgcggcgcacatccgtgaagagatggagggctaagcaatgcacacgacaaccctcgccgcagcccagtctgaggcagccggcaacccgatcctcaacatcgccatcttcggtatcttcatcgtggtgaccctgtacgtggtcacccgcgccggtaagaccaccggggagtccgctgacttctacaccggtggcgcgtcgttcagcggcacgcagaacggccttgccatcgctggcgactacctgtctgccgcgtccttcttgggcatcgtcggctcgatcgcgctcagcggttacgacggcttcctgtactccatcggcttctttgtggcgtggctcgtggcgctgttgctggttgctgagccgcttcgaaatgtcggacgcttcaccatggcggacgtgctctccttccgcttgaagcaaaagccggtacgcgtcgccgccgccttcggcacgctgttcgtttcgctgttctacctcattgcccagatggccggtgctggctccctggtgagtgtgttgctcaacctgcactcgttcacctcccaggctatctgcgtggcaatcgtcggcgtgatcatgatcatctacgttctcgtcggcggcatgaagggcaccacctacgtccagatgatcaaggcggtcctgctcatcgccggtgtggcaatcatggccgtgctcgtcttcgttaacatccgcggcggcatgaacaccctgttcgattccgccatcgccacccacgcggcgtcccaaactgccgcagacaagggctacgacccggcggcgatcatggagccgggtctgaagtacggcggcaccttgacaaagcagctggacttcatttccctaggccttgcgctcgtcctcggtaccgcgggtctgccacacgtgctgatgcgcttctacaccgtgccgacggcgaaggaagcccgcaagtccgtgacctgggccatcgtgcttatcggttccttctacctgctcaccctgattctcggctacgcggccggcgctctcgtcggcccggaccgcatcctcgccgcacccggcggcgcgaactccgctgctccgctgcttgcgttcgagctcggcggctccatcttcatggcgctgatctccgcagttgcgttcgccactgtgctcgccgtggtcgccggcctggcgattaccgcctcggcgtccatcgcccacgacgtctacgacgccgtgttccgcgacggccagtccactgaagaggagcaggtccgcgtctcccgcatcaccgtggtcgtcctcggcatcgtgtccatcatcctcggcatcctcgctatgacccagaacgtggccttcctggtctccctggcattcgccatcgcggcgtccgcgaacctgccgaccatcctgtactccctgtactggaagcgtttcaacaccaccggtgctgtggcctcgatctatacgggcctgatctcagcgctgcttttgatcttcttctccccggcagtgtccggttctccgaccgcaatgttcccgaacgcggactgggcgctgttcccgctgaccaacccgggtatcgtctcgatcccgcttggtttcctcgccggcattgtgggcaccttcctaggcaagccggacaacttcgacgagctgcaggccgagatggaggttcgctcgctgaccggtgtcggcgtcgaggctccggtcgaccactaacacccgcgagcggccactcggcctcaccgcgacagaagcgcggagggagggttcgaaccctccctccgcgttcgtgctgtgtcggcggagtcgcacccactacggcagcagcttgctccaatccgccttggaggagagctcgctgctggttgcgatgaggtcggccaattgggccgccttctcctgctgcgggcggttcagattcagctgcggcagcgatggcgcggtcggcttcgcggctccgcccggcacccactggccccagtcggacgcgtagacgttgttgacgtccacctgcacgccgtcgattaccgcagtccacttcgccttctggtggatggtggtgcgcgggtgaattttgccgccggagccccagtcgtgctgccagaagaaggaaccgatgccgtcctcgatgcaccactggatcacgttgtagttgccgtacacgccggtctggtacccggcgacggtgagcgcagcctggaacgccttgaggtacgggcgaatctggtgcgtgtagtggtcgcggtgcgggttgtcgtcgatcgccacgtagatcggccgcccagtcggtccgccggcggccttgtgcaggcggattgcctcgggcgcgtgccgcgctgcagaggctgcgccgccgagccagtcggcagtttcggcgcggccgaattggtaaaccgaggccgtcgctaagccgtttgcggcgtaatcgcgggtttcgcccagcgacaccggcttgcccagcatccagttcgcgccggggcggcgctccgagacgtagcgcaccgcacccatgtggccggcggctttcactgcgcgggctgatggcacgccggctgaatagtcgacaaccgtgccaaggacccgtccctgcgctgcggcgggggagggggcagcaaagccgaacgtggcggcggcggtcgcgatgccggctgttttcaggaaggagcggcgagaaactttagtcacatcagtaacaataggcccagaagggggcttcaatcacgctgacacggctacaggcccagggttacgaacctcgtgtgccccgccatagcctccagcgcctgctccacgccggcggccgtctctgagtgcgggtggttcatgtgcatcagcacgacagcaccgtctggcgcgtgctggatttgctgcgctacctgaaaagccccggctgaagcgccgaagtcgccgttgacgctgaaccccgcaacccgcatgcccgcgtcgttcgcgatccgcaccgccacatcgtcgtagtgcgcggtacctgcccgaaaccaggtcgaacgaaccccgaaacgctcaagtgcagtggcgttaccggcgatctcctcgatggcttcggcggcgttcgcggtgccgtggatgccgtacgccgcatgcccgctcaccgagagcggaacgtggcgggtgccgtggttctcaagttggaagaggggatcagccgcgagctcgcgagtcaggtctggatgcgcatcaatccacggtttcgcgagaaacagcgtcgccggcacgccatgggagcgaagcatctcgatcaggtgcgcgtcgtaatccccgccgcacgcgtcgaacgtcagggccaccgtgcgctggcccggcaccgtcggcaccgaatccacaatgccgtcgaggtgcgtgccgaaatcgcttgggctcatctcgtcgtacgcgtgcgggggcagcatgcttgccgacgcccccgtcgtccccggaagcgcagtcacctcggtgacctcagccgtttcggtgacctcactcagagctgatgaggtctccggggtaggagcgggcggttttgacccgcacccggcgactccagccgcggcgagcaggctcgcgccgaggaaagcgcggcgggttaacggagacggcatgcgttagcagtgtagtttcctcgagacggtgttgcacaagggtagtaccttgatcgctatgcagaacaccacgcagcgcctcatcgtgcctgacctcgcccgcggcatggcccttctaggcatcgccatggccaacgccgcgcaggcgtggattatcaacgactggtccgaagacagctcccgcgccgggtggtccgtcggcggcgtgcgaccggacgacctcctcgaccagatctgcgccgtcttcgccgcgatgttcgtccacgtccgcgggttgccgatgttcaacacgctcctcggtttcggctttggcttggttgtggccagcctgtttaggaagggctacacccacaaagaggcgcgccgcattctggtgcgccgctacggcatcctcgcgctgttcggtcttttgcacctgtccctgctgttcttcggtgacatcatgctcacgtacggccttgtcggcgtggtcatggcgttcatgctgaaggtctccaccaagtggctgcgccgcatttcgtactgggttctcggcatcttcgcggccttcgctctcttcgctacggcggtgcagtggttcttcgagttcgacccgaccgaagttggtctcatccccaccgcggagctgaccacgttcgctgactacttcagcgcgaacttgcagatggcggtgttcgtcgtgccgtcgctgccgttccaggtggtgcagcttgcggcgctgtcaatcctcgggttcgtgtgggcgcaagagggtgtgctcactgacgtcgccgctcaccgcaaaacactcaagacctggatgtggatcgctatcggcatcatcgtgctgatcggattgccgtgggggctgaccgcggcaggggtgctgccgtcgaacctggagaccaccttctacctgctgaaccaggcgctgggcctctacaccggcccgggtattctcgccgcgttcgcgctcgccaccgacaacctgcacaacgaggtgccgggctgggcgcgcgccttcgtcgcactgggcaagcgctcgatgtcgggctacctcgcgcagtcgttcctcttcatcctgctggtcgtcccggcgtttctgggcatcggcaacgacgccagcgtgagcggcaagatcgggatcggcatcttggtctggttgatcacgctgctgctcgcggtcgcgcttgaggccgccggcaagcaggggccgtttgagtgggcgcaccgccacctttcctacggcaaaaccggccgcatcgaaccgaaacgcgaaaaccccaggttagaggggtaaaaaattggggacagtcgagtaatccctagcccattcactccacaactgccccagctgagcttcctctcgccatttctgagtattcctcacactgcctctgcccgaaatgggatggttccgtcaagacaaaagtttcttgatgccctcggagaggatttcttgtgggcttatgtggtgcgccacgtggaggcgcgcataagtcggggcttgttcggggtcgatggcaacacgcttttcgtcgggtgccatgggggccgtcagggcggcgccgatcacaaggtttgatagccggtaggcagttcccaacggatccgggacgccctctcgttcaagcaggacacacatgcgctcagaaagcgccaggtaagcagggcctctgggggcgcgcatgccgatgacctgaccagcccaccggtgggtcgtgaggtgcgtgaagaaagcttgcatcagggtgggcaggtcggcgttgctgatcgactcggacattgcgggatcatctgcaagcgctgtatctagggcgaggtcgaataggtcgtcaaccgactccacgcgggagtacaggctagctggggcgacgcccacctgttgcgccacagccctcatagtgagcgccttcaagccaccttcgtccaacagtctgcccgatgctcttgcaacttccgcaatatccacggcgcgatggcgttgcaccggtttccgatgttcccagtagctcaccccgccagcctaaccaaacatccttgaaccacctatccaaactatgttagttttgggcgcatgctggatgccgccaaccttccgatcacctttgagaacactcgcctacgccctctcgccgaactggacgcagacgcgtatgcagcaggcacaaaagacgaagctgtgcggcgcttcgctcacctgcctgaacctgattacacccccgagtccgtgcgacggatgatctgtgacgaggtcgcgacgggcctctcgtccggcacgttggcagtcctcgcacttgccgacgccgaaaccaaccggttcgtgggttccatggttctctttgacgttagctccgatgctgccgaggttgggttctggattcatcccggtgcgcgaggggaaggacatgcccgtcggggcttggagctggcatcacgcttcgcgcgcaccagtggacttaaaaccttgacggcacgcacgcttccggaaaacagggcctcccagcactgcttgacgacggcgggattccacgagaccggccgaggcgtagggaccacgcccgcaggacagcgcgaagagttgttccactaccagcgcgatctcgtgaccgtcgcccagtggccgttggtgacagaacgacttcgactccgtctgcatgagacagacgatgtcgcatggcttcacgagctgtactcgcaacctgacgttgctcgttacctgttggacgaaccatggactgtggaagttacccgtgacaagctcgcggagcggctatcaaaaactgaccttgatggtgaggctgctgcacttgcactagtcatcgagcatgacggcacccccataggagacgtcgcactgtggctcacagacagggagcaccgccagggcgagatcgggtgggttctgaacccggcacacggtgggcaaggattcgcaagcgaagccgttcgcgcggtacttgccctcgggtttgaccattaccatctccaccgcatcaccgcgcagatggatgcccgcaacggcgcctccgcggcacttgctaaccgcgttggactccggctcgaagcgcatcacgtccaggactggttcagcaagggcgaatggaccgacacccttatctacgcgcgactcgcctccgagacccatagccaataaatgatgtctgatttgaaatgagcagcggctggacgctattagcggatagcgaactctagttgcgttttcaggcacaggtctcggacgacagtccgcgtatatcaggaaatgcctcgcctacttttgcaggaagaggcattgtttcatgctttcgggggttgttcgaacaatcaaatctaattcttcgaaaccccgaattgaattgcgccccaggtaggaatcgaacctacgacaccttctttaggagagaagtgctctatccactgagctactggggcaacggcgataaggctaccgcagcaacctgcgggccttgaaattcgcccgagtggtttacacttcctcgccggtgagctcgcgaagcttcgcacggactgcggaggcctccgggttcgtttcgtgcgtgccgtcggagtacagcacggtcggcacgactcggttgccgccgttgacgctctctacccacgcggcggcgtcctcgttgccgtcagcctcgacgtcgacgacgtcgtagggtgtctccgtgcggtcaagacgctcgcgcagcttgcggcagaacgggcaccacgaggtggcgaagatagtcacgtgggacgaagtttcaggggtggtcatagcttcctttctggtggctagcgccgctcgaggcgctggaatttgtagcgcagcccgttctcggatgtcagccagtcgccgtcgcggacgagttcgaactcgtcgccgaagcgaggtgcgaagacgggggtgtcgatggggagaacgtggacgtcgataagcgtgcgctcaatcacgtcaacctcgtccagcgtggcctcgtacagctggccaccgccgatgatccacgcgtcggtttcaaggtccggcaggtcggtggacacgtaggcgccgttggaccacgtgcccggctggcgcgacgacaggacgtggttggtgcggcccggaagcgggcgcttaggcagcgcttcccacgtgcgacgacccatgatgatggggtgccccatggtggtgtccttgaagtgtttcaggtcctccggcaggtgccacggcatcgtctcgccatcaccgatcacgccgtcgacgctctgcgcccaaattgctccaagtgttggcattacacggacaccttcgcgctaatcgtcgggtgcgggtcgtagccttcgacctcgatgtcgtcgaaggtgtagtcgaagatcgacgccgctttgcgcagcttgagttgcggataagggcgtgcctcccgggagagctgctcctcaacctgatcaacgtggttgttgtaaatgtggcagtcgccgcccgtccagatcagctcgccgacctcaagtcctgcctgctgggcgaacatgtgggttaaaagcgcgtaggaggcgatgttgaacggcacgccgaggaacatgtccgcggagcgctggtagacctgcatcgacagttttccgttggcgacgtagagctggaacagcaggtggcagggcatgagcgccatcttgtccagctcagcgacgttccatgcggagaccaagatgcgacgcgaatcgggattttcggtgaggtctttcatcacctgctcgatctggtcgatgtggccgccgccgggggtcggccacgagcgccactgcacgccgtagaccgggcccagctcgccgttctcatctgcccactcgttccagatgcgaatgccgttgtcttgcagccagcgcacgtttgagtcgccgcgcaggaaccagagcagctcgcctacgacggccttgaagtagacctttttcgtagtcaggagcgggaacgactcggacaagtcgtagcggatctggcggccgaacacgctgcgcgtgccggtgccggtgcggtcgcccttcgcggtgccgttttccagcacgtcgcggagcaggtcctcgtacggggtggggactgacactagtttgagactccttcgtagctgccgtgctgctcaacgtagcgcgcgcaagcggcgagaatgtcatcggccagctcgggacggcaaatcagaagatccgggatataggtgtcggcgttgttgtagcgcagctcggaaccgtcgaggcgggagcagtgcaggcccgcggccatagacacgcccaccggcgcggcctggtcccactcgtattggccgccggcgtgaacgtatgcgtcgtaatcgccgaggagcacgtgcatggccttcgctcccgcggagcccacctgggccacctcgaaacccagctcgcctgcaacgtgctgcgcgattgcgggcgggcggttgcggctcattgcgatctttcccgcgaacgggccggagacgtggcgcacgtcggacgatttgaaaaccacgccgagatccggcaagccgacggcggcgtgggtgggcaccccgtcttcaaccagcgccacgtgcacggcccagtcttggcggccggtggcgaactccttggtgccgtcgagcgggtcgacgatccacacgcggcggttctcaaggcgcgctgggtcgtccgcggcctcttcggacagcacggcgtctccggggcggtgttgttcgagcacgcgggcgatccagttctgggcgaggtcgtctcccgcctcaccgagctcgcggccgcggagcaggccgacgccgcggatgcctttcaggatctcgccggtgccctgcgcgatcagattggtcagcctggaatccgagtactgggcgctcataggctttaagtttagccggtctgccgagtttcggggctgggctgcaggttggcggggtgcgtctgcccggagcaaccggaggcggcagcgtgcctgcagtgggcctgcagcgtgccgactacccgctgccgtagcggcgttccaagatgctgcttgaagagtgttgcttgcagatggtcattaaccgccgtcgcggaaatcgggctggggccggttactcggttaatgaccatctgcaagcaacactttgggggtgaccatgtgcgtccgtccggggtaactggggttttgccggcacaccggccgtcgccctcccacacgtggcacgtgaagtggcaagctccctagaagcttccatcgaaccccgccgcggtaggatcctcgccatgtccgacaacgtgctcgcccgcttccacccgcaggtggcgacgtggttcgaggaggttttttccgcgcccaccgcggtgcaagaccaagcgtggcgctcgatctcggcgggggagaacaccctcgttgtcgctccaaccggctccggcaagacgctggcggcgtttctgtggtctttgaactcgttggttgagcgctccgggcagcaggcgctgccgatcagcgggggcgagaaatccacgcacggcggcacccgcgtcctctacatctcgccgctcaaagcgctcggtgtggatgttgagaacaacctgcgagcgccgctcgccggcatcgcgcgcgtggctctgcggatggacaagcagatgccggacatctccgtcggtgtgcgctccggcgacaccccccaggcggagcgcaaccgccagctgcgcaaaccgccagacatcctgatcaccacgccggaatcgctctacctcatgctcacctcaaaggcggcggggatcctcaaaaccgtggacacggtgatcgtggacgaaatccacgcgctcgcgggcacgaagcgcggcgttcacttggcgctgtcgctggaacggctcgagcgccttgcggggaagttccagcgcatcggtctttccgccacggtgcggccgatggaaacagtggcgaacttcctaggcccgcgaaccacgatcatcaacccgcccgcggagaagaagtgggagcttgacgtccgggtcccggtggacgacatgagcgacctgccggttccggaggacgcatccaccatcggcgaggcggtcgtggacgaccagctgggcttcggcggcgagccgaccgaaacgttcagcggggcgcaccagagcatctggccgcacattgagcgcgcggtgtacgacgaggtgatggcgcaccgctcgaccatcgtgttcgtgaactccaggcgcgccgcagagcggctcaccagccagctcaacgagctgtgggccaaggagcacaccccggagtcgctgagcgcgccgacgcggcgcccgcccgcgcaactgatgaaatccgtcgacaccgctggccacgcggcgccggtgattgcgcgcgcccaccacggcagcgtgtcgaaggaggagcggctccagaccgagaccatgctgaaagaaggctcgctgaaggccgtgatctccacttcctccctggagctgggtatcgacatgggtgcggtcgatctggtcatccaggtggaatcgccgccgagcgtcgcctctggcttgcagcgcgtcggccgcgccgggcactccgtcggcgcggtctctgagggcattttttaccccaagcaccgctccgaccttgtccaggccgcggtgaccgtcccgcggatgcgagaggggctgatcgaggagctcaagccgccgcgcagcccgctcgacgtgctcgcccagcaaacggtggcggcggtcgcgttcgaggacttgaacgtggacgagtggtacgacacggtgcgcaaagcctggccctaccgcgacctcgctcgcgacgtgttcgactcggtgatcgacctggttaccggcgtgtacccgtccacggacttcgcggaactgcgtccccgcgcgatcctggagggttccatactcaaagcccgtcccggcgcgcaacgagtcgcggtgaccaacgccggcacgatcccggaccgcggcatgttcggggtgttcctggtcggttccgacgcggagggcggcgtgcccagaagggtcggtgagctggatgaggagatggtgtacgagtcgcgggtcggcgacgtgttcacgctcggcgcgtccagctggcggattgaaaacatcacgcgcgaccaggtgcaggtctccccggcgcccgggcatacgggccgtctgccgttttggactggtgacgggttgggtcggccgtatgagttggggaaggcggttggggcgtttcgtcgacaagcaaaaagctccctggacccttccttggaccagcgggcgcgcagcaacctcctgcaatacctcgaggagcaggaggaagccaccggcatactgcccgacgacacgacactggtgctcgagcgcttcaccgacgagctgggggactggcgggtggtgctgcacaccccgtttggcaagggggtgaacgccgcgtgggcgctggcgacggggtggcgtgtgagccaggagaccgggatggacgcgcaggcggtcgcgggtgacgacggcattgtgctgcggctgccgcagggggagaaggagccggacgggtcgctcttccaattcgacccggacgaaatcgcggacatcgtcaccgagcaggtgggcaactcggcgctgttcgcgtcgcgcttccgcgagtgtgccgcccgcgccctgctcctgccgcgtcgcaacccgggcaagcgcgccccgctgtggcagcagcggcaaagggcagagcagcttttagacgtcgcgcgcaactacccgtctttccccatcattttggagaccgtgcgcgagtgcctgcaggacgtttacgacctgcccgcgctgtccgaggtgatgcgcgacatcgccacccgccgcgtgcgtatcgcggaggtgacaacggaaacaccaagcccgttcgcctcatcgctgctgttcaactacaccggcgcgttcatgtacgagggcgacaccccgctcgcggagaagcgcgccgcggcgctgtcgctggacccgtcgctgttggccaaactcctgggaaccgttgagctgcgggaacttttggatgcggacatcattgccgaggtcgacgcgagcttgcgccgcgtgggccgcgcggaaacaagcgagcagttcgccgacacgctgcgcatcgtgggcccgatcccggtagacgagctttcgctgtatacctccgtgcccttgatctcgctggagcaggcgctggggccggcgcgcatgatgcgggtgcgcatcggcggtcgcgagcacgttgcgcaggtgctggacgccccacttctccgggatgcgttaggcatcccggtcccgcccggcgtccctgcccaagtgcagacgattccggacgcgctggcgcagctggtcagccgctgggtgcgcacgcgcgggccgttcgtcttaagggatttagcggacgcgttcgggttggcggttggcgccgcttattccgcgctgcaaccgttggtggacgcgggcaaggtggtggccgggcgctaccgacagggcgtggacgaagaggagtacgtcgccgcggaggtactgcggatcatccgcacccgttctttggcggctgcgcgcgcccaaacccgaccggtcacccagtcggcgtacgcccgctttttgccggcgtggtcgaacgtggctccgcacggtgttacaccggcgctgcgcggagctgacggcgtgtactccgtgcttgagcagctggccggagtgcggttgccggcttccgcgtgggagtcgcacattctgccctctcgcgtgggcgattactccccggcgcatctggatgagttgaccgcgagtggtgagatcgccatcgtcggcgcgggcaaagctggcgcccgcgacccgtggatcatgcttctgccggccgactacgccgcccagctcatgccgcaggtggacgagccgctgctgagcttgacccagtcgcaggtgatggagaaagtgcgtcgcggcggcggattcctcttccaggatctcctcgagccgaccaccaccaccgaggagctgcgcgaggcgatctgggatctcgtcgaggccgggtttgtggccccggattctttcgcccccgttcgagcgaggttggccggcgggaagacggcgcaccgggcgaagcggaggccgtcaagaagcagggtgcgctcgggccgcacctcgttcgctaccctgactccgcccgacatggtcggccgctggtcgctcaccccgaccccggacgctgacgccacgcgccgctcggtggcgctaggggagtcacttttggaccgctacggtgtggtcacccgaggctcagtcgttgccgaggacattcttggcgggttcgcgctggcctacaaaacgctggccgggttcgaagaatcgggcaaggcgatgcgcggctacctcgtcgaggggctcggtgcgtcgcagttctccacgccagcaaccatcgaccggctgcgcggccaccaagattcggacgacgtggtcggctggccgtcgggtgcccgcgacccgctcgtccacgtgctcgccgccaccgatccggcgaacccgtacggtgccgcgctaccgtggccaacccagggaccgacccgctccgcgggggcaatggtggtgcttatcgacggcctgctggccgcccacatcacccgcggcggaaaaactatgaccacattcttcaacgcgtttccagacggtgttggcgacccgatgccgctagttgtcgacgccctggcgcacgccgtgcgcgccgggcggatggagcctgtcggggtggaaaagctcaacggggaacccgcgttcagcctgaagcagtacggcgcgaccgtgacgcacaagggcgtgaagatcggtgcgaaagccactgcgccgccgaagcggcgcggccggagcgtggccgaggcgctcgaagagctggatccagatccgcccgagggcttaagtttcgacgactgatcgaccccaaaagcccccggcatcgcggcgcggttgcgcagggtggttgaaggagacccggacgggtaccctcgcacgcatgcccgaaggtgattccgtctaccagctgtcgaaacgcctccagtggatggccggtcgcgaggtgacccgcacgagcatccaggtcccgcgctacgccaccgtcgacttcaccggcatgacgtgtaagcgggtgtggccctacggtaaacacctcttcatggagttcgcggcgccgggccacgaaccgcaaatcctgcacacccacctcaaaatggagggcacgtggtcgatgcacagggtgggcaccaggtggcgaaagcccgggcatgctgcgcgcgtggtgttgcagcttgacgacgccccccagcccgacatcgaactcgtcggtttttggctcggcctcgtccgcgtgtttccggcccgcgaatatgaggcggagatgggctacctcggccccgacctcttggacccggatttcgacttcgacgaggcggtgcggcggattcaggcccaccccgatctcgaaatcggccgcgcgctgttagaccagcgcaaccttgccggcatcggcaacgagtaccgcgccgagatcaattttctggctgggacgcatccgcgggagaaggtgggggaggtggacgtcggcaagcatgtgctccttgcgcggcgcttgatgtgggcgaacaaggactcccccgtgcgggtgaccaccggggtgaagcgtgcaggggagacgagctacgtctttgggcgcaacaacaagccgtgccggcgctgcggcacgttgatcaagaaggactttctcggcggcgagggagacttggagcgggtgatctggtggtgcccgcagtgccagccggagccttagcagggcgccgacttcaggcaaaacctctatggttgccggtgtcccagacaagctcagacgattggttcgacctcgcggtgtggcttgctgtcgatcatccagagaccaccgacattgctgagcggttacgcagggtggttattatgccttagccggcgcgttcttctcccgcaccgcgcggcggatgaagaacgccacgaacccgaggatgatcagcagcagcaccacgtagatcaccttggagtacgcgtcgacgtagccggtggccttctcccagttatcgccgagcaggtaacccaagtagatcaggatggcgttccaaatgccggagccgagcgtggtccacagaccgaaagtgatgaggttcatcctgtctaggcccgcggggatggaaatcagcgagcggatacccgggatcaaccggccgaagaagatcgatggcttgccgtacttgtggaagaagtccatcgccttatccacgtccgaggccttgaccagccacatccaatcggcgatcctgcgcaggcgctccagcccgagccacgcgcccacgccgtagagcacgtacgcgccgacgaccgagccgagcaccgaccagatgaacacattgagcatgttcaagctgccctgcgcgacagtgaagccggcgagcggcagcaccacctcggaggggatgggcgggaacaggttctccaaaaggatcgcgatgccgacgccgggggcgccgagtgtctccatcaggttgacgatccagtcgatgatgctctgcattgcgccaatcttgccctattcgacatccagcgaccaagtgtgcaccggcgcgccggactcctgattcttcaggtattggcggagcacccgggccagcgcttgccgacgctcccgtgaatctggcctggtgccccctcccacaacgttgagggcgttgagctgccacatcgccccgttctggcgtgtgttcacccggccttcaatgatgccgagggactcgtcgatgcaggcttggtctacgttcagcgcttgcagcccgtcttccgcgatcgcaaggaagtgctcgctgaccagctcggtgacggggagcgtgccgagggtgggccacgtgaggttggcggtcagcccgtgccgggatccttggcgaaagttctcccgcgcgtcgtcgaagcttaaacgcgaccacactgggcgggtttgttcggccagcgttttcacgcaaccgtagaaaaacgcggcgtcggcgacgatgtctttgacggttgggccggcgggtagcagccggttctccagccggatgtgggagagctccccgctgggatcgtagattgggcggttccagcgccagatggtgccgttctgcaagttgaggtagtgcaggccggggttgttgccgtccatcgcttgttttccggcctctgcgcgtccctcgggcagaagcggcgagaagtagcggacgttctcctcgaaaaggtcgaacactgacgtgatccagccgtcgccgaaccagacgcgcgggcgaacgccttggttgatcaactcttgggtgcgcgtgtccatcgcttgcttgaacacggggacgcgggactcgtgccacacccggtagccgagaaacagcggcgagttcgcggacaacgctacctgcacgccggcgatggcctgcgccgcgttccacgcgctcgcgaacatgttcggcgctacttgcaggtgcagctgcatcgaggtgcaggcagactccggcgcgatgctttcgaagtcgtgggcgtagttctcttcgcgccacaggttcatctgcacgagctcgccgcgcgactccatcaccgaattgttgaggccggcgtagcggttctcgggcgtcatccacaccggatcctcgaggaactcggtggtcagcgtgggcaacgagcccaccatggcgacagtggatccggcgtcgcgggcggcgcggcggacgtcgttaagcctttgctctatcccctgttccagcgaagcaagcccgtcacccgcgatggcgagcggcgggtggttgagttcgacgttgaactggcccacctcggattggaactcgtcgcttaaaccttcgagcacggccatgttgtttgggtggggctgcaactggtcgtccacgaggttgagctcgagctcgaggccgatcgtgccgtgcgccacgaactcggcgtcctgcaggtggcggtcgaactcctccagctcctgctcaagctggcggcggtagacagtgcgttggcgcggtgagtagctgtcgcgcgagaccttgtcgcccattagcggtggtgccggtaccaggtgatcagggcgtcggtagatgcgtcgcccgtcgcggcgtcttctttaccttggacggccacggcgagatcgtttgcctgcgtcttgccaagctccacgccccactggtcaaaggagttgatgtcccagaccgcgccctcggtgaacgtgatgtgctcgtagagcgcgatcaacgtgcccagcgcgaacggggtgagttcttctgcgaggatggtggtggtcggacggttgcccggcattgttttgtgggcggcgagctctgtggtgacgccgtcggcctcgacttcctgctgggtcttgccgaaggcgagcaccttggtttgcgcgaagaagttgcccatcaaaaggtcgtgcatggacccggtgccgtccgcggtggggaagtcctgcgctgggcgcgcgaacccgatgaaatcagccgggatcagactcgttccttggtggatgagctggaagaaggcgtgctggccgttggtgcccggctcgccccagaacacttcgccggtgtcgtaggtcacgcgcgtgccgtccctgcgcaccgatttaccgttggactccatggtcagctgctgcaggtacgcggggaagcgggagagatcctcggagtacggcagcacagcgtgtgtctgagcgccgaagaaattgcggtaccagatgttcaaaagccccatcagagcgggaacattctcaccgagcggagcgagacggaaatgctcgtccatggcgtggaacccctcgagcagacgcatgaagtcctcggggccgatcacggccataaggctcagcccgatcgcggagtccatggagtagcgtccgccgacccagtcccagaactcgaacatgttcttcgtgtcgatgccgaaggccgcgaccttctcggcgttggtggacaccgcaacgaagtgcttggccaccgcggcctcgtccccgtcgaagtgctcgagcagccagcgtttggcggcgtgcgcgttggtgagcgtctcttgggtggtgaacgttttggaagcgatgatgaagagcgtctcttccgcgtcgcagcgatccagcaccgcggcgatgtcggcagggtcgatgttggagacgaactccgcggagataccggcggtggcgtaggcgcgcagcgccttcgcggccatcgcggggcccaggtccgacccgccgatgccgatgttgacgatggtggtgatcttgcggcccgtgtggcccttccactcgccggagcgcaatgaggttgcgaaggcgcgcatctgctgcaggaccttgtggacgtccgcggtgacatcttggccgtcgacagtcagctcggcgtcggccggcgcgcgcaaagcggtgtgcaacacggcgcgatcctcggtgttgttgatccgctcgccggcgaacatcgcctcggtgcgacccttcaggtccacttcctccgcgagcgcgacgagggcgtcgagaacatcgtggtcgatgaggttcttcgacaggtcgacccgcagaccggcggcgtcgaaggtgaaatgctccgcgcgtttactgtctgcggcgaagagatcccgcagcgtgacccgcgttttctcggcgtgcagtttctgcaggtttccccaggcggctgtaccggtgatgtccgtcatggctccaacggtagacaacatttacgcataatggcgggcatgagcattgtgaagatcaacgctatttctgttcctgagggacagggtgaggagctggagcgccgcttcgccgcccgcaagcacgcgatcgacgcgcaggcggggttcgagggctttcagctgcttcgccccgtcaagggcgaggagcgctacttcgtggtcacccgctggacagatgaggcgtcctaccaagcctggtgggagggcgaaggccgcgcgggccacgccaagccggcgggggagcgcggcggtgcagaacacgccgcgccggtttccacacgcgcggagctgctcgagttcgaggttgtcctcgactctctggaggaagaccgctaagcctgggccttcagcgcctcgaccacagcctcgccgacgccggtggcgctcatcgggttctgcccggtgatcagcttgccgtctaccaccacgtgcttggtcatcgggatgcgggcggttatgtattccgcagcgtctgccgacaggcgctcttccaggctgaatgggacttcgtcggcgcggcgggcgagtttttcctccgcccaggagtagccggtgaccttgcggccgcgcagcagctcggtgccgtcagccgtgcgaacgcccaagagaccaaccgggccgtggcagacggcggagacaatcttttccgcgtcggcgaagtaggcgacggcgttgttgacctcgtcggtgaggaagtcgaacatcgtcccgtggccgccgatcaagaagatacctgcgtaagcctcgaggtcgacatcggcaatggcgggggagtcgtcgagctgcgacatgaactcggggtcttggtagcgcttgttggtcccgcctagctggatcacgggcggctgcaggctcaccgggtcaacagggatcaccccgccgcgcacgctggcgaggtccacctcgtggccggcatctgtcactgcgtcgaagaagtgggtgtactcgcccagccacacgccggtgcgcaaaccggacgtttcgtaacggtgggcggaggtggaaagcgccagaagtttcatgccccttttctacaccgggaagcagtgcgggcggcgggcttagccgagtttgccgcggcccaagcggagcagaatctgggcgaggcccggtccttcttcccccagctcgtcccggaactggttgatgatcgccacttcgcgggtgtgcaccagcttggtgccgccggagcccatccgggtcttgccgatggcttgggagatctccgtgcggcgcttcaccgcgtcgaggataacgcggtcgaggcggtcgatctccttgcggtattcctggatctccgcatccgacaacgggtcatcggtaccggacggcaggcggatctcaggcttagtcataaacgacaattatgccaccgcctccgggccgcgttcgaacattcgaaaaccgcgttcgggcgtgttggtgtcggtaggtagggtttagcccatgacccagcaaaccgatctgaccctaggactcaacccgcagcagcaggcggccgtcacgcaccagggcggcccgctgctcattgtcgccggcgccggatcgggaaagaccgctgtgctgacccgccgtattgcgcacctgctgcgggaccgaggggtcgccccctggcaaattctggccatcaccttcaccaacaaggctgcggcggagatgcgcgaacgtgtgtcccacctcgtcgggcccgaagccgagagcatgtgggtggccacattccactctgtgtgcgtgcgcatcctgcgccagcaggcgcagctagtgcctgggctcaacaccaacttcaccatctacgactcggacgattcccgccgcctgctcggcatgattgcgaaggatttcggcctcgacttaaagaagttcacgccgcgcacgctggcgaacgcgatctccaacttaaaaaacgagctggtcggcccagaggaggcgcaggcccaggcgcagcagacgcacaacccgttcgagaccacggtggcgaaggtgtacgccgagtaccagcggcggctgcgccagtccaacgcgctcgacttcgacgacttgatcggagaagtggtgcgaatcttccgggagcacccggaggtgaccgactactaccgccgacgcttccgccacgtgctggtggatgagtaccaagacaccaaccacgcgcagtacgagctgatccacacactggtgggcaacggttccgacgcgccggagttagctgtggtgggcgactcggaccagtcgatctacgccttccgcggggcgacgatccgcaacatcgaggagttcgagcgcgactacccgaacgcgaccacggtggtgctggagcagaactaccgctcgactcagaacatcctgaacgccgcgaacgccgtgatcagccagaacgaggggcggaggccgaaaaagctgtggaccgcccacggcgagggcgaaaagatcgtcggctacgtcgcggacaatgagcacgacgaggcgaggttcatcgcctcggaaatcgacgcgctgtctgaccagggaatgaagtactccgacatggcgatcatgtaccgcaccaacaacgcctcgcgcgcgatggaggacatcttcatccgttccggcatcccgtaccgggtggtcggcggcacgcggttctacgagcgccgcgagattcgcgacatcatcgcctacctcaaggtgttcgagaaccccgacgatacggtgagtctgcgccgcatcgttaacgtgccgaaacgggcgatcggcgacaaggcgcaggcgatggttgcgctgcacgcggaaaacaacaaccagagcttcgggcgctcgcttgtcgacgcggcggagggccgtgtcgacatgctgagctcgcgctcggtcaacgcgatttcggccttcgtggacctgatgcgcggcattgcgaacgacatcccgtcgatggtcagcgagggcaccggcgtgacagatctgggccagttggtcacccgcgttctggaggacaccggctacaaggctgagctcgaggcctccaacgacccgcaggacgcggcgcgcctggacaacctcaacgagctggtctcggtcgcccgcgagttttcgtcggaagcggcgaaccagttggcgtacatgacccaggacgagctggacgaggtcatgcaggaaggtgagcccgcgccgggctcgctccaggcgtttttggagaaggtgtcgctcgtggcggacgcggaccagctgcccgacaacgaccaaggcgtggtcacgatgatgacgctgcacaccgcgaaggggctggagttcccggtcgtcttcgtgaccggctgggaggacgggcagttcccgcacctgagatcgctgggggacccgaacgagctcgcggaggagcgccggctcgcgtacgtcggcatcacccgagcgcgggagcggctctacctgactcgggccatgctgcgggcgtcgtggggtgcgccggtgaccaaccccgccagccgctttctcgctgaggtccctgcggacctcgttgactggcgccgggtggaaccggagcccacctacaactcgagcgcgtggggcagcccttcgccggtgtcggcacgggccaagcggccgcgccgcggtatcgcgggcgacatgaaggtgaacaagcaactcgacttggcgccgggcgatcgcgtcaaccacgccaagtatggccttggcacggtgctgaccgttgagggcagtggcgtgcgggagaccgtcaccgtggatttcggctcctccggcacggtgcgcctcatgctcatcggcggagtgccgatggagaagctctaggcagcgcggcgctagatggtgatgccctgcgccttgaaccacggcacggggtcaacctgcttctggccgtcgggcttgatttcgaagtggaggtgcgggccggtggactggccctcgttgccgattttcgcgatctgctcgccggctttcacccgctggcccacgctgacgttgtagtcgcgcatgtgcccgtagacggacacctcgccgccgtcatgcttgatcaccacccagttgccgaagccttgggcggggcccgcgttgatcacggtgccgtccatcaccgcgtagatcggggtaccgaggttgttggcgatgtcgatgccgttgtggatgcgtccccagcgcgggccgtagccggaggtgaagcggccgactgccggggtgaccacctttcggccgtcggctgtgcggccggtttggaagcggacggagttgtcgctggtctccggcgcgaaggcggaactgatttcctcgcccaacgaacgcgggtcgtagacaacctggtagccggcgtagctcagcgtcgccccggacttcgccacggtggtcgcggcgccgacgagtgcgcgaaccgcatcctggctgtccttgatcggggcgccgttgaggtggacggacagcgcgtgggcgggcgccggcgcacacacggtgagcgcgagagccgccgccaccgcggcggcgagggtgttgcggttcgttttcatgcgggcagaagcacctttacgttcgttgggcataccgggataaaacttagtggtgggggcgtcgttaagcaatgctctgacatgcggttttgtcgaatgactgtttcaatccgccgggttttgccagctcaaagggctgttacggatgtgaaaattgttgcagatgttatttgcggcgcgtgaccaatcgggggcaaaacgaaaacccgccacacgaacgcgtgacgggtcggaagggcgtgtttgcgctagagcgaaatgccgcgggccgcgagccacggcaccgggtcgaccgggttcgtgccgtccgggtgaatctcgaagtgcaggtgcgtgccggtggagaagcccatgttgcccatgccggcgatctgctggcccgcggtcacgcggtcgccgacggcgacgttgagggattgcatgtggccgtacacggaaacggcgccgtcgttgtggaggatgcggatccagttgccgtagccctgcgccgggccggaatcgatgaccgtgccgtcctgcaccgcgaggattggggtgccgttgacgttggcgatgtcgatgccgttgtgcatcgtgccccagcgggggccgaagccggaggtgaacgcgccgagcgccggcttgaccacctcgggcaggcgggcggccaggtcggccttggctacctcggcggagtgctcgacggccttggagagctgctcggtcaggttgtcaatcggcttgtactccgggatggccaagatctgcggcgcggcagtggcctcggacaccttcgcggccgcgtcctggaccgcctcgagcttgtccacgttggctgcgagcttgatctcgacgctctggttcgcggagtccttgcccgggatcaggtcggctgcagtcgcgcccgagaggctagcggtagagacagcgccggtggtgacggcgacaatggccacgcgacccttgttcgggctctgcttgcggtgcttgccaccggtgttcgacgacttgaacatgctgcctcttcgttaagatccgtcggccccgggtggttgctgcggcagtcaaccgtgacctttccgttatctagacgaggtaactgtaacgaataggtttcgggacagcaacccacttcgccaacaaaggtctgtcgggaaatagtaaggaaacgttacagggcccctcaagtcacacgcttatcacgggcaccatccgttcgcggtgcgcggcagagtgtctatcggcctgctaccccaaccggggtggcagagtaaacgtcgatgagtacaaacaacgcaccccggtccaccgcgccgcgcagggacgacgccacagcgccgaaggccaccgcgcgccgcaaaccggtgaaggctacggtgtcctccaactcgcggcccgcagacgcgccgcaggccccgaccacgtggggacagcgcatgcgcggcttcatcccgacggccgcggcgccgctgctcatcacagcgctggcggtcgtggcgatctgcttcgctgtcatcctgatcagcggttggcgcctggcatacctgccggcagccatcgggcagacgtggctcacggtcaacggtgcgccgctcagcatcgacggggtagaagtagccaacgtcccgctgttgcccaccatcggtatcgtcgcgctgattgcagcccgcatccgcgccgcggcaagaaggaaggtcagcgtgcgcgacatcggcgcaatacttgcggttctcgcgctgacctcgctcacgctgagcgtgattgcgctgttcatggtcaccgacgcggccaacgtgttcgcgatcgacccgccgaacccagccgcggcgttgctcgcgccccttgttgcgcacctagccggattcgccatcggtgtgggccccaaggtatggcgggcgctcgcgcgccacggcggtgtgccggaggaggcggcggtggccgctgcggcagcgtttcggtttgttgtcgcgcttctcgcgtgcgggcttgcggtgtacgtcgtgctccttggggcaaacgtcgccggcatccgcgcgtcgctcgacgcgtacccgaatctgggcaccggcggacggatcgcgctgtggctgatttgcctcgggtacctcccgaacgcggccgtcgcaacgctcgctgtcctactgggcggcagcttcgactacgcggcggcgtccgtctccctcttcgacgcgaccgctgtgcccgcccctccgctgccgctgttcgccgcggtgccctccgcggttccggcgtgggccccagcgctcatgctgatcccggcagcggtggtggtgcgcttcgtgttgaaggagcagggtttgcttatcgacgccctgtccaccgccacttgggccgccctcttcggagcgttcgtcggggtgtatgcggccggtgctgtgggcgcctacggcgtcgtcggggccaacccgtggacgcttgcgctcaccctgtttgtgtgggcttctgtagcgggccttgccggctggctccttgcgcgtgtgcggggggactagactagcccaccgtgagtgtggacgtagtggtactcgtgtccggatcgggcaccctcttgcaagccatcctggacaaccaggacgataattaccgggtcaacctggtcgtcgcggacaagcagtgccccgcgctcgagcgggccgaaaacgctggagtgcgcactatggttgtgcctatggaggcagaccgcggcgagtggaaccgcaagctcgcggccgcggttggctcggccgactgcgacgtggtggtctccgccgggttcatgcggattctcgggccggagttcttggccgtgtacgaaggccgcaccatcaatactcacccctccctcctgccagcgttcccgggcgcgaacgcggtcggtgacgcgctggcgtacggcgtgaaagtcaccgggtgcaccgtgcactacgttgatgagggcatggacacaggcagaatcatcgcgcagcgggcagtggacgtccgcgacggcgaatcgcaagacgccctccatgaacggatcaagaaggtcgagcgggaacaaattgtggagctacttcaaggaaaggtgacctggtaaatgggtatcgagattaagcgcgcgctaattagcgtctacgacaagaccggtgttgaggagctcgcgcaggccctcggcgccgccggcgtggaaatcgtctccaccggctccaccgcgaagcgcatcgcggacgctggcgtcgccgtgaccgaggtggctgagctcaccggcttccctgaggtgctcgacggccgagtcaagaccctgcacccgcgcgtccactccggcattctcgcggacctgcgcaaggacgaccacgtgagccagcttgaccagcttggcattgagcccttccagctcgtcgtcgttaacctgtaccccttcgaggagaccgtggcttccggcgccgattacgacgagtgcgtcgagcagatcgacatcggcgggccctccatggttcgcgccgccgccaagaaccacccgtcggtggcagtggtgacctcgccggcgcgctacgcggacgtcatcgaggccgtccgcggcaacggtttcgaccttgaccagcgcaaggcactggcacttgaggcattcacccacaccgcgcagtacgacgcggccgtctccacctggctcgccggtcagctggccgccgagattcaggatgctgctgcgccgaccaccgccgaggctcccgcgctgcctgctgacgcgccggcagaaatcccgggtgcgctgcgctacggcgagaacccgcaccaggcggctcgcctagagtcggagggttggggcatcgcggccgctacccagcacggcggcaaggagatgagttacaacaactaccaggacgctgacgccgcgtggcgcgccgcctgggaccacgagcgcccgtgcgtcgccatcatcaagcacgccaacccctgcggcctcgcagtggcggacgagtcgatcgccgaggcccaccgcaaggcccacgcctgcgacccggtgtccgcctacggcggcgtgatcgcctgcaaccgcgaggtgaccctcgagctggctgagcaggtcaagccgatctttaccgaggtcattatcgcgccgtcctacgctccggacgcgcttgcgctgctgcaagagaagaaaaacctccgcatcctcgaggttgcaccggagacccgcggcgaggagcgccgccagatctccggcggctggctcgtccaggagcgcgacacctaccaggcggacggcgatagcgccgtcaactggaagctcgcggccggcgaggccgcagacgaggcaacgctcgcggacctcgagttcgcgtggcggtcggtgcgctgcgtgaagtccaacgcaatcctcatcgccaacgacggcgcctcggtgggcatcggcatgggccaggtcaaccgcgtggactccgcgaagctcgccgtcgaccgtgcgaacaccctcgacggcggcaagaaccgcaccaacggggcggttgctgcgtcggacgcgtttttcccgttcgctgacggtttccagatcctcgcggactccggggtcaccgccgtagtcctgcctggcggctccatccgcgacgaggaagtcatcgccgccgcaaacgaggctggggtgaccatgtatttcaccggcactcgccacttcgcgcactagcgcggcccttcgacagaaagaccctgagcttccgtgtcatctcgtctcaccgcggcgctgctcgccgcgggtatcgcacttccgacggctcctgccgtgtttgaaatccccgtcatcggccccgccatcgtccaggcttacaacgggctgcctccggaactgaaaaaccgcgtccccgagtccgtgcgggcgcagctggtgcctcctgtgaacgccccgggcgccgcaccagcgacgcgggcccacgtagcaccgggagcggtccaagctcagctcgatgcgctggtgcgtgacgtccaggcccgccacggcggccgcgccacggtttcggtcgccggcgcaggtgcgcagttcaccgcgggcgacaaccggcccgagccggcgttttccaccatgaaggtgccgagcggcatcatcgcgctgcgcaacaacccgggcacgtacgccgacgtggaagcgacgatcgtgcgctccgacaaccccgcctcttaccggctcaacgcttctgtgccgggtccgtcgctgaacgacgtgattgccgaggctgggtcgcgcaccaccaacacggccgcgtggcgcatggggacgttgtggaccacgtctgaccaggcgcagttcgcctccggccttcgctgtgtcgctggccacgagccggtgctggagatgatggggcggatcatcccggagcagcgttgggggctcggccgcatcccgggcgctaggttcaagggcggttggaacttccacgaggaggggcatcttgcccggcaattcgggttgatcccggggccgaacggcgacatcgccgtggcaatcacggcccacaacccgcgcggctaccagtccagctacgcgatgctgaacgatcttgccgacggcctgtccaacatgaccagccagctcccaacgtcgcgctgctaatgagatacgcgcgcaccgcagcgacgtgccttgcggcgtgcgcgcttgccgcgtgcgcgccgggtgcgggcgagcagacagctacgttgccgccggcgaccacggtcacgtcgacgtcggcggttccgcccgcgcacggggcacctccgctgtccgcagaaccgggcgcggaggaccccgaaacccagttagcgcgcatcgcgcagggagctatagaaatctttggcggcgaggccagcgttgctgtctcgaacacagcgcaaaccctgacttcgggggacgcgcgagactacgtagcatggtccaccatcaagattcccatcgctgtggctgcgctggaggcagacccgagtctcttgcctgtcgccgaggccgcggtcacgatctcagacaacggtgccgccgagacgctgtggtcggcaaccacacctgcggatgtcgaagcggtgctcgccgcggcgggaacaccaatcgctgtcaacgcggagctgacccggccgggattcacgccgttcgggcagacagtcttcacaaccgctgaccaagccgcgttcgctgccggtctcccgtgctcggcggcatcttcacctgtgctggaaatgatggggcggatcaccgcggagcaacgctacgggctcggtctcctcggcggcgcgcagtttaagggtgggtgggggccagacgaatcaggatcgtacgtcgtccggcaacttggcctcgtcgaaggcaggggagtggcgctgaccgcagcacccgctgacggcacgtatgaaacggcgcagcgcatggcgtcgatgatggctgttgacgtcgaaacagtcatacgccagcttccgcccgccagctgttggtagacgggtgtgacggtacgataagcgtgctaaatggtttcacaaatccgaggtagcaatgtccaatccttatgacaaccgcccgaacgagtgggactcacccagctccgctccgagggattacccgcccacgcagcagttcccgcctcagcagcaccaaacgccgtaccaagcctcgccctacgcccagcaggctccgtattcgtacggcgactggcagcccgcggggtggcaggccgaaccagagaagaaaccgaagtctaacgcgccgttgtgggttgcgctcggcgtagctatcgctgccgcgcttggtgcgggcggctacttcgcttaccgggctgttgatgccgggcaggcggagccgattacgtcgacggtcgtggtcacctcgacgtctccggttgcatcggccccggccggcggttcgagcgcgagtgcagcaacccaagcttccgagccgacgcggtcgcgcgccgaagaggagcgtgaggctgcgaagaacaaggaatttgctcccggcaaatctgagacgtcggtgacctcgcccgagttctcggccgttgtcggcgaagacttcgcggcctactatcgccagcacgggcaggcgccggcgacgcttgagtccaaaagcccggtgacagggaagacgtacacgatgacgtgcttcaaggcctctggcggctaccgctgcaccggcggaaacaatgcctctgtcttcatcggcgagcgttaagatccaaacgcgaggcaaaacaaacacccgctctcaaaccctcgtaggaggggagagcgggtgtttgtgctgctgccaaccggtctttagcggctggtgaacggcagaagagccatctcgcgagcgttcttcactgcggtggcgacctgacgctgctgctgcggagtcagaccggtcacgcggcgggaacggatcttgtggcggtcggagatgaaaagacgcagggtctcaacatccttgtagtcgaccgactcaatgcccttcgccttgagcgggttcttcttcgggcggcgggactgctccatgcgagccttgcgctggttgttgttgcgcttcatagttgtgctgcctccttaccacgaagacttacggacgccaggcagctcaccgcggtgagccatctcgcgcatacggacacgggaaacaccgaacttgcggaggtagccgcgggggcggccgtcacgcgagtcgcggttgcgcacgcgaaccggggaggcgtcgcgcggctggcggttgagctcgaactgggcctccagacgatcctcgtcggaggtttccgggttcttgatgatcgccttcagctcgttacggcgttccgcgtagcgagcgacggtctccttgcgctgctcgttcttcgcaatcttggactttttagccatggattatcgctcctcgcggaattcgacgtgcttgcgaacaatcgggtcgtacttcttcagcgtgatgcgatccgggttgttgcgcttgttcttgcgggtgacgtaggtaaaaccggtgcccgcagtggacttcagcttgatgatgggacggatatcgttacgtgccattagatcttctcacctcgcgcgcggatctgtgccacgacggactcgatgccgtcgcggtcgatgatcttcaaacccttcgccgaaacgttcagggtgatggtgcggccctcagagggcaggtaaaacttccgcttctgcacgttggggttccaacggcgcgagtggcggcggtgcgagtgcgagaccgtcttgccgaaagacggcttgcggcccgtaacctggcaatgtgccgacatggttgacttcctttacttctgccgcccacgcaaagattgtcaaaagtaaagcaccgggaacaagcggtgtgagggtccgcgggcggtgcagtgcaatcggttggcgcaggcgtaaacgtgtacttcgacaacagcgagagctaaccatacacgtccgcacctgtatctcctaatttatggcagtctgcgtggcgtcgataagcaaatggccctatcccgccttcttcctgggggatagggccctgcgttgggcggcgaacctgcgctgtttagagctgcttcggctggccgttctgcgccgccagcaggtcgcgaatctcgctgagcagctcctgctcggtcgggtcctcggcctccgggtcgatgcccttgcggcgcttctgcgcctcgtccagcttgttcatcggcgcgacgatgaagaagtagaccacggcggcgatcagcaggaagttgatcacggcggtgagcagtgcaccgaagttgacgaaggtcgcttcgttgcccggcacgatgcgcacgccgaagccggggatgtctgcgccgccgagggaagcgatgagcggattgatgatgttgtccgagaacgcagtgacgaccgcggtgaaggccgcgccgatcacgacaccgactgcgaggtcgatgacgttgccgcgcataatgaagtctttgaagccctggagcatgatttcccttccgaatatgaattttcaagtgtttggatgacggtacgggaatataacagatgtttcgcttcgtgcgattatgacgacaggggcgcggccggtaggatgttgcaggttgtccggcaccagctggatgaaaacgtattttcgcacccaactcaggcacgatccagccacgccgcgacgtggctggaaccgacctgaagttcaatcctgagggagacgaattccactatgaagaacgatattcacccggattaccacccggtgattttccaggacgcgaacacgggccacaagttcctgacgcgttccaccttgacctctgaccgctccgagcagtgggaagacggcaacgagtacccgctcgtcgttgtcgatgtgaccgcagagtcgcacccgttctggaccggcgcacagcgtctcatggataccgctggccgcgttgagaagttcaaccagcgcttcggtggcatggctcgccgcaagaagaagtccgcagagtaacccagagacagcactttaaggaggaagagatatggcaacccccaagttcaagatgtcccgcgcgaacacccgcatgcgccgttcgcagtggaaggctgacaacccggacctggtgtccgtgaagatcgacggccaggaagtgcgcatcccgcgccgcctggtgaaggcagctcaggcaggcctcatcgacgtcgagcagttctagatcaccgctaaccggcgctgcgttatgcgcgcagcttgtgacgcgactgaagttccgggcccgaacaggcccgggacttttttggtgccgcggtaactaaattggctaatcaaatctacgagataccaatattccgttaagatcttgcctatgaaaattttggttgtggacgacgagcaggccgttcgcgagtctctgcgccggtcgctgcgtttcaacggttacgatgtcttgctggccgaagacggggagcaagctttggcgttcattcgccagcaccgaccggatctggtcattctcgacgtcctcatgccgaaactcgacgggctcgccgtctgccgcatcctgcgcgaggaaggcgatcacacgccggtgttgatgctgacggcacgcgacgatgttgcggaccgcgtcgccggcctcgacgctggcgccgacgattatctgcccaaaccgtttgcgctcgaggagctgctcgcgcgggttcgctcgctgctgcgccgcacccgagatttgagcggcggtaacgattcgctcgagcgcgccacgctcgtgttccaggacctcaccataaacacggaaacgcgcgacgtgtaccgcgcatcgcgtcctatcacgttgacccgaaccgagttcgcgttgctgctgctgctcatgcagaacgcccgccgggtgctgaccaggcaacaaattctcgaagaggtgtggggctacgactttccaacgtccggtaacgcgctcgaggtctacatcggctacctgcgccggaaaaccgaggctaacggcgaagaccggttgattcacacggtccgcggggttgggtacgtcttacgggagaacgctccgtgattctccggcagtccgccgacagccttccccgcactcgcggtgcaggggacggagaggtggaggcgcgcacgtccccattcttcggatgggggctttctttgcgtcagcatctcgggttgctgaccacggctatggtggcggtgaccatcttggtctcaggcatggcgggttactgggcgttccgctcggcgctgacaaatgtgctggacagcgagctggtggtggaagctcaaaccctgctcgcggaagtacaggacgtctacatcgaaccagacgaagacgacgagctcgtgatgcgcgagcgcctcgccttattcaaatcgcacaacccgttcacgcgtgtggcggtgtcgccttccggcacgaacgcgttcttcggcgacccggtaccggtcggcgggcagttccgagaccagatcgacggcgggaagctttcgactcggaccctcggcggcgagcggatcattgtctacgtcgggcccgcagaaaacgcagtcgcgctttcacagacgatcgacccctacgggcgcatctccggcagtctcggagcagcgctgttgatcatcgttggcatcggcgcgctgttggcgtgggccgtgggcggtgccgtagtggccgcggggctgcgccccctgcgccgcttgcagcgggctactgacgacgtgacccgcaccggcgagctgaacctattgcctgtcgacggcgatgacatttactcgcaggtcagtgattcgttcaatcagatgatgacgacgctgcaggagtcgcgcacccgccaagcccagctcgtggcggatgcgggccacgagctgaagacgccgctgacgtctatgcgcaccaatatcgagttgctgatgatggcgacctcggcgggcgccgggaaaggcatttcggccgaggaccgcgctgacttggagcgcgacgtgctcgcgcaaatggaggaaatgtcggcgctcatcactgatctggtcgacctggctcgcgaagaggccccgggaacggtgagcgaggagttcagactcgacgaagtgctgcacgaatcgctggagcgggcgcagcggcggcgcacggacgttcagttcagcgtgcggactcagccttggtcgatgcaaggagatcgcgcggcgatgggccgggcgctgatcaacgtcgtcgacaacgcggtgaagtggtcgccggtcgagggtacggtccgcatcacgctgcgcgcaggtggcaagcaagcggtgctgcttgtcgacgactccgggcccggcattccagcatcggagcgggagaaagtgttcgaacgcttctaccgcgcgaccgagacgaggtcgacccccggctcggggctcggcctggcaattacgaagcaggctctcgcgcgccacgaggcaaccgttgtggtggaggattccgacgacggcggcgcccggttccgcatcgcgttgcccgggtggcctccaggggattactccagctcaacccccacagtaaacactcagtaaaccttatgtgtcgtggggacgggggttaagaccaggcacagcgggagagggaacaatgacgcgaatgagcaatccctttcctccgcaggggcagcagggcccggttggcccgtccgacccccattttgagcagcagcagcagcagtttgggcaaccgcagttctatcaaccggcgctgtcgcctgcaccgaaacgggcgcgtgtcctgcccgccatcgcggcgtctgtggtgacctcgctaatcgtgggcggcgcgaccggttaccttgcggggacggtcaacaccgcggcgtcgagccagtacgaggtccgtgaagcgcttgaaaaacccgctgaggaagatgtccaggatgcgcctgaggggtcggtggagcgcgtcgccgctgcggtgctgcccgcggtggtgtctattgaagtcgaaagtgcgcgcgggtcggcggaggggtcgggttcgatcatttcctcggacgggtacgtgctcaccaaccaccacgtgatcgagtcggcggcaagcggtgccgcgcgcctgactgtcacgctcaacgacggctcgcagtaccccgccgcgtttgtcgcttccgacgtcaacaccgatgtcggtgtgatcaagatcgagggcatcgaaggtctgccggtgctcgagtttggaaactccgacaacctaaaggtcgggcagcaggtggtcgccgtcggctctccgctcggcctgtccgctaccgtgaccacaggtatcgtctccgcactcaaccgcccggtccgcgcaggtcagggtgggggagagagctcgcttatggacggtatccagaccgacgcagctatcaatccgggaaactcgggcggtccgctggtggatatgaacggtcgccttgtcggcatgaactcggtgatcgcgtcgctgtccacaggcgggctgtcgggccagtcctccggatcaatcgggctcggcttcgccatcccctccaacttcgcgcagcgagtagctcgccagctcatcgacaaaggcgaagcttcccagccgatgctgggtgtccaagtcgatgtttaccgcagcggcatgcacggggcagtgatcgcgcaagtggagccgggcagccctgctgaagcggccgaacttgcgccgggggagtccatcgtgcgcctcaacgaccggctgatcgactcggcggatgggctcattgccgctacccgttcccgagacttcggggagacggtgacgctggaggttgagggcgcggacggtaggtctcgatcggtagatgtcacgctcagttccgagtaaagtcccacaggaaaacgatctcccggcccgaatagaggaccccaatggcagcaacgcacgacgcgctcgagtacatggaaccggacgacgagtttctgcaggccgcagagctcgaaaacggtaaaccgggtacgccgtgcgcgctcgtcgtcctgatcggtgaccgccgcttcggcgatcccggcgacgacacgcacaaaatggtcacggagctgctcaccgagatcggtttccaggtcgacgcggtggtgcgggcgaagtcgaaaaagtccgagattcgcaaggcgatcgagactggtgtcgtgggcggcgtcgacctggtgctcaccatcggcggcacgggcgtcggcgcgcgggataaggcgccggaggcgacccgcggcgtgatcgacaagatggtgcccggtgtggcgcaggcgctgcgctcctccgggcaggcgtgcggagcggtcgacgcctgcacctcccgtggtatttgcggcgtctccgggcagaccgtggtggtcaacctcgcaccgagccgccaggcgatccgcgacgggctggccacgatcgggccgctggtgcaccaccttatcggtgagctcaacgagcactctgtggactagatatggcagaccagcagcgccgggtacggcgccgcgtccggcgagtttcggacgccgactacgaccgcaccgccgatgcgccggtgactgcagaggccggcgccgacgcggaccgggcggtgcaaatagacgaggacgccgacgagcagcttgccggcatcgagttctatgaagcggagcgcccgccgcaccacggcgggaactaggttacttcaggaccacggtcagcggatcggcgagcgaagccgcagccacagccgcggcttcggattcgcgcaacagcactaggacggtcccttgatcgccgacggttacgatcttgccgccggaagcaatcactctcggcccttggcccacgacatcgactctggcgccgtggtgcagcatcggcagaatgtctggctcggccaagggcagtggcaccatggtgaacggctcccccggcgcttcgccatccacgagctgcgcaactaaatccggtccgacgaggcgggtcgtggtcaccacctctccccgcgaagccccggccgcaagaatgtgcccgaccacgagcgctgggtcgtcgatcgcgttgtcgggaatcgcggcggctggaagcctggccgtggtcacgtcgtcggcagtgaccagcgttcccgcggcaacctcgcgggcgaaggtggtggttaaggggtcggttttgcggacgtcgacaagaaagctcaacgccgcaaccacaacacagcccgcagcgacaatccggcgaatcaaggtggcgcggcggtgaccgggatgggtgaaggcttggaacttcgatatcgcgtccataggtattggacgcgtgctaccgcgcggcggttccctccacaatgaaaaagccggacggcgtgatcaccgcgtcaacgggtgcgtcgagctggccgtgcggcaccttttccgcaacctcgtggtcaaacaccaccgccgcgaccgggacgtgaagaccagcaagcgcacggtcgtagtagcctgcacctttgccaaggcgcatgccggaccggtcgacagcgagcgccgggacaaccaccaaggcgcattcgcgcaaaacggcggaatcatggcgctcgcctacaggctcggtgatccccagcgcgccgggcgtgctcgcgccctcttggtacatcgaccaggcgaggcgcccctgtgccagcgagatcggcagccagacgcgcgcggcgtaagcggcaagctgcgcagggaaatccgccgtgcctggttcgctgggcaggggagagtaggcggcgatcgcgcccccggttgcctcgaagtggcgcatgcagtcaacggtgtgggccacgattgcctggtctaggcgagctttcctttcagtgtcgccgcgcagctgcctgcgcgcggcggtgtggtcttcgcgcatccgctgtttttcttgcagcagttcggcggcggggtcggtcacggaataggcctttcatcgctgtaagctcatgtcttatgcaagagtctatcgatcaagctcaacagccctcgaccggcgcagtgcgcactgttgttgttccggcggctggtatggggacgcggtttttgccggcgacgaagacagtgccgaaagagcttttgccggttgttgacaccccgggtattgagttgatcgctgaggaggccgcggctcttggggctgcgcggttggcgattgtggtggctccgcagaagcaggagattatggcgcactttggggagttcgccactctgcgtgagcgtcttttgtcccggggcaaggatgagcaggctaagaaggtcagtcgcgcgttcgggttgattgatgcggttgcggtgacccaggatgcgccgcttgggcttgggcatgcggtggggtgtgctgaggcggcgttggatgctgaggaagatgtggtggcggtgatgttgccggatgatctggtgttgccgtttggggtgatggagaagatggttcgggtgcgcgagcagttcggcggcagtgtgctgtgcgcgtttaacgtcactgaggacgaggtgttcaactacggcgtgttcgatgttgaggatgcggacgcgggggttgatggtgttgaggtgaagcgggttcgggggatggtggagaagccggcgaaggaggaggcgccgtcgacgctggtggcgacggggcgctacctgcttgatcgtgcggtgtttgacgcgttgcgccggattgagccgggcaagggtggggagttgcagctcacggatgcgattgagttgatgattcaggaaggtcatccggtgcatgttgtggtgcatgacggtaagcgccacgatttgggtaatcctgggggctatatcccggcgaatgtcgatttcgggttgcgggatgagaagtacgggcctgcgctgtacaccgcgattaagcagattctggccgatttcgaggcggagcaccccgaagtcgtcgacaacaccgggcactaacccggcagggcgagaaggggcagaccgatgcgcagcgttgatgagcagttggcgatggtggttgatgctgccgtcaccccggagccaattcggctcagcctcacggacgcgctcgggctgatgtgcgccgaggagatcgccgcctcggaaccgctgccagggttcaaccaagctgcggtcgacggctacgccgtgcgtagcgtcgacgttggcggggcggtggcgatctccagtgccgccgcaggtagtagcgatgctcccgctggcggcgcaatcgcgctgcccgtggtcggtgaggtggccgccgggtcgcagaagccgctgcgcctgcaacctaagcaggctgttcgcgttgcaacgggcgcgccgctgcccacgctggcggatgcggtgctgccgctggagtggtccgaccgcggccagaagcgggtcacgcctcggcgtcctgtgcacaccggcgatttcgtccgccgcaccggctccgacattcaaccgggcgacattgcggtgcgccaagggactgtgctcggacccgcgcaaatcggcctgatcgccgccgccggccgcgacaaggtgctcgtctacccgcgcccgcgtgtgacggtgatggcgtacggcctcgagctggtcgacgtggaccgcgatccgggcctcggccaggtgtacgacgtggcgtcgtacgccgtcgcagcagcttgcggggaagccggcgctgacgtgacccgcgtgggcatcatcaacgcagaaccgcgccgcctgcgcgaaacggttgccaacgcggtcgcgcgcagcgagatggtggtcatcatcggagcggtcggcggctccggcgccgatgcgctgcttagcgtgctgcgcgagatcggcgaggtggacacgacccgcgtagcaatgcacccgggctcggtgcagggtttcgggcttatcggcgacgagcgcatccccgcattccttctgccgtcgaaccctgtctcggcgcttgtcgtcgcggaaacgctggtccgcccggcgattcgcaagtccctggggaggcagaccaccgagcgccgcactgtgcgtgcgcggtcgctgaagccgatagagtccatcggcggccgccgcggctacattcgcgcgcgcctgatgcgcgacgccaccacgggcgattacttggtggagtcacttggatccgtcggcggtgcggccgcgcacctgctagccggtttcgctgaggcgaacgccatgatccgtctgccagaaggcatcacccgtgttcgcccaggcgagatcgtggacgtcgagtttctccagcagcgcggctaatgctcgaccgtctcgccgcggcgctgcgcgcgcccaccccgggttggccggaacagacccgtgcagtgcagcttgctgacggttccactgtccacctccgcccgctcaaatccagcgacggggacagctggatgcagacccggattgttgatgaggcgtggctgcgccccgtcgaacccaccacacacggcacgtggacgcaggcccattcgtacgccgcatggcgcaccacgtggctgaacctcaagcgcctcgccgcaaacggcgtcgtcgtcccgctcgtcatcgaggtaaacggcgagtttgccggccaggtcacactcggcaacattcagcacggcgcggtgggggagtgctggatcgggtactgggtgcattcgccgttcatgggccgcggggtggctacggcagcctgcgcgctcggcaccgaccacgccttcgggcgcatcggcatgaaccgggtgacggcgacctacctgccgtacaacccggcgtctggcaaggtgctcgcccactgcggtttccgcgaggagggctacatgcgccgcaacctccacatcgacgggcagtggcgcgaccaccactttgtggcgatcaacgctgacgattaccccaccactgcggtgcagcgcctggctgaggcaggcaggattcgaatttgagctctagctaaccggcgcgccggcgcggtgcgggcgtcttgccccgatagcgtaagcgcagatacaagtctgcgacgaaaggtgacacgtcccaatgggcagcccgagcctgatcattttgctgatcattgtcgtgtgggtgattgtgctggcaccactggtgttcggcaacaacaagccgatccgccgctccggcgacggttacgaggagacccgcgtgctgcaccaaggcggcaccaccgcggttgccgctcgccggcgcccgaagctgacggccgccgatgtccaccgctacgacgcgcctgagggcgaggagtacgaggtggtcgaagttgccgaggaggagcaggtgcttgtcgacgacaccccgaacctccccagccccgtcatcatcgacgccgaacccgaaccggaggagccggaggcgccggccgaagagcccgcgcccaccggcggctccaccgcgtactccgtccttcgcgcccgcgcagcggctgcatcgagcacgcaggaagcagacgcgcaggagcgctacgaggctgccgaaacctacctggatgcgagcgacttcggatacgagcctgaaaccggcgccgaggaagcggcgccggctgaggaattagggcccgcagtcgaacctgccgaagaccccgtcgcggaggaggctaccgacctcgacgacgaggatctggcgttcgccgaagctcgccgaggccgcggaggctacgacccgcgccgcgacgagcgcacccgcgcagaccgttataagcggcgccagcgcaccttcttgggccttctgatcgccgacgtggtgacgcttgtggcggccgtagtcgccggcggctgggcgtggctgctcccagcggtcgcgatcggtcttaccgcttggttcttggttgcgctgaacaaggtggtcaaacaggaacgcgcgcttcgccagcgccgcatgcgccagctgcgccgcgcccgcttgggtgtcgactccgagcaccacccgggcatgaaacacacagaccgcgtccgcgccggcgcggtaattctggacatcgacgacgagcacccggacttcgaccatctgccgcgttaccgccaacctgaaccggtccacggcggcccataccgcggcggtgacgagtacgacgactacgaccgcgccagctaaccgccccgtctgttctcccagctcacaccggcgatttagcaatgcgggatgcgcggagtaacgtctagcgcatcgaaggggctatagctcagttggtagagcgttgcgttcgcaatgcaaaggtcaggggttcgattccccttagctccacgcaacacaacccgcaggttggcaacatcctgcgggttttgccgtgtctaccggaaggatccccgttaccacagagagaatccgccgcgccgtccttatcgtcgcgcttttgaatttcgcttacttcttcgtcgagttcgctgccgctgttgctatcggctcggcgtcgctgttcgccgactcggcggattttttggaagacaccgcgattaacctgctggtgttcttcgcggtcgcctggcccgcaaagcgccgccagcgcgtcggcggcgtgctcgccgcgctgatcctgattccggcgatcgcggcgatcgccaccgtggtggcgaaggtgatgaacccggtgccgccgtcgccggaggggctgaccttggttgcggtcggcgcgctcgcggtcaacgtcgcctgcgcggtgatcctcatgcggttgcgcgaggccggatccagcctcaccaccggcgcgtggctcgccgcgcgcaacgacgcggtggccaacgtgctgatcatcgtcgcgggtctgttgaccttcgtgtggcccacagcgtggttcgacattgtcgtcggtgcgatcatcgccgcgattaacctgagcgccgccaaggaggtgtgggaggcctcccgcgaggagcacgcgtcggtggaggaggccttcgccgagatggaggaggactagccccacacgcccgaggcgccgcggcgccacgtgccgatcaggttcgtgtccacgatgccgacagactccatcagcgcgtacatggtcactggccccacgagggtgaagccgcgggacttcaagtccttggccagctgctccgattcaggggagcgggtgggcacctcgtccatggttcgcggctgcgggttcgtgtccggctggtaggaccaaatgaagtcggcgaggtttgtgccctcgccgcggagcgcaagggtggccttggcgttggtcacgcaggcttcgagtttgcggcggttgcggatcagggtggcgtcgtcaagcaggtgccccacctccatctctgcaacttttaccgggtcgaagccgaaaaacgcttcgcgcagggcctcgcgcttggtcaggatgagccgccacgacaagccgacctggaacccttcgaggcacaggcgctcgaacatgcccgcctcgtcgcgcaccggcatgccccactcggtgtcgtagtagcgcatgagcagcgcatcggccgcggcccacggcgggcgagcgcggccgtcgtcgccgacaatcggttcgagtttaggattcgtcatgcccctttagactccgttcgttacggccaggttccatgagtagtgttgttcgcatgaaccggcccgctgtgcgtgatttcgccctgctgcttttgcgctgcgtgctcggcgtagtgttcgtcgctcgtgggtacgagcgctggtttggcaccggcatgcgcgcctcggcgcgggaacttgcagccgcaggggttccgcagccgaagtttagcgcctaccttgtgggcaccgttgagctgatcggcggcgtcttcctcatcatcgggctactcaccacgatcactgccgccatcctcgcggtgatgatgctgttcgcgggctacttcgtacacctgccgaacgggttcttcgcggaaaacggcggggtggagtacccattggtgctcgccgcgtcgttgttcatgatcgtggtgttcggtaccggccgcgccagcttggacggggtgctcacccgcgatgcttagccacgaggaggtccgcgacgcgctgtccgcacggatcgacggagagcaacccctgcttgacgacgcagttgtggacgcccacctcgcccaatgcgagccctgccgcgagtacttctcccaggcgctcgctttgggccgccagctccatgtagcggacggggatggtcaactcaccccgccggatctctccgacgtcatcctcgccggcgtggacgacccgtggcggaagatggcgcagcgccgcattgtcacgctgacaatcgggcgcgtggcacttgtggtcatggcgctaacgtgggccgcgtgggcggtgcaatcggtggccgggggcgcggccggggctggcggtgtgacagatgccgccgtacgcttcggcgtcgcgacctcgctggcgctgtgcgcctggcggccggcgcaggtccccggcgtgcttttgatcgtgggcaccatgttcacgttcaccgccggctttgcggtgcgcgacgcggttctgggcgcgggcgagctggggccgggcgttgttgtggtgccgttgatcaccgcgctcgcgctggtgtggacgtgggtcgctgaccgcgggatcgaagtgcgccgcgcctggtcgtacctcagcgcgaatccgagttagcgccagctcggtagccacatgagcgactggaaatagtcctccggcaccatgtagccgtagaagatcggcgaccagtagatgaagctcgcggccaccaaggcgacgtagacgatgacggccagctgcccggtgcgcagctgggcgccggcgatcttgcccacccagggccagcgcaccggctcacccttgccggcaatgttgcctaaggcaagtgcgatgagcaccgcagtgaacggcacaagtgcggtggcgtagaagaagtacatctggcggtcgaaggcggccagccacggcaggaagccggcggcgaaagcgataagcggcaccatcacgcggtagtcgcggcgcgtcacccacacccacagcgcccacagcagcaccggcaccgtcagccaccagatagctggggtgccgaagaggtagatcatctcgcggcacgtgccgccgttgccgcactcgatgtcggtggcggagtagtagaggatcggccgagcggagaccagccacgcccacggcttggaatcccacgggtgtgagtgcccggaggacgatgtcagcgagccgtggaactcgagcacggagaagtggtagtagagccacccggcgatggaagacggcaggtttgcaagccagggccagtcggaggaggcgatggtgccgtcggcaagcgaatgcctgtacacagaggtttccgaagcaaaccaggcgcgccacgaccacaggtagagcagcgccggtagcagcacgatcgtcgcgagcgcgggcgggacgtccttcgacagcgcgccggcgaggggtttctccacgccgtagcgcttgcgcagccacaggtcccagaacgagccgagcaggccgaagaacgcgatgtagtacaggcccgaccacttcacggacagggcgagtccgagcagcacgcctgtggcgaaacgccaccagcggaaaccagtgcgcgggccgcgggggccggcagattggagctcaccagatgcccacgcgtcgtgccagcgctggtgcgtctggcgcatgtctcccgccagcgtccaggcggcggcgacgataaacagaacttggaagatgtcgagcatgccgaacttggccgcgacgagaagcacaccgtcgaacagcgcgatggtgccggcgaggacgccgatggtggttgactggctcacgcggcgggccaggaggaacgtgaagacgatgacggctgaaccgaacagcgcagtcatcacgcgccagcccaacggggtgtagccgaacagcgcctcgcccgcggccagcagctgcttgcccagcggtgggtgcaccaccaggccgtagcccgggttcgactcgatgccgccgagcaccgggttgaacgaggagcgcaccatgtcccagccttgcggcacgtagtgtttctcgtcgaagaccggggtgcctgaactggtgggcagcgtcacgccgatgaaacgggtcagtagcgccaacacgccgatcaccgctgcggatatcgtgtcgcggcgcgaccacggcaccgtcaccggcgcacctggcgccgggcgcttggggcgggtgacctccaccgcgccggccggatccggggtggggccttgcgcgggcgtattcgcaacgactgtactcacgaggaaggatattagctgcctgcgcgtatggttggggtttatggtcgaccccgtaaccgagctccccgcccgcggcgtggtgctggcggcgacgccgctgggcaacatcggcgacgcatcgcagcgcctgcgcgacgcgctcgagcgggcggacgtcatcgccgccgaggacacccgccgggccaaggcgctcgctgccgcgctcggcgtgaccccgcgtggccggatcgtctccaacttcgaccacaacgaggactcccgctcgggcgagctgatcgacgccgcccgcgccggcgtggtcctcgtggtcaccgacgccggcatgccaatagtttccgacccgggtctcgccctggtcgccgccgcgcacgacgccggtgtggaagtcacctgcatcccgggcccgtccgcggtcacgacggcgctcgccctgtcgggcttaaacgtcggccacttcatcttcgacggcttcgctccccgcaagcccggcgcgcgggatgcgtggctggaatcgctggtaggggagaagcgggcggtgtgtttcttcgagtcgccccaccgcatcgcggccacgctagcgggcgccgcgcgcatcataggtcccggccgccgcgccgcggtgtgccgcgagctgaccaagacctacgaagaggtcaagcgcgccacactgggcgagctcgccgactgggcgtcggagggtctgcgcggcgagatcaccgtggtcatcgagggcggcgcgcccgaggcgcccgagccggaagatctcgtcgacgaggtgctgcggagggtggacgccggcgagcggatgaaggacgcggcgcgggctgtggccaaggaaaacggcgtgaagggctcggcgctttacgacgccacgttgagcgcccgccagcgttaacacagattcctccagttcgagacatgggcgcctttcaggtagcctgcgggggcaattgatcgtcccctaaggtttcgaggagaactcatgtcagaccaagacacctcagcggctagcgagcttgcgtcgctcatcgccgcggaggagcgcggcgagctgggcaccatcaccgcgcctgaggaccaggtggagatgcagtcggagcagaccaacgcgcctgtttcgtggggcattgtcgccaccatcgccgcactcgtcgcggctattgttgcctgggcgctgatcgcccccgagaaattcatcgacttcgccgacaacgcgttcacctgggtcatgaacgactttggctgggcgttcgtcttgttcggtaccgcgttcgtcgtcttcatcttcgtcgtcgcgttttccaagttcggttccatccgcctcggcggcaacgacgagcagccggaattccgcacctcgtcctggatcgcgatgatgttcgccgccggcatgggcattggcctgatgttcttcggcgcctcggagccgctcgcgatgtaccgcgacggcgtgcccggccacgagccgcacgaagtgggcaccgccatggcccagaccatgttccactggacgctgcacccgtgggcgctctacgccatcgtgggcctggccatcgcgtactccacgttccgcctcggccgcaagcagctgctttcgtccgcgttcgtcccactgatcggccaagagcgggctgacggttggttgggcaagcttatcgacggcttcgccatcttcgccaccatcttcggcaccgcttgctcgctcggcatcggcgccatccagatctcttccggcctcgaggcctccgggttcgtggacaacccctccgacaaactgatcatcggcatcgtcgcggtactcaccctggcgtttctgctgtccgcaatgtcgggcgtgggtaagggcatccagtggctgtccaacttcaacatggtcatcgcagccctgatcgcgatcttcgtgttcgtgctcggcccgacggtgagcgcgctgaacatgctgccaacctcgatcggcaactacttctcgcagttcttcgaaatggccgcccgcaccgccgagagcgccgacggcgaagccggcgagttcctctccggctggaccatcttctactgggcgtggtgggcgtcctggtcgccgtttgtgggcaccttcctggcgcgcatctcccgcggccgcacgatccgggaattctgcctcactgtcctgctcgtcccgtcgcttctgtccaccatctggttcgccatcttcggcggcaccgcgatcaagttcgagcagagcggcgaatccatctacggcagcggcagctccgaggagcagctgttcaacctgctgcacatgctgccgggcggctacttcataggcatcttcgccgtgattttgctgggcaccttcttcatcacctccgctgactccgcctcgaccgtgatggcgtccttgtcccagaacggccagaccgaggcgaagccgtggctcgccgctatctggggtatcgccaccgccgcggtcggtctgaccatgctcacggtaggcggcgccgactccttgaacgcgctgcaaagtgtcaccatcgtcgcggcgtcgccgttcctcatcattttggtggcgctgatgttcgccatcgtccgcgacgtttccaacgactccctctacctcgcgcagaaggagcaggagcgtttcgcccgccagctggccattgagcgccgcgcccaccgcgaccaggtccaattcgacaaccgcaaacgccaggtgaagcagatgctcaaaccccgcgggcgtcaatagcgacgcagcgcagctctgcccgttcggctggagttgtaggtctactgtcgtagttcagcgcaaaaactccaggtgggggtggagacctacaacagtagaactacaactcgggcccaggcgcagcgcgtaaccgcggcggcactgcccgcccatacggcctccggtaaggaaaccgggggccgttcattatgcttgagaccatgacttctcccgagaccaaccagaatgttcttgtgtgcgtggcgtggccgtacgcgaacggcccgcgccacatcgggcacgtcgccggcttcggcgtcccctccgacgtcttcgcccgctaccagcgcatgacgggcaagaacgtgttgatggtctccggcaccgacgagcacggcaccccgcttttggtgcaggccgataaagaaggtgtcagcgtgaaagagctcgctgaccgctacaacaagcagatcgttaacgaccttgctggtctcggcctgtcgtacgacttgttcacccgcaccacgacgcgcaaccactacgcagtggtccaggagctgtttaagggcctgtacgcgaacgggtacatgattaaggagacgacgcagggcgcgatctcgccgtcgacggggcgcaccctgccggaccgctacatcgagggaacgtgcccgatctgcggcgccaccgacgcccgtggtgatcagtgcgacacatgcggcaaccagctcgacccggccgacctgatcaacccggtgtccaagatcaacggcgagacgccggagttcatcgagacggagcacttcctgctggacctgccggcgctgcacgacgccctcgaggagtggctgaagggccgccaggactggcgtccgaacgtgttgaagttctccctcaacctgctcgaagacatgcgcccgcgcgctatgacccgcgacatcgactggggtatcccggttcccgtggagggatgggaggacaacccgtcgaagaaactctacgtctggttcgacgcagtggtcggctacctgtctgcctccatcgagtgggcgcagcgaagcggcaacccggaggcgtggaagcagttctggcaggacccggctaccgaggggtactacttcatgggtaaggacaacatcacgttccactcccagatctggcccgcagagttgctcggctacgccggcaagggctcgaagggcggctccgagcacgcgctcggtgagctgaaccttccgacggaggttgtctcgtcagagtttctcaccatgagcggctcgaagttctcgtcgtcgaagggcgtcgtgatctacgtcaaggacttcctcgccgagttcggtcctgacccgctgcgctacttcatcgcggtggccggcccggaaaacaacgacaccgacttcacctgggacgaatttgtccgccgcgtgaacaacgagctggctaacggctggggcaacctggtcaaccgcaccgtatctatggcgcacaagaacttcggccaggtgccggtgccggggccgctgcaggaggcggacgagaagatcctggccttagccgaggacacgttcgcttcagcaggccaggatttgacccgcgcacacttcaaggcggctgtgaccaaggttatgcacgtcgtcggcgaagccaacgcctacatcgcggaaatggagccgtggaagctggcgaaggacgacgcccagcgagagcgcctcgctactgtgctgtggactgcgctgcaggtcgtctccgactgcaacgcgatgcttaccccgttcctgcccaccacagcgcagcgggtgcacgagacgctcggccgcaccggcacctgggcggcgcagccgcgggtggaggaagtaaccgacgacgccgagtacgaccttatcggcgtgggcctgccggagaaggggcagacctacctcacgatcaccggcgactactcgcaggagcaggcggcgtgggcgcgcgtcgacgttgtgccgggcacggagctttccaagccccagccgctgattgccaagctcgaaccggagctcggcgagaccgggccggagtgggccccagtgcagtaattactacccctacacccccaccgcgggcctcgcactcgtgagacgccccgattggggagtgggggtttcacatgcgcgcgaaacgtcacgcaaaattcactttgagtggacggtgtgttcatcttcgggatctacgatgaacgcatcgtccataatccaaggggaccgtgaacgtgacgcgcagcatcattttcgacttcgatggcacgctcgccatcgggcatgggcccgtcgtggcatatgctcgtgagctggcgagcgtggctcgtgtgggttttgtagcccgagttgaggaagcgctgagcagtttcgaatcaggccactccgactacctcgacggctaccaggtcgttgcggagctcgcggctcgagacggggttccttcggggacgatgagcaaggcctacctagcaagccgagaaatgcttgggactgccgaggcgcccgtcaacgcgcccgctggtctcgctgagctgcttcgcacactcagtgagcacgccaccatccacgttgcgaccaacgctcccgctaccggggtggaacgtgtctttgatacgtggggagtgggtgatttcattgatcatcttcacgtcaacgcgggcaagccggaggggttgtacccgatcatcagggatgcactggcaaccggaccggtgatggcggtgggggatatcgtggccaatgatctccaaccagcgttggacctgggtgcggacacagcgttggtcggtgccactgccgtcacgagtggcgcggatgtgacgatgcgaggcgcttcgctgacggaccttcatgacgcgcttgttagctgggctcaaagagaaccccgacctaccgcgaaaggcactcatcatcatgcgtaaacccgttctcgcgctcggcgcaatcctcacagccactgcactttctgtaaccggttgctcctccgattccggctccgactccactgggatgtcaaacgcttcggacgccaacgactggccagaggagatcacgatctctctcgttccagcaacagagggcgagaacctcgccgaagcactgcaaccgctcacctcgtacctctccgataacctcggcatcaaggtaaacggggttgtcgccaacgactacgccgcgacggttgaagcgatcggcgccgaccaggcgcaggtcgccatcaccgacgctggctcgctctataacgcgatgaaccagtacgacgccaagctcatcctgcgcgacgtgcgtttcggtgcgacgaaatacgcatccgtggcctacaccaacaacccggataagtactgcgacgaggccccggtaacagcaacatacgaggcctcaaagaccgagttcgcgtactgcaacggtattgagaaggctggatcgacagccaccggcacaggccccgcggcgacaaacgctctagagaagatcgaggccggcaccaaggttgcgatgcaagccgtcacgtccccagctggctaccagtatccgatcgtgacgatggaagaccagggcgtggacgtggacaagctcgaccaagtgccggtgcagggtaacaacaatgccatgctcgcggtgctcaatggcgatgccgaagttggcttcggctactgggatgcccgtgcatccatcatcaaagaggctccggaggccgcgaccgacatggtcgcatttgcgtacaccgagatgattccgaacggcggcgtggtcgttaccgataccctgccggacgatctcgtggccaagctcaccgacctgatggataactacgcagactcttcggacgaggcgaagcaagttatgcaggacctcgttggcctgaccgattggacggatgagacgaacgaggatgagatccagcgttacggcgagatttacacccgtttcaagtcctaacccggaacgaaagctgatcatggataacgcgcgcgcatcgcagatcacccgcgaaccgtggccgatagtcctcgaccatgtctccgtgacatacccgaacggtacccaggcgttgaaagacgtctcggtatccattgaaccgggggaaatggtcgcggtagtgggtttgtccggctcgggtaaatccaccctcatccggacgatgaacgggctgaccagtgtttctgcgggaaccgttcaagttggtccctacgccatgaacgagttaaacgggaaacaactgcgtgaggcgcgcggccagatcggcatgatattccagcagttcaacctagcggagcgcaccgacgtcttccataacgtcatggtgggcagcttcgcgcgaaacccgtggtggcgcaccgtcttcgacatccccgctgcagcggataaagagctcgcgctcagcgctctggattcggtcgggatgttggagaaagtgtggacccgagcaggggctctttccggcggtcagaaacagcgtgtggccattgcgcgcgcactcacgcaggagccatcggtcatgcttgccgacgagcctgttgcctccctcgatccgcccacgtcgcattctgtgatgagcgacttgcagcgcatcaaccaagagcgcggcctgacggtgatggttaacttgcacctgattgacttggcgcggcagtacacgacgaggctgatcggtttgcgccacggcgagttggtgtacgacggtccaactgccgacgccaccgatgatgacttccagcaaatttacggccgtcccgttcaggccaaggacaggttaggggagcactgatgcagactcccgcgaagccgacaagccaccttcgctgggcgctcattgtgctcgcggtcgtggggttcacggccctgacgatgacgccgcagattggcggcatcgccatcgacttggaatccatcgctcgcaactggcgcaacggtgcagcgaagctagcgcagatggtgcaccccaactttgcgttcctgccgcgaaccgcgctgccgatgcttgagaccttacagatggcctttgtgggcgcggtcctgtccgcaatcgtgtcggtcccgctgacactgtgggccgcacagccgaccaacccgaaccgaatcggacgggtggtaacgcgcaccctaataaacatcatgcggtcagtgcccgacctagtgtatgcatccatcttggtcgccatggtcggagtcggggcgcttccgggtgtgatcacactgttcttgttcaacttgggcatcgtggtcaaattggtttcggaggccatcgactcggcagaccactcctacatggaggcgggtcgggcggcgggtggcacgcagctccagatcaatcacgcgatggcgcttccgcaaaacatgcccctgtttgccaatcagtggttgtacacgttggagctcaatgtgcgcgtgtccgcgatcttgggccttgtaggtgccggcggcatcggccgcctactggaggagcgccgatccttttttgcctacgacgatgtctcgatcatcatccttgagattctggtggtcgtagttctggtcgagatgatttccaactggctgcgaaagagactggtgtagataatgccgggcaagccgaggaaaacgtacgagaccatcgctgccatcctgcttggtctcttagtgatcgtttcgatcgcgacgctgaacattacgtggagtgagctttcgcaggtacccgggcaggtttggcactacctgcaactgatgtttgccgagcccgactggtcgaagcttgaccgcgctttgttggagatgtggcggtccatctcaatggcgtggatcggcatgatcggcactgtcgtgctggccatccctctcggcatgctggctgcgcgtggcgtggggccagcctggctgagggccctgctgcggggccttttcgccgtcatccgcgccttcccggaagcggtgatcgccattatcttgcttacggtcaccgggctcacgccgttcaccggggcgctggctttggccatttcgggaatcggtcagcaggcaaagtgggcctacgaaacgattgagtcccttccgccgggtccggcggaggccgtgcgcgctgccggcggcacgaccgctgagaccgtgcgctgggcactgtggccgcaggccgcgccgtcgttgatctcgttcgcgctctaccgtttcgagatcaacatccgcacctcggccgtgctcggcatggtgggcgcaggcggcatcggtgcgatgctggcgaactacactaactaccgtcagtgggacgtggtgggtatgacgttgatcgttgtcattgtggccaccatgatcgttgacgctatatccggcactatcagacgccgcatcatggaaggggctaccgttcgtgccaacgcaaccgagtcaggccagcccgcccaccgtccggatcgcagcggcgatgtcgtcgctgcaaccgacggagcgaacggtcgttgatttcatcggtgcggatccagcgtcggccgtagagatgacggcgcagcagcttgccgatcacgttggggtaagtcgggcaagcgttatccgtacggcgcaaacgttaggatactcgggatttccccagcttcgcgtggcgctcgcgcaggaagtagcgagcgcccgggcggccacagcgttcgaccccgcaaccggttccatgctcgacatggttcagcacaatgtcgcgcagttttcgcaccgcctcgaggcatccttcggggcgattgatggcacagcgctggccgaaacggtgcggcagcttgacgcagctgatcgcgtactcgtggtcgcgaacggtttttccgcgcccctcggtctcgacctggtgcagcggcttatctcggctggccgatcagcggagttccataccgatgcaatggcgcagcgcattgcggcgcaccacctcggagcacagtcggtgtgtttcgtcttttccggctcgggtgcgaaccggcccacgcttgaggccgcggagcgggcgcgggaaagcggtgcggcggtgatcgcgatgacgaacttctcgccgtcgccgttgacgcagctcgccaccgtggtgctgctcgtgccgccggcgaacaactcgtttcaagacgagctcatccacacctcccgcgcggcgctgatggtgctcacggagcaaatcgtcgagctgctgcttgcctatcgcggtgaacgcggggcggaggcgcgtggagtggtgctctcactgctcggagacgcgctcgaaagctaactgcaacgagccctagcgcccgcccaagaactggtccaagaacacggtgagtttgcccgtttcctcgtcctcgtagcgggtgtccacgaccaccagcggggcgacgtatttctcccccttgtggacgacgaggtcggtgccgtaggcgtcggcaagcaatgcccacacgtagccctcgcgcaccagcgcatcgccgagtgcggtgccgtagatgcgggccgtgtcgccgcgcgggtaggaccgctgcacgtcgcgcggcagggcgaggtagtcggcgagctcgccctcgaagctttccacgatgtcgtgcggggagccgttgatgccgcggccggcggcttcggcgaggtcggcgttgatctggcgctcggtggcgctgtcgatgggttcgaatgccatagggttggattctatgagcaagaaaccccgccctacgccagtgcccgcggaccgcatcgacggcctgattgacgcccacacgcacctcgcctcgtgcaaggtgccggcggcggaactggttaagcgcgcgacagaggccggcgtggcgcgcatctgcaccgtcggggacgggcttcgggaggcagaacttgcactcgccgcggcgcacgagttcgacaacgtctacgccgcgtgcgcgatccacccgactcgcgcgggtgagctcgacgacgccgcgcgtgcgcgcctgaccgagatggccgcagatccgcgctgcgtggctgtgggggagaccggcatcgacacctactggctcacgcacgacccggacgcaaccgcgccgcttgacgtgcaggaagaggcgctgcgctggcacatcgacttggcggtcagctccggcaaggcgttgatgatccacaaccgcgagggcgatgcggagttgatgcggattctcgcggacgcgcccgcaccaaagcacgtgattcttcactgcttctcctcgccgctcggcgtcgcgcgcgaggcgctggagcgcggctacgtcttgagcttcgccggcaacgtgacgttcaagcgcaacgaggagcttcgccaagccgcggctcttgcaccggcggggcagtacctggttgagaccgacgcgccgtacatgacgccggagccgttccgcggggcagccaacgagcccgcgttgatcggtcacacggcgcagctgcttgccgacgtccgcgggacaagtgttgcccaagttgcagacgaggtgcgtgagacgttttcgcaggtctacggggtgtgatgcgcgacaaaaaacgcgcaattacttgaaagtaatagaagcgttaccgtatcgttaccgccatgtctgccgcgaagaaaacgctgaacccgccccacgagaccgcctcgaccccgaagcgggtcatcgccggtgccgtcgcgggcgccgtcatcgtgggcggagccggcacggcactggccgctcagaaggacatcaccctcgacgtcaacggcgaggcgacgaacgtgcgcactttcgccggcgacgtttctggcgtgctgcaggctgccggcgtgaccgtgggcgcgcaagacttggtgtaccccgcgccgggcgagcgcgtctcccggggcgacaccgtcactgtgcgcaccgccaagccggtcgcggtggtgatcgacggtgtggctcaggagctcacctccaccgcggccacggtcggcgagctgatggacgaggccggggtggacgctgcctccgcaaccgacgtcgaccgaaacgctccggtgaccgagggcctttccgtcgacgtgaccaccccgaaggtcgtcggcatcactgacgcaggcgtgcagcacttcaccacggccgcggcgaagaccgtcggtgagctgctctcgtcccgcggggtcacgctcagctccaacgaccgagtcaacgttccgctcgacgcggcggtgacgccgaacatggacatcgtgatcgaccgggtgcaggtgctgcgctcctccgagatcgttgaggtggttgccgagccgtcctacgtcgaggacccgaacttggacgagggggtcgaggaagtccgcgccgaggctgtcccaggtgagactgaggtctaccaccgcaccgtcacggtgaacgggattgaggagtcgcgccacgtcgcgggcgagcgcgtggtccgcgaagcgaagcccgcgaccatcgcgcgcggcaccaagccggtcgcgagcagcgcggccgcccctgctgcccctgctgttgcttccggctcggtgtgggacgcgctcgcgcagtgcgagtcgggcggcaactggtccatcaacaccggcaacggtttccagggcggcctgcagttcacgccgtcgacctgggccgcgtacggcggcactgaatacgccccgctggcgcatatggccacccgcgagcagcagatcgcggtcgcccagcgcacgcaggcgtcccagggttggggcgcgtggccggcgtgcactgcctcgcttggcatccgctagtctcgccgtatggcagattcccacctgctggggccagtcgagatccgggaactggcttcagagctcgacgtcacccccacgaagaagctcggacagaacttcgtccacgaccccaacaccgtccgccgcattgtcgcggccgcggagctttctcccgacgacgttgtggtggaggttggccccgggctggggtcgctgaccctggggcttgtggatacggtctcacacgttgtcgcgctcgagatcgacccgcgcctcgccggccggcttgcgcagacagttggtcagcgcgcgccggagtttgcagatcgcctgaccgtgctcaacaccgacgcgctgcaggtggctcgcgcggatgttgccgccgccgacgcggtgcccaccgcgctggtggcgaacctgccctacaacgtctcagtgcccgtcttgttgcaccttttggcggagttcccctccatccgccgcgtgctggtgatggtgcagaaagaagtcgccgaccgcctcgcggcaacaccgggttccaagatctacggggtccccagcgtcaaagcggcgttctacggcgaggtatcgcgcgccggcaccatcggcaagaacgtcttctggccggcgccgaacatcgagtccgggctggtgcgcatcgacgtcgacccgcaccgcgacagggggcttcgggagcatgttttcccgcttgtcgacgcagcgttttcccaacgccgcaaaactctgcgctccacgctttcgagtgtctacggctcgccggctgccgccgaggaggcgcttcgcgcgtcaggcatcgaaccgggcctgcgcggcgaggccctgggcgtggacgacttcatccgcctaggcgagatgcgaaggagcgtcgccgatgactagccgcgagatcgagccgcgcacgttcaccgcttcggcgccggcgaaggtgaacctgcacttaggcgtctctaacgtcatcgattccggctaccacgagctgatcacggtcttccaggccatcgaccgccgcgaggtggtgcgcctggtagtggagccggacgaggaacccacgcgcgcggaatcggtggtcaccggcatcaccacccgctggctctacgatgacgacctgcccgaggacatcgacacccccgacaacctggcgtggcgcgcggtggatctcgcagtgaactcgttccgcaacggatgcaaccacaccgctggcgtgacccacccggcgctgccgaaggtgcgcatcgaggtggacaagtcggtgttcgtcgctggcggcatggccggcggctccgcggacgcggccgcagcgctgctcgccgcgaaccactacatcgagcactacttcggcgagccgtacgctccagaccatttcaccagctcctcggcgcccgtcctcggcgcggacgtcccgttcgcggtgctgggcggcaacgctgtcggcaaaggccgcggggattcgctcagaccgcttcctggcggcggcaccttctggtgggtgttcgtcaaccccgcaaccaccatcagcacgaaactcgcctttgccaagctggaccagctgcgcgcgaacgacccggacctgactcccaacatggacgtcggccccgtgtccgacgcgctcatcttgggcgacccgcacgccctggccaaggcgctgcacaacgacctcgagctgccggcgcgtctgatgcgcccgcagctcggtgagctgctcgagttcggtaacgccgaagcgctgcgcgccatcgtctccggctcggggccaaccgtggccttgctgtgcgaaagcggagagcacgcgcgtaaggtccgcgcgcgggttagcgaggtcttcccgcgctacacctccttcgcggcgtctggcccggcgcatggcacgcagatgctgccgtgaacctgctcgactcgcttcgttaccacctcgacggcaccagcggtgcgttggactctgcgtactcgccgattactgcggggaagggtcggaaggggaaatacgtgccgtcggtaagcagcctgctccgaagcttcgtcgccgtggactttgagaccgcgaaccgggtcggcggggcgtctgcgtgccaagtcgcgatggtgaaagtcgccgacttcgaggtggtcgacgcgttttgcacgtacctgcgcccgcccgaggaacacatcgcgttcgagttcagccacatccacggcatctaccgcggcgacatcgacgacgccccgagctggttcgacatcgccgacgacgtggtcgatttcgttggcgacgcgcccgtgtacgcgcacaacgccacgttcgacgcttccgtgtggcgcggcctcgaccgctactacttcacgggcacggtgccggcccagatgtactgcaccgcgcgaatggcaaggcggctgctgccggagctttctgaccacaccctgcccaccgtcgccgcgttctgcgcgccgggttttccgctgaaccaccaccgggcggactccgacgcgctggcgtgcgcgcacatcgtcgcctacttccaaagaagccgggggttgcacggtttgcttgcgccgtaagattgggcctcgatggcaaacctgatcaacttagaaaacgtctccaagacttggggcttgaaaacgctgctcgacggtgtgtcgctgggcgtgcagagcagcgaacgaatcggcatcgtcggggtcaacggcggcggtaaaaccacgctgctcgaggtgctgaccggcattgagccgccggacgcgggccgggtgtcgcacaactcctcgctgcgcatggccgtggtgacgcagcgattcgagctcgaccccgcgctgaccgtgggcgaggccgttgtggcgccgttggggctcgagaccttcgagtgggcgtcgaacgccaaagtgcgcgaggtgctcgccggcacgggcgttgccgcgctcgggctggacacgccggtgggcgagctctcgggcggcgagcggcgccgcgtgaacctcgctgcggcgctggtgcaagatctggacctagtggtgctggacgagccgacgaaccacctcgacgtcgaaggcgtgcagtggctggccgaccacctgctctcgcgcaagctcgcggttgtggtggtcacgcacgaccgctggttcctcgacaccgtggcgaacctgacgtgggaggtccacgacggaaccgtcgacgtctacgagggcggttacaacgattggaccttcgcgcgcgccgagcgggcccgccaagccgacgccattgagcagcggcggcagaacctggcgcgcaaggagcttgcgtggttgcgccgcggtgcgccggcgcgcacctccaaaccgcgctaccggatcgcagccgccgaggcgctaatcgccaacgtcccggccccgcgtgacaaggtcgagctgatggcgttttccaagcagcgccagggccgcgtggtcatcgagctggaagacgcgcgcatcgacgcccccgacgggcgcacgctggtcgaccacctcacctggcgcctcgcgccgggcgagcgtatcggtctcgtcggcgtcaacggctccggcaaaactacgctgctgcgaactttggcgggggagtacccgttggctgcgggcaagcgcatcgagggccagaccacgcgcatcggctggctgcgccaagaactcgacgaccttgacccgacgcggcgcgtcatcgacgcggtggaagacgtcgccacctacatcgagctagggaggggccagctttcggcctcccagctcgcggagcggctcgggttctcacccaagcgccagcgcaccccagtcggcgacctctccggcggcgagcggcgcaggttgcagctcacgcgcgtgctgatggcggagccgaacgtgctgctgcttgatgagccgaccaacgacctcgacatcgacaccctccaagaactcgaggacctgctggacaactgggccgggaccttggtggtcatctcccacgaccgctacctcatcgagcgcattgccgacaccacctatgcgctgttcggcgacggcaagctcaccaacctgcccggcggcatccagcagtacctggaccgccgcgccgccgagcaggtcagcaccggtgtgctggatctgggcgcgggcgatccgcaggctggcgccgcccccgccaagacgttgtcttcgcaggaggagcgcgagctgcgcaagaagatgaacgcgctcgagcgcaagctggagaaggccggcaaggacgtggccgcgctcgaggcggagatcaccgagctgtccggcggcgccggccccgatttcgaggcgatcggcgcgaagaccaaggcgcttgcggcgctgcgcgacgaacgcggcgagctggagatgcagtggctcgaactcggggagcagctcgaggcctaatcgtccacaatggtgccatgcgcaccccactcgtcgccctcgtcctcgcaggcggccgcggcagccgcctcacgccgctcaccgaccaccagccgaagcccgcggtggcgttcgccgggagctacaggcttatcgacgtcaccctgtccaacctcacccactccggcatcaacaacgtgtggatcgccgagcaataccgccccaacttcctgaaccggtacttggcaggcgggcgcccctgggacttggacggcaccttggcggggctgcgggttctcccgcccggcgagggcggcaccgaggacggcttcagtgaaggcaacggccacgccctgtaccagcacctcgacgaggtggaggcggcgggcgccgagacactggtggtcatgagcgccgaccacctctgccagctggaccttcgcgatgccgttgcccagcacgagcaactcggcagcgacgtcactgtagtgaccaccgaggtcgccgaggacccctcccgctacggcgttatccagaccgacggcgaccgggtcaccgagtacgcctacaaacctgagtcgccgaagggccacgtgatcgcgaccgaggtcttcgtctttcgcgtggcggcgctgcgcgccgcgtgcgacgccctggtcagcgaaggatctgacggtgctgaactgggcgattacggcgaaaccatcctgccgcacatggtggaaaacgcctccgtgcacgcgtaccgctcggacggttactggcgcgacgtcggcaccatcgacgcctatttccgggcgcacatggaactcatcgacggcaccggtttcaacctctacgaccccgactggcccgttttgagcaacctctcgacttccacgccggcccggattaggcctgaggccaaggtcgacaactcgctcatctgcccgggcgccgacgttgcgggcgaggttacccacagcctgatcggccccggtgtgcgtgtggagcggggcgcgaaggtggaccgttgcgtgctcaccgcggatgtggtggtgcccagcggcgcgcatttggaatccgtcattgcggacaccggagcacacgtcggtcccggccgcaccggggcgacgaaaccgggcccgggaaacatcaccgtgctgaccgcggagttgtagtcccacagttgtagtacagctcgagagccgcaggtggggccggagacctacaactctagaactacaactccagcggacccgcgccccgggcaagacggcgggctctaccataatcgaaacagatgtggcaaaatgatacgcatgtggaatatcggacataactctaagaaagttgcgggcgtcgccgccgtcaccgcagcgcttgtcgccggagcgttcgcaccggccgcctccgcccagccgcagagctctgcgccgtttatggatctccaggtcaacggcctgtcgtcgcaggcgaacatcgtggtgccgcagctgccggacattgaggtgccccgcgaggttgttgacggcgccaagcgcgtcggcatcaccctgccggagcgcattgaactgtcgaagcggctcggtggtgccgcaccgcaggatgaggtcagcgccaccgagcgcgacctcgtcgcggcctccgaggcgcagctggttaaggaaggccaccgccgcgacgacgaggcgcagcgcattgccgctgagtgggctgcccaggcggctcgcggggaggccacgttcaacggcaacgtcggccgcggcacgacggccactgaccgcggcaccggccagatctaccgcctgaacccggcgcaggcagctgagcgcatcacgtggctgcgccgcgacgagactacgaaccgcgtcagtaccaaccccgtcaaggagccgaagcgcttcggcgtcgccaccgcgcgaaacggcgagaccgtctacttggtggagtacttcctcaactagaactaccattggcgcgcaggcgtcggttaccgtggatggtatgagcgaagagtctgtgaagaagccgccgaagctgtccaagaaggcgtatgagaaggagctgctgcgtcttcaagcggagctcgtagccatgcagcagtgggtggtggaaaccggcgctcgcatcgtgatcatcatggagggccgcgacgcggcgggcaagggttccgcgattaagcggatcacccagtacatgaacccgcgcacctgccgcattgaagcgctgccgaagccgactgagcgcgagcaagggcagtggtacttccagcgctacgtggagaagttgccggcggcgggcgagatcgtcatcttcgaccgttcttggtacaaccgcgcaggcgtggagcgcgtcatgggcttttgtacctcgcaggagtaccgccgctttctgcaccaggcgccgatcttcgagcgtcttctggttgaagacggcatcatgctgcgcaagtactggttctcggtgtccgacgaggaacagtacaagcgcttcgtgtcgcgccgcgaggatccgttgcggcagtggaagctctcgccgatggatctcgaatccatcacgaagtgggaggagtactcgcgcgcgaaagacgagatgttcatccacaccgacatcccgtctgcgccgtggtacacggtggaaagcgaggacaaaaagcgctcccgcattaacgtgatctcgcacctgctctcaacgatcccgtacgagcacgtcgcccttgacctgcccgagatcccggagcgccccgagaccaccgattacctgcgcccgccgcgcgacgagttccgctacgtgccggacgccgccgccaagctggaggagccaaaggtggaaggtaagaaaaagaaaaagggcaagaagcgctaggcagcttgtcgacgctacgctttcttcggataccccctcggcgtcgacaccgtcttgttcttggggatccagaacctcagcggggcgtcggcgttcttgctgatgccgatgcgcggccccgccacccattccggctcctccgcacgctctgtgagctggaccggagtgccgttgtccggcagtgttagtcctaaagcttggccgaggttgcccggcccgcgcgccaagttctcgtaggggatgggtgcgcgctccggccgctggcgccgttggcgcgcgagctcctcgccagctacgacttcgccgccgcgcatgaggcaaccttggccctcgccttcgggggcgcagacgatgttgccgttgtggtggatgccgtaggaaaagtagacgtacagccgccccggcggaccgaacatcgacgcgttgcgcgccgtcttcccgttgaaggtgtgtgccgcgggatcgagggagcccacgtacgcctcgacctccgttaaccggatgctcaccccgttgtgcgtgatcacgcaccccagaagctgcggggcaacaatgtcggcggtctgggtgaaatcgatcatccaacaatcgtagcttgtgatgtggaacacttggatcccatggatgctgctatggacaacaagattctgaccgaggtccgggacaccaccggcatcattacgctcaaccggccgaaagccctcaattcgcttgacgacgagatgattcgggtgcttgatgccaccctgcgcgaatgggcggtcgatcacacggtcgagcaagtggtgatctgctcgaactccaagcatttctgctccggcggcgacgtgaagttcgcccgcgccgaaggcctcgccggcaacggggagcgcatcgacgccttcttcgcgcaggagtacgcgatgaacaacttcatcgccgaattccccaagccctacatcgcgctggtcagcggggtggatatgggcggcggcatgggtatctccgcgctcgggtcgcacatggtggttgccgaggggtcgttcgcctcaatgccagagatgaacatcggttacatcaccgacgtcggcatgagctggaaactgcagcacttgccgggccgcgagtcgacgaacctcgggaagtaccttgggctgaccggctaccgcatgaccccagacgacatgattgccctcggcctagccagccacaaggtcgagagcttggagggactcctcgacactctcgttgaccaggggatcggggccctcgatgcggccgcggttcagcccggcgaaagccccctcgcgcgttggttcgacgacatcgaaaccgcattcggcgggtcttgggccgagattgaggcgcgccttgtcgcccagcccggcgagttcgccgagctggttcgcgacctgacgaagcaagtctcgccatcgtcactcgtagccacggccgagcttttcgaggcgaacgcccgccacgacctcgccggcgcgttggaaaacgagcgggtgctcggcgagctcatgcggcgcgaacccgacttcgccgagggcgtgcgcgcggtgctcgtggacaaggaccaagctccggcgttcgcgccccagccagatccggacaagtaccgcgcggtgctgtcctagcctggcctagaagccgttcagcttcaccaggccggtgtggagcgcgcctgcgccgagcgtcgcgagcagcgccgcaagcgtgcccacgataatggcgatgacgccggcggtggaggatccgcgctgcgaggccggcttgtcctctggtgtgagcttggtatccccgctgaggttcgggcgcgccttcgagtggtcggaggtgctgcccagcggcaggcagtcggccagctcatcgatggtgtagaacatcgactcatccgccaccggcacgcagcccgcgtggaacgggatctcaacctcgttgtagagcatgcgcaccagggtgacgccctcgtcgttctggaacgcgtcccactggatgttcgcgcccatcggcgagaccttgtcgccgcgccacgcggagttgtcgtaggacataactgcgtctgccgggaccgccttctcggaaccgggcagcttcaaaagcgctgcgagcgggatgatggtctcggcgtggccgaagcggtactcggcggcgatgtcgccaccgttcgcacggtcctgcacgcctgtgatcatgtggtcgagtaggggagcgaagttgtcgtacgcgacagtttggccctcgattgccgggcccttctcgtagtagtcctccacatcgagcaggtaggcgaagaccgggccgtcggtatcgtccatgtactcgtggaagatccagccttccttcggcttggaggcctcgcgctcgagcgcgggggcgatgatgtagaggttgtagaactgcagcgcggcgtcgacaatcccttccaccgtcttcgagtcgtccttgcggccgacgaaggtttcttcgccggattcgagatcggcgatgaactccggggcaaagatcttgcccagcagtgtctgagcggctttctgggcatcgggctggtcgtaggcctcctgcaccttggcctcaagtacctcgccgtccttccacgccgagtacgccttgtagctgtccgacttcttgtccttgtgggcgtagagaaggtccttgcgggtctcgaggttgacggtgccgttgtcggtgccgtccaccacgtgcgaggcgagcgctgggttcacggacaacaggccgttgccgaactgctggccggactcgatcgcgcggtcctcgccggaggacatgaacttcaccttgtcgttgtcgcttgcgacgacgcggtcgaggaaggccgtgttgcgagcggcgttgcgcacaccgatgccgcgcagttcctcgcggccgaatgtggtcaggttgccgtagcctggctcgcccggaccggtgagttcctcgttgaccttggtcatcgcctcaacctgcgggatgagacgctcgccgagctccgtgagctggccacgctcctgcgcggcttggagcatctgctgcgctaagtcgtcgtacttgaagctggacaggccgcgggagccgtggcggttcaccgaggtggtgtaaatctgcgcaaagcctgccggcgcctcgctgtaggaagagatcggcgcggcgggggagtacggctgctttgtggagtagtaggtggctgcgtccgccgcggaagcggtggggacagcgacaagtggaacagtgattgctgcggctgcggcagcagcggttgcgcggcgggacatgggtgctccttggcggtgaagatgggaaactctgacagcgcaacggtaagaccacgagataacaacgaggtgaaccccgcgtgaacatcgcggggagattgtggcgcggccgcactctggggccggtaggataggggaggttctggggccaaaatcgcccccatttcccacatttttcattccgcgcactaccacttcaaggagcgttcgtgaccgagcccgccatcacccgcgacgattggaacaccaagcttgagctcgcgcagcagatgctgccgctgatcagccgcctgcaccgagagcacaacgtggctacttcgatccacggacgtctgttggtgggggtcaccgacatcgacgtgatcaaggcgcaccgctacgcccgccgcatcgaggaaaaggaactcccgctgcaggagacgctgccgatcctccaagagctggtcgagatggacttgggcaccgcgtccatcgacctgggccggcttgcccgcctgtaccgcaaggccgagaccaccgacatgcgcgcgtttttggaggagcagctcgcggacgtggtcggcacgtcctctgagctggaggcgcgcgacgtggtgctgtacggcttcggccgcatcggccgcctgctcgcccgcattctgatcgcccgcgaggcgacctacggcggcgtgcgcctgcgcgctgtggtggtgcgcaagaagggcgacatcgacattgtgaaacgcgcttcgctgctgcgccgcgactccgtccacggcccgtttaacggcaccatcaccgtggacgaggagaacgagatcatctgggccaacggcaccccgatccagatgatctacgccaacgacccggctgagattgactacaccgcctacggcatcgacaacgccatcgtggtggacaacaccggcgcctggcgcgaccgcgacggcctgtcccgccacctggaatccaaaggcgtggaccgcgtgctgctcaccgcgccgggcaagggcgacatcccgaacatcgtctacggcatcaaccaggacatgatcggcgacgagcgcgtgctctccgccgcgtcctgcaccaccaacggcatcaccccggtgctgaaggtgatcaacgaccgttacggcgtggtccacggccacgtggagaccgtccactcctataccaacgaccagaacctggccgacaacttccacaagggcccgcgccgcggccgcgccgcaggcctgaacatggtgctcaccgagaccggcgctgccaaggccgtgtccaaggcattgcctgagtttgccggcaagctcaccggcaacgcgatccgcgtgcccacccctgacgtgtcgatggctgtgatcaacctcgagctcgagcaggaggtggaaaaggacgaggtgaacaacttcctgcgccgcgtctccaccgattccgagctgcgccagcagatcgactacatcaactcgcccgaggtggtttccaccgacttgctcggcaccacccacgcgggtgtggtcgacggtttggccaccatcgcctccggtaagcacctagtgctctacgtgtggtacgacaacgagtacggctactcccaccaggtggtccgcgtcgtcgaggacatcgccggcgtgcgcccgaagatctacccgccgcgtaaggcagtctccgagctctaaagagctcggctagcgccgcgcggcgtgtgccgcgatagcttcgttgtaaacctccaccacagcttcggtggaggttttccagttccaccggagcgcctcggtgcgcgcggcggtggacatggatgagtgaaggggtgcgtcgataagcaactgctctaccgcggccgcccaccgcgcgtcgctttcctccggatccaccaggaacccggtttcgccgtcggcgacgacgaacggaaggccgcccgcgttcgccgcgaccaccggcacgccggacgcgaacgattcgagggccgcaaacccgagcgtctcggtggtggaggggaagagcagcacgtcgccggaggcgtaggcggcgcggaggtcctcgccggacaggtagccggtgaagtggatccagtcgtcggtgaagtcgtcccgcagcgcgtcgtaaagcgggcccgcaccgatgagcgccaagcgagcgttcggcacggccttgcgcagctcctgcatgatcgggcgggtgcgctcgaccgacttctcggcggagaggcggcccaccactgtcaccagcgggtcctccgggtggccgcccgtcaacctcgcgcgcatctcgcttgtgcgggcatccgggcggaagctctccgtgtccacggctttcggccacaggcggatgttctcgacgccgtagcctgcggctttatccatcatcggtcccgaggtgaccaggttgtattcgcagcggccgtggaaggtgcgaagcccccattccgagatcggcttcgcccagccgatgcccagcttgctggtgtactcgggcacatccgtgtggaacgacccgaccagcggaaggccctgcgcactcgcaatcagcgtggaccacccagccgtccagatcgggttcaccgcgtgcaccacatccggttcgaactgcgcaagccgacgcgctaccagcgggccaaccaggccaaactggatttccgggtagacgggcttaaagcttaaagacggcaccttcaccacctcgcaccccgcgtactgcgaaggtgcgtcaccggtggcgaagatgaggacgtcgtggcccatcgcggcgagttgctccacgtggcgcactgtccgggtgaccacgccgtcgatcttcggtaagaagacctcggtgagcagggcgatgcgcactacttttcgccctcgggcacgcccgcggactgcgcggaggtccacagggagcgcgccgggatcttctcgcggtcggcgcggtcggcgtactttcgcgccacgtcctcgacctcttggagcaggccctcggccaagtaggtcggctcgaggccgaggccgatgaaggtgtcattggccacgaacagctcgttctcagcggcctcgttgcgcgggttgggcaccatctgcacctcggcgccggagatctccgcgatcaggttggccagatcgcgcacgcggtgggtctcggtcatctggttgaagatcttgacgcgctcgccctttgccggcgggttctccaccgcgagctggatgcacttggccatgtcgcggatgtggatgaacgcgcgggtctgcccgccggtgccgtgaactgtcagcgggtagccgaccgcggcctgcatgaggaagcggttgagcacggtgccgtagtcgccgtcgtagtcgaagcggttgatcaggcgctcgtcgcgctccgtctgcggggtgtgggtgccccagatgatgccctggtgcaggtcggtgatgcgcagggagtcgttcttggcgtagtaggcgaacaggttctggtccagcactttggtcatgtggtagaccgagcccgggttggtggggtagaggatctgctgctccacgatgccgttctcgccggcgtcgacttggatgtccaggtagccctccgggatctgcatgccagcggtgccgtagccgtagacacccatcgtgcctaggtgcaccacgtggatgtcaagacccgactccacaatcgcaaccaacaggttgtgggtggcgttgacgttgttgtccactgtgtagcgtttcgtgcgcggggtcttcatagagtacggcgcggcgcgctgctcggcgaaatggatcacggtgtccggttgccactcgttaatgaaggcggaaagcccctcgtagtcctgcgccacgtcgatgttgcggaagccgatctccttgccggagacctccttccacgcctcaaggcggtcctcgatggacgcgatcggggtcagagactctgcgccaagctcctggtcaatcgcgcggcgggacaggttgtccacgatgacgacctcgtggccgatatcggaaaggtgcagtgacgcgggccagccgcagaatccgtccccaccgagtacagcaattttcacgtgaacactccagactagaaccgagaactaacgtctagacaacgttacccggggtctgacacccctgcctgccaagtgctgggttcggggataaagtaacccttgattttccgtattcgcctgcactaattgaggttgcgcatgcttacccccgccggttacgccgttatatccctcgagacaaccgggtttggaggcgccgaccgggtgattgaggtcggcgtggcgttgctcgccccggacatgtccccggagcgctcgtggtcgacgctggtcaacccgggccgcggcatcccgagcagtttctcccacgggttgagttcggacgatgtcgcggacgcgccgcgcttcgagcagatcgctgcggagctggccgggctcatcggcgggcgcatcccggtggcacacaacgccgaagcggttcagcgcttcctgcgcctcgagtaccgccggctgggcgcggacaccggttttacagacggtgcctggctcgacaccgccgcgtacgcccagcggttgtggggcatccgctcgcttaacgacgcactgttgcacaccgccctcgcgcccaccagatccgcctccgcgctctccaaatccgagtcgatcgccgagttgttgcgcgtgatttcccgcgcccacggcatctcgtacaccgaggtcgaacgcctgaacgttgacgccaacggcctgcccgccggcgcgccgccgaagccgcgcgacggggaaggggccgacacgtgggatagctaccgcagcgcgctccgcggcgcggccgctgaacgccccgtcgaccttgatcggatccgcgcgctgcgctcgcggccggagcttgcgggcgtgagcccggaggacgtcgccgctgtccacgacgagttgctgcgccagttggcggtcaaagcgtggttcgacggggtggtcaccgacgcggaacgtagctcggtcgtggccctgggcgaggtgcttggcgcggacccggacgcggtggcgcggttgttcgccgacccagagccccacgagcacggcccgtgggtgccgcttgccgcgggatcacgcgtcgcgttcgccggtgtgctggatttgccgcgtgaagagtgggaggaaaaagccgcgtcggtgggcttgctggtcggggacgtgactgagcagacgagcgtccttgtcgcggcctacccccggggcgaggggccgaagatccaccgtgcccgcgagcttggcgtgccgatcattagcgaaacccgcttcgcccagatcgcgtctggtctcgagccggcctccgcgatcgctgacacggtgtcggtttcgccgtgggcgtcgtttgcgtggttgaacgaggactgggccactgctgccgaggtggccgaggcgtggatcgagcagttcccgtcgcgcccgctgcacgagatgagccacgcgttgaccccgaacaccccgatcgagttcccgccgacaggggtggacaaggcggtctcgcgctggaccgagcgctttgagcggctcctcgacgcgaccgcgtacgacgtcaaggacctcccgggggtgggaacgaagaagctccgcgccctggttgaagcagtggtgcttaccgcacgggacaccgcggaggttgccgtgcccggtctctacgtcgacaacgcgggtagcgaggtgccggagtggaacgccgacacggcacgccacgacgcgctgcacacccagatcaccgtgctctccggatggctgacgctaagcggcgctgcgctgccagagggcaccaccagctcgtcgctgccggacatgccgcagcctgaagcaagtgcggacgcgctgcgcgcactattcgccgcttgcgttgcggagcttacgcacgtgtgcgcatccgacgagcgctacaccgtcgttgccaaacgccgcctgctcggcgacacaacgctcgacgagatcggcacgaacttcggtgtgtcgcgcgagcgcgtgcgccagctgcagtcgggcatgctcgaccacttcaacccgaccagtgggctgtcgcgggccgtcgccaagcagcttgcagccctgctcaccccgctcgcatccgtcgagcagaccaaggcagcgatgcccgccctgttcgaagtcaccgacttcgacgtgacatacgaagagtacttccggcgcttgttcggagcttggcttaacgacggaacgtggatcaccaccaccgatttcgacgacaccgcccgcgctgcgattcggcagcgggatacgggctacggggcgtcggcaatcgcacttgtggcgggcgatcttggggtcgacccggagcttctgactgcgtggctcagcgaagcacctggcctgctcgtgttgccggacggcgagcacgtggtgatcgactccagccaccaagaccgcgccgctgcggtcctgtcgatccacggcgcgccgatgacgacggaggagattgttgacgcgctcggcaacggcgccaacccgcgctcggtgggcaaccagatcgcggtggacgatcgcatcatccgcgtcgcgaactccctgttcggcctgcgcgaatggggccaggaggagttcaacaatatccacgagtggattggcaaacgcatcgacgaatccggtgggcaggtgccgctcgacgaactgatgagtgccgcgccggcgctgcgcatcagcgagaactccgtgtaccagtacgcaacgagcgtccactacgagcttgagggcgggatggtcaagcgcaaggaagcgacgggggaggcgatcaatgcggaccctcaggagtcgcgcgacctgtacttccgcgatggtgcgtggcaccttttggtcaccgtcaattccgagcacctgcgcggttccgggttccaagtgccgcgcggcgtgccgggcatctacagcgtgcccgtcgattcctacgtggatgtcccgagccggctggggccgcaggcggttcgcgtgaacaagctgcgccagccgagcctcgccactatccgccggttcctcgaggacatcggggcgcgggagggccaccgcgtgtggcttcgtttcgacgccgacctggacaacccgaacgcgttcgacgtaacgatggcgcccgaggcccagttcgacggcggcgaggcgggcaccggcggactcgccgcgcttttggaccggatggcgctcgacccggcgctagcgtcggatgaggcgtcggcgatgcgcgccatcaacgcggccctcggcctggatccagacgcgccgcgccgccgcgctgccgccatcttcggacaccgccgccaagacgacctcgcggacgtgatccgctcgctgtagctagaagacgagctcgatcgcgcggatgacggagtcccacagcccagtcaccgagtaggagagctgggtgatggattcttgccacgacgtgggcaaccaatcattggcgaggttagaccatacgaatcggcgggtgtcctgcgcgccgaggtggaagtttctgttcagcgtcgagctcaaaggcgtcatgtcggccataataagccctcagctgaaaaacctctaagacgcctcgacggcgtagtacgtctccacgtactccacggccttgtccaacgcgtcgtggatatcgtcagcctcgaccgtgggcagtttctccgagcggaactgcggccccatgttcttgaacgggctgatcgtccgcccctcgcgcttcgcccgctcaattgaatcgaatagctctttcattcgacggttcacaactcttacgtgcagctggttgtacgccggcggcgcgaacgggttctcccacccgtacacctcggaaacgagccggccaatccgcggatcgaaaacgaagacagccacagggaacgtggacgggtccttcaggttcggctggaattcaacggtgaacgcggtaaacaagtttggtcccgcgtccatcaccgcaatcgtcgccgtcgaagggtcttcggcctcgaacttggtaccggtctcgaggcggaagttcggaagacccggatcgtggatctccagcgtctcctcgtcgattcccttcaccacgagcgcgacagtgttcacgacttcagtgaaaccgtcgacatcaaaccatgcagctgcgtgttccgaatggggttcgacgatcgagagttgtacctccggctccgagccttgccgcggtttaccgacgacgatgatggcagcgcagaattcgtcgaacccttcaccagtttcttttccgtagaacagtttgtacgtagcaaacgccatggtttccccccaagttttctgattccagtgtggtgcgttaggtgatctttcatcccccacggcgaactttagggctgcgttcgtgttgccacccggaaatgcgtgcacacttgagtggacgtgctggggctagacgaagatcagcccgagatgctgtgtcgtcagttcgtactcgccgggcccttttggcaaggaccgaatctcctcctgcgtttcgggcagtactgggatgatccaaccttgacgtgggtcaagaaccggggccgaggacttccgtgtcggaacaaacgtgaccaaacgagaatccgcttcgcctgttaactgaacggcggtggtggcctgtcgtaaatcctcaagggcggcagcggaggtggtgatgatgactagccgctcattggtatcgggggagaggttcgctgtgtgcacggacagggtgtccacatctacccgcgcgacgcgcctcggcacttcaaccagcttttccgctgaactgccgaaacccaacttgtcgaagaaacccatggttggcatctttccacccaccctgaaataggcggcggtgagtgggtagttattatgcgcggcagaatgactgccgcgaccggggtggattatgcgcggcagaatgactgccgcgaccggggtggattatgcgcggcagaatgactgccgcgaccggggtggattatgcgcggcagaatgactgccgcgaccggggtggattatgcgcggcagaatgactggtcttgagtaaggttcaacgcaatgatgtagtggccacccctcaagaattcagagaaaagcatgatctatgtggttcttggtgtagtaatcgcactgttcctttccttgtgcatcgtggcaatggggtatctagtccagtttttcgctaagcgaagggtgctttctccataccgtttcttggccacgatggttttactagcgcccgtttttctgatttacgatttacttagcgatgggatgtgtaatggcctttttaactatgcggtcagcggctacttaattacggcagtcatcatcagttccttagggcgcatctttgcagatggcctcagcgaagcgcggcaataggagtgtcaggccaccatttggattatgcgcggcagaatgactgccgcgaccgggggagggcgtgggcgtcggcaagcaactgctcccttgcgcttgcaggtacggtcgacgcatggctgacgcgaaactcgaacgagtgtttacctatccgtttggcgacatctaccgaaactatgtagccaaggttgagcggaaagaaaggacccgtgagcagctcgatgacgtccttgggtggctgaccgggctgtcgccgacggaactcgacgcggctgccaagtccggtgaaacgctccgcgactttttcggatgcgtcgaactgaaccctgccgcagagcttattaccggcagcgtgtgcggggtgaaggtccaagacgtggaggatccgctcatgcgcaagatccgccagatggacaaggttgttgatgaactcgcgcgcggaaagaaagttgaaagcatcaaacgcagcgccccggtttaaggtgatgggcatgacgcagcccgcctatgaaccagacggcacctcctaccgcgccgaactcattgtcccgtacggcgcgggtgacttggtggtggcgccggctgcggaaaccatgcccgacccgctggctaagggcaaccggctcacgtggccgagtgtgaaactcattcttaagcgcatcgtcttagatttctccttcgatgcgatggtggatcgtgcggcgactttgacttactacacggtgttgtcgatggcgccgatgctgctggccacgtactccgtgtttagcctcttggtgccgcgcgacgagctggcggctgattctgtgatggccgacatcattcggatgtacgtgcccgaggcgttgcaggatgaggcgatgaagctgctgctcacgattatcggcacaccgacgcaaagcacagtcgcgctggtgatctcgctgttgatttcgctcttgtccgcctccggctacgtacgctcgttctcccgcaacgcgaatctgatctacgggcgaacggaaggcaggaacatcgtggtcacatgggtgaccatgtggctgatcacgctggtgctggtggctggcgccattgtgattgtgctcggcgcgctgctgaatgaaagcgtggtcaacgcggtgttgggcccgatcgcgcgcccgctcgggttgcagggcgtgctggagtatctcaacagcatcttcctgccggtgtgggcgtacctgcgcggcccagtcatcgcggtgactgccatcgcgctgatctcggtgctgtactttttcgcgcccaacgtgcggcgcggcaggttccgcttcttcacactcggatcctcgctggcgctgattgtcatcactcttctgtgggtggggttcggctggtacctcgcggttttcggcatccgcagcccgtacggggctttcggcacggtgctcgccgttctgggtttgatttgggtgatgaacattgttctgctcgaaggcgtcaagatcgacgcggaggtcctcagagcgaaggagctgcaagtcggcatggactccgcgcgggtgatccaggctcgtccgaggtcgaacgcgggcgcggcgtggcgggcgcaaacccagcggtggacggatcgcacggtcgcggaaattcagaaagagcgcaggtagtctgggcgggcatggcactgattgatccccgcacgaagtacccgaagacctttgacaaggaagaccgccaggaaaaccccggtcttgacgtgaagatgaccaccgagccggatctgggcgcggacacgtacaccggttctggcaagctcgagggccgcaaagccctgattaccggcggtgattccggcatcggcgcggctaccgcgatcgcgttcgcccgcgagggcgccgacgtcgccatcgcgtacctgccggaggagcaagctgacgccgaccgcatcatcgcgctcatcgaggaagccggccgcaaagccgtggcgatcccaggagacctgactgagcttgcaacctgcatcgacaccgttaccaaggccgtcgacgagctcggcgggttggacatcttggttaacaacgcctcgcgccaggtgtggaacgacggcatcctgaacatctccgatgaggatttcgacgccaccatcaagacgaacatctactcggcgttccgcgtgaccaaggaggcggtcaagcacatgcagccgggctcgtcgattatcttcaccacctcgatccaggcgtatgacccgtcgaaggagctgctcgactacgccatgaccaaggctgccttcaacaacttggcgaagggcctgtcgggtgagcttctgccgtcgaagggcatccgcgtcaacgccgttgccccgggcccgatctggacggtcatccagccggcggagggccagccgcaggaggtcgtcgacgagttcgggcagggctccaagatcggccgcccgggccagccggcggagctcgcgggcgcatacgtcttcctcgcgtccgaagacgcctcgtacatctccggcgagacgctggccgtcaccggcggcgcggtcactccttaaaacccgcccgcagggaccccgcgctttagtagggtcaacctgtgagtgatttgaacagtgttcaaggcgtcgatgtccaaagcatcgacgccgcacacatttggcacccctacgccgagccgggcctgttcgcgtacccggtcagccgcaccgaaggggtgcatttgcagcttgctagcggcgccctcctcatcgacgccatgagctcctggtgggccgccatccacgggcactccaacccgcgcctcaccgccgccgcgaaggaccagatcgaccgcatgagccacgtcatgttcggcgggctcacccacaccccggcagcgctgctcaccgaacgcttgctggacctcaccggcggcaacttcagtcaggtgttctactccgactcgggctcggtggcggtggaggttgccatgaagatggcgctgcagtacgcccgcggccagggccatcctgagcgcactaagtttttgacgtggcgctccggctaccacggcgacacgtttgccacgatgagcgtgtgcgaccccgatggcggcatgcactccttctggggctcggcggtcacccagcagcggtttgcgccgccaccgcccgtgcgaggttcatcacccgtagaccagcgcgcctacctcgagcacttcgccacgcttgtcaccgacgacgtcgccgcaatcatcatcgagccggtcgtgcagggcgccggcggcatgcggttccatgaccccgagctggtcaaggggctcaggcagcttgccgacgcccacgccatccccctcatcgccgacgaaatcgccaccggcttcggtagatccggccagcttttcaccaccctcgacaacggcgttgtccccgacatcatgtgtgtgggcaaggctttgaccggcgggttcatgacgctcgccgcgacgttggccaccgagaagatcgccgccggcatggagccgaaagcgctgatgcacggcccgacgttcatggccaacccgctcgcctgtgccgtggcggccgaatccgtggcgatggtggcagaggggcagtggcgcacccaagtcgccgcgatcgaagagggtctgcgcgagggccttgagccgctccggaacaaccccggcgtcgcggacgtgcgggtgctcggcgccatcggcgtggtggaaatggaacgcgacgtcccgatgcgggcggcaaccgaggccgccatggagcgcggcgtgtggattcgcccgttcggcaggctgatctacaccatgccgccgtacatctgcacccccgagaacatcgagaccatctgcgccggcatcgcggccgcagtcggcgtaagcaccaaggagtagtaccatgatcgtcgctataaccgggacaaacaccgatgtgggcaagaccgttgcaacggcggcgcttgccagtgtgctaaagagcaagggcgtcgacgtcgtcgccgccaagccgattcagacgggggaggccccgggcgaaggagacgcatctaccgttgagcgcctcgccggtattgagacctttgagcggtggcgctacccggagccactcgcgcccaacttggcggcgcggcgggcggggatagcaaccccgccgcttcaagaggtggccgagtgggtgcgcagcctcgacgcgccggaccgcgtggtgttggtggagggcgcgggcgggctcctcgtccgtctcgccgacgactacaccctcgcagacctcgcctctgcactcgccgccccgctcgtcgtcgtcacctcgctggggctcggcagcctgaacctagcggagctgacctgcgtccaggcgcgccagcgcggccttgcggtgctcgggctcatcggcgggatcatgccggagaacccggacctgcccacgcgactcaacatcgaggagctgtcgcaggtgacgggcgcgccgctgtggggttcgatccccgctggcgccggtagcttgaaccagcgtgagttcgcccaggtggcggccagtgcgctggacgcggcgcaggtgctcgccgccttccgctagtcggcgacgaggggctccatcgtcagctccgggtgctccttctccacgaaagccagcttccacttgtcgccgaacagcgcgatgagctcgccgtcggagcgggtgaagatctccacgccgcgctggcggcccagctccggagcactttcggcatcggtgcggcgcgcaaccgagtaggggatcggctccgtgacggtttccacgttatactccagctcgagtcgggcctgcatcacctcgaactgcattgggccgaccgcggccataacgggggcggcgtcgccgcgggcgtcgttgcgcaaaatctgcacaacaccctcggagtccagctggtccaggcccttgcggaactgcttgtacttgcccaaagacttcgcgcgcagcgtgcggaagtgctcgggcgcgaactgcggcatcggcgggtactgcacttttttacctgcgtagatcgtgtcgccaggggcaagcgcaccagcgttgacaagaccgatgatgtcgccgggaaaggcggtttccacggtgtcgcgagaccgtccgaagactgtcagcgcgtacttggtggagaagctgcggcccgactgtgcgtgcgtgacctgcataccgcggtcgaattcgccggagacgacgcgcatgaacgccagcgtgtcgcggtggttgcggtccatgccggcctggaccttgaacacgacaccggagaaatcgtcgccgaccgagcgctcgttctccaaccccgcgcggccttcgggtgcgggcgcgatggcgcaaagcgtgtccaagatctggtggacgccgaagttcagcatcgcggaggcgaagatgatcggggaggtgatgcactgctcgaacagctgctggtcgtgcacggcgccgtcggcaagcaaaagctctgcctcctccagcgcggtttcccacgccgctccctcgcgcgcgagcgcctggtcgggggagaagtgctcctcgggcgcgatggtggaaccgccggcggtgcggatgaagtggatgtactcgtcgacgtcgccgtcggtgttcacgtgtgcgaggccgcggaagtctcctgcctcaccaaccggccagtacagcggcgttggctgcaggtcgatctccgtgacaatctcgtccaccagctcgagcggctcccggccgacgcggtcccacttgttaatcacggtgataatcggcaggccccgggccttgcacacgcggaagagtttgagggtttggggctcgaggcccttggcggcgtcgataagcatgaccgccgcgtcgaccgcggagagcacgcggtaggtgtcctcggagaagtccgcgtggcctggggtgtccaccaggttgatcacatacggttcgccctcgtggccctcgggcgcgtactcgaactgcagcgccgaagacgcaacggagatgccgcggtccttctccatctccatccagtcggacacggtcgacttgcggccggccttgccgtggacggcgccggcctccgagatcatgcgcgcatgcagcgccaacgcctccgtcaacgtggacttaccggcgtccgggtgggcgatgacggcaaacgtgcggcggcgtgcggcctcggcggtggtgctcatggcgtttcagcgtagttgctggctgatctcaatcccagccaaggtccctggtgccgctgccggtcaggtgccgcccgagataggggatgagaaagttgaggtatccgcgccgggggctgtagataagctcgcgcctgatcaaccggtcgcgcaccactgacagctcttgcgtgcgcttgcccatgtgccgggcgatgtcagcggaagcgacagcttcctggccgcgttgaatctccgccatcgcagccagatacgcccgctcgccggcggggacgggagacaacgccgggtcgtgaacgagctggccgagggaatcgagaacggtaccgcgaaccgcgataatgtcgtcgaccgaagctttggtgctgctggccgacacacgctggaagacgtggtagcccagcagctgaaccagaaacgggtagccgcgggtgaaccccaccgcttcgttgagcgcgtcgccctcgaggtcgaggccgccagcggcagccgttgtctggagcacagatgctgtctctgcaggtgtcatcggcgccaagacagcgtgctgggcgcggcgcagaaatgtcgtgccggggtgctggagcaggcgcgccacaccttccggcaggcctgccgcagcgaacgctatgtttctgttgtcccggcgcagatcctgaaccgcagcggtcaggtgccaaagatcggtctggtcgacgctttggacttcatcgagcgtgatcagcaccccggatggcccgggtaacgcatcgcacagctcgtgtaacgcactggttaacgacggcgccggctccgccccttccgcggcggaggtggaaaagccgccgagacctgcgacgctaaccccagtcaccttacggcggtttgggttcgactggcgcagcctctggagcgcacgcggtatctccgtgtcaacgagcggttggatgaggtcgtaaggctgggctcgaacatgcatccagccgcggcgcgctgcttcgtcctccagctcgttgagaagcactgttttgccgattcccctggggccagagatcaacagcgtccggcgcggatcgcctgggccagcttcgagggatgcgccgaaaccggatgttaacgcgtcgcgaccacctaggatggcaggggagacaccgaaggtgggaacaaacggattcactagacacctcgtcgcgcagttggtcgttgttatctttgttatacagcaccgcgttgttatatttgttatattcgcgacatggccaatgacacgtcaacaatcggcattttcctcggatccgtccgcgagggccgcttcggtgaagcggtcgcgcactgggtcctcgagaccgcggccgcgcgcggcaacgggttcaactacaccctgatcgacctcggcgaattcgatgtcccgcacctcgtcgccgcaacgccgccggggatggcgaacaagcagtacgacgacccggctgtcgccgtgtggtcgaaggccgtcgacgagtgcgacggctacatcttcgtcacccccgagtacaaccactcggtgccgggaacgatgaagaacgccttcgactccctcggcccggagtggatgggcaagcccgtcgccttcgtgggctacggcgcggacaacgcgatccgcgcggtggagcactggcgcaccatcgtggcgaacttctccatgttcgacatccgcaaccaggtggcgctgtctgtcttcgaggacgccgccgacggcgcgtttcgcccgcgggagtcgaaggtggcgtcgttaagcaaggtgctcgacgacatcgaggcgcaactgagcgagtaactagcgggcgtggatcacgttctgcgccttcgccaacccttcggtgacaacgagctgcgccgcgtgcgccgctgcggcgatgtcttcctcgccagagatcggccccagcacccagtccggcactgcaatccccgccggcggccgcccgataccgatgcgcacgcggatgtagtcgcgcgtgcccaggtgctcggtgatcgatttcagcccgttgtggccgttctcgttgcctccaagcttcacccgcaccttgccggcgggcagatccagctcgtcgtgcagcacgatgacgcgctcaggcgcaatcccgtagcggcgcaccagcggcgccaccgcttcgccggagaggttcatatacgtctgcggcttgcagcgcgccacgccgtcgatcggcggcagctggtcgagcgccagaaagcccacgttgtgcctcgtcgatgcgtactccgggccggggttgcccagccccaccacgagccactccgccttcgtgcgcctccagaatccaaacacgccgcatactgtacccatgaaactgcccaagattatcgcggcacccatggccggcgggccgtccactcccgcgctggtcaacgccgtcagcttcggattcatcccgctcggcacgtgcaccgcggcgcaggcccgcaagtggctcgcgcaatgcgagccaccgttcggcgcgaacctcttcctgccgcaggaggagcccatgcttgccgacgtccacctcatcgccaactccctcaaccacccagtacccgccatcacttccgactacgacgagaagttcgcggccgtcctcgacgccgcacccgccatcgtctcctcgactttcgggtgcttcacggaacacgagatcgagcgcctgcacgccgccggctccgaggcgtgggcgacggtgaccagccccgccgagatcgctgaggccgccgccaggggagtggacggggtgattgtccaaggcccccgcgccggagggcaccgcgggacgtgggaccagcgcgacgacccggaccagcggccgcttgatgatctcctctcactcgtgaccatccccgccatcgccgccggcggcatccggggcccagaagacgccgccgcgttcgacgttccggtcgcgtgcgggaccgcgtttctgcttgccgacgaagcggggacctcccagcgcaaccgcgaattgctgcgctccgatgcgcccgccgtggtctcccgggccttctccgggcgctgggccagcggggtcgagaccgcgtttgtgagggagcaccccgacatcccgccgatctacccgtacctgcggcccatgacaagcgacaacgattactgcctcgtcggcgcggaccgcggcgagctcctcgcggctcccgccgcggttatcgaagaagcgttaacaccctaagaggtacctgcgattggtggagcatgaagctctccaaacttgccatcgcagcagctaccaccgcgtccgcgcagccggcggacccgaccccgcgcggcggcagcgcgatgtggctctaccaatccctcatgttggacgcgatgcaccgcttcaacaacgtgaacgggcccgacaagcacccgtcggaagtcttcatttccaacatgctgagctccttgccgttggcgatcatgctgttcccgctgcaggtcatcgccgaagctgagctcgcgctgtccagcaccttcgcacgttaagaggtgcgctagtaaatccgcgtggtgttctcgatagcgccgaggccgtcgatctccacgcgcacggtgtcgccgtcgcgcaggtagcgcttcgggtcgcgcgcgtggcccacgccgtccggagtgccggtggcgatcacgtcgccgggctccagcgggtacaagtgcgagatgaactcgacgagtgcagctggggtgaacacgaggtcgtcggtaagcgaatgctgcacccgctcaccgttgagtgtggtggtcagcgcggggcccggccgccacttggtgtccagccaggggccgaagccggcggtcttctccagcgacttgccctggtgccactgcggtgtgcgcttctggtacgtgcgctgggtgtagtcgttgatgatggtgtagccggcgatgaaatcctcgccgttggtcacgtgccgagcccgtttgcccaccaccacagcgagctcgccctcgtagtcgagcgtgttggcgttgaacgcgggcacctccgcgtcgtcgaaggcaccgatcagagcctcggggaatttgatgaaaagcgtgggcacgtccggctgctcgtggcccatctcttcgatgtgcttggcgtagttgaggccgacgcagatgatcttgcccgggttcgggatcaccggcgcgaagtcctgcggcgcgaaggtgatctcctcgccttcgtcataaccgccctcacgaagcagcgtgccgacatccggcgcgctcagcagcacagcccgcgagtcgttgataatgcgcgcggctttcgtggtgtccccggttctgatcgtggcaagtcgcattgcgctagcctagctcgcccaagatcaagtcggccgcattcgcggctgcgatggcgaggtccacctgctcctttgtgccgaagggtttgagcacgtagtcggctggtgccatgcgccctggcgggcggccgatgccgacggccaccttgttgtaggtgttaccgagcgatctggtcaccgacttcaaaccgttatgcccgtggtcgcccccgccggtgcgaagcttcacttcgccgagttccaaatcgagctcgtcgtagaccacgtacaggtcgccgggagagacccggaaatagtctgcgagcgcctttaccgggccgccggagaggttcatataggaccgggtgcgcgccagcaccacttggtcgcttgaggtgaggcgccctgcggcgagctgcgcgatctcggtgttggtcttcttgtgcggggaaagcaccgcgggcataggtaaaaccctggtcagcagttcctcaatcaccaccacgcccgcgttatggcgggtggaatcgtactgctggccagggtttcccagtccgacaatcaagatggtcacacgaccatcttagggttactcggaagcgccctcgtcgccctcgccgccgtcagcgatctcgacgttgtccgggtttgcctcgtcgctgtcagcaccggcgtccgcgccgccctcctcggcctcggcagcggcagcctcgaggtcctcgtcaacctgctcgaaggtgacgttgacgagcagggtctccggatcggagagcagctcagcgccggccggcatggtgacgtcggaagcgaagatctgatcgccgatttccttgccctcgatggacacgacgatctcgtccgggatggacagggcgtcgacctcgatctcgagctcggtcgcctcctggagcacgacagcgtcctgcgcagcctcgccctcggtgataaccggcacggaaacggtcaccttctcgccgcgcttcacgccgagcaggtcgatgtggtcgatctcgagggtgagcacgttctggtcgacgtgcttgaccatgcacagcagcttgtcgccgtcgacgtcgagctcgaggatggcgttggtgccgtcgttgcgcaccagcgcggtcatttcgatgcggtcaactgcgaagtggacgttatcgataccggactcgtagaggacgcccgggatcttgccgtcgcggcgcaggcggcgtgcggagcccttgccaaactcttcgcgcttctcagccttgataaccggaggagtggtagccatggtggttccttctttcaatcgaagggccgcgggcaaagaaaaacctgcgaccactgaacgtaaaaaatgtgctcgtcgagtgatcacagggaagaaatgtcctgtaaatctattcagatcgcgccgataacggctcactaatgagccctcgccgagacgactacaggctagcagggcgctgctgccagacaaaatggccgcttgcctgcaactcctcgtgctcctggccgagcggaatgcccgtgcggtcgcacatcaccaggctcacgacaaacccgatcactgtcgcggtgagcaagtacaccgtgatcgcgctggtgccgccagtggcttcgcgtaaggctgccgcgatggtgggggcgaacgcgccacctaagatcgcgccgagcgcgtacgagatcgaggcgccggaggcgcggatcgaggcggggaagagctcggcgtagaacgcgccgatctcgccgtaagtcaggcctaggccgattgtgaggaacaccagcgcgaacgtgattttgccaagtgagccggtgtttacgagcgggaagagcgcgaggacgcccaccgcttggacgatgaacccgatagcaagcgtgcgggtgcggccgatgtagtcggagacccagcccgcaaacgccgtggtgcacaaccacacagcggctgacgcggtcaccgcccagagaatgtcgccgcgctcaatcgcgagcccttccgtgtcggtgacgtagttctggatgtaaccgccggttgtcatgtaacccacggtgccgttggcggcaaagatgagcgcggccgcgaggaccaaaccggcgtggcgcttgaacagggatcccaccgggttggaggcagggcgcatctcttcaactaccggcgattcctccacacctgtgcggatccaccagccgaggaacgtcagcgcgatagacaagacaaacggcacgcgccagccccactcgataaacgcgtcgccaggcgcaatcaccgtcatcagcgcgagcatgccggacgacaggaggaggccggcgggcacgccgacttgcgggcccgcgccgtagaggccgcgcttatccaccggcgcgtgctccacggcgagcagcacggccgaaccccactccccaccggcggacgtgccctggagcacacgcaggacgatcaacgcggccggggcaagccatccggcggtctcgtaggtgggcagtaaaccgatcagcgcggtggcagtgcccatggtgaacagggtgaccatcagtacctggcggcggccgagccggtcagcgtagtggccggcaaggaccgcgcccagggggcggaaaaggaaggacaggcccacagtcagaaatgctgcgatggtggcggctgcaggacccaacggtccaaacatgactttgttgaacacgaggccagccacggcagcgtagaggaagtagtcgtaccactcgatggccgttccgatggtggtagccgcgatcacgcggcggcgctcgttacgcacgtccgtacgcctttaagaacgcgtccgtttccgcctcgttcgtcacggtgacgcggatgccttcagggaagactcggacgagcacgccgccttgggcgagctgatctgcaacctcctgagccgcacccggcaaccagatgaagttcgcttgcgactcgtcgattcccagctcgtccgttacccgcttgcgctgcgcgaccgtttgatggacgcgctcccgcagctcgtcttgcgcttccagggacgcgatcgcaccggcctgcgccacagaactgaccgagaacggcacagcgaccttgttcagcgcctcgatgaggtggcgcggaccgaacgcgtaaccgacgcgcgcaccagcgagcccgtacgccttggaaaaggtccggagtcctatcacgttggggtacctagtgattgcctctgtggcgatcggcccgtcggaggcggtgttgtactcgaagtacgcctcgtccagcgccaccagcacagcttcggggacacgattcatgaactcgtcgaactcatcgttcgtaattgtcgttcccgtcgggttgttcgggttgcacacaaacaccatgcgggtgcgctccgtaaccgcatctgccatcgcagcaagatccacgcgatggttggcggtcagcggcaccgccaccggcgccgcaccggcgatctgggcgaagatcgggtacgcctcgaacgaccgccacgggaaaacgacctcatcacctggaccggaggtggcaaccaccagctgctggcacagcgcggaggagccggtgccaacagcaacctggtacgcgcccacaccgaggtggcgcgcaagtgcctcgcgcagctccaccgcgcccatgtcggggtagcggttcacgcctgcgagcgacgcctgcattgcgtcgatcacgcttggaagcggcgcctcggcgcactcgttggaggagagctttactgctcgcgcgttgcgcacgcccggaacgtaggccggcagcgtgtcaaggtcgggcctgatcatgcgcgttacggtacaccgtggccgctacgaacagtgccactgaccacgcgataagcgcgaacaatccggcgcggtaatccggcagaaccgccatgagcaccagcacgagggcaaagtaggcagcgcacaggtagttggccaccgggtagccaggagcggtgaagctcgacgactcacctcggcggcggaagttgaggtgggcaaagttgaccgacgcccaggtgatgagctcggacccaaccacgacggcgagcaggatctggaagacgcgtccctcgaagaagtagttgagcagcaccacaacgcccataagcgagcagttgaacagcagcgccggaagcggcagacccttttgggtggtggcggcgaaggctcgcggggcctggccgttaatggccaagtcgcgcagcatgcgggaaccggagtacgtcatggtgttgcagaccgaggcgactgcggcgaggataaccaaattgagaaggttggccgcgccgtcgacgcccacgaacgtcaggacgcggacaaacgggctgacggaattgtccagctcgtcccacggggcgagcaaaaggatgacgccgatgccgccgatgtagaacacgagaatgcgccaaatcaccgagttgatggctttcgggatcgtgcgctctggatcctcggtctcgcccgctgcggtaccgatcgacatcacgccgccaaaggtgaatgtcacggccaccagcgaaaagacaacaccgctcacacccttcggaaggaacccaccgtgggcgaccatgttgtcgaatcccagcgcgggctcgggtccgagcccgagcaccagcgagagaccgagcgcaatcatggcaatgagcgcgaccaccttgataagggatagccaatactcggcttcagcgaagatgctcacccgcgccgcgttgatcaccagcacgacgagaagcgtcaccagcgcggtgacccagtgggggatagaggggaaccagaagtccaagaaggtgcccatcgcggtcagctcgatcatgccgaccacgatcgtggtgtaccaccagttccagcccgcaatgaaccccgcgcgcgggccgatgtaatcgcgggcgtaggcggcaaaagatcctgaaaccgggtgcgcaacggccatctcgccgagcatgcgcatgagcgagtacaccaccgcgcccacgacgaggaaggccaacagcaccccgggcccggcgtacccgatggattccgccgagccgagaaagaggccggtgccgatcgccgaacccagcgcgatcatccgcaactggcggcttttcatcccgcgccggagcccggcgtcgcggtcggtgagcgcgtcgccgttcgtcacgtcgcgctacgcctggccttcgaacagggtcgtgaccgagccgttctcgaagatctcgtggatcgtcttcgccagaagcggagcgatcgagagcacggtgaggttgttccagccttccgtggattgcggcagtgtgtcggtggtgatgacctcttcggcgccgcaatcgttcaggcgctcgcgggccgggtcggagaacacgccgtgggtgcaggcgatgacgacggacttcgcgcccgcctctttcagcacgccgacggcgccggcgatggtgccgccggtgtcgatcatgtcgtcgagcaggatgcagtccttgccctcgacctcgccgaccacgcggttggagacaactttgttggcggcgtcgatgtcgcgggtcttgtgcacaaacgccatcggggcgtcgcccagcatgttggcccacttctccgcggtcttcacgcggcccgcgtctggcgaaaccaccacgaggttgtccagcgggtacttggacttgatgtagtcgaccaggatcggcattgcgtgcatgtggtcgaccgggccgttgaagaaaccctggatctggtcggtgtgcaggtcgaccgacacgatgcggtctgcgcccgctgcggtgagcaggtcagcaaccaggcgcgcggaaatcggctcgcggccgcggtgcttcttgtcttggcgcgcgtacgggtagaacggcaagatcgcggtgatgcgcttcgcggagccgcgcttgagcgcgtcgatcatgatgagttgctccatcagccacttgttcagcggctgggcgtgggactgcatgacgaagcagtcggcgcctcggacggactcttcgaagcggatgaagatttcgccgttggcgaagtcgcgcgccgtggtgggaacgaggtcgatgcccagttctttggccacggcctcggccagctccgggtgcgcgcggccggtgaaaaccttcaggtccttgtggctttcagtcgagtatccagtcatggcgtgtctcggtcctacccttcttcgcgtgctcgctgtgcggccgcagccgcgtcggttcccggccggtttttctccacccagccttcgatgttgcgctggcggccttccttgatagcaagggctccagccggcacatcctgcgtcaccactgtacccgcaccggtgtacgcgccatcgcccaccgtcacgggagcgacgaacatggtgtcggagcccgtgcgacagtagtcgccgatggtggtgtggtgcttgttcacgccgtcgtagttggcgaaaacgctggaggcgccgatgttggactcgcgtcccaccgtcgcgtcgccgatgtaggtcaggtgcggcaccttcgagccttcgccgatcttcgcgttcttcgactcaacgaagccgccgagcttgccgcgggcaccaagttcggtgccggggcggatgtaggtgaacgggccgacggttgcctcttcgccgatcacgccgagctcgccctgggtgcgcaccacggttgcgcgcgcaccgacttccatgtctttcaaagtggtgtcgggtccgatttcggcaccgtcgccaatcacggtcgagccccacagctgggtgttcgggtggatgatcacgtcgcggccgatctccacctccacaccgatccacgtggtgtccgggtcgatgacggtcgcgcctgcgcgcatcgcacgctccaccaagcggcggttgagctccttgccggcggcagcaagctgcacgcggtcgttcacgccggctagctcgcgggcgtcgggggcgatgaacgcggcgaccttcttcccctcgccgcgggcgatgcccagcacgtcggtgatgtagagctcgccttgggcgttgtcggtgttgaggtgggtcagcgcctcgcgcagcacggcgccgtcgaacgcgaagacgccggagttgacctcgcgcacccggcgctcgtcatcggtcgcgtccttttcttccacgatgcgctcgacgtcgccgtctgcgttgcggatgatgcgcccgtagccggtcgggttctcaaactcgagagaaagcacggtgactgcggcgtgctcggactcgtgcttttccaccagcatttcaatggtctcggcggtcaaaagcggcacgtcgccgttggtcactaccacggtgccgtcgaaatccgggatggcgccgaggccgatctgcacggcgtggccggtgccgttttgttcctcctgcacggcctggcgcacctcgatgcccatctgtgtagcgatcgcctcaaccgcgggggagacctggtcgcgctggtggcccacaaccgccacaaggtggctcgggtggacgccagcggcggcgtgcagggagtgggacaacaggcttcgcccgccgatttcgtgaagggtcttctggcggtccgacttcatgcgggttccggcgccggcggccagaacgacgacggcgcgttgctgatcaggcacgtgcggtctccttgtgggggttgagggtttgtttttagggttccagcttaacgcttcgacacgtctttcaagcgcgtcgcaccgagcacgccggcgtatcccacgaccgcgaggaagaccagggcggcctgcggcccgagtaccgaaactgccgacgacaccgcgccgacaaccagcaacacaacgcccatcacggtgttggacgcgccggtgatcatggtgcgcttgtcgccgtccgccatgtccaccagatacgtcttgcggctcaccctcaccgccgtgtgggcgaggttgaccaggaagaacccgagcggcatcacccaggcgttcactccgccgggtgcgaggcgggcgctcgcaaccagcgcaacgatgacggttgacgcgatgcctgcggcccaagccatggtgcttttcgacgacctgtcggagaacttccccgaaatcctccctccaatcagcgacgcgccgcccgatgcgatcacaaacgccccgagcccggtcaggtctgcgccctgctcgcccgccatgaccacgatgaacggtgtggacagcgcggtgaccagcatcagcgagcgcacgacgaggaaacgctgcaggtctttgtcgctgcggaccaaggcccacatttgcctcaagctctggccgtccttgtcagcgggctcggcctccggctcatcaatgccgcggaagaccagggacgcgaacgcccaggtagttgcgccgatgccgagcagcgcggcgagcgcccactgaggcagatcgttcggcagcaatgcgaggacaacgccgatcaccagggtaaaagcgccggcgagcgcggtcgcgcggccggtgatctcgccgcggcggcccttcgaaatggtgcgtccttggacgtctttgccagccaacgagcacagcgaacggaagatcgcgtgggtggccagcaggatgaggatggtggcgccgagtagggggccgtcgataagcaatgcgctcacagcaatcagtgcggcggcgagcgcctgcccccacgagccgatcagccacacgcgcttgcgcgagcgttgcgaggtcacccacgggctcaagatcgcctgggggagcatcgatcccgactcgcggatgggcaccaggaaagaggtgagcaccgccggcacgcccgcggagctgaacaaccacggcaggacggttttcggtgcgacgatctggtcgccgatgttttgcaggccgttcgaccagacaaagcggcgggcgttcgcttcctcgttacgcatagttgcagatagtagtatcattttgcccaaacctgcgagcttggaggagagcatgaggatgacacgacggacgtttttcaaaggcgctgtgttggcgaccgctgcggcggccgcaggggcggccgcatcctgctccacgcagccgaaaccgcgcggcgccgagttcgacgcccgcccgctgcgcatcccaccgctctacgaaggcgagctcgacggcaacgtccgccgcttcgagctcaccgcgcaggagggcgagttcgagatcatccccggcacgatgacgaaaacctgggggttcaacggcccgtaccaaggcccgacgctctacatgcgccacggagagaagatcgagatgacggtgcgcaacgagctgccggaggccacggtggtgcactggcacggcatgcacctgccggcgtcggcagacggggggccggcgctgatgttcgatccgggggagacgtggtcgccgtcgtggacggtcgaccagccggcggcgacctgctggtaccacccgcacccgcacgaaaaatccgcgacccacgcctaccgcggcctcgccggcggccttgtggtggacgacgacgagtcgatcttcccgggccttcccaacaactacggcgtggacgacatcccggtgattatctcggacgcgaacttcaccgaaggcggccaactggatgaggacagcggctgggtcggcgacacggtgatggtcaacggcatgacgcggccgctcttcgagccgaccacgaggcgcctgcgcctgcgtgtgctcaacggctgcgtgctgcgcttccaccacctaaccctgggcgtgccgttcacggttgtcgccaccgaccaggggttcatcgagtccccggtcgaagtcgacggcgtgctgctgagccccggtgaacgcgtggagattgtcgtggaccttgagccaggaaaggagctgacgcttacaagcgacggcatccccaacctcggcggcctgtccgacaaggacaccgcgaagacgttcggcttcccggatcagttcgatctactcgaaatcgccgcgccgccggcggacgcgcccgcgtccccgtcgctgccggagaagctcgtagcgttcgacgtgcccggttcggccgtcgtggagcgcgagttccgcctcaacggcatccagatcaacgagcagaccatggacatggatcgggtcgacttcgtggtcgaccacgacgggccggagatctggcacgtgaccaacgagaacgacgacatgccgcacaacttccacatccacgacgcgcgcttcgcggtgattggggtggagaacggggagcttgcgttctcaacaggctggcacgacacgatcagcgtgccgccgctttccacagtgagcttgctggttgagattggctactacccggatccgagcttggcatacatgtaccactgccacatgctcaaccacgaggaccagggcatgatgggccagttcgtcgtgacgaagccgggggagacgccgaaattggagcgccccggcagtcactggcagtaggagcggagtcaccatgcagtcagagacgctaactgtcccgattacgcggctggaggcgttgtcgatcttggagaagccgtctatccaactcggctagagcggcgagaagttcgtcctctaactcggcattgtcctcttgctgtcggcgagcgctgaacagctcataacgctccccagcaagcctgtctgccgcagatcgtgtaattcttcctcggtctttgagaggctcccgctcattgaactcgatgaagcgatcagtcttttctagccagtcactcatatggatgaccttgcggctctctgcttggaactgggcatagtccagaaactgactcaccagcaggttgaggtgtcgtagctcatcggcggtcagatagttcttggccaccgtgacatcgcgtttgctgacccgcttccccttccagctagtcaggccaaggttatcagcggcggcatcactgcgggtggcaatgatttcgctagcggtgaggcaagtaatcgcgtaatgaagcttgtcttgaatagttgcgtagatttggtgggttcgcggtgcgtccttgtcatagtcgtccgccagggaaacaatgtttcgaagctctagatacaagcgtgcctcgtttgaacgaatgtcccggatgcgttcgagcaactcgtcgaagtaatccaccccgcggggatccttcaacttctcatcgtttagaacgaaacccttaatcaagtagtcctgcaatatcgagctcgcccacgaccggaattgattgcctcgtggtcctcgcacgcgaaagccgacggccatgatcgcgtcgagattgtagtggtcgagcgaacggttttgaataccctgaccttgcacctttcggaacttccgaacaaccctttcgcgcctcaactcccctgaattgaagatggacttaaggtgctcgcttacgctcgatcgcgcgacgtcaaaaagctcggccatttcagcttgggtcatccacacggtgccgtcaataaggcgaagctggacttgagttcggccgtcatctgtgttgtagatgacgaattctcccagttcgtcccgctggatttcgggttcactcgcagccaactttcgcttcaccctttcgcagtcaaaactagtgtgacttgcccccgccaccccagatagaagcgatgctaagcactgctgggcagtgcgaaaccagtgcaactcaaaagttgcgaagcttccccaccaggactcgaacctagaatgacggtaccaaaaaccgtagtgttgccaattacactatggggaaatgcaattggagagtctagctcatggccacccgatcccaaatcccgggctgctccaaggccagtaagctggtcggcatggctcgacagcgaatgaccggcgcgcaacgccgggatcaactcatctccgttggtcgcgccgccttcgccgaacgcggctacgagggcacctcggtggaggagatcgcgagtcgggcggacgtgtccaaaccggtcatctacgagcacttcggcggtaaagaaggcctctaccgcgccgtggtcgagcaggagatggagaagctgaaaggctccatcacgaacgcgattcaggaggggcgctggcgcgagcgcattgagcgcggcgtgttggcgcttctcacgtacgtcgaggaggacaccgacgggttcatcattttggcccacggccagctcccgggtggaacacgaacctactccacggtgttgaacgaagtcacggcccaggtgtcgtacctgttggcaatcgcgtttcagcaccgcggcctcgacgaggacgcggccacgctctacgggcaagcgctcgtcggcacggtgtccaacaccgcgctgtggtggctggatgagcgcagcccggataagcactccaccgcgcgccacctggtcaacctggtgtggaacggcttaagcggcttggaagcgctgccgcatgtaactcatatagctgaggaagagaaggattgatgacggatcagaccctgcccgcgctcgcgggagtgctcaccgccgcccaagcggacccgaagctgaaaggcctttcaagccgcatcggcgacgagtcgctgcacatcaccgcccccgatcaggcccgctcctgggtcgccggaacgctggcgcgcgaggtgccgctgcttgtggtcacggccaccgggcacgaggcggaagaccttgcggcggagctgaaagcactgcttggcgacgccgccgtggccgaattccccgccttcgaaacactgccgcacgagcgcctttcgccggccccggacgtggtgggccgccgcgccaaggtgctccacgagatgccgaaggtggtggtcgccgccgcccgcgccgtgtgccagcccagcctgcccgcagttgccccgatcaccctcgagttggacgccgagcgcgacttcaccgagctcgtccgcgaaatcgagcgcttcggttaccgccacgtggacatggtcgccgcccgcggcgaatacgctacgcgcggcggcatcgtcgacgtgttccccacgacgagtgcgaaccccgtgcgcgtggagttctggggcgacgaggtcaccgacatccgcaccttcgcagtcgccgaccagcgcaccatcgacgaggtcgcgcgcgtctcgctttaccctgcgaggcagttgcttatcgacgacgccgtgaagtccaaagccgacaccctcgcccgcgcctacccgtcgaacccgacgttggtctcccttctgacgcgcgcgtccgaaggcgtgcacgccgacggcgaggagtcgctcctgcccgcgctcaccgacgcgccgtggtcggtcctcccagaactgttcgagcagggcatcgtccttgtgaccaacccggagaaggtgcgcgcccgcatcgccgatctggaggcgacggacgtggagttcctcgaagcgggctgggaggccgccgcgatgggcgcggagggaccagtcgccgtggaggggctcgatgtctccgcgtcgtcctaccgctcgtacgagtcgctggctgtctccgcgcgcaaggccggcaacgcttggtggacgtatgctccgcccggcatgttcaccgccgacgaggccgagacgctgccgctcgagttcgacaccgcccccgcgccgaagggcgaccagaaggcgattgagcagctctacgcaacgctcaagctgcacgtgcaggacaaccacggcaaggcagcgttcgtggcgccggcgaagggcacggtggagcgcaccgcggagcgcctgcgcgagcacggcatttccgcccgcatcgccacccctggccttgaaccggtcgacggcgcggtgaccctctaccaggccctgtcccacggcggcgtcgtcttcggcgggccgaaccttgtcgtggtcacggaaacggatgtcaccggcaaccgtgtcggggacatcggcggagcgaagcgccgcgcgccgaagcggcgcaaccgcgtcgacccgctggcgctgaaaccaggcgattacgtcgtgcacgagacccacggcatcggccgctttctgaaaatggcggagcggaccgtttccgattccaggcgcgagtacatcgtgctggagtaccagcctgctaagcgtggccaaccggcggatcagttgtgggtgccgatggaatcgctggatcttctctcgcgctactcgggcggggagcagccgcacctgtccaagatgggcggatccgattggaagagcacgaagcgcaaagcgcgggccgcggtccgcgagatcgcaggcgagttggtggagctctacgccaagcgccaggccgcacccggtcacgctttcgccccggacaccccgtggcagcacgagatggaagacgccttcccgttcgtggaaacggaggaccagctcaacgcaatcgaagccgttaagcacgatatggagcagccggtgccgatggaccgcgtcatcgtgggcgacgtcggcttcggcaagaccgaagtcgccgtgcgcgcggcgttcaaggcggtgcaggacggcaagcaggtcgcggtgctggtgccgaccacgcttttggcccagcagcactactcgaccttctcgtcgcgtatggacggcttcggcgtcaccgtgcgcgagctgtcgcgcttcacctcggccgcggacgcgaaaaagattatggcggggctcgcggacgggtcggtcgatgtcgtgatcggcacgcaccggcttttggcgacaggcgtgcagtggaagaacttgggcctcatcgttgtcgatgaggagcagcgctttggcgtggagcacaaggagcacatcaaggcgctgaagtctcacgtggatgtgctgaccatgaccgcgaccccgattccgcgaacactggagatgtcgctgacagggatccgcgagatgacctcgatcaccaccccgccggaggaccgccacccggtgctgacctatgtcggcccgcaggaggacaagcaggtcgcggctgcaatccggcgcgagctgcttcgcgacggccaagtgttctacatccacaacaaggtcgcggacatcgagaaggtcgcgcgccgcatccgcgagctcgttcccgaggcgcgtgtggtcatcgcgcacggccagatgtcggagcaggtgctcgagcagaccgtgcagggattctggaaccgcgaatacgacgtgcttgtgtgcaccacgatcgtggagaccggcctcgacatcgccaacgccaacacgctgattgtggagaacgcccagaacatgggcctttcccagctgcaccagctgcgcggtcgtgttgggcgttcgcgcgaacgcgcctacgcctacttcctctatccgaaggacatcacgctcaccgagacctcttacgaccggctggccaccatcgcccagaacaatgacttgggcgcgggtatcgccgtggcgcagaaggacttggagatgcgcggagcgggcaacgtgctgggctcggagcagtcgggccacatcgccggcgtcggcttcgacatgtacgtccgactcgttggcgaggctgtggaaacctacaaggcgctgatgagcggcgaggtcatcgacgccaccgatcagggcccgaaggagatccgcatcgacctgccggtggacgcccacatcccggagacctacatcaactccgaacggctgcgcctcgaggcgtaccgcaagcttgctgaggcccgcacggaggaggacttgcgcaccgtcgccgatgagatggtcgaccgcttcggcgcgctgccgcaggaggtcgagcacttgatggcggtggggcggctgcgtcagcaggcgcgcgccgccggagtctccgacatcttgacccagggcacccggatcaagatccacccggtggagctgccggattcgaagcaggtgcgtctcaagcgcctgtatcccggcgcgaacttccgggcggcggcaaaaacgctgcaggtgccgatgccgcgcgaatcgaaggcgatcaacagcccgaacctgcgcgacaccgaaatgctgcagtgggtggccgacttcatgacgtccatgctggacgcgccgcaagtctcagtcaccgggtcaaccgcggtggagccaagcggcgtcttctcgttcgagggctagttaggcgggcgtgtttcgcctgccgcgccggctgccgtatgattttcaaggcagcaatcgcccctatagcccaattggcagaggcagcggacttaaaatccgccaagtgtcggttcgagtccgactgggggcactacatttcttcgagcgggccgggggagcggtcgccgcgcaggcgcttcaccacgttctcggcggagatcaaacacatgggcacgcccacaccgggaagcgtcgtcgcgcccgcgtacagcaggttgttaagcttccgggagcggttgcgcccgcgcagaaacgccgattgtcgcaacgtgtgggcagggccgatcgagccgccggaccacgcgttgtagcgctcggcgaagtcagcggggccgagcgtcgcgcgcaccacgatgcgatcttcaagatcaacaacgccgcaccactcggcgatctgcgccacggccgcgtccgcgatcgcgcgcaccgcaacggattcctcgccgcggtacagatcgccgtggcctacggattcggccgctggcaccggcacgaggacaaagaggttcgtgtcgccagccggcgcggtggtcgggtccgtggcagacggcttggacacatagatcgaacgcgacgcgtccagagggcgtgacggctctggcgcgttgaacacggcgtcaaagtccgcgtcccactcgcgactgaagagcaggttgtggtgggcaagctggggaatctcgcccgcgacgcccagcatgaccaacacggtgcccagtcccgggtcgcgcggcgcgaaatacgcctcgtcgtaggtgcgcttctccttcggcaaaaggcgcgtctctgtgtggtggaggtccgcgcaggagaccaccacgtccgccgggatctcctcgcccccgaccaagcgcacgccggtcgcgcgacggccctcgtaggtgatcgccgcgacgtccgcgcctaagcgcacggccgccccgttctccctcgccagcgcctgcagcgcatcgaccaccgcagcgaacccgccttgcgggtactgcacgccctgcaccaaatccgtgtggctcatcaagtggtacatcgacggcgtgcgcgacgggtgcgaggacaaaaacactgccgggtacgtcagcatttgccgcaggcgcgtgtcggtaaaccgcttcgccacgtaggcgtcgagtggttgcgcaagcagcttgggcagcagaagcagttgcttatcgacgccccccacacccccagcaaacgtcgtatacaagaaccgctccagcgcgatcgtgtacgtgaacttcgctgaatccaggtactcgccgagtgccgcccccgcgccgggctcgatcgattcgaagagcgcctgcgcctgcgcgcgcccggattgcacgtccacgggctcgctcccctccggaaagaggcggtaggccggggtcaagtcaaccaggtcgagcaggtcttcggtgcgtttgccgaagagcgcgaagaagtggtcgaacgcgtccggcatgaggtaccacgacgggccggtgtcgaaccggaaaccatcaatggcctcgtcgccggcgcggccgccgacggtgtcaaggcgctcgaggacggtcaccgcgtacccttcgcgcccgagcagggcggcggtggcgagtcctgcgacacctgccccgataacgacagcgtgttgcgcgttggtgctcatggcagcgctcctttggtaaccgccgcgcgggcagtgatcataattttgcggctggcgggaacactcacccgcgcagcggccaagtcggcggcgtctgtttgctccagcatggtggtcagctccctgaacagcgcctcagcggccgcgacggcgccgcgcactggtgcgggcaagagcggtattgctgcgcgggcctcggcgagctcctcccggatgccggcggtgacagcggctttcgtcgcatcatcaggtgccatgccctccggaaggtacctgcgtccgagggtgtcgcggtcctcgccgaagtcgcgcaggaagttgatcttctggaacgcggagccgagcgcgcgggccccggcctccatccgggcgcggttcgccggagccgggtcctcgccgacgagaaacgcgctcaggcacagcaaaccgatcacctcagcggaaccgtatacgtactcgtcgaagtcttcccgggtgtagcgcacttggcgtatgtcgcggcgcatggaggcgaagaaggcgcggacgtgctcttcggtgaacccgcagcgccgcgcgctggcggcgtaggcgtgcaggacggggtcggtgtggaaccgcgcggcgggtgcggcgagcacagcccgctcgtagtcagcgatcaatgtcgccgggtctgcgcccgcctctagggctgtgccgtcgacgatctcgtcggcgacgcgcgccatggcgtacaggttgttaatgtcgcggcgggttgtggggggcagtatccgcgaagccagcgaaaagctcgtggaatacgaggcgatgacctgcgcggctgcgcggtcgcacatccggtcgtagcgcttcaaataaccggggactgtactcacccgtttcagcctagaggacgcgggcaacctctcccgccacgaacgccgagccggctcgcgcggggtggtaggccatgttgtagtcgcgggttgtggtgtcgataaagcccgcgacccagcgctcgttgtcgcgcgcgcaggtgttgtgtcctgcggagagcggcttcaggtcgaggtagacggcgccgatctcgcgggccgcgcggatctggttgtcgcgggtgagggtttccacccgctgcacaatcggcaccggtacgccgccgggcaggttgggcaccacgttgatcaggcagacgcgctgggcgccccacggctcggaaatagcgagcatgccgggaatgatgatccgggcgttcggcgccacctcgcggacgcgggccgcggctgcgtgcatgttggcaacgtagttgttctggattcgcggctggtcgaaccgggtgttggccgtgaacatgttgtccggccagtagtcgttgatgccgaccgcgaggaccacggcgcgggtgcccgggttgagatcgcccgcgcggatcgcgccgttgatgcggctcataaccgaccacgaggtcgcgcctgagcaggaccagtcacgcacgtcacgcccggtgcggtacgcgagctggcggggccagttgtccggcccctgcaggcacccgcccatcttggggtagttggcgaggtagtcggagctggccattcccgggatcttcgcggcccagtggcgctgctggtcggggttggcggcgaacgagtcgccgaacaccaccacgtcgcctaccggctgcgcggcagcggagggggcgagcgaccctgcaagcgctgcgacagcgacgagtgccttggccagacctttcaaacgcatgccggaaagcttacagtccgctgcgcatatcttcgtaagcggcgagcgctgtcttacgtgattctttgatgtccaccatcggttctgggtagagcggggtgtgtacctccggcacccagcgcgtgacgtaggaagcgtcagggtcgaacttctcctgttggagcaccgggttgaagatgcggaaatatggggcggcgtcgtcaccggagccggccacccactgccagttgaaggggtttgaggccacgtcggcgtcgacaagcgtgtcccaaaaccactcttctccgtggcgccaatgtatgccgaggttcttggtcagccaagaaccgaccaccatgcgcgcgcggttgtgcatggtgccggtggcccacagctcgcgcatcccggcatccacaagcagcaccccagtttcgccgcgctgccaggcagtgaggtgctcgaggtggacggcgtccggctccatatccgggttcgcgaaggcgtgcttagtgctgcccggcgcagcgcgcggcgtccacgcccactcgaactggtcgaattgttcgcgcacgttgcgggtctcgaggtcctccacgtggaagtaccggtgccacgcgaagtcccgccagatcagctggcgcaaaaaccccgcggtgtgcgggtgctctacagccgccgcccacacggtggcgggggagacctccccaaaacggaggtgggggctcagcccagaggtcgagcctgcgcccaaggtgtcgttgtcgtacgcgcccttggagaggaacgcctcgaggcggcgcagtgctgcgtcttcgcccggttcacaatgcctggccagggtgtccgccgcccagaacggttctgtctccgtagcccagttgctgaacgcctccacatcaacgtctgcgggggtgattcgcggcgccgccgcgggcgcaggcgggctgtcgagcaggttcgcctgcaccgccttcgcaaacggggtgaagaccttgaacggggtgccggagctggtggtgatctcgaacggctctgtgagcaggaaacccgggtgcgacactgcacccgtggcctctaagcggaagcttctcgctcaggcgctgcaggctttcgttgcgccaccagcgcgcggcagcgcccaaactaaagttgtcacggcgtctccactacttcgatttcgatcggaacgctacgcagacgatacgtggccggttcaacatccagtaccgcgataagctccgcggcgaaagcaggtgttgcggggatctcggcgtgggcaggggagaggttgaagggggcgtcgataagcaacagcgcagcgtccctgttgaccagcgcaaacgtgcgcccgaaccgcaacctgaaacgggcggcgcggagcagcgcctgggcggagcgctggtcgatctcgatgtggccgcaaggatcgataaccaggtgcgttgcttgcattgcgcttatcgacgacccctcgtccgccatccccgcctccacccgcgcccgcgcctcgtcgatatccatgatgtcgccgcgggccgggtctgtgagcccgagcgggacgtagtcgccgagcaccccggtgaatttcgccgggtcccaggacagggctgcgtccagctcgcgcgcggtcacgcccaccgcgtaggtgaagcggatgatgcctgtcggtgcgtcggcaagcgtgagcaccgggtcaaccacgaacgtgaaccctccgtcggcggtgaccatgtggtgccccggggcaatctcgctcccggtgcggcgcacctgggcgaccatcccggcgagccgctcagccggccacgcgtagggcaccggggagtcggcggcaacacgcatggtcagctcggtttgcgtccccgcgaccggcaccgacgagcgtacccgggacaacccgaaggtgacgtagaggtaatgcgggaatggctcgtccaccctgaacgcgagcacgtcgagtccgtccagatcatcgaaggtgaacacgaacgggtctaccgccgctgccgcttccgccacacgcttcaacaccgcgtcgccgcccagcggcgggccttggcggacacgcgcggcgaacgccgagagccatcccatgggaactaaactagctgaggccgcgttaaggaagatgaacttccaatttttgaaaacggaaaggagctacggggacgtgagcagcaccaaccctgtgcttaagaacctgcccggggcccaagacggccaagcgcacgggcaaacctacagcccagccgggtttgactacccacagcagaccgaacggccgatgaccgtcaacgacgtcacggccaagaccggcatcactttggcggtgatcgtgctcggtgcactggtcaccttcagcatgtacggcgccggcatgtacggccccgccaccatcgcgacgtttgtgggcatgatcggcgccttcattaccgtgatggtccactccttcgggtccaagtacggctcgcctgtcatcaccctgatctacgccgcgtttgagggcctgttcctcggcggcttctcgttcatgatctccggcgcgtttagcgtcggcggcgcggacgcgggcgcgctgatcggccaggccatccttggcaccatcggcgtcttcatcggcatgctggttgtgtaccgcaccggcgcgattcgcgtcaccccgcgcctgaatcgtttcatcacgggcgcgatcttcggcgtgttcattatggcgctgggtaacttcctgctcttcctgttcaccggcatgtccccgctgcgcgacggcggcaccgtgtcgatcatcttcggcgtgatctgcgtcgttctcgggtcgctggccttcttgcaggactttgaccaggtggacaagctggtccgtgtcggcgcgccggagaaggcggcctggggtgcagcgctcggcctcgcggtgacgctggtgtggctctacaccgagattctgcgcctgctgtcgatcatgtcggaccgctagcagcgcctccaagaacgaacatatcccccgtcagttcacattgtgaaccggcgggggattgctttgtgcgctgacggatctcgcaggttagtactgcgactccgggttgtactgcacgccgtcgacggtgatggtggagaaaaccaccttgccgtcgacctcctgcggagcgcccagggtcacctgcgcaccttcgacaacgcggtccggatcgatggtgacctcggtggcggtgccggtagcgccctcagctgaccactggtcccacacgatgtcctcgaggcggtgcttgttgtccttgcaatcgaggttcaagctcgtcgggcgctgcaggtcggccgtgccgcagttgtccaggaacggggtgttgtcctgcgctgccactgccgtggaggttgcggcggaggagctagcgcgaaccgaggaagcctcagctacgttggttgcggacgcggcgctggactgggcggttgcgccggaggaagccagcgaatccgggttctggctcgacgccgtgtcgatcttctgatcagacgggttctcgttcggcggggtgcaggcggtgattgccagggttgcgagcgcggcgattccggcggcggcgatacgggtggaggaggaagtcacgagatacatccttcggtagttgagctttgggttgtgcctaaagattacttctgccgcggggtagaagccttatccgaatcataaggctcggcggagatgatcgtcaccgaaatctcgcggccgttcggcgcggtgtaggagcgggtctcgccctcggcggcgccgatcacagccgcaccgagcggggagttctcggagtacgtctcgaggtccttgttgtccgtcgaagcagcgcgggtaccaatcaggaaagtctcgcggtcatccttgtcgccgttgtagtagacgtgcaccacggtgccgacgtgcgcaacgccctcggccacaccggagcgctccgtggtggagttcgccaggatctctgagatctgcttgatgcgggcctcttcctggtcctgctgctcacgagccgcgtcgtagccggcgttctccttcagatcgccttcttcgcgacgctcgttgatttcggcggcgatgactgggcggttgtcgatgagctgctggagctcggactccagctttgccttcatctcgggggtgatgtattgctgctgagtctcagccatggggtcttttagctaccttccctcatacgtaaaacgagcccgggccccgagtgggctgggcatcgctggtggtctgggcgcagtttatcacgggcttacgcccgcgcaccgacgtaggttgaggatgtgtccatgtagaacggaatatcctgcgagcacccgtaaatgcgtccggagaccaccggttcgcgggtgggcacctccaccgccagctgctggcgcttctccccgccggcgggcaggatcacctcgcgccggccgatttcagcgtggttgtagtccacggcgaaaacgatgcaatacgagtccttggtggtgtctttgcggttgacgtcgatgaacagccgcgcggtcgaatcgtcgacgcgttcttgggtgatgaattcagcagtcaccggacgcgactgggaccgcacaattgcttggcctgccatcacgagaaccagcaccagcattgcgactgcgaagatcgcgacgaccttgccgcttgcccccttcgcctcgctgccagaagcgccgtagcgcgaccgttgggtaggcctagatggagtagacactgaggtggcctcgctctttccgtagttgtcgtcgggaaaatgagtttgccagtgatcgtactaagatgttgcggagctactgcaccaccccctacgaaagttggaacgttaagtgactggtcttcgcctcatggcggttcacgcgcaccccgacgacgaatcgtcgaagggtgccgcaacgatggcgaagtacgccgcagagggccaccgggtgaaagtagtgacctgcactgacggtcgccgcggcgatattttgaaccccgcgatggaccgtccgggcgtgctagagaacattcacaacgtccgccgccaagaaatggcggcagccgccgaggccctcggcgtggagcacgagtggatgggctatgaggattcgggcttgccgcaaggagacccgctgccgccgctgcccgagggctcgttcgcggtgcagccggtagaagaggtggcgaagaagctcgtcgcctcgatcagggattttcgcccgcacgtgatcatcacctacgacgagaacggtggctacccgcaccccgaccacttgatggtgcacgctatttccatggtggcgtgggaacgcgccggtgacccggatttcgctccggaggcgggcgagccctgggagccgctcaaactgtattactcccacggtttcatcctgcagcgcatggagctgctgcacgacctgctgctggagcagggcaagaccagcccgtacgagcttatgatcaagcgttggcgcgaaaacgaggctgacgtgatgcagcgggtgaccaccagggtggactgcggcgactacttcgactgccgtgcgcgtgctcttgccgcgcacgccacccagatcgacccggctggcgcattcttggccagcccgatcgaagaccagcagcgggtgtggccgacggaggagttcgagctggccaaaacccgcgtcgaggtcaccttgccggagaccgacctatttgaagggatcgagtaaatggctactgagaccatcgtgttgcttgcccaggcagcggcggagacgccgtcggggccagactttggcaaagcccagccgacgggccttttgctgattgtctttctggcagtcatcgttttgtcgctaggctacgcgttccaccgtcgcttctcgcggtttaaccgccgccgggcgttcgccgagatgcacggcatcgacccgtttgacgagcaagcggttgacgcagccatgaaagaagccggggtgctggaccggcagaagcgccgcctgatttagtaagctgcataagtgtgacggcgctcgaaactctcctgtacccgatgtacgaggcgcgtttgcgtcgccagctgcgcggcaagaagcgccccaagcacatcgccgtgatggctgacggcaaccgccgttgggcgcgggaatcggggctgcccgatatctcccacgggcaccgggccggcggggccaaaattggtgagttggtgaaatggtccgctgagatgggcgtcgacgtggtcaccatctacctgctgtcaacggagaacttgaagcgcacctccgaagaggtggaggtgttgttctccatcatttcggacgtgatcgacgacctcgccaccgagcactacacctgccgggtgaagttagtgggccacttggatctcctccctccggacgtggcggagcgcatgcagcgctccgccgacaccacaacagaaaaaggcgggctgacggtcaacatcgcggtgggttacggcgggaggcaggagattgtcgacgctgtgcggtccctcatcaacgccgaagccgaggcgggcaccccagcacaagatctggctgagcatgtcaccgtcgcgtcgatcgcggagcacctgtacacctcgggccaaccggatccggatttggtcatccgcacgtcaggcgaacagcgcctgtccgggttcttgttgtggcaggcagcgtactcggaaatctggttcaccgacacctactggccggcattccgcaaaatcgacttcctgcgagcactgcgcgattactcgcagcgctcccggcgcttcggcaagtagcgcgccttacattttccgcatccgcacccgctgcacggtgtggtcgtggccttttctcaagaccagcgacgcgcgcactctggtcgggaggatgttctccaccagattcggcaggttgattgtctgccacaactcgcgcgctttgtacgccgcttgggcatcgtcgaggtcggcgtactcggcgaagtgcgcacccggctcccggaatgcagtgtggcgaagtttgagaaagcggtggatgtaccagcgttcaatgtcctcggttttcgcgtctacgtagatagagaagtcgaacaagtccgacaccatcagcgtggggcccgtttgcagcacgttcagcccctccaggataagaatgtcgggctttcgcacctcgatgtactcgcccggcaaaatgtcgtaggccttgtgtgagtagatcggtgcgtggacgaggggctggccggatttgacctcggtgacgaagcgcatgaggtttctgcggtcgtatgactctgggaaccccttgcggtgcatcaggttgcgctcttgtagcacttcggtggggtagaggaagccgtcggtagtgatcaggtccacccgggggtgcgaatcccaccgttgcagaagcacttggaggacgcgggcggtggtggatttccccacggcgaccgagccggcgacgccgatgacaaacggcacgtggcctgggtcgcccccgatgaaggtctcagtggagttgatcagcttctgccgcgctcggacctgaaggtggataagcctggagatgggcaaatagatgtcctccacctcctgaaggtcgaggttttcaccgatgccgctcagcgtggtcagctcggcttcggtgaggacctgcggcatggtggcgcgccgctttctccaatcgtcgcgggagaaatcgaggtacgggctggaatcaccgccgcttgatgctcgggacatggaatctattgtcccactggggtgagcttgagcgtgtgtgaggggaatatactgcgttagaccgtctggaaatacacgaagaaaggaccggggctgtgactgaagatctccgctaccaggatcttgcaacctacgacccagaagtgcacgccgctatcgtcggcgagctcgaccgccagcgccacacgctcgagatgatcgcttccgagaactttgtgccgcgcagcgtgctgcaggcgcagggctccgtcttcaccaacaagtacgccgagggctacccggggcgccgctactacggcggttgcgagaacgccgacatcgtggaggatctggcgcgcgaccgcgctaaggaagtgttcggcgccaagtacgccaacgtccagccgcactccggtgcgcaggcgaacgctgctgtgctcatggcgctcgctgagccgggcgacaccatcctcggcctgtcactggcccacggcggccacctcacccacggcatgaagatcaacttctccggccgcctctacaacgtcgccgcctacgaggtggaagaggatacccacctcatcgacatggacaagctgcgcgagcaggcccgcgaggtgaagccgaaggtcatcatcgccggctggtctgcctacccgcgccaggaagatttcgccgagttccgctcgatcgcggatgaggtcggcgcgtacctatgggtcgacatggcgcactttgccggccttgtcgcggctggtctgcacccgtctccggtgccgcacgcgcacgtggtgtcttccacggtgcacaagacgctcggcgggccgcgctcgggcttcatcctcaccaacgatcttgagctgcacaagaagctcaactccgctgtcttccctggccagcagggtggcccgctgatgcacgtggtggccgccaaggcgaccgcgtttaagatcgccggttccgaagagttcaaggagcgccagcagcgcaccctcgacggcgccgcgattctcgcggagcgcctgctgcgcgacgacgcgcgcgaggccggcgtcagcgtcgtctccggcggcactgatgtccacttggtcctcgtcgacctgcgcaactcgaagatggatggtcagcaggcggaggacctgctgcacaaggccggcattacagtcaaccgcaacgccgtgccgttcgacccgcgcccgccggccgtgacctccggtctgcgcatcggcacctccgcgctcgcgacccgcggcttcggcgacgaagatttccgcgaggtggccgatattatcgctgaaaccttgatcaagggcgaggaggccgatctcgatgcgctggcggcacgatctgctgctctcggcgagaagtacccgctctacccgggtatcgaagattggaagatgctctagtcttcagcgttcttggcgcgggcttcgcgcagccagtccggctggtcgtcgagcagcgccttgatctgcgcggtagtcagcggctcatccgcgccgctggccttcagcgcagtaattgagatgcccagcttgcgcgcaacctccggcctcgggtgggggccgttgcggcgcagcgtctgcagccactgcggcgggttgtcctgcaactcccgcagttcggcgtgggtgacggcgccatcttggaaatcctgcggggtggccggcagatagatgccgagcttcttcgccgcggtggcgggcttcatagcggtgccggatggctcacgatcgatcatggttcaagacggtagcatcttggccatgctcaccattgcgttcgctaccggcacagcgccggggaagtggttccggcgctacgaggagctgacgggcatccgcttgacgacgatcccgtcagacgaccctttctccgaaacctgtgacctcgcgctcgtccgcctgcccgacgcgcgggtaggggaggaccaccacgtcgtgcggctctacgaggaagcacttggggtcgccgtgccgaaggactccgagatcgacccggcggatgctggcagcgagattgtgaactaccgcttcgaccctgccgagaacccctcggcgtctgccgacgcgctacacagcgctcttcaggtcgtcgcggccaacgttggcgttgcgttcgcgccgctgcctttgctcaaggcgctgagtaaaaagcaggttcaggcgttggagtacccggggccgagccccgctaccgaaatcgcgctggtgtggttgaaagtgcgcgatgacgacgacattcaggactttgttggggtggcaaaaggcaggacggtcaggtcgtcgagaagcaacgcccaacccaagcaatcccgcaaccggaagcgcatccgccacccccgttagggtgggtgatgtgacagtcgatcgctgggaataggcataatggactgcaaccaacacttaaagaaaggtaatgattttcgtgaatcgcaagattgctgcatctgctgctgccctggccttggccggcggcctggtggcttgctccaatgacgacgctgcaaccaccgccaccgatgccgtgacttcgaccaacgtggcaaccgagaccgaggcttccgccaccgagacgctctcttcgaccgcgaccgaaaccgcgacggagacctcttcttcctcgtctgagaccgcgaccgaaaccgcgacctccaccaacaccgagaccgagaccgtcgccgagagcgctgccgctggcgccaccgaggagatcaccctggctgacggctccgcagccctggttccggccggcgtcgtcgagaccatgaacgagtacgtcgcttctaactggggcgagccgaccgcagtcgaggagatcgacggcggctgggttgtcacctacgacaacgagcactacatcacctggaaggagtccaccggcggctccccgatctggggcgagatcgccaacacctggctcaacgacgtccgcggcgctcgcaccgtcggcttcccgctgatgccggagaccccgaacaccgacggttccggctggaaccaggagttcgagaacggcaccatcgactggtcccgcgacggcggtgcagacgcaccgtttaccgcgacaatcgacgcgaagtaagctcgactccttaccaaacaaaaagctccacccagcgtttgctggggtggagctttttgtttgcttgcggtcgggtttaccgcaacaatggtgcgcgtgacacgcacggagaagcaaggctttcgtattcgtccgatcaagcccgaggactacccgcaggtccgccatatctacgagcttggcctgagcaccggcaacgcctcgtacgaaacgcaaggccaaacgtgggaggaattttcccgcaaaaagatcattgaaacggtcttcgtcgctgtcgacgaagcggatgatgcacgtgtgctcggttgggtggccgccgcaaaggcatccacccgcagcgtctttcacggggtggtggaggattcgatctacacccacccggacgctcgcggtatgggcgtctcgggcgcgctgctggatacgctgatcgatacctgcatcgccttgcacaagtggtcgatccactcgtggatcttccccgaaaacaaaggatccgcggggctgcacacgtcccgcggatttgtgaaggccggcactttccacaacatggccaagatgacgtacggcgaccatgagggaacgtggcgcgactgcgatgtttacgagctcattctgcccatgtccaaggaggactagctcaagtcttccttcagcggctcttctttcacgggaagcagcagcagaagcgacagcacagcgagcggcaccatcaagaggaaaaccggcgtgaggccgtcgttgtagctgctcaagaccacgtcgcgcagcggtgcgggcagctgggtgaccagctcgggggtcaggctgttggcgccgccgttggcaaacttctcgccgtaggccgcgccctccgggccgagctgcgccagcgctccgggcaggcgctcttcgaggttgtcgcgcatgccgtggataaacagcgaacccgacagcgacgcaccgatcgcggagccgatttggcggaagaagttgttagtggaggtcgctgtgccgacgatcttcagcgggaacgagttctgcacgataagaaccaggacctgcatggtcaggcccaagccgaagccgaagatgaacatgtagacgccgagtcgcgtgagcgtggttgtcacttcgagctgcgagaacatgttgagcgccaccgcggtgatcgccataccgatgatcgggtagagcttgtagcgacccgttttcgagatgatgaagcccacacccatgccagtggccagcatgccgatcaccatcggcagcatcatcaggccagcctcagtcggcgacagctcgtgcaccatctgcaggtaggtgggcaggtacgccagcgaggaggtcatggcgaagccgaggaccgtgccagccgccgtggtcagcaccatgttgcggttggtgaacaggccaagcgggatgagcgggtcgtcggcgcgcagctcgacaacgacgaacaagacggcgccaaccagcgcgattgcagacgtggtgatgatggtcggcgacgaccactcgtactgggtgccgccccacgtggtggtgaggatgagcgaggtggtggtcaccaccatgagcagggtgcccagccaatccacgtcgaggttctcggtcgagccgcggcggatgcgcaggacggctgaggacaccgccattgccaggatgcccagcgggatgttcatccacagcgcccaacgccaaccggggccgtcggtgaaccagccgccgagcaccgggcccaagacagaggagacaccgaagactgcgcccatcacgcccatgtacttgccgcgctcgcgggccgggacgacttcagcgatgatcgactgggagttcaccatcatgccgcccgcgccgaagccctggacagcgcggccgacgatgagcatcgtcatcgagttggcgaacccgccgatggtggagccgatcacgaacagcgcaatgctgcccacgtagagccacttgcggccgataacgtcgccgagtttgccgttgacaggcatcgcgatcgtcatggtgaccaagaacgaggagatgacccagctcatatgctccacgccgccgagctcgcccacgatggtgggcagcgcggtggagaagatcatctggcccagcgagctcatcagcatggtgagcagcagggcggagaaaatgagccccacgttgggggcttctttggtttctaccacggtaattcctttgcaaactgggtcaagttgttggcgttgtgacggatttgggtcaccgggtcgccctcaggtcgcgggttccaaaagtattcgccggcggcgctgcggaacagcgcaatgatggcgtgcacctctgacgcgtcggtgtcggaggcgtcaaggagtctgcggtcgcctggaaagcgttcgtagtgctcagttaaggcagcctcgagggcggcaagcgtttcgtgctggcgcgcgatagcgaggtgcagcagcgcggggttcgctccgattaagcgccggcgctgttcgcttatcgacggttccgtcccctccggcaccacctccaccgaagagatcaccaagtcgagaacgttgacgctctgcgtcgagcggatgcgctccagtgagtctgcggtgagttggaacggcacgggccctaggacggcctcgtccttggagtccatgtagttgaagaacgtgcgccgggagatgtccgctgcagcgcagacgtcttcgacggtgacgttgtcgtatccgtgtgcgtcaacgagcgaacccgcctcggcgatgatgcgccggcgggtttcctcgcgttttcgttgtcgattttgcacggggtgcaacattacacccggtgcaagtttatctgccagccgagagcacgccggaggcgaccgccgcgccgttttcgctgtaagtgacctcaacaagccccggttctgggatgccgaaagtccacgtgccgtcgccgacagcgccgccggcgtcgatgagcgcggtgcagccggtcaggggtaggtgatcgaggcggtgccgccgccgaagtgcgctaccgccggccacgcctttacgcgcgcggcagggtcggctgcgttgatggtgccggtgtaggggccttgaaagggagcgtcggcaagcaactgctcctttggccgcgcagtgacggtgaccgtttcgggaaccgctgtgaccggatctggtgcggggttggccgagcgccacgcgccggcaagggcgatcaggatgctgcgagcgccgaaacgccggcggcaatccacggtttgttggagccgccggcgtgacgcaggtcggagaaggaatccgccatttagttgcggtcggtgttcgccatcgagagcacgtcgaggcgcttgtccagctcttcctcggtgagcttctcgccgtccacgaagcccaagtcgatggtggcttggcggatggtgatgccctccttgacggcgtgcttggcaatcttcgccgcgttctcgtagccaatcgcggagttcagcggagtcacgatcgacggggaggactcggccagggtgcgcatgcgctcgacgttcggctcgatgccgtccaccaggcgggtcgcgaactggcgggcggtgttggccagcaggcgggaggactccagcacgttgcgggccatgaccgggatgaacacgttgagctcgaactggccctgggtgccggcgaacgccacggctgcgtcgttgccgatcacctgcgcggagacctgggtcgcggtttcgcacagcaccgggttgaccttgcccggcatgatggacgagcccggctgcaggtccggcaggtggatctcgccgatgccggccagcgggccggagcccatcaggcggatgtcgttggcgatcttgtacaggctcaccgccacggagcgcatcgcgccggagaactcgaccaggccgtcgcggttggcctgcgcctcaaagtggttcttcgcctctgagagctgctcgacaccggtgagcttcacaagctcctcggtcaccttcgcgccgaactcggcgggggtgttgatgccggtgcccacagcggtgccgccgatcgccagctcgccgaggtggggcagggtgttctctacgcgctcgatgcccagctcgatctggcgggcgtaaccggagaactcctggcccagggtgaccggggtggcgtccatcagatgggtgcggccggacttcaccacgtcgtgccactcggcggccttgcgcgagagcgactcgtggagcaccttcagcgccgggatcaggtcgtttgcggcggcctcggttgccgcgacgtgggtggcggtggggaaggtgtcgttggaggactggcccatgttgacgtggtcgttcgggtgcacctcaacgccgtttgccttcgcgatcgacgcgatgacctcgttggtgttcatgttcgacgaggtgccggaaccggtctggaacacgtcgatggggaactggtcgtcgtgctggccgtcggcgatctccttcgccgcggcgataatcgcgtcagccttctcagcgtcgaggttgcccaggtccttgttcacctgcgcgcaggctgccttcagtaggccgagcgcgcgaatctgctgcgcctcgaggccacggccggagattgggaaattttccacggcgcgctgagtctgggcgcgccagagcgcgtccacgggcaccttgacctcgcccatggtgtcatgctcgatgcggtattcctgatcagccattatgtatcctttgcaactatctcgtgcacgccccacactgcaaggtgcgcgcgtgcctgtccattggacgattatgcacgaaccagacacgacgaggaggcgaaatgaccgaacacagcgcccgtaaagcccccactttgagggacgctctggtcgggtgcgcgtcgctggtggttgccgacgcgttgctcatcgcgcaagcgttcgcgctgatgcgccttgaagtcccgcgcgcggtgctgctcacgctcttcccgttgttgattctggtggcgttggcggtgcccaccattttcctgctgcgctacctcaagcggcgcgggatcccccttgggtttgaccggctgggtgcgagagggtggcacttgctgtgggagttcccagtcgcagtactgttcgcgggtgccggggccgcgctcatcggcccgctgctcggcctagagtcaacgggggagacgacgtccaacgacggctccaacctcggcgtcgtcctcactcttgttgcgtacctcgcggtggggccgttccttgaggagatcgttttccgacgcctcgtgatgggctacctggacacggtcgcccccgctgccgtgagcgtcgtcggcagcgcgattctattcggcctcgcgcacatcgccccgccggcgatgctgtatacggggctgatgggcatagccctggcactctcaactcgttggcataagtcgctgtgggccgggctcattttgcacttctgcaacaacctgctcgtgcaggctgtcgttgtgggcgggctttagttcgtcgggtcggagtagtcgatgaccgagtactcctgcagcttggccagcttgtgcatggactcgacgtaacgaactgtgccggacttcgagcgcatcaccagtgagcgcgtggtcgcaccgtacttgcggtaggacacgccgcgcagcatgtcgccgttggtgacaccggtggcggcgaagtagcagttgtccgaggtgacgaggtcgttgatcccgagcacccggtccagatcgtggccagcggcgagtaccgcctcgcgctcttcgtcgctctgcggtgcgagcatgccctggatctcgccgccgaggcacttcagcgcgcacgcggtcacgacaccctccggggtgccgcccacacccatcgcgatatcaatagagctggtgtcctgcgctgctgcgatcgcaccggcaacgtcgccgtccatgatgaagcggaccttcgcgccggcgtcgcggatgtcgcgcaccagctgttcgtggcgcggacggtccagcacgacgacggtgacttcgtcggggcggatgccctttgccttggctacagcatggatgttggcggcaaccggggcggtgatgtcgatgctgcccgcagcctcggggccgacggcgatcttgttcatgtagaacgcgtctttcgggttgaacatcgagccgcggtcggcggcggcgataacggagatcgcgttcgggcggccctcggccatcagacgagtgccgtccaccgggtcgaccgcgaggtccacctgggcgccttggccgttgccgacctgctcgccgttgtaaagcatcggcgcttcgtccttttcaccctcgccgatcacgatgacgccgtccatgctcacggagttgatcatcttgcgcatcgcgtccacggcggcaccgtcgccttcgttcttcttgccgcggccgacccagcgcccggaggcgagcgccgccgcctcggtcacacggaccagctccatggcgagattgcggtccgggaaatattcggtcgtcggttcagacatgcggggacatcctcctcaaggcggtgcggtaaaagacaccttcattctggcactttcttccaccaagaaccgcaaatttgggggattcggggccggcgcgcccccgtgtcatactggtctgcgtggcagacaaagggaaaccccgcgtttttcaagacggccgggacatgttcatcaacgttgtcatcatcgtggtgatgatgctgatcggtgtcggtgccaccgggctgtgtacctacaacccgggacggccggaaaacggtcccgtgcaggaagtcgacgcgcgcacgttcctcggtctcgaatccagagcgacaaatttcccgatccgctacccggacacgcctgagggctgggtagccaactcagcgcgccgcaccatgatcgaccagcagcccgcacccgtggtggggtgggtcaccgccgacggcggctttttgcagatgactcagacgggggcagacattgagaccgccatcgcggcgcaggattcggcgctgcgcccgaacgagcaaacaacgactatcgacggtcgcgaggtgcgtgtcttaagcgccgacgacccggcagtgcgccccttatgggccgtcgatgccggggacgcccgcttggtggtgaccggcgccggcacggaagacgagtttgtaacgctcatcagcgcggcgcttcaggccgccccgatcgatccgaacggcgacgcttaatcttcgcggctctcccgttcagcgatcgcggcctccacgcgctcggaggcgttgtgaagtaggacctcgcagcgcttcgccaggctctcgccgcgctcccagtatttcagcgattcgtccaggctcatctgcccgagctcgagaatcttcaccgtttcaatcagttccgcgcgcgcatcttcgtagttcagcatctccggatccgggaacgcgttctcgccagcttgacctgccccgaaggtggtatctgccatgggtatctcctgtttcgtctgtaaaaaggtcgggttgtagttagtcggcttgggtgacgcccattgacgcggccgaaatcgagccgtcgccgacgcggatgcgcagttgcgaccccggcggcgactgctcgatggaggtgacgacctccggcccagagccgtcgcgggggaggacctggactaccgcgtagccgcgggcaagggttgccgacgggcccagggtggccacttgcgagcgaagcgcgctcaccgtcgacgtctgctgggcgaggtagtgggtgagttcgcgccggatccgggagacttcgcgatctatctcctcgcgacgctgggcgatggcaccgagtgggttcgcaagcgagggtcgtgagcgcacgtcggcaagcgcctgctgctcacgctgcacccagctgcgaagtgctgcggcgctgcggcggcgcgcctctgcgacgagcgcgatttcctcggccatgtcgggcacgacgcgcttagcggcatcggtaggggtggcggcgcggacgtccgccacgttgtctaggacggggttgtccggctcgtgaccgatagcggagacgaccggtgtggcagcagccgcgactgcccgttggagtgcctcctcggagaaggggaggaggtcctccactgagccgccgccgcgggcaatgatgatgacatccacgcctggatcggcgtcgagcttctgcagcgccgcaatgacctcgggcaccgtgcgcgggccttgcaccgcggtgttgaccacctcgaaccggactgcgggccagcgtgcctgcgccaccgagagcacgtcgcgctccgcggcggatccgcgcccggtgatcagccccaccttgtttggtaggtacggcagtggacgcttgcgggccggatcgaacagaccctcgccagcaaggcggtggcgcaattcctcgatgcgcgccagaagctcgccagcgccgacgtgtctgatctccgtgacccgcagcgaaaaagacccgcgctgtgtgaagaagttgggtttgccgtggatgacaacgtgatcgccgtcgcgtggcgggcttgccatcgaggtcagaagcttcgtatctgcgatcagctctacgctggcctcagcctgagtgtcgcgcagcgtgaggtaggagtagctccagttcggcttggtcttgacttgggtaagttgcccctcgacccagatgaagccgagccgttcaacccaacccttcacgctggtgttgagtttggccacgctccacggcgcctccgcggtgcttttgggatcagccaccttgctcctccttcgtttcgccccaaggataggccagcggtttttcttgctagggatttagacgccacttcggtagggtcggttccatgacggatcaaggtcagggcaaaaccctgcttctcgcctccccccgcggttactgcgcgggcgttgaccgcgcggtggagactgtcgagcgtgcgctggagaaatacggcgaaccgatctacgtgcgtaaggaaatcgtccacaacaagtacgtggtgaagacgctccagcagcgcggcgcgatcttcgtcgaggaaaccgacgaggtgccggaaggcgcgcacgtggtgttctctgctcacggcgtgtcacccgcagtgcgcgagtctgcggcgcagcgcaacctgctggcgctggacgcgtcctgcccattggtgaccaaggtgcacaacgaggctaagcggttcgcccgcgacggttaccagattctgctggttggtcacgagggccacgaagaggtcgagggtaccgctggcgaggcgcccgaggtcacccacctcgtcgacggtgtggagggtgtcgctgcgttgcccgacttcccggaagaccagccgctggtgtggttgtcgcagacgacgttgtcggtggatgagacgatggagatcgtcgaaaagctgaaagagcggttcccgcacctgcaggatccgccgagcgacgacatttgttacgccacgcagaaccgccaggccgcggtgaagaacattgcgccgcgctgtgatcttgtcatcgttgtaggttcgcagaactcctcgaactccaagcggttggtggaagtcgcgctcgaggcgggcgcgaaggcgtcccatctggtggactatccccaccagatcgacgacgcctggctggaaggtgtggaaacggtcgggctgacctcgggcgcatccgtgccggagatcttggtgcaggaagtggtcgcctacctcggcgagcgcggattcaccaacgtagatgaggtgaccaccacggtcgagaccatcacgttcgctcttccgcgcgaccttcgcgcccgcaaggcctagcccgcaaggggcttagcgccgagttgagcgcgcccgctcgcggcgcacaagttcttgcacggatacgctgcgagaagacgctgcctggtctgctgcgcgccggtttgaagacgacacgcgccggcgttcccgcgcctcgcgcgccgcgatcacgcggttttgccgcttgatcagctggattcgggcgattcctatcaacgctgaaatgagtgtgacgaagaacagccacgggaatagctccaccagcgggtagaccacgaggagttgcgcggcgcgcgaggatgcgccttcgcctgcgagctggtctttgccaattaacaggccggaggccaccaccgcgacaaggaaaagcagcggagcggtgaccacggtgaggaagacgccgcgcgggttgacaaagagcgtggtgatgatgactgctgcggcgaagagcgccagaagcggccacgtgatggccccggcgctgactgcgagcaatgcgccggtgaacagcgccgcggcgttaatcgcgatcgcggagccggttggaaggcccataaatgcagcagacacggttgattagtctagcttgttgtttttcaccgttttttcaaacgtgtccgcgatcctcttcccgcccgctttgcgcagctcgttgctacggtcgcgcagcttttgccaactcgtcgagccgtggccgggctggggtgcgtccacaacctcgtccataaccggggcggtggaccattcgcgctcctcgcgccactggcggcgggtgtgcaccgactcctcctgctcgatctgcgcgatggcgaggccctccggcgtaaagaagtccagctcgtcggcggtgcgctcgccggagtggatgcgcagcatgtccagcatgtagcggtacgtgaccgcaaccatcgctgctaccggcacggccaggaaagcgccgacgagtccgaacaggccgccgccgacggtgacagagatcaagacaatgaccgggtggaggtccatggcgcgggactgcagcatgggggagaggatgttgccctcgagctgctgcacggcaatcacgatggcgagcacgatgagcgccttggtgaagccgagggagaccagggcgatcagcacggccaaggctccggcgacgaccgcgcccacgatcgggatgaacccggccaggaacgtaatcacagacagggtgaacgccatcggtactccgacgatccagatgccgatgccgataaacagggcgtcgataagcgacactatcgcttgggcacgaatgaaacctgaaagggtgttccaggcgcgggtgagcagctccgtggcgtgcagaccgctgcggccgccggtggccgagcgcagccagggcaggaagcggtggccgtctttcagaaaaaagaacgtcagaacgatgatgaccatgagggtcacgctcaggccagccgcggagctgatgcctgagaacacgccgcccgcgatcgccccagcctggttctggatccagccggagatgtcgttgaccacctcgttaatgctgtcggggtccacattgagcggcgggccctgcagccaaagctggaggcgttgcacaccctcgaacgcctggaggtaaaggacctgggagtggttgaccacgtccggcgcgataagcatgaagatagccgcgagtagcgcgatgaaccccagcattgtgaacatggcggcgaatccggacggcaccttgtggtttctcagccaggtggacaccggtgcgagcaccgtgcaaatgattagcgcgaggatcatcggcaaaataccggcccaaaaagcgccgatgatgcgagcgagggcgtagaggaacaccgcgatgatgagaatgcgcagcgtgaacatcgcggtggacttcacccactggttcatcacaatgccgcggtcaatgcggtcgttgcttgctggccgctgggtggggatttgctccgccgctgcattctcgttgctcgcactcactcgcaccattgtgcacgatgaaccggtcgaatgccacggtcttcggtggactaggatgagccagcgtgagccttactcttggaatcgtcggtctgccgaatgttggaaagtccaccctgttcaacgcgctgacgcgcaacgacgtgctggcggcgaactacccgttcgcaaccatcgagccgaacgtcggcctggtggagctgccggacccgcgcctgacgcggttggcggagattttcgcgtcggagcgcatcctgcccgcaaccgtgtcgttcgtcgacatcgccggcattgtcaagggtgcctccgagggcgagggtatgggcaacgcgtttctggcgaacatccgcgaggccgacgcgatctgccaggtggtccgcgcgtttagcgacgacaacgtgatccacgtcgacggcaaagtggatcccgccaacgacatctccgtgatcaacaccgagctcatactggctgacttgcagacaattgagaaggcgctgccgcggctggaaaaggaaggccgcaaggacaaagacgttgcagcgcaggcggaggaagccaagaaggcgcaggcaattcttgaggacgaccgcacgctcttcgccgcgtccaagtccggggatatcgacctcggtctccttcaccacctgcacctgatgaccgcgaagccgttcctctacgtgttcaactccgatgaggcagtgcttaccgacgaggcgaagaagcaacagctgcgcgacctcgttgctcctgccgaggccgtcttcctcgacgcccagaccgagaccgagcttctggaactggacgaagaggatgccgccgagctgctcgctgccgtcggccaagacgagcccggcttgcagacgctggccaaggccggtttcgacaccctcggcctgcagacgtacctcaccgccggcccgaaggaagcccgcgcgtggacgatccgcaagggcgacactgcgccgaaggctgccggcgtgatccacaccgactttgagaaaggctttatcaaggctgagatcgtcgcgttcgacgacttggactccctcggttcgatggccgaggcccgcgcgcacggcaaagtccgccaagaaggcaaggactacgttatggctgatggggacgtcgtcgagtttcgtttcaatgtaacctaaatacgctatgaatagcgtatgactacacgcgctgctatttacctccgtatctcgttagatgctgccatggacggcctcgccatcgaccggcagcgtcaggactgcgaagccctcgccgagcaacgcggctgggacgtcgtgcatacctacgtcgatcaatcgatctctgcatcaaagaaggacgtggaccgtcccgactacgacgcgatggtggcgtcttttgatcgcggcgagatcgacgcgatcatttgctgggacctcgaccgcctcacacggcagccctggcagctcgaagagtggaccgacagggcggaagagcagaggctgaaactcgtcaccgcgaacggtgatgctgaccttgccaccgacggcggcagaatgtacgcgcgtatcaaagcagccgtggcgcgcggcgagatcgagcgaaaaagcatgcgccaatcccgtgcgcaacagcagcgcgccgagcagggccgctggtactccggcggtgtgcgcccgatcggctacacctccaccggcgagatcatcccatccgaagccgccgccgtgctcgggagactgttatgacccccaaaaagcgcactcggcagtttgcagcgctgctgattgcctctgctctgagcgtttccgtatctaactcagccgttgcttccgcagaagaattccaagaccacggcgccaagggaggctttgcttccggtgtgatggccgagctactcggcgaggcagcaccagccttcacaacctactgggcatctgccggccggaaagtttgctaccctgcaggtggcggtacctgggagtacggattctggaacgctaaggcgcgttcttatttcaccgtgaatcggtgccatacttcgactgtgaccgtcaacggcagaacgcaacgaagcatcaacacccgcggcggccagaagtcgatcgccgagctttgggcaacgaatttgccgggcactaaggacagctactactacaacttctgctagaactcatgcgcattcgacccctagtacttgggcttttgagcctacttcttgctgcagtcatcgcgactactgggtggctgctgacagccctggttgactccaccaagcccttgtccttaggggtcgaatcaacctttagtcttgactacgtcgagcctaagacttcactcgcggaggaacttgagtcagactacgcaccgacggtaatccgtaactcactggtttcattggccgagcagaacggctactacatctaccggctgactggcaccgatgacgcaagcgggacttctcacgaggttttcatcccgctggagcaaaattatccagcaccggaacgcattccccggctcaaccggccggatgccttgagccaagcggccagtgagcttgggtcgctggattaccacggtgactacgtcttggttcccaaagcaacgggtggcaatgcgaaccacttctacgaatcggccaggaatgacgggctcaggctaagcgaaaagacgcagttccttcacctcatccaatcggtcgtattccgcctgcccgcgttggtggcgatcctgtttctatttgtcgtttccctttttgccctggtatttgttcttcgggtttccggtcttagattggcagcgctgcgcacaataaatggcgggcaccgcagtcaaaaaggcaattggcggcaatggacctttgtcatcctcccgcacctagttctcattggccttgcgagtacattcctcgcccgccaagggagctattcttttgccctcctgttcctcaggttctacgccgccgggataggcttggccctggctaccaccggtttggccgtagccgtcaccgccccattgttgcgccgcgcagtagcgctgctggcgcagcgtgcccccgcagagaaggcggcgggaaaagcgctgaaagtaatttcggtctttacctgcgtgacctttgtagcagcgggtcttagctcagcggctgcgctccgctcctaccagcaggaatccgaggcccagcagacctggaaatctctcgcggagtttggagccttgcatttttcagccaacttcgacggccctgctggccgcgtggaaggaggcgagctcttgccgcccagtctgcagcagaacttccgcgacttcgcgctcagctgggaacgggagcacggggctgtcctcagccatactttgccgaaagaaggtaccggtgtgccggactcctgccccgtggcacttgccaaccgccaatggcacgatctgcaggattatcagttccgtcccggagacgacaaccactcggtcgactattccgcagcccaagagcatttcgcagcttccgtggatctgtgggctcaggaatccggcgacctgctccttaaatctgcgcaaattggtccggtcagtgccgatcatgcggtcggattcattagtggaacaatgtcgggggaactggttcccggcgattgtttttacgtgcttgaaacggacgatctatccggcttcgacgcagacttcctaagctccacagcttcgagtgaaaatttgctcttcgcggatttctcggaactgggtccagaacttaccgctgccggcctcgaaggctacgtctacccggtacgcgccgccgatcgcggtctggccgaactagtagccagcacggcgctgttctggctgagtatcctgagcgccctcggagctttgctcgccacgcttgcggccttgatagtccaggcgcgcatccagctccgagttcaccgtcgcctcctggtactcctccacagcgctgggcaatcaccggacaaaacaatgtggcgactattcaaaagccaactggtcagcctgacagttgtcgtcatattgtccgtcctggctccgctactgcttcccaacccgttcctctacaccttcaccgcgctaagctgccttgtcttaatcgtctacctcggttttgtccgtctcagtatttctcagcacatgtccgcctcccctaggagtcacaatgtcattggctagccccaatcagtcccccactctgccgccggagatttccacctctcatctctgtctcgccgcggagtcgactttttctgtggggcgcagcacgcggatggtgaagaagtccctcgtggaaaatgcaacgttttccctacccgggccaggctttgtcgccatctgtggagccagcggttccggaaagactttgctgctcaacaccttggccgggctcctgccgccggcggacggcctcctccggatagacggtgagaatgcctccgcgtggaggatgaagcggaggcggaggttctggcgagaacgcgcagcgataatccaccaagaccacggaatcattcccgaactaagctgcgaagataacctcaccctcgggctatccaggaagcaatactccaaagaagaattgctgcactccctcggcgaagtcggtcttgatgtccccttcgacgggccggcagctattctcagcggaggcgagcagcagcggctggcgatcgcccgagccctgctccgcggcgcggcttatgtgttcgctgacgagccgaccgcctccctcgaccccactaaccgcgaccaagttatcgcgctcctgcggcgagctgcggacgggggcgcactcgttctggccgccacgcacgatgccgcagttattgctgccgctgacagcaccttgcgcatcaatgatcgccaggtcacagtctccggctctgcgcgggattaaatcgcgatgcccgcggccttggccaccttccggtacccggccgcatggtccgcgacgctggcgtgggcgttgagtccgctggggttgtcgagcacgggcctgacccccggaaagtagacacgtcgggggttagctatgctgcttgggtcggcgtagctgatgtgagtgcttcgaagtcattgggggctagaaagttgcaccaggagtgccgtctgcgggtgttgtagcgcatgcaccaccggaagacttcttggcgactgatgtcgaagtggtcgaatttcgtgcgcggtgaacccgcccgccaggaggtgcttgaagtcgctctcgactggatcgctcagcgtgacggcgtgagcatcgataactacatggccaagcaccgcgatgacgaggactgcaaggagctgcagacgtacttcaccaccgtcatcgactgggccgcaagcgtgttcaagatgacggacagttccatgcgtggaatcgcgtggaacaagctctatgagcagtacggcgacaagggctacgacgcagcaaagatgaccgccgaagcacgcgagctgctttccgactcgcaggtccagtcgaagaagggtatctacgagtacctgctcggcggcaagaaagagacgcggctgcttaacgtgcgtgtcttcactgaggctgtcaaaaagcgcgtgtacaagcgccagacagacgccgccgagaagaacggtgtgtccaactgctcctactgcgctatcggcctcgacgagaagaaggagaagatctggccgctcaaggatatggacgctgatcacgtcaccgcatggtcgaagggcggcaagaccgaggaaagcaactgcgagctgctctgcaagtcccacaatcgcgccaaaggtaacgcttaaccagcggcgacgcggggatctaacaatgctgcgtcgctagcgctcgcacccggtaagccgagcatcaggctgcgctagcgacgcccggcgcacatgagtgctgcgctgctgggatacgcctgcgaccggcagagccggaccgaatacgggattgaccgtgtacaccccgtattcgtgcaaaggagcactgccatgtccactcattcccacacgcttgcatcccacggcgagatcctcgcgaacctccccggcatcctcggattctacccgaacaactcgctgatcctcgcgttcttcgtcgacgacgagggcgtcgacaccatccgcctcggcccggtcgcgcggttcgacctggacgaagctgttgcaaagctcaccgagagccgcgagcggttcgcagcgtgggtccaccacctcgaactcgacgctgttatcgcgtacatgatcagcgacgacattgcgcagccggtctttgacgagacggcaacgtatctcactagtggggcagtgcacctaccgccgctgctcggggtggtgcaggtgcccgagatcgtcaccggggctgcgtggtggtctgtgtatcagcatccgctcatcgatgagccgcgccacggtgttgtcggcgaggtcgccgcatcggcggcgctgcgccagatgctagagcacaccggcgagctgccggaaccgagcaaagacgacatcgaagcacggttgaacagcaccgatcacggcatcgacgctgccgagcacgccgacatcatcgaagacgcgctggcgtatatcccgcccatgttcgcggacgtgctgcagcgtgaatacgagcaggcggcggcagggatcacccagccgagcactcgtgctgttcggtctgcgctgaaatgcttcaccacgccgcgcttgcgagacacgctgctcgcagcgctgctcgatgagccgcaggctggccttgcgttcatagagcaggttatgcgcgctgtcccgaccagctggccggggatgcgggcgcagctcaccgccactgttgccgtgctcgctcacgccacaggccagccgggactagctggcgtggctgcgcagcgagccaccgagatcggaccagacgagaatttcccgtctctggtggccaagctgaccgacattggccagggcgagcggatggtcgaactcgtccgcgagggcgctgagaagacccgcacgatcttgttcaccgagtaacaccacacaccccgttgcagcgatgcaacggggtttctttttctcgcggggccgtggccagcagagatgcacacctagcggggcgggggagaaccccctagacagcagagctgtctccaacagacggattgaccatccatccgaacaaggaggcacctgatgcgcgacatcacccacaccgacctggaactgctctaccagctcgccgacggcatcgacggcgaggacgccgatccgggcgcagcacaagaactgcgcgacctagaggcggcaggcacaccgctgccctgggcagtgctgtaacgacagctcaacccccgcagcggcaaagccgctgcttaagtacccaaattgcacggcaaatcacacccactcacgtaaggagaaccatcatgtccaaccccttcaacaacggcaccatcgtcggcaacgcagctcgcgcacccaagctgttcgagcacacaaacggcggcgcgacggtgaagctcagcgtctatgcgcgcaacaccttcaagaacaagtccaccggcaaggtggaaagcgagatcgtggagctgaccggctacgtccaggacgccgcgaaccccggtgtgttcggctgcatcggctccggcgatcgcgttgcggtgagctactcgctcaagaccgacgtctacaccgacaaggacggtgtgaagcagtacccgctggtggcgcgcatcgacacggtgcagctgatcgattccaagaaggagtccgctgctcgcgctgcccgtcgcggaggcgaggcggcgaccgccgccctggctggcgctgagggcgaagaagtaccgttctaactacgaaaccccgcagggaaacctgcggggttattttttcaaccatttcacacgccaatttgctgcgaatcacttgtgcagttttacggtgcagtggtgcggtgcttttactggcgtttctgctgcgcaactcactgcactatgtagtgtctgtgacatttcattaacacgtaggttgcactgtgtattgggcacccatttcatcgacacgtttactgcgcaatcaaatgccctgtcactttaatgacatgtgaattgggcagtgaagtggtttgtcatcctattgacacctttactacgcaacagaatgacaacgacattctgtcggcccttctacggacatctcttctgcgcagcacatgccccgtcgtacacaccgacgtgctgcgcactatctccgccactcaacaggccaattcactgcgcaacgtagtgacaccggccccgcctagccgagatttcttcgattttcgctgaatatcagccgtttacccgccgccaatgacctacgacgccgacggccccctgttaggcccgcagaaggccgtacagggcaggggagagcagtgctacaactccataccgccatcacgatcacgctgctgttgctgctggcggcgcttctcgatgcgctcgcgtgcacgctgctgcgccccgcccttcttgcctgaggtctgcgactgcctgaacagcgtgtaacgctcaagcaactctgggctgcgatgcagttcttgcaccaggaacttcttatccaagtgctccaactgttgtcctgacttcaccgcttcttcgatgatgatgcggcttcatcttcggcgtccgtgtgcgcgttgcggcggatctgatcagcctcatcgcgggcatccttgcgcgttactgcagcgtcgcgtgtggcctcgtcgcggatgctcgtggcctcatctcgtgctttgctgcggatcgtctcggcgtcgcgctcagcctgcttacgggcctcgtcggtcttgcgagtgatcgtctctgcttcgctgcgagctgcggctgtaatatcgcccgccttggcccgcgcagtctcttcggctcgttcgagcagctcgtctgcttgcgcttcggccaggcccaactcctgctcagcatccttgcgtgcttcgctgcggatctcttcggcttcttgctcggccttctcgcgtgcttccttgagcacacgctcggcaacctcgcgagcctgtgcttcagcattctcctgtacgcgctgggctgcttcgcgggcttcttgcgcctgttcaagttccttagcagcctgctcgcggtcacgatcaattgcgtccatgtcgcgctgcacggatcgcttcttgacttccacatcatcctcgcgcttggcgagatcgcgctcccggtcttgttgctcggtgtagcggtcgaggttgagtgactcgtcatgacgttcggagacttctagttccaccggatagccgagcgagtgcatgtgttcgcgcaggccccgttgcgcgtcgatgaacttctggttacccgagatctgcttgcccttcttcgggccggatgtgtaccgcactgaggtgtcagtgttgtacgcgatgccggggcggcaacggagcttgtcgggatcttcgggcttcggtgagaacgtatccgcctggaactggatgtgtggcgttgattcgtcaaagttcatatcaccgccagcgactgcgtcgataccgccggggatgaagttttctgcaagccagcgcattgactcttcgaggtactgctttgcttcctcgtagtcgcgggcgacatagcgcggacgtttcacttcgcgcccgtccacctcactggtgtagtagtcggggatctccttgcacatcgacttcggcagatacacgacgaacagcgacgtcttgaaactgttcttctgcacgcgcactccgtccatccgaggcgtctacggccgccacagggccgtacagccgctgccacaaagatgaaccaatcgagtcgcggcgctacacatttgcatcaacagctgccgctggatctgctgcagcgcgacgcgctgcgaaacacacgtcgctggcggtgctcatcacatgcgcttgcgcgcatatggccgccgcgagcgtgatacgtctgcaccgatagtgtgcttgtggcacgggccgatatgaagtgtattaatcaggcccgtgtcgttgacccccgcagcagcatcaacactgcctggtggcggatggctcgctgcaggattttcaccaccctgcaatgaccgcctgacggcggtgccagagtgcagggtgtggctgtgcgcaccacgtaaacaatgtcggtcttgccgttcggttcgacgccgtggcacgttcgcaagctcacgttgcacacggcgtgcgcgatgacgcgggaacacgccgcaagcggcgtttccacccgtcatcggcccttactttaagaccgacatacaacggctgacgccgcatgtggtgcgcacagcgtggcgacctgcagattttgcgtaggcaccatgtgcgcttcgcgcatcaacgggccgtttcgggtaagggtcgaagaccgtgtcacaacccgaaacacgcaggtcgcagcccccttctgtgtcaaaacccctatatgtttgtcgttataggggtagaagggggaaaagggcataagggggtgcgacgcctccgctgcgctccggcgctcggcatagccgaggcactgcaccgggtattactactcgctggcgctcgcataacccggtgcccggcgctggcgcgccgccccttatagccccagtctcagacctcgctcgctcggtctggctgggtctacctttccctccgctgcgctccggtcaaggtgcccaatagtgcagctggcgctgcaccttgtgtgatgacccatgctttacgtcacgacactgctggcaatccgatatatcccgtcgatatgtattcggatatgccagcatcgatgtgtcgtgtttgggtcatcacgaaacgctccataacggcaagcctgccgagatggatattggcgtatctcacggcgcgtccatgatgcggcatgcgccgcatgtcatctgccgtcgcggttgcatcttcagcagcacagctgctgaaatctgctctgtccgcgctgctgcacgccctcaacccacggccacagctatcggcatatctcgtcgcgcacgacaccatgcctgctgcggccgcgcatcacagcagcgcgacacaccgccagccatgtggcggatgatccaggcgacggggcaggtgtgtatatgccccgtcgccaacaccgtcgcaagcatcgtgacagtgtcacgtgtagcggtgccgcagccacccgcacacacgcgaaaaccccgcccttgcgagcggggtgtgtggcgacatcaaacgtgacggctgtacgtcgtcacgccgcgtggccgtacacacatgaggtgattgcgtgtacggctaaagggttagtcgggtacaacttctagatgccgcttcggcttactgccctcggtgctctcaggcgtgtcgccgtcaccgttctcaggtgtatcgctgtccccttcggtgctggcggacttgtcaccgtccccttcggtgctggcggacttgtcaccgtcgagattcacctcgaactcttcggcatacttgcgcaactgcgcaaggcgctcctttgtcgctttgtgtgcacggcgcgcctcgttcacggtatcttttgcttgctgctcatcgcgcagcgctgctgcgtaatcgtctctgaaagacatggtttgttctccttggttgaatgaactgtttatttggactcggggcacgacggtggagcgcgcgtgtgtagtagcacggccatcacccatcagccctcgcactcagttcaagacccagcctgactagctgagctaagcggcgggatctcgtcgtaggcgggtttgtccgcattagtgcttcacaccgcccagcaccgtgacgagctgctggcgctgctcatctgtcagttggggcgctgcattcacgacggcatcgacgaagccgtcgaatagctgcggggcagggcggcgtgcggccgcgaggtaggcgtcgagatcgtcttggcgaatccgataggcggtgccgaaacggtggaatgaaagacggccctctttaatagcttttcgcaacgtggactcggagccgacgccgagatcggcgagttcctgcagcgtgtaaaagcgtggcgcgacggcggtagtcgtgtccttttcggacatagaaaaacgctcctgggcagattgatctgtcccggagcggggtgctttaccggcttgctattcaggcggcttggagtgccgtgctcaactcgctagaacggtggtctgccgtcccatcgctttacgggagcgcttactccctacctgaccgcttttgtggttggcaatgccgttgccgaccggtctatctcgtcggaggaaccgctcctatcacggtcgagaggctgtctctttatgaattatcctcggggttatcccccgtatgcggctggctaaaccaaaaacgaattaaaacgccacatacggtctgggggccatcgtacggaacttatgcgtcgcgcacaatagcctgcgacctaatctttacgaatcgaaccgagcacgtttctacacgccacgtggcacggctggggtgttgtggtggggcagctgttgtgtggcggcatggtgacacgcaaggggcgcgcctttttgtgacctgtgacacgtctatagtgtgctcgtttcgtagttttgacctcgtttcgtaatttgccgatcaaaatacgaaaaaattacgaaacgctctacctgcggtttcgtagaactacgaaaatcggaaaaccaaattacgaaacacgcgataacgctgtgacctgcacagacacgtcacatttcggggatgtttcgtaattttgcggcatttcgacccaaaccttttaagggagagacacagacacacattacgggcacatgtctacgacatagaccgtcctcattgagggcacgctgcaggggttgtagctatgtgacacggccgggatgctgcgtcacggtgacacgcaaggggcgcgccttttatgacctgtgacacgtctgtagcgcgctcgtttcgtagttttgacctcgtttcgtaatttgccgatcaaaatacgaaaaaattacgaaacgctctacctgcggtttcgtgatttccgcaaacgaaaagaacaaaactacgaaacacgcgataacgctgtgacctgcatagacacgtcacatttcggcggtgtttcgtaattttgcggtatttcgacccaaaccttttaagagagagacacagacacgcattgcaggcacatgtctacgacacagagcgtcctcgttgagggcacgctgcaggggttgcagctatgtgacacgggacacaatcgcaatcaaggtgtctcttcttatttagattttcttcaaaaagtggaaaaattacgaaacgaaaaccatttacgctgctcaacgtatgtttttgtgtttcgtagttttgttcgtttcgtttacgagattacgaaatgacccgcaaatacctaccgtgacctgcggtgatgtgtttcgtatttttctgcgtaatttcacgtcgcccgaagcagacaccctgccgtgtgcttgctgcagggctgcggccgtccctccatgtggagcgtcagtgtcgatgctgtaacttaaacgtacatacatttgtggcgctctcgttacgtgtctgtgcattgccgagctctttactgttgtgtgtgggcgcgcagccgtagtgtccgtgccactccgagtagggcgcgtcgtaccccaaacccatgttcaattaaattccaatccagagaggtcttgcactgttgcggtgcggttgtcttctttctcaccgtattggaccctgcgaaattaattggatacgataggcccatgttgatttcaggttccgttttcatgcggccgctcaccagccgctaaggcggttttctccctcccgcaggttagaaaccgctccggtcctttagccgggcggccatttgccatgcccggctccgtttcaactccacggagcacacctgatgtctacatacggatacggccgtcacgaacatggccaaaattttctcacagaccacaagatcatcaactccatcgtcgatcttgtaaaacaaacctccggccccatcattgagatcgggccaggaagcggtgccctcactcacccgatatcccacttggggagggcaataacggcagttgaggtagacgcaaaactagctgccaaactcacaaaaaagaccgcctcggcgtcggtcgaagtggtccatgatgatttcctcaacttcccgttacccgccactccctgcgtcattgtgggaaacattccctttcacctcaccactgccattcttcgaaagttgttgcatgcgccggcatggactgccgctgtactcctcatgcagtgggaagtcgctcgccgccgggccggggtaggtgcaagcacgatgatgacagctcagtggtccccatggttcacgtttcaccttggttcccgagtaccaaggtctgctttccggccacagccaaacgttgacggggggatcttagtgatccgccgggtgggtgacccgaagatcccgatagagcaacgcaaagcctttcaggcgatggtgcacaccgttttcaccgcccggggacgcgggataggggaaattctccgaagggcagggttgttttcatcacgttcagagacacaatcatggttgcgctcgcgaggaatcgaccccgcaaccctacctcccagattgcacaccagcgactggatcgatctcttccaggtgactggttcctcttcaccgcgccatcggcccatttcacaatcgggaagtagtcaacgccctcctcaacggaaaaatcgaggccggcggcggtaatccccccaccaccaaaaccgaaatccaccagtagtagtgaacgacccatgttcgtctaccgtgagccgcgttatggcagtgacgtgttctcgtcgggcacagtcatagttcccggcgttgccagcgacagggttctacacccagcagcgggaccgatcaaaatcacccgcacggggaacgaccctgctggtggtttcgattttgatgaaagcgaggagacatagcccctcgccaactccccgtagctggcgaacagtagctcctggcgctggcgctcgttggtgagtttgcgtgccacatcgaaagccttatcgacttcccggtccaagttgttgtgagccttgagcagaattgggtccatcgataacgggttgtagtgctccgcgagtgaccgctgggggtgccgctcgcgtgcccgcagcaccaactgtccagcgtcgatgattcgctgctgcgccttctcatctagttcacacagagctggtccgcagttgtagctcccgatgtactccgaaaaacggaaaaaataaatagtggggatacatcaaccttccactttccattcttccggctcagagtattgaggggtctgggaccgggtccgtaaaccctttatgtttttcgcgcacagcggtttttagcgacgcaccctataggttttccgcagaacctatatgtgtttctgtgcacccccatatgttgtctgtttctagcggtatttcgttgtactttgcgcatcgaatagttatttatcgacgacactccgtggagttcaaatttaacgtgtaacgcggagcgttaatgacgtttcgcgttattgggggggtaggttgaagagcgctgtctctaactccggttttcgtgcggcctcggtccattccgctacctcgtgtgtagaatctgcaagcggtatcgggccgttgaactattaggttcacccacagttcccgtgcctgcacgcatcgagaaggaccaggtggtgaactcgaatgactcgcctggtccaacgtgtgtgcgctcggcgcgtggtttaactcttataagacttgccggtcacagcctcagcgtttcgctcgtgcagcccgcaggccgttcaagatcacgatgacttcggcgacttcgtgaaccaacacgacggcggccaggcccagcacaccgctgatcgccagtggcatcaacacgataatgatggccagagacagcacgatgttttggttgatgatcctgctgcctcggcgggcgtgctgcagcgcctgcgggatcagccggaggtcgtggccagtgaaggcgacgtcagcggactcgatcgcggcgtcagagccggttgctcccatcgcaatgcccaccgttgcgcccgccagtgccggcgcgtcgttgatgccgtcgccgatcatcgccgtcggcgtcttggaggagagttcggcgacgatgcttgccttgtcctccgggcgcagctcggcgcgcacgtcgtcgattccggcgatttcagccagcgcccgggcggtacgagtgttgtcgccggtgagcatgctcacttccacatcgttggcgcgcagggtctgcacggcttcgggcacctcgggccgcagctcgtcgcggacgccgatcgctccggcgagggtgtcatcgacggcgaccaggacgcaggtctggccttcggactccatgcgctcaacgtctgccttcagtggcccggcgtcgatccaccgggggctgcccaccagcacccgtcggccttcgacggtgccgctgatgccgtgcccggcttcctcgctgatgtcctgggcggcgggcgcttcgggccccgctgccgcgatcgccgcggcgagggggtgcgtcgattgctgctcaactgccgccgcgaaagtaagcacctgcgcccgatcaaacctgtctgccgggaccacgccggtaacctcgggctggttgcgggtgagggttccggtcttgtccaccgccaggtgacggatgccgccgagccgctcgaacgccgcgccagacttgatgaccacgccgaactggctggccgcgccgatcgcggccacgaccgtcagcggcacggagattgccagcgcgcacggcgacgctgcgaccagaaccaccaacgcacgggtgatccacgtctcggggtcgcccagcagcgagccgatcacgccgactagcaccgccaggatcatcaccccgggcactaggggttgggcaatccggtcggcgatccgggcgcggtcgcccttttccgcctgcgcctgctcgaccaggtccacgagtgtggtcagcgagttgtccgttccagctgcggtcgtctggacttccagcacaccggcggagttgatcgctcccgcgggcacctcgtcgccgggcgcaacctcctccggaatggattctccggtgatcgctgaggtgtcaaggctggagcgcccagaccgaatgatgccgtccgtggcgatccgctctccggggcgcacgagcataagctcgccagccgcgaggtccttcgctgcgacctcgaccgacgtgccgtcgcgcagcaccgtcgcggtctgcggtaccaacttcaacagtgcccgcagtccgccctgcgcccggtccatcgccttgtcttccagcgcctcggcgatcgagtacaggaacgctagcgccgcggcctctccgacgtaaccgaggattaccgcgccgaccgcgctgatggtcatcagcaaaccaatgccgagcttgcgcttcgtgacaaggtttcggatcgcgtcgggcgcgaacgtatacgcccctagcagcaggccgacccagaacagtactgtcgcgggtgtcgctagcccggaccagcccagcgccaggcctacgcagagggctacgccggagaagatcggcagtagcaactcggggtccttccaccatggccgatcgagttcttcgatctccgtggcgggttcgtgttcgcatccacacgccgagctcatgcgtcctctcccttctcgccgcagccgggcaccgagcactcagggtcgatgcacggggcgttttcgtcgacagccaacgtcgcgttcaccagcgcgttgagcgctgccgcgaggtgcggatcggcgatttcgtagcgtgtcttgcggccctccggctcggcaacgacgatgccgcagtcacgcaggcaggtcaggtggttcgagacgtttgagcgggtcaggcccaggtcgcgcgaaagtacggccgggtagctcgggccgtcgagtagtgtcatcaggattctggaacgcgtcggatccgccatggcccggccgagccggttcatgacgtcgaggcgtgaagcaatagtcagcatgtgctgaacaatacatcgtgtgctgaactattcaaagtgtgctgaactgacagttacgcgaaggtcctgcgacctgcaagaattagtcgatgggatagcagatgactgatcctttgtggttcggctgccacccaacgcgggagcgacgtgggtggcgaggttctcgagaaagttactttgcaactacataccgtcgagttcaagttcaacgtgtagtcaacgtgtattcagggtgcaccgcgtcgcgctcatagggacgaggctattgcgacgcctacgctcacgagggcccgcgcattcacaccgggcaaatgaccggcacgccggcgtcgtcgaggatgcgggcgctaatgccgtagacctcgttgaggagctcagggttgagcaccgcggccggggtatccagcgccacgacgcggcccgctttgaccacgagcagctcgtcgcagaaacgtgcggcgaggttgaggtcgtggattgcaaccagggcaagcctgtcggttcccgccacttcatcgcggatgatgtcgagcaggtgcacctggtggcgaaggtcgagggcggacgtgggttcgtcgagaagcaagacgctcggggagcgcacgagcatctgtgcgacgccgaccaactggcgctggccgccggacatgtcggagaccatgcggtcggcgaggtgcgtgatgttgagccgctccatgatgtctgccgttgccgcgactggatcgacttcggccgcgccgcggcgcttcgcggaaaccatgatggactcgaacgcggtgagtgacgcggtggtcagcatgtcctggggcacgtagccgatggcggtggtgcgagacttgccggtgacttcgcgcccgtcgacgacgatggagcaggtgccgtccgacggcttcttaatccccgcgatggttttcaccagcgtggacttgccggcggcgttcgggccgatgagccctacgactttgccttcttcgagtgggccgaaggtcatgtcgtcgatgattgtggtgcggccgtagccgacggtgaggtgctcagcgaaaattgccacggttagcccctctttcgtgcgcgggtgaagataaggaagacgaagaacggcacgccgaccagcgaggtgatgatgccgatcgggatcgccagccccgggatgatggagagcgatacagcataagccacgctgagcagaatcgcgcccgcggctgccgcgccgggaaggaagaacttctggtcctcgcccacgagcatgcgggcgatgtgggggccgacaaggccgatgaagccgatgatgccggtgaaagcgactgccgaggcggccagaaaggatgccacaagcagggtagtgaggcggaggcgcttgacgtcgatgccgagggcggcagcgcgatcgtcgccaagccgaagtgccgtgaggcgccaggagttagccacgcagaaggggatcgctgcggcgacgaccacggcgaggatgatgttcgcagtccagttcgcgcgctgcatcgaacccatggtccagaacacgatctgctggagggcctcgatgttggcgctgtattgcagcagtgagagcagggcctggaagaagaagctcagcgcgatgccgaggaggatcatcgattcggcagtggcgccgcgccacacggacgcggctgccacgatagcgaccgcgagaagtgctgcgatcgccgcagtaagggccaggttgaactgcgggttcgggatgagcgtccagcccatcacgatggcgatcgccgcaccgaacgcggccgccgccgagatgccgagggtgaagggctcggcaagggggttatccaagatggtctgcatctgcccgccagcgaggccgagcgcggcgccgcacagcagtgccatcactgcggcgggcaggcggagggtgcggatgaccacgcgggtctgatcgtccaccagctcggggcggaaaacggcgttgtagacgtcggcaagtgcgatgtcgatggggccgacgacaacggcgacgaggaagctcgcgaaggccgcgatgaccagccccacgatggcgaacgcttttttgcgtccgcgcttgtggtagctcgcaatcgcggcctggcgagcatccacggttgcggcgggctgggcggatactcgagttgtcatgggttagctctcgtccgggttcgcaggatcgtagaagaacacgccgctgtactcgaacggcatccactccttgtggaactcgatgaagtccttggtggggtggtagtcggagaactcctccgggtggatccacttggcgaaggcttcaagcgcgaagacgttgaacgggttgtcgtagaactggtggtacacggcgaagtagttgccggtctgcggcgcttcgagcagctcgaagccgggcagttgcagcgggccgttggaggtttccttcgccagctcggtgttagactggtagcccatctcgacgtggcggaagaggtcggtcttgttcgggtcgcgcgcccactcgccgccggtgacgataatcttctccgggtcgagctcaatcagcttctcgggggtgatggtcttggtttccgggccgaggacttcggggccgaggttgtggccgccggccgcggtgaccagggtgcccaggtgcacgttgcctgcgatggcgcagcactcgttgtagccggccgcggtccacagcagcacgtccggcttctctgcgatcttggctgcgcgctcggagatttccttgaccttcgcgtcgtagaactcgttgtacttcgcggcgcgctcgctctggccgagcaggtcacccaagagctgcatggacacggtggtgttttccagcggcttctggcggaagtcgatgtaggcgtaggtaatgccggcggcatccatgtccgcgatcatgccggcctcttcggcggccttcttctggtcgagcgtcataatgaccacgtccgggtcctgtgcgagcaggttctcaacggtgacgtcgcccttctggatcatgccgatcgccggcaggtcctttgcttccggctgcagttcgaggagcttctcgcggaacgagcccgcgttcttcaccaggtcctggccgtacgcaacgatgttgtccagcgggttctcctgcagtagggcagtggcgtaggctgcgcggccctcagccagcacgatgcggtccggcatctccgcgaactcgatagtgcggcccgctgcatccttcaccgtcagcgctgcgtccgcagtgcgtgccgacgtctgcttctccgccgctgctgccgaggtagcaacctcagaggatgtggtgctggcggtggtgttgccggagtcggagcaggcggccaggccgagcgtggtggcgagtgcaaccacggttgcaccgatctttcgtgaaagcttcaacacttccccttcagttaagtaagcctaagcttagttacaggaacgctgagaacactaaggtaaggctaggctaatgtcaacggtctgagtcgtgcttcacacgctggcgaagcaggacagcgatgagctcccggttcctgtccagcttattgacaggcagcacgggttgaagcctgttaccgcgaatggtgatgcggacctcagtactgagggaggccggatgttcgcgcgcatcaaggggccgtagcacgcagtgaagtcgagcgtaaaggggctaggcagtcacgcgcccaacagcagcgtggagagcgagggcagacatcttcctctccggctacggcgcagcccaggcgatgccaggcccgctgttcacgttcgcgtccttcctcggcgccagtgcacaaggcatggactgggcgctcggcgcgacaatcgcgaccatcgcattcttcctgcccgctgcgcttttggtacttggcgcgataccgttctgggagcgcatccgtcagatgccacgcgcaggtgtcgccctggctggagcgaatgccgcggtggtcggcattctcggtgcagcgctgtacaccccggtgttcaccgccggggtttccggcgtgatcaccctgtccatcgccgtggtctgctacgccgcgctcacctcgtggaaggtcccgccgtgggcggtcgtcgtcgccgcggccctggtcggctggattgtgctgtgaacttcgctctcgcccggtgctcggcgctgaagcgcgccaagggagggaaccgggactagagcgtcacgttggccagcaccgcgccggtgggttgcgccgcgccggcggcgacttcctcggttacgaggactgaagcagttccaccgggcagcggcatccacacgtcgtcgtggggttcttggccgatgactccagccgattccacggcgccgtcatccatgactgcccacacttgtgcccccatgccgtagtcgagagctggctggccgtttaccatggcgccgcccttgcccatgtcagagctgattacgatgtcgaggctcgcgcccatcgcgtcggcctgaccttgacgcgcgtcgtcagcctccatgattgcgtgcatttcgttgacgccttgggctgtcacggattcgcgtgactcgtcgacagtgaattgggtgaccgcgaacccgccaccggcgatgagcacaacggcggctgctgcggcggttgtgagacgccgcccggagcggttcttccgcgcggtgtcgaagtcagcgacctggtcggtggcgtcgatacgctccatgattgcgcgtttgagctccggtggcggggtgaccggcgtggccgcggaattgaagaggtcctcgatatctttatccatcacaggcctcctttcaacgacacggccttgcgaagcttttgcaacccgtcgcgtacccgggttttggctgttccgagagcgacgccagtggcatcggcgatttcttggtgggtgagttccccaaaatacgcgagcatgagcgcacttcgatggggctctccaattgaatcaatgagttcttgaagctcctcagactctagtcgctgttgagcttcgtcctcagcggcagcgacccacgtggtcagttgactgttgaaatcgtcggtgtcgcgggcttgggagctgcgccagctccgcagccgatcgatggctcgcgatttggcgagccgcagtacccatgacttggcgctgccgcggtgtgggtcgaaggtgtgggcgctctgccatacctccacgaagacttcttgggtgacctcttccgcttgggcccggtcacgcaagatgtgggtggtgagaccgagaacctgtggggccagaacgtcgtaaagctcggcgaaggcgcctttatcgcccgcgcgcacgctttctaagagacggtcaggatccacagattccaaatctaacacctgggtcatgtgctacttggattcttccatcatcttgtcttcgctcatcatggcatcggaggacggtgccatggaatcgctcatcatggcatcggaggacggtgtcatggaatcgctcatcatggcatcggaggacggtgtcatggaatcgctcatcatggcatcggaggacggtgccatggaatcgctcatcatcgcctcggaagacggggccatggagccgtccatcctgtcctccatcttctgctgggagtcgttgcatgcgacgaggccggtggcggcgatgactatggcgctgacgctggcgattgcgcggttgatagacatagtgtctccttcactttttcggttcgcaggcgcagtgtttctggcccgtcactgagtactacggagccgggggctgttgcggattggaccaatccggtgcgggtgctcactccgtagtgctgggtgtaggaaaggcaaccggaaagtagaggaaactcatgatcagcgtgattcttgtcggattcatcggaggtgcgatcacggcattgtcaccgtgcattttgccggtgttgccggtggtgctgggtgtcagcgtcgggcgtaaaccgtcgcacgtggtggcaggtttggtcgtgagcttcgccgcgatcgcgctgctgggtacgattctgcttagtgcgctgcatttgccacagtcggtattgcgctgggcgggagtggtgttgctggcatgggtggggctgggaatgattttcccgccggtgggggaggtgttgcagaagccctttgacgcgcttccgcgccccacggcattgcaggagaaaacgcgcggcaagggaggttttctcatcggtctggcccttggcgcggtgtacgttccgtgcgcgggcccggtgcttgcagcggtgacggtggcgggctcgactgggcagatcggctggcacacggcggtgctcactgttgcgttcgcgattgggtccgcgctgccgctgttcgtgttcgccctggcgggcaacaagatcggtgacaaggtagacgcggtgcggcgccaccgtaaggccatcggcgtgctcatcctggtcttcactgtggcgttggctctcgacgcgccggcggcgatccagcgtgcgctgccgaattggacgtcgtcgctgtcgaaccgttttgagaattcggacttggccaatgacgctctcagcaaggtcggcccaactgggagcggttcactgcagtcgtgccgccgcgccgaccccgcgcagctgcaggattgcggcccggcaccggaattcgcggggctgacgaactggatcaacgccgaccagccgccgagcccgcaggacggtggtgtcatgctcgttgatttctgggcgtacgcctgcatcaactgtcagcgtgcgggggagcacatcaccaagctttacgacacttatcgagattccggcctcaccgtggttggcatccattcccctgagtacgctttcgagcacgagctgggcaatgtccgcaacgccgtagaaaaggaaggtatccactacccggtggcgcaggacaatgacttcgctacgtggaggaatttcaacaaccgctactggccagcccgctacctggtggacaagcacggcaacgtccggcagatcgtggaaggggagggaagctacgccgagtcagaaaagctcgtgcgtgaattgcttatcgacgtcaaccccgacgtcgacctccccgaaccggtcgaaggcggcgaagcagcaggcggtacaaagggccgcaacccggaaacgtatctcggcactgcgcgcgccgagtacaccaagcagcccggttacaccgacggcgagcacgacttcggtgaaccggccgccccggagcgcggcatgttcactctgaacggggcgtggattctcgaggaggaatcagtgcagaccaccagtggaggacacctggacatcaacgtcttcgctaagtgggtccagctcgtggtttcgggtgaaggcgagatcgaggtcgagtatccggacggtgcgaaaaagtcgttcccggtcacagatggaaccctcgaccttgtgaaaggcgacacgcccaccgagggagtgctgcgtatccggcccacggcaggcgtgaaattgtattcgttgaccttcggctaggcagagacaaccttgtccagcgcctcggcgaagcgcgcgacggtgcctccgcctccctgccaggctctgcaacctccgcagactccacaaccgcacccgaatccgggtccacccactgcgtggacgtgaccaccacggtctcgggctcgctacctccggcgcaacccgtaaccaccccaacagaactagctacaataagcgcgggcgcgcgacaaaacgcatgtatccaccctaaccggcgggcgcaggaaactctcggctatttcccaagctccttgcgtcgctcggcggcgagtttcagccgctcggcgcgatcagaacgttccttctccagcagttcctcgaggatcttgtcttcctcgtcggagatgtcgaagacggcgtaccaagcgaccgcgagtgcgcccatcatcggccacaccacccaggcgtagtccagatccagcccaatctgcagcacaaaatagaccgccaagccgccaatgagggtggtgtagatcgcggtgtccatcttccgcttcgctgcaagtttctcatccagttcaacctcggacggcgtccgctcctccaatgcgaccggttcggccgggaggtcgtcgaaaagcattgaaagctccccgcgagtgcgcgcaaccgcggcttgacctgtgcgttcttcgaactctcccacatcaaggtagccgtctgcgaacagtgtgcccagccgatccagcgcgtccgaacgctcggcgtcgcccacgcggattccgtccattatcgctcccaacttgcacttgcccttgcggcaagctgttcaatcgcagccatggcagatggtatcgaatacacaatcagcgaggccgccgaagtcctcggcgtttccaccaaggcgctgcgtcactgggagacgctcggcctcatcgcacccgcgcgcacgtgggccgaccaccgcgtttacagggaggcggacctcgagcgcggcgcggccatcgccctctaccgcggagtcggcgtgccgcttgcgcagatcgcgcagcttctcgacgcctccggagccaccctcacccgcgccctcaagcaccaccaagaagcactcgcttctcgacggcgcacgctcgacgcccagctcacatctgtccagcacctcattgacaacgcgacgaaaggatcgatcgacatggatgcaatgaagaagtacctcggcgaagatatgcccgcctatcaggaggaggctgagcagcgctggggtgataccccggagtgggcgcagtcccagaaaaagctcgctcaaatgggcgaaggtgacttcaaacgcctgcaggaagaacaggacgcgctcgccgcggatctgatcgccgcacgcgattccggcgtggaccccggctccgaggaagccgaagcactggtggagcgccacggcgcaagcatcgcccagtggtacgaggtgaccccggctcgccagctcatcctcgcgcgcatgtacgttgacgacgcgcgcttccacgaagcctacggcggcgcgcaggactacctgctcgagctagtcaccgcccacgcggcggccgaaggtgtggacgtgggcaacccgcagtggggttagaaacggagcaggaatccttccaactcttgctggagcaaaggccacggtttggttaggtctagtgttgtcgcgcctatgtgatgaccagcgagcaccgcgtcttttttgcgtatctttacgaaaccgcgcagcagacaccccaccgtgccctcaccggaacccttcttgcgcgaatctctccagtagcactacagcatgaaaactatgtagatttgacgctcatctttccgtgccctgttgcttcgtgagttgctagatgttccgggagcgatagcgccatgaccgcatcctgcgatacttctctggatgtaccttgtaactagtcaagtagggtgcggtactgcttgcgggccttcattgagtgaatgatggtctccgtgccgtcatcccagagaagaacgacaatctccagcaaccgcatagaggaatcaaatccgagccgaagttcacgctgcgggtgatcctcgtcgagtggcgttttgtatacacatcccgaagtggctgcagtgagcgaggattccggttcgataccgtgcttttcagcgctacggcggacctcgatctcaaatggcgttttttagagccttgcggattgcctgcgatcgcgacaacccgtgtgaggcggcatactggtcgagatgaaggacttcgctaggggagaggcggatggaaacaacttgcgcggcttcctcatcccgtggtttccgcccgcgtttccgtagcatctccacgtcgtagccttcttcggcttcggctacccatgcgtcaatctgctcttcgctaatcggcttgccgtttatcgtcttcatacaagatatcgtaatacggaattgcagtcgatactttggccgaacacttaaaactggtcgagttcaagttcaacgtgtaattacgcgtcggggctgcccacgcaaaactcgttaccttccggatcctgcataacggtccaagtaagtcctggtgcctcgtgactgctgagttcagtggcgcccaacgccttgaggtgctccactagggcttcgcgttcagtgccgccgccgtcgatatgaacgcggtttttaccaggggtggggtcggcaacgcgctgaaaacctagtgctggggtggagccgaccatgacaaagtctccgtagtcggcgacgatttcgcatccagtcgcggcggaccagaattcggcgagcttagaggggtcgttgcagtcgaaggttatctgtcggatagcgaaagttgtgtcacgcatagtacgcactgtatctgtgtttcgatgagtcgaggaggctctggcactgctttcggtccttcactgagcggaggcaaaaacgcgcagcctgaggtcgctgcagtgctggagtcctgcggcgtgatgccgtgcttagcggcatatccgctgaggccggtgatctcgacggggattggtggattcatccacgtattagccgtctgttgctctgcttacccacctgaccatctgatgtccgcgggtcctcatcgtatgagcccgccgacccgatctacggcagttggggcttacgcctcgtcgacttcagctccgagcgccgcttcttcgcttcgagacggcgccgcaccgagccgcgcgtcggcttcgttttccgccgcgggggaggcggcggagcgagcgcctcacgcaatagggcggccatgcgttcccgcgcctcggcacggttgcggacctgcgagcgctgcgtcgacgcgctcacggtgagcacagtgccgtccaggcggtgttcgaggttgtggagggcgcggcggcgttgggcgtcggaaagtgatgcacatttcgcgatgtcgatggacagctgcaccttgctgtcggtggtgttgacgccctggccgcctgggcccgacgccttcgcgaaccgctccgtcagatccgcggcggcgacgacgaggccgccggggatccccgggccgggtgcgatggtcaggccctgcatgccgcccaccctacgttcaccctggggccgaggacgaggcggctgagtcggtgctgtcggttgttaatcgcgatagatctcgcggcggtggcctatcgaaagcaccgcgattgtgatcgtgccctcatcgatgagggcaaggatccggtacgcgccgacgcggtatctccactcgccggaacgatttgcggagagccctttcccaaatgcgcgcgggttggtgcagccgtccaaattctctttgatccaggtggcgatgagccgcgcgtcgaagcggtccatcttcttcagctgcttccgtgcgcgggccgtgaattcgactgtgtagtggcccgatggtgccatcatccggggtgctacgtatcgaggtcggcgagaatgtcgtccacgctgtaccgctcgccggtgtcgtgcgcgatggcgtctcgaagctcctgcagatcatgcgcatcttcaatcttttccaagatcgcattgcgggcgaaatcggaaagagttacgccctcgaagcgagcgtacttgcgcacgagttctgcatcgtcgtcatccatccggattgtcatcgtagccaaagtttacccctttaatcagtgtgaatacactgtattcggtaggtgctcgatgtgcaatgggtggggcggagcccgtcgcaaagcacctgcgcctagcgccgcggcagcacgacctcggggtacttgcgtacgtagccgaccgcgatgacgacgagcgccgtgaaggcgccgatgacggtctccgcggtgcgggcgagcagcatcggccagacgggggaggcctcgaccgtctgcaccatcagcagggcggtcggggtgatgaagctggtggcgatggtgtagttgcgggcatgttccgggagcgatggcgccatgaccgcatcctgcggtgtactgacacctagcgccgccggttcgagggcaggttgtcctcgatctcgtttccgtagtaaccgctaccgaaccctttgatgatccggacgatgagccacacgatagagatgatgatgagcgcgatgacggcgaaaatgagcacttcttggtacgagatgttcatggtgttcctccggcggtgtcattcttacggctgatactcgcatggcaccgcaaggagcacaatgcttgacgacgcatcgtggcccaaagtccaccaacccgatccgaaagtaacccgccgatggcaagcgcgcacgcgccccgttaggtagcgtggcctgcgatgttggaagtgctcgcaatcttcacccgccttgggttgacgtcgttcggcggacccacggcgcacctcggatatttccgcgacgagtttgtggacaagcggcagtggatgacagacgaggagtacgcggacttagttgcgctgtgccagttcatgccgggtcccgcctccagtcaggtgggcatggcgatcgggtacaagcgcgccgggtacgcgggcatgctggccgcctgggtcggcttcacgctgccgtcggtgatcctcatggttgcgttcgcactcggcgtcgcgcagctcggcgatgtctctggcgccggctggctggcggggctgaaggccgcggcggtggcggtggtcgcgcaggcggtgatcgggatgagcgggagcatcgtcaccgacggcaagcgcgcagccattgcgctggcggcgttcatcgctgtgcttctggtggttagcccgttcacccaggtggcagttatcgcgctcggcatggtcgcgggcgcggccctgttcggcagtgcacgcacaccggcacgcacaccggcgagcacaccaagcgctgtccccacccgcacccgcgcggttggagccgccgcgctggcggcgttcgcggggctgctggtggtgctaccggctgccgcggccgccgcgcagtccacggccgccgagatgttcagcagcttctaccgggccggcgcgctggtgttcggcggcggccacgtcgtgctgccgctgcttgagcaggcgacggtgccggctgggctggtggaccacgacacgtttttggcgggctacggcgcggcgcaggctgtgccgggtcccttgtttacgtttgcggcgtttttgggggcgtcggcaagcggtgttgcttggtggtggggtgcgattgtcgcgaccgtggcgatcttcctgcctgcggcactcctcgtggtcggcgtcatgccgttctgggagcagctgcgcgagcacccgcttgccgcgtcagccttgagcggcgcgaacgccgcagtggtggggatcctggcggccgcgctctacgacccagtgttcaccgcgggcatcacaggtccgggcaccctggcggtggcggcggcagcgttcgtcgcgctgcgcaagtggaagaccccgccgtgggcggtggtggttgcggcagccgcagcaggggcggtggcactgtgatccgcgtcagggaggcattgcttgccgacgcccccttagtcgccaccctcctcaccaatttcaataccgagttcgacacacccgtacccgaccttggcgtgctgacgaggaggttcgaggcgctgctgccgctcgaaagcgtgctcgtcgtcctcgcggagacagaggaggggccagccgggttcgcgtacctcaccctgcggccgacgccgtactgggacgggccgcttgcgcagctggaggagctgtacgtcgtgccggagctgcgcgggcgcggcatcggcaccgcggtgatggagcgcgtcctcgcaatctgccgcgaaaagggttgcgaggagatgctgatcaacgtcgacgagccggacgagggcgcccggcggttctacgagcgcctcggtttttcgaattacgagatcggcgaggactaccggatgttgtgctacatccggcagctgggcgcggaagcgtagtcgatttaccagcggaggtattcgccgacgactgcgcctccgagctcgtcgaggtcgggtgcgacgacgtggccgccggagcggttagccagggcgtcgataagcgccacaagccctggatcatcaccgaggcggaagaaggtgattttcgcgccgcgcttggtcaccgtgtcgagcgcgtcaacggtgcgcgcgagcgtgatgcggtccgtcggccagttgaagtaggcctcgccccactcggtgaggatggaggtcggctcgccgtcggtgacgatgagcagcgtcgggtcgtagccggcgtggcgggtgaaaaattcgttggccaaaagcagcgcgtggtgcaggttcgtgcccttttcctgcaacggtggcagggcggtgagctcctcgatcgtgagtgtttgcgcgtagaggccgaagccgatgagggcgagttcgtcgctgcggaactgcgtggtgatgaggtggttgagcgccagcgcggtctgcttcatcggcgtccagcggccttccatcgccatggaaaacgaagtgtctacaagcagcgcaaccgcgttcttcgtgcgcgcctcggtctcgaccacctcgatgtcgttcacggtgatcgcgaacggctcgccgcttgcggctgtgcgctgcagcgcgttcgtgatggtgcgggtggtgtcccacgcctgggtgtcgccgaactcccaggggcgggtgccgccggtgggctcacccagctggccggccaggcgggagtcgcgctggccgcgggagagctgggaagttgcgcccttcagcagctctttgcccagcatgcgtagtgcctttggagaaagttgtagcgaaccggattcgcccttgttcagcaacccggattcgcgcaatgctttctccaggtcgcgcagctgcttcgcgctggtggcggcgtcggcgccgagcaggtcggcgatgtcgtccaaatcgatgtcgccggggcgatcgctgctcagggtgtctgcgagctggtcgaggcgcccgaggtcgcgcatcgcgcgggtggcttcgccgaggcccatcgaaccgtcgccgtcgaaagcttcggaccccgtccaatccaaatcggggcggatgccgcgcaggttcgcgtcgagttcgccaaccaggttcatcagctcctccgagccgaaggcctgggctgcgagctgcatcagctccgcgcgctgctcatgcgtcatggagttgagcaggcgctgggccgccgcggaacgctgggcgaggagttccacgagctcatcgatggtgcgcgggttctccgggaactgggcgccgtgtttggccatgaactcctggaagtcctgctccgttgccatgccggcgcggtgcttgcctaagagcacgttcaggtcgcgcagcatctcggcgacggctgcgcggtcctcgtcggtggcgccttcgagcgcctccttcatgccggtgaagcgctggtcgagcagctcgcggccgatgaggtccttgatctcctggtatttttcgcggccttcatgagatgcccagttgtaatcgcccagctcggtcacggcagccgccggggatgcgggcaggttgtccagtgtcatctcgcgcatggtgcggtcgaggtcgtccatgtccacatcgcgggcgagttgaccacgttcggcgagcaccgcctcatcgagaagtttcttagcttcttggatcgtgccgccgaggttggttctttgcagcagctcttgacgacgctccgcaatctggcgaagaaaatcatcgtacccctcgcgccgcaggtactcgcgcatcgcttgttcggcggagtagccgtacatgacgtcatcggcgatggcgcgcaccgccttagccaggttgggcggcggggcgagcgggtccggacccggggtgtacttgcgataccggcgctggctaaccatagatcgtctcgccttcgccggagtccttcgaaatcttctgggtgaggtagagcgcctccaccgccagctcgatagcggctgcgcgctcgccgtcggactgggcgttaaaagaggtagcgatatcgctgtacagcgagccctcgagctgtggtaggccgttcaagaactcgaccgcggtgatgttctcgccggtggtgatgaaggtggagccgtcgagtgcctcaatcagcggggcaaagttgagtcctttaattcgcgggcgcagcgactgcgccaccgcgttgcgcagcaggtactccagaatatcccactcgcgtccctcctcgccgtgctcgaactccaccttgccgccgagcacgtcgacggcggcctcgaggtccaccaggcgcgcgaccggatcctcaccggtcaacgctgcgcgccgggctgcggaggcggcgaccgtttcggcgccagcgatggcgaaacgggccgacacgccggcacgctggttcacagcatcggactcacgaagcgcgcgggtaaaccgggcaagcgcctccatgatgggttgtggaacgacggcggtgagttgcgactcctgctcgatgacgcggatctcgtcgtctagctccaaagggtagtgggtgcggatctcggcgccgaagcggtctttgagtggggtgatgatgcggccgcggttggtgtaatcctccgggttcgcgcttgccaccaccagcacgtccaacggcaagcgcaacatgtagccgcggatttggatgtcggcttcctccatgacgttgagcatggctacctggatgcgctcggctaagtcgggcagctcgttgatggccacgatgccgcggttagagcgggggatcaggccgtagtggatggtctccgggtcgccgaggcggcggccctcggccacgcgcatggggtcgacgtcgccgatgaggtccgcgacggacgtgtccggggtggccaacttctcggagtaacgggccttgcgcgggatccactcgatgggcagtgcgtcgccctcctcctcgatgcggcgcttggtggcctccgtcagcgggttcagggggtgctcgcgcagctcggagccctcgacggcgggcacgaaagcgtcgagcagcaacggcaacgtgcgaagcaggcgggtcttgccctgaccgcgctcgccgaggagcacgatgtcgtggccggcgataatggcgcgctcgacctggggcaacacggtgtgctcaaggccgtggaggcccggccaggggttctcgccggcgcgcagcttggctatcaggttgtcgcgaagctcctcgcgcaccgtcttataggtgtaaccggcggccttcagctcgccgagggtggagattgcgggcttggtcggagtcgcttcagtcatgccggccagggtacgccggggttgtgcggcgcggtgcccgggaacaacgcgtagtagcctggcagcgaaaagggaggagtggttgtcagcggagtacgagaaaatcaccaatcagcaaaacagaggcgacgacgaagattttgtgggtcgtctcacgatgcaagaccccatcgacgattccttcgagtttgagccggttgttatcggactcaaagtgcccgagttctgacctaccatcggcacatgaccgccatctacctcatccgccacggcgagactccgaccacgggcaagatcctgcccggtcgcgcgccggggttgcacctctcggagcgggggcgggggcaggcggaggccgtcgcaaggcagcttgctcacgtggatgcggtgtatgcctcgcccctcgagcgcgcccgcgaaactgccgcacccacgtgcgagcggttcgaaaaggagcttttgcttgacgacgccctcctcgaagccgatttcggcgaatggacaggaaagtcgctgactaagctcgcgaaactgccagagtggcaggtcgtgcagaagcatcctgagcagttccgtttcccgggcggggaatccttcgtggagatgcaggagcgcgtggtggagggcgtgcgcgcgatcgcggcgcgccacccgggcgaggtggtggcctgctttacgcacgccgacccgatcaaggcggcgctcgcgcacttcacggcccggggctggggcgcgttccagacgattcctgcggagccgtgctccatctcggagcttgagctgtgaacaccattgagctgctccaacacggcgaggtcggctttgtggggcagctcgcggactcgtcaaacctgaccgtgctggtcgacctcacactcagcgaggactactgctggggcatcttcaagcctgaggcgggggagcgctacctccacgacttcgagtccggattgtggcggcgcgagcgggccgcgtacctgctcagcgagtggctgggctggaacctggtgccgccgacggtggtgcgcgagatcgagccgctcggcgtggggtcgctgcagtattacgtggacaacgatggttcccactacttcccgctctacgagacgcgcgccgacctgcacccccagtttctgcgcatggccgtattcgacctgctggtgaacaacaccgaccgcaagtcgggccacgttttgctcgcacgctcgcaaaacgcgaaccaagttgaccgcgtgtggggcatcgaccaaggcttgtgcttccaccaggacccgaagctgcgcaccgtgatctgggacttcgcgcacgagacgattcccgacgagctggtcgacgcggtcgaaccgctgcttgaagaggtgccggaagaggtggttgagctgcttgcgccggaggaggtcgcggcgttgcagtcccgagcgtcgcggattgtgcgcctgccgtggctgccggagccgcagtccgagttcccgtacccctggccgctggtgtaatccctactgcgctgggtagcggacgaggaggtcgtcgccgatcaccgcaccgtcactaagctttgctttacttattgatgcaccgtcggacttcaaccccataatgtgatccacgtcgtcgccgtgggcgagaaggtggtcagcgataatccggcggtggcagcgccaccagactgcctccgaacacatgatggcggttggcgtctgcgcggcaatctcgcgcagctctgccagtgcgtcggcgaactccttaccgagcgcgtggtcggcgtagttgtggaagctgcggttttgccagttggcgttgacctcgaaggggacggtcttggacacgttgcgccgccccgccagccccccgatcttggagtatgcgataccgcgatcggggaggttctgggtgagggcgtcgtcgttgaaccacgggtacttccgggagccggtcagcttgcgcacgtcaacgacggcttcgaccccggccgcctcgagcatctgcgcgaattcgttgaactcgaggttggagtggccgacggtgaagatgcgcatgcgtgtcaccttaacaacgccttgtcggcgacgacagcgcccttgatctgcgcaaactggttgagcagatccgcgaccgtgagctcgcgttttgttgcctcgtcggcctcgtagacgatctggccctcgtgcatcatgatgagccggttgcccaccttaagggcttgctccatgttgtgcgtgaccatgagtgtggtcagcccgccttcctccacgatcgagtgagtcaggtcggttacaagggctgcgcgatctgggtcgagggctgcggtgtgctcgtcgagcagcatcaccttcgggtgcgtgaagccggccatgagcagggataatgcttggcgctgcccgccggagagcagccccaccttgtgggtgaggcggttttccaaaccgagatcgagcgacttgagctgctcggtgaagatgtcgcggcgctcgttcgtcagcgcgcggccgagcctgcggggtttgccgcgcaggtaggccagcgacaggttctcctcgatggtgaggttgggcgcggtaccggccagaggatcctggaacacgcggccgacgagccgggcgcgtttgtgttctggggcggtggtgacatcggtgccgtcgataagcacctgccccttatccggccggaggcggccggaaaccgtgttgagcagcgtcgattttcctgcgccgttggagccgatgacggtgacgaaatcgccctttgcaagcgtgaggttgacgtttgtcagcgcggcgcgctcgttggccgtgccggggaagaaggtcttggatatgttgcggatctcaagcacgtgtcttctccttcacagtgaagcgggggatgagcagcgcggcgatgacgagcagcgcggagacgagcttcatgtcgttggggttcaggccgagctggagcgcggcgaagatgatcaggcggtagatcacagcgcccgcgaccacggccaggatggcctggagcaggcggcgctggccgaagatcgcctggccaacaatcacgctggcgaggccgaccacgatgagcccgatgcccatcgagatgtcggcgaagccctggtactgggcgaccagcgcgccggcaagcccgacaagcccgttgcttaaggccagtgtgaggatcttcgtggcgtcggtggacacgccgaaagacgtgatcatcgggccgttgtcgccggtggcgcggatggaaagtccgaggtcggtggtgaggaaccagtgcacgatcagcgccaggaccagcaccgagactgcgaggacggccacgccggcccagttgccgagcagcccgcgctcgcgcagcggggtgaacaccgtgtcttggcggagcaggggcaggttggcaccgcccatgatgcgcaggttgatggaccagaacccgatctgggtgaggatgccggcgagaaggctgtcgatgccgcctttcgtatgcagaagtcccgtgatgacgccggcgaggcagccgatggcgaagcccgcggcggtagcggtgaccgggttcgcgcccgcgataatcagcgccgcagccgtgccgccgccggcggtgaacgacccgtccaccgtcaggtcggcgaagttgaggacgcggaacgtcaggtagacgccgagcgccatcaccccgtagaggacgccgagttcaagcgcgccgatcatgagacggtttcagcctggtccgcgatcgactgcgggatggtcacgccttggcgcttggccgcctccgggttgatgacgtaggagaactcggttgcgctctcgaccggcagggcggcgatgtcggcgccgtcgcgcagcaccttcagcgccatttcgccggtttggtagccgagctttttgtaatcgatgccgagcgttgcgacggcgccgccctccaccgttccggcctcggcggcgacgaccggaatggacttctgctcagccgcctggaccagcgaggagatgccggacacgaccatgttgtcggtggggacgtagaacgcgtccacatcgccgagcgcggttacggcctgcggtatctccgtcacggaggtcacggtttgggtctcgacctgccagccgcgcttcgccgcctcctccttgacgccgtcgacctggatctgcgagttgatctcgccggaggagtagacgacgccgatcttctttgcgtccggcaccagctcagccaagaggtcgagctggtccggaatcggggtggcatcggaagtaccggaggcgttgccgcccggcgtctccagcgaattgaccagctgcgcctccactgggtcggtgacagcggtgaagaaaatcggcgtctcggtgacgttctgcaccatcgcctgcgcggctggggtggccacggccagaacagcgtccaagttctggcccgcgaactgctgtgcaatggtcagcgcggtggcctgctcgccgttggcgttctgctcgctccacttcacgtccgcgcccgcgtcggcgaaggcctccttgaagccttccgcggcggcgtcgagcgccgggtgctgcacgagctggctgatgccgatcgagtacgactcgccggacgcgtcaccggacgcgccgccggactccgacgagcagccggcgagtgcgagcgtggcggcgccgagtgctgcgagcgcgacccgggggcggcagaaagtgtggcgtggcatgggtggatccctcctcaaacgtaggttgcgcatcctggggcggctgcggcaatgagaagagcatagaccaaagggccctaaaacctatacgttttgtgcgcttgttttcgcgagcgccaacagcgcgtccgtgagctgggcaatgtcgtgcggagcgtactcctccggccggtcggtggcgtctttttggtactgctcgaccgggtcgcgccaccgctgcgggatggcgtccgcgccgtgcaacgcgccgaggaaggcgccggcgattgcggcgttggtgtcggtgtcgccgccgaggccgacaaccgcgacgaggtcttcctcgaaggacgtggtgttcgccgcgaaccaacaggtgatgtggaacgcgtggcgcacccagccttgcttgtggacaacgtcgcccggaggggttgagaggtaggtgtccacctcgtcggcgagctccccggcgtgggcgcgcagcgcgtgttgagggtcggcgcctgagatgacgtcggccagcgcggctgtgtacgcggcgttgatgctcaccgggtaggggtgggggtgggtgagcctcgcgtcggtgcgcgcaagctccccggccaccttcgggttgcctgcgtacgccactgcgagcgggctgacgcgcatgagcgcaccgttggtaggcttgcccgcgtcgcgctcgtaggggcggcgaagcgccgcggcgcaggtgcccccgatgtcgaaggggtttgacgacgcccaccggcggtaggcgccgcgcacgtcgtcttcgtcgaaaccgccgcgccgaaccaggctgcgagcgagcgcgagcgcgagttccgagtcgtcggtgggttggccggggacaacgccgtgggggccgccgccggtcagctcgcgcacaccgttcgggtacgcctcgcggatgtcttccgctggttcgaactcgaccagcgcgccgaggttgtcgccgataatctggccgagcatcgcgcccaaagcgcgggaacgggtggtgggtgaggaagtccgtgacgcagtcatgttttcacggtatcggctcgtcccacacacgctgcgcgatgttcgaatctgcgtcgaacacccccagctcacgtggcgtagcatcgtctctcatgaccgagatcaactccgcagacgtttcgcaaaccgtcatcctcccgcagtcgcgcgacgcgatgtttttgaccaccaccatcgtcgagggcggggagcgcgccgcgctggacgccatcaccgggttgagcgggctggtcaacggcgtcggcttccgctggccgggcgcgaacttaagcgccgtggtcggcatcggtgcgaagctgtgggaccgcctgttcgttgtggagaagcctgagcacctgcacgacttcgtggagcttcagggcgcaaagcaccacgcgccgtcgacacccggcgacctgttcttccacatccgcgccgacagcttcgacgtcgcgttcgagctggctcggcgcattaaaggcattcttggcggcgcgatcggcgacttcgacgaagtccacgccttccagttccaagatttccgcgacccgctcggcttcgtcgacggcacggagagcccccgcggcgaggagggccgcgaggtagcactgatccgcgacggcgtgtgggccggcggcagctacatcgtggagcagaagtacatccacgacttgaacgcgtggaacgacttgcccgtagaagagcaggagcaggtcatcggccgcaccaagcactccgatatcgagctggacgacaagccggtcaacagccacgtggccgtgaactcggtggaggacgaggacggcaacgggctggagattgtgcgcaacaacctgaccttcggcgacgcgttgggcaacgagggcacctacttcatgagctacgcgcgcgacgtgcgggttaccgaggtgatgctgcgccgcatgttcatcggcgagccggagggcaactacgaccgcatcctcgatttctccacggcgctcaccggctgcaacttcttcgcgccgccgcgcgcgttcatggaccacgccgcagacttcgcccgccccgaagtcgtgggcgggcaggacgcggctaaccaggacaacccggcgcagcccgcaatcgacttgccccaggccaaggccgtgttcgggagccgggagaacgcgccggtgtcgcacaacgccgagcgcgctcagcgcgcccacgacatttactccttggcggtgaagccgggggagcaggaagccgagaactagagctggggctagagcgagatgaccgccgagatcccgccgccgggcagcggctggatttccaaaccgccgccgtgggcggtggcgatcgcggccaccagcggtagccctagcccgtggccgcggctgctgcgcgagcctgcgaacggctccgccatccgcgcggcgtcctcaacgctgacaacctcgccgctgctcgccacctcgacccgggtcctgcccgcggcgtgcgcaagcgtcagcgcgctggtgcccggttcgccgtgggtgaccgcgttgcgggccagattgtccacggccgttgcgaggagttcagcgtctccttcgacggccacgccgtcggcaacatctgcgcgctcgatgccgttcgcgcgcgccacgcgccggcatatctcgctcagatccacgctctcgcgctgcaagtcgtgacccgattgcacgcgggccagggtcagcagcgccgcgactgtggcggcgttgcctgcgttgacctcccggactcgctggagcgattcgcgtagctcaccctcggtggcgtctgcgtcggagagggcaacgtcggctaacgcctgaatcgtggcaatcggcgttttcagctcgtgcgacgcgtttgcggcgaaacgctggtgcgcggcaagagaggccgcgagcgagtccagcatcgagttcagcgcgttcgccagatcgcccacctcgtcggcggggcccgagtacgccacgcgcgttgccgtgtcgcctgaggtgacggcgcgtgcgtcgcctgcaatcgagcgcagcggcgcgagcacccggcccgccacgaaccacccgaccgcgccggcaagggcggtcagcacggcgagaaccgcaagcgagatcgtcaccacagttcgcaggatctcttcggtgacggggatcgcggcgtcgatgaccgcgccgtccgcgccactgaactcagcctgaaacggcaccggggtaaggcgcaggtacgcgtagaccagaccgatcagcagaatgcccactcccaacaccgtgagcacgaacatcacggtgacccgggcccgcagactcagtcgcatcagtccacctccggggcggcggcgaagtaacccgcgccgggcttggtgtggatgatccacgggtcgccgagcttgcgcctcaggtgcgagatggtcacgcggggggaattggtgaacgggtctgcgttttcgtcccacgcttcctccagaagctcctccgcggagaggacgccgccgtcggcggacatgagcagcttaagaatcgcgaactccttcggcgacagcgcaatctcgcgcccgccgcgggtgacgcgctttcggaaggtgtccaggcggacgtcggcaatccgcagcacttcaccccgcaccggagccgcacgtttggctagcgcctgcacccgggcaatcagctccgcgacctcgaacggcttcggcaagtagtcgtcggcgccgagggaaaacccctccagccggtcgtcgagagtgccggacgcagtcagcatgatcaccctggttgcggggtaatcctcacagatgatgcggcacacctcgtccccgtgcaccccaggcaagtcgcggtcgagcacgacgacatcgggcttgtgcttgtcgacgccctccagcgccgccgagccgtcacccaccacagagacgtccatcccggcgcgcgcgagcgccttgcccacggcctccgcgaggtaaacctcgtcgtccacaacaaacaccctgatcgtcatggaagaacacgttaacgctctcgcaacacgaacctgaatagcctctcacgccatgcagatgcgaaaccgaacccaaggccgcctcgtgggcgtcgacgttgcccgcgccgtggcgctgatcggcatgatctgcgcccacctgacctacccggacggcgtgctcgcggaggtgctctacggattcccgtccgcgctcttcgccttcctggccggtgtgtccatgtcgctgatggcgagaagcggggcgcgcccggcgcacttcgttgtgcgcgggctgttgctgatcgcgctgtcttttctgttgagcgcgataccgacgcagatcgtgatcgttttgggcaccctcggcgcctgcatgatcgcgctcgcgtgggcgcagcggcttccaagccgctggctgctcgcgcttgcggcggtgatgacagctggctccggggtcgtccccctcttcgtctccccgccgctgatgtgggcggtgctgatggtcgccggcatgctgttccaccgccacctcatcgaccgtccgaattacgtggcggctgcggctgcggtcggaggcgctgtgatgacgctggacatcgtggcgcgctggtatgcggacttgccgtactacttcactgcccaagggcacacgggcgggttggtggacgtggtggggtctgcgggggcgtcgataagcatctgctctcttagctgccttgtggcgcggccgcggcaactcgtgctgccgcgcatggggcgcatgccgctgacgctgtactgcctgcatatccccacatccctggtgtgcggcgcggcggtgagcgtgatcgcagcggcggtcatcgcaactgcctggctcgccgcgtttccccgcgggccggtggaagaggccatgcgccgggcggtcagcgccggcgtgggtctgatcgacaacttggaaaggaactaccgtgaaaaaacttctctacccgctgctcgccgcgagcgcgacctgcgcaacagcagctcccgcgctggcgatggagtcgaccacgttcgcaggcgacacccctgaggccgcgcccgtcgtctccgtgcgcgtggaagactccgacccagacgagggtgtgtgcaccggcaccgcgatcgccgagcactgggtgatcaccgcgcgccactgcgtcgaagcggcgcgtaaacccgcagggtccgtgcgcaccgggcagggcggcgaccagaaggtgtacgaggtcgaccgccacgaggtcgcaccggagggcgacatcgctctgctgcacaccgcgcagccgatggaactcgaccacttcgccgatgttgccgacgctgtgcccagcggcccggtgaacatctacggctggtcttccgacggatctggcggttcgacccggttgccgtcggctgaagccgcggtggagggggagtcgccgctggcgctcttcggtgcttccagcgcgctgcatgtcgcgctgaagaacggggcgcgcattcagccgggcgactccggcggcgcgatcttcgccggcggcaaggtggccgggattatgtcggccgggctgttcgaggacccggacaacccgaccgagcaggagatgacctccaacgccgcggtgtcggtggcgccggtggcggaccaggcggcgtggattagggacacggtggcgcagaattccgccggcgagggcggggccgccgccgagggcagctccgacgcgggggccggcggctggctgccgtggttcgcgctcgggctcggcgcgcttgcggtcatcggcgccgcgctgtgggatgtgcagcgaaggaaggccgccccgcttgcgtagttagcgggcttaaccgtggatctcgacgttgttgtaccggttcacccgcagcgcgcccatcggcatcgaggcgtcggtttggaaccagacgtccgacggttcgacggtgatcgtgacctgcttgcccacgagcggcgcccactcggtgccgacgatgtggtcgtagcggctccactccctccggcccaggtccacgtactcggcggttctcgtggacggctcggggcggttgtagtccgtgaactcgcgtggcgcatcgatctcgagcatgtagtactcgctgtccatcgcctcgccgttcggtgtgccttcgggctccagctctgccgcggtcttcatcaccaccgtgccgctgatcacctcggcggggccctcgaccgggttcctgcgctcgatttccggcagcgagacggtgagctcgcccgcgtcgagcggcccgcggtccgccaccggcgtccagtcgacgacgaggtgcagcgcaggcggcgacatcgcgtttatcttgttggcctcgccttcgggcaccaaagtattgccctcaagctggcaccacacgctctcgccgtcgcccgtgccgctggtccactgggactggtacaggccgagcccgagctgcgaggcgtccacgcctgcgcggtacccgccggcgccggccgcgccgtacgtcaggccgttcgaggcctgcgtcagcgacccgctgtcgacggagaacaccagcacgcgggcgaaccggttcgagtgctcgtcggcgctccactggctcaagagcagctcgggcgcgccgccgcctgtcgcctccaccagcgcgtagttgtagtcgccgttgggcaagtactccatctcgatgccggcagggttggcaacgtcgaaattgtatgtctcggccgtgtccagcaccgccgcgtactcgctttgccaatccacggcgcttggcgccacgggcttgtccatcaccgtcgttaccacctcgcccgagtctggatcaacgatcgccgttgcggtgacaaacaccgtctcaggggaagcggaacacgcgctcagcaaaagcgggagggcggcaattgcccggaagcgtttcataaatgacaacatagagcagatgatcttctccggcattgacctcgccgcggatcccgcaaagacgggcgcggcgacgctcaagacctcgcgcaaggggccggtgcttgtcgacgtccacctcaacacctccgacttccacatcttcaaccacgttctcgattccgacctcaccggcatcgacgccccgctcggctggccccggttgttccggaggttcatcaacgaccacgccgccggcgatttagtcagccgggacgtggggacggaggagcggcgcgagctggccaaccggttcaccgacctcgaggtgcgccgcgttgctggcgtggtcccgttgccggtcgcggccgagcgcatcgcctttcccgtcatgcgctgggcgggtgtggaggcgcagttgcgcgacgagcttgggagcgaaggcgtccgccgcgacgggttcggacgcgtcgccgaggtctacccggccgctgcgctgaagatgtgggggttgcgccaccgcggttacaagggtggcagcccggccgcgcaggaggcgagagtggaaatcgtcgcgtcgctcgcccgcgagcgccgcttggattgggcggggtttgaagacgcggccgtctacagcgcagactgcctcgacgctgtcatcgtcgctctcgtcgcctctgagatcagcgcaggggcctgcgttccgcccccgaaagagcacgagagcctgattttggaggaaggttggatctggatcccgcggccagattaatccagcacctccacgtgctcggtgtcgatccagagctggctcccgaacggcaaactcaaatctgaggagtagccgtagcggttcagcggcgaccacacttccacccgttcgcccacgtattcttcccaccccttcgactggtccaggacgccggaggaggagtggtggacaaatcccagcctggcaaacgggctttcctgcgttaccgtgctgcccgccttgttcgcggcgacgctgaccggggagtcgaaaaccagcacgtagtagatgtttcgcgggtcttcgccggctggggtttcgcgtccctgcgccgctttttcggtcggccacgcttccacgatgccggtgaacctggcgttgccttgctcatctaacgtcacgggttcgtacccgctgtccgctcggctcgaaggcgcgagtgcttccgcgtcttccgccacctcgggttcagcctgctcgccctgctcgccctgctcggcctgctcagtctcagcagccacccactgcgtcgaggtgacgaacaccgtcgctggttcgccgccgccggcgcaggcgctgatcggcaacacaaaccctgcggtaaaaagcacaaccgcgcgacgtaaacgcatgatctagaatttagtcgaggtacacaaatccatcagtcggggggacgatcgccgtcgcgtacggagccgacgggtcgttagcgaaccttgtgacgtctgggtcgagactaagctcgatccggcggcctgcgagcttgaagtttgcgccctgcgtcttggttccgagcaggatcgtctgcgttgtgaccgtcgacggtgagctctccgcccctctgatgccagagatggcggctacctcatcgaggtggaggaccaagtaccgctcctctgggccgtactggaagtccccggcgagggcggccagttcctcgcccgacatgtcgcgcacggtgcccaccgctgagcttgcaggttttgctggggcgaccttgtccggtgcaactttctccggtgcggcatcggggaacggtgtgtattcggtaatagaggtcgcacccgcgtaggtgggtttgccggcgtgcagcgcggagcggtcagttgatttcgtccacgcgatgaaacggtggtcgggtagtaagtcggcgttttcgaactcgacgctgtccgaagcagcagtaagggagcggccgctgagcttgtacagcttggagtaggcgtcgggctgcaccgaatgggaatcgacctggtagaggccattgccgctttcagacgcctccacacgcgcccgcgaacctcctgcacctgaagcgcccgcaatcaacacgtcggtggagccggctgctttaccgtccgcgccaaccgtgaacacgatgatcggactgtattccttgctgtccaccatcagcagcatctcgggggtatcgtcgccggtcatctccacaagcgcgtagtgataggtaccgaccggatcgtagcgcgcagccgagttcaccggatagtctcccgggtggtcgagcacccaggcgtactcgttcttccacgcgccggcagccggggttgtcgccgactcagccgcctcggacgcggcggcgctgctggcggtgggcgtgccggcagcttcaccgggcacccattgggtcgaggtgaacagaatagtttcctgtgtgccgcccccggcacaaccggagaccaccgcggcagatccaaccgcgcccaacacagcaaaccgacgcaaacgcatgctctcaacctacccggatgtaccccacctgcgactggtggggcgaaatccgcgccgcccgtgccctcgcgctagaagtgcatacctactgttgtagttccccaaattctcatgagcttttcggccggtatacacaactagacctacaactccggcttcgccagaaaatgcacagacctcaggcacacgtgttcgggtagcatggcgtcacctcgaagaggaaaacgcacggatcaaaggagtgccacatgacgaacccgcagaacttcaaccagcaggaacccccgttcgacccggattacgaccaagttgcccccgccgagcagccggccgagcagcctgctgcggacggccagcaggcagcagccggccagccggagccccagagccctgcccagcagaacccggcgcagcctcagcagcttggccagcagggccagaatgtccaggccggtaacggccagaccggctacgagcaggagatgctcggcgccaccggcgacgcgcaggacggcaacttggagaaggacccttccgagtgggtctccggtgaccagccagcgacggaggcgcagaagtcctacatcgacaccctggccaagcaggcaggggagcagatcccggcgaacctgaccaaggcggaggcgtcgcagcacatcgaccggctgaagaagatcaccggtcagtaatactaggggccgaagctaggcccctttctttttgggtttcttgtccccgctgcggctgtccagcgaggccttcagcgccgccattaagtcgacaacgttgtcgtcctcgtctgcatcctccggtttctcgccgaaggtggcttcggtgtcaagcgtatcgccctgctcgaactttgcgtcgatgagttttcgcagctcgacctggtagtcgtcctcgaactcctcgggcgtgaagtccgaggcgtaggaatcgaccagctgggcggagagcttcatctccttgtccgagatcttcgcgcgcgattttactcccttgaactggccgtcgaagtcgagttcgcggacctcgtcggcccacatcaagccctgcagcacgatcactttgcccaccacgcgaagcacgcccagccgcgtcttttggcgcaatgcgaaacgcaccaccgcggtcagatccgactccttgagcgtctggcgcaacagcaggtacgacttcggcgtcttgccttcgggcgcgaggtagtagctcttctccagcatgatcgggtcgatctggtcggcggggacgaactggactacctcgatctcgtcgttctcggactccggcagcgccgcgaaatcttcgtccgtgagcacgacggtgtcgccgtcttcctcgaacgccttgtcaatgtgtttgtagtcgaccttctcgccgcagacttcgcaccgcctctcgtagcggatgcggcccccgtcttcgtcgtgcacttggtgaaatgacaagtcgtggtcctccgtcgcgccgaacgctttaacgggcacgttgacaaggccgaaggtgatggaaccggtccagattgcgcgcatggttggaaagtctacggatctttaggatgggtgcatggctgcgcaggcgaagcagggttcgaaattccaggtgggcgaccgccaacttaaggtgaccagcctggataaggtgctctaccttgaaaccggcaccaccaaggccgacgtgatgcgctactacctcgaggtcgccgacgtcatgatcccgcagatcacccggcgacccgtgacccgcaaacgctggccggacggcgtgggcgggcagagcttcttccgcaaggatttggaggactccgcgccggagtggatcgaaaccggtgtaatcgagcacaaaacctcaaccaacgactacccgttgatcgacgagccggccgcgctcgcatggctggcgcaagtcgcggcgcttgagctgcacacgccgcagtggcgcttttccgcctccggcaaacaggaaaacccagaccggatggtgctggatctggacccgggccccggagtcacgctggaggagaccgccgaaatcgcgctgtcgtgcaaggacgtcctcgacgggatggggcttgtaagcgtccccgtcaccagcggctccaaaggcatccacatctacgcagggctcgacggcaccacggaggccgagcaggtgagcaaggttgctaaggcgcttgccgacgctctccagaacgaactccccgaccgcgtcacctccgtcatgcgcaaaacggagcgcgccgggaaagtctttttggactggagccaaaacaatgggtcgaaaactactgtcagccggtactccttgcgcggtcgcgaacggcccacggtggcggccccgcgcacctgggacgagatcgcggagcggggccttgcccatctcacgttcgatgaggtgatcgagcgcgtccagggcggcctcgacccgatcgcggagctcgccgcgccgcgcgaggacaagctggctacgtaccgctcgatgcgcgacgcgacgaaaaccgccgagcctgtgcccgagggcacgccgcagccgcgcggcggcacgccgatcttcgtcatcggcgagcaccacgccaggcgcctgcactgggatttccgcctcgagcacgacggcgtactcgtcagctgggcggtaccgaagggtccgccgctcgacccggaggagaaccgcctcgcagtgcagaccgaggaccacccaatcgagtatgcgacgttcgaagggaccatcccgaagggggagtacggcgcgggcgaggtcgcgatctgggacaccggcacctgcgagatcgaaaagtggcaagacgacgaggtcatcgctgtgctcaccggccgacccggcggcggcctcgggggcgtgccgcggcgctacgcgttgattaggactgagggcgacaactggctgctgaagtttatgaagcgccagcccaccgccgaacccgcccacaccgccg

SEQ ID NO: 8 - DNA, 187760 bp, Corynebacterium cassirii
  source 1..187760: mol_type = genomic DNA
ccccaaccccaacccgagcccacgccgccgccacccgcgcccggttcggccgtcggcgagcgccagccccaaggcttcggcggcggcagcgctccgggtggcagctcccgctcgggcggtagccccgctgcgccgcaggcggagttcaagaccacgtccgcgccgcacgcgctgctgcttcccagcctcatccttgcgctgattgccctgatcctcgacgcggttgtgggctttggtccgctgcgctccatcgacacccagtggggcgtgctcaccggtatcgcgtgggcgttgtccggcatcgtgggtgtgtccgcgctcggcctgtatttcaccaagaacaccgaggcacgcgcgaacggcctgtacgaaatcgtcggttggaagcagaccttgttctacgccacggtcgccgcgctggtggttgccgtggtcgtctcgtcggtcatgttcgcgctctggttcggaaggcagtaacccgccatgtcatttcatgtttccctgcgccgcgccgccgcggcgatgacggccgcgtccctcgcagcgatttccaccgcgatgccggctgccgcccaggctccggcccccaacgactccctgcagcagctcggcgcgtgcatggcggagcgcggcgcgctcgacgtcgtgatgcttatggacgagaccggctcgctcgtcggcgagttcgtcgacgaccgcgtggacgagtccctgccgggctcggacgacgagcacaaccgtatcccggcagcccagagcttcgtcgacgagttggtggaccgccacgccgacacgggcgtggacatccgcgtccgcgtctccggcttcggccaggagtaccgctccggcgccacggacccggccaactacggcgagtggcagaccctcgacgagtcttcggctgaccgcgtcaagggcgaaattgaggacttccgcacccgcaccgcggagctctacaccaactacgccaacgcgatggagggcgcgtacaacgacttcgcccgctcgggttccgcgaacccgtgccgcatgctggtcacgttcaccgacggtgaactcaccgccgaggagggcgcggaggttgctgaggagcgcatctgccgacctggcggaattgcggaccgtttgcgtgccggcgggattacgaatgtggggattgggttggcgtcggcaagcaagccctccgacttctccttgctgcggcgcatcaccgaggctgaaggcggcgcgccctgcggcgaccagcccgcgaacggtaccttcttcgaggcgtctaacgtgggtgcccttttcggcgcgttccgccaggcgctttcgtccggccgcgacatggtggtctccggcccggtgggggagccggtcgagttcgcgctcgacaactccatcgacgcggtgcgcctcaacgtcatcgctgaggagcacctcggcccgaacgcacacgtggtgctgaccgcccctgacgggtccacgctggatctcggcgactctggccgcggcgagctgcagggcgcggctgttgagtgggtcgcgactcacgagccggtgcagcgtgtcaccggccgcatgcgcatggcagacggccaggactggtcgggccgctggcaggtcggtttcgccggtgtcgacgacgcgcacaaagacagtcagcacatctccggcatcgagatccagcccgacttgcaggtgcggttcgccggtccggattcggaagatgcgggggcattgtcgcttttcgacgaccagccgctcaccatccaactcgtcgacggcgccggcaacgtgcgcccgatggctggcgaggcccgcacaaccgtcaccttcacgccggacgggcaggagccacaggtgctggcggacaacgccgacatctcctccggctcgctcgaggtggaagcgccgaagctgaacggcgcgccgctttccggccgcctggaatcgcgcaccacggtcaccaccgcgggcgagccgggcacgaccttctccccgttcatcaactcgcaggcgctgagcgtttcgccgcagaacctgccgcagctcgccggcccgatccagttcaactcggactccgtgaccggcgagggcgaagtgacggtgaagggcccgggcaaggtgtgggtcgagccggggacgacattgcgcgccgacaccctgcccgacggcgtcagcgcggtcggcgtcgcttcgacgcacgattccgcagccaacgcgctcgaggttcctgctggccagaccgcgacgctgccggtcacgttcaccgtcgacgagcccaccgagggcatcatcaacggcgcagtggacgtcaccgtcgcagacgtcgacggcgcggttgagccggcgaccgtcccggtgtccgtcaacggttcctacacggtgccgctgaacaccgcgaagttcaccggcgcacttttgggcacgctgcttgcggcgctgctgatcccgcttgtgatcttctacctgatccgctacctcaccgcgcgcatcccgacgcgccgccagctcggcgcgcagcgcttccagatcgatgtggacggcgcgcaggcacgcttcgttaacggggaaccgaagctgtctacccaggaggcgctccgcacgcctgcgacgctcacgccgacgtccttcaccgctttccagtacgagggcacggtgcgcggcttccacccgaacccgttcgcggacgcgccggtggtgcttaagcagacgccgtccctcagcgaggacggcgaccaggtgaagggcgcggccaagctcccgctcgcgttgaccaacacgtggttcgtcgcgccgagcagccgcggaccgcaggcctacgacgtggttgcgctgattaacccgggcaccccggaacagcagctgacccaaacggccagcgagatccgcacgcgcgcaccgaaactcgcgcgccagctgcacgagacccgcgctgcagagaccactccgacggagggcgccgcgccgggcaagaagcgcggtctcggcggccgcggacgcggcggcaacgacgacgcaaaccagcagatgccgccaactccaccgaccccgccgacccagcagggcggtaactacacctcgggtggcttcggctcgggcaaccagggcggcccggggaacaccggcggcccggggaaccagggtggcttcggctccggctggggcgcctccggcggcaacccgcacaaccagggaggctttggctcgggcggatggggcagctccggcgggtccaacccgggcgggtccaacccgggcggctaccaacctcgaccgggcggctttggctccaactaactcaatctccacacgcacacgcagttttaaggaacacacatgtacaaggttttcgtagtcggttgcggcggcagtggcgccaagacgatgtcctacatgatggatcagctcaaggcgacgctggagaagcaggcgccccagtggtggtccaagaacaagcgtctcccggacgcgtggaagttcgtctccattgacgccccgctggtgcccgaggtggtggagaagtcgaagctgccgagcgtgaccgaggccggcggcgactacgttgcctgcggcaccaacgctggcttgagcagcgttcgccgcaacatcgccgacagcgcggcccgcgaggcgaagctgggcaccctgtccaactgggcgctgaaggacggctccctagacacgctcgacgtggccaacggcgccggacagttccgcggcgtgggccgcatgctcgtgctgaaccgcctgaaggaagtcaacgctcagctgcgtcgctcctgggcagaagtgatcagcgccgacactgacgcggacctgatgcagatcgcaaccgagaccggccaaaaccgcgaggtcgccggcccggtcgtgttcatcatctcctcgatggccggcggctccggcgcgtcgatggcggttgacgtgtgccgcctggtcagcgccctgccgggtgtgaataacggcggtgtcggcctctacatggtcacccctgacgtgttctccggcggcgagactggccagatggactccttcgccggcacgaacccgaacgcgctggccatgttcgccgagcttgcagccggccaggccggggcgggtgtgcagaccgacgccgccacctaccaggcgatgggcttgaacatctccatggaggacattccggttggccgtatcttcccggtcggccgcaccgtgggtaccgacgacaagatcactgagatcggcaacggcaccccgtcggacatctaccgctcgcttggtctgggtctcgcgtcgctgttcaccgaccacctggctatggcgaactacgtcgcccacgtgatcaacaacccgcagccaagccgctctcactactacggctggggtgcaaccgagtacccgttcgtgccgtggggcactttcggttacgggcgcgtcgcgatgggccgcgaccgctacgccgagtactctgcgcaacgcctcgcgcactgggccgtcaaccacatcaataacggccacttcgagaaggaagaaatcggtaaggacgaggcccagcagctcgaggagcgcgtggcgaccaactggggtaccttccgcgaccgcatgaacgcggtgttgccgctggtcggcagcaagaaggaatggatcgagcgcaacttcggcggtgtgatcaccggctggtcggaggctcgcttgaacgagacaatcggcgccatcccgaacgcgaacaagcagcgcggcaacgagtggctgaacgtggtctaccgcgagctcagcaacgcctcctaccgcgtcaacaacgagttcaacgcggaccgccgcgccgaccgcccgttctacggcgcgctcgttgaatgggcaggcccagaagcgctgcagagccacctgctggacacgctgcgcctcgaggttggcaagcacggcgccgcatacgccaaggagcttctgagcaagctgcaggccgagctgaaggttgtcgtcgctgagctggaggacttcccggatcacgtgtggttcgagttcaagggcccggtgcacgacaagatcaacaacaccggcaagatcccggacagctccgagttctccaggcagatctacgcccacatgctgccggagttccgcgatggcgcagtcgcgttcatcgcccgccagatggccgagctcctgcgcgccttcgacaacgacttcctcaaggcgctcgaggcggaaatcacccgccagcgcgaggagctgcgcagccagtgcaccgtcacgaccgacccggagctgggtatttcccgtttgcagacgatctacccgaacctctggccggctgagtccgacggcgatgtggactcgcgcttcggcgcgccggcaaccgaggcgtcgattacaccgcgcagcgagttccgcgagcgcttcgtccacgacatcgagaacgcccgacccaacggcggccaggactccgtgtccttcaagaccgggcttgccctcgcgggtaaggccgtggtcgccggcgagtgggagcagggcgccgacaccgagcccgcgccgaaggacctgctttccgtccgcgacggcatgtggtgggtcccgcagcaccacaccatcgacccgcgcaccggcgagcacctggattaccgcaagccgcgcttcgacttcaagatccgttcccaggacgtccttgaccgctcgcggaggttcatcaaccgcaagggcacctcgttcgaggccttcatctccgaatcgctcgccgagtacatcgacgccgacggctacccggcacacgagcgcgagcgccgcgagaacgacctggtgtccaagttcgccctcgctctcgaactggcgctgccgctggcgcaggtggacaaggctgtgcttcaggccatgcttggccaggcgatctcctacgacttcgtcttcaccaagatcccgttcaagaaccacgcgcttgaggcgcgcctgacggacgagctggcgaagttcaagggtggcgccgccaacgcgcaaagccgcaagtcgcttgccgacgccttcggcaacagcggcggcctgcgcgaaatcagcatcaccggctcctttgagaagtacccgccggtagtcttcagctccgtgctgccgcaggcggcggcgcagtgggacgcggcgtcgtcgcaaaccgcccgcgccgatttttggcgcatgcgccgcgcgcgcccgctgtccgcggccctgccgatgagcgacatggagcgcggcgcgatgatccgcggctacttcgtgggcaagctcaccggccgcatctaccactccgaggaagtgcgcgtgtccgcggacaacgagccgatccagatttacgacgtgcgcggcaagagccagaccaaggacaagtggctgaccatcgccacgccgcttctgaccccgccgagccagatgggccaccgtcgcaactacctgccggcgattctggagaactcctccatggcgtgggcgaagatcaaccagcagccggtgatgggctccatccagccctacctcgcgctgcgcgcgctgtgggacgaaggcgagatgccgacccagtggcgccaggacggccagctctacggcggcgacggcattgccaaccacaccagcggccaggaagtgctgcgccagtggctttggtccggcgagcgcaagaacggcgagtacctcatggtggaaggcaccggcccgaacgtgagcgtggaagagcgcctcgccgcggcgaagaagtggctgaacgacgagcgcgagctcgccgtggcctacagcccggcgatggtcggcagcgacgacggcttcctcggcggccgcacggagaagccgtacggtgatgtgaaggacctgcagatcgccgcggcgctgccgctgttcgcagacctcgcgccggactacgtctccgcgatcgacgacctgttgttctccctcgactgggcgtacaagacgggcgcgccgtccgcgggcggcggcttccagccgggagccccggcaggcccgacgggccaggaattcaacggtggcgggccggcgatcagcatgcccggactcgactagggaaatgaagtaggcacggaacatggcagaagcaatcagcatctttcttcacaagggtccgttcgcgcgccgcgtgcgccagtgcgtggccgatatggccgccatcgggcttgtcggcgagagcatctggatcgacgccgaggacggcagctacggaaccctgatcgggcacggcaacgccccggagcacaaccacctgacacgcctgctcaacaacgtcggcggcgcgccggtgcacttggtcgcgctcaacgtgatcggcgaggacagcggcgcaggtgtgctggcccaagacgagatccagcgcctgcagtccgagatccgcaacacaggtgtgggctacgtggcgggtgcggcgaacaccaatttgatcgttgcggaggttggggcgagcgtcgataagcaattcccgctcgtggctggtttcagcaacctgctgctcgcaccggaggaatccgaaagcccggacatcccggcgtcaacggtcttccgcgccgacagtaacgacccggaggagctcgcgctgtctgtggcttgcaaggtcgcgggcctgtgcgggctgtggcagggcgcgcagcacatcccggtggtgcagctgggcagcgacaatggcatccggctggtgcgcacgttctaccgtagggtggacgcgcaggagattcagaagctgctgaaagcacggcttttcgacgtcgcgcagctccccaaagtcagcctcaccgccgggggcaaccaggtgcacgtcaccacgattaacaaccaagcggcgacgaacgagcaaatcgccgcggaggtgatcgcgcacaacgcggcgaacatcgaggcgccgcgcaaggaggccgagaaagaggccaccgagaacatggagtcgctggccgtgatcaagaagatcggggcgctctacgctcagaacctcgtgcgctggccgggaatcttcttcagcaacgtgtcttccggttttaagcacctcgtggagaaccaggtgcagggcatgctcggcgaggattccagcatccgcgtcgggaacctggaaaacatgccgaaggagcgcccgcagggccgccagccgtcgagggatctggacttcaaccgcgaactgtaccggccgatgtgggaggaatacatcgacacctcgttggcgctcgcggacgcgaacccgcgcggccttgtgaacgacgccggccagcccccgtactacctgcagtcttccggcggcggggcggccaccgcccgctctgccagcgacatcatccccggcccgagcacggcgttcaccgccgagcagctgccgccggggttgcgcagcaacgcagaggagctgccgctgcagccctacgacgtgaagggcatccgcgggttccgcgcgcgcctcggcgcggccaactcgcgcggcgtggacgagactctgcagcgattcgacgcctgggagcgcaagcacgccaacagtctggccgcccgcctgggcaaccagcttgattggaatgagcgccgcctgtgggacgattaccttacggcccgccgcgattacgaggacgcgctggcccgcagccgaaacgcgccgaacggaaacggcggggcaggtatctggcgctggctcggctacgtcgtgttctggtccggcgcaatcttcgcgctggcgtggggtatcggcaactggacggcggagcagaccccgtcagggcgcctggtcacttggggctgggtccagaacctcaacaacgcatcgggcaagaccatcttctggatgttcttcatttggttcctgctgtggctcatctgctggctgatccaagtctggctgttcaccaagcagatctttgaggtcgcgaccacgcgcagggacatcctgtcggaagagcgcgccgcgaagatcaacatggaggctgcgtggcaggcatacctcaacattcagcacgcatacctgcagttcctttcgatctcccggatctacggcgcgctcttggagcgcccgttcggcacggtggccaacgctgagaccaagtccccggtgccgatgaaccagatgccggcgtcggtgctgatctccaccgccgagccggatgaagccgcgatcaacaaattcgcagacgacatccgcggcgagtactaccgccagggctggctggacgaacgcgtggatgtgggcctgaagcgcgcattcgacatggtccaggtgggccacggtgaccagggcggcgacaagcactcctacctccgctcccgcggccagggcaccggcgagatcctcgacctacttgcccaagccgtgtcctcgccgcagttcatgggcgaggaccgcaccggcaacaagtggaaccaggtcgtggcgcgcctcgagcgcaacgagggcggaaagcgcgacgagctgttggcgaagcagaagtactacagcgggggcatgctcaccagcgcccgcgagatgccttccctcggcgcagtgaaagattccggcaccttcaacggtgagttcatcactgagggcggctgggccgccggcaccgcgaacaacgttgaccaggccctcaccgaccacagcgcgacccgccagtccggcgaccaggtcggcgcggcggagctgctggtgcagtacggccgcccgggcacccgcgactccttcgtgcttcgcggcaacgagggccaggcactcggcggcggcagcaacgtgcagctgccgggattggattaagcgatgaaagaagatctgctcgccttaaacacctggcgcgaacaggcgctcagccgaggcatcgccaaggaggagctgccgtccgcgttcgagctcggcatcttcctgcgcgcgaaagacgatccggaaaagtggcaggacaagcccacgttgagcaagtggagcgagtccctgaccaaactgctgcaggctgtggccaccggcaactttgtcaagggcaccccgctgccggaccttttctttcgccccaacggcggagccggtcaagccggcgcagccgacaaggacggcagcaacccgccgcgcacagctcaaccggagccgccggcgcagccgaagctgaagcggcgcccgtcgagtgccgagctcaagccggagccggcgcctaccccggaaccagagccggcgcctacccccgagcctgagccggctccggaacccgcgcagctgctcaacctgcgcccggaggatttcgcccgccgcaacgcgctcgccggcgacccggaaaagctcccgggcggcgaggtcaccgtacgcgctcgtgcggacgagccgggcacgctggaggtgtcctgggtcgccccgtcgtccggtgatccggtgcgtatcttccgcgtggtgagcctggatatgctgcttgccagcgacggcctagagccgaccaacggccgcgtgcgcgcgattacctccggccagctctgggtcgacgacgagcgcctcgaccgcgctgtgcgcacgttccacgtgtgggtgaatgagggtgcgaccgaggcggaggccctgcgcgcgcagccgaaagtggtcggcgtgggcgtgtacgtgcgcccagtggacgacttccacgtcacctacgaggacggacgaatctacggcagctacgccgaggtggacgggacctccagcgtggagatttccctgatcgaccagtaccagggcttggtcgagcaattctccaaggagaagaacttgcgcgggttccagctggacccgcagtacaccggccgcacctacgtgttcaaggcccgccgcgttgtggaaaagcacacgtcggactactccgacgagcaggcggtggaggtgccggcggagctgacccgcatctccccgcagatccagcgcgacggcgagcgcttcgccgtcagctggacgtcgcccggcgcgggtgaggttcgcatctatcgctcggcgcagccggtggcggaaggcgccgccggccagctggtggacgcggacaatctctctgagtacgggctgctccccggcgactggtacaaccggcttgcacccgcggcgaagacagacatcgacctggactggaaatccgacgcgttcgcgatgtacatcaccgcggtcaacgtggtggagaaccaggcgatgatcggtgacacccagtcgtgggtacgctgcggcaaagccgagaacgtgcgcatcgctgagcgcgtcaccgagcaggtcatcaccttcacgtggcctgagcaggcttcgggcgttgagttcctccacaccgacccggagagcaagcagggcctcgacttacgctccgcggaggcgatcaaggcggacagctcggtcatgcacatcggccgcatcagcgagagccagtaccgccgctccggcggataccgcgctgagctgcagcgcaactcctgcctgatcctcatgccgtaccgctcccaccagggcaagacggtctacggcgagccgacgctggtggattacccaggcctgatcaagcttcgctacgacatttttcccagcaggtacaacgagcagcagctgcttatttccatcagtgcggaagagcagcgtgacaccgcgaccgcgagctttgtgctgctggcgcaggagggctttttgcctgtcgacgccacccgagacgagcagcgcgtctccgtccagcgggtgtcctccgacggaactccgctggaggacagccgcaagattttccgcagcgggcagccgcgcatcaacaacccgtcgcggcagatgtaccaggagccggacttcttcgccatcaacatgagcgagctgcgcggcagcggctacctcaggttgttcctgtacacccaggtcggcgggtaccagccggtagaggaggacggctacctcaatccagagcctgtgctgttggacccgcccccgcacacgctctactacggcgcgccgccggtcaccaacgtgcctgattcgaccgggctggaaaatgattccgacccggaccaggggagcgaggaaccgcaaggcttgcggggcctgttcaggaggaagaagcgctgatgagcgacacgaattcccgctgggggcagctgacctacgcgtccttcggccgcgcggtgggcgacgggtggggcttcggccccagccgcgacgtccacgacagcgatgtcgagttcgtgcgccacttcgtgcgcgggtcgctaaggcccgtgcacgaggtcagcgatttcctcacctccgaggaagtggaccagttgccgatccgtttcgagtacatcccgtggggcgggcgcggcctgttcatgaacacccgcccggccggcaaggactcctccgggcggaagggcaacacgttcactcacatctacatcgaccacggcgcgcggtacgagaatccgcagcttgcgtacccgatccaggcgtaccgatcgccggatttccggatgccgtttttgtctaagcgcgttgacgcggtcgagctttcggacaacgctgacggaccggatcccggaccgcacttcgacgtcgacctgtcgtgggagatcgtgcgctcgatgtttatgggcatcgaccgcacgacggtcgtctaccgcatcctggacgagttggaggaagcccgccgcctgccggtgctgttggtgaacaactcgatggacgcgcagacctggatcacggtcgtcagctcccttttgtcgcagtgggaggcgcggaacctgttccgcttctccacgtacgagcgcgcggctgatatcgacgcgcagaagtaccgcaaccacgccggcagcacgctggtggcagcgcccgtcgaggacgcagacgcgctggcgaaggtccccggcgtcagcgtgatcaacacgaaggaccctcacgaggggtacgtggggaggggtacgtgggcgtcggcaagcaagcatgccctcgagctgtaccccgaccacctggcgctgtccgcggcgctgaacgcggcacctgttaaccccgaaagagcgcggcttggcgacgccatgcggcagctgcacgacaccaaggagtgagaatggaacacctacaacaaggagctgaagcgttcatcgcgggtgacgacctcaccgctcagatcagcgtggaaatcaccccgcacgcggagttcgactacgagctcgccggtgcaagggagcacgtgaagcgcgccggcacggtctacgctcgcggctttgaacagccggctgagctgatcatccgcccacgctccaccgcgcagttcgccgccgacacgcaggcgcacgtggtcatcgagttccttccggagatcggcgccggcgagagcgttgagctgcagcgcttcaagatcgcgggattgtcagagtttaccccggcgacgctttcgcccgcagccggcggcgtgagcgtgaaagccggccaggtggagcagctcgccgacggccaaagccgcgtctacaccgagatcgtccgcgagatcaccccggaaactggcgacgacaccgcggcagccgccgcgagcgcgaatcagacgcgctcggtgctggtttacatcgaccagtcggcgtccatggcgcagccgagccgcggcgcccagatgcgggcggtggcgaagttcctctccgagttcttgagcaagctggagatcgagctgtccgtggctggcagctccgcggcctccgccccgcgccgcgtgcgcagctccgccgaggcgctcgacacgatgctcgagctcaccccgcgcgccgaggtggggtggccgaactcgctgaacgcggcgctgaagcgctacgaccgcgtcatcgtcgtatccgaggacctgccggcggaagcggccgacccgcgcgtcaccttgatcaccttcgacaacctccccgagcgcttcaacggcgtgcagttcggccccgtgatccagcaggctgtggaaagcgacgaccacgaccggttgaagcagctgtccacgttcctgcaggagcgcctgtacagctccgtccagaacggagcgcggtaaatgaacgtgctcaccacgcgctgcccgtactgcttcgggcacttggacgagaacttaaaccacatcggcgcccccggtgccggaccgcgctgcagccgcaccgattttccgctggggtggcagggcgcgggcgtgatcaccgtcgccatggcaggtgcgcgcgcctctggcaaaagcgtctacctcgcggtggtggttgagctgctcagccagttcactaccgaacagcacggtacgtggcggccggccacgaagaagacggagcagatctacgaggagcatttccactcgcggctgttcgaggaaggccgggcgctggaatccacccgccgcatcgacgacaacgccacctacacggacgagccgctgatcttcaccatgggccggccgatggttcaggggcagcgcagcccgcgcgagattttcatcgtcttccgcgacatcgcgggcgaggacctgcaggactacgacatctcgggagtgaaggaccagctgagcttcctcgccaacgccgacctcgtggtcttcctcttcgacccgcttgccgacgaggacatccgcctcgcccttgcgggcctgcccggcatgtcccagccggaggacggcacccgcaccgacccgtcgatggtgttgcgcaacgtgctggcgcttatcgacgccaaccgcaacccccaccacctgccccgcatcgcgctgaccatgtcgaagttcgacgtgctgcagcagctcgcggagacccaaggcgagccgcgccacatggacgtgatcatgcgcaaccgcggcgccgccttcaaccgcgagggctccggcgtggacagaccgtgggattgggccgacaacgagctgctgcaccaggaaatccgcagcgtgctggccaccctcgacgcccgcggactgttcaaccagctcgacagctggatcacgcacgataacccggagaactactaccgctgcttcgcggtttccgcgctcgggtcccagacccgcgacgacgctgtcgactcctccggcatcgccccgttccgctgcctcgaccccgtgcgttccgtacttgcccagtacggcatcggcgtggctccgcagcaggtttactagagaggttttccactatgacgtaccccaccaacacgatcaccgcacaggaactgcagcaggagaacgaggtctacggcgagaaagaccgccagaacaaggagcgccgcgccagcgcctggatgggtatcgtgtccgcgctcatcgccatcgcggcaatcgttgcgcttgcgatctacctctggcaggtcgtgccgaacgtcaccgacaccgcaggcgacgtccgcgacgcggccaacgaggtctcctcgcaggctagataacggtgccgataagctcggccagcccgggcagctgggtggcgaagtcgtcgccgcctccggggaagcggtcgatcttctccagctgcagatcggcaaccgccgccgcgtccgcttcgagcacgttcaccccggtgacgaacaccgagtgcttgtggtcggagcgcactaccatcgtgtacggcacgatgccctcatcgaggtggtagtagaacgtcaccacgtcgatgtcggggttgaactcggcggtgaccggcaccgggccggtggagaggtcgccttggccagcgcagttggaggcgagccggtctaggtcgctgcccaactcctcgcgcgcaatgccctggtccagcacgagcacgctgtagcgcggtgcgaaccagccctccgcggcgggggagacagctgcctcgggcgcgagggtgatggtcgcttcggcttgggcggtcgccgccgcgtcgttaagccggtaggggccctctgccgcgcaggggtgctcggtgatctcgcccggcaccggcagcaaccactcgacgccgtcgtccgcggtgcggaaccgcgaggacacttcgcccgtgctgccggctgcgagcaaatcggtgtcgtaggggcggatcatgccgttgaccagcggctcctcgcggccggttggggcggcccacgggttgccctcgccgctaccgggcagggcgtagacgagcgctgcggccgcgccgaccgccagcgcggactgcaccagcgtggaaaagaagctgctcattgtgggctaccccccgtttagtacttccgacaagctgaggttccgagatctcctgtatttcatctcggcgttgtgcgccagcgtcggccctgcgaaccagatcagcatgatgcctagcacgctgacgaagtaaccgtctgcgagcatggacgccgcgatcagcgtgagcaccacaaagctcatgaacccgccccagagactcttgcggacgtgagccgcgaaccagccgaacgcgaggcctgcgataagacctggaacaaggcgcccctccggcgcaatcgggatgggccagcgcggggccatgaactggtcgaggagaaccgccgggaccatggtcgcaagggccagaaggaacgagctggtcgttccccgggggaggatgccgagggggcgtttgaggttgtcgtcgaaaagcggcggcgcgggctgctcctgccttcgttgctgacgctcttgttcctcagcctgctggcgctcgagcgcagcgatcccggaggcgatctcgtccaactcagggtggtcgatgctggtggcggttgcgcgcttcagctccttcgacgccagcgccgcgtcttgctgcgccagcgcctgcctcgccgcggcgaccgccgcccgcacctcgttcttgcgcgtttccacctcggcgacgatgtcggtgcccacacccgatttcggcactttgccctgcgctttcagcgtgcccaccagcttggcggcttgcgtcaccctcttttggtccagcagggtttgcaccggtccgtacatggagtggtcgaactccgcggcgcgccgaccaacctcttccggatcctcccggcgcacagccttgggtttcggccgggaccgcggcttcggctctgccgcgggtttagccttgggcttcgcgcttgccgacgccgcgtccgacgccttcggcgcatccccggcaagctgcgcgatgtcggattccaccagcccgtacgtcttcaggcgggcctccacgtcctgccggaacgcgcggcggctgtgcacctcgtcccacagcgccaagtggaacgcgataaccgcgttgtgcagcgcgaggtcggaacccgcgtgggcgcgcagcttggccgcggccgttttctggcgctgggtgttcgggctgcgggtgaaccattcgatcgcggtatccagatcggcgcgcgtgacagtcctcttcgcgtctttgaagtacggcggggagatggtgtagctgctcttcggcgcgccggaggtgtagttctccgggtttagcgcctgcatgatgccgaacgggaacgcctgctcgatctcctgctgcagcgcggccggcagcggctgaatcgggcggatgcccttgccctgcagcttgtgcacgatctggctcatcgcctccggaggcagtccggcgctcgcgcgcatctggtccacctgctccgcggagacgtagttcgaacccggaagggaggcggccagcttgcccacgaaatcggtgatgcgctccgtggcaagccgctcctcctcgccgcgcacgcgcgcgaaaaattgcgggttgtccaggcgttgctccgggtttgccgcctctagccgagcgagcgcgtcgtacacaggcttcgcctccgcgcgcagggtgctcgacggcgacgtggccaacttgcccaagcgctcgatgaactccgcgtactgcgccttcagctcgtccgcgctgggatccgcgccgtcgagctgcagcatcagcgagggctccagcttggccgcgtcgcccgcatcctcaacctccgcccaccgcgaagcgtacggcgtctctttgaggtacttcttcagctcaacgtcgttgaacatcgttactcagaacgaaccatgccggagatcatgttcttgtactcgtccacgcgctcgtctgagagcgcggagatctgcgccgtgagctccacgcgctgaccggtcgtcggctcgctgccctcgagcgagacaatgccgtcgttgctgaccttcatgatcatgtacaccggcgaaccttgcggcaggttcggcaggttgttgagcatcgcgccgttctcaccggagatgcgcttgttcgcgttcatgtcgcgggcggggatttcgccggcctgctcgtaaatgtcgaagcggatgcgggtggtgttgtcgttggacgcgaagccctgcgcggttgcctcggccggcagcttcgcgccggcgttgaggatgtgcatgatgtagggctcctggcggtccggatcccagaactgcacgccgacggccttcggcaggacgttcgtgatctccatggtgcgcgacccgcccggggcggcaaccgtgatcatgctgccggaggtctcgctactgttcgggtcgacgttgatgtcgccacccgcggcgtccaccaaaccctgggcgtagatcgcggcgcccttggccaccgcgaggtcgaactcggtcggcgtgagctcccagccgaaggtgctctcgagcgcctcgctgatcatcggcatgcgcgaggagccgccgaccagcaggtagcggtcgatcttgagatccggcttttccttcttcgccgtctcgatggcgcgctcaaccacgcggatcgtctggtcgacgaggtgcttggttgcgacctcgaactcctcccgcgtgatctccacgttggccttcacgcggttttggtagttgcagaggattttcgcggacttgcgccgcgtcagggcgatcttcgcttgctcaacaccgctcttgaggttttgcacgaagtcgtcgtcgtaggtcgggtcctcgtccaagcccgtggtcatgccgaagttcatcacggcgaggttgaacagctcagtgtcccagtcggcgccgccgagcttgcggtcgccgtccacggccagcacgtcgatgcggtcctcgcgcatgtccatgatggtggtgtcgaaggtgccgccgcccaggtcgtaaaccaggatcgtctggttgctgccgtggcgcatgcccgaggacagcgccgcggcgaccggctcggtgatgatgtcgagcacgttcagcccggcgattttgcccgcctgcttcgtggcggcgcgcgcctcggtgccgaagtaggccggaacagtgatgactacgccgtcggcgtcttcgccggtgaagtcctctgcggcttcaacaaggtaggacaggatcagcgcggagacggactcaggggagtgggtcacgccgtggatcttcacgtcgtaggcgtcgcccatgtggcgcttgatcagctccacggtctcgtctgggcgaagctcgatctcgttcttcgcctcgcggccgacaacgaagctcgtggcgtcgtcgaacagcaccaccgacggggtggtctgctcaccctcgaaattctggatcacctgtggcgagcccagctcatcgatgtgcgcgatcgctgaataggtggtgccgaggtcgatgccgtaaaccttcacgtcgttatcttcctttttcctgtcgctgttgcttagaaactctaaccggcgttcggatcgtagcggtacacggagacctcagccggaaccgagggcttcaccgacgccgggtggccgtacccgcgggcaagcaccttgtgaatagtgtcgttttgcgactcgtcagcggtcttttccacggccaccgtcttgtgccgcttgcggtcgtacggtgtgccgggggctgcgtccacctcttcaaacccgagggcgatgagcgcctcctccagctgctgctcgaagtactcgtacaccgaacgcaattggcgctgcgcctcttcggcgttgagctggctgagatcctggctcaagccctcgtcggtgtctttgaccatcccgccgagaatcttcgcggctggggtgaggaacgtttgaatgatgtcgatgcgggcgtcctgcagcgcggctatcgcggtgtcgcgcgggtcatccgcttcaggggcttcgcttgccgacgccccctttatcccctccagcctccccaccacagtgtccccgagcttctgcatctcattgagcagggtgctggtgctcttgtgcacatcggagcgcagtctgccgacgttgtcgttgagttcgtccgcgatcacgttgagcgacacagaatcgggatccgccttctggttgtcgccggtgtgcactgcggggaactgctcaatcggcggttccgggcgcggcggctgcgggcggttgaagctttggtcgtcgaagcgcatttactggcccaccttctggttcatccaagcgttcttgcccacgaactggttgttcgcgtgcatccgcgcgatctgcacctggttcatcgcttcgaccacgttgccgttgccgtcgacgacgtaggcgccggtcgcgctctggcgccgcggggcgggggttgccggcacgatgcgctgctggcccacgtagtagcccgccacctgcgagccggcgccggcggctttgagctcggtgcgggttcgctccaccagcttgttgaaggcgtcggcgtgcttctgcagctcgcggtttttaaaaatcgtcttggacgcgaactgcgaggcgccgaccgcgacggcaccgaagaacccggaaccgaacagcgcgatgaccgccgggccaagcgtggccagccagccgacgcagccgtctgcgtcgatgtactcctcgatgaacacgccgatgacggacagcacaaagatggtggccaggcagctgaggaaggtgctcgaggaaaacgccgtgtccagcagcgcagcggggatgccgagagcgagcggggtgagccacgcgttggagaacttcggcggcaggaacccgagtgccttgtgcttgccctcgtcctggatgggctggaagtgggtgtccacgacctggtcaatgaaggccgggtcgtgctccatctcgttgacgtacacggccaagtcgccgactgttcgggaatcaacgcaatactctgcaatcgagtccagctcttggcgcgcggcgatcgggttgcgggcgcggatggcctggtccaacgacgcggtgtcgcgctcgagcttgcgggcttgcgactggatgctttcaatgatgtccgcgcccacggaggaacgcgccctctcgcccgactccagcagctggtcgagttcgtacttcgcctgggcgaggcggccctcgccggccgcgcgctccaggctgccgaacgtctggcggtcgatctgctgcgcgcgctccgcggagatttccgggtctacgtgctccgccgcaagacggctcgagccgccttgcgacgccaccagctggcgcacctcgtcctcgtcgacgcccatggaagccagccgctgcgcaccctcgtcgatggagttgcgcacgtcgcgggccttgcggaacgcctgcaggtagaaagacgagaaccagtccctcagctcttcggttcccagccgggaaacgaagtctttttctttgctgaactgggggctggtggtgaagtagttgaccgcggcgtcgcgcacctgagcaccgggttcgccttccgcgccctcgaccgttgcatccacgatcgagatggttgcttccgggttgtcgcggaagacttcggggtagagcgcctgcgcgatgcctttcgggaacagcttctcgatctcgttgaaagtcttctccggaacgtcggcgacgacccggatgccgcggctgccgaggagctgcgtgaccagttgggccgcgaaatccggcaggccgcggtacttcatcgagttgttgagcgagaactcgtcgagaacggggaagccgtccaggcgctccgcccagtagtcggcctcttcagtcgcggcctcggacaccgaatcgaaccaggcgttcttggcaaagcggatgaagtccgggttgtccagcgtccactccgggttcgtctgctcgagcgcggtgagggcggctgcgacggtctcggcagcggagcgccgcgggcccatgccctcggcgagcttgcgcagctcgtcgcggacccgcttgccggttgtgcggatcgtcgcgtcgtcgtcggagtcgtcgacctgggctaggttggtcagctccaccttcggcagagcggttgccaccgcggattcggcgccggcagcgcttgcgccctccgccgcggccttgatctcgctccaggccgccgcgtccatcgtgcccaggtacctgttcagggcagttttgtcgaacttgtccgccccctgagccgccggctcagactgcagggaagatccggtgagatccgattccgccatggcgcgattctccaatcggtgtacaggcacaaaacacaagcagtataaacatcacacacttaactcacagggcgaaggttcgctctggacataaaaacggcgcctgcgggaaccgcaggcgccgtggatgtagcgagtgttacttcgcaaactcttcgacgagagccttgttgaaggccggcaggtcgtccggagtgcgcgaggagataaagccggagtcgaccacaacttcctcgtcgacccagttagcgccggcgttgaccaggtcggtcttcacgttcaccacggaggtgagcttgacgtccttaatcaggtcggcttcggtgaggatccagccgccgtggcagatcacgccgatcggcttgccggcctccttgaagcccttcaccaacgcaacagcgtcggagtcggtgcggatggtgtcggcgttgacggtgccgcccgggaggataagcgcgtcgtaatcggcgacgttggcatcagccgtggtgccgtcgacggcaaccttggtgcccttcttgccctcgatctcgccgctctcggtggagagaacatgggtggtagcgccggcggcctcgacggcctccttcggggaagtcagctcggagtcctcgaaaccgtcggtagcgatgattgcaatcttcttgttgttcaaatcagccatggctcacaccgtacggaaaagttgccgcgggcgtcgtcacacctggtcttcgtccagcttgttctggcgttccttgtcgctggcggtcgctttgtccgggtcgacggcgcgtgcgcggccgggaacttcgtggtcgtaggttttgttcggcgcgtcgtcgttaagcggcacccgcgtggagcccaacccctgcttgaccggagcacccgtggcgaccttctcccgcttggccatgcgcgccatgtgcttgcgcacagcgaggaacgcctccttggagtcgagcgcctggctttgctgggtggcgatttggatgtcgtcggcggtaatttgtccggcgcgcagcgagaccatctcggcccagtagcggaaccacacggcaagcacagccgcgaccgggactgcgaggaaggcgccgacgatgccgaagagggtgccgccgattgcgaccgcgagcagcacgatggctgcgtggaggcccatcgcgcgcgactgcaagatcggctgcagcacgttgccctcgatctgctggacagcgatgatgaggatcagcacgaagatagcgttccagaaaccgttggacacgagcgcgatgatcacggctagggcgccggcggtgaacgcaccgatgatcgggatgaagccggcgaagaaggtgatcacggcgagcaccggccacagcggcacgccgaggaagatgaggcccaagccgatgaagacggcgtcgaccatagacacgattgcctgcgtgcggatgaagccggagagcgtgttccaggagcgcatgagcacctcggtgaggtgccagcccgcacgcgcgccggtgtacttgcgcagccacggcaggaagcggtcgccgtctttcaggaagaagaaggacaggatcagggtgagcaccagggtggtgccgatggaggcgatcgcgccgataccggtgaacacgccggaggcgatgttggatgcttggcccttggcaaaggattcgatctgctggagaccctgctggatgcggtccgggtcaatcagctgcgggtcgaggcgctcgtccacccagtccaggatctgttggataccggtctgcgcctgttcgtagagctggccgccctgcgtgcgcacggtcggcgccatggcggagaagatgccgatgatcgcgccgaagaatgcgaccagcaccaagatgactgcggccgcggagggcatgcccttgttgcgtagccagcgaaccggcggccacaaaacggtgcagaagatcaacgcgagcaggatcggcagcaggccgaaccagacgtagctgaggaggtagaagaggatgccggttgcgacgacaacgataatgaatcgaagtgcccacgcggcggcggtgcggccgtcggcggcgatgacgtcgccgcggtcaattggttcaccggacaactcctgagcggcgtcggccggggtgggcatcatttgaatgtcgtcgacagtggtgtcgagcgcgcccacgtagtccttatctttatcagtcacctgcaacattctgccagaaccatggcaaatcgcttatttagaaaaggttgagtgcatcgggaacaactttgagggcgccgcgttatagacattgagtgcatcaggctcaaggggtacagtggcccttgtgaagttgagtcgaagcacttcaacttactaacaaaatcgtttctaacaggaggaacatcactcatggcacgtgcagttggtatcgacctcggcaccacgaactccgtcgtctccgtcctcgagggcggagagccggtagttatcgctaacgcggaaggctcccgcaccaccccatccgtcgtcgcgtttgcgaagaacggcgaggtgctggtcggccagtccgcaaagaaccaggcggtgaccaacgttgaccgcacgatccgctccgtcaagcgccacatgggcgaggactggacgatcgacatcgacgacaagaagtacaccccgcaggaaatctccgcccgcaccctgatgaagctgaagcgcgacgcagaggcctacctgggtgaggatgtcaccgacgcggtgatcaccgtcccggcttacttcgaggacgcccagcgccaggccaccaaggaggccggccagatcgcaggcctgaacgtcctgcgcatcgtcaacgagccgaccgcggcggcactcgcttacggtctggagaaggctgattccgagcagaccatcttggtcttcgacctcggcggcggcaccttcgacgtgtccctgctcgagatcggcgacggtgttgtcgaggtgctcgcaaccgccggcgacaacgagctcggcggcgacgactgggaccagcgcgttgttgactggctggtggacaagttcaagtccgccaacggtgtcgacctgtccaaggacaagatggcgatgcagcgtctgcgcgaggctgcagagaaggcaaagatcgagctctcctctcagcagcaggcctccatcaacctgccgtacatcaccgttgactccgagaagaacccgctgttcttggacgagaccctgtcgcgcaccgagttccagaagatcacctcggacctgctggaccgcaccaaggcgccgttcaaccaggtgatcaaggacgctggcctgtcggtctccgacatcgaccacgtcgtgctcgtcggtggttcgacccgtatgccggccgtgactgacctggtcaaggacctcaccggcaaggagccgaacaagggtgtgaacccggacgaggtcgtggccctcggcgctgctctgcaggctggtgtgctgcgcggcgacgtcaaggacgtactgctgctcgacgtcaccccgctctccctcggcatcgagaccaagggtggcgtgatgaccaagctgatcgagcgcaacaccaccatcccgacgaagcgttccgagaccttcaccacggctgaggacaaccagccgtccgtgcagatccaggtcttccagggcgagcgcgagatggcgtccgccaacaagctgctcggctctttcgaactggcaggtatcgccccggcaccgcgtggcgttccgcagatcgaggtcaccttcgatatcgacgccaacggcatcgtgagcgtctctgctaaggacaaggccaccggcaaggagaacacgatcaagatccaggacggctccggcctctcccaggacgagatcgaccgcatgatcaaggatgcggagacccacgctgacgaggaccgcaagcgccgcgaggagcaggagacccgcaacaacgcggagaccgctgcgtaccagacccgcaagttcatggacgagaacaccgacaagctgccggaggacatccgcacccgcgtggctgaggcggccgatgccgtggacgaggcgcttaagggcgacgacctcgaggccatcaagtccgcagtggagaagctgaacaccgagtcccaggaactgggcaaggccctctacgaggctgaggcgaacgcaggtgcaaccgccggcggcgcagcagacgctccgttcgacgacaacgtggtcgacgctgaggttgtcgaggacgacgacgcatccgacgcaccgtccgctgagccgaacaccgacgagaacaagtaaaacgcgtaggagacgatcatgactgacccgaacgtgaacccccagatgcccgacaacccgggcgcgccggagaacaccgacgagcagtatgtctcgccggaccaggcagagcagcttgccgacgaggcggccgattccgaagccttcgagcagatgactgacctcgaggctgagggcgaggaccccctcactcaggtctcggacgcggaactcgccgacgcggtcgaggttgaaccaacggatgtcgacggcgacggcgcggtgagcgaaatcgaggtgcagctcgccgaacgcaccgagtcactgcagcgcgtgagcgcggagtacgccaactaccgccggcgcaccgagcgcgagcgctctcagctggtggaccagaccaaggcgaagttcgcttcccagctgctgcctatcctggacgacttggatttggctgagcagcacggcgacttggccgagggcccgcttaaggcgctcgccgacaagctgcgcaccaccttggaaggccagaagctcgtcgcgttcggcgcgccgggcgaggcctttgacccggagattcacgaggcggtgcaggatctttccgagggtgacgagaaggtcatcggaaccgtcctgcgcaagggctacaagctcggcgaccaactggttcgcaacgcgatggtgatcattgcggacgagcagagctaggcgttaggcgctagctatctagcggcctaaagccgaggacaaccagccgggtgcgagcggcatgcaacgcttgccccggctttttccctagaaacgttatttcgagacagaggttcaagtgagaaaggaggagcgtacatggcaatgcagcaagaatgggcaaataaggactactacggcgatttgggcgtgagctcgcaagcgtcggcggcggacatcaagaaggcgtaccgcaagctggcccgcgagaaccacccggactccaaccccggcaacaaggaagccgaggagaagttcaagcgcgtcgcggaggcgtacgacgtcgtcggcgacgaagagaagcgcaaggaatacgaccagttcaaatccatgatcggctccggcggcttcggagggttcggcggccgcttcggagggggaggaggctccgggtttccgggcgggtttcgcacgacgcagacaacgtccgacttcgacttcgacgacctcggagacatcttcggaggtgctggtggacaagctggagacggcggccttggtgatatcctcggtggcttctttaaccgcggcggcggtgctggcaggaacgctcggccgtcgcggggggcggacgtcgaaaccgaaataaccatcgacttccgcgaggccgccaagggcaccaccttcccagtggaactcaccggcgaagccccgtgcaccacgtgccacggctccggttccaagtcgggcaagacgcacacctgcgcgatgtgttccggcaccggctacatccgggagaactccggcgcgttcggcatggcgcgcccgtgcacgaactgcggcggcaccggtgaagtgatcgaagacccgtgctccacctgcggcggcaccggcacggtgcgccgcacccgctcgattaccgtccggatcccggccggtgttgaggacgggcagaaggtgcgcctcgccggccaaggcgaagcgggtccgaatggcaccccgtccggcgacctcttcgtcaccgtccgcgtgcgcgaggacaaggtgttcacccgctccggcaacgacctcgagctgaccgtgccggtctccttcggtgagctggcgctcggcggcaccgtgaccgtgccgacgctggacaagccggtccgggtgaagatcccggctggcacgcctaacggccgcaccctgcgcgtgaagggccgcggtgtggaggcgaaatccggcgccggcgacctgctggtcaccgttgaggttgccgtaccgaagaacctagacgccggcgccaccagcgcgttgcgcgcctatgcccaggcagaaaaggactccggtttcgacccgcgcgccgggtgggccggggccaactaaaggaggtggtggacaatgtctgactcgagaaacgatcacgagcagtactacgtcatctccgtggctgccgagctcaccggcatgcacgcgcagaccctgcgcacctacgaccggttgggtctcgttacgccgatgcgcacctccggcggcggccgccgctactcctcgcgcgacatcgcgctgctgaggcgcgtgcagcagctctcccaggaggagggtgtgaacctcgccggtatcaaggcgatcatcgagctcaccgagcaggtcgaaggcctgcaggccgagctcgacgccgagcgcgaagctgccgcggagctgcgccagcgcttgcagtccggttcgcgccgcggcggggagttggtccacgtgcctcgctcgaccgcggtggtcacgtgggagccattcgcttccaggcgcgcgcgccggcgcgagcaggcgtaggcgtctaaccggtagcgaacgagaaaaccccatcgccggccgctggaaacagcggaggtgacggggtttcgttgtgcctcaggcgcttgagcgccggagtgcgggtccgactagcggcgggtcgtgagcacctgcttctcgtcgcggttgagcacggagcgtgcaccagcagcgccggccagggaggagatcacggcgccgaggatcaggccgccgaaggtccaccaggtgccctcagcagcgtcgtcggagtactcgttgtaggcgtcgcgggccttgttggcagcgtcgttcgctgcatcgcgagcttggtcagcggcgttgtcaacgtcctcctggctgatgttgtcgcgagcggagtcggtagcgtcctcagcgtcctggcgggtcacggtcgcggcgttgccagtggtctcagcgatggtgccggtgacgttgccaagcacggagcccaggccgccgacgatggaggagccgagccagccggccaggatcagggatgccaagagggaggtcgcccaggtggcgaagccgtggaacatgccagcgcggacgccgagagcaccggcgacgtagccggctgcggcgaaggcgacgatcagggagatcagggcaaagatgccggttgcggcaccggtggagccctgtaggcccatcgctgcggcgccgacgccgagcaggatcatgatgcccaggaaggtcacgacgccggcaaagatggcgccccaggacacgttgccgttggacacctcggtggagtcggtgccgatccaggcttcttggccgatgtgctgatcggcgtcggccacggtttcggagcgcacagcggtgctggcggaggccggcgcggtgcgggtggtcttctcaacgcgcttcgttcggcgcgggttctgcggggtagtcataacaggtaaaacctttcttatgaatcaatgacaacgaagcctacggtacagaacagagatgagcatttgggtcacgtagtgataacggttggtcaacgaaaaggggccgtcgttaagcaattgcttatcgacggccccttgaaaaccccaactacccgaattcgatggctgcagcgccaccgatgtggcgcatgttggacttagccaggttaaacagtcggccgacgccgccctcgaggaaggcggtgcgggcaccggacttggcgaagcccttcatcatgtcccaggtgatccccggcggaagcgagagcgcctcggggtcggtgacaatgtcgacgagcaccgggccgtcgtaggcgagggcctccttcagcaccggctttaggtcgtccggatcctcgatgcggtaggactggatgcccacgcccttggcaatctcggcgtagttcgcctcctcgtggtcagtgccgaagtacggcatgccggccaccatcatctccagcttgaccatgccgagcgaagagttgttaaagcagatgaccttcaccggcagctggtgcagcttgatggtgagcagctcgcccatcagcatgcccaagccgccgtcgccggaccaggagatgacctggcggtccgggaacgcggcctgcacgccgatcgccatcggcagcgcgttggccatcgtgccgtggaggaaggacgcggcctcgtcacgcttgccgttcggggtgaggtagcgggacgaccacacgttgcacatgccggtgtcgacagtgaagtaggcgtcctcatcagccagctcgtccagcacggacgcggcgagctcggggtggatcggcttcttcgattcaaaggccttggtggtgtagtggttgatcacgtgctcgagcagctcgtagtggcgcttgagcatcttgtccaagaacttgcggctcttcttctcctcaatgtggggaaggatgttctcgatgacgctcttcacgtcgccaaccaccgggtagtccacggtggtgcggcggccgatgtgggtgccgtcgatgtcgatctgggccacgttctcgtccggcagccagtcggtgtaggggaagtcggtgccgaccataatgaacaggtcgcactcctccatcgcgtcaacgcaggcgccgtagccgagcaggccggacatgccgacgtcgtacgggttgtcgtactcgaagtacatcttgccgcggaaggagtgaccgatcggagccttgaccttctcggcgagtgcgaagacctcgtcgcgcgcgtccttcgcaccgtagccggcgaagatggcgaccttttccgccttgttgatcgcctcgaccaggcgggctgcctcgtgcgggtccgggtaaacgcgcttgtccttgccggtggcgtagacgccgtcggcggtgtgcgggccgtctgccacgtcggcggcgaagacatcgccgggcacgaccatcacggacacgccgttgccggcgagcgtgttctgcagggcgttgtgcaaaacgcgcatgccctggtcagcctcgtggaccacctcgcagtaggaggagcactcctggaagagcagctccgggtgggtctcctggaagaaggaggagccgatctcaatcgtcgggatgtgggacgcgatggcgagcaccttcgcgccgttgcggtgggactcgaacagaccctgcacgaagtgggtgttacccgggccgcaggatgcgccgcacaccgcgagctcgtcggcggccagcgagtcagcgcccgccgcgaacgccgcggcttcctcgttgcggacgtggacccactcgatgtccgactggcggaccgcgtccgacagcgggttcaacgagtcgccgaccagaccgtaaatgcgcttgacgcctagatcttctaggcgccgaactacctgttctgcgaagtttgccatggtgctcgaagctccttaaatgaggtttacctaaatcttcaggtttgcaacagccgatggtaacgaattctgcgcagccgggtcaggcgggcaggtcagagcgttcagcagcacggggcttgcgaagtactcggtgtgcgtgccctcgacgccgtcaataatgatcgcgccgtagcccgggtcgctcggtgagtgcatgccgtgcaggcttgcatcgtcgttgcgcagggttttgatgatgtcgcgcgaagcgtcgacggcatacactcgcggggccgcgcccgggcgtcccgtcagctggaggtcgtcgaccgagttgccgtccacgccggggctgccgagcagccacaaatcgtccgccacgagaccgtgctcgtaggcggcgcggcttgcaaccaccgtgccgtacgagtgggagaccaccgacttttcagcgtgggggaaccgctcgtccagcgcaagttggaacatggcgaggtggccagcgccctccgaggcagcgcggccggagaaccctttggccactgtcggcggcggcgcgtagccctgccacaccaccacagccgcgccggtgtagtccgctatgaacttcgcgcgctctatctcccgcggcagggcgtccggtttgccggttgtcacgccgttgaccaaggtgatgatgcggtcggggtccacgctgtcgccgaccatgacggtggtggagccggggcccgcctccagcacggttccacctgcctgggcaatcgcgcttgccgacgccgccggcaacgtccccacatacctggcatgcagcgcctcgagatcctcttccgggtgcgccacaagccggtcgaccgggtcgtcgccgccggcgccgagttggtccgcgattagcatgtccagctgcttggacatcaggttcagccggatgatcaacgcgcggtgggaggcgtcagcggccatcaaggcggcgcgccgggcaacctcatcgagcagttgctgctggccggcggcgaactcgagcaggtcagccgcttggcgcgcccgggcagcggcgcgggcgaagtcttcggcttgggcctcgaggcgcgcgtaggcagcgcccgctgcggagccagcgaagccggtggccttaagcgcggcagccgcggcccgggcagcgctggcgtgggcgtctgcggcaagtgccgccatccgccaggacgcggccgcggcgcgcagctcgtgggggtaaaggctcgggtggtagatcacggcgttcgtcccttggtcagggcgcggtcgagcgtgcgggctaacgcgtcgtcgatgcgctcgacgcgggtggcgaaggccgcgactgattctaggtgggcggtgagggaggtgaggtgggcgtcgataagcagctgctccttggtgaagcggcgggcatgcgccgcggcggtgcgggaggggcttaacgttgccgcaggtagcggggtgtgctgggggatgaggcgccgggcggttggcgcggtgtgggtggtgagcgtgaggtccatggccggagttaaccaaggtgggcgaattcgatcaaccaagcggctgcgaacctgtggataacgtttttaggatggccggtatgagactcgccttattgcaaacggtgaccggcaaggacaaggccgacaacatcgcgctcgtcagcgggttggtgcgcgacgcagctgcacagggggccacgctgatcgtgctgccggaggctaccagccaggcctttgagcagggccgattagacacccaagctgaggagctggacggggaattctccatcgcgatgcgcaagctcgcggacgagctgggggtcacagttgtggcgggaatgtttcggccgggcgataccaataagctggggaagaaagaactcaaccgcgtgcgcaacactgcgctgatcaccggtgggggcacgcacaccggttacgacaagatccacacctacgacgcgttcgactaccgcgagtccgacaccgtcatgccgggcgaggagctggtcacgttcgtacacgaggcgggcggggagagcgccgtggttggcgttgcggtctgtttcgacatccgcttccccgagcagttcaaggagctcgcccgccgcggcgcgcagatcgttgtggtgcccacgagctgggcggacggcgagggaaagctggatcagtggcgcacgttgaccgccgcgcgcgccctagatgcgggcgttttcatcgcggcggcgggccaagcgcgccccaactggaaaacggaggcgggtgaagaatccggccccaccggcatcggccactcgtgcgtggtcgacccgcagggagcgcgcatcgccgaagcgggttacgcgccggagcttgtgcttgtcgacgtcgacctcaacgccgtcaccgccacccgcaaagccctgccgctcatcgcgatcaccgattcgacggcgatgcgttaacttccaggacctccagccagtcgtttacccgcgccagcgcctggaacaccggcagttcgtagcgctcggcgtccgtgtcgccgaggtagcgcagcgtcacgcgggggcgctcgggttgctccagcagggcgaaaacgaccgccttcgcggcggcgacgctggtgccctcggcggtgagctcaagtgcgtcccggtcgagcggggcgggttcgccgcggggcgcaccgatgaccagcagcgcgccgggcgcgatcgccggcacctcttctgcgcggacgtggaactccacttggccgtgcgcgttcgccggtaccgcggagacccactcgtgccacaccccggggtgctccgccagcatgaccgtgagccgctggcccggcgcgaaagcgatctcggtgccgcactcggcgcggatgatcgagatgtcgctttcgggcaggctcaccctgcgcacgtcgttgacctgcaccacgtaggcggcggggatgccggcggcatccgcctcctcgctcacggcgcgcatgtgcgcggcggcttggataagtgccgcggcgtcctcctcgcccagctccgcgacctccgcgagcatccccgccacggcttcgtactcgccgagcgggaagccgaggcggcgcaggtccagtgcccaggcggtgagtttcggctcggcgtcctcttgcggctgggtgagcgcgaattccgccatgtcgaggatgacttgcggcatctggtccgcgcccggcggcagcagcgtcgcgccctgcgggtaccggcgcatgaacgcctggtggagtgcagcgcggaggcgtcctgcgtcggcgaacggggagtcggtcatgcatccacttttacccgcccggcggcaaacacccgccgttggcagtcaattcacagggttgagcggaacatactcaagcgtccgggcgttacaccgtgtgcgaaagaaaaataaccagtgaaggagtcgcacacatgggttcgtttaatcccacgaccaaaacgcaggaggccctgcagcaagcgctgcagaaagcgtccgccgcaggtaacccggacattcgcccggcgcacctgctggaggcaattcttactcaagacgagggcatcgccgctcccgtgctgaaagcgacgggggttgatccggagacggtggcccgggaggcgcaggcggtcgttgatacgtaccccaaggctgaaggcgcggacatgtccaagccgaacttcaaccgcaacgccttgaacgcgattaacgccgcgcaggagctggcgggcgagctcggcgacgagtttgtctccaccgaggtgctgctcgccgcgattgcgaagggcgacgacgaggcagcggagcttttgaagaagcgcggcgcgacctacgacgtgctcaagggcgcgttcccgtccgtgcgcgggcacaagaaggtcacctcggagaacccggagcagcagttccaggcactggagaagtactcgaccgacctcaccgcgcgtgcgcgcgagggaaagatcgacccggtgatcgggcgcgacaccgagatccgcagggtggtgcaggtgctcagccgccgcaccaagaacaacccggtgctcatcggtgagccgggcgtgggcaagaccgcggtggtcgagggcctggcgcggcgcattgtcgccggcgacgtgccggagagcctgaagggcaagacgctgatctcgctcgacttgggctcgatggttgccggcgcgaagtaccgcggcgagttcgaagagcgcttgaaggccgtgctggatgagatcaaggcctccgagggcgagatcatcactttcatcgatgagctgcacaccatcgtcggcgcgggtgctaccggcgagggcgcgatggatgcgggcaacatgatcaagccgatgctggcccgcggcgagctgcgcctggtcggcgcgacgacgctggacgagtaccgccagtacatcgagaaggacgccgcgctggagcgccgcttccagcaggtctacgtgggcgagccgagcgtggaggacacgatcggcatcctgcgcggcctgaaggagcgctacgaggtgcaccatggcgtgcgcatccaggattccgccctggtggccgccgccgagctgtcgaaccgctacatcaccaaccgcttcctgccggacaaggccatcgatcttgttgacgaggcgggctcgcgcctgcgcatggagattgactcctcgccgcaggagatcgaccagctcgagcgcgtcgtgcgccgcctggagatcgaggagatcgcgctgacgaaggagtccgaccaggcctcccaggagcgcctgacagcgctgcgccaggagctggcagaccagcgcgagaagctcggcgagatgaaggcccgctgggagaacgagaagggcgaggtgaacaaggtccagtccgcgaaggaggagctcgagcgcctgcgcaacgagtctgagattgcggagcgcgagggcgactacgccaaggtttccgagctgcgctacggtcgcatcccggagctcgaggccgaggttgcgcagatcgaatcccaggccagcaccaagacgatgctggtggaagaggtcaccccggacgtgatcgcggaggtcgtgtcgtcctggaccggcatccccgccggcaagatgatgcaaggcgagaccgagaagctgctgaacatggagtcggtgctggcaggccgtgtggtcggccagaacgaggctgtggtcgcggtctccgacgcggtgcgccgctcgcgcgcaggcgttgcggacccgaaccgcccgatcggctcgttcctcttcctcggccccaccggcgtgggcaagaccgagctggcgaaggcgctcagcgagttcctcttcgacgatgagtcggcgatgatccgcatcgacatgagcgagtacggcgagaagcactccgtcgcccgcctggtcggcgcccctccgggatacgtcggttacgacgccggcggtcagctcacggaggcagtgcgtcgccgcccgtacagcttggtgcttttcgacgaggtggagaaagcccaccccgacgtcttcgacgtcctgctccaggtcctcgacgagggcagactcacagacggtcagggccgcacggtggacttccgcaacacggtggtgatcctcacctccaacttgggcgcgggcggtaaccgcgagcagatcatggaggcggtcaagcaccacttcaagccggagttcatcaaccgcctcgacgacgttgtggtcttcgacccgctgaccagcgagcagctggtgggcatcgtcgacatccagctcgcttcgctggcgcagcggcttgcctctaggcggctgacgctcgatgtctcggacgccgcgaagagctggctcgccgagcggggctacgacccggcctacggcgcgcgcccgctgcgccgcctgatccagcaggcgatcggtgaccagctggccaagaagctgctggccggtgagatccgcgacggcgacccggtccacgtggatgtagctgagggcggcgagcgcctggagatcaccaagcgctagttggcggttgctcggcggggtagactgccccgcatgcagctgaccacgacgatcacgacccgcgtcgccacccccggcgtggagaacgagcacttgagcgcccaccagctcagcggcaaccatttcgtggtggccagcgttccgttcgtggacacctcactcgcactcggcgatatcgtcgagtgcgtgctcgttggcggccggtttcatgtggaccgcgtggtggtgcgcggcggcgcgtccacaatccggatcctgcccgagaccgagcacccgcaccagatcgccgagaccctgctcgccttcggctgccgcgtcgagctcggcccgggcgggatgctcgcggccagcatcggtgccgactgcccgcgcgagggcatcctggagtggctcgacgggctagaatccgaaggcgcgatccagcaagcgccgggctacatggcctaataggattggtgcccatgagcgtctttgtctccgcggaagaactgaacgcgcgcatcgaaaccggccagcgacagaccatcctcgcctccctgtgggagggcaaagagaaccgggcgtggtcgaagttccagtctgagcacatccccacggcgctgttttgtgaccccgcctcccagctcaccggcatgcctagccgccagcaagggcgcaaccctgtccccagcctcgaggtggtcacccgcgccgcgaaaacctgggggatcgcggccgaccgcccgacttacatctacgacacaggcaacgggctattcgctgcccgagcctggtgggtgctgcgctgggcgggtatcgaagacgtccacatcctcgacggcggcttcgccgagtgggacaagctggggcttcccaccgtcgcaggcccaggccaggtggtcgtgccccgcccggtggacacctccgagggcaacatgcccacagtcgcgatggaggaggtcagggggacgaaagcactgcttatcgacacccgctctaaacgccgatacgacggccgccgggagatcctcgaccttcgcgccgggcacattcctggcgcggtgaacttgccggtatccgacctgtttacggaggacgacaaggtgaaaaccgacggagagatccgcgaccgcttcgccgaggtcggcatcacccacaacaccgcaccggaagacgtgatcacctactccggctccggcaaccactctgcgctcttgctcgccgccatggagcacgccggcctgccggtggtgacgcactacgtgggcgggtggtcgcagtggtcggcaaacaacgacaacccggttgcgacgaacgtctagggcaaaaacatatggctgcagtgctgttcatcctcgcgttcgcgtgcctcgcggcggggctgtggttgtggttcggcggtactcccgccgcgccgacggccgagccaaagccggctaagcctgccaaacccgccggcaaaaagacgcgccgcgcctgggccgaggccaacggctttgcttacgccaagaccgacgacacgctcaccggcgagtggcgccgcggggccgcggcctcgggggctgcggcgaccaacgtcgccaccggcgcgacgtacgggcgcaccacgatcgtcgccgacctcggcggggtgaccgttatggcgatgaacaccggcgagacgagcgacgtggttgtggacatgcgccgcggtgaggccgctgccggcggggacgacttggtcagggtcgccgacgtcgcggacttcactgtgtacggcaaccaccacggcccggtgcagcggtttattgacgtccgcgtgaccaccgcgctcgagaacttccccgcatccgtgacctccgtgtggtgcgagggcgactgggtgctcgcggagttcgccgccgcgccgagcgccgaggacaccgacgctgcgatcgcgccgctggggctgatcgctgacgcggcgaggacgttgcctccttcggaggtgagggtgttgggggttgaggggggcgtcgataagcaaccaatgcttcgacctcccacccagctgccgacgcgaaccaccggtaccgcgcgggggactgcggagctgaaggtggttggggcggacgacgtggacccgatcgcggagggcgcgccggcgaccgagggcaacgacctcacgcgtgcgcggcgcgcgaacaagccgccgtcaattttttaaaggagatggatatggacaagaagcaacgactcgctgagctggtcaaagagctggccgtggtgcacggcaaggtgacgctgagctccgggcgcgaggccgattactacgttgacctgcgccgcgcgacgctgcaccacgaggcaagcccgctgatcggtgaactcctgcgcgaactgacccaagacctcgagttcgacgccgtcggcgggctgaccctcggcgccgacccagtcgcgaccgccgtgatgcacgcggccggtcgcccgatcgacgcgtttgtggtgcgcaaagaggcgaagaagcacggcatgcagcgccgtatcgaaggtccgagcatcgccggcaagcgcgtgctggtagtggaggacacaaccacgaccggcaactcgccgctcaccgccgtggaggcgtgccgcgccgagggtgctgaggttgtcgcggtggccacggtggtggacagggcgacgggggcggagcaggtgcttgccgacgccggcctggactaccgctacctcctcggcctggacgaccttggccttgcctgacgctgattcgggcgctgagcgcggcccgaccgagtggttccccgcccgaaacggcgtgggcccgtgggaagggccgctgcctgacgacccccgctacgaccccgacctgctcgccgagggtgatacccgcaacgtcgtcgacgcgtaccgctactggtccctcgacgcgatcgtggcggagctggatgcgaagcgccacgacttccacgtcgcgatcgagaacttcgaaaacgacatgaacatcggcaccgtggtgcgaaccgcgaacgcgtttctggcgcgcgaggtgcacatcgtcgggcgcaagcggtggaaccgtcgcggcgccatggtcacagaccgctaccagcacatccgccaccacgagacggttgcggatctgatgcgctgggccgccgcggaggacttggtggtcgtcgcgatcgacaacacgcccggcagcgtgccgttggagacggccgaactgccgcgacgctgcgtgctgctgtttggccaggaaggcccgggggtgagcgaggaggcgcaatccgcggcggtgatgacgtgctcgatcgcgcagttcgggtcgacgcgctccatcaacgcgggcgtggccgcgggtattgcgatgcacgcgtgggtgcgccagcacgccgacttgtcccaggcgtggtaacgaaacgctaacgcttcgcaccgcagcggagatagagttggcgagaacgttcgttatgaggagttgacccgtgcccgaaacttggtcgcaccgcgctgacttggcggccgccgctattgaggagcgccacgcggcgcggttgtggggtatcccgaaaacaaacttggcgctggcggcgtggccgccgtcgtcgaaagacaagctgtttatccactggcatttctggtggcaggcgcagtacctggactgccaggtggatgcggcgcttcggcggccgtcgaaaacaaggcgccgccagctttcggacaccattcggggcatccagcgccgcacccgcggcaagatgacagacatcgcccacaacgacgacaaggcgtggatggcgctcgcgtggaaccgcgcgactgggcttgaggggatcaagcgcacgcgcgccctcgacgcgctggagttcgacctgctcgcggccatcgacccgatcaccggcgtactgccgctgaaaagcggcgagacgtattacaacatcgcgtccaacgcgccggcggcgatcgtgttcgcgcgcacgggccgcctagacaaggcgcgccaggtcacagactggatcttcgacaacttggtgtccgagagcgggctgcttgtcgacggcatccgcatgcgcatgcacggccccgatcgggtggagaagatctacacctacaaccagggcaccgtgctcggcgcgtcgttggagatcgcgctcgcgctgcgcgcggacgtggggctcaaagacgacgagccgatcgactccttcgagttctccgagcgcgctgacgcgtcggtgttctacatcacccacatccgcgcgattgtgcaggccatcgcgctccacatggccacgccgcagggcgtgatcgtaagcccagagcacgaggcgggggagggcgacggcggcctgttcaagggcatcctcgcgcgctacctggccgaggtcgccgtgcgcctgccggaggattcccgggagaacatcgccacaaaaaaggtcgcagcacggctggtcatggcgtctgcggaatcgatgtggtcgcaccgtctcgaggtcgacggtctgccgattttcccggcggagtggacggaagatgcgaagttgccgcacaactacgggttggggccggcgtcgataagcgaagccgttgggcttctgcgcatcgacgagcgcgacctctcagtccagctgtccggctggttgttgctggaagctgcggctgcggtggcagcggcggcgggttaaaccgggcatactgggtgacgtaccacaatcgcgtttagaggttaggaagggtctacaccatgccaattgcaacccctgaggtgtacaaccagatgctcgacgccgccaagaagggcggctacgcctttccggcgatcaactgcacctcgtcggagacgatcaacgcggcgatcaagggcttcgccgaggcggagtccgacggcatcatccagttctccaccggcggcgccgagttcggttccggcctgggtgtgaagaacaaggttgccggcgcccgcgcgctcgctgcgttcgcgcacgaggtagctgcgcactacgacgtgaacatcgcgctgcacaccgaccactgccagaaggagctgctggacgactacgttcgcccgctgatcgccatctcgcaggagcgcgtcgaccgcggcgagctgccgctgttccagtcgcacatgtgggacggctccgcggtcccgatcgacgagaacctcgagatcgctcaggagctcttggctaaggcccacgccgcgaacatcattctcgaggtggagattggcgttgtcggcggcgaggaggacggcgttgaggcccgcgccggcgcgaacctctacaccaccgaggaggacttcgagaagacgatcgacgccttgggcaccggggagaacggccgctaccttctggccgcgaccttcggcaacgtccacggcgtgtacaagccgggcaacgtgaagctgcgccccgaggtcctcgacatgggccagaaggtggcggaagccaagctcggccgcgaggccggctccaacccgttcgacttcgtcttccacggcggctccggctccgagaaggagaagatcgaagagtccctgcgctacggcgtggtgaagatgaacgtggacaccgatacccagtacgcgttcacccgcccggtcgccgcccacatgttccagaactacgacggcgtgctgaagatcgacggcgaggtgggcaacaagaagacctacgacccgcgctcctacctgaagaaggcggagcagtccatgtccgagcgcgtcatcgaggcgtgccaggacctgcacagcgttggtacgtccgtggcaaagtagcgggcaaaagactaacgtttccaagcgtcggcgatccgatcctcgccggcgcttttcttatgcctaaatcacaaccccacagaaggatgagcacccgcgagcggctgcaggtgctcgaccagtcagtccaggcgcgtttacgtcgcatgcgcaaacgccttttgcctattctgcagaccggcattgccgccggcatcgcgtactggctctgtaaggacatcgtcgggcaccagcgcccgttcttcgccccaattgcaaccgtgctgatcatcggtgtctccaacggcgaccggctgaacaaggcggtggacatctcgctcggctgcgtgctcggcgtgctggtcggcgatttgctcttctaccggctgggggacggtggctggcaaatcgccgtcatcgtcgcgggctctctgctcattgcgtcgttcttctcgaagtcgcagctgttggtcaaccaggtcgcgatcggctccatccttatcgcgacgatcatgcctcccggcgccgaggtgaccggcatcgaccgaactatcgacgctgtggtcggctgcaccgtggctttgagcatcctcgcgctgatcccgcaggctcctatgtcgtctgcgcgggcagaaatctcccacgtgatggggctgatgagctcagtgcttgacgacgtcgcctcaggactcaaaaaccgcgatcccaagcacatcgacgaggcgttgaaccacatccgcggctcccagtcccgaatcgacgatatggctgcggccattcaatccggcgaagagtcgacgcgtatctcgccgtttctgtggagctcccgacgctacatccagtcgctcggccgcgttattccgccggtggacagcgccatccgcaacacccgcgtgcttgcccgccgtgcactcgtgatcagccaggacggcgaccaggtgtcgcccaaacaggtggagatcatcgacaccctggccaaggtctcccttgccatttcggagatttacgacgtcaactcccgccgcgcccaagctcaagtcgttcccgagctggtgaacgagctgcgcgccgtcgcgcaggagtccggacttgacgtggtggaggggacgccagaggatccggtgaaagagccggtgttatccgcctacgccatcctcgcacagacgcgttcgttgaccgtcgacctgctgatggtctgcggcatgtcgcgggaatctgcgctcgcggcgctggcgcctacgtctcgcaccccgaagttcaaacccgagcagttcaacctgtagcagttcaggctgtagctcccacggatttgagtagacaatcgagctgggtaaactccggcgatttcgccaccgatttcgctgggagctacagcccttttgatagaagcacgaaagagggccccagccgggtaacccggctagggcccttcgtgctttacagcttgctagccgtggctagcgggctgcttagcgaacgtcgccgtcgatgttgcggtcgcgctcgacgccgtcgacgacctcgccctcggtctcgaaacgctccttgcgaacctgctcggaaacggtctcggtgtcgcggacggtgtcggtctcgagggagaccttctcaaccggcacagactccttggacacgttcacctgctcctcgtggagggtgacggaagcctcagcctcgccgatgttgccgtcgtagttagcgcggtcagcgtcggtgatcggctcacgcacaacgcggacctcttcgcgctctaccggtacctcaacggtctcggtctcgttcacgacgtacttgcgcaggcgaacctggccggactcaacgcgctccttgttcacgttgaggtgctcctcggaacgaacgagctcgtcgttgttcacgtctgcaacgtcgcggcggtcagcgtcgacgaagtcggtgcgatcctcgcgaacctcaccagcagcgtagccagcgccagcggcagcgcctgcagccggagcggcagcagcgtcggtctcgtaggtggtgacatcctgggtctcggtcaggccgtagtggcggtagaacgcctcctggtcctcggtggtgaggtggccgttctcgtcgagctccggagcgtcctcgatgcgagccttcgggaacgcgaggtgcagctcgccgtcgcgcagggtgtggccgcgcagcggaacgatggactcgccgccaccgaaggagccgtggtgcacggaaacgaagtccggctggccggtggtgtcgttcacgtaaacgtccttaacctcgccgaccttgtcgccgtcaacgtcgaaagcggtagcgtttgcgagatcttcaatgcggttgtaatcagccatgattttctcctaaatcagtctgttggattggaaactccctaagcgggaacgagtcccaacgtagctacgttttgcaaatcgccgcggggccaatccgtacccggcttcgggaaccgaaattatgcggacgcgcgccgaaatttcaggtaagagatccgacacaatgccgtgagctgcagcgctggtgcgcggacaccgtgggaactgacaaaccggccgcgctcgacggtctcgaaacggttacgaaatgtcactccagtagcggaaaagaggcgttgtgatgtttatcacatgcatctaaattaggcgtttcgcaccgattggatgtcgcgcaagtggcggtaaaaggtggcgtgggtgagctggcggggtttggggtgggcgtcgataagcagcgaaatgccctctcctcctgtttgcaccgcgcggccggtgagcgccctggagccgtcggtgcggccgcggcgggtgaccagcggcgcgcacgcgatgccgggggcagacatggtgggcacgaggcgcgcgccgaaatggccgcggaagcgcgccgagcggccgccggtgcggaagacgagcgactgcgagtcgacgacaatctcgccgacgaactctttcgagccgtcgccgtgcgtaatcgaggcgctgccggcgaccacttcgccggcgtcggtgcgcacgcaggcggccggaaccaccggtgcctccaccgcgaaggccggatccgcgaccgctccccagcacactgcggcgggggaggaggggtcgatagggatgtaggccacctcggcccacaggtaatcggcgcgcatcatgcgggtgagcaccgcgccgagcgccgcgtcctccccgtgcacgatgacgcgcagccgctcgagcggttcctgcggcgcgaactgcgggtcgcccaaatgcgccacgttcggcgacgcttgtatctccgtgagcgacggtgttgggtcttcgggcaggcacttgctcgccgcggcgtctaagaagcgcaggtccttgcgcgacggaaccgcggggatatcaaaacgctgcgcgcccggaatcgggcccactgcctgcgcttgagcctgagccttggcaccgcacgcgcaatagataagttgcatatgaggcacgctacaatagctgcggttgctgacctatatataaggagcaaaacaatgtccgccattgtgatcgtgggcgcccagtggggcgacgaggggaaaggcaaagccaccgacatcctgggtgggcaggttgattatgtggtcaaacccaatggcggcaacaacgcgggccacaccgtggtggtcggcggcgagaagtacgagctgaagctgctgcccgcgggcgttttgagcgagaacgcgaccccgatcctgggcaacggtgtggtgatcaaccttgaagcgctcttcgccgagatcgacggcctcgaagcgcgcggtgcaaacgcgtcgcgcctcaagatctcctccaacgcgcacttggtcgcgccgtaccaccagacgctggaccgtgtgcaggagcgcttcttgggcaagcgcgccatcggcaccaccggccgcggtatcggcccgacctacgccgacaaggtcgcgcgcgtgggccttcgcgtgcaagacatcttcgacgagtccatcctgcgccagaagatcgagtctgccctcgacgtgaagaaccagatgctggtgaagatgtacaaccgaaacgcgatctcggtcgatgaaacgatggaatacttcctctcctacgccgaccgcctgaagccgatggtgatcgacgccgagtacaccctcaataccgcgctcgatgagggtaagcacgtgcttatggagggcggccaggccaccatgctcgacgtggaccacggcacctacccgtttgttacctcctccaacccgaccgcgggcggcgcgtgcgtcggctccggcatcggccccacccgcattaccgcgtcgctgggcattgtgaaggcgtacaccacgcgcgttggcgccggcccgttcccgaccgagctctttgataaatggggcgactaccttcaggaagtcggcggcgaggtgggcgtgaacaccggccgcaagcgccgctgcgggtggtacgactccgtcatcgcgcgctacgcctcccgcgtcaacggcttcaccgacctcttcctgaccaagctcgacgtgctcaccggcatcggggagatcccgatctgcgtggcctacgacgtggacggccagcgtttcgacgagatgccgctcacccagacccagttccaccacgcggagcctatcttcgaaacgatgcccgcctgggacgaggacatcaccggctgcacgacgttcgacgagctgccgaagaaggcgcaggactacgtgctgcggcttgaagagctctccggcgcccccatctcctacattggcgtggggcccggccgcgatcagacgatcgtgcgccacgacgtcatggcgcgttaggggcaggctgcttatcgacgcccccgtccatcacatcacccctcttcccgagtagcgagaccttcgccgggtggaaaggctcacgctctttacccctaaacgggtggagacttacgggtcgccgctgcgattctcgcgggcaccctgctgttcgacgcttgtgacccgaacggtgggttcaactcctcgaagaacgactcgtcttccaggaacgagtcctcctcgaagaagtagccgttaacggcgcctagccccatctctgctccacgcgggggtggggctttgccatgcgcaagatgggcccacccacgtggaataatgagcacctatgaagcttctaccgcgggttctggtgctcggttcgggattgatcgctgacgagttggctgttgcgtaccgcaggcttgggtgcgattcagcggtcgggtcactttctgacgccacccactacgacatggtcgtggttgcggatgacacagtgaacgcgggtgagctgcgcaccgtggccgagcaaacgcccgtcgtgcctgcggtgtctgcgtgtgccctggcgttcgaccgtgcggcgctgcgtcagaaagcctgtgaggagctcggcttgccgacgctcacctaccaacccacccgcacccctgaggagctcaccgccgcagccgagagcatcggttacccgctgattatgaaaccccgtttgggccgtggtcagcacgtggcgacgtcgcccgatgagctcgcgcacccgttcggggatcaggatctgatggtggagcggttcatcgatttcgattatgaggtcacgatccttacggttcgttcggttgatccggcaacgggggagttggccacgtggttctgcgagccgatcggcacgcgccacgaccacggtgagcttgttgaggcctggcagcccgccctgttgtctgaggccgccgctgacaacgcccgctccatcgcggcgcgcatcaccggtgcgctcgaggggtgcggcctgttcgcgattgagctcttcgttgatggtgaagaagtctacttttctcaagcaacgcccctgccgacgctcgacggcatgctcacccgcaccacccaacgtgtcgaccagttcgagctcttcgcccgcgcgtcgctgcgcctaccaatcgacgtcacactgaccacccccggcgcctccctcctcgcgccgcgcggcgtttccgcacctcgggatgcgttgacgcacgcaatgtcggtggaggaaacaggggggcagttgcttgccgacgccctcctcatccactccaccgccgacaccgttgaagaggcccgcgaccgcgccgcccgcgcggctgactacgacgcttaggcgtttcgacttctgagagaccacccacactttttcacccggctaccacacgcccgcgccggtagaattggtaggcgttcgcgcgctgatcagcgccgctgaccaactgccaacgacgaaaggtcacgcaatgtcccaacaaaatcgcctgctcatcacgtcggtgaaccgttccctggacggggtggataccgaagcactcgcaacccgcctgggtttgaccacggcgaacgtggagggcgcggacctcgccgcggtgtacaactccagcgcaaccgatgccgagaacaccctcctgatcggcaccggggactacaactttgacgcccaggtcgccgccgcaatcggggcgccggtggtgctcatcgctggtggcccgtctgctgagcacgccaggcaccgcgtggaggagcttggcgcggtcgttgcaacgacgctcaccgaggacgcgctcgctagcgccgacatcccggttgtcgaggctcaccccgtcatgtccccagctgtgtttgagaagcagctcatccagcaggcgaaggccaaccgcaagcacatcgtcctgccggagggcgaagacgaccgcatcctgcaggccgccgaccagctgctgcgcgacgatgttgctgagctcaccatcctcggcgacgaggcagacatcaaccgccgcgcctccgagcagggcctggacctttccaaggcccacgtcgtcaaccacctcgagtctgagctgctcgaagacttcgcggctgacttcgcggagcttcgcaagaagaagggcatcactctcgaccaagcgcgggagacgatgcaggacatctcctacttcgccacgatgatggtgcacaagggcatcgccgacggcatggtctccggcgccgcccacaccacggcacacacgatcaagccgtcgttccagatcatcaagaccgccccgggcgcctccgtcgtctcctcgatcttcctcatggtgatgcaggaccgcctctgggcgttcggcgactgcgccgtgaacccaaacccgaccgcggagcagatcggtgagatcgccgccgtctccgcgaagacggccgctcagttcggcatcgacccaaaggtggccatcctgtcgtactccaccggcacctcgggctccggtccggatgtggaccgcgccgtcgccgccgtggaggcagcgaagcaggccgacccgcagctggttgtggacggccccctgcagttcgacgccgcttgcgacgcgggtgtaggcaagaagaaggccccggattccccggtcgcgggccaggctaccgttttcatcttccccgatttggaggccggcaacgccggttacaagatcgcgcagcgcaccggcaacgcgctcgccgtcggcccgatcctgcagggcctgaacaagccggtcaacgacctgtcgcgcggcgccaccgtcgccgacatcgtgaacactgtcgcgattaccgccattcaggctggcgcacagggcgaggtgaagtaaatggcgtatgtgctggtgattaactcggggtcgtcgtcaatcaagttccagatcgtcgacccaaccgcaaccgcctccgacgcaccgtttgtctccggcctggtggagcagatcggtgagcctcagggcaaggtgaccgtcaagcacggcgaggataagtgggtggtgcagcgcgccgtcccgacccacaccgttggactgcaggagacgttccgcctgctcgactcgaaggggctcggccccacccagctggacatcgtggccgtcggccaccgtgttgtccacggcggtatggtcttctccgacccggagctgatcgtcgaccccgtcgtcgagatgatccgcaccctgatcccgctcgcacccctgcacaacccggcgaacatcgacggcattgaggtcgctcgcgcgctgctgccgcacatcccgcacgtcgcggtgttcgacaccggcttcttccgcacactgcccccggccgctgcgctgtacgcgatcaacgccgaggtcgctgaggcgaaccagatccgccgctacggcttccacggcacctcccacgagttcgtctcctcccaggtgccgcagctcatcggccgcgacccgctccacacgcgccagatcgtcctgcacttgggcaacggcgcgtctgcctccgcggtggagaacggccacccgatcgacacgtccatggggctcaccccgctcgccggtctggttatgggtacgcgctccggcgacatcgacccgggcatcatattccacctccaccgcaacgggggcttgagcatcgacgaaattgacgccgtgctcaaccgccaatccggcgtcaaggggctcgccggcgtcaacgacttccgcgagctgcgcaagatgatcgagaacgaggacgagaacgcctggctggcgtacaacgtgtacatcaaccagctgcgccgcttcatcggctcctacatggttgccctcggccgcgtcgacgcgatcacgttcaccgcgggcgtgggggagaacgacaaatacgtgcgcgccgacgccctggacaacatgcacatgtacggcatcgagatcgatccggagaagaacgcgctgcctaacgacggcccgcgcatcatctccaccgacgactccaaggtgaaggtcctcgtcgtgcccacgaacgaggagctcgcgatcgcgcagaaggcggccgccgtcgccgcgcgctacgccaaccgctagaacccgctagaaccaggtggccgggcggaccttgttcgccatgtccaccaacgcgtagcggtgcttggcgtagggggcgacgcgggcttgctcgcgcagcgtgatcgccagcccgcgccgtaaaccccgaacggtgaagtcgtactcaaacaacggcttggtgctcgcggcggcgctgaggcggttatcgctcaggtacgtcagcgccgcgcgcaggacgaagatcttaacctgcaaaaagcgcggctcggtgttggggatcttctccagccggcgcgccgcgcggcggatgcgcgactcggtgaggtcttgcgccaccaggcacagaatcgcggtgagtgatgccatgcggtggtgccgcgaggactgcggcacgcggtcgagggcgctcacagccagctccacctcgccctcgtgcatgagctggcgcgccagaccgaacgcggaagataccgtcgtcgggttggagatccacaccagcgcgtaaaggcgcatcgcgtggaagcgcagcatcgcgggatcatccgtggacatggaccagtcggcctctagcacgccgcgttcgatgaggtggtggaaggtggctgaagggatgtcggcaagcgagctgctcaaacttgcgctggcctgcgccaacgtgtcctccagcagcggttcttcgtggacacctgcggtttgcagcagtagctcgtccaccgcggcgagcgccagcttgggcgccgcctcgccgggcagggtgttgagcaccgtggagaagttttgctgggcggcgcggaaatcgcccagcagcaggttgaccaccccgaagtaccagaagtagcgccagtttttgccgtacttctcgtccaaggagtcgagccaggagcgcgcctgcgaggtaagccccaagtcaaccatggtgcgcaccacaccgaaggggatctccatggattcttcgtactgcggcgtgcgcatcgcttggcgcagcgtctccaaggtttcttgcggctccgcgtacgaggagccttgcagcatggcggcgccgatgtcggagcggtcaatgagcgggctggggagggcggcgacgacttccgccggggtgatctccacggtgcgggtgatgccgtcgatgagctggtcggtgtggaacaccaggtgcttggtgccgaacgtggtgcgctgcggggagaacaacgagtgctgcgcggggtgggtgcggccgtcgcgcaccgcgatgacctcgcgcagcacgccgagcagctgcatctccatcgcgcgggcggagtggaagcgcagctccgggtccgggtggcaggcgcgcgcgatcacgcggtacagcgagatgtaacggcggaacagtggctcgtcgctgggggtggggatgccgtggtcgtacacgccgccggttgcgggcaggtcgatcatcagcgccgccagggtgcgcccgacggtgtagatgtcggactcgatgctgggcccgtcgctgaccacctcaggagcctggaacccgcgcgtgccgtaaatgtagccgtacgcgccgatgccggacaccgcgcccaggtcgatgagtttgacctggtcctcggtgacgatcacgttgtctggcttcaaatcgttgtacaccaccccgcgcgagtgcagataggccagcgcgtcgaggacatccaacatgtaggcgatcgcgatgtccggttccaggtggtggttgggctctgcgttactacgctgtcttaaactagggccccccacgtactccatcacaatgaagccgccgggaacgcgcgggtcgtcgatgaagttgaagatctggacgatgcccgggtgcgtgatctcagccaggaactcccgttccgccgccgctgccgccgcctcgtcggggttgtcggtggagtgcaggcctttgagcacgaccacgcggccggcgacgtagtggtcgtgcgcgaggtagatccagcccatgccgccgtgggcgatcacaccggtgatctcgtactgcccggccaccacgtcgccctgctgcaaaagcggcgggggaatggacttctgcgtcacggccggggtggggtccaccagcgcgtccttcgggtcggtgggttggacccagggcagctccaccatgccgtccgcaacgaggcgggactcgcggcgggtgccgcggcgctcgcggaatgtgtcgatcgcctgcatgcgcgagcgctggctggggtcggcgccggcgcgcaggttctcgatgtcttttaagagcccggccatctcgccgaggtcgctgacatcgtcgtcgtcggcaaacgggtcgaacgccaccgcctcggtgccgggatcggtgccggggcctgtcagctcttcgttcacgagtcttcctcctctcggtacgtctgccgcggcagccacgactccgacagcgagcgcttcagccactcgttgtacatggcattccacgtcccgtcgctgcggatgcgctcgatggtggagttgacctggcgcacaacgtcgtcgtggcccttgggcacgcctacggcgtagcgttgcgacgccaacctgtccgaaaaaatctgcgccagcggatcctgggcgaccatgccggcgagcacggaatcgtccccgaccaccgcgtccgcctggaactgctgcagcgccatcaggcaatccgaccacgagcgggtgcgcagcaccgcggactggccgaagcgctcgcgcaccaggttcatcacgttcgtcccgtcggccacacagatggtcttgcccggcaggtcgtccacggattgcacgccgcggtcgcgcggcacgagcacgcgcacgtacgagtttaaatacggcgtggagaagtcgatcaccttcacccgctccggcgtgatcgacatggtgcggatgacaatgtccacatcccccgactgcagggcgttggtgcgcgaggcggagtcaacaaaccggaagtccacggtgtcggggtcgccgaacatgtcgctcgcgatctcgtgcgctaaatccacctcgaagccgcgcaggtcgccgcgggtggcgtcgcggtaggagagcaggtattgcgactggtccacgcccacgatcaggcggccgcgttcgcggatgcggcgcatgtgcggaccgtcgcggtccgcctccgagcccggctgcagcgaccccggccactgaaacgctttcgcgtcctgcacgaacccctcctcgggttcgacgccgggcggatccaactccgcaccgggcgggcggggcagttcgcgcctggccacgggaccggtgaccgcgtcgctgacggcgtcgctcgctaggtcgggggcaggggtgcaggatgagagaagcgtcgtaaagcaaatgccccaaagcgcaatctttttcatcggtagtactcccccaacctgcggcggatgccggcccagatgcacaccaccgcgaccacggtgagcagcgcgactgctgtagacacgcgcagcgtcgcatccagcgaggcggtgatgtaggcgcgcgtgctctcgcgcgagacgtcctttaagtgctgcagctcgcggtccagctctgcgtaagccgaggcggagccggggcgggcgttgagcaggtcgatcgcagcgtcgaaacgcccgttcgccagcagctccgtgagctgctcgtgcgccgccgcccagtcagccagcgccccgcgtgccgccgccaccgaggcctccgagccctccaacggctcggccgcgtccagcgccgcttccacctgcgcgcgggtctggtcgaacgagcccgccgagcgcgacaccgactggcgcgcgaggaacgtcagcgtctcgtcggtgcgcgcctcctgggcatcgatgcgcgcgctggcaagctgctgccacggctccacggcgcgctcgtagcccaccacgccgttttgccacgactggtagctggacacgccaacccagcccagcgcaacaacgatcgcggcggtggcggccaagaacccgcggttgaagcggcggcggaacgtgcgccacagccacacctgcgcgacggccagaaacagaagcgcagcgaccaggccgcttaagggcacccactgcggcgaggagagccggcgcacctccttcgccacctcttcctgcgtgagctgcgccagctcgtccgcgcgggcgagcatttgctcgcgcatcaccgcgctcgcctccgtcatgtacgccacgcccacggggttgcccaagcgctggttcaccttcgcgcgctccatcagcccggtgtaaacgggcaggtcgcgcaggatgtcggtcacgtcctcgccggcggtggaaagggcgccctcgtggatctcggcggcgtggaccgcagcgctgtctatcgacgcccagtagagctccatctgctcctgggttaaaagccccggctgcacgaacgccgtggtggagacggtatcggcctgcgagagggaggagtacagcgcgtgcgccgaggccgccatcggctcggtggacgtgatcagcgtgtccagcgcccgctgcctggccgccatcgactggctcatggaaatcccggcggccagcagcgcgagcgtgagcaccaccatcatcgccacgatcttgcccggagtggtagtcagcgcccccgccgtgccgcggacgtaccgggcaggctcggacagcgtctgacgcgagcccccctcggcccgctccagccactcatcgtccgccattccccaagaatatacagtggggcacatgcttggcgacggaaacggatgggtccaccacaaccacaccaaatactggggccttcacggggccgcagggcttttcctcgtcgccggcggccgcgcgctgatgcagcaccgcgccgcgtggaccgcccagggcggcacgtggggcatccccggcggcgcccgcgattcgcacgagagcgcttccgaggccgcgctgcgcgagacggtggaggagtgcgccatcgacgtctccgaagtcaccgtcaccggggagctggtcaccttctccgtccccgggtggagctacaccaccgtgcttgcccgcgctgatcgcccacttcgcgtcaccgccaacgaggagagcgaggagctgcgctgggtcccgctcgacgagattgctgcgctgccgctccaccccgggttcgccgcttcgctgcccgctcttgtccaggctgtggtgcatactgaaccgcatgattgaagtacaaggcctgacgaagcgctacggcgcggtcacggccgtcgatgacctcacattcaccgtcaaaccaggcgtcgtcaccggctttttaggccccaacggcgccggcaaatccaccaccatgcgcatgatcctggggttggataaacccacccagggcacatcgcttatcgacggtaccccgtacccctccctaaccaaccccgcccagaaagtgggtgcgttgctcgacgcgaaaggggtccaccccaaccgcagcgcccgcgcgagtcttttgtggcaggcccaggccgcgggccttcccacctcccgcgtcgacgaggtgctggagctggtgggccttaccgacgtggctggtaagcgcgtcggcggcttctccctcggcatgaaccagcgcctcggcatcgccgccgccctgctcggcgacccggagtacctgattctggacgagccggtcaacggcctcgaccccgaaggcatccgttgggtgcgcgggcttctgaaggccttcgccgccgagggccgcaccgtgctcgtgtcctcgcacctgctcgcggagatggcgcaaacggccgacaacctgatcgtcatcggccgcggcaaactggtcgccgacacctctgtcgccgagttcatccgcgcgaactctggggtgatgacggtggtgagggtgaagggggacgcaaataagcaaaagctcctttcggccctgggtggtgcctacaccgaggtcaccgacgccgaggggcgccccgcgatcgagattccggaccgggcgagcgacgaggtgggcgagctggcgtttgctgccggggtgccgcttctggagctgaccgagcggcgcgcctcgctcgaggacgcctacatccaatccaccgaaggccaagctcagtacgtagcgcaggcgcgacaggagggccagcatgcttaacctcatcaccgcagaatggaccaagctgcgctccaccgcctcgctgtggtggaacagcggcatcaccatcctcatcgccgcgctctatgggctgctgttcggctggactgcgaagttttccgcgatgccgtacgtgccgatcaccgtcgtcgcgacggtcgcgctgaccacggcgattgtggtggtggtgcagcaatcgatgatcgtgaccaccgagtaccgcttcggcatccccgccaccaacttccgcatcgcgcccaagcgctggccggtggcggcggccaagctcctgctgggcgcggtgctcgcggcggtggtgtctgttttgagtcttgtcgtggcgttcacgcttgctgatctcaccgcccccgtctccgccaactggcccaccaaccccgccacccagcgcgcgctatgggccgtgcctttggggatggcgcttttggcgatgttcacccagggcgtgggctggctcacgcgcaatacctccggctccatcgtcgcaggtctcgcggtgatgctggtgctcgaatcgatcatcggcatcatcccgcgcttcggcaccgagattgtgaagttcatgccctttggcaacctgctcgcgttcatgaccaaccagccgaccccgcactggtccctcggcgcgtcgctgggcatctacgccgtgtgggcggttgcggtgtgggcgatcggcgtgatcgtgctcgccgcgcgcgatgcgtaaggagctgttaaggttctgacccagtcggggtgatcagggggatcgctccactgtttttggggcttttggggggaagttgtggggactgtattggggccgtcggacacgggtgcggagctggctgccaagcttgtgtgccgctccgaggccgcgcggacgaagtgcctgaagttgtcagcgacgcggtggataccggttgcggaatgggagcagcttaagacttttgagcaggactttctccgctgctacgccgtcggtttggcggcgcggacgtcggtgctcgccggccgctccgccgcgtctgtttctgggatgtgggtgctgccgtccggcgacatacccgtcgagttgatcaaccaacgcgcccggccggtgcgctcgcagtggccggaaggcgtgatttataggcgccacacgctttacgacgaagacatcatcaccctcgaccctccccacaacctgcgctgcacccggcccgtgcgcacggccatcgacatcgcgcgcttccacggtttccgggagggcgtcgtggcgttcgacagcctgttccgcgggctgaagatgtgggagcgtgctgccatgacaaaagacatcaccgaaacattggagcggatggccggcgcgcgcaacatccaggccgcccgcgccgctttcgccgcctgcaacgatctttccgagtcgccgtacgagaccgtctgccgcctcatgctcctggagcgggacatcaccgtcgaggtgcagaagaagatcggcaactaccgcgttgacctgctgtggggcaacctcatcatcgagatcgacggccgcatgaagtacgccgacgtgccccacgacgttctggacaaacaaatggtccgcgagaactggctcaaggaacagggctacgaagtcatccggatctacccgagccagttgcttgccgacgaagccgccgtcctctcccgcatcctcgccgccaagcagcgcgccgacctccgcggcgagccggtggtgaaggctcggtaggtgtgttggaggcggtgtttgtttgccggtggtgcgcttgctggcggcgtgcgcctcgggcgcgagttttacggagttgtaggtctactgttgtagttcagtgcaaaacgccaagtggggaagtagaactacaactgtaggtatttacatcgaggatttggtgtctcgggcggggcgacactcgcttgggtctgggcgaggaccggcttggtgctgggatccggcgcctgcttcggatcgcggtcgccgcgtctggggcgcgagttttacggagttgtaggtctactgttgtagttcagcgcaaaacgccaagtggggaagtagaactacaactgtaggtatttacatcggggaaagggtgcctggggacgccgagcagatgcgttgcgaaagccgtgcgaacgggccgagggacaacgcgaacagtgcgagcggcggcggctagcagcagcgcctactgcagggcggaggtcaacttcatcacgttgtcgatgtagcggcggtgccaggggcgcttcgcccacacttccggggtgagttcgcgggagacggcgaggtagttggaggcgaggtcggcaagcgcggcgagcagggagccctcggcgatgaacaggctgttttcgtagtttagcgagaaggagcggatgtccatgttggaggagccgatggcgccgacgccggcgggggagccggggtcggcgagggcgaacttggtgtggaggacgtacggggcggggaattcgaagatgcggacgccggcctcgaaaagctgctggtagtaggaggattgggcgtgttggaccatgaattggtcggccctttcgccaacgagcaggtccacgcgaacgccgcggtagcaggcggacgtgatggcttctagcagcgaatcttcgggcacgaagtagggggagcacagcaccaggtgctcgcgggcgtggctgatcatggcgttgaacatgcgcaggttcggctcggtgaggtaaccggggccagaggggacgagctgcacaatgttggcgtcagcggcatcgaacgaagcagctgacggcggcgccagctctaacacctcgtcggtctcggtgtaccagtcgacggcgaacatggactcgagcgaggccacgatcggcccctcgagttcgacgaacgcgtccacccactgccgccccgcgcgcacgtggcccggcatgagataaccgcggtcgatgaggttgaaggagcccatgagggcgaggtgggcgtcgataagcagtagcttcctgtggttacggaggtctggccggcgccacctgcggcgcagcgggtcgagcgggagcatcatgtgccagtcgacgccgatggcggtgaggcggcgtttgagcgcgcggaagccggggtacttgcgggagccgatgtggtcgaagagcaggcggacgtggacgccgcgggtaacggcgcgctcgatggcttcgaagacgggtgcggtggtctcgtcccaggccacggcgtagatctcgatgtggacggtgtgctcggcggtgtcgatgagctcggccatgcggcgcatcgtcatgtcgtagtccgtccatagcgcgggcgcgcgggcgggaagcgccgggtagccggtgagcgtgcggttgaggtgcacgatggcgtctttgtccggcggcagcgcgacgcttgccacacctgcgtggatattttccaccgctgccttggcttggtgctggatgcggtggcggcggcgcgacaccagcgtcgaacccatgagaaggtacagcggcaggccgacgaccggcacgaacaggatcagcaacagccacgcgttggcggaggacggtttgcggttgcccggcaccacgccgatcatcacgatcttgatcaggtaatcaacgatcaaaaacgcggtctgcgtcatcgcactgcgtccagctccagatcgtgggtgtcgaagtcggcgaccaccggcgcgtggtcggacgcgcccttgccgcggcgctcctccacgtcgacccaggcgccctgcagccgcgtgtgcatcgggtcggtggcgagcatgaagtcaatcagcatgccttggttcttttgaaagcgcatggccttgtagtcccagaagctgtagcggtcgtcgtggcggatctcggtcagcccggcctccagcagcatctggaacgcggcgcgctccggctcggtgacatgcgtgcggccttcaaaaaacgcgatgtcccacacgttgtcgtcgcgcggcgcaatgttgaagtcgccgcagagcagttggcttgtcgacgccgccacctcccccctcaacgaccacaaaaattgcaacttgtagtcgtagtgcgggtcgccgatctcgcggccgttggggatgtagaggctccacacgtcgaccccgccgcaggtcgcgcccacggcgcgggcctccaccttcggcgcgcccgtcttggcaaacttcggctgccgctcgaaggactcgcgcacgttgtcaaggccgacgcgcgaggcgatcgccacgccgttccactgcgagtagcccacgtgcgcgacctcgtagcctgcggcctcgaaggtggagtaggggaacttgtcgtccgccgtcttcgtttcttgcatacacaggacgtcggtgccgctgcgctcaaggaaggcggcgatgcgctcggcgcgggtgcgcaccgagttgacgttccacgtggcaattcgcatgggtcaaccctacccaagcgggccgtcgaaccgggcgtagcgctcgcggtggtgctcggtgaacccgagcttttcgtacaacccgatgccggcggtgttgctggcgcggacctgcaggtaggcggcgtcggcggcggggtcggcgctcatgccccacgcgagcacgctctcacacatcgcggtgccgataccgcgccggcgccagccgtccgcgacctcgacggcggaaaagcccagccagcgggtgccgtcgccggattcggtgatggtggcgcgggtgacggcgaccgtttcgccattgacgacgtagcgcgcaaacccgatcacgccgtcaatggactgcgccagatcaagcaccgcttcggccggcaagtcctggccgcggtagtggtacagggcgagccactcgtcgtcgggcgcggtgtcgacgcgcacgtgcgggtccatttcgggtgcggggatgtccgcaagcgcggcggacatgaccaggatttcgcttccaagcacccagccctcgcgctcgacaagtttgagtgcgggcttgccaatgcgctccggaatcagcagctgcaccggcatctcgcgcacgcggtaaaactccgcgatctcggcgatcggcaccgggttgaaacccgccgagtggccgatgggggtcgcgctgttggagcgctcagcgatttcggagccggcgcgcacgagccagccgccgaccatcagctgctcctggcccgggaacgcccgggctgtggcggtttcgatcgcgcggatgtcggagttgcgcacggtgcgcggggagagcttcttcatgatgtggagctcaccgatctgcacgagctcgtcgccccggcggatcaccagcggatcgaccgactcgacgaacccgatgacgtcgctcgccagctcgccgcgccgctgccgcaccaccacgcgatccccgaccgcgaccgggtcggagcggaatacccgtggcacttacgcgcggcgggtgaggtaaacgccgcccgcgaccagaagcgcggcgatcgcgagcacgcccagcatcggggtgccggtgtccgctaggtcgtcgtcacgatccgccgtggtcgtggtggtggtcggcttggagctcgaggtggacgaggtcgacgaggtagtcgacgacttcgtgctgcttgccgtcgttgtcgcctcggtcgtgcggttctgcagcacctcggcggtcatgctggtggtcgcttcggtggtggtggacgtgacgatcgtgctcgtcggctccgacgtcgtcgttgccgccgtcgaagaggtcgacgtggaggtcgtcgtctctgtctccgtgtcttggagggtgatcacgcgctgggaaagcgacggcgtcggctcagccggtgacgcaggggctggcgcggtcagctccccgaacgcgacctgcttgtcgtcctcggagcgctcgacagcgtcgagggctacctcgcgcaccacttcgatctcgcccagcaccgttggcagcacaaccgcgtcgtcgtcctgcaactcggcgcgcagctcgcgcacgagcgcgcgctcctccgcaatctcgtcgagcgcctcggcgaaggcctccgcctcctcctctgtgagggtgccctcggcctctgcggcctcgctctgcgcgacgatctcatcaccttcggcgattagcgccttgcgccactgcgccaaagcaaggcggtagtcggcctcaagggaggcgcgctcgggggtgtccaacgtggcgtcgtcaagcagctgctttgcctcaagcgcaacctcgcgccactgcgccaccgtgggctgcgccgaaacggttgtggtgggcgtggtggccagcgcggcgggcgtactggcagcgagggcggcgacggccgccgtgaaggcgaaagcggggcgcatgcgcctaagcatagtcagcgggacccgcgcgttcctactaatgacggaacgggtccggatccgtgcccggcagccacgtgtttccggcctctgtccagccgttatcgcggatcgcgcgcttggcttccttcttccagcggccggtcagcacgtcggtgtagacgtagccgtcgaggtggcccacctcgtgctgcaggcagcgggcgaaaaatccggtgccctcgacttcgatctcgttgccgttttcgtccagcccggtcaccttcgcccagtcggcgcggccggtgggccagccctcgcctggtaccgagaggcatccctcgtcgtcctcgccgtcgtcgcgcggcatcgtcttcgggatctcgctggtttccagcaccgggttgatcacggtgccgcggcgcatctcttcgccgtcggggcagtggtacacgaacaagcgcagcggaacaccgatctggttcgccgcgagcccgacgccgttcgccgcgtccatcgtctcgtgcatgtccgcgatcagctcttgcagctcctcgaccggctgcgtgaccttctcggtcgggttgtgcaggacggggtcgccgtagatcacgattggtcgaatagtcatgcttatatattaggcatgctcccgcccgccgatctcgccctcctcgacttcgaggcccgcgccccgcgctcgctcggcgcgaaggaggaggcgatccgccgcgagctgggcatcagcccggtgcgctactttcaaaagctcaacgcactgctcgactcgcccgatgcgctagcggccaggccccagttggtgcgcaggctgcagcggcttcgcgacgccgccgacacacccctcggccactaacccgtgcgtgcgcgcggcgcgtcacaaaccctcaaggtgaagttgagggtagtgttgcgcgcgtgagtagcagatacaccggcaacggcccgagcgacgaccgtgactacacccagtacaccgactaccccggcgacgattacgcagatttcgaggacgtcgtagacgagcagccggagtacgtcgagcatgacgactacggagattacgccgactccgctgagccggtggaggagtacgccggtgcccaccgccgccgcgacgcggacgattttgaggatggtgttgatgccgggcgtgagtccgccggctccaccgccgcagccgccggcggcgtgccgaagcgcggcctcgccatgatcctcatcgccgtcgcagcgctgctcctactctggggcatcttcgcgctgacccagaaggacgacgcaggtaacgcgggcgactccggcgcgaccagcaccgctgtgacgactgccgcttcggacgctgccggcgccaccgctgcagaccaggccaccgcgaccgcgacggccaccgagttcgccaccgcgaccggcaccgtgatcccgccggcgccgtcgaccgtgccgggcgtggacgaggtcaacgacccgaacaacccgaacaacccggcagcgcctgccgctccggccccggcgccagccacggacggcggcccgcgcatcaccgagcagaacgcgcaggtctacgtctacaacaactccctgcgcaacgacgccgcgaccaacaccgccgccgccctcaaggcggactacaacgtggctaaccgcgacgacgcgcccgagctgatgaacatgccggagcagaccttcggcaccttcggccagaccacggtgctctacgacccccacgctgacggcgcccgcgaaactgccgaaaccatcgctcgccaggtcggcggcgtggtcgtcccgaacaacaacctgcccgcagacgtcatcgaccttccggcagccgtgaagggcaaccgtcaggccatcactgtggtcatcgctggtcagtaaccggaagactgcgagtaagctgatccctcatggatccattccgcgatttcgcccgctcacccaactcaaccctcggtgtcgagtgggaaatctgcgttattgacccagtgacgcgcgaccttgtgccccgcgctgccgaggtcatcgacgaggtgcacgcccgccacccagagacccgcctcgaacgcgagttcctccagaacacgatcgagctggtcaccccgatctgcgcgaacacctccgaggccatcgccgcgctcacccgcgacctggaaaacgtccgcggtgtcgccgagtcgaagggtctgaaactctgggctggcggcggccacccgttcactgacttccgcgagcagccgctgtcgccgaagaacacgtacgaggagatcatcaaccgcacccagtactggggccagcagatgctgctctggggcgtgcactgccacgtgggcgtcagccacgaggacaaggtctggccgatcatcaacgcggtgatgacgaagtacccgcacttgctcgcgatctccgcatcgagccccgcgtgggaaggcctcgacaccggctacgcctccaaccgcaccatgctctaccagcagcttcccaccgccggcatgccgtaccagttcggcagctgggacgagtgggtcgccttcatgcgcgaccagcaaacctccggcgtgatcaaccacaccggctccatgcacttcgacgtccgccccgccgccaagtggggcacgatcgaggtccgcatctccgacgccacgagcaacctccgcgaactcgccgccgtcgttgcgctcacacactgcctggttgtctactacgaccgcatgctggaagccggcgagcagctgcccactcttcagccgtggcacgtcgccgaaaacaagtggcgcggcgcccgctacggcctcgacgccgaggtcatcacctcccgcgccaccgacgaggcatgggtgcgcgatgagctttcgctgcttatcgacgccctcacccccaccgcccgcgacctcaactgcgaggcggagctcaagctcgtcgaggagatcttggaccgcggcgccggttaccagcgccagcgcgacctcttccgcgaaacgggcacttggcaggcggcggtcgacgcgtccgcgcgcgaactcgtcgactggcgcctctaaccgcggcggttcctggggcagcggggcccagattcaccgatgtgtatagctacatgtgtatatcaaccccgcgtcctgcggttttagggttgtcctacaactgtagctatacacatcggggttgatggcggggaacccaggatgtgtgagcacctcggcccagtcctgtcgggagggcgtctggaggagggcgtctggaggatggcggatatgccccctcttttcggtacttccgccctccgctatccgccctccgccagacgcccccggggagcgaggtggcgcaccggccggctcaacccgccaccgcgaaacccttaagtatccttcgccgttgggttgacgcggcccgggtggtaggtcgccgggcgttcattcaccgcgagctcatcctctgggccgtacagaccctcgatgcgcgcgatgcggccgaggcgctgcgcggtcacagggttcgtcatcagcgcaaagatgaccagcagaatcatcatcccgatgtcgccctgctcgtgggggccgaagtcgggggcgccggtgaggcggatgatggtgccgatcatcatgagcagaagccccgtggtctgcggtttggtgatcgcgtggacgcgcgcgagcgtcgagccgaagcgcacggtgcctacggcggccgagaacaccataaacgcgccgagcaagatgaagaagagcgagacgatgtcggtcacaagtgtcatagcgagctgtccctcttgcggaagcgggcgacggaaagcgaggcgatgaacccgagtagcgcgatcacgatcatcacgttgaccacggtggtgtccagcgtccagcagatgtagagcgcaagcgcgcactggagggaggcggtgatggcgtcgttggcaagcagtcggtccatcgacgacgggccgacgatcacccgccacaccaagatggcgaagcctgcggccaacaacgctgccgcgatcgcgaggaacgtgttgtagagcgcggggtccattattttggcctactttcgaagatgtcgatcatctggcgttcgagtttgagcacgttgttgatctcgttctggatggattcaggcgagctggcgtcgagaatgtggatcgtccattcgcgctgtgcgatatcaatatccgtcaccgtgccgcccggctgcaggttgtaggcgcaggtggccaggtagaggacgagctcggagtcgacgcgcatcggcacgcgcaggatcgcgttccgtggcggtgcagctggtcgaagggccagccaggcaacctttgccgacgctacgagcaagtcccacagccactcacccatgaagagcacgagctttccccacgccacgcgatagccctgcagcggcaccggtggcaggggaagcgcgaggacaatcagcagcgcgagaccgatgcccgcgatgacgttgccccaggtgatttcgcccatgagcaggatccacatgaccgtcagccacacgatgaacggccagcgcaggcggtgtttcaaaccttcaagcattagttctcaccgccgttctcagcgtcgtcggcggcgggggccggcgcgcgccccgtcgtcacagcagtggtggcgtgggtgcgaccctcgccggtggtggtgcggtgctgttgcgcgtcgctgccaccgcctgatgtcgtcggcgcgaggaactgctcaggccggcgtgtggggttgtccgtgtcgccgctcagcaccgcgtcgcggtagatggactggtcctgggcggactgggcggcgcggtcggtgatgtcggagatcgggccggccagaaacgtgatggagaccgaggccgccaccagcagcgcggtggacgccagcatgcctggcgggatgcggcccgggtcttcgcgctcggtgatcgtggtggtgttgtagcggtcggcgagtgttgacggccgctccaacgccacttggccctccggtgcgtcctcgcggtcgcggaggaaggccttcgaccacaccagcatcatcgcgtagagggtcagaagggaagtgatgacggcgcccgcgatcagcacccaggcgagccaggtgccggattccgcgccggcctcaatgagcatgatcttgcccaggaagccggagaacggcgggatgccgcccagattcagcgccgggatcatgtacagcgcggcgaccagcggcgcggtgtacatgagcgagccgaggcggcgcagctgcgcggagccggcctggcgctccattaggccaacgaccaagaagagcgaggtttgcacgagaatgtggtgcaccgcgtagaagatcgcgccggacagtccctgcaccgaggcgagcgcgataccgaagatcatgtagccgatgtggctgaccagggtgaacgacaacagacgcttgatgtcgttctgggcgagcgcgcccatgatgccgatgatcatggtcaaaagcgcgacccacatcagaagcgtgtccagcgagccgtcggtgaagaccaccgtgcgcacgcgaatgatcgcgtacacgccgaccttggtcagaaggccggcgaagacggcggtgacaagcgaggcggcggtggggtaggagtccggcagccacgcgtcgagcgggaagaccgcggccttgataccgaacgcaatcagcagcgtggcgaagatcgcggcgcgggtgccgtcggggatctcttccatgcgcacgcctacctgcgccatgttcaccgtgcccacggacgcgtagatcatgccgagggcaaagaggaagatcattgacgacgccaccgagaccatcacatacccaatacccgcacgcacgcgccccggtgaggcgccgagcgtgagcaggacgtaggacgcgacgaggaacacctcgaagcccacgtagaggttgaacaggtcgccggcgaggaaggacaggtttacgcccatggtcagaagcatgtaaatgggcaggaacacggcgacggggtcgtcatcgtcgccgtcgcgaagaccctgcgacatgccgtaccacatcaccccgaataggacgagggatgagacgaataacatgatcgtcgacaagcggtccgaaaccagcgtaatgccgaccggtgcgtcccaaccgcccatctggactgtctggatgccgtggacgtcgacagtcacgatcatcgtcgcggagatgacggcgaggaccaacagcgtggacagcgcgatgaagcgctgcagtcgcaggtgcctgccactgatgaggatcagcgcggcggcgagcgcgggcaggaggatcggcatgaccgtcaagtacggcatgtagccgatggcggtgtccgcgacgtggagcagattatccttcaccgtcggcctccttcacggggttctcgaacgagcgggggccgaaggcgtcgccggagacgctcagacggccggtctcggggtcgtcggaggcgtcgtggtcgggcgcagccgaaggggtggtgggccgcgaggcgatcgcgcggtcctcctcgtcgcgctcgacaacgtcgtcggtgcggtagcggtactggcggtacgccaaagacagcatgaacccagtcagcgccatcgagataacgatggcggtcaggatcatcgcttgggccagcgggtccgccatttgggtggcggcctccgagtcgcggccgaggatcggcggggagccggcctggccgccggactgcagcaccaagaggttggcgccgttgccgatcagcagcacgcccaagatcatgcgcgtcattgcgcggtccagcatgaggtagacaccgcacgcgatgagcacgccggagccgatgagaagaaacaggttggcctgcatttagtcgttgccctccttgcgcgcggcgatgcgctccttggctctggtgaggcgcgcctcgcgctgctggcggcggcgcaggcggttcttctcctgcatctcgcgggcccggtcgcgggcgcgctccttgcgggcgtcgtcttcgcggtcgaggtaggcgcccatggaggtgagcacgtgcatgatcagaccgatgacgatgaggtagacgccggcgtcgaaaatcagcgccgacggcacgtcgaactcgccgatcagcggcagctccagcgagatgtagttgctcatcagcggcgggtagccgaacagcatcggcgccaccaccgcgacggaggagatcaggatgccggtgccgaggatcttcgccgggtcgacgggcagcgcctcctcgatctcgtaccgccccccggctaggtagcgcagggtaaatgcgagtgccgcgacgaggccgccggcgaagccgccgcccggcgcgttgtggcccgagaagaagaagaacgcggacaagagcatcatcgacgggaagaggaggcgggtggcaacgtcaaccatgatcgagcggttttgctcgatttccgacgccaccccagacgccagccaccgcggcttggtggtggacagcgtcggccttctcgattcccggccgaacttaccggtgccgaagatcaggctggccacgccggtggcggcgatgaccagcacgagggtctcgccgaaggtgtcggccgcgcgcaagtcaacgagcaggacgttgaccgtgttgcggccgtggccgatctcgtacgccagctcgggcatgttcttagagatcggctcggcgacgcgcgcggacatcgccgtcatggcgaccacgaccacggacaggcccgtgccgatggagagccaagcgcgcaggcggttgtcctcgttgcgcggctcgatctcggtcggcattttgcgcagcaccagcatgaacagcaccatcacgatggtctcgaccagtgcctgggtcagtgccaagtccggcgcgccgtgcagggcgaagagcatggccattgaatagccggtgagccccaccatgaccacggccgagaggcggttgcgctgcaacgtggcgaagacagccatggccaccatgagcacgaccacgatgccctgccagacgttgtcccacacgatcatctggatcgagttggaggcgcccaggatgaggtaggccagcggcacgatcatcagcgtggcgaagatgacggccaagttgatcgtgagcgagccgcgctgcgtggaggcggtgagcttcaacgagatgttgcgaagcgcgttgaggaggttgtcccagaccacgttggcgtcgccaagagccgggcgctcgagctgcgcctttcgcaccaagtcccgctgccagaacataatggtgcctgcggcgacgatgaccacggtgaggatgagcgggacggtgacaccgtgccacagcgcgagctcttcggcctcggtcgcggggaagcgcacgtcgaggtactcgttgaacgcgtgagagaggaccgtgggcatgagtccgaagccgacggtcaaaaccgcgagcacgagcggggagagccacagggtggggccgatggggtgcatctcgcgcacctcgtcggtgaagccgtcctcgtcggtgtccatgtccgcgtagcgcgggccggtcttggtggcgaacgcgccccagaggaagtacagggtgtaggccatggtgaggatcgagcccactaccagggcgacaagggtgatgctgccgggcatgccgtgcagcagctcctcgtgcaggaccgccgcaagggcagcttcctttgcgacgaagccgaacagcggaggaatgcccgccatcgacgcagccgagacgatggcaatcgcggccaccagcggctccttcttgcccaggccggagaggtggcggatgtcgcgggtgccggaggtgtggtcgatggcgccgacgaccatgaacagcgccgccttgaacatggagtgcgcgaacgtgatcgccagcccggccatggtcgcctcgcgcgagccgatgccgatcaccgcggtgatgaaacccagctgggagaccgtgccgtaggcgaggatgagcttcaagtcgcgctgcttcagcgccatccagccgccgagcagcatggtgaagcagccggtggtgatgaccacgaggtgccaggtggtgacggcggccatgtctggggcgaggcgggcaaccaagtaaatgcccgccttcaccatggcggcggagtgcaggtaagcggagaccggggtgggggcggccatcgcgccgggcagccagaagtgccacggcgcctgggcggacttggtcagcgcgccgagcatgatcagcacgatcgcggcggagataccggtggtgccctcaaggtcggtgaactgggagatctcggagagcttccagatgtcggtctggtggccgagcaggatgatgcccaccagcatggctaggccgccgaacgtggtgaccatgagcgcctgaagagcggcgcgccgggagctggcccgttcgccgtaataggagacgagcaggaaggacaggatggacgtgagttcccagaacacgtacatgagcaggaagttgtccgagatcaccagcccgtacatggtggtggcgaaaagcgtgagctcgcaggcgaacttggccagccgcacggggttctcgtcgaagtagccccagcagtagaacagcaccagcgcgccgacgccgaggatgatcaggctgaacaggccggcgagcgcgtcgaggcggaactccaagttcaggtgtgttgacggcatccacgtgtaggcggcgacgatctcgccgccgtcggtgaacgcgccgttcacgaacagcgagaccatccaaataaagccgccgagcggaaccagcgcgatcagcgcgaacgcccagcggcctaaaactctaagcaggattggcgcggcgacggtggcggcggtgagcgcaataagcagagtcaacacgtccggtggccctccttcttgcgtagtcggtcgggtgaaaatcgacgcaatgaggtagcgcagccgatgtgtgacactttacccataagaaggtgtcgcgtcattaaccctttttgacctgcgtgcttgtgcctgtcttaggttttgtttagttgaagtggttaactacttgccgtagcgggagaggaacgtagcctccgcaaccgcgacgttttcgatctcggtcgggtcgacggactcgtctacgccgtggatgccgcactgcggctcttcgacgccgaagacgacgatctccgcgtccggaaacgtctcctgcagtgtgacggtcagcgggatggagccgccgccgccgacgacggcgaggtcggacttgccgtacgcctccttcaagcactggccgagcagctgaacggcctcgccgtccgggttggtggcgaacggcttgttcacggcgctgatggcgacgtccaccttcgcgccccacggggtgtgggcgaggatgtgctgctctaccttggcggcaatctcgcccgcgtccgcgccggcgggcacgcgcaggttcagctgcgcctcggcgcgggggttgacggcgttgacggcctcggcgaccggggtggaggtgaacccgatcatggtgagcgcggggcgcgaccacaccatgtcggccggctcgtcgtccacggtgccgagcagctgcacgccgtcgaggacgcccgcgtctgcgcggaattcctcgcgggtgtacgggtcgccctcccacttggcggttgcgtcgacgccgtcgatggtggtgcggccgtgctcgtcgaaaagcgagtcgatgatgcgaaccaacgcgtgcgccgcgtccggggcagcgccgccgaaggagccggagtggatggcgccggacagcgtctcgacggtcacgttgatctgagcgccgccgcgaagcgaagtggtgagcgtgggcacgccgacggcggcgttgccggagtcggcgatcaggatgacgtcggccgtgaagaggtccgggtcggcttcaatgagcttgaccaggccgtcgaggccgccgagctcctcggagccctcgacgacgaccttcaggccgaggtcggtgccaccggcagcctcgagcagccgcagggcctcgaggtgcatcgcaaggttgcccttgcagtctgcggcgccgcgaccgtaccagcgcccgtcgcgctcggtcagcgtgaacggatcggaagtccacgcctccgggttgttcgcgggcacgacgtcgtagtgggagtagaggaggaccgtgggggcgtcgtcaagcggtgccttgtagccgatcaccgtatcggcgtcgtccaccgtcgggtggcgcgcgacgtccagcccggcggcctcgagggcgttaaccacccactggcaggcggcctcgtgctggtcggccactgccggggtggagtggacggagttgaaggagaccagcgcggacaggtcggcgaaaatccgctcgcggtcgggagttccaattgcgtgtgcagtgctcatggacccgaagctaccaccgcgccacaacaggcccggctccttgcacttgaggtgggcgagtgctaaaaatgggggctagcactcggacgatgtgagtgctaaatgacatctcaggcaggtgggctgcgctagaccgacagccgtgccgtcgcgggcgcctgctttagaaaacaaaacgaactgaggcatcaactcacatggcaaagatgattgcattcgacgaggaagcacgccgcagcctcgagaacggtctgaacaccctggcagacgccgtgcgcgtcacccttggccccaagggccgcaacgtggtcctggagaagtcctggggcgcaccgaccattactaacgacggtgtgaccattgccaaggagatcgagctcgaggatccgtacgagaagatcggcgccgagctggtcaaggaagtggccaagaagaccgacgacatcgcgggcgacggcaccaccaccgctaccgtgctggcacaggcgctcgtgcgcgagggtctgcgcaacgtggcagccggctccaacccgatgggcatcaagcgcggcatccaggccgccaccgacaaggtgtcgaagtacctgctggacaacgccaaggaggttgagacccaggaggagatcgcttcgaccgcgggcatctccgctggcgatccggagattggtaagaagatcgccgaggcgatgtacgccgtgggcaacggctccgtgaacaaggagtccgtcatcaccgtcgaggagtccaacaccttcggcgttgacctcgaggtcaccgagggcatgcgctttgacaagggcttcatctccgcatacttcgccaccgacatggagcgcggcgaggctgtactcgaggacccgtacatcctgctggtctccggcaagatctccaacgtcaaggagctcgtgccggtgctggagcaggtcatgcagtcgggcaagccactgctgatcgtcgccgaggacgtcgagggcgaggcgctgtccaccctcgttgtgaacaagatccgcggcacctttaagtctgtcgccgtgaaggctccgggcttcggcgaccgccgcaaggccatgctgcaggatctggccatcctcaccggcggccaggtcatttccgaggaggtcggtctgtcgctggagaccgccggcatcgagctgctcggccaggcacgcaaggttgtggtgaccaaggacgaaaccaccatcgtccagggcgccggcgaccaggagcagatcgagggccgcgtgcgccagatccgcgccgagatcgagaactccgattccgactacgaccgcgagaagctgaacgagcgcctggccaagctggcgggcggcgttgcagtgatcaaggtgggtgccgccaccgaggtcgagctcaaagagcagaagatgcgcattgaggacgccgtgcgcaacgccaaggccgccgtggaggagggcatcgtcgctggcggcggcgtcgcgctgctgcaggctgcgaaggagctcgagggtgagcttggcctggacggcgacgaggccaccggcgtgaagatcgtccgcgaggcgctgtcggctccgctgaagcagatcgcgctgaacgctggcctcgagccgggcgtggttgccaacaaggttgccaaccttccggacggcgaaggcctgaacgccgcaaccggcgagtacgtgaacatgatggaggctggcatcaacgacccggccaaggtcacccgttccgcgctccagaacgccgcgtccatcgctggcctgttcctgaccaccgaggcagtggttgccgacaagccggagccggctggcgctaatgccggtatggatccggaagccatgggcatgatgtaaacttcgcccacgctcaggcccgctttacgcgggcctttcgcgtttttaaggcagaggcagctgcttgacgacgcccaccccagctagcccacccccaaattggggaacgcccgccgatgtagtggggcataggtatcgggaccagcatgtcgatgcgttacgccccgattcgggatgtaaactctcttttactttcggctcagcatctgccctgctagataaccagctcggcacaaagttaaagattggtgaacagaagctgtctgtccgcgcgttggtgtgcgagcgatttcgaaaacgaacagcgcttgcgtttctcttgctacgtggcataattctctacgtgatgccccgcgagggtgtcagtacattgtcaagtttttgccaggcaccagctggcacaacctcttaaggggaagacatggatcagcagctgatcaaggacaccatcaaggttctcaaggacttcggcaagttctggaccgagctctacaagatcaccgacggtctgccgtcgctggtcaacaagtggaactcttgggacgccaagagcgactgggatgccaccaaggccgttttcaccggctcctccaagtaaatcgtaaactcacctgattcccacataggagaaaaataatggacaacttcgttaacggctgggttgctctttctagccagtccaccatcaccggccagatcctctactccatgaaggctctgggcgacatggctaaggcccttgctgagcttcttagcttggtctaaagcaaacacctgctttccgacacggcccctccgcttcggcggacgggccgttttgttttttctttcgtgatacatcgggccaaggcgcgtgagtcctacgacgcgcaggggtgcaaggtaccgcgtagaatttacggtatggctgaccacaaagacgacgaactgccgatgatcgacctcgccgaaaccgagggctgggttgtcgatgataccgacgaggatgatccggtcctgctgatgccggacggcacgcctattcagacttggcgcgagcagtacccgtacgacgagcggatggggcgcgacgagtatgaggagcagaagcgcgcgctccagatcgagctgctgaagtggcagaactggacgaaggatactggtcagcgtcacattattctgtttgagggtcgcgatgccgctggtaagggtggcacgattaagcgctttaacgaacacttgaaccctcgtggtgcgcggattgtggcgttggagaagccgtcgccaagagaaagcacctcttggtacttccagcgttacattgagcacttccctgcggcaggggagatcgtctttttcgaccgttcttggtacaaccgctccggtgtggagcgcgtcatgggtttctgcaccgagtcgcagcatgccgagttcctgcgcgaggtgccgatgctggaaaacatgatcctcggctccggcatttccctgaccaagttctggttctcggtgacgccgagggagcagcgcacgcgcttcgcgattcgccaggttgacccggttcgccagtggaagctgtcgccgatggaccttgcttcgttggacaagtgggacgattacacgcgcgcgaaagaagagacgttccgctacacggacacggacgagtcgccgtggatcacgattaagtccaacgacaagaagcgcgctcgtctgaacgcgatgcgctacatcctgagcaagttcgagtacaccaacaaggatcacgatgtggtcggcgagccggatccgaagattgtgaagcgcggccgggaccagatcggggattaataggcaatctctttagtttgtgattacggccgcgagcatggcggcgctaccggacggaagtcggtggcgccgccttcgttttgtcatggagctgtgggttaggtagcgcttttcaggtgacgggtgtctgagatgctgtcagatcgctgagttacgcgcgttgagaacgagcagttgcgggcgcgtgcaggatagtgcacggggaacggccccgcgggccggggtacttcgttcgaacacgcgcggccggggtgagcgagctgttcttgcagctagttcctttgctgcccccgtctgctatcgaaagcccctctcgaacatctatgtggatgtgcgctaaacagcaaattgatgcccgtgtgacggttgtgattgttgagtttaggggttacggtgggtctaaccctgaagtacaggtacagacttgctgtgcgccggtcgttatcttgctttaggatccacttgcctttcacctgtcaaggagagatagatctatgaagcgcattaacaagtccgctattgcggtagcactggccggcgcgctgacgctcggcgtttccccgatggctggcgccgcaaccccagcaaccctcaagcagggcgacgtggtgttcgatgctgacggcaacattgtcacctcgttcagcggcaccaccgacggtttggtggtcctcgaggacggcgacgttgtgtacgactccaactcccagaacgtcaccgctgaccgctccgccacggctccggctgctcccgacgcacctgcaccgcagggcaacacccccgcaactcttcagccgggtgaccttgtctacgatgcggacggcaacatcgtcacctcgttcagcggcactgacaacggctacgtcgttcttaaggatggcgacgtcgtgtacaactccaactccgaaaatgtgaccgcggagcgttccggcaacgcgccggtagttgagggcgagattgtgagctcgaccccggtgacgctgtccaagggtgatcgtatcgttgacttcgctggcaccgagaagctcgttgctgaggctgacggtcagcttgcgaacctcgagccgggcgaccgcgtcgtcgctggcgacggcgttgaggtcaccaacgagcgcaagggtgttgagggtgcaaatgttccgaccccggtgacgctgagctggggcgacatcgttgtagataaagacggcaacgtcgtgctgactgcgaaggccaacggcgagtacgccgttctccagccgggtgacaaggttatcccggcaggcaagatcggtgctggcgtgcttggcggcctcggtgctctgaccctcggcggcattctttacaacgttgtgaagaacgcgcagggcgagaacgtgctggtcccggcagatcgcccggatcagaccccgactgctgaggacgaaaagaagactgaagagctcgtgcaggcgcacgcggacgagatcgctgaccaggctgcaaagcagaacgctgccaacggcgagctccgtggtgtcggcgccaacaccggtaacaacgccttcggcaagggcctcatgaccctgctgctggcttccgtgcttgctgctgcggcgttcgtgttcggccgccgccagctggtctaagccccccttcgatccccgctgtcaagcgtctgcgtagcaagatgcaacagcggggattcttcatgcgctcaccctgcgtacccacatgctctgcattaaattcaggcgcatgtcactgcatcgccacgctcgcgcagccgtcgctgccaccatcgccgtcgccctcgccgctccgttcatcagcccaatcaccgccaccgcgatccagcccgattcacttcccgaatccacccgcccgtacctctattttgaaagcttcgacggagtccgcaacccagcaaagttcacgcatcgcctaccggagggatggggccagaacgtcaccggcgtgacctccggcgaggcccgctggaacggctggaccctgtccgacatgcgcaactgggtgtgggcgtccggcaccgacgagcggcactacttcacccaaggccacgaccagatggccatcatcgactcgcagcagcaggctctcgcaccgcgcgattcgatgaacgcgacgctcacctccgcgccgatcgacgtcaccggcaccgggagcgtggcgctcgagttcgaccaccactaccgccagggtcgcaagggccagtcggcgaaggtcagcgtttccttcgacggcgcagagccccgcaccgtcgccaccttcaccgaaaaccgctacacccagcacgagtactacgagatcgacgtgcccaagggtgccaaggagatgcgcgtcgagttcagctacctcggcggcaacaacgactactggtgggcgattgacaacgtcgctgtgcgtgagcccttcacccagcccgccgacaagccggtcacgatcatcgacgtcatctccgacacccaggacgaccccgaggactacaagctggccatccgccacctcaacgcgatgccggacaaggcgcaggcgctcgtcattaacggcgacatcgttgataccggccgccaggagcagtgggacaagttcatgaaggctcgccgcgaggtcacccacgattccggggtggagctgtggaccatcggcaaccacgagctctacggccaggagctcgacttccaggtgaagatggaccgctacttcaagtacgccggccaggtcaccgggcagacaaagccgtggcaggagatcgtggtgaacggcacgccgctgatcggcatcagcacggagtactaccaagactccgaccgcgacggcaaggaaccgttccagcgcatctccgccgagcagctcgcgtggctcgacgagcgcctcgctctctgggacgccgagggcgtgaccgcactcgtctttactcacccgctgctgccggaaacggtctccatgtcgcactcccgcaactaccaaaacgacttcgaggacctcaccgcgctttccgacgtcctctccaagtacaacgacctcgtcctgttcaccagccactcgcacgcctcgctgcgtcagccgaactggtggggcacaaggctttacgacggcaccccgcaaggctccatcggtttccccgtgttcaacaccggcgccatcctcaacgagtacatgccgcttggcgaccacgccgagcgcatcaccgactcccgcgccgccaccggccttcgcgtgaagatctacgacgaccgcgtccgcgtcgaagcctgggacttcaagtccggccacggcctgaccaacctcaaccccggcaagccggagatgatcaagtaccaggacatctcgaagcagcgccgcctctccgacccgactccaaccccgacaccgaccgaaaccaccacggtcacccagaccgcaacacgcgaggtcccaacgacgctcacgtcgacggtcaccaccgctgtgcccacgactatcgaaaccacggttgaaaagaccctggagaccacggtcgagaagaccgtcgaaatcccgaccaccgtcgagaccaccgtggaagcgactgttaccgcaacggtgcccaccccagtccccaccacggtgacctccgttatcccgacggtcatctccacgacggttacgaacacggtgacgaccccagtcccgacgacggtgatctcggaggtatcgaccaccgtgacaactgaaatcccgactacagtgaccgagaccgccaccgagaccgtcacccagaccacgaccaggaccgaaccgcagcctgctcctgcgtcttccggttcctccaccgggggagtgatcgctctgttgctcgggcttttggccctcgtcgcaggcgcactcgtttacttcaccccgcaaatcgaacagctgctggcgacgcttcctggtttctaaacccgcacttccaaacccccatttctcgagtagattgcttcgccctcgtgcgcggtactcgagaaatgggggttacgaagtgggtgtttagaagtgcgggtttcggggtcggggtcggcttcgttgcgacgatgcggacagtcgctaaaagtaataaatgaggctcatgtgaattgagttgcaaaagtgtcttgaattaacgcgtgagtatgcggatcgtctgctgcagagtctcaacccgaagttgagagtcttcgtctggcaaggagaagaaatacatgaagcgctttaacaagaccgtcgtttcgctggcaaccgccggtgcgctcggcttcggtgttgcaccaatcgcattcgctcaggacgctcagttcggcgatctgccggtcaccgagggtgagggtgctctcgcggttgacgcgaactaccccgaaaacccggttgacaacaccccaggtactaccgtcaaccttcctgagggtgctacttgggatgagagcatcgcaccggcaccaaatgctccggccaccagcatcgatgagctgaccaaggctcagcccgaggcgcagaacacaactgctcctctcgcgaacgtagtttgcaccgacggtgacggcaaccgtgttacctacctgcgccacgctgatggcctgaactacgtgaaggacggctacgacaccactggcgcgcttccgggcgcggctggcgcataccgttcctacgctgaccttcaggcagaccagagctgcgacctcgtcgaaggtggcgacgtccagggtgccgtgaccccgggtgaggtcaccacggatccggctgacatcgccaaggcagtggcggctgtcgttggcgctggtgttggcgctgccatcatcatcaacggcgtgaagtacttcctgaacaaggacggcaagactctcgttgagaccccagagcgcgtccacatggacgcgaccccggaggagaaggcgaagtctgagcagctgatcaaggagaacgctgctgagatcaacaacgctaacaacgcccagaacgagcgtggtatcgctgccgctaccggcgtgaacaagatcccggctgcgctcatgaccctgctgctggcttccgtgcttgctgctgcggcgttcgtgttcggccgccgccagctggtctaaacaccatccgctttccccgctactgaacgcctggaagtcaggcgcagtggcgggttttgcgtttgtgcgggcgcaattccctaaaacaccagctggtcgaggaaccgctgtgcgcgctcgctcttgggagcggcgaaaaactcctcggggggcgccatctcgacgatgcggccggcgtccatgaacgccacgcggtccgcgacagcgcgggcgaaagccatctcgtgggtaaccaccagcatggtcatgccctcgcgcgccaacccaactacgacgtcgagcacttcgcgcacgatctcggggtcgagggacgctgtgatctcatctagcagcagcgctttcggttgcatcatcagcgcgcgcacgatggccacgcgctgcttctggcctcccgagagctcgcgcgggcgggcatcggctttggcggcgagcccgacgcgctcgaggagtccgagggcgcgctcctttgcctccgcctggtcggcgccctgcaccaccttcggcgcgagcaggaggttctccatgaccgtcaggtggggaaacaggtcgtaggactggaacaccatgcccacgtcggagcggacatccttcagtttggtcgaacccgctgtgacttcgcggccgttgaccatgatttgcccggaatccaccggctcgagaccgttgactgtgcgcagcagcgtggacttgccgcagccggacgggccgatgatggcaaggacttcgccggggtcgacggcgacggagacgtcgttaagcgccttgtgcccgttcgggtacgtctttgaaacgtgggacagagagatgagcgacatctaactccacctttcttccagcttgcgcgcggcgagcgagatagggaaacacacgagaaaatacagcaggaagaccaccccgtagatccacaacgcggcggaggggtagtcgaagcggttggcgtcgataatctgctgtgccaccttgagcacctcaacaacgccaatgagggcgacgagcgacgtcgtcatgatcatgcggttggtcaggttaatggtggcgggtaacaagccccgcaacgcctgcggcagcacgacgtggcggtagagcgcgcgaccttcgatgccgagcgccgcggccgaaaggtactggtgccgcggcacggattcaatcgcggcgcgcaccaagtcaccgagctcggcagtgccccacaacgtaaacacaattactgcggctacgcgggcgtcgaggttaagaccccacgcacgggttgcgtcgaagtagaccaggaacagcaacaccagctgcggcatgatgcgcacaaactgcaggtagatctgggtgacgatgtggataattttactcttgcgcgtcatcgcgacgcccatcaacgtgccgagcacgatggacagcgccattgacgataaggcgatttggatggagacgccaaggccttggaggaggcgggtgaaattgttgccgtctgcaagcacctggagatcagaaaacattcgcgcgcaccttcttctccacctggccggcgatcaatgaaatcggaagcaggataatgaggtagaacgtgaccagcagcaggagcgcctcccgggtttcatacgtctggccgatctgttctttcgcggtgaacaccagatccggcagcgcgacgatgctgaccacagacgtctctttgatcagaaagacaatgttcgcggtaatagccggcagggcgagggcggcagcttgcggggccacgacgtggcgcagcgcctgcatgcgcgacatgcccaggctgaggctcgattgcatctggatcggtgcgacgccctccagcccggcgcggatcgcctccgccatgtacgcgccgcctaggagtcctaggccaatgactgcgcaagtctcgctttcaagcaccacgccgagcttcggcagaccgaaatacagaaagaaaagctgcacaagcaggggggtgttgcggaacagttcgatgtagcccctggcaagctgggtgaggatcggtagctggaagaaccggataccggctacgacggcaccgataacaaaggccagcaaaatgccttcggcggcaaccctcacggtgaggactgccgccgctgcgtagaccgggatgttctcggcgataaccgaaaagtccatgagcgtcgtggttgaaggcttagagctggccaccctcgacgaccaagtcgtcggcggagaccgcgtcgccgtagacgggcttcaaggtcttgtcgtaggcgtcgtggaagaagttttccttgcccagctcaaccagctcgtcgttcatccagttgcgcaggtcgtcgttgcccttggcgacggcgcccgcgatggtgtcaatgtcaccgagggacgggatggtggtggagaaaccatcggtctttgccgcccaagcgagggcctcggtgttgtctgtgacccaggcgtccccgcgtccgtcgataagcgcgttcgtcgcctcggtgtactgctcgaacttggtcagcttcacctctgggtggttcttctccaggtaggcctcggccgtggtgcccttgaccacgatcacgttcttgtcggccaaatcctcgacactcgtgatcggtgcgctatccggcgtgaccgcgccgagggacaccttcatgtacgggttggcgtagtccaccttttccgcacgctccggggtcacggtgaagttggcgaggatgatgtcgaccttgttcgtgtcaaggaattccacgcgggaggctgcctcgaccggaacgtactcgacgtccacaccgaggtcttcgcccaagcggttgccgtactcgatgtcgtagccggcgaacttgccgtcggagtccacgtaaccgaacggggacttgtcggagaagaccccgatcttcactgacccggcgtcttggattgcggcgacgtcgcggaagccgtcggaggacgcaccggtgttatcggtggactctgcggagcacgcggtcagggaaaccgcggcgatcacggacgcggctgcagcggcgaggcgcggacggtgagagaagaaggacatggtgtttcgctttctgagacgggaaaacggttctaagaaccactctgttcagtcaaactacaccacttggtacagaactgggaatagtcgcgtacgcccttccccgccgcaacccctaccgcacgggctcgacggggttgccctgccagacggtcatcggcgggacggagtcgccgcgcatgaccagcgagcccgggccgatggttgagccggtgcccaacaccgcgccggggagaatgacggagttggggccgagggtggcggcggcgtcgatagtcaccgtgtcgagcgacataacgcggtcctggaagaggtgggtctgcaccacggtgccggggccgacggtggcgcctgcgcccacgcggcagaggtccgtctccgggaaccagtacgactcgacccaggcgccgcggcccaccttgacacccagggagcgcagtgccaggttcatctcgccggagccggtggcccagtcgaagaaccacggcgctgcgatcatctccacgaactgatcctgcagctcgttgagccagacgaaccaggagtacagcgggtgctcggccgggcggtggcgctgaacgagagcccacttaaacacgagcgtgatcgctagggccaccgcgccgaccgccatccacagcaggccgccgagggcataggcccacaggccgatgcggctgagcagctcggtcagaccgatcgcgaacagggcgaccagcagcgcgtgggcgatgggggcgagcaggcgcagcgtctcgacgaagccgcggcgggcgcgaaggccggcactaggggcgaaggttgcggcatcgccggcttcggcctcgacagcgacgcggcgcatgcgctccggcggggagccccaccagttggacttcgccttcgatttcttcggcgcggaggagagcactgccaccaaagaacccttggccagcttgcggccaggcgcgacaatgccggagttgcccacgaaggaacgcttgcccaccacggacttctcggcgtgaatccatccgctggagagttggtaggggccgatgagggtgtcgtcggcaaggaaggagttctcgcggacgtcggtaagcatgggcaccaccagcgctgtggaaacctctgctcccttgccgatatgcgcgccgagtgagcggaaccagactggggtaaggcggctggcgtagagggggaagaggcgggtgcgggcggcgtcgagaagcctgaccactgtccacagcccccagccgcgggcggagcgcaccgggtacgtgccgggtttgacggcgagctgcgcgaggcggacgaacacccacgtgatcgcgaggtcggcgaagaagtaggcgaggccgcctgcggcgatggcgaggatgaacggtgagccgccaacaagcaggaatagaccgatccagatgccgaaggcagcggcgatgacgggcacgccggcgatcgcgagtgccgtgagggcgtatagcgcgacccagtagcggcgcttcggcggacgtgtgtcggggaagacctgcgcggccttcgcggccttgcccactttgcgggcgggggagcccgcccagcgcgagccggccttcacagccttgtcgccggtgacggtggagccggcctcgatgtaggcgctctcgcggatttccgcgccgggcatgagcgaggagcgtgcgccgacgcgggcgtcagcgccgacgaacacctcgccgacgtgcagctcgtcgccgtcgagccagtagccggagaggtcgacgccgggttcgatggaggcgccctcgccgatggtgacgaggcctgtgaccggcggcaacgactggtagtccacgtccttgcccacgtggttgccaagcatgcgggcgataattttgacaaacggcgcggccgagatgttgagtgcgccagaggcggccagccacttctcggcggcccacagccgcaggtgtgtcgcgctgccgcgcttgtacacgccaggttgcaagcgaccgcggatgagccgcgcgccccaggcgccgatgggcacgcgaccgatcggggtgcagaggatgagccacaacagcagcagaccccaccagggtgccgcgggggtgagcaggctgagcgcgatcaaggcccaggtaatcgcgctggcggcgcgcagggtcatgatggggatgagtaggagtgtttgcgctgcgcgggtgcccgcccctacgggttggacggtgcgttcgcgggtggtgggggaggagatgaggtgggcgtcgattagcgaagcaagcgcccctaagcgcggatgatcgtagaggtcgcgcaccgcgaacgtggggacgcgctcgcgcaggcgggtgaccagggcggctgcggcgagcgaggtcccgccgagcgagaagaagtccgcgtccgcgccggagacgtcgacgccgagcacctcaacccacagccccgccacccactgctccgtctcggtgaggccgaccgcggcgacctccgccggcagcggccacggcagcgccttcttgtccaccttgccggaggttcgcaccggcagctcgtccatcacgtgcaggcgcggcacgagcgcggccggcatcacctcggcgagctcggcgcgcatctccgcgatgtccagcgtcgcgcccgcctgcggggagacgtagccgaccagcaccttgtcgctgcttggcagcgtctgcacggccacggcggagttgtacacgccgtcgagcgccgccacactcgcctcgacctcgccgagttcgatgcgccgcccgccgatcttgacctggtcgtcggcgcgcccgatgaacgccaggccctggtcggttacgcgcacgtggtcgccggtgcggtacgcgcgcgcccactcgccccacggggcgtacttctccgcgtccttcgcgggatcgaggtagcgggccagtcccacgccgccgatgatcagctcgccgtcctcggcgaccgcaaggtcccagccgtcaagcgcccagccgatggtgacgggcttgcctggttcaagcttggcggcggaggcgaccaccgtcgcctcggtcggcccgtacgtattccacatctcgcggccgtttgaaagtctgtccgccagctcttgcgaacacgcctcgccgcccacgatgagcaggcgcacgttatccagcgcctcggctggccagagaccggcgagcgttggcacggtggaaacgacggtgatatcgcggcggatcagccacgggcccaggtcctggccggagcgcaccagcgagcgaggcgctggcacgaggcaggcgccgtggcgccacgcgagccacatctcctcgcagctggcgtcgaacgcgaccgagaggccggcgaggacgcggtcgtcaggcccgagcggctcgtcctggcagaacaggcgcgcctcggcgtccacgaacgcggccgccgagcggtgcgtcacggccacgcccttcggcgtgcccgttgacccggaggtgaagatgatccagcagtcgctgtctaggtcgggtcctttgaggtcgctcgtttgcggtcgttcggccacgatgtcgaggccgtcgtcactgaacagcgcgtcgattgtggcctcgccgaacaccagctcggcgcgctcatcggggtcgtcggcgtccaccgggacgtaggcggcgccggcaaacagcgtggccaggatggccaggtataggtccttcgaccccgaggtcatgcgcacgccgacgcgcgagccgcgcccgatgccggcgctgtttaactcggcggcgagctcctcgacgtttgcgacgagttcggcgtaggtgaggatctcggagccgtcgtcaatcgctgctgcatcggggtgcgcgtcggcgctggcgcggacgatgtccaccagcgtgcgcggcggcggcgcgaggtggccgcggttgagcccgttgagattttgcatgcggacaaggctaattgtgctcgccgtttctgtaaaatggtgggaactctccacgatttgtgtcgccccactgtttgtggggtggtcgcggagttgtaggtctagagttgtagttctccgccaaatcgcaagtggggctgttgttatatacaagtagacctacaactccggagtctgggcaacggcgcgtggggcccggcgtaacatcgcagccatgactggcgacacctacgttccgcgcaggccccccgaactgccgcggtcgagccgctacgacgcgcagcaaaggcgccgcccgaaccagccgggccatgcaaaccgcccaagccagccgcgccgcccgcgtaagccgcagtgggtgtactgggtgcgccgtgccggggcgctgatcatcctcttcctgctgctcacgggtattttccgcgcgtgcagcgggcccgccgagcctgaaacgacgccggtagagaccacgcagccgaccacgaccaccgaagcaaccaccgagcagtccacaccgccgcccacgcacatcgaggcggccaggcctgtggagatggtcattcccgccgtgggcatgagcgcgaagttcgacgacggcgactgccgggtggcggacggcaagattgaccccgccgggctgtcgaaggcctgcgtgtacaccgcggaggacaagccctacgagctgccgggcactgatgcgggcgacattgtggtgatcgcggggcacgcggcggcgggcgtgccggcggtgtttgacaagctgtacaaaccctcggaggacgcgcacacgctcaagctcggcgacaccctcttcatccgcaccgccacctccggcgagtggtggctcaagtacgtggtcaccgatctccacgagccgatgaaggatgcgcttgccggcgacaccgccatctggggcaccggcgccaccccgggccggctgctcaccatctcgtgcgtgcagccggcgaacccgttcgaggactcggtgcgcaacgccgtgatcggctggcagtttgagggcgtcaccgccgaagctgcctagtagaaaaggactagctttcctcttccaggatcgcgcgcgagagcttcttcaggctcttcagctgcttgttcgtggacatgtctagcgcgcggtcctcggcgtcggcgacgtctttcgccagcgcgctgtgcaacttcgcgcccttcttcgtcggggtgatgatctggcggcggcggtccttggggtcgcgatcgcgcttgacccagtcgtggctctccaacgaatcgacgaggcgcaccatatcggaggcgtcgataatcagcacttcagacagttggcgttgggagagcggctgctccataacgcagctcaaaatccagtactcgcgcatgctggagccgtgtttccccagaactcgctccacctcgtccttggtatggcggcgtacgcgctcaatctggaacgagggtgactgcgtcagcgtgctgggcaactctaccgtctgggacatgcaataaagcgtaggcggaattggcgggcaacggaaactatttgcacagtcaattaatgatgtttggggagtatttactccgtcggcaagcctgcttcaatccatgccgacgtgccgcccgcgacgttgatgacgttgtcccacccgcgcgactgctcgaggtactccgccgcctgcgcggagcggccgccggagtggcagatgaggtagatgtcgcggtccgggtcgatctcgccgacgcgcgcgatgaactcgctcaaggggaggtttgcggcgccggtggcgtgggtgtgggtgtactcgtggggctcgcggacgtcaataagctgtgcgcccgcggggacgtcggtgacgttgacttctttcatgggagccaagtgtacggcgcgggggcagatgcttatcgacgccacgtgtgaccaaaatcacccactagcctggaggtctccgatgggagccccgcaccttaaaaacgtcgtataacggcagcttaaaggcgggaccgttgttgaaaatttgatcacctgcttaaaaaatcagctgctcgctcacgtacagcttcctgtcaattgttgtcagaaaattttacggctagtgttttagctatccgccggagattgggctccaacccccagagtctgggcggtgtcgggaagcccccggcgacaccgtgcgcctgaacagtgaggactgtgatggtggatagcggtatccgaatttcaatcgactgcaggctgtcggcctgcaccaacccgaagggttcacacgtgaaaaaccactctgttgcagtgcgctccgtgacgatcgccgctgctgctgcactttccattggcgtgtccgcgccgatcatgcctgcgaacgcgcaggccggtgttgttcgcaccgatggcaacgtccgtgtgtcggactccaccatcgacaccagtgccaccggtacgctgaccatcttcaagcgcgctaacccggagaacactcacacggctaccggtgaggttgacagcactgctgaaggcactgcgcttgagggcgcagggttcaccctgtaccgcgtgaccaacgcggacctaaccaccaacgatggtctcgctgccgcagcaaaccttactgtcgcagaagcccagtatgacaaaaacgctccagtcggtggggctgagaagaccaccggtcctaatggtcaggcgaagtgggacgacctccccgttggcgtctacctcctgaaggagaccacgaccccggagggctactccccggcagctgactccctggtcttcgtgccgatgacccgccagaacgccaccaacggcggtacccagtggctctacgacatcactgcgtacccgaagaacacttctcagcaggaaccgcagaagaccgttaccgactccggtcagaacgtcggtgacaccgtcacctacaacatcgacacctacgcacagaccgttcgcgaaggtcagttccgcaccttctaccgcgttgaagatacccttgacccggcgctgcgcctggtcgaaaacaacccggttatcgtgacttcgaacccggaccgcgcgttcgaggaaggcaccgattacaacatccgtactgcctgggttaacgcacagggtgaggaagttgaagcgggtaccgagggcgcgcgtcagcgcgttcgcgtgaacttcaccaacactgaaggcaacggcgttaacaagatccagaacggcgaccagatctccgtccagatcaacgccgaggtgaactcgaagccgggcgagggcgacctgttcaaccaggctacccagtaccagaacaaccctaatgacagccaggcgtatgagcctgacaccgacacgcctccggaagagggcactccgaccaacgaggtccacaccttctacggtgacctcgagttcacgaaggtgaactctggtcacgagggtcttgagggtgcagagttcaaggtcttcggtgtcaagggcagccagacctgtgatgctctcgactggaagaacccgggcgataacgcagcagagcaaaccgcctccggtaatgacacctggacctccgatgctgacggcaaggtgaccatcaccggcctgcacgcgaacaacatcgcaaacttcaacttggccaaggacgaagacggcaacgtcacggcaaccgagaccccgaacgagtggaccagctactgcctcgtggagaccgagtctccggcgggttacgagctcctcgctaagccggttgcgttcacgatcaccgctgcgaacaacgacggcgtctggtctgtgacgaacggcagcgtgaaggtcggcaacaccgacaacgagatcgtcaacctcgaggactccaccccgaagctgccgcttaccggtggcacgggtatcggcatcctcgcagcgcttggtgctctgatcatcgcggctggtgcgtactccgcaaagcgtcgctccgcgtaagcgaagcgcgtaaaccccacatcccgtagaacccaggacgcgtgagtgcctgggtgggcgggtgtgggttcaagggggcgtcgtcaagcacaatgccccctcagcaaggaggaacggggagacctcttgctttgcactaccgccttcgggcgggatctcccccaagttttctttggataggtggtgaccatgacggttgttgagcagccgaagaagcagtctgctctgctgccggtcatcatcatcctgttcggcgtgctggtgctggtgtacccggttgtagcgacgcagtggaacaacatccagcagcaccgcgtggccgacgagtacgcgaagatgcagcagagcgaacccgaagatgtgctgcggaaggtgtacgactcggcgctggtgtacaaccagacccacactaagggcccgattctggacccgtggctgacgcgcatcggcaccgacaacccggagtacggccgttacacggccgagctgagcaatttcccggtgatggcgcgcctcatcgtgccgaccggcgatattgatctgcccgtctaccacggcacatccgacgaggtgctgcagaagggcgtcggccacctcttcggtacggaccttcccgtcggcggcgagggtacccacgcggtgctgaccggccacacgggcctgaccacggcgacgctattcgaccacctcaaggacgtcgaggtcggcgacggcatctacgtgcaggtcgccggcgagaagctgaagtacgaagtcgacgagatccaggtggtcgagccggacgacacggaaagcctgagggcgcgcgcgggggaggacctgctcacgctggtcacctgcaccccgtacggcatcaactcgcaccgcctgcttgtgcactcgcaccgcgtgccgatggacgcggagacgacagtcttcgagaagtctgcgacccagacccagtggtggatgtgggcgatcatcggtgccgcagcactcattctcgccctgctggcgctgtggctgctacgacgccgcaagcagcgcgagcaggaagtaacaaacgatcaggagcggaagttttggcctcacgaacagtaacgatggcgcttgccggcgcaatcgccgtcggcgcgtgcgcagctcccgcttacgctgatacgcgccctgtggtcggcgcttgccgcgagatcacggacgcatcgctcatgcgcgacaccggcgagccgctccggcttaccgtgcgcaaaacccaagccaacccgtacgacgaaggttcgctcccgcccgggtccgtcgaggggatcgagttcaagctctttgaggttcaggggcttagcttgacgacgccctccggcctctcccaagcccaaaaactcacgctcgacgacgcacgcgacctcggcctcacccaggttgcgtctggccgcacgggatccgacggcacgatcacgttcgccggtctgaagcccgcgatgtacgtggtggaggaggtcgctcctgacgacgacacccacgactaccgcacgtcggacccgttcctgattctcttgccgacgttcgacgccgactgcgaaaccacccactccgacaccgtcaccgtggtgaagagccgcgcgaagacaccgcccacggtcactaccgtcagcaccacgccgccgaacgtcccgccgccgtcatggccgaactggccgccggaaacgtcgacagtgacaacgacgccaccgacgactcccgtcaccaccaccgtgactggcgggccgccggttaccaccacggtgccgggcgggcctggaacgccggggtcgcctggttcacctgggaacccgtcgaaaccgggccggccggatggcccgctcgcgtacaccggcgccaacgtgatctgggcgctgttcgtcgccttggcattgatcatcggcggcgtgctcttagtccgtcgctcccgcgataacgagtccagcaaacaaccgaagcaaagttagtgagtgagaggttctagatgatgtttagcaacaccgacagccgcgaagcggtgagcggagttgacgcagccgtcagctctcccactcgcgcagcagttcaccgcgccgtcgcggttgtttccgccatcttcatgtcggtcgcgctgatcgctgggttgtccgtatctggggtggctgtttctcgggctgaggcgcaggagtgcactacggagacttcggtgaagacattgaaggtggattcctcgatccagtacggaagctcggctgcgagacggctcgctatctctggattgacgcctggggaaacggttactgagttggagttcagtaacaccaagaactcatttggtaagtccgcgagctactccagcatcttccgcaactctgcgggagaactggttccttttaaaaacaacaactacggtgacgagcttggggtcccgtttgccgacatttcgggactaggcagcaagacgctgacctacaggctgccggcgagtacgactgctggtcctgcgggaacgtttaccgccgtcgtgccgatcagcgacaataacgcggcgaacttctccgtacgagcgaccgtcgagcgcacgacgtgtactacccctgaaccggaacctacctccgaagccccgtcgccggagccgacatctgaagccccgtcgccggagccgacatctgaagccccgtcgccggaaccgaccccggacacttccgagcccacaactaagccgaccagcgagcagccttccacggagccgacgtcaacggcaccttcgagctcggagcagccttcttcccccacgcccacagaaacgaagtgtgtcgtgggcaatatcccaacgagcggcggcaggacaaacggagcgaccgaccccgtcgcgagcggcgggttaaaccagcaactcgatttctctttcggcagctttaacggcacccgctacctggagaagttgacgataggctccccatcgaagttcggctcacagccatttgggccgagtggcttgaactggcggttcgttcacgatggcaagacctacgtcgcgggcaccgactttatagtgagcccggccaacggcaatgccacatcggtatccctagttttcaccactcccgtgcctttgcgtgcaaactcctctgcgcgggtgtacctgcccgtaaccggaccaaacggtgcggcgccggtagtcgctaccgcatctaactgtgagccggagaatctgccggaggatccgccgacggagaatccccagccgacggacccagacgagccgggtgacccagagatgcctgccgagccggaagaggcgaccgaacggcgtgatccagcagttggagaacagcgactcaccgtgtctgcacgagcgttcgtcccaatgttcaccgcggggagcttcgatgaccacaacgcccgaactagtaccgacacccggtatacggccggcatccggttcgagctatggaacacgagcaacgatatcgccgtagctctcagggacgggcccagtagcaaggttgatgagccgtgggcctattgcgtcactgattcaacgggtgaatgcgacattttcgtaccggatagctatttgggcgcgggcaagcggttttacgtgaagcaagtctccaatgcacccggaaccttccacatcgacaaggtcaactggggtagatacggcgcggcaaacgaccgtttcgaggcatacctgccaggaccggttgactcccacccgacccactccagccggggtgttgtcaagcccggtggaaagaacgtccaagaacgctcttacgagattccgccttcgaagcgttacgacggaccggacgtgaaatctatcaactctaaccgcgaccgcgatgcgtcgcagtggagctcgtttggttccgcagcacagtctctcaacaacccgcccctttctcaggcgcgtaagtgtcaggcaagtggtggccctaaaattgccttggtgatggacgtaaccgcgtccatcgacgagaatggtagcccgcaaaagtatcgcgacgcggtttacggaacgtacgggttcttgcagtcgcttcgcggaacgggtgcggagatcgctatgttcaacttcaacgagtcttcgcctggacgggatcagaactacccggagcccctctccgtcgatacgaacatgacgaagctggaagggcaggcaaagagtattctgcggagcttcagtagtggcacaaactgggatagcggtcttaatgcggtgaagtctgcaattgagagtggccagaagtatgacgaggttattttcattacggatggcgacgccaacgggtacggcaagaacggcagcggagacttcaacgacggacgttcaggctacgtgcgggcaatcgaagcagcgatttaccgaagcaacgagattaaggagaagggcacacgcgtcgtttccattggtgttggctcggcagaggacgcctccaactgggacggctcaggccagctggaagccatctccggtctgaagtacggcgaggactacttcggcacagattgggaccgccttgcctccaccctccgcgccgcagcgagccaggtaacgtgccagaacgagatcgtggtggataagaccatcgtcgacgagaatgggcgcaagttgcccgaccagtcgcaagcaacgaaatggaatgtcgacatcaatgtggacaatgtcgtttccgagatcaactggtcccacggtgacgatccggtgcagccggccgtgttgtctccgaacgcttcgacatccgacgattcattgaacccgctaaagattcatgatcgccgggcgacaccggactcgcgttggttcctcaccttctacggcaacgcagagccaggttctaaaaaggcaaaccgtgccgatatctcgatttccgaagacacgaatagtcgcgcgggctatatctttgttccgggcacggggcaaaagagcaccggcggctactccggacggggatcttggtacgagatccggaatctccgctacgatacggtgctcgaaacggggccgatgacgagcccgaatatgaagttcccggagctacctcaggaccggaagctgatagtgcacctacagaaccagccatcagtggcggtgcataaaggcactgcgcagagcgtggtgagcgtgaacgctgacaacacgtggaccgcgcgctacgaagtccgcgcaaacggcacttctgattcgaaaacgcggatcccgcgcatcactgacgaaccgggttttcctgacgggttcgaaattacgaaggttgccgttgatggagagccgcgtcagctgaaagacgggaagtttgaggttgccgctgaaggcagccgcagcctgagcaaaaacgacattgccagctacacggtggtggtggagggtgtttatacccgcaaaaacgctcaaggcacgctcgtacctctcgagacgctgggagacgagctgaaatgcgaagctgacggctctgacggcccggggaaggggatgttcaacgaagtctttatgacaccggatgtcgatgggcaagcgaataaccgggcatgtattccgattgtgccgaacccgccgaagaagccgtcggtggagaagacattcgtcgacgtcacgccggtttctacgtccacggcgggtgagcagcttgtcaccttccgcatcaatgtgaagggggatccgtcctcggaccttaacttcgacctgacagaccgcacagcattcgcacccggtattgagattcaggaggtgcgggcgcgcttcctgggtggatcttcaagcgggaacccagggttgggcaggagctttactactctgaccaaacaaaccgacagtcagggtacgtactggaaggtcgccagcggcactgtgccaaagcagggtgtattcgagtatgagattcagttccgcgtcaaaggtttagacaaggtacagcccgaagaccggaagtgcgagagcaccggaaacaacgacttccgccggtggacgccacaggaggggttctacaaccaggcaaccctcggctgggggacaacttcgaaccgccaaacccaggatgtagacgcgtgcggcgacatcgatgtccagccgaagctgagcgtggaaaagtcggtcgcgcagcacccgcagacggttaccactgcggacgggaagcttcacgacgaccgctcgacaggtctgcagtaccgcattgttgtgtccaacaccggcaccgggccaggcacgtacacacttcgagacatgccgctctttgccaacggggttgaactactgagcgaccaccatggaattgtttcagccgaagtggtgaacgcctccacgggaaacaagacggaccttaaacttcccgggtataccgtctacgtcgacgggaataggaaactcgttgggttcggattcgcgagggacctcgaaatcgccccgaacacctcgcacgtgtacatcgtgcaggtcgcgtacggcgagaagaccgacttctttagcaacgagaatcagcgggacagcgtctgtgcgtcaacacccggcgatgaccgaaaggggctgaataacaaggcgcagctggtgtccgtgaagaacccggccgccggcaatgcagaggtacccggtgatcccggcgagtacgttgattatgcgtgcgcgaacatcccgccggagccctccatcagcaaggagatcaccaacgaaaagctgacgttggacgacaccgtctcatacaacgtcaccgtgaggaacccagatggcggtgtcgcccggcgtatcgacgtgaccgacataccgaagtttggaaagaacatcacggttgatccgaagtcggtcaaggtggacggtcgttcaatcgaatatgaagccggcaaagagcttgcccttgggacggtggagcttaaaccgggcgagagcaagacgttcgttgtaagcgcgaagtacacagcaaaatccggtgagttcaatcctgaggcaatctgctccaccagcgactacggtttgaacaacaccggcaagatttacttcgcgtacttcccggaccgctccgcaggaaaacgcccgcgtctttcggactccgacgacgcctgtggcctcgtgcggacggatctcaaaattggagtgcagaagttcggtgcggacaaggccggaaacgtagaagagattgacccgacaacgggtgggtaccagttcgaactacgcgaaaccggtccggacgctgcagcgccacgggttctggatgccgtggcggagactcagaccgggacccaattcaacaccgttgatgccccgctaaaagctaacaccgagtatgagttggtagagaccaaggcacccgctggttactcgctgttggccgaacccgttaagttccgagttgtcgccaccgcggatggcgtccaagtgcagttctatgacagcgtcagccagaagtgggcaaacaagctggtgaatgtatctgcatcttcaacgggggagaacgccgggttgcagttgatatcggtgacagacgttcactccgggacgctcccgcgtacaggtggcaacggcctgtggcccatcacgttgctcggtctaagcatcgtcggcctgggcgccgcggttggtgcacgtaggaagtccgcctaagatgcgtaagcgatggcgacagtaaggacggagcgggtggggaggaagggtgcgtcgaaaagcaacctcatgcccgtcctcctcatcctcctaggcctcgcggtgctgctgtacccggtggtggcgacgcagtggaacaactaccagcagacgaaggtcgcggaggattaccgcgccttgatggatgaagcggtggagaaggacccggacgccatgcagcaggcgctggacgccgctcgcgagtacaaccgcgcgggcaggggcgggccgatccttgacccgtggcagtcgcgcgacgcgacgggcaatgaggagtaccaggcgtacctgcgcgagctctcgggtctgccggcgatggcacagattgtcattccgtccatcaaggtgaacctgccggtgatgcacggtacgagcgacgaggtgttgaacaaggctgttggccacctgtttggtacgtcgctgcctgttggcggaccggatacgcacgcggtgctgactggccacactggtctgacgaacgccacgctcttcgacaacctgatcgacgtggaggaaggcgacgcgatctacctcgcggtcttcggcgagaagctgaagtacgaggtctacgacatccaggtggtgctgccggaggagacggacagtctgaagacggtgccgggggaggatctgctcactctggtcacgtgtacgccgtacggcatcaacacccaccgcctcttggtgcacgcgcaccgggttccgatggatccggaggaggcgtcggtgtttgatgaggccggcagtccggtgcagtggtggatgtgggcgatcgtcggcgtcgcgctgctagttgtactgctgcttgcgtggtggctgctgcggcagaagaagaagcgtaaggaagaagaaccggagccggtcaggcattggcccggggaaattccgggcgctggttcgaactaacgtgccgccaagcactggttgaccagcgcattcagcgagatcccctcggctgctgctcggataaccagttcacggtgcagtgatggggaagtgcggacgttgaactttcccgagtaacgccgctcgcccaatggctccgggatcgtctcattgttggacgtcatatcctcaacgatctcggaaagaaggtctgtcagacctgcctcggcctcggttcgggttggagcgagccaggaaacggacggaaactcgagaacagttgcaacgaactcttcatcctcttcagaccaaaaggtctggaatgtgtatcggtcaatcttagtgctcatttactgctcctctcgctccaaccggtcgatagcttttaacacctgccgcacttggtaagccttggccattccgttcgcgttctgaatgttcactcgaggatcccctgtccaaggggtcttatacgaacggtgtgacgagcctgagtggggacggggctcaaagaagaaatcgcaaaccttctgcaggtcggcatatctcacgtttgcgggagagcgcctcatttgcgccacgatcttcgcgaggttatctcccacaacgaagatagtaccgtatgcagtactaggtgaaaagtttacccgcagcccctccgatccgtcagcaagtcaccatgatgatgaagaagaaaaggaggtcgacgatgacaaccaagatgaccgctgaagaacggcgcagggagtgggccaagctcgcggttcgcgcgagtgagttgactggagaccggttgccacccgagatctacgaacgagcgcgcggagacgcagagcgccccgctagcggtcccaagacaagaaaccgttaagcggggcgcaacaggccaaagactagttctccgtcttcgcttccttctcggcctcgaggttctcgcgggagttctgctcaccagcggcctcgaacgcgtcgagcgatgccttaaggatcttctcggcctcctcgcggccgccccaaccggagccggtgacttccttgttcggctcgaggtccttgtagtgcacaaagaagtgctcgatttcgtccttgacaaagtcggagacgtcgtcaatgtcctggtaggactcgtagcgcacgtcgtcgatcacgcaaagcagcttgtcatcgccgccggcctcgtcggtcatcttgaacacgccgatcgggcgcgcgatcacggtcacgcccgggaacaccggctcgggggtgatgacgagtgcgtcgagtggatcgccatcgtcggcaagcgtgttgtcaatgaagccgtagtcggctgggtacgccatcggggtgaacaggtagcggtcgaggaaaaccttgccggtttcgtggtcgacctcgtacttgttgcgcgaacccttcgggatttcgatgatgacctcgatagccatgatgctcctttgcttgtgcggatgagactggcactcatcctagtccgggcggatcttcgggttcgatccggagcacatcggcgacaacatgttcacgcaggtgctcgcgcaagaaggggaggacgaaatcggcggtgcctcggtcggttgttacaaggtcagcctcgtagagacgggcgcgatagttgtaggcctgctggtcgctcacgccgagacgcttggctacgtccgtgatcttggaaggcccgtcatccagtgacattgcggcaaggaaccgccggtcctcactggagagatcgcttagcgcgggttcatgcaccagttgacccaatttcttcctcgccttagccaccccctcctgggctgcatcaagcgatatcacctcgtcgttagcaaacctccaggcaaagttgccgatgagctggatcatgaacggataaccgccggatgcttccacggcataccggagcgcccgctcgtcccacgttctgcccgcttccaccgcgggaacctcgaggccgtcgcgcacttttgaggcgggaatggcgccgaggtcaatcctgttcgcccttctgaggaacgtaatcgggtttctgccgtcctggctcgccaacaacggtcggatagacgttgggattcccgcgagaacaaccgcaatctcgcggttctcgcgcacgagatgctggaccgtcgtggcgaactctgtgatctcgtgttggtgcacgtagtggagctcatcaattgtgataagaatgcccgttggttgaccgttaaatttatcgcgctcagcaaccacgtccaaagcttgtccgaggaggcttcggaggctgtctccggtggaaccagagtcttgactttcccgcttgtagcggaggaagctgggtcccacgtgcagactgcgtttggctttcgacaactcagcgtcgagaaactgaaccacctgctgcttgaggctttccacgaacccttccgtggcggtttcggaaaatgccagccaaccttgccgggtagccgtgtcctccaattcgttaaggagcaccgttttaccaacaccgcgagcgccaacgaggagggatattcgctcatgcgcaccggggccttctcgtagggccaatgcaaaatcttcgatgacctcgtcccggcccacaagtaacggcgggctcgatcccaaagatgcgcggaacgggttattcggcgtggtcatgcggttattgtacccagttgtgtgttcttatgtggtttgtgtggagttgtgtataaacaggccggaaccgatgtgttcttgtgtggtttgtgtggagttgtgtactacgatctagcccgatgaaggtctggtcttgggtcgtgtccgccgccgcgctggcggctgtcggtggggtagcgggcttcggcgtcgcggcgcacgagcagctctccgcgctcgagcacgcccccgcctacgccatgccggagcccgcgcccatgctggcaccagctacaggagctccagtagacagagcattgcttatcgacgccctgtccaacgcctccaccaaccccgccctagcagacttccacgcccacatcaccgacgccaccaccggcgacgtgatctttacccagctcgcggacgtgcccttgcgacccgcctccaccacgaaggtgctcaccgccgccgcggcgctgtatgagctcggcgccgccgacacgctcaccaccaccgcctaccgcgtcggcgacgatgtctatgtgaaggcctccggcgacgtgtggatggacgcggacgcgctggacgagctcgccgccgcgatccccggcgcgcaggccgtctacgtcgatacctctatctgggacggcatgccggagatgatgcccggctggaacgaggccgacatcgacggcggattcgtagcacccctgcagccggcgatgctcaacggcggccgcggcttggaggaagcaaccggcgacgtgccccgctcccacaccccggccctcgacgtggcccaggctttggctgatcgggtgggcgccgcccacgtcgacttcgccgccgttcccgagggcgccgagcaggtggccgaggtttcgtcgccagacctcattacgcgccttgacgtaatgatgaagaactccgacaacgtctacgccgaggccatcgcccgcgaggtgcgcctcgccaccggctcggacccgctgaccgtcgtggcgaaccacggcttcgacaccaccggctgcgtcgtcgaggacggctccggcctgtccacgctcaacctcatcaccccggcgctgctggacgcgattcttgccgacgccgccaccaaccccaccctccgcccccttctcaccaccctgcccgtggccgccggcgacggtaccttgatccaccgctacggcgatctcccaggccgcggctgggtccgcgcgaagaccggcacactcgacgacacctccggtctcgccggcaccgtgaccagcgtgggcggcaacgtctacacgttcgccttcctatccaacggttccaacatcctcgacgcccgccgcgccatggacgagatggcctccatcctccgcgagtactagcgcatggaccccttctggccgcgccgctcgccccacttcctcgcgtgccgccgggcggtgcgccccttcgccggatccggtcccgtggtcatcggtctttccggcggccccgactcgctcgcgctggtcgccgccgcagccgccgagggtatcgacgcgaccgccgtggttgtcgatcacggtctgcaggagggatcggcggacgtcgcaaagcatgcttccgaacaggcaacccgcttcggtatccctgccaccgttgtacctgtgaccgtcgccgactctcccgacggcgtcgaggccgccgcccgcgaggcgcgttacgcagccctcttcgccgctgcgcccgccgatgtctgggtcgcccacaccgccgacgaccaggccgaaacgctcctcctcggcgcgctgcgcggcaaccccgccggcatggcgccacgcgacggacgcctcgtgcgccccttcctcaccatccgccgcgccgacaccgtgggtgcctgcactgagctcggcatcgagccgtggcacgacccgatgaataaagacactgcttatcgacgccccgccatccgcacctccatcatccctcaactcagcgagctcatcggcggcgatgccgtcccagcgcttgccgccgccgccgaccgcatcgccgccgacaaccaactcatcgcctctctcgtcgacctcacccccacctcctcgtgcgctgagctgctggcggagccgggggcggtgaggcggcgtcgattagcagcatggcttgtggaaaacgatgtgcccgtccagcgcgaccaacttgccgccatcgaatccttaatcaccgactggcacggccagggtcccatcaacgtcgccggtggggcggtggcgcgccgggctggcgtgctggtgatggaaccgtcgggcgtttcggcgcgtctaaatggccatgggaatgacgacgcaacgccagcaggagatccgcaaccacatcgttgatttgcggcgactctcgcacgcgcaggctaccgaactgagtggcgggtacacccggctcgatccgtcgattgtgtacccgacagatatgctgaaaacgcttgcctaccacgaacgcaggtggctcgaggtcgaagcggccgcgatgaccagtcgcggtgccgtcctcgtctcccgctcagcggcgcggaagctgggtatgtgggtgatcgcgctcgatagcgagctggtcgaactcgccctgcgctcccgggcgaaatgcccgtctcggggcagtcgccgcaacatcgtctaccggcgcagccagttgttggacagcgagattgaggaaatcgacggacacccaaccaccacgccgtttcgcacgtttgccgacatcgcccgctaccactcgttcgccgaggggcttatcgccgccgactacctccgccgcaacgggtatacgcttgagcagctccggggggaaacgatccgcctcggccggttgaaggggatcgcaaccgttcgcgagtgcgtcgcccacagtgtggacaactccgactccgcgtacgagtcattcgcgcgggctttgcttattcaggccggcattggtcccatcaccacccagtacgagattaacggctacttcgccgacatccttatcggcaactggctcatcatcgagatcgacggcaacgtcaaatacgaaggccccgacgccgaagccgttcgtcaacgcgagttcaacagacagaagcgcattggcaacatgggctacgtctttctccgcttctccccggacttcatccgtaaccacccggacgagttcatcgcgcaggttcgccaagcgatcgccgcccgcgcggcaatgttggcgaaatagtcgtggccgcggtttcgtcgcgccgcgccgaccgcgccggccaaatggtaacccccacctggtaactaccaaaaggtcattaaccgccgtcggcaaagatcatctctttcccgcgactcggttaatgaccatgtgccagcaacactttggaagcaacactctgcaagcaacgctttgcgccgtccccgcagccaccgccgcagcagccgccgcacccaccccaaccccgtcaccgcgtcgtttgttgataccccagcgattgaggtggcaatatgagagttcacccgcgtacgagggtttgccaaaccgagggaagggctttccatgactcagctgcaggacaccaaggacttcaacgtcccggccaaccgctacggcgacgacgttgaggcgatcctcattccggaggatgtgctgcaggcccgcatccaggagctggcggacatgatctccgagaaatacaaggacgcggaagacgacctcatcttggtctgcgtgttgaagggcgccgtcttcttcctcacggacttcgcgcgcaagttgtccatcccggcggagatggagttcatggcggtctccagctacggcaactcgaccaccagctcgggcgtggtgcgcatccttaaggatctggacaaagagatccaggggcgcgacgtgctcgtggtcgaggacattatcgactccggcctcaccttgtcctggctgctgcgcaacttgaagggccgcgggccaaagagcctcgaggtgatcacgctgttgcgcaagccggaggtgcagaccgccaagatcgacctgctcgatgttggctttgacatcccgaacgagttcgtgattggctacggcctcgattacgcggagcggtaccgcgatctgccgtacgtgggcacgctgcacccgaaggtgtacacggagcagacgcaggaaccagtcaccgagactgaaatctaggattaatgagcaaaaatcaaaatgtgatgcggtggggcctgatcggcgccaccgtcttaatcgtcctctacctgtttaccctgatcggggacgattcccgcgccttccaagacgtggacacctcagttgcgctggagcaactccaagaccgcaacgccgagacggtgcaaatcgacgaccgcgagcagcgcatcaggattgagctgcgggagccgattactgtcgacgagcgcgagaacattgaggcggtttcggcgcagtatccggcgcggacgtcgccaagcatctttgaagcagtgcaggactctggtgccgactcgttcgaaacgaacgtgacgcaggagtcgttcctgatgtcggtgctcggcttcatgctgccgatggtcctgatcttcggcctgctgacgtacttcatgtaccgcatgcaggctggcggcggcatgttcggcatcggcgcctcgaaggcgaagcagctgaacaaggacaatccgaccaacaccttcgcggacgtcgctggcgcggacgaggctgtcgacgagctgcaggaggtcgtggacttccttactgatccgtcgatctacgaaaagctcggcgccaagatcccgcgcggcgttctgctgtacggccctcccggcacaggtaagaccctgctcgcacgagccgtagcgggcgaggcgggcgtgccgttctactccatctccggctcggacttcgtggagatgttcgtcggtgtcggcgcctcccgcgtgcgcgacctgttcaagcaggcccgcgagaacgcgccgtgcatcatcttcgtcgacgagatcgacgccgttggccgccagcgcggctcaggcatgggcggcggccacgacgagcgcgagcagacgctgaaccaactgctggtggagatggacggcttcgacggtcgcgagggcgtcatcctgatcgccgcgacgaaccgcccggacatcttggacccggcgctgctgcgcccgggccgctttgaccgccagatcccggtgaccaacccggacctcgccggtcgcgccaagatcctgaaggtgcacgccaagggcaagccgctgtcgaaggatgtggacctcgacgcgctggcgaagcgcaccgccggcatgtccggcgcggacctggccaacgtgctcaacgaggcggcgctgctcaccgcccgcatcggcggcaacgtgatcaccccggacgcgctggaggaggcgaccgaccgcgttatcggcggcccccgccgcagcaccaaggtcatctccgagaaggagaagaaggtcaccgcgtaccacgagggcgggcacacgctcgccgcatgggcgctcaaagacatcgagcgcgtgtacaaggtgaccatcctccagcgcggcaacacgggcggcttcgccatgaccgccgacgaggacgacaagggcatgtacacccgcgacgagttgttcgcgcgcatggtcttcgccatgggcgggcgcagcgcggaggagctcgtcttcggcgagccgaccaccggcgcgtccaacgacatcgagcaggccaccaagatcgctcgcgcaatggtcaccgagtacggcatgtccagtgtgctcggcgcggtgaaatacggcgagcagcaaggcgacccgttctctggccgcggcgccggcggcacgctcgagtactccccggcggtggctgagacgatcgaccgcgagatgcatgagcttctcgacgcagcccaccaaaccgcctacgccatcctgtcgcgctaccgcgacgagttggatctgctggtcaccaaactgctggagaaggagacgctccgccgccccgatctggaggagatcttcgacacgatcaccccggagcgtccggagcttccgcttcacgacgcccgcttcacccgccaggccgaccgcgaacctgtcaagacccccgtggagcttgcgatcgagcgcggcgaggagccgccgaagcgcttctcgatcctcgaggcgtcgaaggcgacgcgcgagcgccgccgccaagagcgcgaggccggcaacaacgcccagcagccgcacctcccgaagcacagcaagaagccgacctacggcggcccgaccccgccgccgaactggcagtacccgggacagggccagcaaccccaaagccagcaaccacgctggccggaacagacgggacaggcggaggagatcggcttccgcttgcccgagcacgagcagccggacaacccgctgccgcagaacgcgcgcgatatgccggagcagcgccctgtccgcgatgccgaggaactagagaacgaaggcgagaagtagatgagtgaattcgaccgcgaacgcgccgaggccgcgatccgcgagcttttgctcgccgtgggggaggacccggagcgcgagggactcaaggagacgccggcgcgcgttgccagggcgtacgaggaggtcttcgcgggcctgcgcgaggacccgaccgagcagctggagaagacgttcgcggagaaccaccgcgagctggtgctggtgcgcgacatcccgatctactccacgtgcgagcaccacctcgtgccgttctacggcgtggcccacatcggctacatcccgggcccggagggcaaggtcaccggcctgtccaagctcgcgcgcctggcggatctgtatgcgaagcggccgcaggtgcaggagaggttgacggctcaggtggcggacgcgatcgtcgataagctgcatgcttccgcggtcattgtggtgatcgaatgcgagcacctgtgcatggcgatgcgcggcatccgcaagccgggcgctgtgaccaccaccagtgctgtgcgtggcgggttccagacgaacgcggcctcgcgcgccgaggtcatgagcctgatcaggagctagacagatggcgatcacgctcgaacaactcaccgcgccgggccgcacgacggtcatgggcatcgtgaacgtcaccacagactccttttcggacggcggacgctacctcgacccgcaagccgccctcaaccacgcgcgcgagttggtgcggcagggggcggacattatcgacgtcggtgcagaatccacccgccccggcgccacccgcgtgccggcggacgtcgaggccgagcgcgtcagcaccgtgatcgagctcctagccaaagagggattcaaaacctccgtcgacaccatgcgcgcgtccaccgcactcgctgccgcggaggcgggcgcgcacctgatcaacgacgtctccggcggcctcgccgacgccgacatgtaccgtgtcatggccgagacccagctgccggtgtgcctgatgcactggcggacggacaggtttgagtcggcgtctggaagtgccgaccacggcggggacgtggtgcgcgacgtgcacgaggtgctgaagaccatcaccggcaacgcgatcgccgccggcgtggaccctaagcagatcaccgtcgacccgggcttgggctttgcgaagacggccgaggacaactgggcgctgctcaacgcgctgccggagttcaccgaaggcgagttcccggtgctggtcggcgcgagccgcaagcgcttcctctccgctatccgcgccgagcgcgggctcgaccacgaccctgttgccgccgacccggcgaccgcggccgtcacggcgcttgcggcgcaggccggcgcgtggtgcgtgcgcgtgcacgaggtcgccgtctcccgcgacgccgtcgacgtggccgcgaggtggcgcaatggctgaccggatcgagatcaaggggctcaaattccacgccaaccacggtgtgctcgcccacgagacggagcacggccaggcgttttcgctggacatcacgtgctggctcgagttcgctggggccgccgcaacggacgacctcacacagaccgtcaactacgcggagctcgctcagctcgcacatggcatcgccaccggcacgccgcgccagctaatcgagaccgtggccagcgagatcgccgacacggcgcttgcccgcttcccgcagctacacgccgtcgaggtcacgctgcacaagccgcacgcgccgatcccgctcgtctttgacgacgtcgcggtggtcgcccgccgctcgaggaaccggcggtagccatgcgggcagtgctctcgaccggctcgaacatcggcgacgcccgcgcgcacctcgccacggtcgtcgaggctttcaaccccatcgcccaaagctcgctctacgccaccgcgccgtggggaggcgtcgagcagcaggatttcatcaatcaagcactgcttatcgacgctcccttcacctccccccacgccctcctcgaggcgtgccaagaactggagcagcgcgccaaccgcgtccgcgacgtgcgctggggcccgcgcaccctcgacgtcgacatcgtcgcgatcgacggcatcgagtcggacgacccggtgctcaccctgccgcacccgcgcgcgcacctgcgcgagttcgtgctgcgcccgtggctggagatcgacccgcacgccacgctgcacggacagcccttggagtactggctggaacgcctcgaacctcaaggcgtgaggaggctctaaggcatgaaccagggcatgaaccgcacctccatcccgggccttgccggcgccgccgcgtttacggcggccgcggcactgatattggtgcgcaggtattactccgcgttggcgtcgttaagcctgctctggcccttgagcctctggatcgccgcgttggtgtgcttcttcatcgcccacatggtgagaaagcgccgcgaggagggcggcgttggcttagaccgcagccaactcaacccgatgatggtggccaatttcatggtcttcggcaaggcgtgcgcgtggacgggcgcgctgtgcggcggggcctatgcgggccttttggcctacgttgtcccgaggatcgggatgctcaccgcggcagccgaagattttccctcgctcgcctccggagcgctcggcggcattgtgctcgccgcggcgggtgtggtgctggagcgcgcttgcgaggtgtcgccacctgcatcgggcgagggcgcaagctaaggtgaacgccatgaatgaccgcaattcgggaaacttttgggtaattgccccgttcgtccttgccgtcattggcactgtggtcatgctgttcaccaactcggccaacgcgctgaagatcgctctcattttcgcgctgtgggcggccgccgccggcatcctggtgattgaccgcgtgcgtcgcgaccgcgaccgcgcggttgccacattgtcggagcgggaggcggcgcttgccgacgccaaccgtctcctccaggagcgcccccaggtcgccgcgccagctcccgccccggcgccggcgatggcgtccgaggacgtcgcgttgctgcgccagctccaggaggagatccaggcgctgcgcacgcagcttgaggagatgcgcggcgaggtcttcgagtacgagccagccgccgtgcgcgcttccgcccgccgcatccaagagctggagccagaacccaaacccgagcccaaaccggaacccaaaccagaaccaaagcccgagcccaagccgggcccgtccagcgacgatacgatgcgcatcacccgcgtcaccgccccgaagcccggcacgacccggcgcacccgcccggcgggcgcgccgagcgcggaggccatcgctggccgcctgggccagcaaccatcgcgcgagcagcccaacccgctgtccacgctgatcagcgagcgcgcgcaggaagcaaccgaggcgccgaaggttgaaaaacccgagccccgtggtgggcgccgccgccgcgacgaggccggcgaggggtcgctgtccgtggccgacctgcttgcgcgcagccgggacgaggaccgttaagtagtgccacctcgtcttactgtcggggcggtcttcgggccgactccgctcgcggttgaactcgagcgcgcgagtcaccttgtgagcccggtggactccatcgagcacgttgatttggtgttgcttgatggggaggctggggaggttgttcggggcgtcgacaagctgaaagcccaagcgcgggacaagcaaatgttcctgcacaccgcgttgggtgccggggcgcagttgcttgatgatgtcgagacgtccggcgccatcgtcatgtgcgcgtcgaacctcttcggcaacgtgtgggtgacttccgccgcggacgaggtcggcgagacgatcgtcgggctcatcgtctccgagatcggcggcacgagcatcccgatctcggacacgcagcggcctgccctggtggcggcccagcgcctgcgcgcgctggagagcgtgttgcgaaacgacgcagccgacatccttcgcgacacgctgccaaccttcgacgtgttcgaagccgggtacatggcggcaccgtccggcacggcgggcccgatcgccgtggaggaattggagtgggtggtctcagccgtgggggatgagcaggtgcgcgccctgctccgggacgtcgagcggcgccgtgccgaacaggaaaggaagcagtaaatggcgtttgaaccgggccgagcggtggtggtgaccgacgaggcgcagctcgcgcagtacgggcgcgcgtttcgcaaagtgggtaagaagatcgcgctggtgccgctgggcgaggccgtgcacgcgggccacgtggagctgatccgcgcggcgaagtcgctgctcggcgcgtacgtgttcgtgacgttttccggcggcgaggtgccggagctgttcgcgcgcgagggcgtggacgtggtgtttcacgggcagatcgacactgccgcgcgcatcgagaccggtctggaccaccttgaggacccggagcagatcgcggcggagaccgcgcgcatcgttgccgcggcgaacctcgcccacgccaccgacttggtgctgggagagaaggacttcgagctgctcgtcgcggtgcagcgggccgtgagcgctttgcgcatggaggtcaagctgcactcgctgcccacggtgcgcctgacggagggcctcgccatctcactgagcaaccagcgcttaagccccgaggaccgcgaagccgcgctcgccctttccgccgcgttgaccgcgggtgcccacgccgctgagcacggcgccgaggtggtgctcgagaccgcccgcggtgtcttcgaggccgccggggtgacgcctgcctacgtggagctgcgcgacctcggcttccgccccgcgcccgacaagggcgacgcgcgccttctcgccgccgtcgacttcggcggggtgcggctcatcgacaacgtgggcctgccgctcggtgtgggctttaagtatgtcggggacgtctaagccgcctgcgctagactcgctgacatgtctgcgcccctgatagccgagatcttaaacggccgctacggtttcgacttcgccgccgatcgcatcaccgagatcggccgcacgcccgcctcgaccctcttcgaggcgaacaacgacgagggcgcggcagtggagatcgaggtcttcgacgcacccattgcgcaggacacgaccaccttggacgaggagtttgccaaggtccaggcgccgggcgcgtttcggccgaggcacgccggcctgcttgacgacggccgcgtgtacatcctccgcgaagcctccgtcggcacgccgttctccgacctggtggccgcgaagaagcaggccggcgagcagttcaccgacgccgagacacgcgacctgctttcctccgtggcccaggctgtcgacgactacaacgccgccggccaccccgagttcctcgcccgctcgatcgcggcgaagcagcttttggtgcagccgtcgtggtctgacatcccggtgaagctcgcccttgtcggcccgagcccggaatcggcggcagccgaggacaacctgcacgacttctggaatttggtcgcagacgtcaccggccgcccggtggacgaggaagcggcggcgaagaacgctaccgcgctcggctacttgcaagacgtgtgcgcctcggccgcggataacgtcaccggcccgggctcaggccttgtcgcccccggcgaccacgacggctaccgccgcccgcccgagccgtacccggcaggctacgtgcccccggcaccggaaaaggaagcgcgcaacccgtggccgtggatcatcggcgcgctcgccatcgcgctgatcgcgatggcgctggcctggtacttcaccacccagcgcggcgaggagtggtccgtggcggagaaggacatcgcggccgcttacccggaaatcgtgtccaggaaatccggccagcgcggttggcaggacttaaagtgcgagtccgcggcgcccgacgccggccaagaggccaagatccgctgcgccggcgaggagttgggcgtgtctgtggccaagtacccgaccgaggcgcagcgcgacgaggagcttcccggccagcagtacgccaccgtgctgggctcgggcgagtgcatgatcgaggactacgagatccccgacgcctacccgcaggctttcgccatggcgccgcgcgataagggccagtacctgatcgtggtcaacggctacgacgcggaaacggtgcgcttggatctgccggtgtgtgagtaggacacccacggccgacgggctacgattgtcggtcgtgatgaaccagcagccgcagaaccagacccaggacttatccgagcagcagcagattcggcgcgcgaagcgccagaagctgattgatgacgggcgcggggcgtacccagccgaggtcgcccgcaccatctcgctgaaagacctgcgcgcgaaatacccggatttggagcctggccaggagaccgaggacgtggtctccgttgcgggccgcatcatgttccagcgcaacaccggcaagctctgcttcgccacgctgcaggaaggcgacggcacccagctgcaggttatggtctcgctggcagaggtgggcgaggagtcgctcgccagctggaaggccgacaccgatctcggcgacatcgtttccgtcaccggccgcgtgatcgcgtcgcgccgcggagagctctccgtccaggccacctcgtggcagatggcgtcgaaggcgctgcgcccgctgccggtcgcgttcgccgacatgaacgaggagcagcgcgtccgccaccgctacaccgacctgatcatgcgcgaggctgcccgcgacaacgctatgacccgcatcaaggtcatcgccgcggtgcgcaagtacctcacgggcttggactacgtagagattgagacgccgatgctgcagacgctgcacggcggcgccgcggctcggccgtttgtgacccactccaacgccctcgacatcgaccttttcctgcgcatcgcgcccgagctctacctcaagcgcgcggtggtcggcggcatcgagcgcgtcttcgagatcaaccgcaacttccgcaacgagggcatcgactcctctcactccccggagttcaccatgctggagacctaccaggcgtggggcacctacaaggacggcgcggagatgatgcagggcttggtcaagttctgcgcccgcgaggtgttcggttcggaagcagtcacgcttgccgacggcaccgtgtacgacttctccggcgactggaaagtcctcgacatgtactcctcgctcaacgaagccctgcaacgcaagttcccgggccagcccgaggttaccgtggagtcctcggtggacgaactcaagtccatcgccgccgccatcggcctgccggtgccggagaacgccggctggctgcacggcaagctggtcgaggagatctgggagcacctgtgctccgaccagctctacgaaccgacgtttgtggtcaacttcccggtggagacctcgccgctgacccgcgaccaccgcgagaagcccggtgtgactgagaagtgggatctttacatccgcggcttcgagttggccaccggctactccgagctggtggacccggtgatccagcgcgagcgcttcgaggatcaggcccgcctcgccgcccacggcgacgacgaggcgatggtgctcgacgagaacttcctcgccgccatggagcagggcatgccgccgaccgcgggctgcggtatgggcgtggaccgcctgctgatggcgctgaccggcctcggtatccgcgaaacggtgctcttcccgctggtcaagccggaagcgaactagggctttctacccgaaggcccacacagccttcgcgccgtcggtgttggtggcgatgatgacgaactcgtcccactcgtagatagcgtgttcgctttcgccctggaaggtttcggtggcgcccacgtcgagcgagaagctcgcatctcttttcagagcgacctggtcgccgttcgggtacatcgcgacgaattcctccggcaggtagaacgttgacgtgccgggggtgtccttgtttccgagtgtgaacgccgcctcgtaacgcagggtgcggtcctcaaaccacgcgttggtgaacgtgaactgggagccgtcgaactcctcttccggcacctccacggtctcacccggcgcgagcgccacctcgcgcgcctcgcggtacgcgtcggagacggccgagacgggctgtaccgcgacgtccttgtactcaggcgcggagaagtcgaacaacccgcgcttgtccgaggagaactggtattggtcggccaggttgtccagctggttgatcagcgggttcaccgcttcgcacggcccgtcgacggtgatcgagacttctttgtactcctccctcgtgctcaccacgacgcactcggcgccggtcttggtggtgtaggcgacggcatcaagcgagcgcggcgcggcggcctcgcggtacatccagttgtggtggtggatgtcgggcttgaactccccgctcgggcggtggtgcgggtcgaaggtcacggcaaggggaaatccctccccggaatcaatcaacccctcgcagccgcgcgtagaccagtccacgctgcgcatgccgacgctgccgtaaaactcgtcgccgaggttgcaggtcttcagctcgccggcctcgaagaactcgttcacctccttgtcactccagccaagcggacccgcaggcacgtcgcgcacctgttggaaggcgagcagcccgccgaagaccaccacaatggcgccgagcacagacccgaccgcgatacctgcggtgttgcgctccttctccggctcgggctgcggcgcttggttgctgtagacatagggagagccggcgaacggctcgtgttgcggggtgtcgtaggggttggtcataacaatccatcatgctctacggcggttgcgggcgcgtgcgttactatctcgccatggcccactacaacctctacgactcgatcggtctggactcctcgaaggacaccgccgcgctggctgcggagatcgacgagcggatccgctccggcaacacgtggaaccgcgggggcattgaggagctgcaggttgcaagggcagttttgggcaacgcctccaggcgcgccgcctacgaccacaaactctcagacccccacgccccagacgtgacggtggattcgctgcgccggttggccaacgtgaacttcgacgccaaccccgccgcccccgcgtaccagtacagccccagcacaacacagcccgcctcgcccgcgcccgccccagaaacgaagaagcgccccgtgtggccgtggattgccgcggcagcaggtgtactcgctgcagccggcggcggtttctggttcctcgccaactccggaactgagtgggacgagacgcacgcgcaggtcgcagccgactttcccgcgctgatcgcggagaaagacggcggcaagggatacctcagcatgacgtgcacctcccgggagaccgagggcgaagaggaagcgaagatccgctgcgagaacgccgagatcgggttgaatatctaccattacggctccgccgagcagcgcgacgctgtcgtcggcggaggcgagccggagttttacggcaacgacgtctgccagttcaccgcagtcgagatccctgaccaggcttaccccacctactacatcgcgcccaacggggactgggatacctacttgctgctgctcaacggcgaggacgccgaaaagatgaagacgcgccttcccatttgctagctaaggttgaaccttatgagctccccctacaactacagcggttaccagccccagcacacacagactcagtacggccagatggagccgtacaacgcctacaccccgccggtgggcgtgaagcagaagagcaaggtgctcgccgctgtgctgttctttgtgctcggcggcctcggcgtgggcaacttctacctcggccagaccaagcgcggcgttttcacgctcctgctctcgctgtttgcgggcttctgctttctcactatcttgctcatcccgctcgcgtacttgattgagggcgcgctcttcctcgccatcgtcgcgcagatcatcttcgtgctcaccggttcgctcggctacgaccgcgacggcgacggcgtcccgctccgctagttcttatggcggcgcgcacggttctccgcggcatcggggtctccaccggagcggtggtgggcccggtggcggtggtggaggggcaggtgggcgtcgataagcatgaagccccttgcgccgatcctgagctggtgcgggacgcgctcaaccaggtggcggagggctaccggagccgcgccgggcaggcaaactcggacacggcgcgggaggtgctggcggcgacggcggcgctggcaggggaccgcgcgcttgcaaaggccgtggacaagcagctcgcccagggcgctggcgcgacggctgcggtttatgaggccgtcgaggtctacgccgcgaagttccgccagctcgggggcaccatggcgcagcgtgtgagcgacctgtacgacatccgcgatcgcgctatcgcccacctccgcgggcttcccgagcctggcctgcccccgctcacgcgccccgcaatcctcgtcgccaaggacctcgcgcccgccgacaccgccacgctcgacccggagctggtcctcggcatcgtcaccgaggaaggcggtccgacatcgcacaccgcgatcctcgcggcgcagctgggcatcccggcggtggtgcaggcaaagggcatcaaagcactgcttgccgacgcccccctcatctccctcaacgcccacaccggcgaagtggtgatttccccaaccgaggtcgacgtccgcgccctccaggacggcgagcgccgccgcctcgccgcgttcaccgctgcttctggttcgcgggcgccggtcgcgctgatggccaacatcggatcagtgcgcgacgcttctgccgcgcccggtgccgatggttgcgggctctttcgcaccgagtttcttttcctcgaccgcgactgcgcccccggtctgcaggagcagaccgagacctacacccgggtgctgcgggcgttcgggccgcggagggtggtggtccgcaccctcgacgccggcgccgacaagccgctgcgcttcgccgacctcggcgcggaacccaaccccgcgctcgggcggcgcggcatccgactcgcgcaggcgcgcgaggatttgctggacgtacagcttgaggcgcttgccagggcttcgcgcgccgtgcccggctcgcaactgtgggtgatggcgccgatggttgccacggtggaggagacccgctggttcgtcgaacgcgcccgcggatacgggctcgcggacgtcggcgtcatgatcgagacacccgcggcggcgcttacggcggcgcagatcctcgaggccgccgacttcgcctcgatcggcaccaacgaccttgcgcagtacacgatggccgcggaccgcatggcgggcgaactcgcgccgcttctttcgccgtggcagccggcggtgctcacaatgatccgcgaggcttgccggggcgccgaaacccacgccaaacccatcggcgtgtgcggcgaggccgccggtgatccgctgatggcgcttgttcttgctggcctcggcgcaacctcgctgtcgatggcccctgtccgcatccccgccgtgcgcgctgccctgcacgcccacggcttgcaagcctgccgggagatggcgcgcgccgctctctccgcgcccaccgccgacctttcgcaatcagctgccgctgacctgttcgctactggcgaacatagccgctgagctggcttgatttggctgcagccgacagtgtgtgcggaaagcggggaagttgtgttgggcccgcgcgttatggttgtggacaactgatttagggactgcttgaaaaaggggtagccacatgtttgaacggttcaccgaccgcgcccgccgcgtcatcgtcctcgcccaggaagaggctcgcgagctcaaccacaactacatgggtactgagcacatcctcctcggcctgattaaggagggcgagggtgtcgccgccaaggcgctcgagtcgatgggcatcaatctcgaggacgtgcgccgcgaggtcatcgacattatcggccacggcacccagcccgtgaccggccacatcccgttcaccccgcgcgccaagaaggttctcgagctctcgctgcgcgagggtctgcagatgggccacaagtacatcggcaccgagttcctcctcctcggcctcatccgcgagggcgagggcgttgcagcccaagtgctgatcaagctcggcgccgacctgccgcgcgtgcgccagcaggtgatccagctgctgtccgggtacgagggcggcgacggccagaatccggagatgccgcagcagaccgccggcgccgcaaccgcaggccccggtccgcgcgggggcgggcaaggggagcgctccaactcgctggtgctcgaccagttcggccgcaacctcaccgcagccgccaaggagggcaagcttgacccggtggtcggccgcgacaaggaagtggagcgcatcatgcaggtgctctcccgccgcaccaagaacaacccggtgctcatcggtgagcccggtgtgggtaagaccgcagtggtggagggcctcgcgctcgacatcgcaaacggcaaggtgcctgagaccctgaaggacaagcaggtctactccctcgacctcggctccctggtggcgggctcgcgctaccgcggcgacttcgaggagcgcctcaagaaggtgctcaaggagatcaaccagcgcggcgacatcatcctgttcatcgacgagattcacaccctcgtcggcgcgggcgcggcagagggcgcgatcgacgcggcttcgctgctcaagccgaagctcgcccgcggtgagctccagaccatcggcgcaaccacgctggacgagtaccgcaagcacattgagaaggatgcggctcttgagcgccgcttccagccggtgcaggtggacgagccgagcgtcgaggacaccatcttgatcctcaagggcctgcgcgaccgttacgaggcgcaccaccgcgtgtcctacaccgacgacgcgctgaaggccgccgctaacctctcggaccgctacatcaacgaccgcttcctgccggacaaggctgtcgacctcctcgacgaggccggtgcacgcatgcgcatcaagcgcatgaccgccccggaggcgctgcgcgaggtggacgaccgcatcgcggaggtgcgcaaggagaaggaagcggcgatcgacgcccaggacttcgagaaggccgcgggcctgcgcgacaccgagcgcaagctcggcgaggagcgctccgagaaggagaagaagtggcgctccgacgacctggaggacatcgccgaggtgggcgaagaccagatcgcggaggtgctggcgaactggaccggtatcccggtgttcaaactcaccgagagcgagtcgtcccgcctgctcaacatggaagacgagctgcacaagcgcatcatcggccaggacgaggcagtcaaggccgtgtcgcgctccatccgccgcacccgtgccggcctgaaggacccgaagcgcccgagcggctcgttcatcttcgccggcccgtccggtgtcggtaagacggagctgtccaaggcgttggcggagttcctcttcggcgacgaggattccctcatccaggtcgacatgggcgagttccacgaccgcttcaccgcgtcgcgcctgttcggtgcgcctccgggatacgtcggctacgaagagggcggccagctcacagagaaggtgcgccgcaagccgttcagcgtcgtgctgttcgacgagatcgagaaggcccacaaggagatttacaacaccctcctgcaggtgctcgaggaagggcacgtgaccgacgggcagggccgcaacgtggacttcaagaacacggtgctgatcttcacctcgaacctcggcaccggcgacatctccaaggctgtgggcctcggcttcaccggcagcaccgcgacggattcggacgcgcagtacgagcgcatgaagaacaaggtccacgacgagctgaagaagcacttccgcccggagttcctgaaccgcatcgacgaaatcgtggtcttccgccagctgacgcaggaggagatcgtagagatggtcgacctgctcaccgcccgcgtggacaagaacctggacgcccaggacatgggcatcgagctcaccgccgacgcgaagaacctgctggccaaccgcggcttcgacccggtgctgggcgcgcgcccgctgcgccgcaccatccagcgcgagatcgaggacgcgctgtcggagaagatccttttcggcgagatcggcgccggcgagatcatcaccgtcgacgtcgagggctgggacggcgaaggcaacggcgagggtgcgacgttcaccttcaccccgcgtccgaagccgctgccggccgacaccttcgatgaggaggatgtggagctcgagagcgaagtccgcgagatcgacccctcgcgcgtgagcgaaccgtccaccgcgtccgagttcccggatgagctggatgagctggacgaggacgacgatctcggcggcgaggacgagggcgagggccgcggcccggtagagccggcctaagcccagcccaaggtaagccccgccgttgaaggaccgcccggcgaagcggtcgtccatccgggagcctgctcgaaggggacgatgtcgtcggtcaataggccctttggcgcgaggtgtaggtgatgcgcttgccgctgaaaatttccgcggcggcggcaaccgcgcgagcatgtggcatgggtggaaagtgtatcctgctgcgcatgggtcttcagtacagaaagaaacacaaggtgggcaagaacgtctggatcaaccagaccggcactggggcgtccgtgtccaccaagctcgggcctgtgaccgtgaactcgcgcggcggtgtgtgggtgaacctgccgggcgggatgacttaccgcggcaggtggaagtagccgcgttcgttttgttctaggagaccgtcggcaagcaagctgcccagcgccctcgagcgctgcgccgcgtccggccacacgacgtcgatttcggactgtggcacgggtccttcggcttcgcgcagggcgcgcatgattttgccgcggacctggcggtcggtgccttcgaagcgctgcgatttctttttctgaaacgttttcgggtagccgcgctcgcgccactcgcaccggctcaccgggcacgccccgcacagcggcgcggttttgcacacgagcgccccgagctcgatcaggccctccgagaacaccgggccgttgcgcgacggcagcagctcggccacctccgcaacctcggacttgcgcgccgcctggttctctaggcccttgatcgcgcgggcgtgcacgcgcctgacgttggtgtccaccaccgccacgttgcgcccgaaggcgaagcaggccacggcgcgcgcggtgtactcgccgatgccgggtaacgcgagcagctcctcgacggtgtcgggcacgcggcctgcgtgcttatccacaatgacctgcgcgcactccttcaggcgcagggcacgccgcgggtagccgagcgagccccaggcgcgcaaaatttcgtctgtgcccgcggcggcgaaggactccggcgtgggccagcgcgcgatccactcctgccaaatcggggcgacccgctccacctgtgtttggtggctcatcacctctgacagcagcacgccccacggagtcgtgtcgcggcgccacggaaggtcgcgcaaattggccaggtaccaatcaaccacttcactctgaaagctcacaagtgggagaatatcggccatgactacatcgcagaatcctcaggaagtttgggaagcgctgctggcgggaaacacccggttcgtcgagggcgccgtcacctcaccgcaccgcgaccccgcgcgtttgaacgagatagtctcgggccaggcgccggtcgccgccgtcatcgcgtgcagcgactcgcgggtcccggtcgagttgcttttcgacgccggcttcggcgacatcttcgtcatccgaaccgccggcggctgcgtcgattccacggtggccgcctcggtggagtacgcggtggaggggctcggggtgccgctggtcgtggtgctgtcccacgagtcgtgcggtgcgattggtgcggccgtcgctgcggtggacgctccggacgagaccccgctgggtctgaccagggtgttcgtggagaagattgcgccgtcggttctggcggcccgcgcggcgggggagacggaacgcgcccaggtcgaggcggcgcacgcgcggattacggcgcagcacttggtggatagggtgccgtcgataagaagctccggcgcgggtgtggtggccgcgaggtaccaccttgatgggggccgcgtcgagaccgtctacgagcacttcgctggctaaagtgggggcatgacgaaccagcgcccgctccccgatgagatttacatgcgccgcagggtcggcgcgctcgtaatcatcctgctcgttgtcattctggcggtgtgggggctcagcgcgctggcgcgttccggtggctcggacgcgacacctgctggcgggacagaatcggtgagcacgagcaccgaaccggcgccggtgacggaaccgacggtgcccgcaccttccgacgacacagagaccacagagaccacggagaccaccgaaaccaccaccacagagacgaccaacgcggccgaaagcgagaccaccgcggccgcagcgaagaagggcagctgtgaactcggcgacttggtcatcaccgcctcgaccaagcacccgtcgtttcccgtgggcagcaagccggagttcttcatgaacgtcaaaaacccgaccgacaccgactgcgtgatcgacgtcggtgacgacctgctgcggttcgaggtctacgagatgcgcaccaacgcgcgcgtctggtcggacaccgactgctacccgggtgttgagacgggcgtccaggagttcccggcgggcacggagcgcggcctcaacgccgtgtggtctggtaccggttccgcgccgggccagtgcaccaaccgcgagcaggtgccggcgggcgcctattacctgcacgctgtgatcgacgacaacgcttccgacccggcgccgtttaacctcacttagccgggaaaactagagccggcgcaggccctctgcgatgtggcgggcccacagtgccgaaacgtgttctgcggcggcgagttcctcgggggaggcgtccaagatcgcgggcagctcgccgaaggcggagacgatgtggtccatcaggaacttcttcacgcgcggcacgcgcgacagcgcgcggtagccgcgcggcaccacgccctgcatgaggtgctcctccgaagcaggcaagccgaggccgcgggcgagggctcccgtgttgagcaactcggcgtcgggaagctggtcgaaggcctcaagcgcggctgccacctgctcgtccgtgggcaccggcccgagcgcgaggtagtcgcgcaccagcatctcgatgtcgctgctgtttgacccctcgagctcggacagctgcaggatgagctggcgcgcgtcggtgccgagctccacaattgtcaagtctaggtctttcgccgcgcgctccagcatcatttggcgctggagcacgttgaccacgtcgcccacggtggcgtagccgttcatctcggcggcgaagaggcgctggttagccaggtcgaggcgctggcggtagcgctcgatggtggacagcgcctggttcgcctgcgcgatcagaaccgccggctcttcgaggcggtggcgctcaccctggtagtacagcgtcacggtgttcatcgacgcggagacggacaccacgggcacaccggtctgcagcgctgtgcgctcggctgctcggtggcgggtcccggattcgacggttgggtagcttggcgacggcaccaactgcacattcgcccgcgtaatccgctccccatccgcggagaggatgacagcgccgtccatcttcgacagctcgcgtagcaacgtgggggagaacggggcgtcgaaggttactccgccgtcgcagatttgggtgacctcggcggcgtcgccaagcacgatgagccccccgcccctgcctcgctgaatgcgctcaaccccgtcgcgcaggggggtgccgggggaaagtttggatagggcgtcgcgcagagtcacgcgagcaaccctatcgcctcggcgagcgtggacgcctgctggacgcgcatgccgtcgaccgtgatcttttcaccggcgggcacgatggcgcgctcgtagccaaggcgggcagcctccatcaggcggcggcccaggttgggcacgcggcgcagctcgcccgcaagccccacctcgccgatcaccacggtcttttcgggcagcggcttctcgtgcaggctcgaccacgtcgccagcgccaccgcgaggtcggtggcggtctcggtgatgcgcaccccgcccacggtggcgacgtaggcgtccttgtcgttcgtgcgctccccgcagcgggcctgcagcaccgcgagaaccatgggaacgcggttgccgtcgagaccggtgacgacgcggcgcggcgacttgttcaccgggtcaacggtcagcgcctgcacctcggcgagcatggggcgcacgccgtccatcgccacggtgaccgccgaaccgtccggggtgcgcccgcggtgggagaggaagagccccgacgggtccggcacctcacggatgccgtcggcggtctgctcgaagcagcccacctcgtcggtcgcgccgaagcggttcttcaaaccgcggagcattcttagcgacgactgcctatcgccctcaaaattcaacaccacgtccactaggtgctccagcacacgcggacccgccacgttgccgtccttggtcacgtgaccaaccagcagcacggggaggttcgacgtcttcgccagggtggtgagcgcggcggtcacggcgcgggactgcgccacgccaccgggcacgccctccacgcccgaggcgtgcatggtctgcaccgagtcgacgatgagcaaggtcgggttgacggccttgacgtggccgaagacggtgtcgaggtgggactcggcggcgaggtagagggtgtcgcgcagcgctcccgtgcgctcagcacgggcgcggacctggcccgcggattcctcggcggtgacgtagagcgccttcttcccctgctgcgcccagcgtgaggcgacttcaaggaggagggtggatttgcccacgccgggctcgccagccatcagcactacggagccggggacgacgccgctgcccaaaacgcggtcaagctccccgatgccagatgttacggcgtgggtggccgcagcgtcgatagaggtgatcggcttcgcggcagttgtgggcgtgagtgcggaggtggaggtgaggggggacgacgtgacgtcgttaagcaggtgctcctcctgcagcgttccccacgaaccgcactccgggcacctgcccaaccacttgggggaggagtacccgcattcggtgcaggtgtggattacccgcgcctttttggccaagctgcttcgggacttacttggacgggtcgcggtcgacctggccggacgccacgatcggcgcggagacggtcgcggtgacttcgatggagccggtgtcgaagttgaacttcaccggcacgttgccgccgtacgcgaagttcttgttttccacggaggttgcgacgtactgggtgcagtcgctgtcggtctgcggcatgcgctcgaggctggacgccgtgtcgcccaccagcacacagttgtaggtgatcttctggctggagccgaggttgacaggggtgccgtcaacggtggcggactggagcgtgtggtccttcatcgaggtgtcctggttcgtcgcgacgaacttcagcgcggcctggccgttctcctcaaggatgagcgtgacgtcctgaactgacagggctccgtcctcggtgaagacggaagcgccgtcgaccgcggccacctggctcgaggtctgggtaatctggccggcagagcagctggccagggccaatgcgcaggcgatcgcggcaaccggcttcagggacttcacgtcgatgtcctccatcgttgttggaaaaattgctgtgaaaattataggcgaattaccccggccaactctactcgcaggcccgccttatttccgagtttcgcagtggtactctagccggcatggaattcaacgtcggagaagtagtggtctacccgcaccacggtgcagcccgcatcgctgacatcgagcagcgcgagatcggcggcgagacgctggactacctggtgctgcagatcctccagtccgacttggaggttcgtgtcccggtcaagaacaccgagcttgtcggcgtgcgcgacgtggtgaacgaggagggtctgcagaaggtcttctcggtgctgcgcgagaccgacgttgaggaagctggcaactggtcccgccgctacaaggcgaaccaggagcgcctggcttccggcgatatcaacaaggtggcggaggttgtgcgcgacctgtggcgccgcgaccagggcaagggcctgtccgcgggcgaaaagcgcatgctgggcaaggcacgccagatcctcgtgggcgagcttgcgctggctgagccggtcgacgaggcgaaggtcaaggagatggagtccggtatcgccaagattatcgaggagcaggtaaaggctggcatcgtcgaagatccgcgcgatgcagtcgaggacgatatggacctcgacgacttgagcttcgacgacgaagacgacgacgagaactagctcagtgcagcgcccggtcgtcgccgttgtcgccgccgcggggaagggcacccgcctcggtgcggaggtgcccaaggcgtacgtgccgctcgctggctcaagcctcgtcgaacgctcggtggctgcgatcgaggcttcgggagttgccgacgacatcatcgtgaccgtcggcgaggggatgctcgacgttgccgtgcgggaactcaaaggccacagcgtgcgcttcgtcgccggcggtgcggagcgcgcagacagcatccgcaacgcgctagagagcatttcgcttgccgacgcctgcgttatcatccacgacgccgcccgcgcactcaccccgccctcgttgttcacccgcgtggcttccgccgtgctcgacggcgccgatgcggtcatccccgtcctgcccgtcgcggacacgatcaaggtggtgtctggcgggcgcgtcgtttccacccccgaccgagccagcctgcgcgcggtgcagaccccgcaagccttcgacctgcgcaccctccgggccgcgaacgaggcgtttttcgcgtctccgcagaccttcgccgcaacagacgatgcttcgcttatggagtggcacggagtggacgtgcacaccgtcgacggggaccccttggcgttcaaggtgacaaccccgctcgatcttcgccttgccgaggccattctcgctcgttaacccgcttttattcttcttcgcaacgctatgttcgtcgcgtttgctataagtgtttcaacctcttaacggggcctgtttgggatcgaaaacaactgctaaaaacgatgtttggagcggttgttatagtcccggtaatcgattgcatgtgcgaagaagaaagtgggtgaaacgatggcgtatttcgcaacggagcgcggcggcgacgagctgtgcgccttggggcacttaagtcgagagatcgagtacgaggtgttcatccgatacgcggtcaacgtggcggagatagacgacgctgacctcgacctccaagtcaaccgcctcagcgcggcgttggggtggcgcccagcccgggtgcgggacgggatcctggcgtactacacgctgcgcagcctgcccaagttggcggcgatgcagaaggagacgaagcgcctcgatctcgaccgggtgcgggcgatctccgaggtggtgaccctgctttacgaccttccccaagaagacatcttcgaagagttcgacgactacctcgtcaccatgttcaccccgaagcgtgacggtgcggagctgccctcaccgcgaacgatcaagcgcaagctcatcgaactcgtccgcaagatcgacgcttcgctcgccccaaacaagaacgagaagaagaagcgcaaggacgacaaagatcagcgcgacggcgcgtgcgaggtggatttagtcgccctcgaccaacgtaattcgcagttgaccttgggcggcaacaacctgctgatgggcctgatcaacaagtcggtggaaacgactgcgaagatgcggaacctctccaagggcgagaccgtcaaaaagctgctgctcggcgagatttccccagcagccaacatcaccctccacctttacgcgcccaagggcgagcccgagtcctactacatcccccagattggctggaccgacgcggaggggaccgaggccgtcgcgcagttcctcgcggaccacgatcaccgcgtcgtcgacctcgaccaagctgccgaagcccgcacgaacgcgtacgtgcccaccgacgccatccgagcctacgttcgcgcccgtgacggcttctgcatcttcccgggctgcgaggtggaggcggagcgctgccagctcgaccaccgcatccccttcgacgacggcggcgagacggccccgtcgaacctcttctgcctgtgccagaagcaccacaacatgaagaccgaccgccgcgcgtactacgtcgtcgaccccgtcacggccgacatcgtctggctcttcgaagacggcacctaccagctgaccaagccagacggcatcatgggcagctacaccacgccgcagcgcccgcgctggaagcagacgattaaacagcgcatcgagaaacgcaccaaacgcgcggcgttcgacgcccgctgccacgccacaatcgacaagtacctcagcgacgccgacttcttcacctgcatccaaaccctccaccagctagagaagacttacgcgctgaagttcgacttctggccggacgcgccgccatgggtgacctgcagctacggggaatggcgggcgttcaggctcggtgcctaccgcgacggttacgtctccgccgacacgttgattgctgagttcggcgacgaaatggccgagaccttgggggtgggtgtgccgttctaggtacggttgagcacatgcacaatcttcgcgcggggaccgcgttcgacgcccaccaactccaggcgggcaaggaatgttggatcgcaggcgtgctccatcccggctacgacggctgcgagggccactcggacggcgatgtggtcagccacgccatcgtcgacgccgtgctgtcggcggcgggcctcggcgacttggggtccttcgtgggagtcggccgccccgaatacgacggcgtgcgcggcgtgcagttgctgcaggagctcaagcagcttgtcgacgcccacggccactccatcatcaacgcctccgcacaactcatcgcccaaacaccgaaaatgtcgaaagtcagggaggagtgcgaacgcaccttgagcgaggctctcggcgcaccggtgtccgtgtcggcgacgacgaccgaccacatgggcttcacgggcagcggccaggggcgcgcagcgattgccaccgcgttggtggaacttggcacgaaagtaccgacttcgggaacttaggtacctgacctgctctttcagcttctccccagggggttgtgcgggttaggttacccgtatgaagaaaaccttgaccgccctgtgcgccgccgcattcgcagctgtgggcgcgccggtcgcttttggtgtgcctgccatgccgcaggggtacccaattgagggtctcgacacgccgtgcgacaccgccactttctcagacccgcagtggcgttacggcgagatcgcaaggcgctaccttgctgacggcaccctccaattcaccaaccgcaccgaccaaaccgtgccctacaccgcaacagtggaaaccggcacaaaccacaagatcgaagccaactcgaaggccgcgctgcccaacgggtggaacaccaccgcgaagacggacatcggtctgaaggaatccaacggttggatcgagggcgagaccttcggcccgatcgagctggggccgggggagtcgttccgcgtcgactacggcgtgctggagaaggacttcatctccatgttcatgacgtgcgacaacggggtcttgcgcaacgggcccggcgcgaacgtgatccgcggaaccggtcctgcggagcggtacgccttcgcgtacgtcgttaaggcggacgggacggtgtcggatgtggcgttggaggtgccgtcgagaagcgaaggcgcaaactcgcggccggtcggtgacacatacacggcgacgtcgggcccgagtcttgagcagatcgccagcccgcgcgacacgcgcgtggcgccggggccgaacttccgccgcgacccggactggccgcagctcgggcagaaggcgcggccgggggacaagtcctactacccgtacgacatcgaagcggtggcgccgacgttccgaaaacccggctactcgcaggactttctgaactggtcgaagggcacctacacgttcacaccggtgaccgactacgtggtcggcgcggagttcaacggctacctcaactggatgggcggcggcgggcggttgcctgcgggctggctggaatcggtcggcgccgcgccgcgcgccctcatgccggtgggcactgcgctcaaacctgttgagctcgcgccgggcgagcgggtgcgcgtggagtacggcacgaccatgacgcggatcaactaccgcgagatctcggctgggcgcgacggcgcgtacagccgcgtgaccgcgcacccgcaagctagcgccccgagcgggttttgggccgaggccctgatcaccagcccggacggttcgacccggaccgtggacatcacacccaacctgtaagaaagaagattcccatgaagcgcgcaattgtttcctccctcgtcgcagccgccctcgttgccgcacccgccgcccaggcgctgccgcagcgcaactacaccgccgtgaacccgaccaccatcggcgcgtactgctcgaacccgggcgaccggggccaaacggtgaacatcgtccgcagctacttcgacggatccgcgggcacctggaccgtgtcgaactacaacgacgagccgctgccggtgacccgctcgatcacggagaccaagacgaagacgtggaacgtcaccgcgggcgtgagcttcgatgtggccaagctgatccagttcacgttctccaccagctacaccgacacgcagacctacaccgttggtgagcaggtcggaccgtacaacatcgcgccgggcaagaccgcggtgctgcaggccggctggatcgtctccgacttcgagggccaagagacggtttgcggcgccaaccacacctggcagggcgcgggcaacacgttcaccgcgaccatgccgaaggagcgccacgtgcgcgtgagcacccgcgacaacatggactggggggcgtaggtggggaaataccgagcagctgcggtggttgtggcggcgtcgatgttgatggcgccgtcggcaagcgccgagccgtacgatttcgaactcccgcagcgctggaacaccgatctggctccgggcagcacctgcgccacgccggggttgaaggacacctacgtcaccgcgacgcgccgctggttcaagcagacggacgccgccagcgtggctaacgacacggaggaaacagtgcccgtcacgcagacggtgaaagagaagcgcgtgcagacgctcgaggtctccggcacgttcacccccaagggcgacctggtgaagaacgtctcgcgcgcctacgggtggaagtacgtgcacgaggtgtcgtgggcgctgaaccagaaggtggggccctacatgctcgctccggggacgcaagggcgcttggtgtgggggttcaccatgctcgacggtgacgcgcaggatgtggtgtgtggggaggggaaggtgtgggagggcgtcggcaagcagtacagcttcaccgttcctgaggcccgctactcggagcttatggtgggttcatcccagctgtagacttgggtgccgtgactcaacgcatcttcgacaccgccacccgctcgctgcgggacttcgagccggtgcgccccggacacgtctccatgtacctgtgcggggcgacgccgcaagccgcgccccacatcgggcacctgcgcagcggcgtcgcgttcgacatcgtgcgccgctggttcatggccaacggcaacgacgtggcgtttgtcaggaacgtcaccgatatcgacgacaagatcctgacgaaggccgaagagaacgaccgcccctggtgggagtgggtgtccacctacgagcgcgaatttacccgcgcatacaacacgctcggcgtgctgccgccgtcggtggagccgcgcgcgaccggtcacgtcacgcagatggtgaactacatgcagcggctcatcgacaacggctacgcctacgcgcgcgacggctccgtgtactttgacgtgccggcgtgggtggaagcgggcggggattacggctcggtgtcgggcaacaaggtagaggacgtaaggggtgagggaggcaccgataaaaagagccccctcgacttcgcgctgtggaaggcggcgaaacccggtgagccgcactggccgacaccgtggggtgacggccgcccgggttggcacctggagtgctcggcgatgtccacctggtacttgggcgggcagttcgacatccacggcggcggtctggacctgcagttcccgcaccacgagaacgagcaggcgcagtcgcacgcggcgggcgacgggtttgcgaactactggatgcacaaccactgggtgaccatggcgggcgagaagatgtcgaagtcgctcggcaacgtgctgtccatcgacgccatgctcgagcaggtgcgcccagcggagttgcgctactacctgggctcggcgcactaccgcagcgtgctggagtactccccggaagcgctgcaggaggcggccgcggggtaccgccgcatcgaggagtttgtgaagcgcgccggctaccccgagccgacgacgtggaccgacgggttcgcggacgcgatgaacgacgactttggcgtgccgcgcgcgctcgcagagatccacaacaccgtgcgcgagggcaacaaatctggcaacccggccgaagcagcggcccaggtgcgcgcgatggcggcggtgctcggcatcgatccggggcagtggcagcagcttgacgacgccaccagcaccacccgcgccctcgacatcctcgtgagcgccgagcttcagcgccgcgcggaggcgcgcaagaataaggactgggcagaagcggacgcggtgcgcgaccggctggcggaggccggtatcgaggtcaccgacaccccggacggaccgacatgggagatgaggtaaatggcgaaaccgtaccaacggccggacaagcagaagaagaacaagaagggcccggccaaggggtccggcggccagatccgccgcgggctgcggggcaagggcgccacaccgaaggcggaggaccgcgtctaccacgcggcgcacaagcgcaagcttgagcgccagcgccgcgactctggtcgccacgagaaggagcaggcggacttggtcgtcggccgcaacccagtggtggagtgcctgcacgcgaaggtgccggcggaagcgctttacgtcgcgctcggcaccagcaacgacgaccgcttgaccgaggccgtcaccctcgcgcactcgaagggccttccggtgcacgaggtgccgcgccagcagctcgacgacatgacgggcaacggtctgcaccagggcatcggcttaaagatccagccgtacaagtacgcggatgtgttcgacctgatcgccggagcgaaggacgaggccggcatgttcgtggtgctcgacaacatcacggacccgcgcaacttgggcgccgtgatccgcagcaccgctgcgttcggcggccacggcgtgattattcctgaaaggcgcagcgcccaggtcaccggcgtggcgtggcgcacctctgcgggcacggcggcgcgcctgcccgtggcgaaggcgaccaacctcacccgcaccatcaaggagttcaaggacaacggctacatggtcgtcggcctcgacgcgggcggggagcacaccctggacacgttcgagggcggcacggacccggtggtcatcgtcgtcggctccgagggcaagggcatctcgcgcctggtgcgcgagaactgcgacgtgatcatgtcggtgcccatgcaggactgggtggagtcgctcaacgcgtccgttgcggcgggcgtggtgctgagcgagttcgcccgccagcgccgcgtgaagaacgcccaaaccaactagcccttatgccgtcgctcgcgtccctcgccgcggatttgggggtatcgcggaccacggtgtcgaacgcgttcaatcacccggaccagctgtcgaagccgctgcgcgacaagatcctcgcggcggcacgagcgcgcgggtatgccggccccgaccccatggcgcgctcgcttcgcacgcagcgcacgggcgcggtcggcgtcgtgctgaccgaggagctgcccttcgccttcgaggaccgcgcgtcggtggacttcctcgccggtctcgcgcagatcagcggctactcgctcacgctgattccccaccacggcagcgtgcacgatgcaattgtcgacggcatcgtggtctactccgtccccgacaacgacccccagctgctccaggcaagacagcgaaacctgccgcttgtggtgtgcgaccagccgaaagataccggcgtgccgtttgtgggcatcgacgacttcgccgcgatccagccggcggcgcaggcgctcaagaaggcgggccacagcaaggtgggcatcttggccaagcggatgttttcgcgcgcctacaacggcgaggtcggcgatgttgcggcggcggacttgcaggcccagcgcgcccgggtggagggcgcccgcgcggtgctgggcaacgttccggtggtgacgcgccacgcgaacgacatcgattcggccgccgacggcgcccgggaactgctcacccgccaccccgacctcaccgccgtgttgtgcaccaccgactccatggcgctgggggtgctcgcggcctacggcgaccgggtcccgcacgagctgtcggtgacagggttcgacggcatttccgaagcggagcactaccgcttatcgacggtccgccaacccaacaaacgcaaaggccaagaagccgccgccatgctgcacagcctcatgaacggggaggaaccagaaagcgttatcctcggcacggagttcgtcgcaggcgctacggttgctcccgcagcactctgatgctgggcgggtcgaggagctgctcggtagaaacgaggagcttctcgcttggcgacgcctccctcacctcaaacatcgcgccctctttagcaacagccgtcacctggttgtgcgtgtagcgggcggcgccgaggcaggtgtcggcgggtgtttcctgggtgagggtggtaagggtgagaagggcgtcgtcaagcgaaaagctcccctcgagctttgcgcagggcgtggcgccctcgaaggttgaaccgtggacgcggacggtggcgcgctcgggcagggcgccgggcaccgtcgggtcggtgtagacctcgaccacttgccacgtctcgcccgccgagcagccggaaagcgcggcggccgcaaggagtgcggcgagcgcgcggcgagacattagtccttctcggtggtcttcttggcggcctttttcgtcgtcttcttcgtggtctttttggtcgccttcttggtggccttcttcgtcgtcttcttcgtcgtcttcttcgtggtcttcttggtcgactttttggcggccttcttcgtggtcttcttcgccggcgcctcctcggcctccgccttctcctgctcgagctgctcggcgtagcgcttgtacacgaagcccttcggctcgacgcccagcattgacatcaaggtcacgccgtcgaagaaatcctccgcgtaggtggccacgatccgccgcgcaccagcggcggtctgctcctccatctcgatgacggcatcgggagctgggcgggagtccgtgatcttcggtggcactagaggttcctccttgggcgtttacgagatacttgggtcatggtaccgaaggtggcgcgcccgactcgcttcagcgcccggtagggcaggtactcctgcggcgcgcgcagccggcgcgccagccactcgccgaagaccacgcctccggcgagcgccatgcaggtggcgatggcggagaagatgttggtcagcccaacgaccatctgctcgttcatcacggcgtacatgccgcggtagatgcccgaaccaggcaagaacggggtcacgcccgcgaccgcggtgatgacggggctgatcatcgtgcgtcgcgcgatgagaccgccggcgaggccgacaaccatggcgcaggcggcggtggccatgaagcggtcggtgccgaacggaatgaggaacacgtagtagatggtggagccggcggcggctgtgatgaacgagacgaagatcgcgggcttttccgcgaagcacgtgactgcgaacgcggcggcggcggtggcgccgccgagaatgcgccagaccacgctgtcgagcgaaggtcggccgagcatcgtctcgatggggggcaggcctacgcccatcaggtccgaaaacgacagacccatcgctacgccgccaacaatgccgccggtgaacagcaccgtttggaagaagcgggcggaggcggtcacgggggagccggtgatgccgtcaagaagcgactggaccagcgtcaggccggcgagcagcaccacgatgccggaggcaatgacctggctcggcacgatcgtgcgcccgatgactgtggaaaagtcgtagaacactgctgcggggatcgtcgcaaagaagccgcccaccacgcagtggaaaaagtacggcaagttgttcctcgagagcaccttgttgaagcccatgatgaggaacgcggtgatgccgccgacgatcgacatcaagaagtctccgccgagcaagatcgcaatggccgcgcccatgaccgtccagccgaggaggaagcgggtgttgcggtagggaatcggggagttgtcgatgctgtcgaggaccttctcggcgacctccggcggcgtcgcacccgcgcggatggagcggatcaggcggtccgcctcctggagcttgtggtagttctcgctcatcatcgtcaccacgcggaacaccgtcaccggcgttcgcttgctgttgtgcacgatcaccgcgttcatagtgatggtgttcaccgtgatgtccacgtgacagtagtgcaggccgtacgaggaggtcacggtgcggatctgcgcaatggcgtccgaggaggtggtgccgttggcgatgaggatctcgccgatgcgggccgcgattgtcatcacagccgcgacctgcgtcgagtcggtcaggtcgaccggggcgagcactgatggtgggggcgaggtgcgggcggcgtcaatggtggccacgcgttgccgcgaaccgcgcagcatatccctcagagatgtcacgcgatagaccctagtctgtgcgtggttcgtcggcctgtgtaggctgttggagcattgctggagtggcgcaatcggtagcgcaacggtcttgtaaaccgtaggttgcgggttcaagtcccgtctccagctccatttcttcaacttgggtgacgcggtacagcgcgcgttcaggaaacatacagttgcggggtgttggattatcggaagttggaagtactgacctctgttcaaaggagatgacccccggatggctgaaaaccagggtgtgaaggtcctcgttgtagacgatgaaccgaatatcgtcgagctgctcaccgtgtcgctgcggttccaaggtttcgaggtggagagcgcgaattccggcgaggaggcgctcgagctggcccgctcgttcaagccggaggcgtacatcctcgacgtgatgatgccggacatggacggcttcgaactgctgaccaagctgcgctcggaggggctcgatggcccggtcctcttcctcaccgcaaaggacgcggtggaggaccgcatccacggcctgacaatcggcgcggacgactacgtgaccaagccgttcagcctcgaggaagtgatcacccgcctgcgcgtgatcctgcgccggggcaacgtcaccgacgacgcggagggcgacggcacgctgcgctacgccgacctcacgctgaacgatgagacgcacgaggtgaccaaggctggccagatcgtcgacctgtcgcccaccgagttcaacctgctgcgctacctcatgctcaacgctgaggtggtcgtgtccaaggcgaagatcttggacaacgtgtggcactacgacttcggcggcgacggcaacgtggtcgagtcgtacatctcctacctgcgccgcaaggtggaccagggtgatccgcagctgattcacacggtgcgcggtgtggggtatgtgttgagaacgccgcgtcaataagcaaaagcccctttgaccgcgatgttgattacccgggcttacgcgcagaaccggccgctgcagaagcggctggtgggcattgtcgtcggtgtgtcctcggtggcgatggcggtcagcttcatcatcgtgtacttcctgatgcgcgagctgttgtaccagcgcgtcgacgaccagctcgaagaagcgatgaacacctgggtggggcaaaccgcgtggctgcccacctacggcgcgccgagcgacttccaccaggcgattatggtgcctggctacagcacgccgtgggagccctcgcgcagcacgaccccgccggactacgcggagctgacgaagttcgaccagccgcagaccgtggggtcggttcccggctccgaattcaaccgccagtggcgcgcgatgaagcacgaagccaacggcacggtggagctggtggccaaaaagcttgaccaggaacgccgcacgctgaccagcctcgcgatgacggagagcctcatctggttcctcgccaccgtcgcgctggtctacgtcagccgccggcaggtgcagcgcgcgctggcgccgctgagggaggttgagaccactgcgctggcgattgccgacggggccaacaggcgcatccccgcttggtcgagagaaaccgaggtcggcaaactcggctacgccatgaataccatggtgagcaagctgcaggactctgtgaacgaggcggaggcgaaagaggagcaaatgcgccgcttcgtcggcgacgcctcccacgagctgcgcacgccgctgaccagcgtgcgcggctacgcggagctgtacaagaagggtatggcgcccgacgtggacatggtgctggacaagatcgaccaggagtccgcgcgcatgcagcttctggtagaggacctgctcgacctcacccgcgccgagggcgcgcgcctgaacacgcgcgaagtggacatgaccgagctcgtggcgagcgtggccagctccatccacgcggcgttcccggaccgcgagctgagcgtcatcaacgactgccagcgcgcgcccgccgtgcagggcgaccccgaccgcctccatcaagtgctgatcaacctggtcaccaacgcttacaagcacgccggcgcggacgcggtggtgacgatcaccctgcgagacaacttagacaggctgtttatcgacgtcagcgacaacggcatcggcatgcaccccgaggacgcggagcgcatcttcgaccgcttctaccgcgcggactcctcgcgccagcgcggtaagggcgggggctcaggcttggggctggcgattaccaagtcgatcattgagcagcacgacggcaccatcaaggtggccaccgcgccgggcgaaggctcgacctttactatttcgctgccaatgcctgcgtaagcttctgcgccgcctcgtccatcttcttctcgtcggtctggtcggcggggatggcgcgggacaggtcgtagccggacatgtcgtcggccggaaagacgtggatgtgcgcgtgcggcacctcgaacccggcaatcaggtagccggcgcgctcggagccgaagacctcaatgattgcctggccgatgtcctgcgcgacacggttcagcttcgcccacagttcaggctcgatgtcggtccacttgtccacttccttcaccggtacgaccagcgtgtggccgtacgccacgggctcaatggtgaggaaggcggcgacatcgtcgtcgcggtagataaaccggcccgggatctcgccttcgatgatcttggtgaatacggtgctcatacccttgcacgctaccggtaaatttgaggccatgcgcatccttgttatcggttcgggcggccgcgaacacgccctgctgaaaggccttgaaggccacgaacttttcgccgcgccgggtaactccgggatggccgcgctcgccgagctgcacccggtggacgtttccgacccggcggcgatcgtcgccctggccaagaacatcgaggccgaactcgtggtcatcggcccggagatcccgctggtggcgggtgccgctgacgcgctggaggacgccggcatcgcggtcttcggcccgtcgaaggcggcggcgcagctcgagggctccaaggcctttgccaaggacgtgatgcagtccgcaggcgtgcgcacggcgcaggccgcgcaggtcgcggacgccgcgggcatcgatgccgcgctcgacgccttcggtccgacttacgtggtgaaagacgacgggctcgcaggcggcaagggcgttgtggtgacaaaagaccgaaacgcagcgcgcgcccacgccgaagctgtgatcgccgcgggtaacccggtgctgctcgagtccttcctcgacggccccgaggtaagcctgttctgcctggtcgacggcgagacggtcgtgccgcttcagcccgcgcaggaccacaagcgcgcctacgacaacgacgagggcccgaacaccggcggcatgggagcgtacgcgccgctgccgtggctgccggaggacggggtggagcgcatcgtgcgcgagatcgccgagcctgtcgcccgcgagatggtcgcgcgcggcaccccgtaccacggtctgctctacgtcggcgcggcgtggggcgcgcagggcccggcggtgatcgagttcaacgcccgcttcggcgacccggagacccaggcggtgctcagcttgctggaaaccccgctggtggacgccctaggagcagttgcttatcgacgcctcgcccaactccccagactgtcctggaaacccggctacgccgcgacggtggtgctggccgcagagggctacccggccgcacctgtgaccggcggcgcgatcacgggcgagccgctggcagatcccgagcgcgttctccacgctggcaccggcaacaacggcggcgaggtggtcgccgccggcggccgcgtgctcaacgccctcggctacggcgagacgcttgaagatgccgtcgctaacgcttattccgtgctcgaccagatcgaactggccggctccttctaccgccgcgacatcgccctccccgcgatcgagggtcgcatccagcttccggaaaggtaaacacccatgcaaaaacccgcaaacgccaacgtcttaagcaaccgctacgcatcacccgagatggccacgctgtgggcgccggagcacaagatcgtgctcgagcgccagctgtggatcgctgtgcttcgcgcgcagaaggagctcggtgtcgaggtcgccgacggcgccatcgaggcctacgagtctgtcatcgaccaggtggacctggccagcatcgctgagcgcgaaaagatcacccgccacgacgtgaaggcgcgcatcgaggagttcaacgcgcttgccggctacgaggagatccacaaggggatgacctcgcgcgacctgacggagaacgtcgagcagctgcagatcgtccgctccctcgaactgacacgcgacaaggccgttgcgctgctcaaagccgtgggcaaccgcgccggcgagtacgagtcacttgtgatggcgggccgctcccacaacgtggccgcgcaggcgaccaccctgggcaagcgtttcgcctccgccgccgacgaggtcctcgtcgctgtggagcgcatcgaggagctcatcggccgctacccgctgcgcggcatcaagggcccgatgggcaccgcccaggacatgctcgacttgatgggcggagacgaggcgaagctggcggagctcgagacgggcatcgcgcgcgggcttggcttcgaccgcgtcttcgactccgtggggcaggtctacccgcgctcgctcgacttcgatgtggtgagcgcgcttgtgcagctgggtgcgggcccgtcgtctttggccaccaccatccgtctgatggccggcaacgaaacggtcaccgagggcttcaaggagggccaggtcggctccagtgccatgccgcacaagatgaacgcccgctcctgcgagcgcgtgggcggtttccaggtgatcctgcgcggctacctcgcaatggtcgctgacctggctggtcagcagtggaacgagggcgacgtgttctgctccgtggtgcgccgtgtggcgcttcccgacgcgttcttcgccatcgacgggcagctggagaccatgctcaccgtgctcgacgagttcggtgccttcccggcgatgatcaaccgcgagctggaccgctacctgccgtttttggccaccacccgcatcctgatggcggcggtgcgcgcgggcgtgggccgcgagaccgcccacgaggtgatcaaggaaaacgctgtcgcgatggcgctcgacatgcgcgagcgcggcgccgagcagaacttgatggagcgcttggccgccgacgagcgcctgccgctcgaccgcgatcagctagacgccgccctcgagaaccgccacgccttcatcggcgctgccgagtcgcaggttgagcgggtgcgcgcccgcatcgaggaggtcctccagcgccacccggaggcggccgactaccgcccgggcgacatcctctagccgctactgccaggtgacagtctggtcccgggtggaaagcttcaccccggtgccggcgatgccgtagagcccgtcccagctcgcgacgtaaaaggagtactcgcggccctcgcgcatctccccggtgtagccggtgggcgggttgacgtcctcgccgcacagcgacgtgtcgttgaggtagttggcgttctcgtcgccgttgacaggggtgaacctcggcagcgggaccgtcacgtccaccgggtagtcgccgatgaaggtgggcgtcatccgcaccctgttgcacaaggcctttggaaaggttggggtagcagggacgagcttcggcttgtcgacgctcacctcccacaacaccggcaccccgtgcccaacatcgcgtgtgagcacctccgccggtttgccgtaggagcgggtgagctccgatcggactttcgggatctcgccggagtagggcgccggcggggcgcaagcgaccagcgcaaacgtcgcggcggccgctgcggcggcgtgacggcgggccccttttcgcatgcgtcggagcctaccaggcatacacttggaagccatgcgcgcagatttgtctgactacaagcacctggccggcggcaaggtccgcgagatctacgaggttgactccgacacgctgctcatggtcgcctcggaccggatctccgcgttcgacttctcgctggagcccgcaatcccggacaagggcaggatcctgaccgccacgtccatgttcttcttcgatcttctcgacgtgccgaaccaccttgccggcccgatcgacgacccgcgcgtgcccgactccgctttgggccgcgccatgctggtgaagaagctcgacatggtgccgttcgagtgcgtcgcccgcggctacctcaccggctcgggcaagaaggagtacgatgcccgcggcaaggtttgcggcgtcgaccttccggagggcctgaaagaggcctccaagctgccggagccgattttcaccccggctaccaaggcggagcagggcgaccacgacgaaaacgtcaccttcgactacatggccaacaagatcggcaccgaactggccgacaagctccgcgagctcacgctggccgtctacacccgcgccgccgagcacgccgagtctaagggcatcatcctcgccgacacgaagctggagttcggcatcgaccaagacggcaacgtcgtgctggctgatgaggtgctcacccccgattcctcccgctactggccggcggacggctacgcggagggtcaggtgcagcccagctttgacaaacagtacgtgcgcaactggctcaccggcccgaaggcggactgggatccggcatcgaacacgcagccgccggagctgcccggctccgttgtggaggcgacccgcgaccgctacatcgaggcctacgagcgcctttcgggcaagcgcttcgcggattggccgggaagcaaagcctagactcgacgtctatggcatcaacgcacatcaacccacctgagccagccaagcgaccagtcacccgcgccttccacggccgcgagttcgtcgacgactacgagtggctgcgcgataaggacaatcccgaggtcatcgctcacctcgaggcggagaacgcctacaccgacgcgatgaccgaagacctgaaaccgctcacggacgcggtgtacggggagatcaagtcgcgcgtgaaggaaacggacatgtccgtaccgcagcgccagggcgactggtggtactacggccgcaccgaggagggaaagagctacgccacctcgtgccgcgtgccggtcgccggcgacccgtgggccccgcccgaagtcacggacgacatgccgggcgagcaggtgctgctcgatttgaacgaacttgcggacggccacgagtttttctccctcggcgcctcgtcggtttccacgtcggggcgcctgctcgcgtactccgtcgacaccgagggcgacgagcggttcacgctgcgcatcaaggatcttgagggcggttcgctttacgacgaccacctgacagacatcttctacggcgccgtatgggccggcgacgactacctcttttacatccgcgtcgacgaagcgtggcgcccgcaccaggtgtggcgacacaaggtgggcacgcccgagtcggacgacgtgcttgtgtacgaggaaaccgacgagcgcttcggtgtcggcgtgggtgccgaccgcgcggagcgctacctgttcatcgcgtcagcatcgtcgctgaccagcgagtaccgcgtcgcgcccctggacgacccgaccgcagactttcaggtcatgtggccccgcgagcccggtgtggagtaccacccggattacgcccaggtgggcgaccgcgattactgggtggtcacccacaacgccgcagggcccaacttcgcagtaggcgtgtgcccagtcggtgagctgccggcgctgacggagctcgacacgattctcgagcactcggagaccacccgcgtggagggcgtcgacacgtaccgcgacttcatgttcgtcagctaccgtcgcggcggtatcgcccgccttgcggtggcgggactgactgacggtttcggcggctggcacgagcttgagttcgacgaggagctctacacggcatccctgatcggcaacccggagtgggacgcgccggttgtgcgcatcggctacacctcgttcaccacgccgtcgacggtgctggactaccgcgtgggcagcggcgagttcaccaagctcaagcagcaggaggtgctcggcgggtacaacccggacgagtacgaggcgttccgcctgtgggcgagggcttcggacggggtagaggtgccggtgtcggtggtgcgtcgtaaagcaactgcccctgggccgcagccgaccttgctctacggctacggctcgtacgaagcctcgaccgacccgggcttttccgtggcgcgcctgtcgcttttggatcggggcatggtgtgggcgtgcgcccacgtgcgcggcggcggcgaaatgggccgcacctggtacgacacgggcaagatgctgcacaaggtcaacacgttcaccgacttcgtggcgtgcgcggacatgctgatcgatgggggctacaccacgcctgcgcagatggtcgccgaaggcgggtccgcaggcgggctgctcatgggcgcggtggcgaacctcgccccggaaaagttcgcgggcattcaggcgattgtgccgtttgtggacccgctgacctccgtactcaagcccgaactgccgctgactgtgggcgagtgggaggagtggggcgacccgtaccacgacccgcaagtgtacgactacatggcggcttacgcgccgtacgagaacgtctccgcgcagaactaccccgcgatcttggcggtaacctcgctgaacgatacccgggtgctgttcgtggagccggcgaagtgggtagccaagctccgggaggtcggccgcggcggaccgttcttgctcaagacggagatggccgctggccacggcggtgtgtcggggcgctacgcgaagtggaagcagaccgccttcgaatacgcgtggacgcttgctacgtccggcgcggttgacacgagtgtggaaaaatagggcccatgcctggccgcctcctcgtctccgtttcctcgatttttgatgaaacgttgcccggggtgcaggccctgatcaacgagctggaccgcgaggacgtcccggtctcgctgctggtcgccccgcacatcgacaaccggtggcacctggcgaaggacaagcacacgcgcaagtggctgcgcgaccaggcggggcagcgcgcgatgctgctcaacggcttcgaccaggcggtgcagggacggcgcgccgagttcgccaccctcgagcagcacgaggcgaagttgcggctgaagggggccactcgccagatggagtcgctgggtttcgacttcgacatgtttgccccgccgcgctggcagatgtccgcgggcacgcttgaggtgctgccggacttcgggtttgacgtcgcggcgtcgacaaagggcatccaccacctgctcaccggagaattcacccagtgccgcaacctgtctgttggcgagggctacggcgcggcgaagtggtggcgccgcaacatcatcaaggcggcggcccgcggcgccgagcgcggcaacacgatccgcctgtccgtttccggccgcgagctgggtacgaagaaggtgcaccgcgacttcgtggccgcggcccgcgaggccgttaaggccggcgcggaaccctccgactaccgtgcctaccaataatccggcacaccaagtagatcccgaacgagataaacgcgacgaacacgctgaccggcacgccgggcgccagcgacaaaatcatgccgccgaccgcggcgacctcggcgaaaataaccgagtaaagtaccgcgagcttcgggttcgcggtgatctgggcggctgcagcgccgggcgtgatcagaagcgacatgaccagcagcgcgccgacgatctgcacgctttgggcggacgcgacgccgacgagcacggcgaaggtgagcgccatggctttgacgggcacgcctgccgcagcggccatctccgggtcggcggaggcgaacaggagggggcgccacaggacaaccaccgcgccggcaaccagggcggtggtgagtccgagcaggacgaggtcttggcctgtcacgccgactatctggccggtgagcagcgcgagcgcgcggttggcgttgccggggtagaggtggatgaacagcacggataagcccataccgaaactcatgaccacgccgacggcggaatcctgctggcctttgagcccgagcgctgcgagcacgaccgcggcgacgacggcgccgacgatcgcgcccaaaccgacgttgatgccggtcagcagggcggcggaggcgcccatcagcgcgagctcgctcgtcgcgtggacgctgaacgacatctgcctcagcacgataagaggcgccatgacgccggagagcacacccagcagcgcgcaggcgataagggtggcctggacgaaatcgagggaaagcagttcaagcgtcgtcacaggaccacaagcttcccgtttacttctgcgacgtcgacgtgggtgccgaagagatcgctaagcacctcgctgcgcatgacctcgtccacgctgcccaagacgtggccttgaggcccgatgtagaggacgcggtcgacgacgcttagcagcgggttgatcgagtgcgtgacgcagacgaccgcggcgcctgagtccttcaaccttcttgtggtttcgtgttggcgggcggggtcgagggagagcaggggctcgtcggcaagcaagagctccggatcctgcgcaaacgcctgtgcttggcggatgagctgctgttgcccgccggacagtgtgccgacgcgctggtcggcgaaactgcgggcgccgacgaaatcgagcagcttatcgacgccctcggtgcgcccaaagggtctcgggttcacagcgagcgagacgaggtcgcggccgcgcatcggcagatccggcgggaacatgcgctgctgcggtatcagtccgatgcgtccgctgacgctgacagtgccgctggtgagcgagcgcgtgcccaggaccgtgccgatcagggtggacttgcccacaccgttcggcccgagcacggcgaggaactcgccacgctccagctcgagattcaagttcgaccagagggggtcgacggcggcgccgcgaaacgaaaggatcactgtgcggattctacgagcgcgtccgcgatctgctcaacgtagtccagcacgctggtgccggcgggtggaatctcggtgatctcgacgatggtggtgttgtgcgatttcgcggcgtcgacgatgcgctgcgccgcgctggtcattgactgggggttgacgatcagcacatcaacgtggccgttctcgatctcctggatgaagtttgctacagcgcttgccgacgcctccccgtgattcaacgccgccttcctgtaatcagccggcgtggtgtcgtgcatctcggatccggcaatcaggtggtctgcgatcgactccgtctgcgcgacgtgcaggtgtggcaggttgccgatcttctgcttgagcgcggccatgcggctttccacctcggtcgcgtcaccgcccactttcgcctcaacctccttggccacggcggtaatcgcgtcgggggagaaccagacgtgctcattcacgctgtggtcgtggtggtcgtggtggtcgtggtggtcgtcgtggccgtggtcgtgcgcgtcatcgagacctgcgaggtcgaacgcgttgatcacccggtcttgctctgcgacctcgtagagggccgcgtcgtacccgccgccgttggcgataacggtgttggcggctttcactcgagcgaggtcctgagcagtcggctcgtagtggtgggggtcgatactcgtgccggtgaggatcgcgggtacgtcgttcccggtcactgcggaggcgacgtcggcccagacgcctgtggtcgcgacgagttctgcttggtcgctgctggtcgtgccgtcgcacgccacaagggttaccgcgaggagggggactgctgcaagggtgggggtgattcgcatgcgcaaattttaagcactaatgaaaatcgttttcaatttgagtgtggggtaaaaacgcgagaactccacccccgcgcagggaggtggagttctacggctgcgcggtgttagttggaagaaccagcgtcaccgcacgcggagaccagcgttgcgatcgcggcagcgccgagggagatcgccgccaggccggtaagggcctgaaccgcgccgatgcccatgctgctcagctgctcagcggtcaacgcgagctgcgggacgaagacgttgagctgctgctgcgcgagggtgttgagctggttgacctgatcctgcaccggttggagcgccgggatgccgattgtcgctgcgaggccgagcggaaccagcgcgaccagcggcagaccccagccgacagctgcggcgatgcagcggccgttagaggaggcgttcgttcccggagccggggccggcgccggcgtggagccggtgaccttgccgaggttctgggtggtgccgtcggagtaagtgagcacgagctcgccgttgtcgttgacctccgcgctggtgacgccccgtccgtcggtgcctggctgggccgcgaccttgcccaagttgctggtctcaccgtcgctgtaggtgatgatcagatcgccgtcgttgttgatgacagcatccgccacgaagcgtggcttgttcacgttgacggtgacctcgacgctgtcctgactgccgtccgggtaggtgacaagcacagcgcgcttttgaccagcgcctggctgatcggtctttgcgtccgaccactggaatgtggtgccctcaggcaatgcgtcagcgttcttgatcacggatttcgcctccggtagctcctcgttctgagtcaccgtgatcgcatcgccggactccggctcgtgctgatctttctcgcgctcggggaagctgatgccgaccttcaccgggtcgtggtcggaagcagcgaacgggttgtcgttctggaagagatccgcaccgtggtagttgcggcgcgagtactggaaaacaatcggctcgtccgcgttaatgttccacaccgccgcatcctggacgagtgcgcgcgcagcctcgtttgcgagcacgtggtcgagggagccaacgtgcttgccgaaggagtaggacgactcttgtgccgcggcgccggcgccagcgacgttgtgctcggcgttgtgctcaacgatctcgaatccgccgccgttgagcgccgtgatggaatcctcgcgcgagtacgagttcaggtcgccgaggatgaagactggtttgttgtcccactggttttgctgttgcaggtgatcgagcagcgcctgcgcttgggccttacgcacgttcgggttgttggcctggccatcgttttggtcggcatcgccccgtgccaccgatcccttcgacttgaagtggttcacgatcgcgacgaagctttcgtcgtcggagccgcccttgggcttgaattcctgtgccaacggttggcgggcggtccctgtaaacgcggggtcgtcaaaaatgacggattcgccgaccggctcaaccttgtctttgttgtagatgaacgcgacgcggatgaagtcctcattggtgccgagctgcgccggcgacttgacgtagtcccaggtgccgccagcgtcgttaagcgcctcaacaagtttcccgagggattcgtcgcgcttggcaacgtcgccggaggtcttcgccgtgttctcaacctccatcaggccgacgacggaggcgtccagctcgttgatggccagcacgatcttgtcctgctggtccttgaacgcgtcttgggtgaacgcgccgcggacgttgcagcggttcgcagcgatgtcgttgccgaaacggtcctggtacgccttgcagccagcttcggtctcgccgagggtggtgaaatagttcagcacgttgaaggaaccgatggacagatcgcccttgacctggctcggcacattgcgcactgcttcgcgggtatctgcccactcgaccgggaggtcctcctccgggctcttgccggtgagcggcacgagcggctggaagcgccacgcgttgaaggagtactcgacgatgacaccggagtctttaaactccagttggtcgccgacgcgcatcgacttgatgcccttgtcggaggtttggaggtagggaagcgggatgtctttgttgttgcggaagtagttgtaggtggaagcgtcgtcaagcaggatgatgctcttgagctgctcctgctcgagcgcgtatgcctcctcgccgggcgccatgacgtcggtcggttggcgcaggggctcttcgcccgggacgatgcccatctcgccgtaggtgttgaagctgtagttgtccgtcaccgtgtggactccgggcttgaccagcatgccttcgtagcgttcgcgcgcctcgtcgccggcgggcagggagtcgaactcaacaggggtgaccggttcgaaatcttcgttcagtgcggtgatcctggggccagacagctgcgtggaggtgttgaactcctcgaccttgccggtgacctcgatgtaggaaccacgcgcagggtaggtctccggttttgcgcccttgcccatgtagacaaagacagcgtcagatgcgtcgccgtcgtttttcaccttgcccgcgccgggggtctgcatgtagaagccgtcgcggccgccctcgttgtacaccgcggtgacaacgccgcgggtggttaccgtttggccctcgagcggagaggaagcgcccggaccctgaatgtctgcaatggtgactggttcggtcggctgcggctggggttgcggctggggatcggtcggatccggattgttgggctccggagtctcctcgccgttcgatgcgcccggggtcggggcgtctactttgaaatcgttcgcgttgttgtcggtgtcaacgccgtcccgcttgcgctgaactgaggtgccgttgttcgtgcctgcagcaggggagtccccttcggcttccttggcagcgccccacccaaggaggtcgactacactgccgttggcgtcgatgagctttgcaatggcctgcttgcctgcgaaatcgaaattcaaaatttgatctggagccggcagctcaccggtagcgttgttgcccgcccaaccttgcacaaggaagaaagattttggctgaatcgtgccgttgagcacgtgcgggtgacggcccccctttccgccgtttgcggagtactgctcaatctgccacccggtgatgtcaatcggggcgtccgtcgggttatagagctcgacgaagtcgttggagtacacggaaccgctgttaccgccgcctccgtaaacctcgttgatgacgacgttggtgccgtcaacggcggcggaagcggaaggagcgacgacggaaacggtgccggctgcgagcgcgatggcgaacgtcgcactaagtgccttgcgattcgagttacgcatgggaaacgaacctctcgtggatagctaggtggccagtaagggaagcggtgcaaagcttgcaccgccaaagtaactccgctagacggcgtacgggcggtctactgacagggttctccaacagttcacccaccgtttaccgaggctgttccgagggcctttgggctgtgtggtggctcggatatacttatcgccgacctaatacaggcgtccaacctccctcaacacgaaggattctcatggcacgagtcgtcgtcaatgtcatgcccaaagccgaaattctggacccgcagggccaagcagtgctgcgcgcgctgggccggatcggggtggagggtgtcaccgatgtccgtcagggcaagcgcttcgagatcgaggtggatgacactgtctccgatgaggagctgcgccgcatggcggagaccctcttgaccaacaccgtgatcgaggatttcgaggttgtgcgatgagcgcaaccatcggtgtaatcacgtttccaggcacgcttgacgacgttgacgcgttgcgtgccgtgcgcctcgccggtgctgagcccaagcagctctggcacgcggacgacgatctgactggcgtcgacgcggtggtcgtccccggtggtttctcctacggtgactacctgcgctcaggcgcgatcgcagcccaagcaccgatgatgggcgcggtgatcgaggcagccaagggcggtatgccggtgctcggtatctgcaacggattccagatcctcactgaggcgggtcttctgccgggtgcgctgacccgcaaccagaacctcaacttccactgcgtggacacgtacctcgaggtggcgaacacctccaccgcctggaccaccgagtttgatcagggccagcgcatctacgttcctgctaagcacggcgagggccgcttccaggccgcgcccgaaaccatcgaagcgctggagaaggagggccgcgtggtcttccgttataccgacaatttcaacggctccatcaacgcgatcgccggcgtgaccaacgaaactggccgcgtcgtcggcctcatgccgcacccggagcacgccattgaaacgctcaccggcccgtccaccgacggcctgggcctgttcacgtccgccatcaacgctatttcgaagatcggagcgtaaaacacagatgactgtggtgaatgacaccgtcgaaaacgcgaaggcgaccccggatacggtgcagccctacgccgagctcggcctcaaggacgacgagtaccagaagatcaaggacatcctcggccgccgtccgacggacgccgagctcaccgtctactccgtgatgtggtcggagcactgctcctacaagtcttcgaaggtgcacctgcgctacttcggcgagacgatgacggatgaaatggcgtcgaagatcctcgccggcatcggcgagaacgccggtgttgtggacattggcggcggcgacgctgtgaccttccgcgtggagagccacaaccacccgtcgtttgtcgagccctaccagggcgcggcgaccggtgttggcggcatcgtccgcgacatcatggcgatgggcgcgcgcccgatcgcggtgatggaccagctgcgcttcggccccattgacgccgacgacaccaagcgcgtgctgccgggcgtggtgcacggcatcggcggctacggcaactgcctcggcctgccaaacatcggcggcgagacggtgttcgacgccgcctacgccggcaacccgctggtcaacgcgctgtgcatcggcacgctgaaggtggaggacctccaccttgcgttcgcgtccggcaccggcaacaaggtgatcctgttcggctcccgcaccggcctcgacggcatcggcggtgtgagcgtgctcggctcggccaccttcgaggagggcgaggagcgcaagttgccggcggtgcaggtcggcgacccgttcgcggaaaaggtgctcatcgagtgctgcctcgagctttacgcggctggcgtcgtggtgggcatccaggaccttggcggcggcggcctgtcgtgcgccacctccgagctggctgcggccggcgacggcggcatgcgcgtcgacctcgacgctgttccgctgcgcgccgagaacatgaccgcggcagagatcctggcctccgagtcgcaggagcgcatgtgcgcggttgtggctccggaaaacgtggacaagttcatggaaatctgcgccaagtgggacgtgggcgcggccgtcatcggtgaggtcacggacgagcacgaccgcctcgccgtgtaccaccagggtgagctggtgctcgacgcgccgccgtcgacgattgacgcgggcccggtttacgagcgcccgtttgcgcgcccggattggttggacggtgtgcagggggaagggggcgtcgataagcacctgcccctgaaggacacctggttgaagatggttgcttccccggcgctgtgctcgcgcgacttcatcaccgagcagtacgatcgctacgtgcgcggcaacaccgtgcaggcaaagtacgccgattccggtgtgctgcgcattaacgaggagacgaagcgcggcgtggcagcgtcggccgacgcgtcgggccgctacacctacctggatccgaacatgggtgcgcgtcttgctctggcagaggcgtaccgcaatgtggctgtcaccggcgcgaagccggtcgcggtgaccaactgcctgaacttcggctccccggagaacccggacgtgatgtggcagttccgcgaggcggtgcatgggcttgcagacggcgcggccgaactttctatccccgtctccggcggcaacgtgtccttctacaaccagaccggcgagaccccgatcctgccgaccccggttgtcggcgtgctgggtgtcattgaggacgcggagaagaccatcccgcacgcggcacccgcgggcgaggagtacacgctgatcctgctcggcgagaccaaagacgagttcggcggttccgtctggcaggacatctcgggagccggccttgcgggcctgccgccgcaggttgtcctggccaacgaggcgcggctggcggagtacttcgccgagccggagggcatctcggccgcccacgacctctccgagggcggtttgtctcaggccctgttcgagctgctgctcggctcggacttgggcgcggagatcgacctgtcggtggtccacgaggacgcgtttaccgcgatgttctccgagtcagcttcccgcgtgctcgtcgcggtgaccagggaccgcgccgacgccgccgtggcgcgcgcgacctccgccgggatcccggtggcggtgcttggctccaccaccgaggacggcgtcatccgcttcagcggcgaggagatcgccgtggctgagctcgccggcgcgtgggcggccaccatgccgggccacttcggacacgcgacggcgccgaactcggcggtttagtccacgcgctgggcggcctcgggcagccgcaccagcggcaccggctcgtactggccgcgcagatctttcagggtctgcgtgtgctcccagagccgcttgtcctcgtccgtcaccggggtgaactggcgggcgggcagggggtttccgtcgatgtcgatacccaggtacgtcaccgaggcgtggatggcctcggtgagctgctcctgcccgccgcgcgggtcgccggagcgcaccgagatcgaggtgtgcaacgaccgggtgtcggtgcgggtgagccgcgcctcaacctcgatcaaatcgccgatgtggatcggcttgtaaaagcggatgccgcccgcgtacaccgcgacggtgcgctcgcccgaccattccatggtgcaggacaaaccggcctcgtcgatccactccatcgccgtgccgccgtgcacgttgccgccccagttcacatccgtcggcttggccaggaagcggtggatcgtgcgcggggcggtcgaatcgcgcgtgtaggtctgctcgctcatctcttgctcgatcgccttgcgcagctcgatgcgcgacagggcggcctcagccacgcggcgctcctcgtcgtcggagggaacgaacgtgggcaccggcgtgggccggccagtagccgggtccttcgccacgaaaatcaccaggcagtcgcacgcgcgggtgaatacgccctggcgcgggtcggcggaaagcacctcgttgacaatgtgcatcgaggagcgccccgtcatcgccacgcgcgagcgcacctccacgatgtggccggaggggatcgggcgggtgaagtggatgtggcccacgtacgcggtcacgcagtacgtcgacgaccactgtgccgcacacgcgtaggcggccttgtcaatccactccagcacgcgcccgccggcgacgccttgcgcgccggcgtgcagcacgtcggtcggcgccgccatgaagcgcagcgtgatggagggggatttttcggtcggcacagcggtgttcggcatagccacaccttaaacgcttggggttaccatctgcgctatggctacgaagaaggtcgatccgcacgaaacgcgcgccgcggtgcgcgctgttgaggcatggcttaaagacgcctcgttacccgccccggggcgccaagccctggcagcagcgtgccgcaccaccgcacgcacgcttgcggaggagttgcccggccacaccgttgagctgcgcgtcccgccgttcgtcgcggtccagtgcatcgaaggtccgcggcacacgcgcggcaccccgccgaacgtggtggagtgcgacccgcgcacgtggctccgtctcgccacagggctgaccgacttcgacgcggaagtcgccagcggcgccgtggatgcctcgggttcgcgcgcgggtgaggtcgcccgcggcttgccggtaattcctttgtgagggcccgagtccgatacagtggtgggtgtgcatgacctagtcaatcagggtgcaaatcagcaaaacgatgagccgcgcgaggagtgcggcgtcttcggcgtgtgggcgccgaaggaagacgtgtcgaagctgacctacttcggcctcttcgcgctgcagcaccgcgggcaagagggtgccggcatcgccgtcggcgacaaggaaaacatcgtggtgtttaaagacaccggcctggtaagccaggtgttcgacgagtcggcgctggacgctttgcagggagatgtggccatcggccacacccgctactccacagccgggggcaactcgtgggacaacgtgcagccgatgttccgcacctcgccgaacggcaccgacgtggccctcgcccacaacggcaacctggtcaactacatggagctgcagcacgaggcgattgccaagaagctcatcccggccgctggggtcaagggccaggggtcgagctcggatacggcagttgtttcggcgctgctcgccgatctaatcaccgaagagcattcgcttatcgacgcctgccgggaactccttccgcgcatccgcggcgctttctgcttcatgatcaccgacggccacaccctctacgccgcccgcgatccccacggcgtgcgcccgctttccctgggccgcctcgacgggggctgggtcgtggcgtctgagacctgcgccctcgacatcgtgggcgcgtcctttgtacgcgacatcgagccgggcgagctcatctggatcgacgaaacgggtgtgcattccgagcgcttcgccgagacgccgaaggcgcactgcgttttcgagtacgtctacgtcgcccgcccggattcggtgatcgagggcaagtccgtcaacgccgcccgcattgagatcgggcgcaggctggcaaaggtccgcccggttgaggcggacttggtgatgccggtgccggaatcgggcaccccggccgccatcggttacgccgaggagtccgggatccccttcaaacagggcatgatgaaaaacgcgtacgtgggccgcaccttcatccagccctcggacacgctgcgtcagctgggactgcgcctgaagctcaaccccgtgcgcgaggtcattgagggcaagaagctggtcgtggtggacgactctatcgtgcgcggcaacactcagcgcaagctgatccgcatgctgcgcgaggcgggtgccgccgaggtgcacgtgcgcatcgcgtcgccgccggtgaagtggccctgcttctacggtattgacttcgccagccccggcgaactgatcgccaaccacggcaaggccggcaccgatgcggaagtagccgaatccatccgcacgatgatcggcgccgactcgctcgccttcgtcccgatcgacgacatggtggaggcgactacccagccggcggaaaacttgtgcgcggcctgcttcaccggcgactatcctttgggcctgccggacggcaaccccaacgcagaccttgtccgacgcatccagaaaggtgcatagagcctccatgaccactcctgagaaccaacaccccgtctcgtacgaggctgccggcgtgtccatcgaggccggcgacaaagcagtagagctcttcgcgccgcacgccaagcgcgccacccgcccggaggtccgcggcggacttggcggctttgccggcctgttcgcgctgggtaagtacaaggagccgctgctcgccgccggttcggatggcgtgggtaccaagcttgccgtggcgcaggccatggacaagcacgacaccatcggcatcgacctggtcgcgatgtgcgtcgacgacctcgtcgtgtgcggcgcggagccgctgttcctgcaggattacatcgccatcggcaaggttgtgccggagaaggtcgcggagatcgtgtccggcatcgctgagggctgtgtgcgcgccggttgcgcgctgctcggcggcgaaacggcagagcaccccggtgtgatggacgccgacgagtacgacgtttccgcgaccgccgtcggcgtggtcgaggcagatgagctgctcggcccgcaccgcgtgcgcgagggtgacacggtcatcgcgatggcgtcgtctggcctgcactccaacggctactcgctcgcccgccacgtgctgctggagcgcgccggcctgccgctcgacgggcacatcgaggagctggggcgctcgctcggcgaggagctgctcgagcccacccgcatctacgcgctggactgcctcgagcttgccgccgagtgcgaggtgcgcacgttttgccacgttactggcggtggactcgccggcaacatggaacgcgtcatccctgaaggtctggtcgccgacatgcaccgcacgtcctggacgccgagccagatcttccgcaccatccgctcgatcggccaggtgccggacgcggagatggagaagaccttcaacatgggtgtgggtatggtcgcgatcgtcgctcccgaggaccgcgaccgcgcgcttgcgatcttggcggcgcgccacattgacagctgggtgctcggcgaggtgcgcgcggccgctgagggcgaaactgcccgcgcggtgctgaccggctctcacccgcagtactagcaaaggagcgcaccccggccggggtgcgctcctttattgctttggtggtgagatcctagcgggcgactcggtgatcctcgccgtcctcgtcatcccaggcgccgtagtttgcgtactcgtcgtactgggaatccacctcgtcctcgtcgtcccatccggctgccggtgcttgacccgcaagctcccgctgcagcgaatcgagatccatttccggagagttgtacttgagctggcgagcgaccttggtctgctttgctttggcgcgtccgcgacccatggcgtgacccccttgaggtggtattattcgatacgtttttgtcctgccagacataatagcgggtagggcaaaaaaattcccttccggcccccgagctgcgccgacgccgcaaacctgcgttaccggcctcgcagcgcgtccaccgcccggcgcccggcgcgttcgccctcgtcggtgggcagcgagtcggggtccacgcgcgctgcggtgccgtcgacgtccagatccaccgcggtggccgaaccgtcgccgagcgcagagcgcttcaccagcgccagcgcgatggggccgtagtcaacgtcgtggaccacggtgccaaggcggcccacagcgcggccgttcaacgtaaccggtgcgcccggctccggctgggtgggcgaggagccgtcaagttgcagtgtgaccagaaggcggggggagcggccgaggttctccacgcgcgcgaccgtctcttggccccggtagcaacccttgttcaggtggacggcggctggttcggcgccgcgggcgatgaagcgaggcacctcgtggggaattgccttggcgtctaagtcgcggtggatttccggctcgacggcgcgcacgcgggcggcctcgtacgccatgaggccggcgatgtcgaaaccggcagaggtgaagattgagggggagggagaggggatgagagcgtcggtaagcagcaatgccccgaacgccgaagtgcggatggcggcggcctccggaagttcgggagcgctaccgcgggggctgaggacggaaacgagctgcaggtcggagtcctcgatggtgacgtcggaccagaacaccatgcggcgcacgtagtcggtgaaggattcgtgctgctcggagggcatgtccaggtagaacgtggtgccgtcgtacatcacgccgacgtggtgcaggatgcggccttgggcgtccaggtcgagcgcgaagccgccgaaactggcgggcgcgtcgtcgagcttctgcgtgagcaggttgttcaggaacgtgggcgcgtcggggccggaaacctccaccacgcgccggtgcgaccggtcgatcacagccggtgtggtggcgaggcgccgctgctccgcgagcgggtcgccgtaatggagggcaacgccagtttcggggtcggggacagcgccggggagatcgagaaattcagacacgatgcccgatcttaagggcataatgggatgctatgtcgctgctgcctccggaacccgtgatttacctggtagagccgttcggcggttcgattcggcggcagaaccccaacatgccgcacgtgtattgggacgatgcggcggtcacccgcggcgacggtgtgttcgaaaccatcctcgtgcgcggtggcgaggcccggaacctgggcaaacacgtcgagcggttccagcgttccgcgcgcgccctagcgctgccggaaccggacgcggagcattggatccgcgcgacgacagaagcggtggcggactactgccgcgagcacgcgggcgcccaggcgcaagaagatattgaggcaaagtgcgtgtggacgttgacccgcgggcgcgagaccacaggggtcgcgtcggcgtggctgacggtgcggccgatcccagaggacgtgcttgcgcagcgcgagcgcggcgtcaaggtggtgactacaccgcgcgcgttcgcgccgaactcggatgtccagtgggccggggcggaggcgaagacgctgaactacgcggcgaacatggcggcgctgcggtgggcgaaaacccagggcgcggacgacgtgatttacgtggaagcggataccggtcgcgtgctcgagggcgccaccagcacggtgctcatggtgaaaaagggccagcggatgcgcacgccgaaacccgaggccggcgtgcttcgcggcaccacccaagccgcggtgttcgaggacgcggtcaagctcggctggaagtgccgcgagaaggacatctacgtcaacgaactggcaaaggccgagtccgtgtggctggtcagctccacgcgcatctgcgcgcaggtgacgcacttagacggcgtgaagcttgccaaacccggcaacgaggcggagatccgcgagctcattgccggcgcgctgcgctagccggcgacgcgcttgagctcggcggacatgtatggcaccagctcgccgtccaccacgcgctcgtccacccagccgaggttgttgttcggcatcaggccgtaaaggcgcttgcccgggccgtggtcgaccgggccgcgctcagttgcgatggtggaggcggattccagctgccaggcgcgctcgttgagcaggctgccgtagagcacctccaccaagccgcgggagttggtcaaggtgacttcgatctcgtccttctcggagatgcgccagaaacccacctcgcgctggtcggccccggtggattcgccttcctcgttcaggcgccactggcgggattcaaagcgcaggtaatttccgccgtcgtgggaaatcaccagctgctggccgaaggcgtactcctcgccgtggtcgttggcctcgccggtgccctgccagacgccgacaagggggaggagggctaacaggccgtcgtgaagcgagggcccctggcgcaggtttgctgtgtcgtcctcgagcggaaagccctcgaaccccaaccccgggatgttcttgtcggcggtgtgcttcgactgctcggctgcgaggttgaccgcagcggaaccatctaacttttcgttttcagtcatagcaaccaagggtagcctggctgcatggatcacatggagatcgtccaagccgccgaggcgcacgacggtgtcgcgccgctgtcagagcagttcctgcggggattgaccgatgaaagcctcggccacaaacgctacgaggtggaaggcgggtttgcggcggttgcgcctgacggagcggtggagctggtggtgcacccgggccaccggcggaaaggccgcgggagggagctcatttcgcttgtcgacgatcccttgaaccccatccaccacaccttttgggcccacggcaatcttcccgccgcgcagcaaaccgccgcggcgctcggaatgcagcccacccgcgaactgctcgtgatgtcggccaccgctgacgaactcgatgcggctggcgcactcgacgcgcagctgccggaggggtttgaggcgctcaatcttgtccaggcagccgcgcgctacggcgaagatgcggtgctagatagctggctcgaggtaaacaacgacgcgttttcctggcaccccgagcagggcgggtgggaccgcgcgcggctcgaccgcgggatggatacggaatggttcgacgcggaaggggtctggttcctctacaagggtgacgatctcgccggattccactggacaaagcggcacccagatgaaacgggtgaggtgtatgtggttggtttagcctcggcgtgtcggggggagggcttgggggtacccctgctccagatggggttgaagcacctcgtcgagcgcggatcctcgcaggtcatcctctatgtggaggccgataacgcacctgccgtcaagcggtaccgtgagacggggttcacagttgccgaatcgcacgtggtgtatgaatttcccatgatctagctgggagtttggggtctgggacgagaattcactgattgtttaccttcatttacaccggaggttaaccagcggcacgtagctttatcagccgtgagtaatcggagttgatttgcgcctgcatccagcaggtggatttccagcccgaaggacgggccgattctcttccattgatctacaaagaccggaaaggttaccccgtgatccgcaacatcaagcgcactgccgcaatcgccggcgtcgttgcagtttcctccgcttccctcgttgcatgtggcgactccaacgacaccaccgcaactgacaccgcgacctccaccgatgtcgcgaccgagaccgctgcttccgcaaccgagaccgctggtaccgacgcagctgctgctccggctggtgactacgagctgaccggccagaccggcaccctcgttgctgagggcgcttcgtcccagcagaacgcaatggactacttcggtgctgtgtacgccgagcaggttccgggcgcaaacctggcctacaacccgtccggttctggcgctggccagaagaacttcatcgcgaaccaggctgtcttcgccggttctgactccccgctgaaggacgaccaggtccaggctgccgctgaccgctgcggcggcaacgaggcatggcacctgccgttcgtcatcggcccggttgctatcgcttacaacatcgacggtgttgacgagctgaacctgaccgttgacaacatcgtcgacatcttccagggcaccatcaccaattggaacgacccggctatcgctgagtccaacccgggtgcaaccctgccggatctgccgatccaggtcttcttccgctccgacgagtccggcacctccgacaacttccagaagttcctcgccgccgcttccgacggcaagtggaccggcgagggcaaggccttcccggctgaggttggtaccggtgctaacggctccaccggcgttgccgaggaggtcaaggctaccaacggtgctatcacctacgtcgaggctggcttcgcggacaagaaggccaacatcgacttcggcaacggcccggtcgagctcaacgcggacaccgtgggcaaggctctggacaacctggagttcaagaccaccggccacaacatggtcgttgactccagcgcactgttcgcttccaacgaggctgactcctacccgctggttctgaccacctacgagatcgtctgctccgccggctacgacgaggcgacctccaacatggtcaaggacttcctgaacgttgctctggaccaccaggacgacgagctggctgacgagggcttcatcccggtttccggcgctcacgctgagcgactgcgcgaggccatcaacgctatccagtaaggcattttcaaagccttccgcccaataacgcgtgggacgactagcacctgacgcggttggcgagtgcgccccccactgacattcgtctttcggggggcgcacctgtgcggggatgcgatttctgcgccgcgcgcacaccaccttttctccatcacgatccttatatgcgaaggaaaagcgaaccatggctgacaatgacatgccagcaactggtcacgatggccgcggcgcaggcccggcgacgcagactgatccagtagtgcagcactcgaccggaagcccggtccaaaatggccaagatcaggcgaccaccggcaccccgattgccgacgaggcgaacaccaccgctggtgtgaagcgcccgggcgaccgcgtcttcgaatttctctccaccgtctccgccgcgctgatcaccgtgctggtggcggccgtcggtatcttcctcctcctccaggcaatcccgccgctcgcccgcaacgagaacggacttctcggcttcttcacctacggcgggccgtggagcaccgctgacctggagaacatgaagttcggtatcccgaacctgttcttctccacgatcaccatctccctgatcgccctgatcatcgcgatgccgatcgcgctcggcattgccctgttcctttccaactacgcgccgaagtctctggttcgcccgctcggcaccttggtggacatgctggccgccgtcccgtcaatcgtcttcggtctctggggcgctcaggtgctcgggccgaagctgggcaagttttacaactggctccacagctgggccggcgacttcttcctgttcgctacctaccagaactcgccgccgttctccacggcccgcaacatgctcaccggcggcatcgtgctcgccatcatgatcctgccgatcatcgccgccaccgcgcgcgaggtcttcgtgcagacccctccgggccagatcgagtccgcgctggcgctgggcgccacccgctgggaagtcatccgtatgaccgtgatcccgttcggctggtccggctttatcgccggcgcgatgctcggcctcggccgcgcgctcggtgagaccatggcgctctacatggtcgtcgccccggccaacgactaccgcggttccctgttcgacggcggcaccaccttcgcaaccgcgatcgcgaacgccgccgcggagttcaacaacccgatcagtgccggcgcctacatcgctgctggtctggtgctgttcgtccttacgttcatcgtcaactcgatcgcccgcgcgattgtgaacaagtaggcaggaggagcaaacataatgtctaccgctattccgactcacggttccggttccgactccggctcctccaaggtcaccacgaccaccaccgctgacaccgctgtagccaccggcgggcgggagggcaacggtgccccgttcgttgacatcgccggcagccgcaagaccacgaacaccctcatgggtgggttgatgtggctctgcatgatcctcgccctcatcccgctgctgtgggtcctcatcaccgtggtctccaacggctggcgcgccgtggtcgacccgtcctggtggaccgaggacatggtcggcgtccgcgcctccaaggagggcggcggcgcggcccacgccatcgtgggtaccctgctgcagaccttcgtcgcgtccctgttctccatcccgatcggtatcttcaccgcgatctacctggtggagtactccaacggcaaccgcctgggcaagctgaccaccttcatggtggacatcctctccggtgtcccgtcgatcgtctccgcactgttcatctacgccctgtggatcaccatcctgggccagcagcgctccggcttcgccgtgtcgctgtcgctgattctgctcatgatcccggttgtggtccgcaacaccgaggagatgctgcgcgtcgtgccaatggatctgcgcgaagccacctacgccctgggcgtgccgaagtggaagaccatcgcacgcatcgtgctgccgaccgccctgtccggcatcatcactggcatcatgctggccgtcgcccgcgtgatgggtgagtccgcgccggtgctgatcctcgtgggctccaacccggccatgaactggaaccacatgttcaaccagccgcagtcttcgctgccgctgttcatgctcgacatgtggaagaccggcgccaccggcccggcgaacgaccgcctgtggggcgcagccctgaccctggtgatcatcgttgtcgctctgaacctgctcgcgcgcttcatcgccgcgaagtactcggtgaagaagaagtaacccgccgtatccccccttaaccaacaggagaaatactgatgtccaagctctctctcaacgacgtcaacatttactacggcgacttccacgccgtgcagaacgtgaacatggagatcccggcccaggctgtgaccgcgttcatcggcccgtccggctgcggcaagtccaccgtgctgcgcactctgaaccgcatgcacgaggtcatccccggcgcgtccgtcaagggcgagatcctgctcgacggcaacaacatctacggcaagaacgtcgacccggtggcagtgcgcaacaccatcggcatggtgttccagaaggcgaacccgttcccgacgatgtcgattgctgagaacgtggtcgccggcctgaccctgcagggcgtgaaggacaagaagaagctcgccgagatcaccgagcagtccctgcgcggcgcgaacctctgggacgaggtcaaggaccgtctggacaagccgggcggcggcctctccggtggtcagcagcagcgcctctgcatcgcccgcgcaatcgcagtgcgcccggaggtcctgcttatggacgagccgtgctccgctctcgacccgatctcgaccctggcagtggaggacctcatccacgagctgaaggaggagtacaccattgtcatcgtgacgcacaacatgcagcaggctgcccgcgtgtccgacaagactgccttcttctccctcgaggcaaccggtaagcccggcaagctggtggagttcaacgacaccaccacgatcttcgagaacccggaccagaaggagaccgaggactacatcgctggtcgcttcggctagagcatttgcttgacgacggcaccgtttcccacctcggggcggtgccgtttagcgttccccggttatgaacacgacttgctgaccgatggccacgcagtggtcggcaaagcgctcgtagtagcgggcgatcagcgcggtttccactgcctcgcacgcggtgtgggcccaggctttgtctttggccagcgcagcgagcttgctcgccgcctcgtccaccggctcgtcggcggcgtcgagttcgcgcgccgcatccgcatcaggttcccggaggaactccgcggtcagcgccgccatctcgtcgacggcctcggccatggccgcgatctcggtgcgcacgtcctcgggcaccgcgtaatcgggatagtgttgccgcgagattttggccaccagcttggccaagttagccattcgcacgaggtggtcttcgatgcggatgtaggccataacgcggcgcagctccgaagcaacgggggcctgcagcgccagaagctcaagcgcgcgggcctcgcactggcgctgggtgtccaccacggcgtcggagttgctgattgctgtctccgcagcctccaaatcaatctccaaaagcgcgagcgacgccgtggccatgccagagcgggcctgctcgcacatggagacgatgtcgtcggtgtacccggcgagaagggcgcggtactgcccgcgcagctcggtgcgtgtgtcagccgccattgttctcaatctccgcgccttctggcaccgtcgcatcttccgggtcgtcgagccagccctcgggcagtgcgatcttggaggccgagccctgccggccccgcgcgtcgtccgcgtggtcggccagcgcatccgagtccatgatcggcgcgaggcgcccactcagctcagacagcgacgtgacctgcgccagttccctgcggaactcgccgccgacggggaagccccgcaggtaccacccggtgtgcttgcggatgtcgcggcaggcgtgcgactcgccgtcgtgaagcgcaagaagctccgcgtggcggtagatgatgcgcgcaaccttgccgagcgtcggctcgggcggaatgtcctcgccgcggagctgggcgccgagctgcgcgaagagccacgggcggccgaggcagccgcggccgacctccacaccgtggcatccggtgagctccatcatcttcgcggcgtcgtcggcggcgaaaatgtcgccgttgccgatcaccggaacaccgcttccgtccatgtgctccacaaggcgcgcgatctcgtcccagtgagcctcgcccgagtaacgctgcgcgcccgtgcgggcgtgcagggccaccgcagctgcgccggcggctgctgcaatgcgccccgcgtcaaggtgggtgtggtggtcgtcgtcaatgccgatgcggaacttcactgtgatcggaatgcccgacccctcggccgcgcgtaccgccgcgtccacgatgttgccgtagaggcgccgcttgtacgggatggcgcagccaccgcccttgcgggtgaccttcggcaccgggcagccgaagttcatgtccacatggtcggcgatgtcttcctcgacgatcatgcgcaccgcgtcgtacgtgaacttcgggtcgacggtgtagagctgcatcgaccgcgggcgctcaacctcggcgaaggtggtcatgtgcagcgtcttctggttgcgcgccaccatggcgcgggccgtgatcatctcgcagatgtagaggccggacgcggtgccggtgagctcttcctcgatctcgcggcacaacacgcggaacggcatgttggtcaccccggccatgggcgcgaggatgacgggggagtcgagctcgatgcccccgatgcgcagcgcggtggtggttacagtcataggccctcattgttcccgcaggcggcgtttcagtccaatcacactttcgggggtggcctgcggggcttgaccgcggtgcttggaacaacctcccccgcagaaatgcaagataggtcacaatagtctggcactgtaacccggaacgaaaagagggatccatgagcgagcgcatcgcaaacgccaaactccgcgacaaggtcatgaccgcgcaggaggctgctcagttcatcgaccacggcgcgaagatcggcatgtccggcttcaccggcgccggctaccccaaggccatgccggccgctatcgccgaacgcgcgaacgaggcccacggcaagggccaagatttctccatcgacctttacactggcgcatccaccgcgccggaatgcgacggcgtgttggccgaggttggcgcgctgcgctaccgcatgccgtaccagtccgacccgaccatgcgcaacaagatcaacgccggcgagatgaagttccaggacatccacctgtcgcactccggcatgatggtggagcagggcttcttcggcgatatcgactttgccatcgtcgaggctgtccgcatcaccgaggacggcaacattgtcccgtcgtcgtccgtgggcaactccgtggagttcctcaacgccgcgaagaagatcatcatcgaggtcaactcctggcagtccgaggatctcgaaggcatgcacgatatctggaccgtgccgccgctgccgaaccgcattccgatcccgatcaccaagtgcggcgaccgcatcggcaccacctacatcgagatcgacccggagaaggtcgtcgcggtgatcgagaccaacgacccggaccgcaacgctccgttcaaggcgccggatgccatctccgagcagatcgccggcaacttcctcgacttcctcgaaaacgaagtgaagtttggccgcctcagctacgacggctacgtcatgcagtccggcgtgggcaacgtcccgaacgccgtgatggcgggtctgatggattccaagtttgagaacatccaggcctacaccgaggtcatccaggacggcatggtcgacctgattgacgcgggcaagatgaccgtggcgtcggcaacctcgttctccctgtcaccggagtacgccgagaagatgaacaacgaggcagcccgctaccgcgagtccatcatcctgcgcccgcagacgatctcgaaccacccggaggttatccgccgcgtcggcttgatcgcctccaacggcatgatcgaagcggacatctacggcaacgccaactccacccacatcaacggctcccgcctgatgaacgccctcggcggctccggcgacttcactcgcaacgcctacatctcctcgttcatctccccgtcggtggccaaggacggcgcgatctccgccatcgtgccgatggtctcccacgtggaccacaccgagcacgacgcgatggtcttcatcaccgagtacggtgtcgccgacctgcgcggcctggccccgcgcgaccgcgtggccaagatgatctcgatcgcgcacccgtcctaccgcccgctgctggaggagtacgtcgagctcgcttccaagtgcaagtaccaggcaacgccgcacgacctgcgccacgccttcgacttccacacccgcatcgaagagaccggcacgatgcagaagagcgggtcgtagaacgcatcgcttctcccgcgggttaatagcgcctcgccccgattaccagcagcggggcgctaccggctaccattgagacgcacgggcctttagctcagttggtagagctacggacttttaatccgcaggtcccgggttcgagccccggagggcccacgcacgcaaccccgtcgcttaccgcggcggggttttgtggtcgatgccacacttcgtgctggaagtggggaagaaatcatgctacctaaaccggatggtctctacgattggtggtcggcgcaggaagcgccgcaagaacgcaccgagagaggtacctatgaccaccaccgtcggccactacctggccacgcgccttgagcagatcggcctgaagcactacttccaggttccgggagactacaacctgcagctcctagatgagctgctaaagaacgagaacctgaccatgatcagctgcacgaacgagctgaactccgcttacgccgccgagggctacgcgcgcgcgaacggcgcgtccgcgtgtgtgatcacgtttaacgtcggcgcgttctccgccctgaacggcgttgccggcgcctacgctgagcgcctaccgatgatcttcgtctctgccggttacaacacaaacgacgaagcctcgggacgattcctgcaccacaccatcggcgaaacggactactcctaccaggaggaaatgttccgcccgatcacgtgcaagactgtgcgcatcctgtccgcagaggaagcgccgagcaagattgacgacgcgattgccgcggcactgcgcgagtcgaagccgtgctatatcgagatcgcatccaacctcgccgatgctgagtgtcccgacccgcagccggtcgagttcccacgcgcctgggagtgcacctactcgcacgaggcgatggacaaggcaacgaccgacgtggccgaaaagctgaacgccgccgccaacccggtcctcttggctggcccgcatctgcgcccttacggcgccatcgacgcgttccaaaagctcgccgaggcgctgggctgcgcggttgcggtgcagccaaacgcgaagagcttcttcccggaggaccacccgcagttcatcggtcactacctgggcaacgcgtccgcaccgggcgtggaggcgatcgttgatatgtccgactgcgttctggcggcaggcccaatgttcaccgactactccacggtcggctggaccacctccgtcccatcagatgagggctacatcgctgtcaccgagcaaggtgtggttaccccggactcggagtacacgcgcctgcccatcgcggcgtttctgcgcgagctggcggccaaggttgagtgcaacgactcgtcgttgacgcagcacaaccgtgatgacatcactggcgaggctgcggcctacgagccgttggcagaccacgcgcagctcacccgcgcggagatggtgcaccagattaacgagctgttggtcactgactccacgctgttcgtcgagaccggcgactcctggtttaacggcatgcacatgcacctgccccacgatgcgggcttcgagatcgagatgcagtggggcgctatcggttggtccgtgccgtcctcgcacggctacgccgtggcgcgcggcaacgagcaccacacgatcctgatggtcggtgacggctccttccagctcaccgcccaagaggtatgcaacatgatccgctacgaggacaacatcacggtgattgtggtcaacaacaagggctacgtgatcgagtcggctctgcacgagggcccgtacaactactacaagaactgggactacccggctctcatcgatgcgttcaacgccgaggatggccagggcatcggcatcaccgccaccactgcggggcagttccgcgacgcgctgaacgtcgcacgccagcacaccgaccgcccagtgctgatcgaggcgcaaatcgaacacgacgacatgacccaggatctggtgaagtggggcaagccggtctccggtgctatcggccgcccaccggctgacgctcagtaacaacgctgacgcgttaaggctacggcggtatccttgcccgcatggatgtcgccgttgctttcgggatgacgttgctcgccggcctggccacgggcgtcggcgggttatacgtcgcgttgaaacgcacgccctctgaccgcttccttgcggggagtttagggttctcggcgggggtgatgctgtacatctcgcttgtggagctgctgggggagggcgtggcgtcgataagcgagggctcctcccacgccgagctgaaggtaaccgtggcctttttcgccggcatggcggcgattgctttgatcgaccggctggtgcccggtggtaccgggatgcgccgcgtgggggtggtgacggcgctcgcgatcgcggttcacaacttccccgaaggcattgccacgtttgtttccgcgctagcggatccggtgatggcggtgccgatcgcggcggcgatcgcgattcacaacatccccgagggcattgcggttgccgtgccgcttcgtgaggccaccggttcgaagtggaaggcagcgggttgggcgacgttgtcggggcttgcggagccgctcggtgcggcactgggctacctgctgttgcgtccggtgatggggccgcagacgctcgggtacgcatttgctgcgattgcaggggtgatggtgttcgtgagcgtcgataagctgctgcccactgcgcttgcgacggaccgccatgaagaagcggtgtacggcgcggtcggtggcatggccgtgatggccgcaagcttgctgctgctggggtaagcacgctcgcctgcctatttggtgggggccgaggccgtgatctatgatcaacaagctgtcttttcagcgcccccatcgtctagaggcctaggactccgccctttcacggcggcaacacgggttcgaatcccgttgggggtacggccctgtggcgcagttggttagcgcgccgccctgtcacggcggaggtcgcgggttcaagtcccgtcagggtcgctcttagctcgaggttctcctcgagcttttcgttttgtggtgacgggcgcgagtgagaacaaccacgctgtccggcggcgaacggcagcgccttaagctggccgcaagtctgaagaagccggcctctacctacctgctggacgagcccaccaacggccttcgcctcacggacacggcgcggttgctggccttgttcgaccggcttgtggacggcggtgcgtcggtcatcgttgtcgagcacaacctcgcgctggtttcgcgagccgactacgtcatcgacctcggcccgggcgcgggatcagccggcgggcacgttgtggctgcggggacggtgcgcgaacttgtggataattacaaggggaccgggtctgaaacgggacgctatctgtccgtgcttgcacacaattgatgtacccctttaccagccgatttgtggtggaggtgacgcgctgtgtaatctttcaactcgtgcaagcgacagcgtgaaagcgcgggagcgagtacagaaatgcatatggccctgtggcgcagttggttagcgcgccgccctgtcacggcggaggtcgcgggttcaagtcccgtcagggtcgcagaacagcttgcgaaagccgttctggctagatagctcagtcggtagagcacacgcctgaaaagtgtggggtcgccagttcgatcctggctctagccacagcatgaaaggtagccccttcgcttcgatgaaagcggaggggctactgctttgcgacgcccgcgtacactatccccatgcaatacgagctttcacgtaacgacaccgcccagcagtatgagttgacgatcggcggcgaagtagccggctacgcgtcgttccaggagcgcggggacgtgctcgtgcttccccacacggtggttgagccgcagttccggggccagggcctgtcgaagccgctgattcagtacgctctcgacgacgcgcgagaccgcggcctgaaggtcgtcccggcgtgctcagcggtggccgggttcatcgacgccaccccggagtaccgcgacctggtgtagcccgccgcggcgcggccgcggcccgttagatgatgtagctgcccgggtcgacgtagttgtccgggtccaccagccggacgtgctcgccggacttgcgcgggcgcactttcgcgggaatgcccaccgcgatcgagttttccggcacgtccttggtcaccacggcgttggcgcctacggcggagccggcgccgattgtgattgggcccagcaccttcgcgcccgcgccgatggtgacgttgtccccgatggttgggtggcgcttggtctgcgtgagcacctgccctcctagtgtgacgccgtggtagagcatcaccccgtcgccaatctctgccgtctcgccgatcacaatgcccatgccgtggtcaatgaaaaaacgccggccgatggttgcgcccgggtgaatttcaatgccggtgaggaaccggttgatctgcgcgaggatgcgcgccgggcctttccacccgcgaccccacatgctgtggcagatgcggtggatccagatcgcgtggagacccgaataaacgatcgcgttctccacgtttccgcgcgcggcggggtcgtggtcgcgggcgttcgcaagatcttcgcggatggtggaagccacttttgagatcaccgaaagcatggttggcaccttactaaaacgagcccccggcaaaccgggggctcgagagttttatgcgcggggttgtgcgccgcggcgttgcggactagtcgcggatgtcctcgtagaggacggtggaaacgtagcgctcaccgaagtcggggatgatgaccacgatggtcttgccctcgttctccgggcgctcagccagctcgagagcggccttgacgttcgcgccagcagagatgccgccgaggacggcgtccttcacagcaagctcgcgggacgtcgcgaccgcgtcctcgttggaaacggcgatgatctcgtccacgatggagcggtcgagggttcccggcacgaagttagcgcccaggccctggatcttgtgcgggccagcctcgcccttggacagcagcggggaagcggccggctcgacggcgacggccttgacgtcggacttctgctccttcaggtacttgcctgcgccggagatggtgccgccggtgccgacaccggctacgaggatgtcaacctggccgtcggtgtcgttccagatctccgggccggtggtggtgtagtggatgcgcgggttggcctcgttctcgaactggcgggccaagatagcgccctcgttctcggcgacgatctcgttggccttctccacggcgcccttcatgccggcggcgcccggagtcaacacgatctccgcaccgaacgcgcgcagcagcacgcggcgctcggtggacatggtctccggcatggtcaggatgaccttgtagcccttcgccgcgcccgcgagcgcgagggcgataccggtgttgccggaggtggcctcgacgatggtgccgcccggcttcagctcgccggacgcctctgcggcctcgacgatggccttaccgatgcggtccttcaccgagttcgccgggttgtagaactcgagcttggccagcacgcgggccttcgagttctcggtgatgccgtgcagctccaccagcggggtgccaccgatgagctcgaggacattgtttgcgatcttcgccatgtttcgctccttgtgaggatcgttagtttcaggactgcaggcgactatacacccgacgaatagacaatgcggttttagcaaaaaagacagagcggtctaaggggctttcgcttatcgacgccctccccccacccacacccgcactccccgacaaaacgcaagtacgggacacgggaggtgaagtttggctacccccgttcacgggttatcatcattgccatgactgtggatgctcaacgggtcaaagacgatgacgattcgatccgcgcagctctcaccgcgctaaagacggccaccgggatccccgtggccatgtacggaacgctgctcgcggataaccgtctgcagatcacgcagtggatcggtttgcgcacgcccgcgctccagaacctgatcattgagcagggtgcaggcgtcggcggccgcgttatcaccacccgccgcgcggtcggtgtctccgactacacccgagccaacgtcatttcccacgagtacgacaaggccatccaggatgagggcctccactccgttgttgcggtgccagtcattgttcagcgcgagatccgcggtgtcctgtacgtcggtgtccactcgaccgtgcgcctcggcgacaaggtgatcgaggaggtcaccctcaccgcccgcaccctcgagcaggacctcgccgtcaactctgcgctccgccgcctcgacgggggcaagggtgcggccgcgaacaaaggccgcgtgatgaacagcgccgagtgggagcaggttcgggcaacccactccaaactgcgcatgctggcgaaccgcgtcgacgaccaagacctgcgcaaggagctggagcacctctgtgaccagatggtctccccggtgcgcgtcaagcagtccacgaagctttcggcccgcgagcttgacgtgctgtcctgtgtcgcccttggccacaccaacgtggaagctgccgaggaaatgggcatcggcccggagacggtgaagtcctacctgcgcagcgtcatgcgcaagctcggcgcccacacccgctacgaggcggtcaacgccgcccgccgcatcggcgcgctgccctaggaacctgtttgggtacggtgggggacgtgaaagaacgatttctggtctccggcggcactcggctcgaaggcgtggtcaaggtggacggcgcgaagaacagcgtgctcaagctgatggcggcctcgctgcttgctgaagggaccacaaccctccacaactgccccgaaatcctcgacgtcccactcatgggccaggtgctcgaaggtctcggttgcgaagtggacatcaacggcgccacggtgcgcatcacaacccccgccaccgtttccccaaacgctgactttgaagcggtgcgccagttccgcgcttccgtggccgtgctcggcccgctggttgcgcgatgcaacgaagcgcgagtggcgttgccaggcggcgacgccatcggctcccgtccgctggatatgcaccagacggggttggagaagctcggcgcaaccacccgcattgaacacggcgccgtcgttgccgaggcaaaagagctgcgcggcgcagccattaagctcgacttcccctcagtcggcgcgacagaaaacatcgtcaccgcgtcggtgctcgcgaacggaaccacggtgctcgacaacgccgcgcgtgaaccggaaatcgtcgacctctgcgacatgctcaacgccatgggcgcgcgcatcgacggtgccggcacctccaccatcacaatcgagggcgtcgattcgctgcgtccagcggagcacactgtcgtcggcgaccgcatcgtagcggggacttgggcctacgccgccgctatcacgcagggcgatatcaccgtcaccggcatcgccccgcgccacctgcacttggcgctgtccaagctgaaactcgctggtgcgaacgtggagacctacgacaacggcttccgtgtccggatggaccagcgcccgaaggctgtggactaccagaccctgcctttccccggtttcccgacagatctgcagccgatggcgatcgcgatctccgcaatcgcggaaggtgtctctgtcatcaccgagaacgtcttcgaagcgcgcttccggtttgttgacgagatgcttcgcctcggtgccgacgccaacgtcgacgggcaccacgttgtcatccgcggtgtcgacaagatgagctccactgacgtgtggtcgtccgacatccgcgccggcgcaggacttgtccttgcgggcctcgttgcggaaggggaaaccgtggtgcacgacgtctaccacatcgaccgcggctacccggcgtttgttgagcagctcaccgacctaggcgccaacatccagcgcgtgggtggccggggacgccacgctgccgactaaccgcttttaagcacttacgtttaaatcggaaaaccgtttctgtgctgggggtttgtgttgtgttggtgtggtgtgtaacttagttcgagtcagcgagaccgacagcgccccgcgagagagtgtgaatcttcttgtggtgtggcgataagaaaacgatcgtttggcgaaaattttttactgctgcttgcgcaactggctgtgtttggttggttgtggggtgtgcgtgtgttgtttgagaactcgatagtgtgccaatacttttttgtttggtgtgattgttgtgcgtgtgcgccatgattttttgttgtggtgtgtgccggtggcagtgctgctttttctttg

SEQ ID NO: 9 - DNA, 185787 bp, Corynebacterium cassirii
  source 1..185787: mol_type = genomic DNA
ggcaggttggggagccggcgccagctcctgcccccgcgccggctccccaacctgccccggcacctgcacccgcaccgcgtgtggcaccggccccggcgcctgccccggcggcgaaggcttaccgcaactgcaccgcggtgtggaacgacctcggccgcccgatccgccgcggcgaggccggctacggttcgcacctcgaccgcgacggtgacggtatcggctgcgagaagcgcccgcgctaatcgaccagcgagggaagatccaatatgaaaaggcttgtgctcgccgcgtacgccggtgctctcatactcaccgccaccgcgtgcggcgatattgaggaccctgcccccacaacgggtttggccacggtgagctcgtctacctcgtccgcgagcgaatcgacgacgaccacgtcgaccacgacaagcgacgaggcagccccggaaaccgttcccgatcctgcgcctgtcgaagaaccggcccccgaaccggatgcgcctgcaccagacgagcgacctgctcaactgatcgcaccagcgccagcgcccggccaggttgaagaaccaccagcacagcagcccaagtccgcgtactacggcagttgcgatgcggctcggtccgcgggtgcggctccgctctacgcgggtgatgccggctaccgcgccggcttggatcgcgacggcgacggcgtcgcctgcgagtaggggttagcgctgaggcagtaccgcggtgaccgctgcgccgagcccgaggattgcgagggccgggagcacgacgtcgaaccagcgcaccgtggagctcgctgcgggcaccgacccctgtgagctcgccgcgcgcgctccctccgaacgcgtaccgccccactttgggctcgcgacgtagccggtgcgcccctgggagcacatgatgttggcgtcgatggctgccatctgcgcttggtaatagaagtccgtgtagcgatgcatctcggatgcatcggaacgctgcaccacggcgaggagcgcggctgagggctccgagtgcgggtcaaactgcgcgtcaccaaccatgaatccgaggtaccccaagtagaagaacccggggtcgtcctgcgtgaacttcgaagcaagaacgtagataacctcgtccggcgtctagccagcggcagcgaggtcggctttgacggctaccagctcaccctcgccgaagagttcctcaggcggcaacgctgggtcgaacgcgaatgcaaccgcgtccaaatcatcgagttcagcgagctccgcagctgtcgtcacatcctcccgtacgcgggtctcgagctcggtggtgatgtagcggtgagcgaccgcgtaatcggcgatctcgcgcgacgaggcgtcgagccagcagacaccgccgtccatcggcgttgcgacgagcgcctgcaccggggcggctgcggaaaccgctaaggccgttgccaccactgcggcgtggagagtccttcgcatgaccgcagtataaagacgttttcccgtgcacaacgaaaggcgaccgcggacaccgccgcagtcgccgttttacctcgtttgcgttcgagttactgctggaactgtgcaatcagctgatcgatagtaatccccgaggcgttcatcgcaccgagaaccgcgacgatcccgccaatcgccgccaacagtccaagcagcacacccagcggggtggcagtcacactggagccgaccgtcgccgagctgccggcgatcgaagaaccaccgacactggaagacttcgacgatccgtccgacgagcccgacggggtcggcgtgaccgtcacggtcgccgtctccgtcacggtttcaccaggcttcaccacggtcgtcggagagaccaccgtggtcggtgttgccaccgtcgtggtcgcccctggggtggcggtcactgtcgtagtgacggtcgtggtgaccggcggcacctcttccggtgcctcagcggtgaagacgcgcaggttgctgtagcgggtttcgtcgcggccatctacgttgccgttggaacgagcgaaccacacgtactcgtcgcccttatccaggtcgttccagtcaaacgtcacagcgctacctgcgcgaagctcggcggaaccgacggtctccgctgtgccaaaggcggcgatgccggaggttgcaacgaccttttcgtactgcagaggaacctcgaacgtgaactcgtcagactcaggtgtgtaacccaagtcgcgcacgtcgttcttccacggctcaaaggactgcagtcgcggcgagtaggcgttgccggcgaggatgccgctgtccagatccacctggtaaaggcgggtgtagagtgcgtcgcgcgcgccatcttcttcgtacgactggtagtcggcgacggtttcgaacaccttcgtgccgtcttcgcgctctgtgaggcgctgacgcacaccgtgcaggtggccggagagcactagcaccacgttcgagttcggctcgacaaggcgctcgaagaggacgtcaccctgggccatccagcgaccgttggccgggttggaacgctcatcgatttcgggcttgaggtactcgtgcgtgccgaagacaacgttgtggtccgggtgcgccttgatcacgccgtccgcccactcgatctcctcttcggaggagtcgtagcccatctgcaggaacagccacttcgagccgtccttctcaagcgtgaagtaattcgacgccataccgtccgggccgtggtcgccgaaccacggcttgttctcaaagcgggagaccgggtagtactcgttgaacatgtcgttcgagttgccccacgcgttgtcgtggttacccggcaagatgccgtacggcatgtcagcgtcttccagaatcttcatgatcttggatgcgcgctcgttctctagaactgctcggtccggctcctggttgccacgcagccagttctggatcacgtcgccagtgtggaccgtagcgatgatgtcgcgagcgtcgcggttggcgacgaggaacgcgatcatctgcgtaaacgaggtcgggttctgctcaaccaggtactgggagtccgttacgtgcgcgatagcgaagtcgtactcgcccggcgtcttaaacatctggttggcttcggaaccgctgtcggagaacggatctgccgtacgcttgccgtcctgcaccaagacgtccaccttgccgtcgcggtagtagtcggcggctgcaccggagccgacaagagtgagttcttcgccctttgcccccgctgccgtacccacgcggtcccacgtacccgtggtgtggttgaagaagtacatctgcacctcgtggcggtctcgggaagtaccgctccacgcgatggagatgtcgttgccctccggcttctccacggccaactcaaaacgctggtacgggaacgcatgcgttgcgtcgaccgcctggtccatgttgcggacgtcggccgcgcgggtctcgttctcgccaacccgcgtttcaagggcctcacccttcgaggtgccaataaagcccgcggagttctcccaatcgatcttggcggtctttgccccgagagccgtggcatcggcggcgctgccggccttgacggtcagcgcgcggccgctgtcggtcgcggtgtccgagatctgtgccggcgcgaactcctgcttgcggtccacctgaaccgggtcgagggtgccctcgagcggctcggtcacgtcgcggtactcaggcccctcggcggaacccggcgtcgccttgtccgtgaagaagtctgcccagttgttcccggtggcctgcacgcggtgccatgcgtagtcgtgcttctgcgcttcctcaatggaggtaaaacgcatgcggcggtcgagcggcaccgaggtctcaccgctgcacgggccttccggagcgttggtgaccttgcctacgtcgtcgtagtagacagcgacgcggtcgaggagggctccggtggcatcggtgagcattgcaccgtagccgtcctgttcgaagagctgctcggtttccagcgcaccgtcaaccccagcctcagctcgagccacggtgaacacgccgccgggagcgagcttgatgccctccggcacgattgccgcggacttcgacatgcggcggccgtcagcggcgcagtagtcaacgcgcaagcccgagaggtcctcctccgcgtcgccgcggttgatgatctccacgtactgcgccttctgccccgtcgcaccgcctgccgcgatctcgttgataagcaggttgcccagcttcggctcctgcagctcgatcggggtaatctcggcggggttatggacgcccggggtgcgcgtcgcgcgcacaaagtcagccttgttgttgtcggtgtcagcgacgcgctggaacgactcgttggacgggaaatcgagggtgttcggcaacggctcaccgagtgaacacggggaatcgacgcggtcgaagacaccgacggcgtcgacgatgtccaagttctgatcaacaagcatcacgccgaagccgtcgttcgcgttgaacgaggtgccgtacgtagcatcgggactatcgacggtggacgccgagccctcgcgagccgcgaggaacacctggcccggctcgagcttgcccgcaggcatgttcagctgcagcatctcgttgtacacgcgacccgtgcccgtgcagcggtagacctgccacccggtgacatccacggcttcggtgccgaggttggtgatctcgaagaagttgtcacccgcgccaccttcaccgccgttcgcaacctccgtgatcttcaccgaagagggtgcgcgccgctccgaaggagcttctgcgttacgacgccccggagtacgcggcgccacaacaaaatcttcacgcgcgtcaccggtgatgccgacacgctgccacgactccgcgtgcaacccgttcagcgtgccgggaagcggcgagccattggcacagaagctggcgacatcgggacgcgacgagccgatacgatcgacgatcttgccgttctggtcgaagatcatcagcccgtactgcgtagcgaaggagataccgaacgtggcatcctgaacggccttgatgtcgtctccggcctgacccgcgcgaccagccgtgaagcgctgacccggctgcagcacgacaccgtcgagctgctcgaccgacagctgcggcaccgatgcgcgcacgcccgtgccgatgcaccggtagaccgaccatccggtgagatcctgcggcgcatcgccgtagttttgcatctcgaagaagatgtcgccgttgccacccgggccggtgttggtcatctccgaaatgaggacgttcgccccaccagtagtcgacggctccgaaccagtctgtgctggtgctgcctgcgcgagcggcgaaacaaccgctgtcatcggcaatgtgatgatgatgcttgaagccaccgctgcacagctacggatggcattccacttccggctcatttgactctctctgacgtaggtacgcgccgctgccccggcgctgaacccgacgctagaaccttgagagaaactcgggattagattgagattaaatggaagtaaactgtttttggacgtctaaccacttatatgggaagcgcgcgcccagatggtggggccagcggggctcgaacccgcgaccaacggattatgagtccgtagctctaaccgactgagctatagccccttaagtcgcaaaactctgattactataacccgtcgcccatcgagtgaagtaatgcgatgctgttactgacgataacccaaccggtagtgttagccccatgtaccaatacatcgtcggagctgctgcaggatacgttttgggtacgaaggcgggccgcaagcgttaccaccagatcgtcaacgcgacccaagcggtagcgaactcaccagtaacgaagtcggttaccaactcggcgcggcgtgcgatcgccaacaagatcgatccggagccgcggatgaaagaggttcgcggccggaaacgcggtggcgatcaaattctcgaaccagatcaggactaattcgcaacttcaaacagccccgccacaatcccgtcgaggatgtccttctcgctaatgatgaagctggaggcgttggcggcttgctcgaaggcattagctagctcctcgacgacggtggagccggaaccgatgacgtcggcgcgcccgggatgcatcacggggttctcaagccgctgagccgcggtcttggagcggagatccgccgtcacttcccgcatgcggaggaacgggatctccgacatgtggatgcgttcggggtcatactcaggcaaaccctgggcgagcgcggacagggtggtaaacgtgcccgcgcagccgacgaacgtggtcgcttggttgaatggaactactgtcgcggcctccgcgatgcgctcgcggatgtaggcgcgggcttcctccgtttcctcgcgcgtgggcgggtcggttcgcatgaagcgctcagtgacgcgcacacaccccatctgggtggacttggcgcgcaggccgcccggcgtcatcatcacgaactccgtggaaccgccaccgagatcaatcacgcaggcggggccccgttcggggtcgaggtccaccgtcgcgccagcgaaggaaagcgcagcctcttcctccccggtgatcacttctgcttgagcccccggtgtgatgcggccgaggagctcgcgtgtcatggcgaagaagtcctcgcggttagcggcgtcgcgggtggcggaggttgcgaccatgcgcacctcggatacgtgttcgcgctgcatctcgtcgacgtactcggcaagcgcctggcgggcgcgctcgatggcctcgagcgcgaactggccggtctcgtccacaccttggccaaggcggacgatggtgttgcggcgcacgacgtcgacggcctgtccggtggtggggtcgatctcggagatcagcaggcggatggagttggtgccacagtcgacggcagcgacgcgggttggctgggtggtcatgcgagcccctcccctgcttcggtgagtgtgatgttgagatcagcaagcgtgggccagtccgcgggaatagcggtgccgcggaggttgccgtgctcggcggcaagtgccacggcttcggtgccgaatcggacgcggccgggaccttcggcaagtgcgtaggcgatgagcacgtggaggcacttcacgcggtctggcatgccgccgccggagaagtcggtgccgaggtcgtgtagtccgttccgcttggccaggtagtgctcgtgggcagcgaggtagtcggcgcgcagcgccgcgccgactacggtgtcagcgttgaggcgcgactccatccacttcatcacctgcgcgacttcgaggcgggacgcttcggcagtgaggcgcgggtctgtgaggtagtagagggtggggaacggggtggcgtcggcaagcataggctccgtgagcaccaccgccggctgaccgtccggcgtgcggtaggagacctccagaacgccgcggggtgtgcggccgagctgggtcgtgatggtgtcgaggtcttgctgggtgacaggcatgggctcgatgttactgagccgccgagtggccggttgtcttgaaggtaccgatatccaccgcagttgctgccggcagctggctgtccagcgcggcgatcgtgggcgcgatctgggactgctccacgaacagcaccggcatcgggcataccttggcgttgttcgaggtgtcgaaacgctcgtggtacaggttcacctgcacgggctgcttgagctgggacgctgagcggccgcggactgcgaacacgatggcgcggacggtgcccggaagcatcgatgcctcgtagatgcacgtagagacggcgccggaggcgaagcaggtcttagggatgatcacgccgaggtcagtctggacgaactcgagtttttggttccacaccttcgtgtccaccatgatgctgccgcgggggctgttgaccaagtggtcgatgttggcagagacgttgccgttcttgttgatctctagatcatcgatgagcaggaatgaatcatcaagaccgtcctggatgagccatgaggtctggatctcccccgccgcgccgatggcccaggtcttgtcctcaccatcgaacaccgtgcccgtggtcttgcccgtgtcgatcaccttctggaaatcgtcgtggacgtgctgcttgaccgcctcgagctgctggaagtactcggggtgggattcggcgaggtcgatggggacccgcttcgtttcgcgacgatgcatgaacgtggaaactgcgtagaccacgattgccgcgcacgagaggaacacagtcctagaaagcgggtagtcatctgtgattgacaggaccaccaacgcactgatgatcaagaacgccgcccagccgctgtctgtcggtgtgacggcgctcgagttgggttcgaagcggtactcgcgcttgggttccggcggcgataaccgcgcgacagcgttgtccatcgcttgttttaccgcaccacctgcggcggttccatacactttagccatgtgggaaaactctagcgccccggtgcgggcgcctcgtggcccggcgtcaggggctcggggatttcgcgcaggctatcccagaggaactcgcgccacccgcgggtgtcgggggcctcgtcggtggtgatggcggggttttgcgtcatgcgggggtcgatgatgcgccaggctgtttcgccctctgcgagcacgcctagacgacgccgcgcttcctgctccacaaacgtaggatcctcgtagcgcgcgatgtccgattccaagctgcgtttctgcgcctcaagcgcctcgatcgcggcgttggcgcgggcgatctcgccgcggccctcgtagtagttgcgcagcggcaccgcgattgcgacaaggacgaccaaaacgacggcgaggaggatgccggcagacttcagatcggcgttctgcatccgctcccgggcgcgttgacgcccgcgagtgcgcgcggccttctcttcgcgccgcttctgctgcgcgcggtccctcgaggccacggggaccgtcttcggggcgcggcgcttgcgtccgccagttggtgcgtttggggtcatagtgattgttgagcttagcgctgttgtgagcgggaaaccggtttgacgtggcctgggagctagacccggaccttcagaacttggaggaaatcgagcggggtgagcacgggaaccccaaagtgttgggccacatcagggatcttcacctttttcacgcctttaggcgcggcaacctcggcggttacaatagacgctccatgtcgtgaggctgaagcgaccaaccaagaatcagcggcactgtagaactggtccacggcataaggccggtactgaggctgccgagtgtttgctacccaccgcgttacgtctgtgtagtggtccagttccaactgatcgacactcagaatctgtttttggtcgacatgggcgttgtaccaatggagccggggatgagcccaccgctgtagttctttgtccacctcatggtgaaagaaaacgctgggcacaaacagcctatgaactagctggctccatagtgacgggaacactgcatcagggtagaagttctcgaggtgccccagaaagtttgtatcgactaagtacacccactacacctctgctggacccgttatgcggcgatcaccatcaggtcggtgaagctgccctgccatcggcttgcgcttttctacgagcgactggaaagtctcaaaactccgaacgcctaagtagcgcgccgcttccaagtctgacacctgtccgtccacggcagcctgggtgagtgtgtcaaagaagagttcaccaaccctggatctcgctaagacatggaactggggcccgccttctcggcgttcctcactctgccgcaccaccccgagaatcttccgcgccgcatcctcttgctcagcgcggctaacaagctcgagttctcgaagcctcaacagtgaggcttcgcggctcaaaccgaaacgccgagcgacggtattgactgcctccagcacgtcacccggctcgaaagtgctgcgcaccgcatccaccggagctataaattccgctccgaaagagttgcaccatctctccaactcctggtgctcagagtggtcagagagcccgggtttgccgcgaaccacgtgcccaagctcgtgagcaagactaaaaagttgcgccgattttgcgtcattagtgttaacaaagacgagcgcaaacccatcgtcttcaatagtgaagcctcgaaactcagtgacgctgagagcgcgccggttggcgttaccgaccaccgagtttcgcgagacaaggagacctgtctcctccatcgcgcgcgtcagcgtcagcaccttgtcgttgcccggtatcggttcgtttgtctcgaaaccgagtaactctcgtgtcacaatcgctgcggttcgcggactggtttcattggagactgagccgataatgcttggcgcctcgaccccgttagattcggcgtggtccgagtaccaggcaagccgattctgcgctgcgaagaatacttcctggaggtccggactcatttcgcccacagcagcactacgcaccgtccggaaatcggcaacgttctgatccccacttgaaggcgcctctaggagtaaacggccgaacggaatacgggccttgtcagcaagctttcgagcttgcgccagcgttggtttcgcttcttgggcaatccacttatccagtttggggaactgcgcgtgaaggtcgtcgccgtccataccagtacggcggatagcccattccagcacggcgggcgcgatggtgacctctacaggtgtcatcgccgctccttccgtttagcaataccgtctacgcagtataaaggcgggatccacattcacgtggatcccggtctagcggcgcctacttgaagcgcgggaacgcagcgcggccggcgtaggctgcggcggtgcccagctgctgctcgatgtccagcaggcggttgtacttggccacgcgctcggaacgggccggcgcacccgtcttgatctggccgcagccaagggcgaccgcgaggtcggcgatcgtggtgtcctcggtctcgccggagcggtgggacatcatcgtgcggtagccgttgcggtgggcgagctcgacagcgtcgaaggtttcggtgagggtgccgatctggttcaccttcaccaaaagcgcgttcgccgccttctcctcgatgccgcgggccaggcgggtcgggttggtgacaaagaagtcgtcgccgacgagctgcaccttgttgcccagctcggcggtcagcgaggtgtagcccgcccagtcgttctcgtccagcgggtcctcgatggagacgatcgggtagttgtccaccaagtcggcgtacaccttggccatctcgtcggcggtgtgctcaccgcgctcgaagttgtagacaccattctcgaagaactcggacgatgcgacgtcgagcgcgagggcgatgtcgtcgccgagcgtgtagccagccttctccacggcctcggcgatgaggtcgagggcggccttggtggagtcgacggcgggggcgaaaccgccttcgtcgccaagcgcggtggaaagccccttgcccttgatcacggacttcagggagtggtacacctctgcacccatgcgcagggcctcggcgaaggtgggtgcgccgatcggggcgatcatgaactcctgaacgtcgacgccggagtcagcgtgcgcgccaccgttgacgatgttcatcatcggcaccggcaggacgtgggcgttcgggccgccaacgtagcggtagagcgggaggttcgcggcctcggcggctgcgcgggcgttggccatagaaacacccaggatggcgtttgcgccgaggttcttcttgttgtcggagccgtcgagctcaatcatggtctggtccagcaggcgctggtcgtcggcctcgatgccggcgaccgcgtcgttgatggcctcgttgatgttttccacggccttgagtacgcccttgccgccgtagcgctcgtcgccgtcgcggagctcgtgcgcctcgtgctcaccggtggatgcgccggacgggacggctgcggtgccgcgggagccgtcgtcaagaaacaccgatgcctcgacggtggggttgccgcgggagtcgaggatctcgcgcccgaaaacgtggatgatgtcagccatgctggttcaactccttgaatggtgctatttcgttccagcacccaattgttgcagaaactacctgtgcgcgggctggttaagcgcgtaattcgctgctgcgtcgcggaccttggccacgtagtcgttcgagtggttgtacgcgaagatggcgtcgcgccagccgtcttgggttgccagatcgcgtcctcctgcgcagaggaggttggcggcggacagcgctgcgtcgtcaatctgctgcgggttgggcgtgccgtcgccgtctgcgtcgcgcccgaagcgcgcccacgattcggggatgaactgcatcgggccaaccgcgcggtcgaactccgtgtccccgtcgaggaggccgccgtcggtgtcttgaatcagcgcgaagttgcccgtgccgtcgagcgcggggccgatgatcgggggttcgggaatgccggcgtcgttcaggcgggcggggtcgaaactgcggcccgtgtaggtgccgtggcgagtctccacccagccgatgccggcgatagtgttccaacggatgttgcaggcgggccaagcctcgcgcgcgatgagttcggcgttggcgtaggcacgaagtgcctgcgggttgatgcgggttgcttcggcgatgggcgccgcccactcggcgagctcgttggcggtgcggcccggcgcgtggacgtcaatccgaggcggcgtctccgccgcgtccggaggcatgtgcgtgggcacgggggcgcgctgctgaccgggggcgggggtgtcggtgattgaggcgagccacgacacaagcgcgacaacgaggacgatcgccagcgtcaccgcgatcaggccgacgcatccgcagcctttcgcgactcgggaagcgcgtcgagttgtcatggcgggagattgtacttggcggggattaaggcgggcgaagtgctagcgggcggaaggctttcactttcaccacttgcgtcacttcagtaacatgtatagtccttatttatgcgaaaactcactgcttccctcgcctccgccgccgtcgcgttcgcagctctgacctcgtttgcccccgcccacgccgtcccgacgaacaacgcccctgccccaagcgccgtcgagctggtccgcctgctcaacggcgagatcgcgaccgccgactgcggccgcctcggcaccaccctgcgcgtcaccggcatggccaaccgcgagaccacccgctcccagctggtggcgaacgtcaacaacgccgtaggccagaacgcgccgctgcgcctcgttgcggcacccaccgtcaacgcgcttggcgaccgcgccgtcgagtgcggcgtggtcaaaccggacccggccaccccgatgacccagttcctccaaatgagctcgaagctctcctctgacgcgggtctgccggatctgcgcacgatcgctccgacactggcgggctagttcttctgtagaacttccgcttcccgtcccttgccctcggtccagtagcggtcctgggtggtgacgtcgacggtgccaacggagccgtcgaaaaggtaaggcgaacgcgactgcatcttggtcacgaacgagtgcgccacatccgcaaaggtgaatgcgcgcgctcggcggaaacttcgacgtggaagaggacttgcaggaggacatcggcaggctctttcttcagttcctcatcgcccgcatgctcctcgattgcctcggcgacctccgctgcttcctccttcgagtacggcaagaggcgctcgcgcgttacggattgctcccaccccctgcgtgtgcgcggtgtgcgtcaccgcaaccgcacaggcgacgggatcgtccaaggcggggaccgacagcgactggtccgccgagaagtacggcaactacctcgcgcgcctgcgaaaagcccgcgacacccacgacgcgacgctggcgttagacggcgttgagtatgacgcgcgcgagttcgcggacaagtaataccgcccatccacggtgccgatgaataggactatcggggttgctcgtaaacccaggtaccgcctatcgatataacgcgagaatcatttcggtcagttgtcgataaatttcgtactcgcagcatcatttaacgacgtacatcacttaaccgcagccaactgccctgctgtccaaccgcgtgtggtggtgcttccattcttctcaacccttgtcattctatgggagtttaagggcgtgaacccttactcgagcgttttggtcagctcatcaacaccggccgaagctcgagattcaacagcactccaacattccccgtactacgttgcaacactggatttggctatcagcaaatgtgagactttaagatctgcctgggccaacttttgagagctgcgcccgagtccaatgttccgaggtttagcacggcccgaaagattttcaacttcctcccgcgtgaacctcattctcccaagtcacttttggaccgcgtcagcaaccatcacctcgaactttccgagtgatggcctaaaatagtcattcacattgcaaccgcagccgagccgaggtagtagatgaacgaaacaagtcgcgaaatcattgtcacgatgaaaaatcagccatggccagagcctcatgggtggttcacaatcgcaatgccgcgcgtttccgctcagtcaatcatggaaaacgggtggaggttctcaaagaagccgaccatcaaggtgcagcaaggcatggactggctgagcccggggaaagaagatcgcagttggggcttccacttacacacatgggaaatgatggatgctgtcctaggagagtttgcgacgacgcgcgacgaagcgctattgaattggatgctggacattgccgatgattgggcccagtttgagaaatctgactctactgatggatccatgatttggtatgacatgtctcttagcttgcgcatggcccgcctagctcggttgatgatctacgcatcccatctaggcttggatcgtcgcgttgaagcactactacccgcggctgaacgtcatattgaagagatgttcaaacccgaagcatttaactcgggcaacaaccacgggttctacgccgcagcttcttcgctcgattgggcccgactattacctcagtttcctcgaagctccgaacttgcggccctcggggaagagaggctgaaagacatcgcatcgcggcagttcgctcccgacggtgggcaccaagagcattcccctggttaccaccggatgcttttgaagtctttcgaaaccggcttgaacgacgggataatcgaagaccccaccgtccaagcgacggtcgagaatgccacggatgttctcggctggtggatccagcctgatggctatttcgtccagttcggtgacaccgaccatcagtcagccgatcaaatgaagttaagctcgtcgaacgaacaaagccagttcattatcacaaacggacacgagggaaagccaagcagcgaagaactgcgcgtacttccagacgctggttacgcaatgatccgatctcctcaaccggcaggaccagacgagcggataaacagtagctacctcgcactacaggccgcattccactcacgtgcccacaaacacgcggatgacctgacttttgtctggtttgaccgaggagtggaaatcttggttgactccggtcgttttgggtacgtcgatcttctaccggccgattcaccggaccggcttaaagggttctactacgcagcgccggagcgccagtatgttgaatcgacggttgcccacaatacggtgtccgtcaatggtgaagatatcgaacgacgattccgcaccccctacggctccgcgctgaaatcgtggtcccatgaaaatggtatttttcgcattgaagctgaggcggactgcaagacatatacacaccaccgagtaatcactttgagcccccgacagtttctgatcgtcgaggattcgctcagcggtctcgctcctggagacgaagcaatcgcctggtttaaccttaacggcgaggcacaacgtgtggccggccaagacaatgagcttcagttcttacttccaggacaagctggctatcttacggttgaaggtgaccaggaagtggttacccccgttagaggccagcaagagcccctccgaggatggagagctaagcgagagcgcagttttgaaccgatctggaacctcggttttaaactcgatgcctcaaatccagctctgagaaccgaatggaagctcagcaaataagactgctagtctcgcccccacaagggtgagacaaacactgccgtcggttcctcatatagtcctaagccctacatagctttcgccgcccatccgttcggcgtcaagccagttcctgacaatctgctggtaggaagcaggcgcgggagcgacgtgcccgtcccccataaactcttccttaaactggataccatgggtcgatgatgatcggcccactaaatctttcagtggcaaaaagtgctctgtgaagtggtgatcatctcctgtgttctgcaaaaccaacccacgaacatcgaattcgatctcctgaaaccgtgtcaacacgctccaacgtttaagttcgtcgacactgaattcttcaatagctgttttgccgaatactgcccaggctgcttggtcagctagcagcggggtgtagcgttcgatatccgtttggccatttattgagatgaatgatgcgcctctaaggtgactcgcgacttgcattgcgctaaagcctcccccagagttccccacgatagttactcgttcgaccccgtaacgccttgcgagactgtcaaccatctgtgcaattacccggtgcaagtcaaggtcctcgtgccctatataccaagacagaatcatgcgactatctagatctaatgtcggatccgaaaagaatgcgaccggaccttgcgcaacgtaagagagagaacggactcgctcgtagcgtggcatcgagtgccgagttctatcggtcgcaccatgaaggtagacaagtagtgtgtcaccggatttgggacgaaccaacgctgaaggcaccacttggccacaatccacactccagacaaaatcgtcctgaggaggctctccatcggctaattcaggagaccgcgttgaaatgattggcgtcctgtagaaagtttgctcctcgccctcgccccacgacactagattggtccttttccgtgcggtcaccgcagcgtggctcggtaaatctgaaatgtccacccccgctagatcgaccatcgctgcaccgagagcatgatcgcgtagacctgtcactcggtgttcttcacaaaacgaatcaaggtatttgatgagacgctgacgattttccacgcttggatctttccaagccttttccttgacttcctctattacgcttcgtgttcgaagccgttgcgcaagcgcctcggagtcggagatttcgccttgtgcaagccttcgttcagcttcctcgatggattgttcaaccgaactcgtgggatcagcgagaatggatccctcggtagaattgaccaaccgttccgagacacccttgtcagtatgatcgagtacaatccaatgccccggagctggttttcgagtaattgagaactctgtggcgtcgaccacatccgctatcgccgtaatgattcgagaggactggccagtaaatgatgcgcttaatcgtcgagccgcaattcctccgctaccgtctttaatctcctgtagctctaagtcggaatcgatggttccaaaaatgcagatgcaaagagttcgactgccgtaggtgcaaaaagccctatccccgcgaagagtgacttcaacttctgggtgaataatccaatgcacgtaaccggagatctctgacgacgctcggatcgtatctttcaccactacataatggttgctcttgacaaaaactaggtcccggttccactgagctggcagatacgttttcggggctacaactacctcatccatgagagcgtctgaactcgaacggatgatttggctcctcgcgttgtctcggaagcgcctttgctctacctcaacaattgagtgatgcgccgctgcaccaaattcatctcctggcaaatcgataatccagggaatcccctgactgtggaaggtaactcgtccgctgtcttgatgtgccccgcgtcctctcgcaggccccgtccacatagtccaatgcgtttcttcgctgagatcccgctctgtttccccccacccactgcggctagaggaaatcccgccttcttccgcaatcagcccaaatgcgggcgggcttccaaaacgtccattggtccgaaggtagcgaaccccgccggacatcgtgtcccaaaagttctcgagcggcagcgagctacctaaggatgttggagctccgctaggagaaatcagatgagaccaaaattccgtggacgcgaagcttttcgagatcggtccaagatcgaaccccagcgtttccagacgatcgatccaaggtttccaagtgtcttttgcgattgacatctccttaagatctgttccgtaaagccctcctgaaggtctgataaatgcgcttatggcggcacgtaacggcccctcgatgtcggtcgaaaagtcttctcgacccgcattcagcaagatcagggaatctaccgccgctctgaaagattggggcgttggagcttcctcgagtcgccgagcaagaacgacagaatggttctttatcattaccgggtcgagcgctgctacaagttcgccgccgagtgccaaggcttgcactcgttgcgccaaaacggggaacgcccagagtctggacgctgacctatcttggttttggtttaacctccaccattcgttagcgagcctctgccataacccgccgaactcgtgcttatccgcacgtaccaactgatctagccatctcaagctgtggagagcgagatagaaagactcggtctcatatttcggggccgtcaaactttctgggcctatacttagttcaacgccgccgagaggcagggttccatcagctatctgaagggcccgacgtcggtcagatgctctcggttcgaatagtccagttcgaagtgacgaaaataattctgcttccctttgagcatccacgcttaaagaactcctctctcggtattaagctgcgcgacatgccgatagatttggtcgatccagatggcgcgattcatccatgattcgtgtactggggtcgcttcttcgttgcggacgagctcttcaaacttgaccaacgagtcggcgttgaggaactttttccaatggtgggactcttcccaaacaccccaaaagccgtcggggtccgtttgataagtgcaggttccctgccgcatcagacgtttcgaatcgtcccccgaggctttgtaagtttcgacttctgcccattgtgggattgctcggcggacaatctccttcggcacggcttttgaaaccttgtcctcaggcgtcacgctaaaagccaagcgcacaaaggcaggcgctgcaaggaggaccgccgaggtggaacctaaagcttggttaccccaccttcttagcttttcagttaggtacaggaaatcgagacgttcaagccccacaacgcccaaatcgtcagctttccgcccagcgaaactaaaggcctcatcaatggctctgtgggctgactcggtaagttgggcgaccccaaatgaccgcctagccgcaagcatgggatcggattcttcgcgtaatttctcaatctggcctggtcgagaatagtagtacccatgtacaatctcacctcccaccccgccgatctggatcaccgaccgtccagagggtatggcgacgttacgcttcatattccccggagcggcgtctccatcccacatagcaaaagacctttgtagtcgctcttccaaaggcatcgtgatctcggcgggatttggcagggtaacggtatgccgaatttccgagctatcctcccctccgcgctcttccaagtagatcctcatcagctcagaggcaatctccgactctcggggcagggctcccatagtcacgacgttggcgcgttgtactgcagatagccaaactcccgcagtcattcgtgagtctcttcctccgctcaggaagacggtcggcacccgatcaacgagacgcgcaatgttcctagaaaccagctgcaattgttctagggtttcagcgtaacctgtttcttcgtcgacaggttcaaacatcccagtaaaaccatcatagcggttctcgtgaatggccccggcggagtcgatcgagaaaacctgggcttcagaaaaccgtgtaattccggagatgggcgaatcgttgttcatgaagaaccccgcgccagcgaatttcgctacagcactttcgttaaccgaaatccgtccttggatgaattctgttagcgcaccaatgtggtttgacgcagcgaaaaaatcgtccgtttggatatagtaacagcgaccgaatcccaagatatcggcccacacttttacgtcgccgttggctgagacggcatacccgaaataattaggttgaagctcctggaagcgatcctgatcaacgatctgcttcaccagcgtccaatagttagaggcctcgattgtcgccgagtttggaatcggtggttgagagaatgcgatcgcaacatcgtcatcggcgaaaactggatcttcggaccaagtacctgagatccgattagcgttgtatgccctaatcctgccgttctggtagtgccacgaatctggggacttgaacacattctccactcgagtgattgcacgggcaaactttgaatcaatcgtttcgagcccgtgggcggatagtgcaaccgcgatgaggttaacgttcatattcattttgataccagaagtcccgcacgtggtttgataaacccgccaaataccatcggtttcgacctgcgaactgggatcgagggccgggagcgacactctgcgatacgatctcgaaagcacactttctaattggaggtcgggatgaacaaacccatgattaggattcaactggctgccgccagtctaagctggcttgtggggtgggctgccctgctcaaagacgggtttacatctggtcaaacggtcgtcaccgtcgctggaatcgccgtcgcgttgtcgcccattccagtggcttgggctgtaatcgataccgttcgtaggagagacaaagctaaagatgagcttgtagaaaaacttcgcaaagaagtgcggtcgaagtgcgatacggagaccgtagagctacaagttaagcctttaaagtcggccattgcggacgtcaaaaacacccacaagttggaaaattctcagatcagcaacgagcttatgaaacttcagcggcgcgttgatgaagacgaggtcgcactggaacaaatacagggatcactagagcagtctcatgcccgcgtcgaccagatccagacgagtacgaagcgatttcagtcacaggtagatcagacgcacagtcagcacaagatattgaaaagccaggctacccagacccaaaggctaactgagaaagcttaccagaccctcgataaactcgtcgcttccctacacgcggttgaaggcgatctccggtccgcgagcctcaggatccttaagcttgcttctcgccaagggatcaacgtgggccagggcttaacaaaagaggagctcggagagcttctcctccattccctcaaagccgatgacgcactggcaaaagggcttctcacacgcgaaattgaaagcgcaccgagtgatctatcgctgactgagctccgccaactcatgaagggtcttcgccatagcggatacctctccgagtctagtaaggtcatggggtggatcgcagagaggtcaggaaagactagcgacactgaacgcgccgcgattatgaagagcgaagcctcccttttcgaaggtgcgtacatgccgcaagttgagctcccaatttatcgaccgtacccagagtccaaagtggtcgttcaccttgttggaaagagtctgcccgaaactcaaaccggctacactctgcgcacccactacaccgctcgcgcaatagcgaagctcggggttgagcccgtcatagctgttcaagccggcggcgatggcatcgaatacagctcaatccaatctgactttgtcgacgatattcaatactgcacgctcgctggtccggtccggaacaccgtgccttgggatcaatgggtggagcagaatatcgtcagcttcgcagagcttgtttgcagtctgcgtcccgctgtaatccacgctcattctgacttcttcaacgcgttgattgcgcaatatgtgggtgaccggtacgggatccccgtggtcaatgaaacacgaggcttctgggaggaaagctggctctcgcgaacgatggacgcacagggcgaggcggggttccgtgaattggttgaagccttggggttaccgattgcatacacgggtcgccgcgccttagaagctaagctgcgcagcgaagcagaaacagtcatcactctcgctcaggttatggctgaacatattgaaaaaactgccgacgagtacggtcttcagcgtccgcgtgtcaaaattgttccgaacgcagttgaaagccgttccttcccggtcgtcggtaaagatcgtgatttgctgatcaacctcggcctccctgagcattcaacgattgttgggtatatatcctccatcgttgagtacgaaggaatcgataccctaattcgcgggttctacgaacttctctgcgcgttcaaggcttttgaagatctttgcgacgcctgcggcttgtcgctgaacgacttccagaatgaatcggaggcctcactcgacgcaataggggccggtcatgatcgtgttctttcgggttggcactcattcgaccaggaagtgtttgcggaaacagctgcgcggctggaggcacatctacgcgatatattccccgagttctaccaagagagcggatttgctgcggacctactgaacgacgttgtagaactagccaacatccccggctctgctgttacgtccgaactccgcctcgtgatcgttggtgacggagccgagctcgagaacctccgaggtttagctgttgaacttggaatcgatgaatatgtagttttcaccggccgcgttccacacgaagagatcctacgcttctacggattaatcgacgtctttgtcgtacctcggaaatcttccgacgtaaccgaattggtcactccgttaaaacctttcgaagccatgtcgacgggtcgcgcctgtgtattctctaatgtccgcgctctcaaagagatagctgacgaggctggctgtgtggaagtattccaagccgatgatcatcacagcctcgcaaagacacttctgcccatggtgtctgatcctgacaccatcagatcaatgggtagccagagcgcgcgctgggttcgtgatgctcgatcttgggacctcaacgcaatttcgtacgttgaagcctaccaagagctcggaatgcaaactgaccttcctgaatatgcgtctctcttccgcgacatgactactcagggccgccacccgagactcatgctcgaactgcttgagaacgcaccatgccccaaaccaacaggttggttcactaccacaaagttggcagcgagtgccgaggagattatttccgaaggctggaaaatggctaagcgtcctcgaattctgtttgagccaggttttgactggatggccccgggcaaggcagatcggacatggggattccgactgcatcggtgggaaatggttgaccctgtcctcgaagagttctaccgaactcggaaccgagaccttttggagtggctccttaatttctccttagactggtcgagatttgatgcacaagcggatgagcaagaatcaatggcttggtacgacatggcaatgagtctccgtatgccgcgtctcgcacggatcatgatctacgctgcgcaatctgggtataccaacgaggttactttgcttcttcccacggcagttaaacatatccgggagattctcaaaacaagcgccttcaacgccaacaataatcacggcttcttcaatgcaagtgcctgtttagattgggcaaagttactgccatcattccccaatgccgataagctctcagatgttggccaccggcgtctgtcaagtattgtcgatagccagtttgctagcgatggcggccatctggagcactcccccgcttatcaattgatgctcctgtctggtttcgagggtgcaatttcggatgagctcatcagcgatgcagcgctcgttcaaaagattgatcgagcgtcatatgcactcggatggatgattcaaccggatggtcacctagttcaattcggtgacacagatcaaatcgacgtcacagtcgaagaagtggggctcagcgatcctcacgcccgatttatagaaacagacggggcagaggggcaaccggataccgcccagatgatgatcctccccgaatctggctatgcctttgttcgcagcccgcagccggacagagtagagcagcgccgtaacagtagctatttagcattccaagctggcttccattcacgtgcgcacaaacacgcagacgacctaacatttacgtggttcgataagggtcgtgaaatcctcgtcgattcaggcaaatatggctattttgatctattgtcgaaggatgccccagcgcgcttggatggcttttactatggttcccccgaacgacagtatgtggaatccacccgcgcacacaacactgttgcgattaaaggattagacatcgagcgccgtaatcgcgaaccttttggttccgcgttagagacgtgctttgaagacaacggtaccttcatcctctcgggtcgcgttatccacgacaacctagagcactggcgtcgcattgaactatctcccggacgatccctccgcgtgcacgatttaatacacactacagaggaaaaccaaactgttgtctcttggtttaatatcgatggttctgcgctgctccaaattgagcaagaatcgctactattccactttcccaatgagaagtggtttctcgaagttgcaagcaacgctcgtctggttgaaccggtcaggggacaacataacccccttcggggatggcggtctcgagaggaagggtccttggaaccaacctggaatttcgggtttgaatgcgacacaagctcccaagttcatatcgtcactcaattcacgatccacgacaccgagggaatgtccatctcagccagtgagtccgtccccaaatagtgttcggttgcctccgatctgatataggcggtccagttcggcttggggactagcacctaagccgagagaaggaccactccgtaccttcgactccaagcgattggcgaggtgattacaaaaagtgattgctgactttaagacttggagttgtcatgatcattttgtggaaacttccgtacgaaactcaaacctcggctggttgtaaccgctgcgagtttcttcgataaccgcagcggctgattcttcatctcgcttcgagatgcattgagtccatcgctggtactcgtccgcaacttcttcagatgctccatctgcaatcaggtctccgttgtggatccagagtatgcgactgcacatgtccttcatcgtggttggcgcatgcgaaaccagaaaaatcgtcccggccgttactaggtattcgctcatccgctgctgtgcccgcgacttaaaggcgatatcaccagtcgccagggcttcgtcgacaagcagaatgtcgcggtcgacagcagtggcgattgcgaatttaagtcgagcgttcatccccgaagagtacgtccgcataggcctatcgacggcactgccaatgccagcgaaatcgcagatgtcttcttccagctctggaatagctgctgggagtgtcccctgcgcgagcaacccaagcctgatattctgccggcctgttaagtctgggcgcagcgcggctgagacgctcagcaatgtaggttgcgctgaaactagaatacggccgttagtgggctgttcggctccggcaataagacgcataagtgtggattttccggaaccattgcgtcccaacacgcccacggattctcccttcgaaaccgcgaacgagattcctttaagcgcctcaacatctagattgctggaaccctgccaaaaacgccgatcagatgccttatatattttggaaactctatcgactacaacagccggctcatcgcacctgcgcataacgcccctctgctaaccagaaatatgtgaaccccgcaatggcaacggtgactgaccaaacagccatgtacacccattcgtcagtagctggaagcgagtggtacatcactgccccgcgcacagcgtccaggaatcggtaggcgggattcagctgcatcgcatcctgaatgaattgcgagttatcgaatttctctgggaggaaaaagacaccggaaatataaaaccacgctcgaccgatcacgggaatgagcgactttacgtccggaacgatggccgtaagacgagcagttattaacgtgagccctaaaccgaaaacgtgaacaagaagaaatagcggtactacagcaagaatctcccaccccggccagttgccccattgcgcgcaaagcgcaagaacaattgcgaccattaccggagcgagactcgttagcacatttttcgtccacgcaccgaaaacgatagcggcccttggaaagttaaagcttgatatcagtggtttcgaggccttcatcagtcctgatccgctcgtcaaagactgctgtagaatacggaaaaatgtcgttccgagaattacgtatcccacaaagttctcaataccacgggacgtgttcagaatgacgccaaacataaacccgtacatcgcggcaaacaacaacggttccaagatgatccagagccgacccaggaatttgtcttggtgtagaccaaaggccctgtggtgagcatcttgataaatgaagaatcgatggccccaaagacgcttcaaataggaccctagcgcctctcgttcggactgttctcgtaacccggctcggttaatcacaataaaactgtcagtccgagtctcatgagcttcgtccagcggaaacaatgattgctcattcgcatcagcactcatccaccaattctccttttcccgcgccgaaggtcggatcaattgtagatgcgcgtccgagtatctaaaaatgattcgaagtgtagggcgaccccgcacaaaacgaacgataaatttcgtcgattgtcgccgctgcgctgtcccaagtgcgattacgcagccattcattcatagcgttctcactctcgggctggttctcgtcggccagagccgcgacaattgcttctgcaagtgcctccgcatcctctggaggaaaatagttcgcgaatccaccagtgacttctcttaaggccggaagatccgaggctataactgggatccctaacgccattgcagtgagcggtttaatgggggttacattgcgcgtgacgtcgctgttcacacgaggaagtacaaaaacgtctagggcagcataccacttccaaatatctgcctgcggtttcctgccaacaaagtgcactcgcccagcgagatcgtttcgctgcgcaaatttttccagatcggggcgcgcttggccgtcgccgacgactatcactgagattccactgggcagatactccaaggcctctatgagagtgtgcagcccttcataactcaccacggaggtcacggttccgaccaatgggcctttcaagccgcccaaaccgaggtcatttctaatactggcaacatcaaaccgcttgtcaaggattgatgcatcgatggagtttgggacaacaaaagtcttgtctggatcggcgccattgctgaccaagcgattcttggacacctcgctgagaccaatcacagcgttagctttacttatcgcatcattctcagcttccctcatccgtcgatattgctcagacctttgcgcgaactcacgatggtcactcggccgttttgagagccacgtgttttccaattcgcctcggacctcgtacacccaaggcagaccgaatcgctccgcgacggtgctgaccacattcgcgttgtggaaatcagtagtggtgtgcaataccgaaggcttcagttctcggaccaagttactaaggaggtcaactgattgctcgaacttcgcgctctcgtcgctactgactacccacggcaggagatggtggtaagtaaccgactctaccgtggtttgatctgatcccggccatttgcccacaataaccgggtagttgagacgcgtacacgcatccacatccacgcctttccgcctcaacgcaaccagcaagcgctgggtacgaactgtatatccgctgttggtatacggcagacagttattgaccacgtaaagagcgcgtgtcggctgtgcgggctgcacacggggtacaactctgtaacgaggttggtcatatccggcttcgattcggtcgattcttcgaactagcgcttgatcgccctggtctgctgcgaactgtcgagccgcggcgagatgaccatcgtcaagcaatctgtggccctcgtgagttgtgtgcgaaacgaccgtaatcgcaacatccagagccttttcaactacctctttgccgacgggcacattcaaccgcgcccattctctaaacttgcgcaaaaagtcggaggcattggtcgacacatgacgatacaccgctgaaacagtgagagtcaccaaacgaaggctgtgtttgattgtcatccgatccctcgtgcaacctcgatcaactccaagaaacgcttaggcacaacttcctcgcgttgagtcctcacccactgggttccaacgcttgaaacggctagccgagaccgatcgcgcgcgattgcgacccagagttgagccaagagctcaggcgattcggggggcactgtatctccagcacccatgtcttgaatgagaacggcagcttctccgctgactacgccagtgatgtggatcccctgcgccatcaactcgtaggtctttgatggaattgttctctcgagcggttcccagtcagtcaaatgaacaagcgctgaatcggcccacccgtagaactcgctaagatcggccgcaggcttcgtctcatagaactgcacagggatatcttcttggagcgcgagtttctccaaccgatcgcgggcatcccccgcacccacaacgcgcagttggacgtctacccccaagctccgtgcaatccgaaccgcccggagagcattgcctaggttctgcgctcgcccagcagttccagcgtaaagcacccgcagggcgttccctctttccgcgttgtccctgcgcctttgagcgtaggtctgcgctgggaacacgttgcggataaccgcaacattatttgaggctttccgaagtctcggatcgctgaggatttcatccttcatgccacgggtagtcaccatgacgcctgccgcataacgcaaagagtggttgatcgaccaagcagtgacggctttagtcaactgaagcggacccagtaacgcgagtttcgccctcagagatttcgtccctgtcgcgctattccagtgttccgagttcctcagcaagtctggccaagcatcacgcagatcaatgatgtacggcgcccgtaaaagtaaagccgctacccgtgtgacaaatgctgtaggcaaagcaggaacggtaccgataactaggtcgaaattatcgcagcgaggtgaaaccattcgcaacacttgtctcagttggccgccagcgcccacagcttgcgaggcgatcttcgacgtcagagttttccttgcaggagcaaagcccgagcggactatggtttcaccgctcggtcctgtctgcgtcttcccaacataatgccggttgagagagatgacggtaggtcgatcgatttcctcgttgtaactgggcggaggtgcgatgacagtgacttcgtgcccctcttgagcgagaatctgcgtcaaccactgccaccgccgttgagggacaccattttctggaaaccaatactgggtgacaatgaggattttcactgtcaccactccatttccatgaaaaatcgttacatctaacgcaccctaatgcgaaaaactagcgacgaatcatgccgcgagtatcaatgacatccttgcccgcaagaaccttggggtcgagattcttaaattcggagtggtcaaccaaaaccaaaataatgtccgcatcttcaagcgctgcatgaagatcggtgagctcggagttctccttgccatcgaatcgtgctgggagagcttgtatgttcggttcaaccacgcggattggcttgtcggggtactggtcagtcaaacgatccacaatatcgagagctggggattctcgcagatcatcgatgtcagccttgaaagccaaaccaagggcagcaattgacgcgtcaggtttccgttctacagcctctgccaccttacccagcacaaactccggcttggagtcatttgtctcacgcgctaaacgaatgagtttcgcctgttccggcacggaggacacaatgaaccacggatccacggcgatacagtgaccgcccaccccggggccagggttaagaatgttcacacgcggatgatggttggccagctcgatcagttcccagacatcaatatccagtttatcgcagatgagggagagctcattcgcgaacgcgatattaacgtcgcggaaggaattctcagtcaacttggccatctccgccgttgttgcgtcagtcataagcaactcggcgctgcaaaaagtcgcgtagaggtcgcgagccatctccgtaccgcgcggagtcaaaccaccgatcacgcggtcgttattctccatctcttccatgatctgaccaggcaatacgcgctctgggcagtgagcgatgtagatggcgttctcggcgtcctcctccagcgacaggtcgggccgctgctggatgatgtagtctgccatccacttggtggtgccgggaggagaggtcgattccagaacgacaagtgcaccaggacgaagatgcgacgtcatagcgtcgatcgccgaggcgatgtacttagtatcgacctcatggttggatcctttgaacggtgttggcacgcaaactatgtacgcgtcagccggaacctgctctgcctgggcaacgagcagctccttctccactacatcgcgcagaaggctatcgaagcccggctcgacgaatggaacctcaccccggttgatcgaatccacaaagcgctggttcacgtcaacgccggtgactttcacaccttttgaggcgatgaacgcggccgtgggcagaccaatatatccgagtcccacgacgcacactgtgtcgaatgtgtaaggagtgcttgacactattaccacctttgcttcattcaacaggttctctgtaacctgtccttaactaggaaatcttaccccccggttaccacctgcatggctcgggctggcctaggcttgggcagacaactgtggatcaaattctgccaggcgttctcccactcccgccagcgcggcaatagccccgacggctcgctgagctgcatttccgtcgccataaggattcaccgcgttggccatcgccttataagcggcatcttggtccatcaaattcgatgcctcggcgacaataagaccacggttggtacccaccagcttcacagtcccagccacaacggcttctggtctctcagtgttgtcccgcatcactaggacaggtttacccagggaaggagcctcctcttggactccgccggaatcggtgagaacgaggtaggaacgattcatcaatgccgtgaactggtcgtaagggagtggatccgtaatgatcacgttgcctaggtgctccacctcaggcagcacctgctcacgtactttcgggttcaggtgcaacggcaacgcaaagataacttcgggatatgcccttgccaagtcttgaaccgctccaccgatctccgtcattgcatcgagattctcgcgacggtgagtggttaccaaaaccacccgctggtctgtgtcggtcagcgcttggaggcgttcgtcctcgaatttgacattccaggttgtggaaatcttgagggaatcgatgaccgtgttgccggtgaccacgatgtcctttgagcgcacgttctcgcggcgcagattttccctggattcactcgtgggtgcaagatgcagactcgagacttgcccgatgatcttccggttcgcctcctcggggaacggagaaaaaatattccccgttcgcaaacctgcttcaaggtgaacgatcttcactccctggtggaaccccgctaaagctgcagccattgctgtggacgtatcgccctgggaaatgatcacatcaggtttctccttggagatgatctcatccaaccccgcaattgcacgagcaactagctcgttgagactctggccgggtttcatgagtccgaggtcatagtcaggaacgatgccaaacctgttattgacctgctcaagcatctcacggtgctggcctgtggaaacaacgaccgcgtcgaatcgatcatcgtcatttagtgcggtaatgacaggcgcgaccttgattgcctctggcctcgtcccatagacagtcatcaccttcggctttgatgaaatcactgtgtctccttgaaattcagctgtatcgcacagactttataggaactgagcgttgctgtctcaccatgtccgcttcccgcgccttgccctcggcccagtaccggtcctgggtggcgatgtcgacggtgccctcggagccgtcgaagaggtacggcgcccgcgattccatcttggtcacgaacgcgtgcgccacgtccgcgaacgtgaatgcgccgcgctcggcggcaagttcggcgtggaagaggacttggaggaggacgtcggcaagctctttcttgagctcctcatcgccagcctgttcctcgatcgcctgggctagctccgctgcttcctctttcaggtacggcagcaggcgttcgtgcgtcatggactgctcccactcccctcgcccacgcgcggtgtgcatgacggcaaccgcgcgggcgacggggtcgtccagggaaggggcacggacggcgtcaccgctgtcctcggttgtcagcgtccacttggcaccgggcacatacggccacacgcgcgcttgctcagggacctcgggcgtgtagtccacaccgcctgcgaattccttcgtaaggtgcgcgggcaccatgtctggccagcgggggtcgagcacgagcgtaggcatgcatgaaacaatagacgccatgacgaaccaactttcagaggcgcttgccgccgtcaaccccagccacgccgacgtcatggagcactccgtgactttctccccgctgcgctggaagaccggttggccgcaccacctgcgccgcgtcccgccgttccgtgacgacgcccgcgcctccatcacccgcgccgaggtcttcgacttcgccggcgatgtccgcgagtccggctacaaccgcgaccagatcatcgacttcctcggtgccgcgttcggctacctggccgggcagagcaaccaggtgatggagctgcaggcgttcctgcgcaacaagggcaacgccgcgaagcttttgaacgctatccgccagaccgagggcaagaacgccgttgacgcttacgctgtgctggcggaggccggcattgctccgaaggtcgcctccgccatcgcctacttcctcgccggcgagcaggcagagggcgagagcgacaagcccgtgatcatctgcagcaaccgcgcgaagatcgcaggtctcgagtccgacagcgattggtccgccgaggagtacggcgactacctcgcgcgccttcgcgaggcccgcgatgcacacgacgcgacgctggcgctggactccgtggagtacgccgcgcgcgagttcgcgaacaagtagcgccgattaccgctccgccgcgtgcgcccgcagcgcgcgggtgttgagctcccgacgggcctgctccagggccagtaggtcggagaacagcgcgttgtaggcggcctcgtcgtcggacgggcgcatgcgctgcagctgcgccttcaactgggcgatctggtcgcccacccgcgtttcctgcaggcgcgagagcaccgcgtcgatgtagacgtccaagttgtcggcgttgatcgcctccaccgccagctcggagacgaggttgcggccggccaagtcccgcatcccgccggccacagatgcgatccagttcgacccctcatggtcggcgatgccgcctgccgcggccatcgcgtcgcgcacctcccggtacgccgcgttggtgaacgcgtccgggttgatgccgtcgaagtagctgccagctttctccggatactgcagcgccgctttcaacgcctcgcgctgcggccagagcaccgggtcgttcggcgcgggcgccaccagcgcgttttgcccagtggaaccaccgtcacccccagcgcccgctgccttccgcgccggcgtcttcagcgcgcccttcttcggcgccttcgccgcctcgcgcacctgcgccagcacctcgtccgggttcggccagccaacccaccccgcgagtcggcgcgcgtactcgttgcgcaggactgggtcgtggatctccgcgaccatcggcaccgtgcggttcagcgcctggatgcgccccaccggggagtcgagcgaaaagtcagcgagcgtggactccagcacgaactcgatcatgggcattcggcgcgccaccagatcgcgcaccgccgcgtcgccccttgcctgccgcaggtcgcacgggtccatcccgtcgggcgcgatcgcgacgaaggactggccggtgaactccaggtccgttgaaaacgcgcgcatggccgccttctgtccggcgtcgtcaccgtcgaaggtgtagatcagctcgccgcggaagaagttgtcgtcgagcatgagccggcggatcgtctgcaggtggtcgcggccgaacgcggtgccgcacgaggcgacggcggtttgcacacccgcggcgtgcattgccatcacgtccgtgtagccctccaccaccacggcctggtggccctcggcaatatgcttcttcgccagatcgatcccgaagagcaccttcgacttgtggtacagcagcgtgtcctgggtgttcatgtacttgcccatgggatcgtcgtcgaacagcttgcgcgcgccgaagccgatcacgttgccagccgcgtccttgatcggccagattaaccgccggcggaacttatcaatcggcccgcgcttgcccatggagctgatacccgcctgctgcagttcctcggcgtcgaagcccttgcgcagcaggtgcttcgtcagcgtgtcccacccgtccggggcgtacccgcactcgaagtggtagatatgctcgcggctaaacccgcggttcagcaaaaactcgcggcccacctgcgcctcgggggtttctagctgctcgcggtagaactcgtgcgctgccttgttaatggctaacaggcgctggcgcgttcctggcttcacgtcccgcgcgccggtggtgccgccctggtagttgatgcggtagccgatttggtcggcaaccgcctccaccgcctccgggaaggtcagctgctccatctccatgaggaaggtgaacacgtcgccgcccttgccggtggagaagcagtggaagtacccgcgcgcggggcggacgtggaaggacggcgtcttctcgtccttgaacggcgacaggcccttcatcgagtcgtggccagcgggcttgagctgcacgtactcgccgacgatctcctcgatcgccgcgcgttcacggatcgcttcaatgtcgctctccggaattctccccttggccatgcgcctaacggtacaacctcaccccaacatcagaaagcaccgcttctacccgcgcactctcgcccgcaggcagctgccaatcgcgcaccacgagctgcttcaccgccccctcacgaatcaggtctgccagcccgtcgaggtttgtgggggcatcgcgggcgccgtcaagcactgccctggagagcgcttggagcagctggcttatcgacgccaccttccccacccccaccggatcccaccgagtactgcccatcgttttcctacctcgcaatctcgcagaacgattcgtagtggtcggccgtgtagtaccactcgcggcctgcaccttcgcccccggtgatgatgcggcgcgcgccgcggtggttcacaccaggcgtgtccaccgtgtactcgcggtagtaccccaaagactcctcgggcaggtggccctcatagttgccgaagcgctggtcgtcgtttgccgggtacttgtacggcccgccgcgctcgatcacctcgatcgtctcctcggcctgcgccggcagccgctcgcacgccggtatctcggtttccgtttcaaccggcgccgcgcaccccgccaccagcagcgctgccgccgccaacacccagcctttccgcatgtcgcacatcataggaccaacgtatgggcggacacacatagcggcatgtaggtgcggtgtcatacaatcccagtcaccctatgatgcacaccacttttgaaggaggattatgagcgcggtcgtactggcccttatcggcctaggaatgatggcactcgggtacctgctgtactcgaagtttttggggaccagggtctaccaactctcggacgcctacaccacgcccgcccacaccatgggagacggcgtggactacgtacccacgaacaagtacgtgctgtggggccaccacttcacctccgtcgcgggcgccgcaccgatcatcggcccggccgtcgccgtgatctggggctgggtccccgccttcctgtgggtcacgctcggcaccgtcttttttgccggcatgcacgacctcggagcgctctgggcctcccagcgccaccgcggccagtccatcggcacgctgtcgggccgctacgtcggcgcgcgcggccgcaacctcttcctcgtggtgatcttccttctgctgctcatggtcaacgcggcgttcgccgtggtgatctcgaaccttctgatctccaccccgtccgcggtcatcccgacctggggcgcgatcgtcgtggcgctcttgatcggccaagccatctaccgcttcaactggaacctgccgctcgtctccctcgtcggtgttgccgccctctacggcctgatggtctggggcgaccgcatgccgctggcgcttccggaggtcatgctcggcatcccggaccgcggctggtggatcatcttcctgttcacctacgcgtttatcgcctcccttttgccggtgtgggtcctgctgcaaccgcgcgactacatcaacggcctgcagctgtttgtcggcctgttcatcctctacgcctccttcttcatcgtccgcccggagatcgtcgccccctcgcttcgcgatgctgtgccggacggcacccccggcatcttcccgcttttgttcgtcaccatcgcctgcggcgcgatctccggtttccacggtgtggttgcctccggcacctcgtccaagcagctggataaggaaaccgacgctcgcttcgtgggctacttcggcgcggtcggtgagggcctgctcgcgctcggtaccatcatcgccaccaccggcgggtttaagaccatcgccgactgggagaacgtctacagcgagtggaacgccggcggcgtcgacgcgtttatcgccggcggtggcgcgctgatgaatgaaggcctgggcatcccgacctccctgtccgccaccatcctcgccaccatggccgtgctgttcgccgccaccacgatggactccggcgtgcgcctgcagcgcctcgtcgtcgccgagatcgccgagctcatgggcatcaagctctccgggcttgtcgcaaccatcatcgcggtcggcttcgcgcttgcgttgaccttctccaccggcctcgacggctccggcggcatgctgatctggccgctgttcggcaccaccaaccagctcatggccggcctgaccctgtcgattctggccattatgctcacccagctgcgccgcccgacgtggccgatcctcatcccgctgctgttcgtcaccgtcatgtccctgtgggccgcgatcctgcagctgcgcaccctgtgggccgcgcagaactggctgcttctggtcatcgacatcgtcatcatctgctgcgccatctgggtcatcgtggaggcgttcaccgcgatctccaaggcgcggagggcaccggccgttacctggcgcgacgacgagaccatgccgggcgagcacgccgcgcagccagctagcgtctaaaccatgtgggagaagatcaaggcgttcggggccggcctcgacgagttctacaaggccccctaccgccgcgagttcgcccgagccgcccgcgaggaggacgacctgttcatgctgctcgtcgcatcggagatgctgggcatccccaacccggcgagctactacacgctcgaactgctcccgctgctctacagcgacgtccacgcctggcacacccgcatgggcatggagaaatcccccctggacggtgtgcgatgctgctaaccaccgcgcccgtcatgttcttcggtggcaaaggcggcgtgggaaaaacaaccgtctccgctgcaacggccgtgcgcttggccgaggccggcaagcgcgtcctgttagtctccaccgacccggcgcacaacttagggcacgtgtggggcagcacgcttgccgacgcccccgtccacctcgagcccaacctccacgggatagaactcgacccggacaaaaccacccagcggcacctagacaccgtggccgcgtcgatgcgccacatgatgccggagcgcctccacagcgagatcgaccgccacatggagctctcccgccactcccccggtatgcacgaggccgccatgctcgagcgcattgcggagctcgtggcggagcttaccgacaagcgcggttacgaccacatcatcttcgacaccgcgccgtccggccacacctcgcgcctgctggaacttccggagatcatgtccgcctacaccggtggactgctcgcgcgccgcgaggcctccgacacgttttcgcgcgcggtgcgcgggttcgggggcaagggcgtcaccgactcaagcgccaccgagcgccgtaatcagcagattcgcgcgacgctgcttgcccgccagcgcaagttcgagggcttacgcgcagtgctgaccgacgcccagaagtgcgtcttcaacatcgtgctcaccgcggagcgcctgccggtgatggagtcggcggagctctaccgcgacatcaccgcaagcggcattcacgtcggcgggttagtcatcaaccgccgcacgcctgccggaggggaggcgtttttggagacgcggaggggcgtcgaaaagcaagcgctcgagctcctcgacaacctgctacccggggtgaagcgggtggagctgccctggctgccgggtgaggtggggacgcgggaggcgctggggggcgtcgccaagcacctgtagccccttagctgtaacccccgaacgccgcggccttcttcgcggcgcgctccaggcgcgactcggtcatggacgcgatctggtccacgatgacgcgctcgcgggcaaggtccgtctcggcggtgagccaccactgctgatacatcgtgtcgagagtgcccggcgcgcccgctgcaaggtagtcgtagacgcggaagatgcgctcgcgctggcggtcctggcgcggggtgtgggcgggcaggtccataacgtagagcacggcgatggttttgagcagcttgacctcggattcgatgtcggccgggaccaccagatcgccgtgcatgcggcccagcggggagtcgtttgcgtcaagggtcgcctgcaccaccccgccgacgtagcgcccaaccagctcgctggtgagctgcttgagctccacccatgactgcagcgtgtagttgaagtcggctgcgcgggagatggaggggagggattggaggtgggcggcggcgtcgataagcgagctcggcgagcccccgaacgctgccgcacccttgtccgccagggcggcgagctctacgaagtcccacaggactttgagcgagatgcgcccggagatgatgccgtcctcgacatcgtggacggagtaggcgatgtcgtcggcgaagtccatgacctgcgcctcaatcggcgggcgggcatccgtgtggccctttcgcacccaggccagaagctccgcgtcctcgtcgtaggccgagtacttcttgttcaccgtgccgtctgcgttggtgcgcgtgcgggggtacttgcacgcggcgtcgagggcggcgcgggtgaggttgagcccgaagctttcggcgcctatgaccaccttcggttccagccggctcaaaatccgcagtgtctgggcgttgccctcgaagccgcagttggacacctcgtccagcgcgcgctcgccgttgtgcccgtacggcgggtggccgatgtcgtgggagagacccgcaagctcgcagatgtccgggtcgaggcccaggccctcgccgatgctgcgcgcaatctgcgccacctccagcgagtgggtcagccgcgtgcgcggggtgtcgccgtcctgcgggccgacgacctgcgttttgtccgcgaggcggcgcagcgcggccgagtgcagcacgcgcgcccggtcgcggctgaacgcgccgcgagtatcggcgccggccgcgatctgggagcccttctccccctctaccgcgcggcgctcggcgtccgccgcggtgtattcgtacttcttcacgccttcccagcgtagaggccaagatgcgtgttggaggttgcgactaccctaggagggcatgaaacaccgttacctccgtgtcctccttgctgccccggcgcttgccgcaggtgtcggcctcgccgcggcacccgtggccatggctttagcacccgctcacgctgcttcggcgccggccgagtatgcccaggcccaggcgccagctcaagccccggctgtgtcgggcccgcgcctgcttacccaacccgtcaccgacgaggccggcgtgctgtccaccggcgacattgccaacattgaaagcgcgatccaaaaggtcagcgccgagaaaggcaagtcgctgcgcgtgatcttcctcgagtccttcggcggtatgcagccgagcgcctgggtggagcagtcgatcaaggccagcgggccgaacaccgcggtgctggcgatcgccccggaggagcgctcctactacgtcaacggcggtgagcagtggacccagaacgaggtcgacgccatggatagcgccgcctacgccaagctggcagaggaggactgggcgggcgcggccatcgccgcggctgacgctgcggtctccgctgggagcggatccggctcgggcggttctggcggcggcgacggcacaggcgccggctgggtcgccggcggccttggcgttgcggcccttgccggcggcggcatctacgccgcgaaccgccgcacctcgcagaagacgcaggccaagcagatcgagtccgcccgcgcgctggatccgtccgacaccgattcgctcggccgcctgccaacgccgacgcttgagcaggtcgcgcgcgacgcgctggtctcggccgacgagtcgatcacgcagggcaaggaggagctgcgcctggccaccagcgaattcggccccgaacgtgtgcgcccgttcaccgcggcgatgaacacggcgacctccacgctgcagcgcgcgttttcaacccaccagaagctctacgacgcgatccccgagaccgagcccgaaaagcgtgcgatgctggtggacatcatttcgtcttccggccaggccgagcaggcgctgcgcgacaagacggccgagttcaacgagatgcgcggcgtgctcatgcgcgcgcccgaggaggtggataacgtccgccagcgcaccgtggacatccgcgcgcgcctcgagcccgcgcagcaaacactgaacgatctgcgtgagcgctactccgaggacatgctccactccatcgccgacaacgtcgacatcgcctcggcctccctcgacgaggcggagaagcacttggacgaggcaagctccatcgcacggcagtcggcgggcaggcagggctcgcttatcgacgtcctgtcagccgccacccgcgccgtcgacatctccgacaccaacttggccgccatcgagcacgccgaggacaacatccgtcaagctcagacaaacctgccggccatcaaggccgagatcgaggacgagctgcgcgagatcgagcaggtcaaggccgcaacgcagcagggcgcgcgcatcgacgtcgccgccctagacaacgtcgccgccgccgcccgccaggtgctcgccaccgtcccggcccgcgccgatcgcgacccgctgtccctctacacggacttaacggacgtggacgcgcgcattgacgagcagctggcgattgccaagggcgccgccggcgaccagacccgttccctgcagctgttcgaccagcaaatgcgtgtcgccaccgcccagatccagtccgcggaagacctgatccgctcccgcggccgcatcatcggctcgcacgcgcgcaccttacttgcagaggccaagcgccagtacgcccaggctcaccagctgcgcgtgcgcgacactcgccaggcaatcgacttcgcccgcgccgcaaccgagacggcgcgccgcgcggcgaaggcagcgagcgacgacatagaccgctaccgcgcggcgcagaaccgccagaccgcgaacaacgtagcgcaggccgtgctgtggggctcgatcctctccggcggcttcggcggtggtggcggctacggcggcggcaccatgggcggcggtttctccggcggtggcggcggcccggccggccgcggcggcacgttctagtagcgggtgttattcacgggggtgtcgacaagcagcagccccctcgcgatgaactccaggtcagcgcgctcctcggcgctcgccacccgggtttccagctcgatctcgccgctcgggcgcgcgagcgtgacaccgacgaggttgccggccgcgtcggttatctcgcggcgcttgcgcaacaggccccctcccgcgcgacgcacgctataggtgcggccggcgcactcggcctcgtagtgcgagacggttaggccccgtttggtgagtcggtaggtgcgcccgtccgcggccacggcgcggatgtcggccgggttgtcggaggtgaagcgcagcggttcccgcgtcacaggaagaacaccaggactgcgacggcggagaacagcgtcagcgcggcaatcagcgcgttcgccgaggcggtctggcgagactccatcacgctgcgcgagagccaggcgagcgccgcgacatccgtcagcggcagggcggtgtcaccttcgaactcgaggatcgccttgcgcacgcccgagttcgcgcgggagaactgcgcgaccttttcgccggcggcgtcgtcgatgacccagttgttggacgtctccttgaccagcgtgtagccgcggccctccacgtccacgcggacctcgtcgccgcggcgcagcgagtcgaacgcccgcacgatctcctcgccgccgcgcgtggccaccgccccagattcaggcgagaccgctaggtcccagatctccccgcccacgctcgcgcggtcggtgcggaacacgccgagcacatccggacccgcctcggcgagcagcttcggcgcgtcgcgctcggtgcggtcccagctgacgtagtgcatcgctattgcaaccccggcttagcagccgatcaggcgggccgccaggtaggactcgagctccgcaagcggcacacgctcctgctccatggtgtcgcgctcgcggacggtcaccgcgccgtcttcaagcgaatcgaaatcgtaagtcacgcagaacggcgtgccgatctcgtcctgacggcggtagcggcggccgatcgcgccggaggtgtcgtaatcgacgttccagtgcgcgcgcagggtgtccgctagctcctccgccgggccggagagttccggcttcttcgacagcggcagcaccgcaaccttcaccggcgcgaggcggcggtcaaggcgcagcacgacgcgggtatcggtgccgcccttggcgttgggggcttcctcttcgtcgtacgcgtcgatgaggaacgccatcatcgcgcggccgagacccgcagccggctcgatgcagtacgggatccagcgctcgttcgcctcctggtcgaagaagctcaagtcctcggccgaggcctcggcgtgcgtcttcaggtcgtagtctgtgcggttggccacgccctcgagctcgccccacttggagccggtgaagccgaaggcgtactcgatgtccacggtgcgcttggagtagtggctgagcttctccttcgggtgctcgtacaagcgcaggttctccgggtcgatgcccaggtcgatgtaccactggtggcggttgtcaatccagtactggtgccactgctcgtcctcgccgggtttgacgaagaactccatctccatctgctcaaactcgcgggtgcggaaaatgaagttgcccggggtgatttcgttgcggaagctcttgccaatgttggcgatgccaaacgggggcttcatgcgcgcagacgtcatcacattcttgaagttcacgaaaataccctgagccgtctcggggcgcatgtagtgcagcccctccttgtcatccaccgggcccaggtaggtcttcataagcccggagaactctcgcggctcggtccacttgcccggctggcccgtctccgggtccgggatgtccgcgaaaccgttgaccggcgggtggccgtgcttctcctcgtacgcctcgagcaggtggtcggcgcggtagcgcttgtgcgtgtgcagtgactccaccagcgggtcagtgaacacctcgacgtggccggaggcctcccacacctggcgcggcaggatgatggaggtgtccacgccgacggtgtcgcggcgcgactgcaccatgtggcgccaccactggcgcttcaggttttctttcaactccacgccgagcgggccgtagtcccatgcggagcgggtgccaccgtaaatttcgccagcggggtagaccaagccacggcgcttgcacaggttaactacggtatcgatcttattcgcgggcactggctccaaagcctcctcttggcagtgatcaagtaacgtgctcagtctagcgaagcgggtagacccacgaacgaccacggtgaggaatgcttttcgctattttctaactatgagcgttcgacgacagctggacgcgcgggagatcgagctcaccgcgcagctgctgagcgccttggactccgagctacgactgagtttgctgttcctgcttaaccgcgacgcccgcgtcgtccaccaactcgtcaccgagctaggaaaatcgcagccgttgataagccagcacctgcgcgtgctcaaagccgcggggctggtcacgtctcgccgcacaggtcgtgaggtggtgtactcgctggcgcagccaggcatcgtcgatgtcattatggagctcgccacctacgcctcccccggcgcgagcgcgttctcatccgtttccgcgaccatgtcgtcggcctcggcggtggcgatcatcgagccgccgatgcacccgcgtccaggcgaggacccaggcctctacccgcagacaccaaagccgcagcgggactaagctcgccgcttatggacgtccccaaactcggcccccgcaccacccgccagcgcaccgccgtcgtggaaacgctccaagccatcgaccgcttcgcgtccgcgaagaccatccaccaagagctggaagcccgcggagagaaggtggggctgaccaccgtctaccgcacactgcagtcgctggcggagaaggaagccgtggacgttttgcaaacgcctgagggcgaaacgctctaccgccactgcctcaccgagcaccaccatcaccacctcgtgtgcaccaagtgcgggcgcagcgaggaagtcgaaggcgggcccgtggagaggtgggcggagctcgtcgccgcgcgctacggctacaacctcgtcggccacgacgccgagatctacggcgtgtgccgcgcctgccaggccccttagcgctgaccagcgctaaggggcaaatttgtccacagcgccgccgaagcgacggtcgcgcttggcgtactccagcacagcgtcgtacatgtgctgcggcgtaaagtccggaaacagcgtgtcctggtagaccatctccgcgtacgccgattgccagagcaggaagttcgacgtccgcttctcccccgacgggcgcaggaacagatccacgtccggcatgtcgggccggtagaggtagcgcgacagcgtctcctcggtgacgtcgccggggtgcaggcggccctcgttggcgtctttgatcatggaccgggtggcgtcgacaagctctgccctaccgccgtaattgatgcacatcgcgagtgtgacaccggtgttgtcgcgggtcagctcttcggcttcctcgagctcgcgcagcaccgagcgccatagccgcggcctgcgtcccgcccacacgatgcgcacgttcttctcgtggagctcgtcgcggtgtcggcgcagcacgtcgcgggaaaaccccatgaggaagcgcacctcagagtgggagcggcgccagttctcggtggaaaacgcgtacgccgacagccactccacatgccccagcgcgatgcacgcgtcgacgcaatccatcagcacactctcgccgcggcggtggccttcggtgcgcggcaacccgcgctcctgcgcccaccggccgttgccgtccatcacaagcgcgatgtgcttgggaatgaactcggggtcaatctgcggcggggcgggaaacgtcatgccacccattattacgcctgctccatgatgcgaagcgacttcagccccgattccacgttgtactgcagatgcgccaccgtgagccggtggaccacggcggtaagggcggcatcgtccgcgggcagcgggtggcctccccggatcaaccacatcgcgtgcagcgcctccgggtccacgtccgctgatccgcgcgggcggcactcagcgcacaccgcgccgcccacagccgcgttaaacgcgcggtgcgggcccggcgcgccgcagttcgcgcagtcgaacaggcttaagccccagccggcgtgctcggtggcgcgcaggatgaacgcgtcgagcaccactgtcggcgtttcctcccccgcgcggatgcggcccagggcctctgcgacgaggtcgaagagctcgggatcggcctcttcgtaagccagtttctcggcggtttccatcacggcgcaggcagcggtgtagcggtcgaaatcatcggtgatggtgtgcccgaagtaggcgacggtgtcggctgaggtgatcgtcgataagcctgatgccctttttggcgggtagatctgcgcgtcgatctccacgaagggctggagcctggagccgaagcgggacttggctttgcgcacgcctttggccacgccgcgcaccaggccgtgggtgcgcgtgagcaagacgatgacgcggtcagcctcggcgaagtcgtacgtgcggacgacgaaggcgcggtcgcggaaggggttagaagccaagtcggccgagcgccttcgggtcggactgccagttcttcagcactttgatgcgcaggtcgaggtagacgttgtggccgataagctccatgatctgctggcgcgagcggtgcgtgatgccgctcaaacgccgcccatctgggccctcgaggatcttcttctggcccgggcgctcgaggtagatcacggcgtagatcatcatgcgcttgggatcgcgctcgtcggcttcgtcgacgtgcatctcgtcgatccgcacagccaccgagtgcggcagctcctcgcgcaggccctgcagcgcttcttcgcggatcagctcggcgatgcgggtttccatgtcctcgtcggtgacgtcgccctccgggtagaagcgcgggccttcgggcagctgggacaccagcacgtcaagcagcacgtcgagctgcacctgctccgtggcggagacgggcacgacctcggagtcctcgcccagcatctcgtgcagctcgatgaggcgctcgccgacgacgtcttttgccaccttgtccagcttggtcacaatgcccaccactggcgcgttcggtttgacggcccggatctgctcgaagatgaagcggtcgcccgggccgagcttttcgtccgccggcacggtaaacccgatgacgtcgacgtcggcgtaggtgtccttcaccacgtcgttgagccgctcgcccaaaagcgtgcgcgggcggtggatgcccggggtgtccacgatgattacctgcgcgtcatcgcggttgacaatgccgcggatcgggtggcgggtggtctccggctggtccgccataatcgcgatcttctcgcccaccagcgcgttggtcagcgtcgacttgcccgtgttcggccggcccacgaacccgacgaacccggagcggaagccgtcgggcgtgtcggtgaaccctgcgtaatccgcaggtgcgctcgcgttcgcctcggcgggcaggtcgtcgaagtcggggaagtccgggaaatcgctcatggacaccaagtctacttgggtacgtttggggcttatggctgtgcgcattgtgctaatgggcgtgtccggctgcgggaaatccaccgtcggccccgtggtcgcgagcgcgcttggcgtgccgtatctcgacggcgacgcgctgcacccgcccgcaaacattcagaaaatggcgcagggcattgcgcttgtcgacgccgaccgcatcccctggctcaccgacattgccgaacacctcgccgcaggcagcgaaggtgccgtagtgggatgctcggcgctgaccaggcgctaccgcgacatcatccgcgcccgcgtgcccaatgtggtgtttgcgcaccttgacggccgcgaggacgtcctgcgcgcgcgtctgggagcccgcgaggaccacttcatgccggcgtcgctgttagattcccagctagccacgttggagccgctagccgacgacgaggcgggtgccgtcttcgacatcgagctgccggctgcggagatcgcccgccgtatcgttaaatgggtgacatgagtacgccacacactgcaggaattgccgccaccttcgactgggatctcgccgagcgctacggcgagatcctcgccttcggcgcccgcgaacgcggcgaggacgccgtgtcggtgcctgggcggttatcggagaacccgttcctcaccggcgtcatggccaagcacatcacgatgggtattcagaagacgggcgtggacgggcaagcggtgttggcgcctgcgtctgccggcgagcgcgcgcttcgcgagcacgacctcatccccttcgagatgtccatcaaagacggcaacctcgcccgcgtgcaggtcggcgtttctgagggcgcggcgggtgctgagcgtgtgttgcgcgacgagtggggcttttccggcttcgtctctgaagacgcgcccgccgaggttgccgccggctacgaggacgagctcgccgccataaccgaccgcacggtggtgcttttggacaacgctgcgggtctgttgccgctggatcccgcgtctgcgagttcggtggttatcgtcggtgcttccgacttggcggagcatctgcgcgctgcacttgcggagctcggcgctgacgctgatgtgcgcgcggcaggtgctgatagtgatgttgatgcggcgggcgctgttgtggtcgtggactgcgcggattcttcggaacttcggcggttgggtggggctttggcggtggtggggtgctttggggcgtcggcaagcaatgcccctgccgttgtccgggcgctgactggtgctacgaacccctctgcgaagctgccgctcgcgttgcctggttacccgtttggggccggcggcagctacaccacgtttgagcttggccgtcccgaggtcgctcgcgaggtgcgccgcggcgacgacatgtttgtcgtgcgcgttgacgtgacgaacacgggcgatcgcgcgggtgctgaggtcgtgcagatctacgtggacattcctggtcagccggagcgtcgtttggtcgggttccgcagcgtcgaggttgctgccggtgcttccgagaccgtcgagatcgagatgggcatcgattggcccgaccatccgtttagcgtctgggacgaggatgcgcgcgagtgggtgacgccgcggggcacgcacgtgctgcacgtggggacgtcgtcggtggacacgccgcacgcgcttgaggtggagctttaggcgtgtagttccttggcgtcgaaccgcgagcgcggttccaccagcaggttctggcactgaaccagcggcaactcggggaggtcgcgctcgcggacttcggtgacgatgtcgaacatcgaccctgcgaggtgggtcaggcgctcttttggttcttggtccgcgagcgccgcgtagagcgccgtcgcgagatcgcccgcgccgaccacgttgccgccgagtcgcggcgtttcggtgaagtaggtgctctcgggggtgatgtcgagcagcccgagggcgcccggcttgtcggcggcgaccgaggtgaccagcgccgtgtctttgaggttgcgcgcggcttctgcggtggctgccggggagtctaggttctggcccgtgaggagcgagagctcccactggttcggggtgatggcgtccgcgagcgggatgaggcgctcgcggaagacatcggggatctcgggcgcgacaaacgagccgatctgcgcgttgccgatgacgggatcgcagatgtagcgcgcgttggggttggcgtctttgatgcgcgtcaccgcgttgtggacgacctcagcgagctccgccgagcccaaataccccgagacgaagacatctacctgcgggtacgcgaaggcgaagccgtcgaggatgccggcaacctcgacgggtgtcatcaccggcccaccccagtccgggtactccgtgtggttggagaagttcaccgtgtagacgggccacacctcgtggcccaggcgctgcatggcgaaaacggcggcggagttgcccacgtggccgtatgccacgtgcgactgcaaggagacgatgttcacggctcgatcatacgaaccggccggattgcgccgcgcataatccgcttggaacgacccgcatatggtcaccgccagatggtcaccagtaagtggtgaccggcaaaaggtcattagccgagtagctggcacccgcggggacgcggtgctgtcggttaatgaccttcttccagcaacactttgctggtgaccgtgtggaagaacatctccaccgtaagccagtcagagaaacgatcagcgtgtcaccgaggctagagatggggcatgaggtgggcgtcgaacaagttctcacaggcatttcttaggaacgcaccattgattcgtacgtgagtccagcgttacagtagccacacttctgtgagcttggacatactcgtccactgatctggaaaggattacagtgcccatttacgaattcaaatgcgtcgatggacatgtcaccgacatgcagctaccgatgtcgagcgagacgcgtgagatcaactgcccggactgcgggtcgcaagcacgccggttgatcagcgcaccgtcggtacgccgtgttgatgccggcctggccagtgccgtggaagcgacacagaagagcgcgtacgagccgcaagtggtctcgtcgctacccagcgctggcaatgcgcgcgtcacgaaagtgacgcacaacccgcagcacgcgaaattgccccgcccctaaccaacccctcaaggaggcactgcaatgccaaagaatctcttccccctcgactcatccaaacgcttcgccgatcaagaaatcgtcggtcacaaccgttggcaccccgacatcccgccggcggtgaccgtacaacctggcgacaccttccgtgtcgattgccgcgaatggttcgacggtttcattaagaacgacgactctgccgacgacatccgcgacgcgccgatgaaccgcgtccacgcgctttccggcccgttccgcatcgagggcgcgaagcccggtgatctgctcatcgtcgacatcctcgatgttggaccgattccgcaagaggagggcgagctcgcgggccagggatggggctacacaggaatcttcgccaagaaaaacggcggcagcttcctcaccgatcagttccccgacgcttataaggccgtgtgggacttcaccgggcagaccgcaacgtcgcgccacgtcccgggggtgagcttcaccggtatcatccaccccggcttgatgggcactgccccatctcacgagctgctcagcaagtggaataagcgcgagggcgagctcatcgctaccgatccccaccgcgaaccgccgctcgcactgccgccggagccagacgaggccatcttgggcacactgactggcgaggacttcgaccgggtcgcagccgagggtgcgcgcaccgccccgccgcgcgaaaacggcggcaaccaggacatcaagaacctgtccaagggcacccgcgtgttctaccccgtctacgtcgacggcgcgaatttctccgttggcgacctgcacttctctcagggcgacggcgagatcaccttctgcggcggcattgagatgagcggttacatcgatattcacgtcgacatcatcaaggacggcatgaaaaagtacggcgtggaggaaaacgccatcttcatgccgggcaacgtggagccgcggtacagccagtggttggcgttctccggtacgtctgtcaccctcgagggcgagcagcgctacctggactcccagctggcgtaccagcgcgcctgcctccacgccatcgactacttgaccacgttcggctggtccccggagcaggcctacctcctcctcggcgccgcgccgatcgagggccgcttctccggcgtggtggacatcccgaacgcgtgcgcaaccgtgtacttgccgacggaaattttcgacatcgacattcgcccaggcgcgggcgagacaccgaagatcgacccgggcatcggtgcgccgcgctcgagcttctagcggtcggcgcggtgcagaaagctggagttgtaggtccaggtgtgtatagcaacctgcccacttggggttttgagggagaactacaactgtagacctacaactcgggagaaacaggcccggctgcggcctaagctacagcgcctcgacggtgaactgctttgccgggttggcgaagaactcctgggactccacaagcttgagttcccttgagtcggcctcgtgggtgagcttcagcatgtcgtagacgctcgaggcggtcttggccagcgcgtcagcggcgtcgcgggaatccaagtagtggccggtgaagagggcggcggtcacgtcgccggagccgttgcgcttgaacggcaggcgcggggtgcgcacgatccacttgccgcggtcgtcgacggcgatcatttcgatgacgtcgtcgccggcggtttccgggcgctcaacggaggtgacgagcacgattgacgggcccatctcccgagcggcgttgacggcggcgagggtggagtcgagatcggtgacgtcgcgctcggtgaggtagcccagctcgaactggttgggggtgatgaggtccgcgaccggcaccacgcgggaacgcagcagcggcgggatggtgtccgcgacgtggcagcccgactttgcgttgcccatcaccgggtcgcaagcgtagatggcagacgggtgctgctccttgacacgggcgacggcgtcgatgatcacgtcggcaatgtcgtcgccgccctggtagccggagaggacagcgtcaacgctagcaagcgcgccgcgctcgtcgatgccgtcgatgacggctgcgacgtccgaagccgggatcattgggcccttccacgcgccgtacccggtgtggttggagaagttcacggtgtgcaccggccacacctcgtggccgatgcgctgcagcggaaagacggcggcggaattgccgacgtgcccgtacgccacgtgggactggatggagagaatgttagccatgggggttattgtgcccccgcaggtctaaccctcttgtatcggggcgggttcgtccgcgggcaccggcacctcaacgagcacggaacgggtcttgacgcggccgcggcggtcgcgcccgccctcggcggtgtaggacaccccgtccatcgtgatggacgaaccaggcaacggcacacgccccaactcgtaagacaacaggcccgcgacggtgtcgacggaatcgcgcacttcgtcgtcgtactccagctcgtaatcgaggtggtcggcgaggtggtccacgaggtcgtccagcggcaggcgcgcctggacgcgcatgaggcgctcgtcgatgtgctcgattggggcgacctcgtcctcgtcgtactcgtcggtgatttcgccgacgatctcctcgaggaggtcctccatggtgaggaggccggcgacggtgccgtactcgtcgataagcactgctatgtgggtgttgacccgctgcatctctttcagcagcacgtcgagcggcttggagtcggggacgaaaagcggttcgcgcaccactttggtgacggcggtggacggctcgatcggggtgccgccctcgccgaacatgtccttgagatacgccacgcccacgacgtcatcgacgtcctcgccgatcaccggaacgcgcgagtggccggagcgcaccatcaagcgggtggcctgtttcgcggtcttgtcgtgctcgatccagatcatctcggggcgcggcaccatcacctggcgggcgtgggtggaggcgaggtcgaaaatgttctggatcatgcggccctcagtggtttccaccacgccctgctcctgggcgatgtcgaccatctcccgcagctcaacctctgtggagtacggaccgtcgcggaaatcctcgcccgggtggaacaggttgcccacgcggatcaacagcccggagagaggtcccaggatggtgtggaacgcgaccagccactgcgaggccttgagcgagatcgagtacgggttgcgcttgccggcagtgcgggcgaaaacgccgatgatgccgaactgcagcagcgtcaccaccgcaatcgcagcggcgattgcccacgcgtctgagtcgatgaggtccatcgctagcatcgcggcgaacacggcggccaccacgtccaagatggtgtgcagcatgaccagcgtgttgatgtggctcgcgcggttgtccaccacgcgcagaagcgactgggaaccgcggacgtcgtctttgaccatgttctccacgcgcgcccgggaaatcggggcgagcgcggactcaaccgaacctaaaagccccgaaagcagaagcgcgatcaccgtggtgagcgcgtacgcgacggtcgcctgcacctactgccccgccttcatcttgcggtcgagctcgtcgcggtcggcggccgaggggaaggcgtgcgcgcccgtgggcttcggctggtacttcaccccgcgggaagcgagcgagtcgtaccactcggccaagatctcgttctgcagcgcgaacatctcgcgctcgtcctccggcgcgacgtggtcgtaccccagaaggtgcagcacaccgtggacggtgagcagcgccatctcgtgggcgaggtcgtggcctgccatttcggcctgcttgcggtcgtaggccgggcacaaaatgatgtcgccgagcatcgcgggacccaagtccttggcgtcggggcgcccgccgcccggggtgagctcgtccatggggaagctcatcacgtcggtggggccctcgaggtccatccagcggacgtggaggtcggccatggtggctttgtccacgagcgtgatggtggtctcggtgtcggggtggacgtccatcgcggtcagcgcgtaggagcacacgtccacgagcatctcttcgttgacgtcggcctcgccggactcgttcagtacttcgatgctcacttggtgtcctccccggcagcgtcgttaagctcttgctccctctcgcgctcgatctcgcgctggcgcttctcgtagcgcgcggcgttctgcgcgtcgtggcggtcgtaggcggcgacgatgcgcgagatcaggtggtggcgcaccacgtcgtcggcgtgcagttcttggaagttaatgccctcgatgtcgccgaggatgcggcgcgcgacgcgcaggccggagacggtcccgcgcggcaggtccacctggctcacgtctccggtgaccaccattttggagccgaagcccaggcgggtcaaaaacatcttcatctgcgcgccagtggtgttctgggcctcgtcgaggatcacgaacgcgtccgacagcgtgcggccgcgcatgtacgccaagggcgcgacctcaatgatcccggcctcgatgagtttggggatcatctccgggtccatcatgtcgcgcagcgcgtcatacagcgggcgcaggtaggggtcgatcttgtcgctcaacgtgccgggcagaaagcccagcttctcccccgcctcgacggccgggcgggtgaggataatgcgcttgacttctttgttctgcagcgcttggacggccttcgccaccgcaagatacgtcttgccagagccggcggggccgatgccgaaggtgatcgtgttgtcgtcgatcgcgtccacatagcggcgctgtccggcagtcttcgggcggatcaccttgccctttcgcgcgacgatctccgcgccgaggatctctgcggcggactcgggcgcgtcggtctccatgatccgcacggcgtgcaccacggtgtcggaggtcacgggaacgccgcggcgcgccatcgactcgagttcatctagaacgcgcaacacgtgcgccacgcggtggtcctcgccgcgcacggtgacggtggtgccgcgcgcgtgcacgtccaccccaaggttctggttgagtacccgcaggttctcatcgttgatcccgaggacggattgcgcgtacgccgaatccagatcgatcttgcgggtaacaagttcttccataatgccactcagactaccagcgagctgttctcactccgatcgcgcagagcccggcaaacgcggcactcgccgtgcgtagaacctcgggcccgagcttgaccggggtgccgccgatcaactccagctcgtccgcgccgatgccgccctccggcccgacgacgaggaagagctcgtccgcaaggtcgacatcctttaaagagacggtcgcgtcctcgtgcagcacaagcttttgcttgtcgacgccccccagccaccccgagcccaccggcatcccaacttcaggaatccatgcccggcgcgactgcttcgcgctggcgaccgcctggttgcgccacttctccaccagcttggcctgcttgttctcgggccagcgggcgatggtgcggtgtgagatccacggcaggatctcgtcggcgccggcctgaacggcgaggtcgacggcaagctcggcgcgctccgacttcggaatcgcctgcaccaccgtcacgcgcggcgtgggcgccggcaccacctcctccgcaatgacgtctccgcgcagctgcgacttggtggtgtgcgtgacggtgacggtggtggtgagcccgtgaccgtcggtaagcacgatgcgctcccccacctcgatgcgtttgacgtgcgcgtgctgggcttccgcaccctcgagcacgccggcgcgcgggtcgggtgagacgaagtacggcagcgacactagcggcggaaccgatcgcgcatccgggagaagaagccctcgtgcgcggggccgtcctccgtgtggacctcggtgttgtcagcgctgccctcgcgcaggtcgcgcaaagcgtcgcgttccttggcgctcaggtcagtcggcacgacgacctgcacctgcgcgaccagatcgccgaagcggtcggtgcggatctgcggcatgccctcgccgcgcagcgtgatcgcatcgccaggctgggtgccggcgggaacctcgatcagcgtctcgccgcctgcgaggttctccaccgcgatctcggtgcccagcgccgcgtcgtacatcggcacgttcaagcgcagcagcaagtcgttgccgtcgcgcaggaagtacgggtgcggctcggtctggacctcgacgtagaggtcgccggccgggccgccgccgtggccgacctcgccctggcccgccatgcggatgcgcatgccggaagcgatgcccgccggaatgttcacggtcaggtcgcgggtggcgcgcacgcggccgtcgcccgcgcactggcggcacgggtcggtgatgatctcgccgtagccgcggcacttcgggcagtcgcgggtagtcatcacgttgcccaagaacgactgctggacttcctccaccgagccggtgccgtggcagtagtcgcaggtgactggcttcgactcggtctcggagccggtgccgtggcacttgtcgcacaccacggcggtgtcgacggcgacggtctgcttcacgccggagtaggcctcggcgagcgtgacggtggtgcgcagcagggcgtcgttgcccggctgcacgcgcgaacgcggctggcgggtttggcccccgccgccgaagaaggcctcgaagatgtcgcccaggcccccgccgaagccgccgcccatgcctccagcagcctggtccattgggtcgccgccgcggtccacgatggagcgcttcttcggatccagcagcacctcttgcgccaacgaaatctccgcgaacttctccgcggcctcctcggacgggttcacgtccgggtggtacttgcgcgccagcttgcggtacgccttcttaatctcctgttcggtggcctcccggtcgacgccgagaatgccgtaataatcccgagccaaaatccttttccctcctactcgccgcggagaatgcggctgatgtagctcgccaccgttgcaaccttttgaatggtactcgggtagtccatgtgcgtcggaccgacaacccctaagccaccaagcgcctcggcgccagctccgtacgctgtagtaacaacgctggcgcgggataattcctcgtcctcgttctcgctgccgatgcgtacggagacgtgctcgagctcctgcgcgctggcgagcagcttcagcaccaccacttgctcctccagcgcagcgatgacggagtttaagtcgcccgcaccgtagagggtgaggttgccggcgccggcgattaacagccggtcggaggtggtggccaccagcgtgtcgatcagcaccgcggtggcgcggcgggcggcggcctgaatttgcgccggcgcccgagtgggaagctcggccaacgactccgcggcctctttgagcgtcttgccgtcaagcacctcattgagcagggtgcgaagaacccgcacgccctcgtcgtccaacggcgcgtcgagttccacgttgcgctggtccacgcggcccgagtccgtgatcagcacgagcaacaggcgagtcggggtgagcgcgaccacctcgcagtgcttgacgcggctgacgttcagcgtgggcagctggaccacggcagcctggttcgtcagctgcgcgagcagggtgacggagcggcgcagcacgtcctccatgtccaccccggagtcgaggaaggtcatgatcgcgcggcgctcggcggacgacagcggcttgacgtcgtgcagcgcgtccacgaacgcgcggtagccggcctcggtggggatgcgccctgagctcgcgtgcgtctgctcgatgaagccctcgctctcgagcacgttcatgtcgttgcggactgtcgccgggctgacctttaagttgtggcgctccaccagcgctttggagccgactggttcttggctggcgatgtagtcggcgacaatcgcccgcagcactgcccttcgtctcgcatcagccgcactcatgggctacagggtaccgtccgcggttgcgggtggttcttgggcgaggatgtcggtgacgatgccgtcgacaagcaacctgcccttgtccgtgactttgagccgctcgccgcgggtgacaagtccgagccgctcgtgtttttccgtgggcgcggtgaccagcgccgacgggatgccttctttgaggcgcaggcccagcatgaccgcctcgaagtgccggatgtcgtcggtgagctcttcgcgctcggcgacgggcagctcgccagcagaaagcacgtcggcatagcgctccgggcgcttgacgttgtagaagcgctgcttgccgacgctactgtgcgcccccggacccgcgccccaccaactgccgccgcgccaatacaaaaggttgtgctcgcactcgccgccgggcttggcccagttggacacctcgtaccagtcgaagccgttctcctcgagcgatgctgcgatgagctcgtagcgggtggcgtagacctcctcgtccggctccggcagctggcctttgcggatcttgcggctcatcgccgtgccgtcctccacgatcaggctgtaggcggagacgtggtcgacgggcgtggataaaatggcgtcgagggttgcgcgcacgtcgtcgtcggtctcggtcggcgtgccgtagatcatgtccaagttgatgcgcgcaaaacccgcctcgtgcgcttcgcgcgcggcggcggtggcgcggcctggggtgtggcggcggtccagcactttgagcaccggcgtggaggccgactgcatgcccagcgacacgcggttgaagccgtggcgcagcaggccctcgaagtaggcggggctggtggactccgggttggattcggtggtgatctccgcgcccggtttcacgccgatggtgttgcgcgcggcggtgaggatgcggcccaaaccgtcggcgccgaggatgctgggagtgccgccgccgatgaagacggtgtcggcgggaccgaaaccctgggatgcgagaatcggcgcggcgagctccaactcgcgctccaacgcgtcgaggtacgtcgcgtgggacgtgtccacctcggttggcgtgtaggtgttgaagtcgcagtacccgcagcgcgacgcgcagaaggggacgtggatgtagatgccgaaaccgctcacgcctagctaaggtacagcgcgcttacgcgccgcggcgattgcgcttcgcagcgacgcgggcgaccacggcgtcaatgcgcgcgcgctcctccaagaactccggcgggttggagccgcgcatcgtgcgggtaaacgccgggtggtccatgcacacggtgtccatccaaccctccacggcggcctccaccagctcgccggcgcgggcgtagaggtgcggcagactgaccgcgcccagctcgcgggcgaccatctcggtctgctccagcacgtaagcgacgacctcgccgatgtgctgcaccaccaagtcggtgcgcccggtcagggcgtcctgcatcgtctgcacggagtacggcgcttcgagcgggaagaggtcaatcagcccgctgccgtcgaggtactccggctcgggaattttctcctccggccccgcggtggccgaaagctgcccggcgcgcatcccggaggtgagcgcttggcgcagcccgatcagctcgccgaccacgcggcgagcgtcctggcgcgcgtcgtcgacgatttcggagaactcggccaggcagtcgtctgcaagctcgccgtcgtaatccgcgatcgcctccgcgatgtgctcggcgtattccgcaacctcgtcgccgatgttgtagatctcctgtgtcagttcgcggtggcgcagcacagcggcggtcttgtgcatgtgtgtgcgccccctttgaaacaggtgtgaatagccggtcaagtgctagaaggggatgctatgccacgcaagcgcgcgcgtcgggaaggcgcgccggttggccgcccgccggcgcgggttcctatcgctggtagagcttgtcgatgtcgtcttggaaacgctggaagaccacgttgcgcttcaccttcatcgtcggcgtcatctcgtcgttctgctcggacaggtcgcggtccaagatgcggaacttcttgatcgcctcggtgcgcgagacggtagcgttggccatgttcaccgcgtcctgcacctcggcgcgaagggccgggtcctgcgccagctcggacaacttgcggttggccgggatgttgtggttcgccttccagcgcttcagctccgactcgtcgagggtgaccagcacgccgatgaacggcttgccgtcgcccaccaccaacgcgttcgagatcagcgggtcctggcggatgatctcctccagcgggcccggcgagacgttcttgccgccggcggtgacaatcaggtccttcttgcggccggtgatgcgcacgaagccctcgtcgtccacctcgccaagatcgccggtgttgaaccagccgtcggtgatcccgtcggcggtggcctccgggttgttccagtactccgagatcacgccggggccggcgaactcgatctcgccgtcgtcgttgatgcgcacggagtagccgttcatcggccggcccacggtgccgatcttgttggcgtcggcgttgttcacgcaggcagccgcgcaggtctcggtcagcccgtagccttcgtagatgggcacacccatgccgcggaagaagtggctgagatccgggttcatggcggagccgccggtgatgccgtaccagacggagccgcccatcgcttccttaatcttgctgtagaccagcttgtcgtagagggcgaccttggctttctgcacccgggtcgggccggattcggtgtccagcgccttggagtagtcgatcgcggccttctccgcctcgagaaagacgcgcttgcccagcgcggaaccgtccgcagccttgcggtacgcaccctcgcgcaccttctcaaacacgcgcggcacgccgacaaccaagttcggccggccgcgctgcagctccacggtcaaggttgaggtgtcggaccagtgcgactgggtcgcgccggagagcgtccacgcgatcgacacggcgcgcgcgagcacgtgcgccagcggcaggaacgtcaccatgcgctggcccgggaaggatacttggccgatcttgttctctagcagcgcccagcactggtaggcccagttaccgtgcgtgatcttcacacccttcgggcggccggtggtgccggaggtgtagacgatggatgctgggtcgtcgtgggtcaggggttgccaacgctcgtcgacaagcgcctgctcaatgctcctcccctcgaacttaatgatctccgtgccagaggcgttgaactcgtagacccgctccagcttcgagttcttgtacacaccgtccggcaggaagggggtgagcagctcagtgtggtcgcgcgtttcgctgaacgcgatcttcgcgccggagtcctccagaatccactggatctggtgtgtggagctcgtcgggtagatcggcacggtcaccgcgcccgcggcccagatggcgtagtccaccagcgcccactcgtagcgggtggaggagaagatcgcgacgcggtcccccggtgcaacaccggcggcaatgagccccttcgccacctcgaagacctcctcgatgaactctcccgccgtgaccgagacccactcgtagttgcgcgggcgcgagtacagcacaaggtgcggttgggtctggcacatctcgaccaaccggcggatcggcgtgtccttgtccgtgagcgtgaaaccaagttccgtggtgaaagagttcgacggcatgcgggcaattctaccgcgcgctgtggcagaatcgcgtgatgtgagaaacggtgacttgctgctcgaactggccgaggcctatggcttcggcaccacctaccgcgcctcgaacggtctgatcacctcacccccgctggtctcctacgtcaagctgttgcgcgcgttggggctcacgcttgacgacgacccgtcgcaagaagaactccagttccacctggatgcgcgccgcctagagctggccacccgcccgctgccgccgaccgtggtggcgaccgcggggcacgagaagcacttcaacgtccacgttcacgacgggcactgggcgcactgctggatccgcttagaggacggctcctcgcgcgacgcgtaccaggacgagaactgggccccgccggtcaccggcgccgacggcgtggtgtggggcgaggccaccttccacgttcccggcgacttgccggtgggctggcacgagctgcacctagaatccgacacggtccacgcgaccgccacgctgatcgtggtgccggagcagctggagaccaaccagcggcttatccacgacccggtttggggcgtgatggcgcagctgtactcggtgcgctccgagcagtcctggggtgtgggcgactttgaagacttggggcgcctagcagaggtcgtcgccgctgagggcgcggactacctgctgatcaacccggtgcacgccgcgcagccggtgccgccggtggaggactcgccgtacctgcctacttcccggcgtttcgtcaaccccatctacatctccgtggaggcggtgccggagttttcctggctcgccgacgaccagcgcgccgagatcgacgagctgatcgccccgctgaaagccatgaaccgctcggcggagccgctggagcgcgacaccgtgttccaggtcaagctcgacgtgctgcgcgagttgttctacctgtccagcgaggacgaggagcgcacccggggtttcgagctgttcaccttcgacgagggcgagggcttagaggagttcgcccgctggtgcgcggggcaggcgctcaacgccgcgcccgcccgccacgccggcccgcagaaaggcgacccgctggccgaggccacccgtttctacatgtggctgcagttcatcgcagacgagcagcgccgcgtggcccaggagcgcgcgctggccgccggcatgtcgattggcatcatgacggaccttgccgtgggcatccaccccgacggcgccgacgcgcacactttgcacgacgtgctggttgccgacgcctctgtcggcgccccgccggaccagtactcccaacagggccaggactggtcccagccaccgtggaacccagagaagctcgccgccgaggggtacgccccgtggcgcgacctgctgcgcaccgtgcttcgccactccggcggcatccgcgtcgaccacgtgctggggctgttccgtctgttctggctgccgcgcatggattcgcccgccgagggcgcgtacatgaactacgactacgaggcgatggtgggcgtgctcgcgctcgaggcgcagcgcgcgggcgccgtcgtcgtcggcgaggacctgggcaccttcgagccgtgggtccaagacgtgctgcgcgacaagggcatcttcggcaccaccgttttgtggttcgaatccacgccgtgggacaactcgccgctgccgtcgaaccagtaccgcaacctctcgctcacggcgatcggcacgcacgacttgccgccgaccgcgggctacatgaagggcgcacacaacgagctgcgccacaagctgggcctggtcgaggagaccctcgacgagctcaacgccaacgacgcggtgtggatcagccaggtgctcgcccacgcgcagtcggagggcgcgttcgacggcacctcggttgcggagctcgacttcctcgaccgcgacttgggcgagtacgaggacgtcaacgcgttgctggtggggctcacccgcttcatcgcctccaccccgtcggcgatgacctgcaccaacctcgtggacatggtcggcgacgtgcgcattcagaaccagccgggcaccaacgccgagcagtactcgaattggtgcatcccgcttagcgacgcacacggaaacgccatcctcatcgaggacttgaaagacctgcccctgttccacgacgtggccgaggcctcgcggcgccggtagcgctagagcgcgccggcgatagccgcgatcaccacgatcgcgatcaggatccacatcacctgcgtgaccagcgagcgcgggtacttgcgctgcggccgaggcagcttctggtcctcgcgccgcagctcttctgggtttgccatggtgtgtaaccctactcgacgatatctgccacctgcgcgccggcaagcccgcgccgcacgagcagcgggcgggtgtctttggctcggccgcgaaacgcttcgtacgccgcagcgtagtcgcgcgacgcgccgcgcgaaagcaccgtatcccggaagcgctggcccaccgcgcggttgatgccttcgcgcttcaccagctcgtaaccgtcggcgtccagcgcctccgcccagaggtaggagtagtacccggcggagtagccgccggcgaagatgtggttgaaccaggtcgagcgatagcgcggttccagcccctccacatccaaccccacagcgcgcagcgcctcccgctcgaactcgtcgactgcggccacatccgtgggcacctcgccctccaggctgtgccacgccaagtcaatcgccgcggctgccaggtactcggccgtgtcgaagccctggccgaactgacgcgacgcgcgcacggcctctaccagctcctccgggatcacctcgccggtatccacgtggcgcgcgtagttgctcaccacctcgggggcgaacgccagattctcgttgaactggctggggaattcgacccagtcgcgcggcacgttggtgccggacagtgaggggtagcgcacgttggacagcagcccgtgcagcgcgtggccgaactcgtggaagacggtggtcacctcatcaatagacaaaagcgggctggtcacgctcatcacgttcaccaccaccgggcgggtgcccagcagctcggactggtcgacgaacgagctcatccacgccccgccgcgcttggtctcgcgcgccgcgtagtccgtgagcaggagcccaagaccggtgccgtcggcgtctttgacctcccacacgtcgacgacgtcgcggtagccgcgcaggtcggggcgcttgtccacgctgatgccgtagaggaggtgggcggagtggaaggcgccgtcgacaagcacctgctccaaggggaagtacttgcgcagctcagcttcatccaccgagagctcggttgcttttctgcgcgcctgccagtacggccaatccgccccgtcaacgtcgtaaccggcgagttcggaggcgagcttgcgctccgcctcggcattcgcggcggccgccggcgcgaggtcagcgatcagcccgcgggcagctgcggcggtaccggctgtctcctccgcgatgacgtaatccgcgtgggaggcgaaacctaaaagccgcgcgcgttcttggcgcagccgcaccgcttccagcacgatctcccggttggtttcggtgccgcgagcgcgcgaggcgtcgaaaagcttgcgtcgcgcagccgggttctcaagctccgcctgcagcgactgggtggtgggcagctcgatgggaacgacgtagcggtcgccgtctttcaagccctcgagctgcgtctcgctcaggcctttgagttcctcttcggccagttcgacggcgagcgccttcgtgtccgcgagcaggttgcgtccgaagcgctccgacagctccgaaaggcgctggttgatctcctgcaggcgggtcttgccggccgcgtcgagcagcgcgccgcggcgctcgaaccggcgggtcaaaagctcgtggagccgccccgattcctcatcgcccggcacctccaccgccttgatgcgccggtagagctcctcgttctggtaaatcgaatccacgtgcgcggatagcttcggcacgatggcgtcggcgacccggtcgaactccttgtcgccgtcggtgccctgcaggttgaaaaaccacgcggtgacgcgctccaagtcctgccccgagcgctcgagcgcctccaccgtgttcgcccacgtcggctgggcttgcgtcacaatcgcggtgatctcgtcggcctgcgcccgcagcgcccgctcgaacgccggctccacgtgctcgaggcggatcgccgcgaaatccggcaggttgtagggcaaaacagagggttgcagcagggggttcgtcatagggaacaccatagctaggatcggagcacgtgctgcttgccgacgccctcccccacctcaccacccctcacggtgcacgccccggcgacgacttccccgtcgtcgcctggctgggcgagggcggccccgaccccgtgagcgccgcctcggccgggttggtccacgcccgggttgcgtaccgctccgggctaaccgggtggctgcagtttcccgccgacgcgccttcccactaccgcgccgtcgccgactgttcggccagccttgtgtggctgcagcgcaacgtggaggccttcggcggcgacccgacgaacatcaccgtggtcgggtcgggcgaagcggcggccatcgcgttgtggctgaccaggcgcgatcactaccgcggcgacttccgccgcgccgccgcaatcgcgccagcgtttccgcgccgggggctgcagtcgcgcaagtggatcatccgcggagcactcgggatcccgctcaccgagtccgcggtggatgacctcgccgcgagaaagccggagaagttcgcgcgcgcggagaggcgcctcgccctgctttcacccgccaccaccccgctcggccccttccccttcgacgccggcgagctcgccgccgtgccgctgttggtcgcgccgggcgccgacgagcgcggcgcatcatttgccgccgcgctcgcagacgaagcgcccggccccgtcaccgtcgaacccctccgggtgggcgatgacctgtggcgcaaccctttcctccgcggcggcagctaaggggggcggatgaaggagtgcgtccgaaggatggcggatctacggtgaaaaatggctacttccgccatccttgggacgccatccttgagacgccatccttcggacgccccccgctgagaggcccagcccgcagggcgcgctaacgcaagccgagctaacccaaggcggcgcggaggcgggggtcggcgagctcctcgacgagccacggcgacaaaagaaacggcgtctcctcggcggcgcggaccaccgcctgcggcgcgacccacgcgaacgagtcgacctctgcggggttggggttgagaacgacgccgtcggcgagccgggcgacaaagacggggcagatttcgttttccaccacgccggatgagtcgacggcgcggtaacggaactcgggaagcaccagttcaagcgagaccaaatcctcactggccagaccgagttcggtgccggcgcggcgcgtcaccgcttcttcacaccgctcgcccggcgcggggtggccgcaaaacgagttggtccacacacccggccacgtcaacttgcttagagcgcgccgggtgaggagcagctgccccgacgaatccagcaaccagcaggaaaacgcgaggtgaaggggggtgtgggaagtgtggatgtcgactttgggggcggtggttgtggggttgccgtaagcgtcgacaagctgcactagctccatcagttattaaggttcccctcgaaggtgacgttgccgatggtgaagcgggcgtcccacaggttgccggtggacacgtcgaaggcgtacttcgcgttcaccgtggcgccgggcccgagcggcaggtcgaggccgatgatgtccacgtccgcctcttctgcgcttaaggcttccgccgtgcgcatctcgccgccgccagcgttgtacttcagctccggcgacagcgtgtccaccggcatcggcgcgtccgactcgttggtcaccgcgacgaccacgatcgagccgccgcccggcgcgtacgaggtgccctgccacttgtagctgagctccatcgccgggtcctccacgcgcgcgcccttgatctccgtcgacggggccggctcgacgctggacgaggtgaactcctgcgcggggcgcccgatggtgctggtggcggagacttcctcctcggcgctccgctgggccgcgaccgggtcgtcctcgccgccggcgacgcagccggcgagcggcagcacaagcaacatcgcggcgaatctcatgcggtggttcatttgggcgcggctccaagcagacgtgttcgggcagttcctcgcaatactacagcgcgcggtagcgtgaccagcatgcagccaatcacccgtgttctacgcagcgcaaaccaactccgcccgtactacatcgcggtggtggcggtctcctcgctggtggcggcgctcgggctggtgtcgccgtttttgctgcgcgaggccacggacaccatcgtcgaaggcggcgaggcgcgcacggtgatctggctggccatcggcctgttcgccgcggaggcaacagcgtcggttttgcgcaacgtctccggctacttgggcgacgtcatggttgcgcgcatccgccagatcctgtccacgcgatactttgaaaagctgctgtcgctgccgcagcgctacttcgacaaccaggtcacgggcacgatcatcgcgcgactcgaccgctcgatcgccaacgtcacccagttcatccagtcgatggcgaacaacttcctgcccatgctgatccaggtcatcgcgatcctggctatcaccggcttctattactggccgctggcggtgctgctcgcgctactgttccccctctacacgtggctgacggcgctgacgtcgaagcgctggcagacgttcgagggcgagaagaacgaccacatcgaccagggcaacggccgcttcgctgaggtggtcgggcagatgaaggtgaccaagtccttcgtcgccgaatcgcgcgagctgaacacgttcgcagaccactaccagtccaccgtggacatcacgcgcccgcagtcgcgctggtggcactcgatggacaccgcacgcggcctagtcatgaacgcgatcttcctcggcatctacctgatcctgttcctgcgcacgctcggcggccacttctccatcggcaccatggtcatgctgattcagatggtgaccatggtgcgccaacccgtgaccatgatgagctggatcgtggattccgcgcaacgcgccgtcgccggctccaagagctacttcaaggtcatggacgcgccggtcgaggaagcgttcgcgcgcaaccccgctctctcacccctgccggttgcggagccggtggtcagcttcgatcacgtcagcttcgggtatgaggagggggcattggtgcttgacgacgtcaccttccacgcccaccagcaccaaaaaattgcgctggtcggcgagtccggcggcggcaagtccaccatcgtgagcctccttttgggcctctaccccatcgacgccggccgcctgagggtctgcggccgcgacgccgcagagatctccgccgctgaactgcgcgcgtccaccggcgtggtgttccaggaaccggcgctgttctccggcacgatccgggaaaacatcgcctacggcaaacccggcgcgacgctggaggaagtcatcgaggtggccaagcgcgccaacgcgcacggcttcatcagcgggttcgacaacggctacgacaccgtcatcggcgagcggggtttgcgcttatccggcgggcagaagcagcgggtggcggttgccagggccatgcttaaagacgccccgatcctcattctcgacgaagccacctcagccctcgacacgaaggcggagcgcgcggtgcaagccggcctggacgagctgatgaagaaccgcacgacgatcatgatcgcgcaccgcttgtccaccatcgccgacgtggacaccatcatcacgctcaaggacgggcgcatcgacgagatcggctcgccggctgagctcgccgtgtccggcggtatttattcggagcttctgcagctcaccgcctcgtcttcagctgcagaccgcgagcgcttgaagtccttcggcttccacgtggactccgaggacggggacgacgaggagccgcaagagcgctagccttgggtgccatgcagtttcctagccttgacaccctgaaagcccgcggcacccgcaagtggacggtgtacggcgaggacgtgatcccgctgtttatcgcggagagcgacttccccaccgcaccggccgtcaagcgggcgattatcgacgcctgcgagcgcgaaatgttcggctacacccccgccccgcgcgcccaccgcttgggcgaggcggtcaccgacttctacgccgaccgctacggctggcgcccggatcccgcaaatgtcttccccgtcgccgacgtggtgcgcggcgtgctgctgtccattcagtacttcacggaaggcccggtcattgtgccggtgccggcgtacttccccttcctcgagatcgccgaggccgctgggcgcgagcgcgtcgacgtcggctcggtgaacggtcttgacctgatggaggtcgaagccgcgtttagaaacggcgcgggcagcatcatcctgactaacccgttcaaccccggcggctacgtgttcgacgccgaggagctcgaccagatctgcgccatcgcgcgacgctacggcggccgcgtcatcgtcgacgagatccacgctccgttgacgttcggcgcaccccacgtgtgcgccgcggcgaacaatccggacgtgtgcatcaccgtcaccgccacctccaaggcgtggaacgtcgcggggctcaaatgcgcgcagatcatcttctccaacgacgaggacgtcaagcgttggaacgggatgaaccacgtggcgaaggacggcgtgggcacgctcggcatcgtcgctgcggaggcctgctacaacgacggccgcgagttcctcgacgaggaggtcgcgctgctcaaggcgaaccgcgactggctggtggagcacctgccggaggcgatccccggcatcgagttcgtggtgccggacgcgacgtacctgatgttcctggacttcagcggcaccaggctcgccaccgagctgggcgtggaccgccccgcagcttggctgctcaagcacgcaaacgtggcgatgagcgaaggcgccgacttcggccccggcggcgacaacaaggcgcgcctgaatttcgccaccagcccggagatcctcgaagaggccgtcgggcgcatggctcgtgcgattacgagcgcctaaacccagtacgctctagggccatggagcaaacgccgcaggcctcgcagttcatgacccccgcgcccgccgagcaaccgtgggagcgccccgacccggagtggtacaaggatgccgtcttttacgaggtgctggtgcgcgccttctacgatccggacggcactggttccgggtcgctgaaaggcctcgaggagaagctggactacctcgagtggctcggggtggactgcctgtggatcccgccgttctacgactccccgctcaaagacggcggctacgacatccgggacttccgcaaggtgctgccggagttcggcacggtggaggacttcgtttcgcttatcgacgcagcccacaaacgcggcatccgcatcatcacagacttccccatcaaccacacttccgaccagcacgcctggttccgcgcatcccgccaggacccggaaggcccgtacggcaactactacgtgtggaccgatgacccggagcagtacgagggcacccgcatcatcttcatcgacaccgaggagtccaactggacgtgggatccggtgcgcaagcagtacttctggcaccgcttcttctcccaccagccggacctgaactacgacaacccgaaggtccaggaggaagtcctggacgtgatccgcttctggctggatctgggcatggacggcatccgcctcgacgcgattccgtacctgtttgagcgcgagggcacctccagcgagaacctcccggagacccaccagttcatcaaacgcgtgcgcgcgatgtttgatgaggagtacccgggccgcttcctcttggccgaggcgaaccagctgccgtacgaggtggtggagtacttcggccagggcgaggacggcgccggcgacgagtgccagatggcgttccacttccccgtcatgccgcgcatcttcatgggcctgcacaaggaaacggcgcagccgatcatcgacatcctgcgcgagaccccggcaatcccggagagcgcgcagtggggcatctttttgcgcaaccacgacgagctcacgctcgagatggtgaccgaagacgagcgcgactacatgtacaagtcctacgcgttcgagcctcgcatgcgcgccaacgtgggcatccgccgacgcctcgcgccgctgctgggcggcgaccgcgaccgcctcgagctcgcccacgcgctgctgttgtcgctgccgggttcgccgtttttgtactacggcgacgagatcggcatgggcgacaacatttggcttgccgaccgcgacggggtgcgcacaccaatgcagtggtcgaacgaccgaaacggcgggttctccagcgccgacccggagcgcctctacctgccgccggtgcgcaacgatcagtacggcttccacacggtgaacgtggagtcgcagaagagccgcgagaattcgctgctgcactgggtgcgcaccctcgtgcacattcgcaagcagtaccgcgcgttcggccgcggtgcctacatcgaggtcgagcacggcaacgaccaagtgctcgctttcatccgcgaatacacggacgagacgggccgcaccgagcgcatcctgtgcgtgcacaacatgtcgtctcggccgcaaccggtggagatgcagttagctcgctacagcggactcctgccgcgcgagctgtccggcggcgtggacttccccgcgatcggtgagctgccgtggctggtcaccttggccccgcacgggttcttctggttcgacatctcgggtgcggtggagcagcgatgatcgacatctcaaaggagcggttcttcggggcgaaggcgtcgggggtggggcgggtgagcgtcgtcaagcagctgcccctcgggccgtacgagtggcaactgttgcaggtggacgacgacatctaccaagtggtttcggacggcgcccgcgacgtgcttgccgctaaccccaccacctacgtggagcacctgggcaagctgggtgaggtgcgcggcgagctggtgcgcggtgaggcgcgcgcgatgggtgcggagcagtcgaacacgaacctggtggtcggcggcacgttggtgaaggtgttccgcaagctcgagcggggtgtaaacccggatgtggagatcctgagccgcatcgacaacccgcacgtcgcgcccgtgaccgcgtacgtgacctttgacgggatgacgcttgcgatgcagcaggcgatgctcgacggcgacgacggctttgagctggccacctccggcgccgagctcgactcgcgcgctctcggcgaggccgtcgccagcgtccacgcctcactcgcagccgagtttggggtgcgggagagcatctcgcttgccgacgagctcaattcccgcctcaccgactccatccgccgcgcgccggtcctggccgagtttgaggacgccatccgcgcgcgctacgaggtgctgaaccagccgctggaaatccagcgcgtgcacggcgacctgcacttgggccagacgctgaagcgccggggcggtgtgagccactggtacctcatcgacttcgagggcgaacccgcgcgcccgcttgcccagcgcgtggagcccgaccacaggctgcgcgatctcgccggcatggtgcgctcctacggctacgcgcgccacatcggcgggcacagcaaggcttgggaagacgacaacgtcgcggcgctgaaagccggctacggcggcgttgacggcattgacggcgttgacgaggacatcctcgcggcctacatcgcagacaaggcggcgtacgaagtggtgtacgaggcgaacaaccggccagactgggtggacatccccctcaccgctcttcgttccattgtgtgggactaacttcccaaaaacactccgtggaaggtactgtgtacgaaatcattgatttcccacaacgactccaacggaggttttcatgggctccacagcagtgcgcgccgagcaagccggtcagaccggcgctgggcgcaaacagggcagcaccaaaacgattctgatcacctcgctcgcccttttctccatgttcttcggcgcgggcaacttgatcttcccgcccatgttggctgtggaggccggcgacaacttctggcccgccatcttgggcttcctcggcaccggcgctctgttgccggtgctcgccgtgatcgccatcgccatgtcgggcgcgtccgtgcgcgacctgtccaagcgcgccggccacgtcttcggcttccttttccccgtgcttgcgtacctgtccatcggcgccttctacgcgctgccgcgtaccggcgcggtttccatggagacagcgatcaccccgctgttcggtttcgagggcacgctcgcgtccgcggtcttcaacatcatcttcttcggcgtcgcgctggcgctggcgtggaacccgtccaccatcatggacaaactgggcaaattcctggtgcccgcgctcgtcgtgctgctggtgatcatgatcgccgtctcgctcgcccgctggaacgctgaaccgagcgcgccgagcgaggtctacgccgacggcccgtttacttccggactgctcgagggttacttgaccatggactcgatcgccgccctggcgttctccatcgtcatcatttccaacctgcgcgccaagggctttgccgagggccgcgagattgtcaacggcaccatcatcgccggcatcggcgcgggcgtcatgctcgcgctcgtctacctgggcctcggcggcatcggccgcgtcatcccgaaggcgggccagtacgacaacggcgcgggccttctggcggacgcagcgaacctgaccatgggcaccgtcggccaagccgtcttctcggcggtcgtgctcctcgcctgcctgaccaccgccgtcggcctgatcaccgcgaccagcgagtacttctccgggaacttcttcggcacctaccgcgcctgggccatcggcttcaccacctggtccatggtgttcgcgacccagggcttgagcttcatcatgaccatcgccgctccggtcatcggctttttgtacccgccggccatcgcgctgatcttggtcaccctgattgagccggccttccgctccaagacgcggtttacctgggcactgatccttccggtgtggaccgcggtcgtgttctcgctcgttgaaaccttcgtcaacctcggctgggctgccgacgcgctgtccccgatcgtgtcctgggcgccgttgttcgaagctggcctgggctgggttgtcccggtcgcagccgccttcgtcatcggcctggtgctcgacttcgtgaacccgaaggcgccgatggaagtgggcaccaaccacaccgtcgagggcgaggtccccgtcgccgccgagtaggaagcgcgtagcgtggggtcatgactaccccactttccctcattgatttctgcatccgccgtcccggcgaaaccgtcggggcggcgatgcagcgttctgtggagttcgcgcaaaaagcagaggcgctggactacaagcgcatctggtactccgagcaccacaatatgtccacgatcgtgtcgtcctcaccggcggtactgatctcccacatcggcgccaagaccaactccatccgcctaggctccggcggcgtgatgctgccgaaccactccccctacgtcatcgccgagcagttcggtatgctggcggagctctacccagaccgcatcgacttgggtctcggccgcgcgccgggcaccgaccagcagacgctcggccgggcgctgcgccgcgacccgcgtgccgcggagaacttcccccaggacgtcctcgagctgcaggcgtggttgtccgacgagtcgccgatcccgagtgtcgtcgccttcccaggcaagggcaccgaggtcccgctgattatcctcggctcctccatgttcggcgcctcgctcgccgcaaagctcggactgccctattcgttcgcctcccacttcgcgccgcagcacctagagcaggcgaccacctactaccgggaaaactacgagccctcggagcgtcacccggagccgtacgtcatcgccgcggtcaacgtgattgcctccgacactgccgaggacgcggagcgccaggagcggctcgtccaccgcgagcgtgtgcgcaccttcgtcggccgccagggaaccccgctgaccaacgagcagctagacacggtagtggcctcgtaccagggccagcagatcattgacatgctgcgctacaccgccaagggcacgggtgaggacgtggccgcgtaccttaaagaattccaagagcttgcgaaggcggacgagcttatggtgtcgctgcaggcgccctcacatgaggaagtgctgagaagcatggagattctcgcggcccaccgcccatagattcacccccgcccgcgcaatgtaggctgatgcgcgtgtcggattctttgtcatccaaccccttgcgccgcccgcagcagcaccaggagattgctgattacctccgcgacgagatcttcgccggccgcctgccggtcggcgagtcgctgccgtcggaagcggagctgtgcgagcagttcgcgacgtcgcgcggcccggttcggcaggccgtcgcaacgcttcgctccgaagggctgatctcctcgggccgcgggcgccgctccatcgtgctgtctagcacgcgcaccgaaaccttcgaggaagtgctctccacctcctcctgggtcgcgcgcatgggcaaggtgccgggacagtccctcaagtggttcgggttgcacccagcccagccggagatcgcgaaagcactgcagcttaaagacggcacgtcggtcgtctccctgcgccgcatccgcaccgccaacggcgcgcccgtagtcgccgaggacatctttttcagccccgctgtttccgcgaccgtgctgcgcaccgacccgaacgccgaatccttccaccgcaccttgatgcgcgagggcgtgaacttcaacaacgtttcgcgcgccgcgtccatcgagcgcgcaaccgaggcagatgcggagacgttggccgtttcggttggcgcccccatcctcgctgtcgagctgcgcgcttacacccacaccggcaagccggttgagtacgcgctgcgccgttaccgcaccgacgacatcaccttcggcatgaacaacgtgcgcgggcactcctcgccgctgtggctggagatgaccccggagcagatcggatgagcgcaccccgcctcgcaggcccactcgcggtggcggcggcgctgagcgcgtgcgccacgcctgcgccgcaggtcgacgtcgtcactgtcgctgcctccgccccgccagcgagcctcgacttcaccgccaccggcggcgccgcggccccgcaggcgctgatgggcaacgtgtacgaaacactcgttcgcatcgacgatcacggggtgccccagccgtttctggctacctcgtgggacacctccgacgacggcatcacttacaccttctacttgcgcgacgacgtggcgttttccaacggaaagccgttcaccgccgaggacgccgcgttttccatcgactacgtgaaaactcagtgggcgaacgggttgaaatcccagatggacccggtggtgcaagcccgcgcggtggacgagcacacgcttcaggtggtcctcagcgaaccgagcgagagctggctgtggtccatgggcaccttcaccggggcgatgatgtgcgaggaaagcatcgcccgcctcgccaccgacccgctgggcaccggcccctacacggtcgcccgcttcgacgagaacaccgcgatcagcttcgacgcccgcggcgactactggggcgaggtcgcgcacgacgcgcagatccgctacttcaccgacgccaccagcgcggtcaacgcgctgcgcgccggcgacgtggacgtggtgtggcaaatgcaggccccgcagctcattggggcgttgcgcgacgacgtccgcgtggaagtgggcaccacaaacggcgaggtcctgttgtccatgaacaacaacgccgcccccttcgacgacccggacgtgcgccgcgccgccgcctacgccatcgacagaagcgcgctcaacgacgtggtctacgacggcctggccaccgacacgggcggcgcgccagtgccccccaccgacccctggtacaccggcaccgactactaccccttcgaccccgaccgcgcacgcgagctactggccggtcggacgccgcagctgaccatcaccgtgccgagtctgccgtacgcccaaaccgcggcggagctcattttcagccagctgcgggacgtcggcttcgacgtcaccttagaaaccgtcgaattccccgcggtgtggctgcaaaaggtgctgaaaagcgcggactaccaagcctcgatcatcgcccacgtcgagccgcgggatatggcgtcgatgttcgctaaccccgactactacttgggctacgactcggcccgcgcacgcgagctgatccaggccggagacgtggccagcatgcgcgaagccgtagacgagatcatggcggacgcagcggcgctcacgctggtcaacgccccgaacatcgtgctgctgcgcaacggtgtttccggcgtggacccgaacatcgtcaccgactcgctgccgctgaacacaatcacgttgaaggaggagccatgatcgctcgagttgggcgcgccgtgggacggttcgcgctgctcatcgccgcggcgagtgcggtgattttcctcctgctgcgcgcggttcccggcgacccggcgcgcgtggctctgggggttaccgccacagaggaggccgtcgccgaactctcgcacaagctcggcaccgaccgcccgctcggcgtccagtacgtcgactgggtcacgggtatgctcaccggcgacttcggcatctccatggcgtctggccgcgagatcagcgacaccgtggcagagcgcgccggggtttcgctgacgctcacgcttgctgcgatggcgctcgcgctcgtgacagcggttccgctcggcatccgcctcgcccgcaagccgagcgccgtgctcgcggccgccacccaggtcgggatggcggtgccgtccttcctcgttggcatcctcgcagtggggctcttcgccgttcggctgaactggctgccggcgggcgggtggggcacgcccgcgcacgcggtgctgccggtgatctcgctcgcggttgtgcagggcgcgatcctcacccgctacgtgcgtgcggcggtggccgaggagctgtccaaggattatgtgcgcacggggagggcgcagggggcgtcgataagcaatgtgctctactcctctgtcctgcgcaacgccgcgctgcctgtgttgaccgtgaccgggctgcaactgtccaccatggtggtcggcgcggtggtggtcgagcgcgtgttcgccatccccggcctgggaacgctccttttaacctcggtagccaaccgcgacctcaccaccgtgcagacggtgatgatgcttctggtggcgttcaccctggtggtgaacctgatcgtggacctgttgtacgtggtgatcgacccgaggagtaagcggtgaagcgcgcgggctacatcatcctcgcggtgtttagcgccgccgcagtgctctcgctgttctggacgccgttcgacccgctgcaggcggcgcccgccgagcgcctgcagccgttcggcgccgcgcactggatgggcaccgacgagctcgggcgcgacgtgctcagccgcatcatggcaggagcgcgcttgacgttgtcggtcgcggcggcctcggtggcgttgtctgcccttgtcggtatcccgctggggattttcgccggcatgcgccgccgcgccgggaaggtagtaatgggggcttccgacctgctgctcgcgttcccggccctgttgctggctatcgtattcaccgccgtcttcggcgcgtcgatgtggatcgtggtgctggcgatcggcatcgcgggcatccccggcttcgtgcgcgtcgcgcgcgtgggcacgctgcaggtcatgagccaggactacatcctcgccgcgcgcatggcgaaggtgccgggcccggtgatcgcagcccgccacgttttgccgaacatcgcgcacctgctcgccgcccaagcaacagtcgcggccgcgctggccatcctcgccgaggcgggcctgtcgtttctggggctcggcgcgcccgcgccgtacgcctcgtggggacgcatgctgcaggcctcgcagccgtacctggccaccgctccccacctcgcgctgtggccgggcgcggcgatagcgctcacagtcctcgcctgcaacctgatcggaggcgaccgtgatcgtcgttgaccgtttgcacatcgccgacctcgtgcgcgacatctcgttcaccctcgcccccggcgaacgcctcggcatcatcggcgaatccggctccggcaaatcgctgaccgcgctggccatcatgggcctttcggagttgccgactaagggcaaggtgcttatcgacgccaccgagatgctccacagccccgaccgcgtcacccgcgccgtcaggggctcgaaagtgggcatggtcttccaagaaccgatgacggcgctggatccgctgaaaaaggtgggcaagatcgtgccccgagagctgctcaaagaggtaggcgtcgaccgccccgacgcctacccacaccaactctccggcgggcagcgccagcgcgtgctgatcgcgctggcactgagccagaaccccgactacttgatctgcgacgagcccaccaccgccctcgacgccaccacgcaagcccgcatcctggacctgatcgaccggctggtggaagagcgcggcatgggcctgattttcatctctcacgacttgaacgtggtgcgccgcatgacgcagcggcagcttgttttccaccgcggtgaaatcgtcccgcccgattccgactacgcgcgcgccttggccgccgccgcgcgtcctgggaaaccggccgcaccggttgacccagcctcgctcggcgaggcggtggtcgatcttcgcggagtcaccgtgcgccgcgggtcgacgctggcgctcgacggtgtgtcgctcaccgtgcgcgcaggcgagcgcctcggcatcgtcggcggctccggctccggcaagacgacgcttctgcacactatcgccgggcttatcgcgcccgacgccggcgcggtggaaacgagcgggcgcatgcacatggtgttccaggacccgtactcgtcgctcgacccgcggatgcgcgttgcggcctcggtgcgggaggccggtgtggacgccgcgcgcgccgaggaggtgctcgccgccgtcgggttagaaggcgcgggcgggcgcaaaccgcgggagttctccggcgggcagcgccagcgaatctcgatcgcgcgcgccgcggccccgcacccggacattctgcttgcggatgagccggtctcagccctcgacgtctcgcttcgctcccaggtgctcgacctgatcagcgccacagtcgggaacaacaccctgatcttcatttcccacgacctgcaggtggtgcgcgagatctgcccgcggttggccgtgatgcacagcggacgcatcgtggagcacggcgacaccgaggcgatctgggcaaatccgtcccacgaatacacgcgcgagttgatagcgtcggtggcacgatgagcacccacattacggtcgtcggttccatcaacgccgacctgactgtcaacgtcgccgcgcacccggcacccggcgagaccctgctgggctccggcggcgggatcaccgccggcggcaagggcgcgaaccaagccgttgcggctgcccggctcggcgcgcgggtggcgctcgtcggggcggtgggcaacgacgcctacgccgaacccgctaccgcgctgctgcgcagctcaggcgtggacctggcccacgtggagaccgtcgactcggtgacagggcttgccgtgattaccgtggacgccgccggcgagaacaccatcatcgtggtcccgggcgcgaacgctgcggtggacgcgcagtacgtggagaagcaccaagcccctatccgcgacgccgagctggtcctgcttcagggcgaaatccccgcagacggattcgcccgcgccgccgcgctggccgccgggcgcgtggtggtgaacctggcgccggtggtcgacgtgccgcgtgaagcgctgcttgccgccaacccgctgatcgcgaacgagcacgaggctggcctcatccttgcccagctgggtgaagaccctgcgggggagcctgctgcgctggcccaacgcttggtcggcgccggtttcgcatccgttgtgctcaccctcggcgcgcgcggcgcgctggtcgccgacgcgggcggcacgcacaacatccccactccgcgcgtcaccgccgtggacaccgtcggcgcgggcgacgccttcgcgggcgcgctgtgcacccgcctcgtcgccggcgactcgctgctcgacgccgcccgcttcgccgcgcgcgtgggcgcgttcgctgtgaccaagccgggcgcgcagccgtcttaccctgccgaaagcgacccactgcccgatgtgtagcgggtggcgctagcgcgtgatgtagaacatcagcgaggggtccagcacgtgctcttcgacccgctcaaactcatcggtcaacgcctcgaacgccttaaactccccaggcgaaagctttgcctgctcgcgcggaaccggtgtctgcatgggcgttattgtagtccccatgcccttccaccgcctcgccgccgcgcgccctggccggttcgcggtcgtcgagctggtcgcggtggcggtcatcgccctcgggctgcaggtggtcttcttccaaacgcttgaaagcttcccgcttgccgacgccctgttgatctccaccaccctccccgccccatttctcgccgcgtggttgaccaagcgcaaccccgccgagctgctctctgtcgaaaggcggattcgctggggtgtcgccggccgagcgctcgccgcctcatgcgccgtctacggcgccgccgccctcgcagccgccgcgagcgggcgcatgatcgccttcggcgaccccgcccgcgcactgcggttcaccgcctacgcgctggtggtggtcaccgcccaatcagccgccgaggagctcatcttccgcggcgcgttgccgcagatcgtcggcacgtgggcgcgctcgccgtgggtggcgtacggcgtgcccgcggcactgtttctccccctccacgccaccgacgggtggggctacgtggacatcgccgtctttaccgcctgcgctggctggctgacgtggttcaccggcggcgttgaggcggcgatcgcgctgcacgcagcgggcaacctgcttgtgcagttcgcccctgtaagcccggccgcatcgatcgcgctgacggtggcggcgaccgcgctaagcggatggttcgcccgcgcccgcgcctaatccagtatggcgaacaggcctgtggccacctcggcgccgtggacccagatcgcgtcgtgctcccaggtgtcgtgcgaccacaccttgaggctggcaatgcttgccgccgtctggctcacgcaggctattcttcgtcggtcgacagcgcggcgacgaacgcctcctgcggcacagtgacggagccgatggacttcatgcgcttcttaccggccttctgcttctccagcagcttgcgcttgcgcgagatatcgccgccgtaacacttggacaggacgtccttgcgcagcgcgcggatgttctcgcgggcgatgatcttggaaccaatcgccgcctgcaccggcacctcgaactgctggcgcgggatgagctctttgagcttcttcgtcatcttgttgccgtaccactgcgcggactccttgtgcacgatcgcgctgaacgcgtcgaccggctcaccctggagcaggatgtccaccttcaccaggtcgccgagctgctcgccggcttcctcgtagttcagcgaggcgtaacccttcgtgcgcgacttcagcatgtcgaagaagtcgaagataatctcgcccagcggcatgatgtagcgcagctcgacgcggtcctcggagaggtactccatgttcttcatggtgccgcgcttggactggcacagctccatcgtggtacccacgaactcctgcggcacgatgatggtcatgttcacgatcggctcgtagacctcgtcgatcttgccgcccggccagtccgacgggttgtgcacgacctgctccgtgccgtcctcgcgcatcacgcggtaggtcacgctcggcgcggtggagatcaggtcgaggtcgaactcgcgctcgaggcggtcgcgggtgatctccatgtggagcaggcctaagaatccgcagcggaaaccgaagccgagggcaacggaggtttcgggttcgaaggtcaacgatgcgtcgttaagctggagcttctccaggctctcgcgcagcgcggggaagtcctcctggctgaccgggaacaggcccgagtacaccatcggtttaacctcttcgaaaccctcgagcgggtcgtcggcacccttggaagcccaggtcaccgtgtcgccgacgcgggtctcgcgcacatccttcacaccggtgatgaggtagcccacttcacctgggcccaagcctttggtctttttcatcgtcggcgacaccacgccgatttctaagatgtccagcttggtgccggtgttcatcatctgcacctgctggttgggcagaagcttgccgtccaccatgcggatgtaggtgaccacaccgcggtaggtgtcgtagaccgagtcgaagatcagggcgcgggccggcgcatcagccgcatccgagccgtcctccatctcggacttcggcgccgggatcagctcgaccaccttgtccagaagctccggcacgccctggccagtcttaccggagacgcgcagcacctcctccggctcgcagccgatgatgttggcgatctcgagagcgaacttctccgggtcggccgccggcaggtcgatcttgttcagcacggggatgatctcgaggtcgttctccatcgccatgtagaggttggcaagggtttgggcttcgatgccctgcgccgcgtcgacaagcaaaatagctccctcgcacgcgtccagggagcgcgagacctcgtaggaaaagtccacgtggcctggtgtgtcaatcatctgcaggacgaactcctcgcccgcgtgctcgccggtcttcggcacccacggcaggcgcacgttctgcgccttgatggtgatgccacgctcgcgctcaatgtccatgttgtcgaggtactggtcgcgcatgtcgcgttcgtccaccacgccggagagctgcaggatacggtcggccagcgtggacttgccgtggtcgatgtgcgcgatgatgcagaagttgcggatccgggccggatccgtgaacgtctcttccgcgaagttcctcttttgagcagccataattaccacatcctactgggtggccagacgaagagaaatatcggcgcaaaccgcttgtaggcacgtgtttttgcacctaaagtggctccgaaaggttcggtagcaaggaggccgaaggtggcacgctggttccgtggcaaaggttggggcagcaccagcgacaagaagcgcgcccgcgagctggacccgtcgctggagaaaggcctcgcgctgctgaacgagcggctggcgcgcccgaactcgcagcgccgcgaacgcctcgcttcgcgcgtgcacgtcaaacccaccgccgcggttccgcggaacatctactacgcccccgacatggacggcggagcggagcccggcgaggtggtgtgggtgaccgtgccgtcgcagccgccgtcggagcgctccatgctggtggtgggccgcgaccgcaccgacgtgctgggccttttaatctcgcccgagaaggaccacgccaacgactcgcgttggctcggcatcggctccggcgggtgggacgcctccggcgagccgtgctgggtgcgcctggacaagaccctgtgcgtgcctgaatccgacgtgcaccgccgcggcaccaccgtgccccagctgcgcttcgagcgcgtggccaacagactgcgcgaccacttcgattggggctagcgcttttgccttttggttccggccgcggtgagctgctagctttgaggagttgttcgcatccgggtgtttaagggtgcgcggcgctacgcgggcaggaccttgggtccgcgttcatacccaaagcgccgtgcgcaaagccctgccggatcttcgacatacccatcagtatcgaattaagaggtgattgctcatggcaaacattaagcagcagaagaagcgcaacctgaccaacgagaaggcgcgcatccgcaacaagtccatccgttcggctacccgcacggagatccgcaagttccgcgaggctgtggagtccggcgacaaggctgccgccgaggcgcagctgcgcgtcgcgtcccgcaagctggacaaggctgtgaccaagggcgtgttccaccgcaacagcgctgcgaacaagaagtccaacatggctcgcgccctgaacaagatgggccaggaagaagcgtaaagctttttggcttgtcgacgccccgttgatcattttcagcggggcgtttccttttgcccgcgccgcgctacaccagctctgcgatacgccgcaccgcgttctccagctcgaactcctcgtcgccgccttggcccttcaccgccgcgtccaagtcagcgacgatgatcacggcttcggacaccgcctcccccgaccactggcgcgccacctgcatcgccttcttcaccgcgaaagggtgcatgccgagctccctggccaactggtcgtggctgccgcgcgcgccgtagagcttggcaatgtctccgactttcatcgccagcgccgcagcgatcgcgaccggcgaggcgcccagctgcagcgccctcctcgtcgacgccagcgccctatccgcccttcccgccaccgcctggtccgcgatatcgaaacctgcgacctccgcaacaccggtgtagtaatcgcgcaccgacgccacggtgatctcaccctctgtgtccgagaccagctggctgacggccgaggcgagctcgcgcaggtcgctgcccaccgattccaacagcgccgccaccacgtcgggcgtgggccgcaccccgtggcgcttgaactcggtggtgagccacgcgtgccggtcgcgctccttaaggggatcgacctggtgcacctcggcgagctttctgaacttctccagctgcgatttctgccgcccgccgccggtgtgcttgataatgacggtgacgcccggcgcgacatccacgcaggccttgagcagcgcctccacaggttctttgcccgccagttccgtcttctccacgatgagcacgcggtcctcggcgaacagcgacgggctcatcgcttgcgccagttcgcccgcagtggcgtcgacggcgcgcagcgtggtcacttccgccgtcggcgacgcctcggcgaggatgtccttcgttgcgcgttcagcgaggaactcgtcctcacccaccactaggtgcacggggttgagcatgcgctccattgtaagtgcggtctctgcacgggttcacggcggtgagcgcgacccgtcggcgcgcagcgtaatcgccccgtcgcggttagggaagatcaccgggatgccggccggtgtcttcgtcgggcgtttcgtgggcgcgcccggttctagcaccaccaccagctcggttcccggcgggaccggctcgatctcgctgcgcgtcgccaccacgtgggcgcgcagcgcggtctggtccaccaccggcgcaggcagcggttggaggtgcagcgctccgatcactcccgcggtgatagcaaaggtgatccgcggccgcctcgccatcagccccgcgatgacccagccgtaggccaccagcaccatcacaggccctgcttcaaccttggcaaacggcagacgcgcaccgttggtggccacggcgtgcacccaccacgtcaacggctcaatagcgatgagcagcggcacctcgaggccgcccggcagaagacacagcaccgcggcgagaagccccagcaccgtcaccgcacccgtgacgggcgcaactagcacgttggcagcggcagagaccagcgaaacctcccccgccatcagggacacgatcggcatggtcaccacgtccgccgcaatcgccaccgctaccgctcgcacaaggatgtcgggccacccagttggcgcaagccagcggtacagcagcgggtgcagcgtcacgatcccagcggtcgcggccaccgacagggcgaaaccgtaatggacggcgaggtccgtatccgcaagcaccagcgcgatcaccgcgatgcacagcgcgtggaccggctctgcccgcgtcgaggcgataaccgctaccagaccgaccaaaccagtgacggacgcgcgcagcacgctgggttccggtcccaccaaccctgcgaaaaggaggagagccgctgccgcgcacgcgaggcgggtgcgcagcccgcacccgatcaacgtggctgccaccaccgcggccgtggtgacgtaggtgacgttgcttccggacaccgcgctcaaatggctcaagccagtcgcaatgtacgcctgctcttccgcggccgtctgcgccgatgtgtcgccgagcaccataccggggatgagtcccctcgagctcgggcccacggttgcgtccacactctcggcgaatgtgcggcgcacgtgcgcggcaaacgcggcgtagccggtaggcggctgcaccatctcgacctccccgttgaacacgtacgggttcacggcagcgacacgggacgccttcagggcaccggttgccacgacggtcgcgccaggctccacgccgtcaggcaattgggtgctgaacacggcgagggtggaggggtgcccgtctggcgaaatccgggtcagccacgatccgccgctggtgagcttcggcgccgaagtgacgcgtcccgtgatgcgctccccgaactcccagttttgcgccacgcgcacacgcaccgaggccaccgcgcacgacgcgcagccgagccccacagccaacagcgactgaccggggtggccgcagaccaagcagataaggcccgctgcagcgacgagtgcaagacccgcccaggtgccgacggtcacgcacaggatgctcgccagccacaccgtgagcgcggcgggaacaagacgcaactcagacacggctacagcgcgatctggtctttgagcgccgcgaacttcgcgggcccgatgcccttgacgtccatgagcgcctcgagcgaggtgaacggaccgttcgcctcccggtgcgcaacaatcgcggccgcggtggcggctccgacgccgggaagtgtctccagctcggtggccgatgccccgttaatcgagaccaatcccccgcccgccgagaccgcgccgaccgaaagggcaggaaccgcacccggcggcgcggcagcgttggagggtaggacgaggatctgctgcccgtcgacaagcaactgcgcctggttcagcgctaacaggtcggcgtgctcgtgcggcgccgcaaccgctaaggcatcggcgacgcgcgccccctggtgcaaggtgaccaggcctgggttggccacctcccccaccacagagaccaccagttgctccggcaccgcgtcctcggcggcaaccgtctcccactgctgggccggcggggctgcgtccggggtgcgcgtgacagcccacccggcgacgatggcgagcaccgccgagacgcacaccgcggcttgcttcggctccacgcggaggcgaggttcggggtaggcgacggggaggagatcctcttctccggtgggcttggtcagctctttgatgcggtcggcggcgctcataggcgaaccgtacggccagctccccgacccgcggaagcccctggtggcgcacctgtggataacccggcgggcgcgagcgtggcaccaaaaggttgtccacacgcaacgcccgtgctgaaaacgcaacgggccttattggaaacgggacgtggtggatttagccgtagcggcgctgatcgacgaaccggccgaacgaatcggatacttggttgtcccactgcgacggccacagatagtagcggccgtggttgccgccgttgtggcgcgccgaaccctcaagcgtctgcactgacaggtcgcacacgccgtcgagcggcaggcagtagttgacgcggttggtggtccccgctgcggagcgggagttgaacggcagccagccgagcatgccgcccgacccgccgccggccacgccgacggtcgctgggtcgcccgcggcggtgttcgggttgccgaagtacacggcaccggcgagctggccgcggcgcgcgagctcacgctcgtgctccagaagaatcatcgcgccctgcgagtacccgaccaggatgtagccagggcggcagccggtggcgcgttcgtagtcgttgatctggcgcagcacaccggcacggcccgcctggaccgagtcggtgaactcgcctgcggcaccgcgcgcggtgcgcagcaccggcagcgcgtactcgagggcgatgtccaaggcttgaatgaccgttgccggggtcggaacggtgggcacggagtactcggggtaagcggccgggtagtagcgcggctcgaggccaagcacctcaacgtccttcatcagggaggcgccgccgtgggttgcgcggtatcggttctcagcgtggcgcaggaaagcgcggatcgtctcaccttcccagccgttggacacccacggtgcctcgtttgcgtagctggtgcggtaaatgtggccattctggccggagccgcgcgcggcgattacggcgaccgacgggcagcgctgctgcgcatccgcgctcggcgcctgcggggtaaaggaaacagataacgtggcgacaagcgcggtcaccagggcgacgaggacaactcgagcctggcgcgagagggtggtttgcacgcgcaaaactctagcgaatctcgctacgtcgcgctgaacacggccgacacaccgatggcgccggcaccggtgtgggtggcgatgacgggcgcgaacgcctccacgagcaccttggaaccgtccggcagcacatcctcaagcgtgtgcgcgacctgctcggcggcgtcggccgcgtcggcgtgctgcaccgccacgaacacgggcttgttgtcggcgccctccaccacgagctccgccagccgcgcgaacgccttggtttgcgtgcgcgtcttggccgccaattcgagcttgccgtcgcgcatgcgcaggatgggtttcgtcgcgagcaaggtggcagacagtgcggtgcccgcgctcaagcgtccggacttgcggaggatatcgagctgctgcaggtacagccacgtctccgagcgctcgagggtggacacggccatcgcctcgcattcgtcgaggctcgccccctccctggcgagggtggccgcagccatcgcggccgccccgacggccatgccgacggcatcggtgtccaccacgcgaacggtatctggaaacaccgccgacgccgtgacggcggcggaccacgtggacgacattgccttgcccaagtggagggcgaccacgccgtcatcgccgccgcgctcgagctggcgggcgtaggccgccgttagctccaaggcgctgagccccgaggtcgactcctccccctcggatgcatcgatgacgtgcatgtcgacgacggtgatgccgagctcatcggcgatctccggcggcagacttgcggaagaatcgactacaacgcgcacgctcacgagatgctcaacccctggttccaggcctcgaggtaccactgcaccttgtctggttcggcggcgtcgaaatcggtgggatcggcatcttggctgtagtgcggcatcgcgacaagccgcgaggtgttcgtgttgcccagccccttgagcagcgggtactgctccggcgcaagacccagcaggttcgacgtcagcgcggagatcgtcccgccgtgggcgacgatcagcacgctcgagtcgtcccacccgctataagacgccatcagctcgtcgaccacggggcgggcgcggcgcgccacgtccaggcggctctcgccctcgggcggcgcccagcccgggttgttgcgccagtgggcgcgcacacgcgcgtctgcgctgtccacctcggcatgggtcttgccctgccactggccgaggtgcgtttcgcgcagccgctcgtccacggtgaagtccagacccagcacggcggcgacgatttccgcggtgcggcgggcgcgcgacaaatccgaggcgacgatcttgccgacgccgagttcgcgcatcatcagcgcggcggcgcgggcctgctccacgccggtgtcggacagctcagtatccaagtgcccctgcatgcggcgggtggcgttgtactccgtctggccgtggcgcagcaggataagtcgtcggttcaccgtgtgcgtccgcgaactagtactcgtccgcgtcggggccttccccggcgagcggcaagtcctcgatcgtctccgcctcgcgcacaccggcgttgtcggcgaaggcgcccgggcgctggtacggctccaagccctcgacctcgatgacggggcagtcggagtacaggcggtcgaggccgtagaactcgcgctcggcctcgcgctggacgtgcacgacgaagttgccgtagtcgagcagcacccagcggaactcgcggttgccctcgcggcgcttgggctcaaggcccgcgtcagtgagctcggattcaatctcctcgacgatcgcggcgacctggcgctcggtctccgcggacgcgatcacgaagatgtcggtgatcgccatgacgttggagacgtcgatgacagcaatgttcgcgccgagcttttcgtcagcggccttggcggcgatggtcgcctgctcgatggacagttgcgtggcagtcaagaatgtaggtccttaggtctgtggtactaggtacctgtaagtctaacggcagcgtcgtcaggcatacagttcatgcttggctatgtactgcaccaccccgtccggcacgaggtaccacaccggcctgcccccggcggcgcgggcgcggcagtcggtcgacgagatcgccatcgcggggatgtccagcaggtggacgcgctgctggatgtccgagggaagcatgtcctcggtcagctcgtagccgggccgggtcacgccgacgaactcggcgagggtgaacatcgcctcccagtcgtgccaagacatgatcgagctcagcgcgtcggcgccggtgatgaagtacagctgcgcgtccgggtaatccacctgcagatcgcgcagcgtgtcaatggtgtaggtcggcccgccgcggtcaatgtccacgcgcgagacgctgaactgggggttggaggcggtcgcgatgaccgtcatcaagtagcggtcttccgccggcgagatggacctgcccgccttctgccacggctcaccggtgggcacgaagaccacctcgtcgagctggaagcggtgcgccgcctcgctcgccgcgaccaagtggccgtggtggatggggtcgaaggtgccgcccatcaccccgatgcgccgtgccgcgcgggtcacgccctcacctgccccgtgccttcgagcacccacttcgtggtggtcagctccggaagcgccatgggaccgcgcgcgtgcagcttctgggtcgaaatgccgatctctgcgcccatgccgtactgctcaccgtcggtgaacgctgtcgaggcgttgagcaccaccgcagcggagtcgacccggtcggcgaaacgctgcagcgtgtacgcgtcgcgggaggcgatcgcgtcggtgtggccggtggagtacgcggcgatgtgctcgatcgcgccgtcgacgccgtcgacttccttgtacgcgatgtccatcgagaggtactcctcggcccagtcggcctcggtcgcctcaacaaaccccagcgcggggtcgccgtggatggttactccggcgttgtgcagggcgtcgataatctgctgctttgaggcttggtccaagctcgcgtccaccagcaccgtctcggtggcgttgcacacgctcacccggcgcgttttgccgttgaggagcatctcgatcgccgagtccagctctgcggccttgtcaatatagaagtggcagttgccggtaccggtctcgatcgtgggcacggtcgcgttggtgaccacggcctcgatgagcttcgcgccgccgcgcgggatcaccacgtctaccagcccgcgggcggtgatcaggtgctgcaccgaatcgtgggtctcgcacggcagaagctgcacggcttcgcgcggcaagccgtggtctgcgagcacgtcctgcaggatggccaccagcgcctcgttggagcggcgcgcggtcttggacccgcgtagcagcgccacgttgcccgacttcagcgcaaggccgaacgcgtcgaccgtgacgttggggcgtgcctcgtagaccatgcccatcacgcccagcggcacgcgcacctgatgcatcttgatgccgtttgccagcgtgtggcctcgcagcacctcgcctaccgggtctttcaggcccgctacctggcgaagtccgtcggcgatgcccgcgatgcgcgcctcatccagcgccagccggtcgagcagcgcctcgtccatcccggctgcgcggccggcttcgaggtcttgcgcgttggcggcgaggatttctgcggtgcggttttggagcgtggtggcggcgtcgataagcagcgcgttctttgccgactgcgaaagcgcggccacctccggtgcgacgtccttggcgcggcgcgccttggccaggacctcgtcgcgttcgtttcccatcagtagcctgcttccacgtcgatctcggttcgcatcttctcccccgcttcgaacaggcgccagttctcggcggttaggccgccgatgcggcgtctcatgaaccgcgggatgttggcggtgtgcggggtgatcacacacgtgtcaatgccccacagcgggtggtcctccggcagcggctcgggctcggtgacgtcaaggccagcgccggcaatcttgccccgctgcagcgcgtccgtcagcgcgtcggtgtcgatcaggccgccgcggccgacgttgatcaccactgcgttctccggcatctgggccagggtgtccgcgtccaccatgtggcgcgtctcatccgtcagcggagtcagcagcacgaagatgtcgtggctcgaccacaccttctccgcatccgccatcttcacggtccgcgccgcgccctcgacctcgttgccggagcggttcacagccgtgacctcgacgccgaacggccgcacgtactcgatcagtttcttgccaatgccgcccgcgccgatcagggccagcttcttgtcgtcgaagaggtactccgtctcgccgaaaagctgcttctggttccacgaaggagctactgcttgatgacggtgcatcaccgccaacgtaagcgcaagagccgactccgcaaccgtgtcgtcgtagagcccgcccgcgttggcgaaacgcacgccgttagccgcgtgcttggcaaagatctcctggaggttctccacccctgcgtagacgatctgcacgaccttgacgctttcaggcagatcctgcgggaagtcgtccggcccgccgccgaagagcagcaggtccggcccctcgtccagaccaacaagttcgtggccggcggcctcgagatcggcaacgggcttatcccagggggtaggcaaatacgcgaacttcatagacgcccagattacaagcgcgaagcgtagttcgacaggtaatcggcgtggacaacagggcgctgccggtgggcttcgagctccgacgtgtggcgcccgagcatgccggcgaggtcggcggcgtcgtaggcaacctcgcctcggcccaccacctccgaatcaggacccaaaatttctacgatgtcgcctgcgtggaaatctccctcgattccggtgatgcccacggcgagcaagctggtccccccgcgggtgacggccttgaccgctcccgcgtcgaggcgcagcaccccttccgcgtccgccgcgtagagcgcccagaacttccacgcgttgagcttgctttccgggcgggtgtggaacacggtgccgccctcggcggttgcgagcgcgcgctcgatgtcgctggatgcggtgagcagcaccggcacgccgccacgggtggcgaggcgggctgcggaaaccttcgccgccatgccgccggtgccgaacacgcccccgtcgccggcctgcacgtcttcaaggtcagccccggtgaccacttcgtcgatgcgacgtgcgccgggcagcgcagggttggcggtgtagaggccgtcgacatccgaaagcagcacgagcgcgtcggcgctgatgagcgttgctacgatcgcggacaacctatcgttgtcgccgaagcgcatctcggaggtcgccaccgtgtcgttctcgttcacgatcggcaccgcaccgatctggcgtaaccgatcaatggtgcgctgcgcgttgcgggcccgctcccgggacccggcgtccgactgggtcagcagcacctgcccgatcgtgcggccgtagcgcgcgaacgactggccccaggactgcgccaagtggatctggcccaccgcagccgctgcctgcttcgtggccaaatcgcgagggcgggctttcaaccccagcggccccattccggcggcgattgcgcccgacgacaccacaaccacgtcgctgccgcgcgcaatgcgggcctcgatcgcgtctacgatccgatcgattttgggttgggagacttgccccgtttcgtcgacaagcgaggacgtgcccagcttcaccacgatgcgcttcgccgcggaaatctgctgtctgagaggggaacctgccatacgtgcagtgtaaacggggctctacagcgtccggcgaagtgaccgaaacatctccatgggaagaacgcaggccacgccgaattcatctgccacgttggggatcttcacctttgtagagtttggatctgctacccgctcttcgtacgtgacaaccactgcggcctcagtagccgcagcagcgatcagacggggatcagcatggcgaaggaaattgttgacgtgtcgggaagcgtacgggcgtgcagggtcagtcacccaatccgccacgcgcgccagcattctggcctgggcgaggttttcgtacagtacgtcaccgcgtcgctggtcaacgttgtttttcagccagccggttagccatttgtcttccagcgttgtcacctccctgtacacagcttccgggatcttcacctcaccgttagctacggcgtcgagtagttggtcccagaagccggggacaacgtcaggcggataattcctctcagcagccgaaatgagtacgtttgcgtcgaggaggtacatggatcagttctcttccaacgtggcaaagaggtgttccagagctgttcgctttgatagcccagtcagatccagcgcgtcgcgaactgggagcagagacgtgcccatcgagtcccgcaatgcagacagcagccgctctcccgtccttgcttttacattgcggaaggtgctcccgccgcttgaccgctctcgtaggggaatgtcgagagcggcgtgttcagccagcaaagaatccacggtttcaagtgaggctagcccgagctccctcagcctgtagacgaatgctgggacgctgaccccaaacctccgagctgcgtgctggatctcctccaaatccgcttccttcggcagcccgagcgagtggaccgcttctgcaggcatgaggaacgctgcggcgaacccgttgcaccaccgctcaatctcctggggtgccccgtttgcgacttcgctggactcgttagagatccctggtgcaccaaggactgcgtgacctagttcgtgcgcgaggctgaacagttgcgcagatttcgcgtcacgggtgttaacgaaaaccagagcaaacccgtcctgaatcagcgtgaaacctcgaaactcctcgacacgcaacggtttaaacgaattgttgccaaccatggagttgcgggtaaccagcactccgctttcttctatcgccgaggacagcgccgcgatagcttgatctccaatgacccggcttccaggcacccagccaagcagattccgcactctttcagcgacactctcggcagcctgccccaaggtcgcactgcccactatccctggcggcatcaacccgacttcgtccgcatactcgaggtaccaatccagctgccgttgtgcccgctcgatcgccgctgccaattcaacgcttggatcgaccaccagttgggaaccgaccgtgcggaaatcaggcagctgcacgtccagcaaacgcggcttcgccagcaaaaggagagggtaaggcacagacgccttagcagcgagggcttccgcctgacggatggtcggctggctcgtcccattcacccaattctctatctggttgaattcagaagatcgtgcgagctcctcaaccgttgaacccgtgcgtgcaatcgcccagtccaagactggcttggcaatggggatgcgaactggcgcggccacgggtgcgtcacctccctacggagtcggttgcccgaaaatatagcacccctggaacacacaccgccggagcttcgtcgctcccctacccctgccagcgctcggtgtcggcggcctcgtcggtgccgtagtcgtactcgtcgatcaggccgcggcgggcctgcgaggcacgcttgcgctcggcagcggacgcgcggtcggtgccaccaaatcgcgcgtcttggccgcggccggcaagtgtcgggtcgccgcctcgcgatggctcccagtcgaaagagatgtcgccgatggtgaccacgtcgccctccttcgcgccgatcttgcgaagcgcgtcttccacacccgccttctccaaacggtcggagaggtagccgacggcctcgtcgttttcgaagtccgtctggcggatccagcgctccgccttttcaccggtgacaatccagccctcggggtagatcgggtcgcgctcgacggcgatgccggtgtcgcgggaacgcgaagcgtccttcggccggatgacctgcggctccgcggcgcgtgccgacttcggccgagccttgcgggactgctggacaatctcccacatcgcccacttcagctcgtcgaggccctcgcggctgacggtggagatgagaaacaccggccagccgaacttggcctcaatgtcgtctttgaggaattccgcgagctcgcgcgcctccaacacgtcgatcttgttcagcacgacaaggcgggggcggtcgcgcagatcgcccaagcccgagtcgacgtcgagctcgtccgcgtaggacgaaagctccgcttctagcgcctcgatgtcagaaatcgggtcgcggccgggctccatcgtggcggcgtcgacgatgtgcgcaagcacagcggtgcgctcgatgtggcgcaggaagtccaggcctaagcccttgccctggctcgcacccgggatcagccccggcacgtcagcgatggtgaaggtgtcgctgccggtgtcaaccacgcccaggttcggtgccagggtggtgaaggggtagtccgcaatcttcggctttgctgcggacagcacggagattaacgacgacttgcccgccgaggggaaacccaccagaccaacgtcggccatggacttcagctccagtatcaggtcgtgggcctcaccgggttcgcctttcagcgcgaaccccggggccttgcgcttcgctgtcgccagcgccgcgttaccaagaccgccgaagccgccctcggcggcgacgaagcgggtgcccggctcggtgaggtcggccaagacttcgccgtcggcgcttcgcaccaccgtgccgaccgggacctcgaggatcaggtcctctccgcgggcgccgtttcggtggtcgccctcgccgtttgcgccgcgctgcgctttgacgtgcgggcggaactggaagtcgagcagcgtgtgcacttgcggggagacttccaaaatgatgtcgcctccgtgcccgccgttgccgccgtctggcccgccgagcggcttgaacttttcgcggtgcaccgacacgcagccgtgcccgccgtcgccggcttgcaggtggagaacagcttggtcaacaaattgcgccatagtcagccagcctacttggtcgcgcgcgctacaaagatcccagtgagcgcagatcgtccgcggtgatcgtggtgcgctcctccgcccccgccggggcgaagttgccgccgtaggtgcggaagagacgaatcgagatggcgtcgacaagcttgcgctccgccctacccaggttgtcggggctgacggacgcgagcgcttggcgcagctgcgcctcgtcaaaggtgtaacccttcgacctcaggctgtccaccaccgccgacgccgcatcggggccgggttggcccgccgctgcgccgaccggacgcgccgtaagacggttcgcctccgccgccgggcgcggcgcgcgcactgccggcttaggctgaccggcttcggatccaccggtctcggatgtgtcgacccactcgccgccgcggcgctcaaacaaccgcgcaccgggcgcgttcaccgtgctggtgcccccggcgtagacgcggaagtcggacttcggcgcggccaccacctcgtcggcgcgaagcgcggagtcgccgaggtagagctccgtgtcgtaggcgagtagcccaagcgcggtcagatcgatgtcggtgccggccttcgcgtgaatcgcgcgtttgcccgcgtggttttccataatgctcacctcaccggtgatggtggcgccttccgcctcgaggtagtagatccagtcgccgtcgaagttggcggtggactcgtccacgcgcacccagccaagcatgctcgcctgcgaatacagctcgctgttctccgccgccaccacgccgacccaggggcggctttgcggcgactccaccacgcactcgtcgaactccaacacgccgccgttatcggcgccgatctgggccatgttgatcgggtgctgccccggcacgaaccgcacctcgtaggcgcggacgcggccgccgtggttgtaaatgaccatgtcatcgggtgcctggatcagcgtcataccgctgacgttgagctcttgtccggcgtcgacatcgacgctggcgctcacccacaccgtgcactcgtcggtaccagggccgataaacgtcagcgggccggcgtggatagacaggcccgtaatcacgtactcgccctcctccatccgcacgaccgtccctggtgcgagctgaggcacgatgaggtcgtcgaacttgtcgccgtccgcggcgcgccagaggacctcgcccgcattcgacccgccgccggcaacgacgcacatctccgaatcaaggttgatctgggcgccgtcctcggcgttgacgcggacgcgctcgccgtcggtttggatgcgggggatgtccacatacgcgtcgtcgacgctgatgtaggggttatcgcccttgaagtagagctgcggggcggtgaacttgccgccggaatcgaccatcagcgccgaatctccacctgcaggcgcaatggcgcaggccccgtcgagcgccataatcgcaccgccgttgacgcgcaccgcgcccagcgtggactgggaaacagacgctttcgactcggcgccgacgttgatgtaccccacgcgggatcgctcgataagcaggtgcgccttcgtagcaacgagggcgggccgctcctcggtctcctcgaccacgcagctatcgagctcaaggccggcgtcgttgactcgcaccgcgaccttctcagcgtcagggcgcaggcgcgccgcgcaatgatttagcgtgggaaaaccagagaccacgtcgaaggctgggccgtccttgggtgcgtggacgccgatcgcccacacctgcgacgcccctgacaacaccaccgtgccgtggatgcgggcgacgtcggcgccgttgccctgcaagaagcggtcatcaacaatgagggggcggtgaaggaagtagtctccgccggagagcacaagcccgtcgccgggcgccacagacgcgagtgccgcctcgaggttcgacgacgggtccaccactcgggaggtgttgttatccataaggcgccagtctacaaaacgcaaaagacgcgctgcggatcgtttgacccggcaacgcgtccgtccttcaagcggaaagcccttaagcggtagcctccgccacggtgccttcctcgaccacacctgcggcctcggcagcctcgagcacctcggaagcaacgccctcgccgtcagccgggacgatgttcacaacgcggcgcttcttcttgatgccgaactggacagcgccagcggtgagcgcgaacagcgtgtcgtcgccgccgcggccgacgttgtcgcccgggtggaacttggtgccgcgctgacggacgatgatctcgccggccttaacctgctggccaccgaaacgcttcacgccaaggcgcttggactcagagtcacggccgttcgcggagctggatgcacccttcttgtgtgccatggttcaaatctccttgattgaaaagtcttggtcagcttacttgatgccggtgatcttcagctgcgtcagctgctgacggtggccctgacgcttcttgtagccggtcttgttcttgtacttcagaatgttgaccttcttgcccttggtctgctggacaatctcggcctcaaccttggcgtttgcaagcttgtcagcgccggaggtgacgtctgcgccatcaacgagaaggatcggggtgagttcgaccttgtcgcctgcttcaccctcaagcttctcgaccttgaccaggtcgccctcggcaaccttgtactgcttgccgccggtcttgacgatcgcgtacatagagggttaccccttatctcttactcgcccgctgcctgcatgccacggcggcggaatggaacatggaaagcgtttcggggccgtagttgatggccagccgtgcccgcatgcgtgggcatcgaggcggcgcaccccgaaacagcgactgtcaaagactacaccggcgacttatgaatcaccaaaactagctcgacgtgcgacgcgtagcccggcggcggccccggcgcggcgaggattccggctgcggcttgtccgccggctcctccgccggcttccgcgtcgctgcggcgcgcttcggctgctgggccgctgccccgctcgtcttccgggtcgcccggcggcgctcgcgtgtgcggggcttcggcttgtcgacgccctcctcaccgcttcgcgcgccagacttcctgaccggccgctcactgggttcgctcggctcgctcacatcgctcggctcgctcgcgctctcgaagttctcccggcgcgggcggtggtcggagcgcgagttgccgcgggtgcggcgcttgcggcgcggcgaggcctcgaactcttccaccgcttcctcgtaggagatgccggcagtctcggaggtctcggtgttctccgtctgctgcggctcctgcttgcctcggccgcgggagccgccgcggcggccgcgcctgcgggagcgtttctcgccggtgtcctgcttctccgagatgaccgaatccgcgatctggtcgagctcgtcctcagcgagcgcgtcgccgcgggaagcgtcagtgtcagtgtcagtgtcagcgtcagcgctgtcgtcgtgctgcgccccgcgcgccttggctgccgggtggtcccccgccgggcggcggcgctcctccttgaactcgctcttggtctccggctcgaccgggtcgtcctcaatgatcagcccgcgcccgccacaggtttcgcactcgtgggcgaacgtctccaccagcccggtgccgaggcgcttgcgcgtcatctgcacaagacccagggaggtgacttcggagacctggtggcgggtgcggtcgcggccgagcgcctccttcaggcggcgcagcaccagatcctggttctcgggcaggatcatgtcgataaagtcgatgatgatgatgccgccgatatcgcgcaggcgaatctggcgcacgatttcctcggctgcctcgagattgttgcgcgtcaccgtctcttcgagcgagccgccagaaccggtgaatttgccggtgttgacgtcgatgaccgtcatcgcctcggtcttgtcgatgataagagtgccgccggacggcagccacacggtgcgcgaaagggctttttgaatctgctcgtcaacccggtacacctcgaaggcgtccttgccgccgtgcttcttcgggttgaacttgaccaaacggtctgccaggtcaggggccacggtgtccacgtaggagcgcaccgtgttccaggacttctggccttcgaccaccaactcggagaagtcctcgttgaacaggtcgcgcaccaccttgaccaaaaggttcggctcctcgtacagggtcaccggcttggcgcccttggagttcttctccttctcggcttcgcgctgaattgcttcccactgcgtgtgcagtcggttgacgtcggcggcgatcgcctcttccggcacgccctcggcggcggtgcggataatcgccccgcccttgcccggcacgacgttgttcaggatctcctttagccgcttgcgctccggggccggaagctttcgggagatgcccgcgctgcggccgcccggcacgtacaccaggaagcggccggccagcgagatctgggtggtcaggcgcgcgcccttgtggcccaccgggtccttggtcacctgcaccacgacctggtcgccggacttcagcgcgtgctcgatgcggcgggagcgcccgcccaggccagccgccttccagtccacctcgccggcgtagagcacgccgtttcggccctggccaatgtcgataaacgccgcctccatgctcggcagcacgttctgcacgcggccgaggtagatgttgccgatcatcgacgcctggctgtcggaggtgacgaagtgctcgaccaacagaccgtcttccagcacgcccacctgggtgatgcggccgcggccgtcgtggcggtcgcgctcgcgcacaaccatttggcgggtcacagactcgcggcgcgccaggaactcggcctgggagacgatgcgggagcgcttgcggccctcctcgcgcttttcgctgcggcggcggcgctgcgcttccagccgcgacgagccctggatcgccttcggctcttccagcacctcggcggcttcggcgacttcgaccacctcgtcgacgcgatcctcaacctcctcaacgggcgcggaggaaggcgcgtctttaccgctcgggcggctggcgcggcggcgctccccgcgcgcgggcgccttgaacagcggcgcgtacgccgcagcctcctcggcgggcaccggggtgacatccggctcgatgtcggtcagcagcacgtcttccgagtcgacgagcgcgtcggtgtcgtcctcgtcggtgtcgtcctcgtcgtcagcggcgtccacggtgtcgtcgtcaagcgccgaaagctccgcctcaaccttgcgctcgatctggttgatctcgttggcgacgtccttgcgcacgcgctcgcggatcttcgcgtccgcttcgctctctgcggcaccctcggtctcctccgctgccggggcctcgtcgccgcggggcgcggcggccgttgcggccagcgcgtcaagcagttgctcgctctccgctcgcgtcagcgtggactgggcaaccttgaccagacccatttctgacagcgccactaccaggtccttcgaggggacgttcagcgccttcgccagctggaacacgcgcgtcttctcggacagggtcgagcggtcgaagtcggcgtacgggttcgccgctttcttcgtggtgcgcttcttggtggatctcttcttcggcttctcgtcgctgcgtgccacgttatgctccttatgtcttcgcgctgcaccgaacgcgacctctgccaccgggcgctggcgatacaactcgccgccgccgcacagcggctcaagacaggtccgttcgtgagcggaacggtttttcaatatttgtgaaagcttttcagctccagcgcgcacaagatgcgggcgcggcgaagcctcggtgaccattgtggcacacggcgcacgaaaaaacgccccgcagggtgcgcggggcgtgcggcggaagaagcgattagaggttcgggaaccagatcgcgatctcgcgctcagcggactccggcgagtcggagccgtggacaacgttttcgcccacagtcagggcgaagtcgccgcggatggtgcccggggtagccttctccaccgggtgggtgccgccggcgagctggcgccacgcggcgattgcggactcgccctcgacgatgccggcaaccagcggagcggaggtgatgaagtccaccagctcgccgaagaacggcttgtccttgtgctcggcgtagtgcttctcagcggtctcgcggtctgcggtgcgcaggtccatctccaccagcttgaggcccttgcgctcaatgcgggagatgatttcgccgacgtggccgtttgccacgccgtccggcttgatcagaatcagagtgcgttcagtcatgcgcctgatcttaccttttcctaccttttcgcgttacacctcgcgcacgatgcgcgccgcttcctccgccggcggattccggaaccacagctgcacctgctggatagccagctggtggttgccctccgccttcatacgtttgatagtggcgcgctgctcgtcgtcgagcacaatcggcttgggctcctgcttggacgcgacgtcatagaacccccagagcagaaacacgccggcgatgacgatcgcggtgacggcgatgccgcgcggcagacccatccactgccccgcgatggcgacgacggaaaacacagcggcgacggtgaaggcgaggtagcgcatggcaccgtttataccgcgtttatgcccggttattcacccgcgtacgcttgcaccatgttctacgccagtccgctgccagacatcgcgctgccgaacaccgacatcttctctctcgttttcggcgggctgggcgcggacgccgctttgcctgcgatcacggaggttgactccggccggacgctttcctacggcgagctgcgcgacatggcggagcgcgtcgcttccggggtcgccgatggcgaggtggtggcgcttcggcagcccaactccgcagcgttcgcggcggggcttttcggtattgcccgcgcgggcggcgtagcggtgctgctagggcatgtgcttactagcgccgaagccgaccacctcacaacgctctcgcgcgccgcgcgcgtgatcgaccccgccgaacagccccgcgactcgtttgcgccgccggcgcgcatcgacccgcagcaggtggcggtcatcccgttctcctccggcacgacggggctgccgaaaccggtgcagctcacccacgcagccgtcaccgccaacgcggcgcagtttggcgccgcgctccgcgcgagcgggatcgagcgcggcacacgcacgtttgcgccgctgccgtttagccacatctacgggctgaacacgctacttctctcctccctcgccgcgcgccaccacgtccacaccaccgcccgcttcaacctggaggagatggtgcgcgtccaccgcgaacacgccatcgagctcagcttcatcgcgccgccgatcgcgcggatgttagccaaggagcagctcgacgagcgcgccttcgacgcctgccggttcatggtgtgcggcgccgcttccttggacgaggacctggcccgcgcggtggagcgccgcctagacctcacgatcctgcagggctacggcatgaccgagaccgcgccggtgacccacgtcggcatcgcggggaaatctaccccgggctcgatcgggtttgcggtgcccaacacccagtaccgcatcgtggacctcgagcaccgcgcggatgtcgctgcgggcgacgctggcgagctgcttgtgcgcgggccgcagctcatgcgcggctaccttggtcaacccccgcttgaagaaggcgcgtggctgaaaactggggacctcgcgcgccagctggacaacggcaccgtcgagatcgtcgaccgggtgaaagacgtgttcaagtaccgcggctaccaagtctcacccgctgagctcgaggcggtgctgctcacccacccgcaggtagccgatgccgcggtggcaggggtgaaacgtgacggtcaggacgtgccgtgggggtttgtggtgttcaggggggcgtcgacaagcaacgaagccctcatgcgctgggtggcggcacgcgtggcaccgtacaaaaagctgcgcggcgtcacgcgggtcgatgaaatcccgcgcaacgccgccggcaaaatcctgcgccgaaaactacctggcgccgtcggccgatgagccgaggtgctgcgtgaccaggtaaccgaagcgcatgcgctgcatcatttccgagcgcattttcacaatgtagtaccagacgatgccgaacacgatacccaccaccgtgaccgaccagtggatgaagaacccgaagatcagcgggatctgcaacgcgagatcgatccacagcgcgccgggcacgcgctgcagaaacgccatgatgaggtgggctgcgccgatgacggtgatgtagacccagttgaatgtggtccacagctcgccgttatccaccttcagcaccaccagcaggatgaggaagatggtgatggcctccatcacgagcgtgccggagagcacaccggtcagcgccttcatcgggtccttgactggggcgtggccggggccgagcgggccgtacagcggtgcctcattcttcgcgcgcctgcgtggggtcatcattgcggatcctttccaaacatctcgcgtgcctcgccggcggtaaccaccgaacctgtgatcacgatgccgttgccggactgcacgcccggctcgtccagctcctcctcggcgagctcgaccgcgagcgcgtaggccgacggcaggtgctcctcgacgtggacgcgctcgtcgccgaagacctcgcgcgcggtttccgccagatcataggcgccggctgcgcgcggcgacgaattttgcgtgatcacgacctcggtcagcacaggctcgagggcctcgaagatgccgcgggcgtccttgtcctccagcaccccgagcacgccgatgagccgcgtgaagttgaagtcgtgctccagcgccttggccagcgcgcgggcgccgtgggggttgtgtgtggcgtcgacgaaggtggtcggcgcggtgtgcacgcgctcgaggcgccccggcgagctggcgaggcgaaagcccgcgcgcaccgtgtcggcgtcgagggggcgttcagcgttcgcgccgtaaaacgcctccacggcggccagcgccaccgcggcgttgcgcgcctggtgcggcccggcaagcggcaagaacacgtcgtccaccacgccggacaggccgcgcagcgtgagtagctggccgccgacggcgatctccgcgtcctcgaccgcaaactcctggccgaggcgcgcaactggtgagccgaccgcgacggtctgctcgaggatcacgcgcatcgcgtccgcgtcctggtcagcgatgacagccaccgcgtccgcgctgcggatgatgccggccttttcgcccgcgatctcctcgatggtctcgccgaggtactccgtgtggtcgaggcccaccggcatgatcacgtccacgtcggcgtcgaccacgttagtcgcgtcccagcgcccgcccatgccgacttcgaccactgcgacgtccaccggcgcgtcggcgaacgcggcgaacgccaccgcgaccatgacctcgaagtagctcattggggtgccggcgcgctcgtccaccatctggatgtacggctcgatctcgcggtagacgcggacgaactccgccgggtggatcggctcgccgtcgatgccgatgcgctccgtgacctgctgcagatgcgggctggtggtgcggccgacgcggttgccgaaggcgcgcagtaccgactcgatcatccgcaccgtcgacgtcttgccgttggtgcctgcgacgtggatgaccttgcaggccttctgcggctcgccgagcaggtccatcagcagctccacgcgctcgagagtggggtcgatgacggtctccggccatcgggccttcagctcgtcctcgacctggaccaacgccgccaagtcgtcctcggtgacggggcgcggggcgtactcctcgtcgtcggcgctgtcaggttcgccgcctagcggggtgcccacgctgccgaggtggagcgtccggccgtgctcgttgtcttcgacctcgtagatctccgagttttcgaggctgtccgagctatccattgagcccctcaagacgcgcggtgacgcggtcgaactcctcgcgcgcgacctgctggcgctcgcggatcttcgccacgacgtgctccggcgcgttcgctaggaactggtcgttgcccagcttcgcggcggtggtgtcgagctccttctgcgccgcggcaagctccttttccaagcgcttgcgctcggccgcgacatccaccgtgcccgaggtgtccagctccacgttcagggtcgcctggctgagacgcatttcaatgcttgacgacgccgcgaagtcctccccaggcgcctccacccgagcaatcgcgcgaactgcgccttccatcccctccaggtcagccgacgcgaagtcgagccgggccggcaccgtctggctgggcttgacgccctggtcggcgcggaagcggcgcagctccgtgatcagcttgaccgcgtcctccacgcggcggcgggcgtctaagtcggactcggcgccgccgttggtgtcgtccgcggtcggccacggcgccagcgtgatcgtctcgcggccggtgagtgccttccacagcacctcggtgatgaacggcatcgtcgggtggagcaggcgcagcaccacgtcgaggacgcgacccagcacgatctgggtggtgcggccgcgctcctgctcttctgccgacgcgtcagcgttcacgtcgacgcgcgggatctgggtcttggcaatctccaagtaccagtcgcacagctcgtcccacgcgaagtggtagagctcctcgttggctttggcgaactggtaatcgtccaggtaggcgtcgacgcttgcgcggacctcctcagcgcggtccagaatccagcggtccgcgtcggttagggtttcccgctgcggtagatcatctaccgcagcgccgttcatcagcgcgaacttcgtggcgttgtacagcttggtggcgaaattgcgggcgctggtcgcgttgtcctcgccgatcggcaggtccacgcccgggttcgcgccgcgtgccagggcgaagcgcagcgcgtcggcaccgtagcgctcgacccagtccatcgggtcgatgccgttgccgagcgacttcgacatcttccggcccttctcatcgcgcacgaggccgtggaggtagaggtcggtgaacggcacctgcgggcggccgcccttgccctcccccagcacctccggggtctgagtgccggcgaaagtgccgaacatcatcatgcgcgcgacccagaagaacaggatgtcgtaggcggtgaccagcaccgaggtcgggtaaaacttctccagctcgggggtcttctccggccagcccatcgtggagaacggccacagcgcggagctgaaccaggtgtccagcacatccgggtcctgctcgtagcccgccggcgcctcctcgcccgggcccacgcacaccacgtcgcgttcgccgttgtcgtcctcggggccgtaccagattgggatgcggtggccccaccacagctggcgcgaaatggtccagtcgtgcatgttgtccacccagtcgaagtagcgcttctccatcgactgcgggtggatctttgtgtcgccggagcgcaccgcctcggcggacatgcgggcgagctcttcgaccttgacaaaccactgcaggctcaggcgcggctcgatcggctcgccggagcgctcggagtggcccaccgagtggacgtacggcctgatctccttgacaatgcggccctgctccgcgagcgcctcgcgcaccttcacgcgcgcttcctcgcggctcaagccgtcgaaggcggtgccggtgttcgcgatccgccccttctcgtccatgatgatcggcatgtccaggtcgtggcgcaggcccatctcgtagtcgttggggtcgtgcgcgggcgtgatcttcacagcacccgtgcccagctccatgtcgacgtactcgtcggcgatgaccttcagcttcaggtcgtcgcggaacgggtggtcgaactcggcgcccaccaaatgcgcgtagcgctcgtcgtccgggtggacggcgatggcgacgtcgcccagcatcgtctccacgcgggtggtggcgacgattaagtgcggctcgtcgtcgttcagggaaccgtagcggatggagacgaactcgccctcgacgtccttgtacaccacctcgatgtcgctgaccgcggtttccagcaccggcgaccagttcaccaggcggtagtcgcggtagaccatcccctggtcgtacagctgcttgaagatggtctggacagcgttcgacagcccgctatccagcgtgaaccgctccctcgaccagtcaaccgagtcgccgatcgcccgcatctgggtggcaatggtgccgccgtactcgcgcttccactcccagaccttttcaacgaactcgtcgcggccgtagtcgtagcggtccttgccctcttcagccttgagcttcgcctcgaccttggtctgggtcgcgatgcccgcgtggtccatgcccggcaaccacagcacctcgtatctctgcatgcgcttgcggcgcaccagcgcgtccatcagcgtgtgatcaagggcatggcccatgtgcagctgaccggtcacgttcggcggcggcagcatgatggagtacgccggcttgtccgacgccgggtcggccgtgaagtaaccggcctcaacccagccctcgtacagcggctgctcgtgctccttcggctcccacgacttgggcagcgcgtcggcgcggtttgtgcctaccagttgatcattcgcttcagtcacgaacaatcatcttagtaggtcagaaaagcccgtcggccacctcggcttcggcgcgcagcgcctcgatgttggcgtcgatgcgcgggcgctggaattcgttgatctcaaggtcgtccacggcttcccactggccgttgacacccacggcaggaaaaccgaagaccaggccctcgtcgacgccgtattggcttgtcgacggcaacgcaaccgtcacccagcgcccatccgtacccagcgcccaatcgcgcatgtggtccaccgccgcggacgcagctgacgcagccgacgacttgccgcggacctggatgatctccgcgccgcgctttgccacgcgcgggatgaactcgtcggtgtaccacgcctggtcgatctggtcgccgacgctttggccgttcagctgggcgtacgtcacgtccgggaactgggtgtcggagtggttgccccacaccaccaggcgctcgaactcggcggagtccgcacccagcttctcccccagcatcgacagcgcgcggttgtggtcgaggcgcatcagcgcgttaaaacgctcagccggcacgtccggagcagctttcgacgcgatgtaggcgttggtgtttgccgggtttcccacgacgaggacgcgaatgtcgtccgcggcggcgtcgttaatcgccctgccctgctcgatgaagatccggccgttggcctggagcatgtcggcgcgggattcgcccttgccgcgcggcttcgcgccgaccaggaaggccgcgttcgcgccgtcgaacgcctgggccgcgtcggtggagacggtgatgttgcgcagaagcggcagcgcggaatccgacagctccatcgcggtgccttcggcggcctgcacggcgctgtcgatctccagcagcgtcagctcgactggttgatccggcccgaagacgtccccggcggcgacgcgccacagaagcgagtaggcgatgttgccggcggcgccggtgaccgttactttcagcggggttcgattctcagacataccccgagtataggtcgcggccactccccccgtttgtgcttggaagtgtggccttcctcgcgcaaaaacgcgccgagcacggcgaattcgggcaacattgcggctatgacacacggaagcgctgagccatcgcctgaggaggcggtcgcggtcgcgcttgccatgttcgcccgcgacggttacgagggaacgaagcttgacgcggtggcgagagcgtgcggcgtatcgaagcgcatgttgcactaccacttcggcaacaaagccggcctctaccagcgcgcgctctcgctggcgatggagcgcgtcgccccgccggagcggctgatcagccgcaactacgccgtgccggtggagggcatgcgccgctttgtcgacgccaccttccactccttccgcgaccaccccgagtgcgtgcggctgctgttgcgcgaaaacctcgaccccaccaccgacgtggacgactctggctccgacgcgcgcgagcactcagtgcttttgcacttggagcgcattcttatgcagggccaagatgccggggcgtttcgccccggcatcagcgctgacgacgtgctcgcactgactgtgtctctgtgcgagttccaggtcgctcacaccgcgaccgcctacaccgtcagcagaatcaaggtggacgacccgcgcaatgtcgaggggctgcgccgtttggtcatcgacaccgtgctggcgtttttaacgtcgcacatcccccactcgggctacgactcctacctggtctccgagccggccccggagaccatcgacgtcgccgacatctactaggcgggtctacgccgagcgcttctcgctggatgcccggtactccggctctgccttgccgcgcgccactgcgtccgagatgaccacctcggccgcgtcctcgcggtctggcaggtcgtacatcacgggcacgaggatttcctccatgatcgcgcgcaggccgcgagctccggtcttgcgctccgccgccttgtcggcgatcacaccgagcgcctcgtccgtgatggtcagctccgccccgtccatagcgaacagccgctggtactgcttcaccagagagttcttcggctccgtgagcacccgcaccagcgagtcgcggtccaagtcgtcaacgtgcgcgatgatcggcaggcggccaatgaactcggggatgagcccgaacttcaccagatcccccggctggacctgcgccaagagattcgcctcgtcgcgctccgacttggagtcgatctccgcgccgaagccaatgcctttcttgcccacgcgctccgcaatcaccttgtccagacccgcgaacgctccggcgacgatgaacaggatattcgtggtgtcgagctggatgaactcctggttcgggtgcttgcgtccgccctgcggcggcaccgaggcgaccgtgccctccaaaattttcagcagcgcctgctgcacgccctcgccggagacgtcgcgggtgatcgacgggttctcgctcttgcgcgagattttgtccacctcgtcgacgtagataatgccggtctgcgcgcggttgacgtcgaagtccgccgcctgcagcagtttcaaaaggatattctccacgtcctcgcccacgtacccggcctcggtcaagctggttgcgtccgcgatggcgaacggcacgttcagcatccgcgcgagcgtctgcgcgaggtaggtcttaccggagccggtggggccgagcagcaggatgttcgacttggaaatctcaacttcctcgtcgcggcgccggctgcccagcaccgtctgctcggcccggatgcgcttgtagtggttgtagacggcgacggcgagcgtgcgcttagcctggtcctggccgatcacgtagtcgtctaaaaacgccgtgatttcggacggccgcggcaggcggtcgtcgcttgcggacgagttcgacgcggagccggctagttcctcttcaatgatctcgttgcagagctcaatgcattcgtcacagatgtagacgccgcccccggcgatcagcttgcgaacttgcttctgcgtcttgccgcagaacgagcacttcaaaagttctgagctgtcgtgcgttactgccatgtactttctgcaactcccagatgtcaaagtttgtagttactccagcatacttcgtcgcgcaaacatcccttttgggcacaacgcgcgaaaccgtgtccggcaatgatcgtgcacaatgggccgcatgacaaaccttgaggtacacgagttcggtcaacgcggctccggtgtggaaacggtggtgctgctcagttccatcgccaccacccacgagtcgtggaacgagatcatcgcggcgctcgagcccaactaccgcgtggtcaccgtcaaccaccgcgggcacggcgcgtccgaggtggcgcgtgtggcgccgggctctaccacggtcgagcagctgtgcgacgacgtcatacaggcactcgattcggtgggtgtagaccgtttcaatgtcgttgggctttccctcggcggcgccctcgcccagtggatcgcggccaactccggccgggtagaaaaggcagtgttctgctccaccgccacgtacctcggcggtcaggacaagtggtcggagcgcacggcacaagctcgaagcgagggtatggcactgcttgccgacggtttcgtgaactcctggttcacgccctccttccgcgagagcaaccccgacgaggtccgccgcatccgcgacatggccgcgggcgtggacccggagggctacgcccaaaacggcgacgcgctggcgggctgggatttcgccgacaccctcgaccgcatcacctgtcccgtgctcacgatcgcgggcgcgcaggacccgaacacggggccggaggaacttgccgccattgccgccggtgtgtccggcccgagcgaatccgcggtgatcgaccccggctcccaccaagtcgctgtggagaacccgggcgaattcatccgggtgctgaaacggtttctggccggcgcatcggctagccttgagggttgatacacacgaactgccaaaggggtctcacgcgtgaaccgtgccacaacagccgtagcgacactcgccgtctccgcgctcgtgctgaccggctgcgcgtccgaggacgacgaggtgcgcctcgccgaaccggtgctcgacttcccctacaccagcaccaccgccgccccaaccccgacgatggcggcgcctgctgagaccgaggacgccgacgagacggaaacgaccgcgtctgagtcttcgacgacgtcctcctcaacgaagacatcgacgcgcacgtccacgaagacgtcgacaagcacccgctccgcaagctcgacccgccagcaggaacccgcacccgcgccggcccctgccaacccggagcccgttcagcccggcgccaactgcgcgtggccggcgcagggtgaggcaaacgggggcgagttctccaccttctgcgaccgcgaatgggcccgcaccatgctcgacgggcagcagtacttctggcgcgccgaaggcaacggctgggtcagcatcgacccagaagccatggtcgacgacgaggtgtgctggccccgcgacgagttcgacggcgctccggaagctatccgaaacgccgccgtgtactgcgagcccgccgccgaggagccggcggactaggctgcagccttcgcgctgtccgcggtttcggtgggcttcagcccggccaacgcaaccgcgctgacgacgaacacgcacgccgaggtgacgtagagcgacttcggcccccacccggcttgcgccaagtagccgatgattagggggcccagcacagagccggcgcgcgccaccgcaagtgcggcgccgacgcctgttgcgcgcagacgcgacgggtaggacagcggggtcacggtgtacatgccggtcacgcagccgttgagcagcatgcccaccaggatgccgagcgggaaggccacccccggctggtccacgcagtagatgaacgcgaccagggccgcggcgccaaggaccgcgaagaccatcagcagcgtgcgcggcttgaccttggtcgtaagcaccccgaagatcagcgaaccgatcgtgccgccgaacgcgatcatgatgccgccaaggatgccctgctgcgcggtcatgcccgactcgttcagcaacttcggcgtccacgagttggcgaacgagaacccgaagttcaccagcgcgaacgcgatccagagccgcaccgtggtggcgaggaacgccggcgagacaagctcggagtacggggtcttctcggaacgcacaaccggcgccagctccacgtccgagccgtggccgatgcgcttcgccactcggcgaacgccgtcgatatccccgcgggcggaaagcacgtccaccgactccggcagaacgacatacgcgagaaggagcgcgaccgccgagaggatggcgccggtgaagaaaatccactcccacccctggttcgggatgaggcggccggcgagcacgccgcacagcgtggcgccgaggccgtagccggaggcgtagatcgccgtagccaaaccgcggaagcgcaggttggaaaactcggtgatgaccacagtcacgcaggcgagcacaccaccgacgccgataccggtaacaaggcgccagaaaatgaacgtgccggcgctgcctgcgaatccggtcatgacgaggccgacgatgtcgaggatgagggagaccaggacgatcgtgcggcggccgaatttatctgccagcggtcctaagaccgcggcgccgacacccacgccgatcagcgccgcggaaagcacccagccgagcgttgcgggaccgatcccgaactcctcactcagatgcggagcggcaaaagcggtggccacgaggtcgtagccgtcgagggcgttgaggtacgtaatcaccgcgacgatcagccactggtagccggtcatcgggcgcgtatcgattgagctgcggatgttcacgcaggcgaactgtaccgcacggtctagtgaacgagaaaacggtgcgcactggtgcgcaccgtttaattcatcgagccttaagcgcttacgcgttcaacttccggtaatcaaaaacctggtcgatgatgccgtactcgacggcctctgccgcggtgaggatcttgtcgcggtcggtgtcgatgcggacctgttccggcgtgcggccggagtggtgcgccaaggtctcctccatgaggcggcgcatgcgctcgatttcggcagcctggatctccaggtcggaaacctggccgcgggtgccctcggtcgccggctggtggatcagcacgcgcgagttcggcaacgccgcgcgcttgcccggcgcaccggcagcgaggatgacggccgcagcggaggccgcctggccgaggcagacggtctgcacgtcggggcggacatactgcatcgtgtcgtagatcgccatcagcgcggtgaacgagccgccgggcgagttgatgtacatcgtgatgtcgcggtccgggtcctgcgattcgaggaccagcagctgcgccatgatgtcgttggcggacgtgtcgtcgacctgggtgccgaggaagacgatgcgctcctcaaacagcttgccgtacgggtcgatctgcttcgtgccgaagctggtctcctcgaggaactgcggcagcacgtagcgggagctgggcatttggaaagtcatggaattctccttcttcgttgcttgccggttagtcgccgatggagtactcgccggcctgcgcggcgttctcgatcacgtggtccacgatgccgtagtcgcgcgcctcctgagcggtgaaccatcggtcgcggtcggagtccttggtgatctgctcgaaggtctggccggtgtgctcggcaatgagttccgccatctcgcgcttggtctgagcgaactgctccgcctgaatggcgatgtctgccgcggtgccaccgacaccagcggacggctggtgcatcatgatgcgcgcgtgcggcagggcgtagcgcttgcccttggtgccgccggagagcaggaactggcccatcgacgccgcaagacccatgccgtaagtggcgatatcgcacggcgagtaacgcatcgtgtcgtagatagccatgccagcggtcaccgaaccgcccggggagttgatgtaaaggttaatgtcgcgtgtcgggtcctcagcggacagcaggaggatctgcgcgcagagcttgttcgcaatctcatcgtcgacctcctggccgaggaaaataatgcgctcgcgcagcaggcgctcgtagaccgagtctcccaggttcattccttgagtcggggaagtcataacaccgctccttcgctagttttctcgtgtaacgccccaaccctactcggctgtagtgggaactcccagcgcgttcgctaccggcgtacgcctttgcacaaggcaaacaaaaaagcagccggggctttgccgcccaggctgcttagcgcgttgcgcgaagaggtttactcctcggtcgcgggagctgcgtcctcgacaacctcgtcgtcctcgatctcaccgaagtactcgttcgggtcaacggagttgccctcggagtcggtcacggtagtgcgcgagatggctgccgccagcgccttgccgcggcgcacgtcggagaacaggttcgcgatctggccggactgctgcagctgagccacgaactgattcgggtccatgccgtaggactgcgcggtgaacaggatgtggtcggtcagctcctcctgggtgacctccggctgctcctggtcggcgacagcgtcgaggaacaactgggtgcgcacggattcttcggcctgggtgcgggcgttcgcgtcgaactcctcgcgggtggtgccctgcgcctcgagcagctgggcaagcgcgttgtcgtcgtgcgccagctggcccaggatctggtggagctggttgtgcacctgctcgtccacgatggactccggcagcgcgaactcggactgcgcgagagcggccttgagcacctcgtcgcggatgtccgcggcctgctgcgccttcagattctcctcgagctgggtcttggtggactcgcgcagctcctcgacggtgtcgaactcggacgccatctgagcgaactcgtcgtcgagctccggcagtgcgcgctccttggtctggttcacggtggccttgacgacggcttcctcgcccttgtgctcaccgaactcgatggtggtggtgaactcggcgctctcgccggacttcaggccggtaattgcggcgtcgaggcccgtgatcaggtcgtcggagccaacctcgtagttcaggccctcagcggacgcgtcctcgagcttctcgccgtcgacggttgcctcgaggtccagcacagcgaagtcgccctcggccagcttgcggtcggtgtccttcagctcgccgaagcggccgcgcaggttctccagctcagcgtcgatcgcctcgtcctcgacgttcagcgccggaacggtgacagagatttgggagaagtctggcacggtgatctccgggcggacgtcaatctctgcggtgaactcgactacgtcgttgtcctcgatcttggtgatctcgatctcgggctggccaagcgggttcaggtcgttctctgccagcgcctgctcgtagcgggtcggcagcatgtcgttgacaacctgctccaggatcgggccgcggccaaagcgtgcgtcgatcagctggcgcggcgccttgccgcggcggaagcccgggatggtgacctgctgggcgatcgccttgtacgcctggtcgatctcgcggcccagttcgtcgaacgggacggagacgtcaagcttgactcgggtgtcgctcagcttctcgacgtttgtcttcacggatgttgtccttctagatcggtgtacatgaccttgtcggggcgacaggatttgaacctgcgaccccctgctcccaaagcaggtgcgctaccaaactgcgccacgccccgtgagtggaacccacgaccgaccattgtagcgaccggaaaaccgacggcgttatgggggccgagaaaaataaaaagcccggcctgagctggccggacttggagggaacgacgggaatcgaacccgcgtcttcagcttggaaggctgaggtattagccactatacgacgttcccacgcgcgaaaaagcgctgttcggaatgttagcgcagccggtaccgttgaaccaaacacgtgactgtatctattaaggagccaccgtgtccttgctatttatcctccttctcttctttatcggccccatgctgttttttcccatgatgggcggcgggcagcagcggccaatgtcgcagcgccaggtggcgcagcgggagcaggtttcgcttgacgacgcgctcgcggacgccaaacgctggaccgatcgactcggctcccagattctgaacctcgagggcaccgacgccgcctccaagcaggccatggcggacgcgtccgagcgcttcaacgccgcccgcgccgggcttgcggacgcgcgcacgccgaagcaggcgatgctggcgcgcgaatccgcgctcgagggcctgcactacgtcaacgcggcgcgcgagatcatgggcctgcccgcgggccctcagctgcccgagctcgagggccagcgccaggccggccgcgtgaccgaggagcgcacggtgcgccaggacgacggcacgctggtcaccgcctcgccctacgcctcggcacagacgccgcactactaccccggcggcgccgtggccggccgcccggtcccggccggctggtactccaccgcgtggtgggcgccggcgatgatgaccggcatgtgggcggcgagctccatgatgttttattcggccatgttctccggcatggcgggcgcggcacccgctgccgcgttcgaggcgggcgacctcggcggtgacctcggcggaatggacggcgccggcgacattggcgacatgggtgacatgggaggggatctcggcggggacttcggcggcttcgatttcggcggcttcgacttctagccccgcatcccgggtgcgctagaatctgcacgtctacccgcgagaatgaaggagcgcccgtgcgtatcgccgtgctgctgaaagaggtcccggacacgtacagcgaccgggaaatgagtttggagactggcctgacggaccgcaccggcgatgtggtggcggacgaggtcggcgagcgcgcggtcgaagccgcgctgcgcatcaaggaggcccgcgagggcgacgcggaggtccacatcctcaccgtcggcccggaatctgcggctgacgcggttcgccgcggcatcgccatgggcgcgtcggagggttttttgcttagcgacgtagccctcaccggcgccgacctcaccctcacagccgaggcgctcgccgcgatggtggagaagaacggttacgacctcgtcgtctgcggcgcaatgtcgtcggacggcgcggccggcgtgatggccccgatgctggcagagttgctgaactggcccgcgctgacgaacttgtccgagctcgcgctcgacggtgagtccgtggttggggttggtgtgggtgaggggggcgtcgtaaagcttcaagcccctctgcctgccgtggctgcggtgtccgacgagttccccgacgcccgctttcccaacttcaagggcctgatggccgcgaagaagaaggagctgcacaccttcgccctggctgagctgggtattgacgcggaggactactcccgcccgcgcgcgatcatggtggatgtcgcgaagcgaccggcgcgagagcgcggcgagattattgacggcgggaagaccgcagcgagccagctggtggacttcctcgattcccgcggcctgctgtaaggagaacccgatgactgacactgtgcttgttgtgctcgaccgcgccggcgacggcgccgagctgatcgcggccgcgcgcgagctgggctccgtggccgttttgaccacgacgcgcaaggaggtgcccggtgcggaccaggtgctcgtcgccgaggttggcgaaggcgccgtcgcgctggtcgacgcggtggaggccgctgtttcccgcctgaaccccgccgctatcctcttcgcacacacggccgccgggcgcgacgtcgcagcccgagtcgcggtgcgcctcaggagggcgttgcttaccgacgccaccgcaatccgccgcgacgcccacggcatcgtgaccgagcactccaactacggcggcgcgttcaccgccaccgcggcggccacccacctcgcgccggtggtgaccatgcgcccgggcagcgtcgacgccgccgttgaggcgtcctcgtccgaggtcgtcgagctcgatgtcgccgcttctggccgccgcgacgtgaagatcctggaaaccaccccgatcgagcgcacctcgacgcgccccgacctgctcaccgccgacaaggtggttgccggcggcgtgtccctgggcagcgacgacatgtttgaggagcttgtcggcgggctcgccgacgccctcggcgccgccgtcggcgccacccgctccgccgtcgacgagggccaagtgccctacgaggcgcagatcggacagaccggcgtgatggtcagcccgaagctgtacatcggcctcggcatctcaggcgccgtgcagcacttggtgggcatgcagacatccgacaccatcgtcgccatcaacagcgacgaagacgcgccgatcttcgacatcgccgacttcggcatcatcggcgacatcttcgacctcgtcccggacatcatcgccgagatcgaggcccgcaagtccgtgtccggcgaggtgagcgagtaaccatgcagatccccgtccgccgcggattgccgcgcaccccgggcggcgaagggtggccgcccgtcgacgccgtcgaagtcgaagacgccctcgcccctgcccctcttgcagagaccgccgcctcggagcccgaaccggccggcgaccgcgtcgccgttgcgttacgacgcggcctgccccgcacccccggcggcgacccctggccgcccgccgacaccgcactcgtcgacgcctcccttgtccccgccgagccagcctcagcgcccgaaccggccgcggagcccgttcccgtgccggctgccgctcccgccaccgagcccgcgccagcgccgcagccgcagcaaccgcgcaagcgcccccgcggactcggctggctcgcagccgcggtcgccctcttcgtggtcggcgtggtgttctcgcgttggttcctcggcactgacaccggcgccgacttcatcacgcgctacgacggcaagcagccgctccccgactccgcccccaccggcattcccgcctggttggggtgggcccacttcttcaacatgttcctgatggcgttggtggtgaagacgggctgggcgattcgcacgcaagcaaaggccccggcgtactgggctccgcgctccaacccccgggcgaagatctcgctgaaccaatggatgcacttggtgctcgacgccgcgtgggttgtcttgggcgccgtgttctacgtgctgctgtttgccaccgggcagtggatgcgcatcgtgccgacgagctgggaagttatccccaacgccgtctccgccggcttgcagtacctctcacttgactggccgaacgaggacccgtgggtggcgtacaacgcgctgcaggagctgatgtacttcgcggtcgtcttcctcgccgcgcccttggcgattctctccgggcttcgcatgagcccgttctggccaaagaggtggacgggactgtcgctcaaggcggcgcgccgcatccacttcccagtgatggtgttcttcgttgtgttcgtggtcatccacgtggcgctcgtgctgctgacgggcctgcgcggcaacatgaacgcgatgttcgctgcctcccacgacgccgaaagctggaccggcgtactggtgttcctcggcggcctagtggcgattgcggcagcgtggttcgccgcgcggccgatggtcgtcgcaccggtggcggcgaagttcggcaacgtcacgcagcgctaacgccggccgggccactaccgccaaagggggggggcggatagcggatggcggaagtacgggttcttactcgcatatccgccatccttcatccgccatccctcatccgccatccttcatccgcccccctgcgaatgcgcgggcacccaggcggtctcatcgcaccggtggcggcgaaattcggcaacgtcacgcagcgctaacgccggccgcggccactaccgccaaaggggggcacccaggcggtctcatcaccccggtggcggcgaagttcggcaacgtcacgcagcgctaacgccggccgtggccactcaccacagggggggcggatagcggatgacggaagtacgggttcttactcgtaaatccgccatccttcatccgccatccctcatccgcccccccctggaaaaggcggtccctggaaaaggcggcccgtggaaagggagcccgtggagggaacccgtgaaaaggcagactgtgaagggcacgggaaaaggagcgcggcacaccggctggcggggctgaagaacagcccttcccgcgctactgcgggcggcccatctcaagcccggcgatgcgctccgcctcgtcgatcaccttggctagcgcctccgtcacacggacaaaagcttcgccacccggggcgagcaggtcgtcgcgcacttcgaacatgatgcccagcactgccgggttcatctcgtactcgacagggatgtagacgccggtgaacggggtgttgcgctcgacgcggaagccggcttcggtgaaaatgcgcgccgcggtgtcgacgaggatcgccggggagtgcaccgagtgcgtgccgatgcagatgtccggggagagccggccgccgtggatctggtgctcttcgggcgggttgttatacgagtggatgtccacgatcaccgcgccgcccgtggcgcggatgcgctcgcgcacaagctcccccaccgcgtcgttgtacgggtggaagtacgttgccttcagggcggaatcgtcgaagcctaaggggcggagcagctcgccgtcggtcagccgagtgtaaacggcgccgcggccggaggcctccatggagtcgcgctggctgtagaagcggcccggatccgcgaccaggcgcgacagctcgttgaccacgagccagctgcgctgccccgccgcctcgtgcgcggcgcgggcgagcgcgtcggtgcctgtgtcggtcacgcggtccagttcctgctcgacctgctccggcgtggcggcgaaatcagccgcgactgcatctgggatctcgcgcgatgcgtgcgggacgtggaggatgacggggctggcgtctgtgccccggcttacgcagaggtgctcgtacatacctcgcaaggttaagggtgtttgggggtttgtgcttgccaggtgccgtcgataagcgaaacagccccttccgcctcgaaggccttcagccagccacccatgggaaactcgccccacttcgagtggaagtagttggcgttgcgcacgatgtcgtccaagtgctcccacggcggggacgacaccgggtgccactggtggaacgcgtgcgcgccgccgacccagtagaggtcgatgccgtgggcgcgcagctgccaggcaaaatcggtgtcctcgccaccgtatccggtgtagccggtgtcgaagccaccgaagtcgcgctcgatgcgccgccacgtgtcggccgtcagcgcgaaggagagggaccagaacaggttgtagtcgtcggccttcaccagctcgccgggcgccgggttggggcgcgcggggtgcgggtcggggcgcacggtgcgtaactcgccttcgcgcatgtacgtcactgggcccgcgaccaccgcatccgggtgcagggcgagcgcgcgcgtgtagtgcgcgaccaggtcgccggaggccacgcagtccgcgtcgaggaaaatgatgatatcggcgccgcgctcaatcgcggtgcgcgcggcgaggttgcgcgccgccgcgaggttcggctcacccgccacgacgtgcgacttcggcacggctttgcgcaagccttcagcgtcggcgagcgcaacggtgatgtggtcggtgccctcgggcttcaagttcacctggtgggtcaggtgcccagcgcggttggcattcgccagcgtgaccagagcaatttttttgcttatcgacgcccccctagccaccttttccaccacatcggccgcccgcgccgccgccccgtccgtctgccaccgcgaccagtcaccagccgactgcgcgcgtcgcagcagctcgggccactcgcttgctggcgggaacgtgtcggcgacaacagcaaggcccgcctcgccaacggtggctgcgttgagcttctgctcgatgaacgggcgcggctgcggcagcaggacggcaggtgccccgcacgcggcgatgtccgcgatcgagttctgcccgcccgcggtgacgaccacacccgccgactggaggagctccgtcgggtcgtcgacgcggttgtcgccggtgaggtacgtgaaccggtagtccgggcaggctcgctcgacgtcctcccaatcctccggctcccacgtggagccgccggtgcccgccatcaccacgacgtggtgcgggtcgcgggcaacccccggcttggggcgaagccgcgagatgccgccgactgcgtgcaaccggtcttcgtgggcgcgcaggtgctcgggcacgtcaacccagtccggccacgcggcgatcagcgcgtcggcctgggcgtaggcgagttggtgcggggtgtcgtcgcgcagccccggcatcgcgtgcgccaccaccggcacgcccataagacggatgaacatccccacctcggcggagacatcgacgtagaacgcgtccgggttgtgctccgcgatccaggtggcgatcgtggcgaagcgcttcttcaacccctcgttgccgtagggcgcgtagtgcaaagatccgccggcgttcatggagcggccgtagtggccgtggccggcgtcgtcggcaagcagaatgcccccgcgcgggtcggtggacaggattgtcacgtcgtgtccgcgcgcgacgagctcccgctggatctcgcggcagcgctggatgtggccggagccgtggtggtgggcgtagatgccgatggtgctcacgatgcgcggacctcctcgtagagcgcgatgtagttgcgggcggtttgcgtcagcgagtggtgtttgaccacccaatcgcgcaccagcttgcggtcgatctcgcgcgcgcggtggatcgccgcggccaacgagtcgatgtcgtcgggaacggccagggccgccggcgcgcggtgcaacaactcgccgagaccgccgcggtcgaacgctgcaaccggcgtgccgcacgccatcgcctcgaaggcgacgagcccgaacggctcctcccagcgcgggctgaccaccgccaccgagcagctggccaccagctggcgcagctcagcgtgcgacatcgcgcccagccacgtggccacgccgggagcaagccgcggctcaatctcctcgcggaagtagcggtgatcgccgttgcggccggccagcaccagctcgacgccggcggcgcgcgcggcgtccatcgccatgtgcgcgcccttctccggcacgaggcggccgaaccataccgcgcgctcgccacctgggccgggctgccaggtggtgacgttgacgccgttcgggatcacggtcgcggaccgcggcaggtcccaatcggcggcggtggtgtggctgacggcggcaaagtgcccggcgcgcgcacccgcggcggtgatcgcgtcctgcagctcatccacgcgcggggtgtgcagcgtggtcagcatgggcagcggcgcgctggagtgctcgccggggaagatgcgcgggttcaggctgttgttgtgcacgacgtcgtagtcgcgccgcgccaacagctcgcgcagctgcgtgaacgcttcgtcctcgcgctctttgccaccctcgggataggtggtgtccgtcgcgtcgtcggccgcatcgccccagtccacgccgggcagctccaagccggtgtcgttgccgtcggagccggcggcggcgaagaagtcgacctcgtggccgagctgccgcaacgcacgcaccatggtgaggcagaacgcctcgagcccgccggcaaacggctcgcgcactgggtaacgggccggcccgataaacgcgatgcgcactctacctcctcactgtttggtcgatcactgctcggtatatctccgcgtgggcgtcgcggacctgcgaaagttgggcgcggcggtcggtggtcaagggcaccgcgccgcgctcaagcagggttttggaagcattgcttgcttgcgccccgtcgcctaccccgtacacctcaacggcattaggggtgtccacttggtccgcgtagcacccgatgtccgggaccgcgacgtttgtgccctggtcccggcacatctccaaccacccggagtgggtgccgcgggtgtacggcagtacgcacacagttgcgcgggcgacagccgcgtgcagctcggcgtcgctcatcggctcgtgcacgtggagggcaaggtcggcgccgcccggcgcgtccgcgagtgcgcggcgcagcgtagctgtggcgtcgacgtcgtggacgtagacgcccagcggcacgttacgtgcgatctcggtgtagaacgccgggtcggcgaccacgttgccgcgcagcgacttcacaaacaccgcggcgcggggctcgcgcgggacgtcgacaggctcggcgatctgggggtgcggcagcacccgcacgccggccgcgccgaagcgctcgcgcaacatgcgcgcggcgtggtcggtgagcgtgatgacggccgcggcggcgctgacaagcacctgcaaccgctcgtggtgctcgcgctggtcggccaagtgggggttgtcgatgtcgtgcaccgtcaccaccagcggcacgggcagcgccgcgaccgtcttacgcagctcgtctggcgagacgtgctcgaagccgaagtggatgtgcaccaggtcaacctgcggggggttcgcccagtagtcggcgcgcagtgcggggtggggccaccagcggccttccccgtcgacgtccgggtccggaacatactccacaccggcaggcaaaacagcctgcgtgtaggggtgttctgccgggatcgcgaggacccgcacggcgcgctggtcggttgtcaccccactaatataatcgttttcgcattaatcacgggctcccaggaggtccacccccaccatggccacgctcaccgtcgtcggcaactgccaagcagagtccacgcgccgcttgctgatgtccacaggagaattcgaatcggagcgcatcaagcccgtccacgagctcgagcaagacgacatgggctggttcaccgagctgctcgctagcaccgacgtgctggtcacccagccgatccgcgacgattaccggggattgcccgtgggcacgcgccaaatgcgcgagcatttaaggcgctctgcccgccacatcacggtgccggtactgcgtttcgacggtctgatgccgtaccacgccatcatccgcaaccccgccaacatgtcggagaacccgccggttgttccctaccacgacctgcgcatcctcgccgccgctgcgaggggtagagacgcgcccgttgaggctgacccagaccatgtcgcgctgcgccgcgccgccgccatgtcgatcgagcagatgcgcgtgcgcgagcgcgcctacggcaccgtggtcgtctccgactacttggaaaccaccccggtgtggcacaccatcaaccacccgaacaacgccacgctcgcgcacatggcgcagcagattctcgccgcgctcggcagcaccgcgcagccacagatgcctggttatgagatgttgggggccttgcaggggcccgtcgataggcaagctgccctcgcgcttggtgtggaggtgcgccgcggcgagtggaccgaccggacgctgggcgtgatcgaccagcagttgatcaccgaggggcacttcgactactaccgctcgcggccggacgtggtcgcgcacgggctgaaacgccacgcggagcgccttgaaaacctagggttgatgccgtgaaacacctgattatcgggcctgacggccacggcgtgaccgactacgccctcaaactcgcggcggcgtgcggcgccgagaccatccgcgaagagcggttcagcggcgccgaactgccggacgaacccatccacgtcgcgttcaccgacaacctctgcgacaccgacgcgctgattgagcgggtgggcgcgcgcccgctgtccgtgagcttccacgacgtccctcagccggaagaaggtaaagcccgctacgcgcgccgcgccgccgcgtaccggcgcttagccgacgccgcgcagctgaacgccacgaactccaaccacgaggcgcggtttttcggcggcgacgccgccgtgatccggctgccgattccggtaattgattcgccgttcgcgccggaagccggcaccgtcggcgtgctcggcttcctctaccccggcaagggccacgaggacgtgatcgaggcgcttgcaggcacgaactggcgcatgcgctttctcggcgcggtctccgacggccacgaggaatgggctgcgggacttgcccgccacgcggagatcaccggctggctcaccgacgagcagatggcggttgagatgggccgcatcgccgtgccggtgtgcgcgcaccggcacttctcggcgtcggggtcgatgatggcgtggctcggcgccggccgcacaatcctcgcgcgcgactccgactacgcccgcgaaatcgacgattggctgccggggcgcattcagcttgtcgacggcccgtggcgccccgcaatcaaagacttcgagccgcgcgtcgtcgacccgccggcgtacgggtgggcggacgtggcgcgcgcgtgggaggacgcatggacttcagctggccttgtgtaagcgtggtgatcccgcactacaactcgcccgagtcgttggcgcgggtggttgacgcagtgcgtgcgcaggactacgcgggtgaagtcgagatcatcatcgccgacgacggttccgcggagacgccgcgcatcgacggcaccaccaccgtcacccagcccgatctgggtttccgcgccgccgccgcccgcaacctgggcgccgaggcagcccgcggcgaggtgctcgcgtttttagacgccgacacggtgcccgagacgggctacctttcggcggtggtgccgcacgtggtgggcgactaccgcgccgtggtcgtgggcacgcggctgacgggatcgcagcggcgcgaaccgcagtggcttgcagacgcctgggagcgcaccaacgacctccgcgacgcagaccacacctcgtggcgcttcatcatttccgccgtgctgacgtgctccgccgagttctttaaccaggtcggtggcttcgacggcacgttcgtcggatacggcggcgaggactgggagttcgggtggcgcgcgtggaacgccggcgcaacgtttatccacgaaccggctgcggtggccatccaccccgaggaggatttcggcgggcgtttcgacgacgccgataaagccgcgcgcgtgaaaaacgccgagtcgctggcgttggcgcgccgcatcacccacccgctcgcccgccccgagcacgtcttgttcaaaaacttcgacatcgccgtcaccgtgccgctgctggacggcgagggcgtggccgaattcgtcatcgccgaatgggtgaaggtcggcgcgtacgtgcacgtcgccgacgtgccggaactctttaacgccgacccccgggtgggcaccgagccccgtgacgcccgcgtgcacgtcgctatcggcgcaggctgggcaccgcaagatctggacgcgctgctcgccgtcgagcacgtgctgctaaccgacggcaccgtgatccgcacggcgcgcgcgaaagcgctgcagctcgagcccgtcaacgcctcccctgaggactgcgggctcaccccgattaccggcccgctgcagctcgagcgctacttcgccggctggtaattacctcgcggcggggatttccggtgccacaccggtgcgctcgtagtcggcgaggatgtcgatgcggcgctggtggcgctcctcctcgctccacggctgggtaacaaacgcgtcgacgatagcgagcgtttcctcctcggtgtgcatgcgccctccgatgccgatcagctgcgcgttgttgtgctcgcgcgccagcttcgcggtctccaccgaccacgcgagcgcgcagcgcgcgcccttgaccttgttcgccgcgatctgctcgccgttgccggagccgcccagcacgatgcccagcgaccccgggtcggcgaccacggcttcagcggctgcgatgcagtacgccgggtaatcgtcggccgcatcgtactcgagcgcgccgcagtcagtcacctcgaaccctttggcctcgaggtgggctttgatctggttcttccgctcgaaaccggcgtggtctgctccaaggtaaatacgcatgtccctaccctacctgcgggtcctcggtgcgcgaacgcttcagctcgaagaagtaggggaaggaggcgagttgcacggatgcgtcgaaaagctgccctgcctcctcgccctccggaacgcgcgtgatcaccggaccgaaaaacgccgtgtcgccgaacttgatcaccggggtgcccacgtcgtcgcccacggcctccatagcctgcgcgtggtagccgcgcagcaggtcgtcctcggtgtcggtgttggcagcctcagcgaacgacgccggcaagcccaccttctccagcgcagccgcgatgatctcgtcgtaggcgccgtagcctctcttgccgccctcgccgcccgggtggaccatggtgcccatcgcggtgtagagctggtcgaccttctcgggcgcctcggacttcaccttggcgaagacgcgcgcagggccccagttcgccttcatcatttcgcggtaggcctcggggagttcatcgcggccgtcgttaagaaccgcaagcgacatgggaacccactccaccgtgacgtcgcggactttctccacttccttcatccagcgggaagtctgccagcaaaacgggcaggacacatcgaaataaaacgtcacgttctcgctcatgggccccactgtagagaacttgtaacgtggtgcgcatgaaaacgaacctgacgcgcgacgccgcgcaacaccgcaaagcactgattgacaacgtgacctaccgcatcgaggtcgacgtcacgggcgcggagcagttcacctccaccaccaccatcgagttcgactccggcgaaggcgaaaccttcttcgatctggtggccgacgagttctccgcaacgctcgacggtgagccgctggagggcagggagctttcgcttaccgacgcccaccacaccgtccaagtccacgccaaagagacctataaccgcaccggcgaggggctgcacaagttcactgacccggtcgacgggaaggactacctctacacgcagttcgagcccgcgatggcgatgaaggtcttcgcctgcttcgaccagccggacctgaaggcgacgtacgacatcgccgtgacggcgccggagcgctacacggtggtgctgaacgaggcggccgagcgccgcggcaacggcgacggcaccgcgacgtggaccacacgcatcgacacgccgctgtcgacgtatttgatcgcgatcatcgccggcgagtacgagcaggtgcgcgacacctacaccacgggcgaccgcaccatcgacctaggcatttacgcccgctccagcgtgatcgagcacctggacgccgagcgcatcttccgccagacgaaggacggcttcgacttttaccacgccaacttcggccggacgtacccgttcggcgacaagtacgaccagatcttctgccccgagtacaacatgggcgcgatggagcacgtcggcgcggtgacgtaccgcgacgagtacgtcttctcttccgaaccgacgccgtaccgcctcgagcggcgcaacgacacgatcctgcacgagatggcgcacatgtggttcggcgacctggtcaccatgcagtggtgggacgacctgtggctgaacgagtccttcgccacctggtcggcagccacggcgcagaccggcatcggcgagtacccggaggcttggaccacgttcgccgcggtggagaaagcgtgggcgtactcccaggaccagctgccgtccacccacccgatcgcggcggacgcgccggacatcgagacggcggagcagaacttcgacggcatcacctacgccaagggcgcctccgtgctcaagcagctgcaggcgtacgtgggctacgaggagttcttcgccggcgtgcgcacccacttcgacaaccacgcgtacggcaacgcaaccttcgccgaccttttgggcgcgctggaggaggcctcagggcgcgacttgtcgcagtgggctgaacagtggctgcgcaccaccggcgtgtccacgctgcgccccgagatcggcgagacgttcgcggtggtgcaggaagacccacgcccgcaccgcgtgcgcgtggggctgtattcgcttatcgacggccgcgtcacccgcacccaccaaaccgaagtcgaccttacgggcacgcgcaccgagatccccgagttcgctggcgtggagcacgacctggccctggtcaacgacgacgacctcacctactgcctgatggagctcggcccggagcagcagcagttcgcggtcgagtacctgggcgcaatcgacgactcgttggcgcgcaccctggtgtggtcctcgctgtgggaggccgcccgcggcggccggctgcccgcgcgcgagttcgtccgcctggtggcgaagttcggcgcggcagagtcgcacccgagcgtgcaggagcgcctcctgtcgcaggcgacgctggcagtgcgcagctacgtcgacccggcctggcgcggcgagggcatggacctgctcaacgctgcgttccggggcgctgagcctgcggcggtgttcgaccgcgccctggcgcgcctgaccccgacggaggagaccaccgcgtacttcaaggagctgctggagcgctccgacaaccgcgaagtgcgctggctggcgctgaccaacctgatcgcctccggcgcgctgccgctgagcgcagccgacgaggaggacgacgactccaacgagggcgcaatttcgcgccttcgcgcacgcgctgccgtggacaagcgctgggcgtgggacaagctggtgagcgacgacctgaccaacctcgaggcccgcttcctcatggacggtctcaccttcaccctcgacgggttggaggggctgaccgacgagtacttccgcgccgcgccggcgctgtgggaccgcctcaccaacgagatggcgcagcgcacgcttgagggcatgtacccctcgtgggatgtggacgagcaggctatcggcaaagccgacgcgctgctgaacgacgggaaagccccggccggcctgaagcgggtcgtgtcagagggccaggaccgcgcggcgcgtgcgctgcgcaaccagcaggtcgacgcagcgagcgctgctggcgctgaaaactaagcgccggtgacggcgcgcagctgcgccgcatcaggccgcagggtgatcagcgtgtactcggccagctgatcgcccgcgtagctgctgcgcgacaccttctgcaccaccgctcccctggccagccccagcgcctcgcactcgcggtcggtggcccgcgttgcggtgagaatgtcctcgcgccgcacgggagcgttacctgcggcctcgggcccgccgggcaaggtgtacgcggcggcgaaaagcaccggctggccgtcggaggcgtagatcacctcgcgctcgaagacttctgtaccggcagggatgtcaaacgcggcggcgacgacggacggcgcgggcactgccgtcgtctgcgtcgagacaacctctgcgccgctgagggcgaagtgttcctcgaaacctgcgaccgaggtcagctcgagcgagggcggggtggcgcgcacaaacgttccgccggtgcggccgcggcggcgctcaatcaacccttcgtcctgcagcatgtcgagggcgtggcgcacggtcatgcgggccacgccgaagcggtcgacgagctcgcgctccgacggcaggcgcgccccagccggcaattcctgcgagacgatctgctcccgcagctcgtcaccgatcaccatgtacgcgggctttttcgccacctaccgcctccttcaaacgcaccgtcgacgctagtgagactacagcgcgcgcaacgccttctcgagatcggcaagcaagtccgcctcgtcctcaataccgacggaaatgcgcaccagctcaggcggcacctcgagggcggagccggccaccgacacgtgcgtcatggtcgccgggtgctccaccaagctctccaccccgcccagcgattccgcgaggcagaacagcttggtggacaagcagaatttcttcgcctgctcctccgtgttgaattcgacggagaccatgccgccgaaacggcgcatctggcgcttggcaacctcgtggcccgggtgcgattccagccccgggtaatgcacgcgcgcgacttgatcttgttcgctgaggtagttggcaacagcctccgcgttgtcgcagtggcgctccatgcgcaccggcagggtcttcagcccgcggcccgtgaggtaggtgtcgaacggcgaagggatagcgccgacccagccgaagaagaagcgcaggttctcctccaggtcgccgatcaactcgtgcttaccgcacaccacgcccccgaccacgtccgagtggccgccgatgtacttcgtggtggagtgcagcactacgtccgcgccgaactcgaacgggcgctgcaggtacggcgaggcgaatgtgttgtccaccaccagcttcgcgtcgcccttgatgcgggacaccgcctcgatgtccacgatggacagaagcgggttggtcggcgtctccacccagatcaccttggtgttgggctttacagccgcggcgacagcgtccacatccgtcatgtccaccacggtgttctccacgccccactgggtgaagatctgctggatcaagcggtaggttccgccgtaggcgtcgttgctgatcacgatgtggtcgcccggtttcagcagcacgcgcagcaccacgtccaccgctgccatgccggacgcgaacgcgacggcgaagtccgcgccctccagcgccgcgatcgtcttctccagcgcagtaatcgtcgggttgcccacgcgggtgtactcgtagccgccgcgcagctgcgccagcccgttctgtgcgaacgtggtcgaggcgtagatcggcgtgttgattgggccgtacaggctatccggctcgtagcccgcgtggatggaatcggtcgagggtccaagaggtgaggattgcatggtttggatggtagaccacccactagaccaagctgtccacttgggtcgacttttatccaaccgcgtacacttaccgtcgatgaacgagaacctggaaacctccgtcgacaccaccgttgacgacgtcacctcgtggtggaacgacccggcgacccacgagatgcttgtggagaagccgctgaagatactgctcattctgctcgtggcactggtgctgaactggctcgcggtgcgcattatccgccgggccacgcagcgcgctatcgagacacccgcaatactgcgcgaatcgggctcagacaagaactctccgcaggcccgcgcccaggaaaaccgccggcagcagcggatgcgcacgctggcgaatgtgggccgctcgatcgcggcgatcattatctggacctgggcggtgctggcgattctggaccagctcggtgtcaacgtcgcgccgctgatcgcttctgccggggtggtcggcgtcgccattggtttcggcgcgcagtcactggtcaaggacttcttcagcggcatcttcatcctgctggagaaccagtacggtgtcggggacacgattcaggttggcgacgtggtcggcgaggttgaggagatgacccttcgcatcaccacgatccgcgacatggacggcgcgctgtggtacatccgcaacggcgacatcgaccgggtgggcaaccactcgatccagttctcggtcgcgcgcctgcagatcccggtctcgctcatggcgaacccggataaggtctcgcgcgtggtggaggacgcctgcaccgccgcgatccacgacccggaggttaaagacctggtcatggcggcgccgcagatgctcggcccgtccgacttcaacccgaactacgtgtcgttccgcgtcacggtgaagaccatgccgggcgcgcagtgggcggttgcccgccacctgcaccaccgcgtgctggtcgcgctgcacaaggaagatgtcgtactcgcgccgatggattcgatcctggtggagttcgcagataaggacagcaacaatgaacgagcctaaggagcagtcgctttacgacgccctcggacactccttcttcacccgcctcgtttccggtttctacgagcaggtgaaaaccgacgacctgatcggcccgatgtacccggaggacgactttgcgggcgcagaggaccggctgcgctggttcttggagcagtactggggcgggccgcgcacctaccaggagcagcgcggcaacccgatgctgcgccggcgccacttccccttcgccatcggcgcggcggaggctgaccgctggctggagctgatgagcgcctcgctcgaccagttcagcgaagacgaactcagcgccgaacaccgcgcggtgctgtggaaccacatgcagcgcgtggcgttcatgatgatcaaccaataagcaggttcagccccgcgttccggaagattgagccgtaggccgcgtcgaggcgcgtccacgagccgcaggtggagatgcgcatctgccgcgggatattcgccggtgcatcgaatccggggatcagccccagcgaggtcgccgcgaagatcatgctcatcggcacctcgacggggttggatgattcggcgtcagcggtgatcacggtgttgctgagcagggagcgcggcggacctgcgggcccggagaactgccgggcgagcgccctaccctcgtccgccaacttgcgcaccgtggcaatcggcacggtgtcccgcaaaacgaagccgtcgaccgggggaagtgccccgggccacgcgcttgccgggagggggtttggggtgttcgggagcgcgtcgataagcaactgcccctgaaacaccccttcctccagcgctgtgctgcgccgggctgccgcgcaatcgaatggggtggtgacgaagacgttcgacgcgtcggcgccgaccgcctggaccctcgctaccgcgcccgcgtcgagggcgaccgcgcggcgcaggagggtgagaagtccgcggtcgctactcaacgttactggccgcagtctgcgaaagaatcccgatttctttctgcgtgatctcgcgcggcgtggtcgtcgcgttgtcgattgtcacttggacgcactcgatggtgcagcagacgcggccctgggagtccttcacttcctgacgggtagtgaaggaggtggtgccgaggttgaccacctgcgtttccacgcgggcgaggaccgtgttcggcaacagcggtcggacgtaatccgcctcaatgcggcgcacgaacgagacgaactcgtggccctgcgagtagaagaactcgttggcaaaagccaggcgcgcctcctgggcgatctcgatgtacgcggagttggtcacgtgcccgtagcggtcgaagtcgctccaccgaagcgggatgttgtggacgtggacgttgcctgcgttgccgttgtcggccatggagatcacaccttttgcgtttgacgaccgttactcattcgcgatgctaccccgccctcaggcggggtgcccgcgtgttagcgggtgagcttgcggtgggtcacgcgcgacggcttcgccgcctcttcgcccaggcgctcaaccttgttgcgctcgtaatcgccgaagttgccctcgaaccagaaccacttgccctcctcgatgttgccttcccaggcgaggatgtgggtgcaggtgcggtccaggaaccagcggtcgtgcgagatcaccacggcgcagcccgggaacttctgcagcgcgttctccagcgagcccagggtttcgacgtcgaggtcgttggtcggctcatcgagcaggatcaggttgccgccctgcttcagcgtcagcgccaggttcaggcggttgcgctcaccaccggagagcaccttcgacggcttctgctggtccggacccttgaagccgaacgcggacaggtaggcgcgcgacggcatctcattctggccgacgtgaatgtagtcgagtccgtccgagacgacctcccacacggtcttctccgggtcgatgttttcgcggttctggtccacgtacgagatctgcacggtctcgccgacctcgaccttgccgtcgtccggctcctcgaagccgacgatcgtcttgaacagggtcgacttacccacaccgttcgggccgatgacaccgacgatgccgtttcgcggtagcgtgaacgacaggtccttgatcagcacgcggccgtcgaagcccttgtccaggtcctcgacttcgacgaccttgttgcccaggcgcggcggggtcgggatctggatttcctcgaagtccagcttcctgtactgctccgcctcggctgccatctcctcgtagcgctccagacgcgccttgttcttcgcctggcgggccttcggcgaggaccgcacccactcgagctcgttcttcagccgcttctgcagcttctgatccttcttgccggcaacttcgaggcgctcagccttcttctccaggtaggtggagtagttgccttcgtacgggtaaagcttgccgcgatcaacctcgcagatccactccgcgacgttgtccaggaagtaacggtcgtgggtgatggcgagcacggcacccgggtaggtctgcaggtgcttctccagccacaggacgctctccgcgtcgaggtggttggtgggctcgtcgagcagcaaaaggtccggctcggacagcagcagcttcgccagcgcgacgcggcggcgctcaccgccagagaggttagtcaccggggaatcggacggcgggcagcgcagcgcctccatcgcctgctcgatcttggagtcgacctcccacgcgtcggcggcgtcgagctcctcctgcagcttgcccatctcctccatcagctcgtcggagtagttggttgccatctcctcggcgatttcctcgaagcgctgcttcttggcgaagatgtcgccgaggccctcctcgacgttctcgcgcaccgtcttctcctcgttcagcggcggctcctggagcaggatgcccacggtcgcaccgggttggaggaacgcctcgccgttattcggctggtcgatgcctgccatgatcttgagcaacgacgacttgccggcgccgttggggcccacaacgccgatcttggcgcccgggtaaaaggccatggtgacgttgtccaaaatcaccttgtcaccgatggccctgcgaacatttttcatcgtgtagatgaactcagccacgaaacgtttccccttgttagaaagacttgaaactgcttttcacagggtacattacgtggcctggtgcaccgcgcgctagaacggcgcagcgccctctgagtcaccggccgcggctgggactggctcagcgctgcggccgtcacggccgccgtggccgccgccgtcggcgaagttcggctcggcgccgtcctccgcgctgcggcgcgcctcaggctgctggatgaaatccgcaacggttttcaccgtcatcggcacggtgccgttcgcgttgtgggtgacgttggtggtcttgatggagttgagctggaagttcgacagatcgaaggagacctgggtggccttcagcgcaatcttggagcgcatgttggagtcttggccgagcgccgacttgtcctcccacatttcggtgacaaggcggccggtcaccgtgaccgggaagccgcgcttcagagacgccatgcagttgacggcgagctcgttccagcaggcgacgtcgatgtaaaggtggtcggcgtcctcccagatgtcgcggccattggagtccttgtcgccggtgttgcgccggcgcgaggtggcgaggcggaacttggtcagcgggagctcgtccgctcccgcaacggtcaagacgggatcagaggtgaggttgccggaaatagtgacgatgttgctcatggtggtgcctttcttggggttgatgggggcgtcgataagcaattgcccctaggggcagcgtggcacctgccgccaccccggcaaagcggtaatccccaacccggcgcgaaacgcggaaaacactccacagcttattgaaaacgcgcagcttaactgttgtagcgcgcgagcatctcgttgtactgccgccactgctcatcatccgactcctccgcctggcggtcggcggcctcggactcggcgcggtcactgctcagccactggcggaacagctcggcgaacacgatgaccagcgggaacgagccggttgcccacgcgataccgccgccgaccttctggtcgtcgagcagattcgggttccacggcaactgcagggaggtgtagaactcctcgccgagcaccacgttgagctgcatcaggtacacgcccatgaacaggtgaatcggcatggaaacccagagccaggcgaggcggatgcgcgcgtcggtgcgcggctcgatctcgtccgggccgatgagttcccaaaaatagaagtagccggaggtgaggaacacggcgttcatgatcacgtgccccgcgtgctcagaaatcatcagctcatacagcgggatgaacatgtagagcgcgtagaagaagaagatgaactgcacaaggctgaccggcgggtaggtgatcacgcgcaaaaacgcggagcgctggaagctctcggcccacaaccgcgggttgaactcccccgccgggtacgccgcccgcacgagcgtgagcggcgcgccgagcaccagaaacaccggtgccaccatggacagcgccatgtgcgcgagcatgtgcgcggagtaactcgccggcatgtgcatgccgatgttggacgacagcgtggcaacgaccgtcgcgcaccccgccaaccaccacgcggtgcgcgaggcgcgccagccgtcaacccggcgcgcaaggtgcaggtagtacgcggcaagcaggacggcgatcacgctgaacagcagctcgaagcgccactgcgtgaaccaggtggcgaaggtcagcgggcgctcgaggtcgtagcccatctggatctgcatcgcgctcaagttcacttcgcgcggcgggggcggcggggtgcgcccgagtgtggccgccaacccggtgacggcagccatcactagcacctcgacggcggcgaggcgggtgaatgcccgcggttcggtggcgagcttgggaatcgtgcggcggcggtgcagcgcgccgaaaactccgagtacgaccaagccgatgagcttcgctaccagcacgagaccgtagtcgtagtccagcagctcgttggggcggatgcggatccacgcgttgacgacaccggaaatcaacatgccgaaaaacgcgaacagcgcgatgttggagtagcgcgtcacggcagcctccatgcgggggccgagccggcgcccgtgggcgatgagcgccatcaacgcaccgacccacaccaccatgcacactaggtgccagatgaaggaatttgtgccgtagtcgtggttgccgccggttgcggagtggccggttagcgcaagcggcatcagcgaggtgaccgatccgataagcagcgcaacctgcggccaccacgtcttggaaacgaatccgccgagcgcgaccgcccccgcaaacgccgcgacggtgagccacaccttcgcatcgctgacctgctccagcgcgatcgaccacgagccggcgttgaagaacacctcgccgagcggctggcccgacacgtccgacagcgtcaggggaatcatgatgagcgcaatgagggccatgcttgccgacgcccacgcccccgcccgcgccgccacccacccgtcaaccgtgagcgctgcgttgttcaggtcgtcctcgtacgccgggggaaaaaggaacgacgagaacaaaaacgagcccacggaaagtgctgcgcacatccacgccgcggcgcgcagcgccggcagcccgaacgtggtgggccagcccgggtccgggataccgagcgccgcgagcgactcgcccacgaaactctgcgccaccgccccagcgaccaccgcggccaccaccacggcgacgagatagaacggccacgcgaccctggccggaagcttctgctgcatggcttgcatggctcaaacgatacgttcgcgcgctgcgagtccaccaaacggcgtgcgttacaatgacgcacgcttactttttaagcgcgcctccatagctcagtggattagagcaaccggcttctacccggtgtgtcgcgggttcgagtcctgctgggggcacatttttctccgcgtggtgtagtacgtgcgtacccttgggagacacggtttttacaaaccgacgtatttcgaaggagtacccatgactgacaacactggccgcccgccgaagagcgaagacagcgtcgacgatctcggcgatccagacgcaaccgccaaactgcaggagcagacttctgacgacgagggtgaggagtaaaagaccatgaccaacccgaacagcgaaaccgaccgcctgctcgatgctgccgtgcaccgcatcggcaacgagccggataacggcgagaccttcgacgacttcgaggacgccgaccagaacgcctcccggggcgcaagcgacctcggcaccgacggcgctgacaccccggtgcaggacgagcgctccaccgacggtctcggtgtggaggacactgatcactaagcgggaccagctggcggagctgcgcgcgattgaacgccgcgcggccgacgtccccgtcccgtgggctggtatcgcagcgaccggcgcggcctgcgggttcgtggtggggtccgcgctgatggagctgcccgccgtcaccttcgcggcggtcgtggtgctgctggcaggtgtcgtcgtcctcgagcgcccgggcaagaagaccgtgcgcaccgcgatgaaacaagacgtgcgccccgatcctccgacggactggcgcctcgtggtgtacattctcctgctcaacatcgcgatgcaagcaatgatgcgccgccagccgcacgcgagccttggagtggcaatcgcagcaggtgtggccacggctgtggtgtggactgttttctttggtttgtggtggaagcgggcgaagccgtgaacttcgatgccctgaaaatttgtgcggcgctcaaaggcgccggcgccacggacggcggcgtccgccaagagatgaaacgcagccgcatctcagagctcaccgggctgggcggcgacgcggtggcggcggcgcttactgaactcgaggccgccggccacgtcaccacgtttttcgagtacggatcgcggcccgagaagaacaccgtttgggtcacgctgaccaccacggggctgcaggcgtacaacgcgtacgtggacgggctcgagcggggggcgggtacggttggggtatgagtttcccgcagccgtcgataagcaactatgccctcatcaccggtgcaagccagggcatcggcgaagcgatcgcccgcaaacttgcggcgggcgggcacaacctgatcctcgtggcgcggcgcgaggacgtgctgatgcgcatcgccgatgagctggcgggcaagcatggcatagacgtggaggtgttcgccgctgacctgtcgaagcaacgcgacgtcgatgcgctgcttgagcacattggcagcaagcagatccacatctgcgtgaactctgccggcatagccagcttcgggccgttcatgcaggccgactgggggtacgagaccaaccagttcaacctgaacgcggctgcagtgttccgcatcactaaggccgtgctcgaccagatggtgccgcgcggcgagggggcgctgtgcaacgtcggctccgccgccggcaactcccccatcccgaacaacgccacctacgtcttcaccaaggccggcgtgaacacgttcacggagtcgctgcactacgaactcaagcccacaggcgtgcactgcaccctgctcgcgccggggcccgtgcgcgacgccgacatcgacgaggcgagcaagagcttcattgacaagctcgtgccggatttcctctggacaacctacgaatcctgcgccgaggacacgctgcgcgccatgcgcaagaacaagcgccgcgtggtgccgggccccctgtcgaaggcgatggatgtggtgtccacctacgcgccgcgcggctcgctcgcgcctattctgggcagcttttacgcaaagatgggagaagaacagcatgcctgacgtacccgcacgcgacgaccggattgtctgggtcgacctcgagatgaccgggctcgacccgaagcgccacgtcatcgtggaggtggcggcgctggtcaccgacgcggagctgaacattctggacgagggcatcgacttggtcgtccacgccaccgaggcggagcttgcagagatggacgatttcgtccgcgggatgcactcggagaacgggctgctggccgcaatcagcgagtcgaccgtgagcatcaccgaggccgaggacgctgtcttggagctgatagcgaagcactgcgatcccgcccaccccgcgccgctggccggcaactcgatcgccacggaccgcaccttcatccgcgcgcagatgccgcgcctggacgcggcgctgcactaccgcatgatcgatgtctccaccatcaaggagctttcgcgccgctggttccccaaggcgtatcaaaaccaaccgccgaagggcatggcgcaccgcgcgctggcggacatcgtcgagtcgatccaagagctggactactaccgacgctgcgtgttcacccccgccccaggccccgacgggactgcggcccgtgccgccgctgcagaggcgcacgaagcttacctgccgtttttgtaaacgctgacgcccgtactaaggtagtcggagttgccttacggcagcgatggtggctgtagttcagctggtagagcaccaggttgtgatcctgggtgtcgcgggttcgagtcccgtcagccaccccaaaggctaaggcccggcttgcagttgttgcaggccgggccttactcgttcgggtcctcggatccgcccgaacggcgctcccaatcgaggttccagtaccccagaccgtcgtactgcgtgagcgtgtcgccggccgtgttcttcactatcactgggtcaccgcggcgcacgttgtcctggaaccacttggcgtcctctgtggaggcgttgatgcagccgtgcgagacgttgctggacccgatcgcgccggcggcccacggggccgcgtggacgtaaatgccggagtatgacaactgcgttgcccatttgaccggtgtgacgtagccgcccttgcccaggtcgagtccgaaggtgcgcgaatccatgacaagctcctcgtggcggtcaccgacgacgtaggtaccgtttggggtgtcgtaggtgccgtcgcggcccagagcaatggggaacgacctcaccagctcgccgccccggtacacgctcaaggtcttgtcggcgttatccacgacggtctcgaccgcgtcgccgatggtgaacgagatctccacgtcgtcgccgccccacaagccttcgccgaacttgtgcccgtagatgtcggccgccacggagacctctgtgtgcggctcccagaactccttcgggcgccagcgcagctcgtacgggtcgatccagaagaacccgccctccgtgccgttggaggtggtcaccgtaatcgcctcctccacggccttcgtgtctttcacgggcgtgttgaagcggaatgtaaccgcctgggcgatgccaacggtcgagccgtcaatgggaccgacagcgacggtgagttgctggctcggcacgacggtggtgaacgttgcgctagagctcttgccctcgacgttcttcgcggtaacggtgtaggtgcgtccgtagcccagcggctctgccacctcccacgcggttttgtcgtcgttgaattccgcgtcgatctcgcgcccttgttcgttgaccatggtcacggtttgcagtttgcttgccgacgccaccttcaccccatcccacggccccaccccgctcgcgccgtccctgacagagatggtcgggggcttcgccgccgcggttgtggtagccgcggcggttgcgcttgtggtacttagctccgcttcagcaccagcaacgtggcgctcgcttgcgtcaccgccgcagcctgccagcgccgcgccagccagtacaccggtaagcgctgccgccgtcaccctggtccgcatctgacaccccttcccgtccgcgggcggaatcccgcacaaccaatgcaaccctagttggtggcactcaaaatgagtactctgccgggctggttaaccaaaccgttgcacaacgaaggaaatgtcgtttaaccaggcgatttcacactaaaacaacacgctgctatagtcatatcccgttgcgccattagctcaattggtagagcaactgactcttaatcagtgggttcggggttcgattccctgatggcgcacaggtcgaaggccaagttgattttctcaacttggccttcgttttgtctatacactgttacccatgactcgcgcacttgtgattgttgatgtccagaacgatttctgccccggcggctccctcgcgaccggccgcggcgacgaggtcgcaggcaagatcgcgcatctgctcgatggcgctgaggataactagtcccgcgtgcttgccacccaggactggcacatcgacccgggctcgcacttctcggagaaccccgatttcgtcgactcgtggccagtgcactgcgtggccgatgcggagggctccgcgatgcgagctccgcttgacgacgccccctacgccgggatgatcaccgaatatttccgcaagggcgagtacaccgccgcctactccggcttcgagggtaagaacacggacggcgcgctgctgtcagatttcctccgcgaaaacggcatcgacgcgatcgacgtggtcggtatcgcgaccgaccactgcgtgcgcgccaccgtgctcgacggcgtgaaggagggctttgccgtacgcgtactcgctgacctgtgctcccccgtggacgaggcacgcggccaagcggcgcttgaggagatggccgcggccggcgccgagatcgtgtaacccgctacatgctcggctcgtagccgaggatgtcttccatctcagccatttccgcggtctgaacgtcgatcatctcgcgggccatatcctttaagggctcgtaagccccgccgtcgacctcgccctgcgtcatgtcgatcacgtgggcgtggtggaagtgcatccactcgaggaacgtggtgcgcagctgatcgcctttgagcgcgcggaactggtctagctgctcgggatggaacatgccgttggcaatgtgcttcgagtgccgctccatgtcctcgtcgatgccccactcgtcggcccatgcgcgcatctggtcgttttcgcgctcttggccgtccttgatgcgctgggccagatcgcggacgtgctcgtcgtcgacgtcggaggccaaaaggacgtccgacatctcgatcgcctgctcgtggtgcggcaccatcatgccgaggaagtgaacgtcgaagtcgttgtactcgtctgaagcggccgtgtcggagccgccgaggcgcgggatgagcagggcggccagaagcaccaccaccgcgacaacggcgagtccagcgacgaggggtcggcgggacggctgagcgggttgcagatcagaattggtcatacctacatccaagcataaaaaaaccgcctggccagtcgatccagtcaggcggtgagcaaccccacagtcggggttaaccgtttagcggcgggaaagcaggcgctgcagctccttgagctccttcttgcgcttgcggccgttaaggaacttgataccggcaagagccgctacacctgccgcaatgccgccgagcaccttctgcacggtctcgtcctgcagccacgacgcggcctggtccttcgcgttgtccgcgaggttggacgggttggtgcgatccgccagctcatcaagggtgcttgcgagctgggagcgggtgcgggcgaggtcgcgctcgatgtcgttgatgtctcgtgccacgataaaactcctactaatcaaagcttgtcagtacttgcaaccacactaatcgaaaaccatgtacaacggatgcatgacgaacgacaaccgccttgcccccggcgacaccgcgccggccttttcgctgaccgacgaccgcggtgagaccgtctcgctggcggactttttcggccagcgcgtgatcgtctacttctacccgaaggcgaacaccccgggttgcaccaccgaagcctgcgacttcacggaaaagttccccgagttcgacagcgcgggcgtcaaggtgctcgggatctccctcgatacacccgaggcgcttgcgaagttccgcagcgaccacgacctgcatattgagctgctctccgatccgtcgaaggacgttctgcgcgaatggggcgcgttcggggagaagaagaactacggcaaggttgtcgagggcgttatccgctccacgttcctcgtcagcggcgagggcatcatcgagcaggcacagtacaacgtccgcgcgtccggccacgtcgatcgcattctgcgcgactggggcatctagctcgaatatctctagaagtggtgcgcccggagagacttgaactctcacgccctaaggcactggaacctaaatccagcgcgtctgccaattccgccacgggcgcagtgctacaacactctacacacagggaagcctaaaactttagtttggctgcacagagtgcgggggtatggtttgaagacgtgagtgacacgcgtgcaacgaccgagacgcagacgccgccgaagcgccagcgaattagggtgcgcgcgtggcacatcttgctcctcatcgctgcggtgatcaccaccttgttgctggcacggtggcagtggcagcgctaccagtccggcaccggcacgttccaaaacttgggctacgcgctgcagtggccattctttggcgctttcttcgtctacgcctaccgcatggggctgaggatggagaacgagaagattgacgcgatcaactcgggcgaggcaatggacgacctgtacgaggcggacttgcgaaagtttggcaaggacggcgaagaactcaaaacgaaaatcgacgaagacttcctgcctgcccgcccccaggtggacgtcgaggagtacaacgagatgctgacgcccaaacgtcagcgcccgaaacaaggagaacgcgagctatgacagaaccgcagccgacagcaccccgcatccaccccgagcgccagcgacgcgtgcgcaccgcgctgaaaatcttttccgtcgccgcgtgggtgaccggtgtgctgctgcttctgctggtgctgcgcatggtgctggagtacggcttcggcatggacgtctcggcgcttggatgggtcgctcgcgtgcacggcttggcctacatcgcgttcctcatggcatcgctgaacctcggcaccaccgctcgctggccggcgtcgacgtgggtcatcaccgccatctccggcgtggtgccgtttctttccttcgtcgtggaggcgaagcggcgcaaggaagttagccggacgttccagctgtagcggcaagcgccgcgatcgccggcgcgagcgcgcgcaacgcctgccccctgtgggagcgggcattttttgcctccgcggaaagttcggcggaggactgccccggcgcgtccgcgggggcaaaaatcgggtcgtacccgaagccgtgctcgccgcggggttgacgcagcagctcgccctcccagcggccctcgacggtggtctcctcgccggccggtgtgaccagggcgcagcacgagacgaaggcggccgcacggtggtcgatgtcggccatctggttcaacagcagccggttgttggcctcgtcgtcaccgtgggcgcctgaccacctcgcggacaagatgccaggcatcccgttcaacgcctcgacggtgagtccggagtcgtcggcaacgcaggcgagacccgtggccgctacgccggcacgggccttgatcagggcgttctcggcgaaggtgagtccggtttcggcgggttcggggtatgaggggacgtcggcaagcgaaacaagctctataccgccgatctcctgctgcttaagcacctgctctaactcccgaagcttcttcgggtttcccgacgcgacgagcattttcacagcccgagcgcctccttctgcgcggcgatgagctgggtgcagcccttctcggcaacgtcgagcatctccgcgagctgcgcgcggccgaacagcccgtgctcgccggtgccctggatctcgacgaagttgccgccctcctgcatcaccacgttcaagtccacctcggcggcagaatcttcgacgtagggcaggtcgaggaccacgcggccgtcgacaatccctgcggacaccgcggcaaccggggcgagcagcggctcgccggggaccaccccgcgctccttcagcacggtgatcgcgtccgcgagcgccacgtaggcaccagtgatggaggcggtacgggtgccgccgtcggcctgaaggacgtcgcagtcgatctggatcgtgttctcgcccagctggcttaagtccaccgcagcgcgcagcgagcggcccaccagccgcgagatctcgtgggtgcggcccttgaccttgcccttcatcgactcgcgcggcatgcgttcgtgcgtggccgacggcagcatcgagtactcggcagtcagccagccctcgcccgaatccttcttaaagcggggcacgcccacctccacactcgcggtgcacatgacgcgcgtctggccgaactcgattaagacactgccggccgggtgggaggtgaagccgcgggtgatgcgcaccgggcgcatctcgtcgaacgcgcggccgtcgaaacgggtaaacgttgctggttcagtcatgcccccaagcgtacttggcgctacagcgtgaagacgtcgcccgcatcccccacgacaacctcgccgccgaactccgcggccgcggcctggcgggtcgcttccttgtccgtccacggctggatgtgcaccagcacgagcttttccacccccgcctcgcgggcgacgcggccagcctcttcgccggacaggtgcatgccgctggggcggccgtcggcaattgggccccacgcggcctcgcagaacagaagagaagcacctcgtgccgcctcgatcaacgacggggtgaacccggtatcgccggagtacgtggccaccttgccggtcgccttgtcttcaacgcgcagcgcgcacgcctccacggccgggtggtccaccaaaaacggggtgatggtcacaccctcaaacacggcgggctcacccggcgtccaggaggtgaactcgaacgtgtctgagatatccgtcggatcgctcgggccgtcggcgcccatcagcgccaggtgctcggcggtgtagctcgggcccataaggcggtggcgctcatgcgccggcgcaaccgggtggtagcggcgccacaccagaagcgacgcggcgtcagagcagtgatcggcgtgcaggtgggagaagacgacgtgcgccgccgacggatcgaacccgtgctcctgcatcgcagcgagcgcgccgggaccgaaatccatcaccacgtccgggttgccgtctgtggaaaccacgtaggacgatccggggttgccaggcgcacccacacttccggagcatccgaggatggtcagcttcatggacctactgtgccacggatgcccacggcgtgcactcttggccccacgatccgctccgccagcgcgtcgaacatcactgggtcgcccgtggactcgaacgtgcgcgtcggtgcttcgcggcccggcgcgcccgcaggcgcggcgagtaagtcgagctcggtgagcacgcgcagcacgtccttggatgtctcctcagcggagttgaccagggtgacgtgctcgccgatagccagctggatcacgcctgaaagcagcgggtagtgggtgcagccgagcacgagggtgtccacgccggcggcctgcagcggctcgaggtagccctgcgcgacgcccaagacctgccggcccgaggtcaccccgcgctcgacgaactccacgaacgcggggcacgcggcagcggtgacctcaacgttcgggttgagtgcgaacaggtcttggtagacgccggaggtgatcgtgccttgggtgccgatgaccccgatcttgccgttgcgggtggtggccatcgcgcggcgcacggcgggctggattacctcgatgacggggattgagtagcgctcgcgggcgtcgtgaagaaaagctgccgtggccgtgttgcacgcgatcaccagcatcttgcacccgcgttcaaccagctcgtcggcgatgcgctgcgcgtgcgagcgcaccgtggcgatcggctgcggcccgtacggtgcgtgggcggtgtcgccgatgtacatgattgactcctccggcaactggtccatcacggcgcgggcgacagttaacccgcccacaccggaatcgaagatgccgatgggggcgttgttgacggcgccgaccgggctcaccatccctgcgtccgccgcgtcagctgatccagctcgttttgcgccatccgcttctccaggtccttctgctggcgcttcgccaccagcgcaggcgggtcgtcggaggtgatcaccatcgcggccacggcgccgccgatcgcgccgaacatgtgtgcctgccagctcacacccgcgtcgcccgggaacatgccccacaccaggctggagtagaagaaaccgaggacgaggcccaggatgatttggcggccagagcggttgaaaaagccgcgcaccaccaggtacgcccaccagccgtacaccaatccggaggcaccgatgtggttggtgccgatcccgccgaagacccaggtgcccaagcccccgatgagcaccacgaacgtggagacctcccagaacacacgcttgcccgaataccccaccaggtacgcaaacacagcgccggcgacggtgttgcccaggatgtgctcgaggttggcgtgcagaagcggcgaggtgaagatgaacggcagcgacgacacatccagcgggtggatgcccaagtagttcaggttcccgccgaacacgagcgcgttaaggaggaacacggcccagatcgccacgacgtagaggaccacgaaacgccagccggagcggcgctgcgcctggcgcttggccttccgcgcctgcagctgctgctgcgcggggttcaccggttgcgggctgggcagcggcgcgaacgccggttgctgggtctccgggtgggaaaatggccgctggaacggcttgccgtagccgggctggccggtatcgccgtaaccccacccggccggcgggtagtactggttgttcgtcatcgaggctaaagcttagcccgcgatgtcgcaccacgctgtcgcgccgtgggcggtgcgggcagtcaccaccgcgttcactattgccgcttgcacgcagcctgcggctgcttcaccgagcattgtttgcttgtcgacgcccccctcaaacttcccttcccccaccgagacagcgaacaacgtgtctccgtccagcggcgaatgcgccgggcgcacggcacgcgcgatgccgtcgtggccggtcatcgccagccgcttcaactgagctttgttcagcggcgcgtcggtggcgatcaccccgatggtggtgttcagcttcggggtggggcgcgtcagcgaccggaacgcctcgaggtccaccgccgggtaagacgcgtcgccgtacagcttccccgagaccgggtcgatgacagagccgacagggttggccacgacgtacgcccacaccgtgtactgcccgatgtgggcgtgcgcgctgccgaagccgccgcgcagcacacccgcggtcgccccgcagccggcgccgacgctgccggtttccggctccgcgccgtcagacgcaaacgccgcacgaatggcagccgccccgtcgtccgggcccggccggtggtgggggtcgccgacggcgaggtcaaagatcacggcagccggtacgatcggcacaatgggcccgccgggcagctcgtcgccgaagactttgaagcccgccccgcgctgctccagctcggccatcgcgccgtcggcggcggcgaggccgaacgctgagccgccgcacaaaagaaccgcgttgatccgctccaccgtgttgtggggctccaaaagatcagtctcgcgcgtgcccggcccgccgccgcgcacgtccacggccgcggccatacccgctgggtcctccgccaccagcgcggtgacgccagtgtcgccgagggaggtgtgccctacaagaaggttcacggctctacccatcatcaatccatcatggcctgcagcagcgaatcctggcagaacgccagccagtccaaaagcatcgcgcggttttcctgcgcagcttcgccgccggaggtgtcttccgagacgtagaggcgcatgtcgttgagggccgcgacaaaccgcggcgcgtcgtcctgctcgattgttacctccaccccgccggtggggccgagcacctcgttgaccacctgcaggttctgcagcttggccttgatgatgtcgttctcgtgcaagctgcgcaacagcccgttgtcgccgtcgaactcctcgtcgccctcgcgctcaaaatcgggcaaaaggcgcgccatacgcgggtcctgcggcgcctcggtgtggccggaggagacaccgagcatctcggcgaactcgtccttcggcgcggactgggcgcgcgcgatcagcgcttccgagaccgttgctgtcaggtcgccgatcagctcgcgttcaatcggttcgaaccgagtcgagtactttacgcccgagcgcatcaagccctttttgcgccgccactgctccatctttgtctcccgccccgctttcgctacccggcctgctgcatcgtggcccacaacccgtgggtgtgcagtttcttcacgtcgccttcgaccttgtctttctcaccggaggacacaaccgccttgccctccgtgtgcacctgcatcatcagctcgttcgcgcgcttgcggtcgtagcccagcaccgtctggaagacgtaggccacgtagctcatgaggttgaccgggtcgtcccagacgatgcacatccacggcagattctcgctcgtggcgacatcaacctcgatcgcctcgtccaaatcgggcgacgccatcggcgagcccatccgcgggtgcattgcattcatgcgccccacattacccgaggtgtgctggagctctcagccgcgaagccgggtagccttacacaccatgaacgatcagacggcaaaggcgcccgcgcgggtgagcgactcgcgcaccagcggctgctccgaatccaccgcctttttcactgatatgtacgagctgaccatgctcgacgctgcgatccaggagggcaccgcgttccggcagtgcgcgttcgaagtcttcacgcgccgcctgccggtggagcgccgctacggcgtggtcgccggcaccgcgcgcgtgatcgacgcgatctcgaacttccgcttcaccgaggagcagatcaaaaccgcgccgttcctctcggacgcggcgaaggactacctgcgcaactaccgcttcaccggcagcgtcgaaggctaccgcgagggcgacatctacttcccctattccccaatcctcaccgtccacggcacgtttgcggagtgcgtcgtgctggagacggtaatcttgtccatcttcaactccgactcggctgtcgcctccgccgcctcccgcatggtctcggctgccgacggccgcccgatcatcgagatgggctcgcgccgcacccacgagcacgcagctgtgaccgcggcgcgcgcggcctacatcgccggcttcgacgcgacctcgaacatggaggcgtccctgcgctacggcatccccgcctctggcaccgcggcgcacgcgtggaccctgctccacgtggacgagaacggcgtgccggacgagaaggcggcatttaaggcccagatcgaggccgcaggcaaagacaccaccttgttggtggacaccttcgacatcaccaaaggcgtggaaaacgcgctcgaggttgccggcaccgaactcggcggcgtgcgcatcgactctggtgacctgggcatcatgtctcgccgtgtgcgggcccagctggacgaagcgggcgcttacaacacccgcatcatcgtttcctccgacctcgacgagttcaccatcgcaggcttgcgcggcgacccggtcgacggcttcggcgtgggcacctccgtagtcaccggctccggcgcaccgaccgcaggcctggtgtacaagctggttgaggtcgagggccacgcggtggcgaagcgctcctccggaaagcgcacctacggcggcgcaaaaaccgcgctgcgcgcctaccgcgcctccggcgtggcggtcgccgagattgtcaccccgcgcggtgcagacatctcccgcaagccaaacctggactaccgggagctgaccgtgccgatgatcaaggacggtgccgtcaccgacgccaccttcgaccttgagtcggcgcgcgagaaccacgctaaggcgcgcgagacgttgccgtgggaaggcctggcgctctcgcgcggcgaggcggccatcccgacgcagtttgtcggtttcccggagccgacagagtaggcgtggcctcatcgaccgaggacctgctcgccgccgcagtcgccgcaatcggcggcgcgccgcggcctggccagcaggcaatggcgaaagcggtgacgacctccctcgacaccggcaagcacttggcggtgcaagctggcaccggcacgggcaagtcgctggcgtatttggttcctgcgatgctgcacgcgcagcaaaccggcaccacggtggtggtctcaaccgccacgattgccctgcagcggcagctggtcgagcgggacttgccgcggcttgcagacgccctcgagccgcacatgggccgccgccccaccttcgccatcctcaaaggccgcaacaactacgtgtgcctgcacaagctttcgcttgacgacgcagcgccggaagcactcatcgaagaagacaacctttcgcgcatcggccgcgaggtcaaacgcgtggctgactgggcgtcggagacagacaccggcgaccgcgacgacctgcagcccggtgtgagcgacctggtgtggcggcaggtgtcggtcacctccgccgagtgcctgggcgctacccgctgcccgcacggcgacgagtgttttgcgcaactcgcccgagaggaggcgagcaaagtcgacgttgtcgtgaccaaccatgcgctgctcgccatcgacgcgctcagcgacgtcaacatccttcccgagcactccgccgtcatcatcgacgaggcccacgagctcgacgcccgcatcacagccgtggccaccaacgtgatctcggaccgggcgctcacgctcgcggcccgccgcgcgggcaagctcggcgctgataagcagatcttagaaagcgtggtggacgacttcaacgcggccgtcgctatcgaggcgcccggacggtgggagaccatcaccgaacccgccgaagcagcgttcaccacgctttcctccgcgctgagcaagacgcgactcgcgatcaatgacgcacctcccggcgagtccgagaatgaccccgaaacctacgccgaacgccagaatctgaagaaccacctcaacgagctggagggcgccgtcgagcgcatcctctccgtcttcgaggaggaagacccgaaaaagcagcgcgacgtcgtgtggctcacccgctccgagcgcggggacgacgcggtctccgtcgcaccgctgtctgtggctccgctgttgagcacttcgcttttcgacaccacccctgtcatcctcacctccgccaccctgacagtcggcggcaacttcgacgccatggccgcggcctgggggctgccacgcaactcgtacgagacgatggacgccggcacaccgttcgacccggcgaagtccggcatcctctacaccgcgacgcacctgcccgcccccggccgcgacggtttggcccccgccaccctcgacgagatcgccgagctcattaccgccgcaggcgggcgcacgcttggactattctcctcgaagcgcgccgccgaacaggccgcggccgagatgcggtcgcggctgccgttcgacatctacctccaaggcgaggacacaaccggagccctggtggacaagttcgccaagtcggagaactcctgcctcttcggcacgctcaccctctggcaaggtgtggacgtgccgggcagctcctgctcgctggtgatcatcgaccgcattcccttcccccgccccgacgacccgctgctgcaggcgcgcgccgaagctgccgacgccgccggccggtccgggttcatggaagtctccgcgacccacgccgcgctgctgctcgcccagggcaccggccggctgctgcgctccaccacagaccgcggggtcatcgccgtgctggacaaccgcctggtcaccaaacgctacggagcatttctgcgcaagtcgctgctgccgttttggcagaccaccaacccggagacggtccgcggctcccttcagcgcttggttaagcggtaaagctcggcgttacactccggcggcagcgtgagcgccgtgatcgaaccaggtgccacttcggtgaacccggcgtcgcggactgcggctgcgcccggggcatcaacgagcgcgttaaacgcatccgcgggcacctcgcgcacattgagcgcgaacccttcgcgcgcccacgcttggaccgcgtccagcgggagtgccgcggcgtagagcatggaggcgtgccccacctgcgcggccgctttgccggcggacatgcccagggaggcgttgatgaggatggtggggtgggcgtcgacaagcgtgagctcctcccccgcctcaatctcagtgcctttgatctgcagcttcgctatctcgtgcgggacgtccgaaaccggagacggcacaaacgcccggactgcgccgactgtcgcgccgggaagggtttgcacgtcgtcccacgccttgttgcgggcgcggcgggcaaccttacggatgcggtgcgagtaccagccggcaaggccgtcgcgccagaacccgtcctggctcgcgcgggggtcgaggcacacggcgagcactgcgcgggccgcgtcgacaagcacggcgttgcgcgccggcggatccgccttcggcaggttgatggccatctgcatggcttggactgttgacgggtcgtcggggtcctccgtgcggtccttgtagtcgcgcgcgggcaactccgctagcagcgcgtgcgcccgggcgatgtcgcttgtgcggtcgggatgggtcacagtccgtcgatctcctcgcgcgggatgccgaggatgtacaacacctcgtcgaggaacgggtggttgaccgaagcgtcggcgacctccttcagcgctggcttggcgttgaaagcaatgccgaggcccgcgcgcgagagcatgtcgatgtcgttggcgccgtcgcccaccgcgacagtctggttcatcgtcagaccagagtccgcggcgaactcctcgaggaactcagccttggcggtgcggtcgaccaccttgccgatgacgcggcccgtcaacttgccgtcgacgatctcgagggtgttcgcgcgcacgtagtccagttcgagctcgtctgcgagcccctcgagcacttggatgaacccgcccgagaccaccgcggtgcggtaccccatcgagttcagggtgcggatggtcgttcgtgcgcccggggtaagctccaccgccgcggcaacctcgtcgataacggacgcgtctaggccagccagcgtcttcacgcgttcgcgcagcgactcctcgaaatccagctcgccgcgcatcgcgcgctccgtcacctctgcgacctcctgctctcggcctgcgtgagcggccagcatctcgatgacctcgccggtgatcagcgtggaatcgcagtcgaagcacaccaggcgcttggccctgcggtgcaggccagcgtgctccatggcaaggtcgacccccagctccgcagacagctccgcgagctctctgcgaatctcctgcccgccacccggtgtgtaatccgggatggtaatgcggaactcgagacctgtcaccgggtactgcgcgatgccgcgaatcacgttgatgttcgccccgtaggacgccaacgtggcgccgaggcggctaacagattccgcggtgaccgggttacccagcgcgacaaccacgtgcgtcgatttcgcccggggaacctcagcagccgcggaaccggtctcgatggtgacgtgctggccgaactcccacagttgcgaacgcagatcgcgctccagctcggtcagcaccgcgggatccatacccaccagggccgcaagcaagaggcgcccgcggaagttcgtctgctcgacgtccagcagctgcacgttgtggcctgccagcgccgcgaagaacgccgcagatacgccggggcggtctgggccggaggtgctgatgactgcgggtttcaggcctggctgcagctcgacctgaagagcggggttctcgggcatcgcgtgattccttctgcgtacggttcggatagacaaaatgccccccatcttacgatgggaggcgttggtcaagcagatttacttgctcggcgcggtgtgcgcgtgcgggccctcttcggcaccgagctcgtgggtagagcccttccaggtggcgggggtgtcctcgttgtgaccggtgtgagcctcgcggcgcatggtctcaaccatgtgcgggtagtgcagctcgaacgccgggcgctcggagcggatgcgcggcagcgaggtgaagttgtggcgcggcggcgggcaggaggtagcccactcgagagagttgccgtagccccacgggtcgtccacggtcacgatctcgccgtaacgccaagacttgaacacgttccagatgaagggcagcataccgatgcccaagatgatcgcaccgatcgtggagatctggttcagggtggtgaagccgtcggtgtccaggtagtcggcgtagcggcgcggcatgcccatgttgcccagccagtgctggaccaggaaggtcatgttgaagccgatgaacacgagccagaaggagatcttggccaggcgctcgtccagcatgcggcccgtcatcttcgggaaccagaagtggacacccgcgactgcggagaacaccacggtaccgaacagggtgtagtggaagtgcgcgaccacgaagtaggagtcgtggagctggaagtccagcggcggagccgcgagcataatgccggtcaggccaccgaacaggaacgtgaacaggaagcccatgacccacatcattggggagtcgaaggtgatgcggccgttccacatggtgccgacccagttgaagaacttcacaccggtcggaaccgcgatcaggaaggtcatgaaggagaagaacggcagtagcaccgcaccggtagcgaacatgtggtgcgcccacacggccatggacagacccgcaatggccagcgttgcgaacaccaggccgatgtagccgaagatcggcttgcgggagaagaccgggacgatctcggagatgatgccgaagaacggcagcgcgaggacgtacacctcagggtggccgaagaaccagaacaggtgctgccacaggatggagccgccgttagcggtgtcgtagatgtggccgccgagaagacggtcgtacaggacgccgagagccgcagcgagtagcagcgggaagatcatcagcgcgatgatggaggtgacaaagaccgtccaagtgaagaccggcatacggaacatggtcatgcccggtgcgcgcatggtcagcacggtggtgagcatgttgatggcagaagccacggtgccgacaccggttgcgccgacgccgacgatccacaggttcgcagacaccgacggtgtgtgggtcgcgtcagccagcggcatgtacatggtccagccgaagtcggcggcgccgcccggggtgatgaagcccgcgagcatcgcgacgacacccacggtggtgatccagaagccgaacgcgttcaagcgcgggaacgccacatccggggcgccgatctgcagcggcagaatgtagttagcgaagccccacacgattggggtaccaaacgccagcagcatcacggtgccgtgcatggtgaacagctggttgaactgctcgttagacaggaattgcaggcccgggctgaacagctcagcacggatcaacaaagccatcaggccggctacgaagaaccagatgaaggacatgatgatgtacatgatgcccagttctttgtggtcggtcgtggtcagctgcttgtaaattttggaacccctgcgggcgttacccgtgggttccggacgtgtcggtgggacatagttgtccaaccgtggcgccacagcggtcatacgatcctcctgattcgggccttccaacgaaaagccacttaacgtaccgaatcatcgtaacgattggcacatggaattgccagccatcacaggcttgctatgtgtacagagtgtatcccccgcgcacccctcgggcagtccgcctgcgccgcggggtgagatcccccagttcacgtggaataacgaacgtgcgcgagccccctcggttaacccgatattgggggttttttccgcgcgcttcaggcaggaggcccaagggggagcccagccggtttagaaatcccagtcgtcgtcctgggtgtcctcagccttgccgataacataggaggaaccggaaccagagaagaagtcgtggttctcgtcggcgttcggcgcgagcgaggccaggattgcgggcgaaacccgggtctcatccgccgggaagagcccttcgtagccgaggttgttgagcgccttgttggcgttgtagcgcaaaaagcgcttgacgtcttccgtccagcccagcgggtcgtagaggtcttcggtgtactggatttcgttctcgtagaggtcgtagagcagatcgaacgcgtgctccttcagctcgtccctgcgcgcctcggactcgtcgcgcagccccacctggtacttgtagccgatgtagtagccgtgcacagcctcgtctcggatgatcagacggatgatgtcggcggtgttggtgagcttggagtgcaccgcccagttgagcggcaggtagaagccggagtagaagaggaacgactcgagcatcaccgaggcgatcttcttcttcgccgggtcgtcgccgcagtagaagctctggataattttcgccttgcgctgcacctcctcattctcctcggtccagcggaacgcgtcgttaatctgcggcgtggaggcgagcgtcatgtagatgttggagtaactcttcgcgtggacggactccatgaacgcgatattggtgtagacggcttcctcgtggagggtcttcgcgtcggggatgagcgagacggcgcccaccgtgccctgcagcgtgtccaagagcgtgaggttggcgaagacgcgcatggtggacaactgctcagcgtcgttgagcgtgttccagctcgggatgtcgttggagacgggaatcttctcggggagccagaagttgccggtcagccggtcccacacttcctggtccttctcgtccggaatctcgttccagttgatcgccttcagcggctgcgggtgcgctgcgacgtaatcctcgtagtcctcgtactcctgttggctcatggcgcttatagtagccgacccctctaacacagcatctggcgccgacaaaccgacccgatgacaccgaaatgccagggcaagtgagatgatcattgatatagagcagattcgagacagaggagctatctcaaaatggcggctgcgaaggaatcgtccaccgagccacttcttgcttcagtgctggacaagctcggtgaagagattgtttctggcaccatgccgacgggccacacttttacgttgcaggacctctcgacgaggttcggcatttcgcgcaccgtcgcccgcgaggccatgcgcgcgcttgagcagctggggctcgtctcctcgtcccgccgcgtcggcattcgcgttctgccacccgaaaactgggcggtgctcgatcgctccgtgatcgcgtggcgcctcgcgagcgctgagcagcgcaacgcgcagattacctcgctcgatgcgctgcgcaccgcagtggaaccggtcgcggcgcggctcgctgccgcccacgctgaacccgagcacgtcgcccgcctgaaggaaatcgccgcgcagctcgtgactctgtccgaggagggcgccggcaacacccctgagttcctcgacatcgacaaggaattccacacgttgctgctcgtcgcatccggcaacgagatgtttaaagcgcttgccgagccgattatgaacgtgctggagggccgcacccgctacggcatcatgccggacgacccggcagtggacaccatgcgaatccacgtcgatcttgcaaaccagatcgcggccggaaacgcgaaagccgccgaggacgcctcccggcgactcctcagcggcatcagcgagttcatggagtactgagccccctcccccgctgctacagcatgcaggacacgcagccctgaacctcggtgccttcgagcgccatctggcgcaggcggatgtagtagagggtcttaatccccttgcgccacgcgtagatctgcgccttgttgatgtcgcgcgtggtcaccgtgtccttgaagaacaaggtgagcgagagaccctggtcgacgtacttcgtggcctcggcgtaggtgtcgatgatcttttcgtagccgatctcgtacgcgtccttgaagtaggccgcgttctcgttgtccatgtgcggcgcggggtagtacacgcggccgatcttgccttccttgcggatctcaatcttcgacgcaatcgggtggatcgaggacgtcgagttgttgatgtacgaaatcgacccggtcggcgggatggcctggaggtagcggttgtaaataccgtcgcgggccacctgctgcttcagttcctcccactgctcagcggtcggcaccgcaatgtcggaggcctcgaacagcgccttgatcttctccgtcttcggctggaagtcggccacgtcgtacctgtcgaagaaggcgcccgacgcgtactcggattcagcgaagttttcaaacgcctcgcccttttccacggcaattttgtgcgacgccttgatgcactcgtacatcaccgcggcgaagtaggcgttggtgaagtccaggccttcctcggagccgtactctatgtgctcgcgccccaggtacccgtggaggttcatctggccgaggccgatcgcgtgggaggcgtcgttgccttcgcggacactcggcacggaatcaatggaggttgaatccgccaccgcagtcaggccgcggatcgcggtctcaatggtgcgggagaagttgtccgagtccatcgccatcgcaatgttgagcgagcccaagttgcacgagatgtcgtggccgaccgtgtcgtacgtcaggtcttcgttcagcacggacggcgagttgacctgcaagatctccgagcacaggttggacatgttaatgcggccggtcttcaccgggttcgcgcggttcgccgtgtcctcgaacaggatgtacgggtaacccgactcaaactggatctccgcgatcgtctggaagaactggcgagccttgatcttggtctttcggatgcgcggatcctcgaccatctcctcgtagttctcggtcaccgagatgtcggcgaacggcttgccgtacacgcgctcgacgtcgtacggggagaacaggtacatgtcgtcgttgcgcttcgccagctcaaaggtgatatccggaatcaccacaccgagcgacaacgtcttaatgcggatcttctcgtccgcgttctcgcgcttcgtgtccaggaaccgcaggatgtccgggtggtgcgcgttcaggtacaccgcgccggcaccctggcgggcaccgagctggttggcgtaggagaacgagtcctccaggagcttcatcaccggaatcacgccagacgactggttctcgatgtgcttgatcggcgcgccggactcgcggatgttggacagcaacagggcgacaccgccgccgcgcttcgacagctgcagcgaagagttaatcgcgcggccgatggactccatgttgtcctcgacacggagaaggaagcagctcaccagctcgccgcgctgcgccttgccggcattgaggaacgtcggggtggctggctgaaagcgcccagtcatgatctcgtccaccagcgcggtcgccagcttttcgtcgccgcgggccaaaaacagcgcggtcatggacacgcggtcttcgaaccgctcgaggtagcggcgcccgtcgaacgtcttcagcgtgtaggaggtgtagtacttatacgctccgaggaagctcttgaagcgaaacttgtaggagtacgcgcgcttgaaagtgtctttcacaaactcccagtcgtactgctcgatcacacccggctcgtagtacttgttgtccaccaagtaccccatcttctcttccaagtcgtggaagtagacggtgttttggttcacgtgctggaggaagaactggttcgccgcctcgcggtctttgtcgaactgaatttggccgttctcgtcgtacaggttcaacagcgcgttcagcgcgtggtagtccagctggtctgccgcggaagcgggcttcggaacgctcgtgccgaggggctgggcgggagttggcgtggtcacggtgaacgggcctttcagtgagagactttcgtgttccgggagcgagagtacttcccggtgtacttggcgcgcaggcgggcgagccgctcagcgtttgggtcgtcggtggtgggcgcgggtgcgtggtcagctggtgcaaggcccaagcgctcggcctgagcaaccagctcagatcgtacgtggttcacgtcctccgctccgcccatcagctcaaatcggtagaggtagggcaccttgcacttcgcggcaatcacgtcgccggcgcggcagtagtccgcgccgaagttcgagttgcccgaggcaatcacgccgcggatgaggcggcggttgtgctcgttgttgaggaaccggatgacctgcggcggcacggggcgggagttttcgtgcgtgagcgagacgccgcccccgtaggtcgggcagatcagcacgtacggctcgtccacgacaagctcgccgtcgtgcttgtgcagggggattcttgccgacggcaaccccaccttctccacgaaccgcttcgtgttctcggtcgccgaagagaagtacaccaccaacacgccgcttccccttcttttacggcttacgccgctgcgaggctgcgaatgcgctcggggcggaaaccggaccagtggtcgccgtcaacctcgaccaccggggcctgcaggtggccgagcgccatgacgtaatcgcgggccgcgtcgtccagagagatgtcgaccaggttgtactccaagccggccttgtccagggcgcgggtggttgctcggcactgctggcatgcgggcttggtgtaaacggtgatagacatctcgacgcttccttgtaaaagtttcgtgggcttgaaaatgctcttcgccgatcccctcggcggttcaggagagacactataccttggggcaaaaatcggcaactgatactatatgtagtagttacacacgtggtattcgcaggtggggccgggaaattacccacatgtagtcttcggcgtgaatcgctgacttacaggtgtggtattaaattttcctgagacttcgtccgccgccgagaaacgccgaaaaatcccgcctcggccgtaaagccgaaagacgggattgatcggttggttagcgctctagccctggcgagccttgaagcgcggctccttcttgttgatcacgtagaccttgccgcggcgacgcacaacctgggcgcccggcttgttcttcagcgaccgaagcgacttgcggaccttcatcgggcgctcctttctgttagagactgctactttatgcaacgcatggccgaaaacggccgcgtcgcgacacgagcgaacactctacacgcaccctgcagcaagcaccaaacccctttcgggaacaggttagcctctcccgcgggtgtagcggcgttccatttcatcggcgacggtgtcgaggctcttacccatcgtctccggaatctgccgggcgacgaaaacggcggcgatcacgccgagcaccgcgaaaagcacaaacgtcgtcgtagcggatagcgcgttcaccagcggaaggaagaactgcgccaccacccagttcatcgcccacaacgccaggccggccaagcccatgcccacgccgcgaatctgcggcgggacgagctcggagatcaaaagccacgtcgtcggcgacaccgccgcctgctgggaggcgatgaatcccgccatgcacgccagcgccacccacgccagcgacgtgttcgactccgccgcgcggtaggtcaaagacagcgcgaggaggaagacgatgttgccgcacaacccgaagagcagcagccggcgacgcccgatgcggtcaacaagtttcagtcccacccagcacgcggccacactcacgaggccgatgacgatagaggtgtagacggcgttggcggtggaaaggccgaccttgttcatcatcgtcggcgcgaagtacacgattgcgttgacgccggtgatctgctgagtcaccccgagcagcgccgcgaaaacgaccgtgacttgaagccacctcgcctccgccagcgcgcgccactgcgccgacacacgcgggttgtcctcggcctcagcgcgcgcggtctccagctcgtccgcgtcaataccagccttggcggcgattgccgcggccttctcgtcgtgtccccggcgcgcgagccacagcggcgtctcgggcacgaacgccatgccggcggcgagcgcgagtcccggcagcgcggcggcgccgagcatgagccgccagttctccagcggcgcaagcagcgagttgaccacgtaggcggcaagctggccgatgacaatcatgagcgtgttcagcgacacgagctgaccgcggatgctgctcggcacgatctccgagatgtacatcggggtgacaatcgatacagcgccgaccgcgaggccgagcagtgtgcgggcggcggcgagcgagccgacggaagctgcgagcgcgcaccacagcgagccggcgacgaaaagcgccccggcggtgatgagggtgcggcgccttcccagcgcgtccgcgacggcgccgccgctgatcgccccgacggcggcgcccaccagcagcatcgaagtgacgaacccctcctgcgcgggactcatcccgaactcgggcgtaataaagagcagggcgccgctcatcaccccggtgtcgtagccgaagagcaggccgccgagcgccgctgtcgccgccaccttgcgggcgtaagtaaattccatgccgccaaatatgccccgcgtctaccatgaatgtcatgtccagcgacgaaagcgacctgcagcggcacattatccgggcgttgggggtctccccctcaatcgatccggcggaggagattgaccgccgggtggagtttttgagcgactacctggcagccacgggcgcgcgcgggttcgtgctggggatctccggcgggcaggattcgacgttggcggggaagctggggcaggaggctgtgaataagcaacgggccctcgggcgggacgtggaattcgtcgctgtgcgcctgccgcacggggtgcaggcggacgaggacgacgcgcagctggcgctgaaattcatcaacccagaccgcacggtgacggtggatatcaagccagcaactgacgcagtcgatgctgcggtggcagccgctctcggcaccgcgcggttgggcgacttcaacaagggcaacgtcaaagcgcggcagcggatgatcgcgcagtacgcgatcgcgggcgagcttgggatgttagtcatcggcaccgaccacgccgcggagaacatcaccgggttcttcaccaaacacggcgacggcgccgccgacctcatgccgctggccgggctgaacaagcgccagggcgcgcagctgctagagcacctcggcgccgaccggcgactgtgggagaaagtgccgaccgccgatctcgaggaggaccgcccggcgctgcccgacgaggaggcgctcggcgtcacctacgcgcagatcgacgactacctcgaaggcaagccaatcgacgcggatgcgcgcgagcgcctggagcacctgtggcgcgtcggccagcacaagcgccacctgccgcccgggcctgcggacacctggtggcgctaggtcccttggtgccctaggcgccgagaacgctttcggcagcgcgcacgagcgcgtcgccgtagctcgggccgtgggtgtaggagtggacggccaaggggtgcagctggtgggccgggatgcgctcgcgccagttggcgctgagctgcccgccggcggccaagtagccgtccacgaaggactcgaagtacggggcgccgaagagctcgagcatcgcgatgtctgtcaacgggtggccgccgtgtgcggctgggtcgatgaaccgcacgccggccgggctgtagagcacgttgccgctccacaaatcgccgtggaggcgcgccacgggggcgtcctcgtcttcggcgagcagcgcgtcgcaggcgcggcgcacggtatccaggccagcctgatgtaggttgcccgcctcgtgcgccttctgcgcaaacggcagcacgcgctggtggacatagaaatcggcccaacgctcggttggcttacactcctgttgcgcgcggccgatgtagttcgggccgtcccacccgctcgccggagcgccgaatgcgtccgcccccgcggcgtggattgcggcgagctcgcggccgccctcgtgcgcagcgtgtgcggtggggcgtgcggtgggcaccttctcaatcacgaggtagttctcctcgtcgctgacctcgaagacctccacgactgcgctggatccttcgcgcaaccaccgcaagtacgccgcctcggcagccgcggcgtgcgggccgctgccccgtttcacaaacgagttagctcgtgtcttagacaaatctcgcctccatctccagcaggaatttcttcatttccactcccccgccatactggccgatcgccccgcccgcgcgtacgacccggtggcacggcaccacaatcaccagggggtttcttgcgcacgcggtgccggcggcgcgcgccgcgcggggggcgcctgcggcctttgcaagctcagcgtaggtggcggtctcgccgtacggaatggtgagcagcgcccgctgcatgcgctcgtagactcccgaggtcaaactccagtccagcgggaggtcgaaagtgcggcgctgcccagaaaaaaattgggctagttgcttatcgacgtccgcgtgatcggatttcaccgccccgtcggcaagcaactgcccaaaccccacccgaaccaacccattcggtgaacacacgcttgtcagcggtccaaccggggtgtcgtgcacgcggtaggtgtacatgttgtggagctaacgggattcgaacccgtgacccccacactgccagtgtggtgcgctaccagctgcgccatagccccgctgttcggaaggagccctcccgaacggcttcgataaatataacagccgctgcaatcagcgaccaaatcccgccgtgactaggaattcttcagcgtggtgacccacgcctcgcggtcgccgagatcctctgcgtccttgccgtcgatccacacgcgcggggtccacgcctcgccggtctcgtcctcctgcagcttcaggttggccgcgccgacttccttcgccttctcgatgaacgcgccctcgcgtatgtcgctgacagcatcctccgaggcgccgtagtccgcagccagatccgccaggtcgtcgttcgagtacttcgcggtggcctgctggttcacgtacaggaagtcgcgcaggctgaacgcctggtccatgtcgccgcggctgatcagcgccagcatcgccgccagcgagcgggtggagtggccctcaataccgcggtcctggaactccatcatgtgcaggtccacgttgatgtcgccggccttgagcgcctcaaccatctctgcgtcggtctgcttgtgcagctctgcgcagtagccgcaggagaaatcttcgaacagctgaccggtcggcgcatccgggttagcgccgaccaggtggatgacgttgtcgtcctctgcccactcgacgttgatgccgctcatgtcgatcatgccttcgcggacggcgttagcacgctggctcttgccgttggacacaatcaggccgattaccagagcggcgatcgcgatcacggcgacaatcgcccaaatgaacgcgttgccacccttctggttcgggttctgcactttgcgcgtagtcacagctacatctcctcgacggtaaacagggttaatgtgatgggtcagtctacgggtagaccgcaaacttcttaaatggtcggtacatcatgaatgcagttactgccagcaggaacacatcgcgccagatggcttgcattatgtccccgtgctgcggctcgcgctggttggggtcgaaacacccgcagtcaatcaccatgccgcgggcgtgcacagaccacaagcccatgatgaacataatgagcaccaccatggagaccccgccagcccagcggatcttgatgccgagcagcaacaacaacccgcctgccagctccagcgggccgatgaagtttgccaagatgtcggaccagtacggggtgaagacctcgtacgcctcaatcttctggaacacctcgaggtggttgccgattttggtgtagccggcgtagatccacacggccgcaagtccgaaacgggccgcggcggcggcgaagtcgagcacccgcgtcatgggagcgggcgcagtttgtacaggtgagctcacaggtgttgacactagcccaccgcgcgccggcaatggtgcgacgaacgatgtgttcagcgttactttccaagcaccccgttcacaatcgctgcggcttcttcctgcacctgcttgaggtgctcctcgcccttgaacgactcggcgtagatcttgtacttgtcctcggtgccggacgggcgcgccgcgaaccaggcgttttcggtggtgaccttcagcccgccgatcgctgcgccgttgcccggggcctcagtcagcttcgcggtaatctcctcgcccgcgagcgtggtcgccggcacctgatccggcgacagcgccttcaacgcggccttctgctcgcggtcggcggcagcgtcgatgcgcgcgtacgccggagcaccgtacttctgctcgagctcggcgtagcgctgcgacggggtctttcccgttaccgcggtgatctcggcagcgagcaggtcgaggatgaggccgtccttgtcggtcgaccacaccgtgccgtccttgcgcaggaacgacgcgcctgcggactcctcaccgccgaagccgatggtgccgctgaccaggccggggacgaaccacttgaagccgaccggcacctcaaccagctttcggccgagcgctttcaccacccgatcgatcatcgacgacgagaccagggtcttgcccaccgccgtatcctgaccccacccatcgcggtggctgaacaggtactcgatggccacggccaggtagtggttcgggttcatcagccccgcgtcaggggtaacgataccgtggcggtctgcgtcggcgtcgttgccggtggcgatgtcgtacttgtcgcggttgcgcaccaggctcgccatggagttcggcgaggagcagtccatgcgaatcttgccgtctgtgtccagcgtcatgaaccgccaggtcgcgtccacctccgggttgaccacggtcaggttcagcccgtagtggtccgcgatcgcgccccagtagtccacggacgccccgcccatcgggtctgcgccgattgctaggccggagcgcttgatcgcctcagtgtcaacgacgtggtcgaggtcggagacgtacgcgcccttgaagtcgaacgcgctcgcgcgctcgtcgcgcacgccgctcacgcttacccggcgcacgccctcgaggctggccgcaaggtagtcgttcgccttcgccgcgatccagtcggtcgcgtcggtgccggcaggaccgccgcttggcgggttgtacttgaagccgccgtcgcgcggcgggttgtgggacggggtaatcacgatgccgtcggcgcgcttcgcgtccgtgccggtcaccccgccgccgaacttggcgttgtgccgcaagatggcgtgggagaccgcaggcgtcggcgtgtagcggccgtccgcgtccaccatcacctcaatgccgttagcgatcagcacctcgagcgcagaaatcatcgctggctcgctcagcgcgtgcgtgtcgcggccgatgaacaccggtccgccaatgttgtggttgcggcggtagtccacgatcgcctgcgtagtggccagaatgtgcgcctcgttgaacgcgttgtccagcgccgaaccgcggtggcccgaggtgccgaacgcgacttgctgcgctgggtcggacgcgtcaatgtcgcgggtgtagtacgcggtgaccagctccgcgatgtcgatgaggtcctcgggtcgggcgggctgacccgcgcggtcgtgtgccatgatgcgctccttgcggtggctggtggtttcggcggacgcttacaaccccacttttacccaagttggcagcttcgcgttcgggtttgggcgggagcggccaatagactcgactcccgtgcgcactgactctcttcacaccggcatcgcggtcggacttggcgcagccctcggcgcgctcgcgcggtacgcgctgaccttactcaccaccgacggatcgccgcaggccgcggtcttggtcctggcgatcaacatggccgggtgcttcgccatggggcgtttcaagcccgggccattctggggcatgggctttctcgggggcttcaccacgtactccgcggtcgccctcggcgcgctcgacttttcgcttgccggcgcgacaatcttcatcctggtcaccttcaccgcgtgcgtggcgtcctggttggccggcgacgccgcctcgggaggtgcccgccgtggctaatctcagcttgttcgcctgggtcttcatcggcgccttcttcggcgggctggcgcgctgggccctgtcgcacatcccggccccgagggtgggcacgttcaccgccaacatcgtcgcgtgcgccgtgctcggcttcaccttagtgttccccgcgccgtggcaagcgggactcggcgccgggttcgcgggtgcactttccacctggtcaacactggcgaaggagtgcggcgagctgtacaagcgccgccagtggggcaagctggccaaatacgccagcttcaccgccgcgatgggcatcgcagccgctggctggggcgtgatgatcagccgccggggaatgtggggctaaccagccggcggcctagtccgcgatcgcgtcgagcggaggcgtcttcgaagcccggtgcgccggccagagcgcggcaacaacacccacggccacgctgccggcaagcatcagccacaccaggttccacggcacgacgatggtgtcgaggccttggttggcgagcacggtgaggaacgtccacccgagggccaggcctaagacaacgcccaacaccgcgccaaagaacgccatctgcaccgattctaagatgatcatggtgcgcacctgcctgcggtgcgtgccgacggcgcgcaacatcccaatttcttggcggcgttcgatcaccgacagcgtcagggtgttcacgattcccagcaccgcaatcaccacagccagcgacaacagcgcgtacaggatgaacagcatctggtcgatgaggcccagcacttctccagagatatcgtccttcgactgcacctgcacaacaatgtcgtggcgcacctcgtcctcgaggttgccgcgcagttgatcggtcgagaccgtgccgtcgccgctgacacccatcatgatgattcgggcgctgccggggacgatctgattcgcgacgtcggcactgaccaccaccgaagtgaggatggaagagttctcgaagatgcccccaacggtcgcttccaccttcaccggggaggcaccaggcgccgcgacagtgacgctgtcgcccaccgaccagccgcgttcttccgcccagtcgcgcggggcgatgaccacgtcgccggccagcgatgacgacccgtccaccatatccatcgaaatcaagtctcccgggtcgccgaagaggaccgacgtcgtgccgaaggggccgaactgcgctgagtactccccgtcgacctgaatttgggcctccgtgtaggcggcgacggcgccaaccccgtcgacggcggggatgcgggacatcagggcgctatcaagcggaaaagccccgaacgccggcccggaaagcacgtactccgcgctgacctcgttgtctgcgacgctgtccaccgaatacttcatcgacgcgccgaacatgccgatcaagttgaccagtgcaatgccaagcatcagcgcgaaggcagttgcggaggtgcggcgcgggttgcggctggtgttggtggaagctagcttgccgacggcaccaaacggcgcacctattacccttccgacaggcggaacgatcggaagactcatcgcgggacccgccaagaagatgccggcgataaccagcaccgccgccgcgccgaccaataatgcgcgctgggccgtgcggccgtcctcccacccgagtgctgcagcgccggcagcgactgcagcggcgatgagcagcgcgccgatcactgtgcgcgtcttcagcggctggggcgcggcggattcgctggcccgcatcgccgcgaccggctgcacccgtcctgcttggcgagccggcgcccacgccgacagcagcgtcacaacaacgccggtgacgatcggcaccaccaccgcgtcgagcgacaacccgagcccgcccgccggcagcgccatgccgttttggcccataccccacttgatggcggcgaccatgccgacgccggcaagcacaccgagagcggaaccgatgagaccgacgacgaacgcttccgcgatgacggatctggtcacttgacgctttgatgcgcccagagcgcgcagcagcgcgaactccttggtccgctgcgcaacgatcatggagaacgtgtttgcaatcaaaaatgtgcccacgagcaggcccacgaggccgaacgcgatgaggaagtaggacacgaagctcaacgcctcgcgcactgattcgctggcttcctctgctgcttcctccccaggacgtatggtgagctccgggtgctgctgcgcgagctgctcgcgcagcgtctccgggtccgtgatcccgtcagtgctgatcaaaagcgctgtgacgtaccccggtgtcatgtatgcgtcgaggtagtcctgcgccggcaacaggaacttcattgaagtctcctgggtcagttcgtcatcgtagaaacccacgatggtgaatgtccgccggtccttggtatcaaccgcgataacctcttggcccagctcgagaccgtagaacgcggcgccgttgccgttgacgatggcctcgatcggttcaccgccgctattgtgcggctcgcggccgtcggtaatctccggcaccgggccgaccgcctcggtctctgggtagtacagcccgccagccgacatcccttgccgggtctggtacgcctcctcgtccgtgttcgccacgacgagcaccttcgagtcagtcacgttaacgtttcttacgccctcggcaccgcggatcgcgttcgcgtcctcctccgtgatgccgccttcaccgtcagcgggttccaccaccacatcggcgccctcgtagcgcgtggaaacggctgagtcgaacgtgcgctccagcatgttcgtgaacatcatggaacccgcgatgaacgcggtgccgagcaccaccgccaacaccgtgagcgcaagccgcaacttgtgcgcaccaatgtttcgcagcgagaccttcgtcatcgcccgtgaacccaccgccattactgttcgatccccgacatcacgcggagaattgcgtccatcgacggttcatagagctcgtcaacgatctgcccgtcccggaggaagacgaccctgtcggcgtacgacgcggcacgcgcgtcatgcgtgacgatgacgacggtttgcccatcgtggtcaaccgcgtgcctcaagatgctcagcacctcgctacccgcgtttgaatcgaggttgcccgtcggctcgtcgccgaagatgatctcgggcttgctcaccagcgcgcgggcgcacgccacacgctgctgctgacctccggaaagctcacttggccggtgcgccagccgctgatcaagacccaacctggtcgtgatctcgtcgaaccacgccttgtcaatcttcttacccgcgatatctgtcggcagcgtgatgttctcagccgcgttcaacgtgggtaccaggttgaacgattgaaagatgaacccgaggcgatcgcgccggagctccgtcagctgcgcgtcgttgagtgaggacaacgccgtaccgccgatgtacgcctcgccagaggtaaacgaatccagccctgccatcgtgtgcatgagcgtcgatttgccggacccagacggccccatgatcgcagtgaacgcgccgcgcgcgaactccacattcaccccagccagtgccgacacctcagtatcgccctgcccgtaagttttgactagatccacggccttcgctgctgcttccaccgtgactacgctaccccaccagtgattcgagcccgcggtcgtgcgcctcgggtagctgctcgctgtcaggcgctaggtgatagcgggtatctcggcgacagttgtgtgtttccgcaggtcgcgttgcgcggtcgtgggagttacccgctatcagtggttgtggcctgtagctcccaaggtttcagtgtgtcaacgacagggggttttgcacctaccgatgaggctgtttgtcgtcgggagctacagggcgcggcgcgtgcgtcgcccgtgtcactgccgcctatgtgccgggagcgccccgatatgtcagtgcagtcggcgccttgtagctcccaaagttccgtggtgtcagcgacctggggttttgtgggccggtttgaggctgtttctcgttgggagctacaggacgcaggctgtgacgatgcccgagttgcccggcgtgccagcggtgcggcctttaaggggggcggatcgtttgacgctgctcgggtttgtgtgcgggcatagtaaagcacccgatctaccggttgtggccggtggatcgggtgcttcggtattttgttgttgttttgttgttgttgggtcggcggtaacctactctcccacaccctcccgggtgcagtaccatcggcgcgggcgggcttagcttccgggttcggaatgggtccgggcgtttcccc

SEQ ID NO: 10 - DNA, 150251 bp, Corynebacterium cassirii
  source 1..150251: mol_type = genomic DNA
gtgctggcggtggtgggtgcgtgtggtggggtgggggtatcggtgttggcggcgtcgataagcatgaaagcccacgctcacgcgccgacgctgatcgacgggcacctgcgctcgggaggtgccgacctgctgctcgggatcgaggagcggcccggcgcgcggtggggcgagattgcgctgggggagggcacgatcgcgcgcggggacatccgccgggcgctgcccgccaccagcggcgatgtagcggtgctgacctcgactcgcgcgaccgtcgccgacggcgccgcgatcactccgtccgacgttgagaccgtggtcggcgcgctcgccacggggggtgtgacagtgctggatgtgccggtggaggctatcccgcagcgctgcgacgccgctgtcatcgtcgtgcccggccagcttcgaccggctgccgccgcggcaaggatcgcggccgagctcgatgcccgcggtgtgccgcacacgctggtgctgcgtcgcgcggggtgggagtcgctgacggacgccgaggtcgagcgcgttgccgggtcgcggatcatcgcgcagctgcccacatccgcagggctggctaaaaccatcgagcgcggcgggctgccgcagcggctcccgcgcccgctggctgcagccgccgagcgttgccttgctgaggtgctgcccgccgcggcccgggaaaagagggcagcgtagatggccgcgaaccacgatgtgctcgagcgcgtgcagcgccggcttgcggacgagccgcccaaccccacccccgaacgcctcgcccacctcatccgggaagaagctgtggtgatcagcgacgtcgacgtgctcgacctgctgcgccgcctgcgcgaggacaccaccggcgcgggaccgctcgagccgctgctcgctggcggcgacgtcaccgacatctgcgtcaacggcgcggacgaggttttcatcgacgctggccgcggcctccagcgcgcgccgcagcgcctcttcgacaccgacgacgacgtgcgccgcttagccacccgtttggcgatgcggtgcgggcgcaggcttgacgacacccacccgtactgcgacggccacatcacccgaccagacggcacccttttgcgcttccacgccgtgctggcaccgacctcccagccgggcacgtgtatttcgcttcgcgtgctgcgcacagccacggcgagccttgcgtcgctggtcgagcgcggttccgtcgatgcggagcgtgccgagctgttgcgcgggctcgtccgcaagcgcaagacgtttctggttgtcggcggcaccggcagcggcaagaccacgctgctttcagccatgctcgccgaggtcgacgcgtccgagcgcatcatcgccatcgaagacaccctcgagctgaccccagcccacccgcacgtggtgaacctggccacccgcggcgcgaacaccgaaggcgccggtgagatcaccgtcgcagacttggtgcgtcaagcgctgcgcatgcgccccgaccgcattgtcgtcggtgagatccgcggcgccgaggtcatcgacctgctcgcggcgctcaacaccggccacgagggcggcgcgggcacgctccacgcgaactcgcttggtgaggtgcctgcgcggttggaggcgctcgccgcccttggcgggctcgaccgcgcgggcctgcacgcccagctcgccgccgcagtggacgccgtggtggtggtcaaacgccgaccggacggcactcgcctcgtccagcagattggcgtgctcgacggcttgcctgtgaccgcgcgctgcgtgtgggacgccggcaccgggcccgccgaggggtacgaggagctcgcatgcgcgcggtgatcgtggcactggccgtggcctgccttaccggtccgccgcgaccgctcggccgcatcgaagcccgcagcggcgagaccgcttctttcaatcccgcctggattcccgtcgctgtcggcgcggtggcgcttaccgctttcgccactggtcgcgccggggtggtcgttgccgcggcgtgcgccggcgcttgcgccgtccacacggttgctgcccggcgtgccgcgcgcgccgaccgggcccgcgcggcggcggccgccgagttcattggccacctggcggagggcgtcagcgcgggagcaacgctcgcgggtgccgcagcgcgcgccaccgagcggctgcccgaatccgctccggcgacgctgcgccgcgattgcctcgtcttcgcagcagccgctcagcggggcgacgccccgccggaggtcgccaccccggaacttcagcgcgtcaccgcgctgtgggcgctatccaccacccggggcgtgccagttgccgggcttttagccaccgcccgcgacgagatcgaccaccaactgcgccaccgcgctgcgacgactgccgcgctttcagggccgaaaaccaccgcggttgtgctctcgctcttgccgctggctggcatcgggatgggcgcggcgatgggggcgcagccggtcgcgctgctcacctctcccggcatcggttcggtgcttttggtcgctggcaccgcgctcgtgagcgcaggtgtggtgacctccggcgagatcatcaggagggcggccgcatgatctccccgctcgccttgtgctgcatcgccggcgcgctcgcgacgacccgccccaggccccgcggccgcctcagccttggcgcgccggatccaacgcaccgcccccgcgacggacccgcgggggcggatccgaaccggtgcgccagcgacatcgcgctgttcgcggcctgctccaccgccgggctatcgcccgcgcaggcggcggccgcggttgcggacacgtacgccggcctcagtgccggctccggcactgcctggcacaccaccgccgcgcttctggcgctcggggccgaccccgagcgcgcctggtccgaactccgcgccgtcgacggcggggcggacctggccaaccttgtcaccatgtccaactcgtccggctctgcgctcgctgcgggctgctaccgcatcgcggagcgcctccgcagcgagggagccgaccacgcaaccgcgaaggcggaacgcgcgggtgtgctgatcgctatcccgctgaccgcctttttcctcccggcgtttttcgccctcggccttgcgccggtggtgatcagcctgggatcaaccgtcctccgatagccaaaccttgaaaaacgaaagcgagaacaaccatgaaccgcatccagctagcaaccatcgcctcctacaacgctgccgtcggctgggcacagaacacccttgccaaactcggcaacgaccgcgggatgagcaccatcgaatacgccttcgggtcgttggcggccgcggcgcttgccggcgtgctgtatctggtggttaacggcaacggcgtgacctcggcaatcgagggtgtcatcaccgacgcgctcagcgaccgcccgaactagacatgactacggtagaaaccgcgctttcgctcaccgtgctggtcacggtggcagcggcgatcgtggccggaatcgcgacgatcgcggcctacatctccgccgtcgacaccgccggggcggccgcgcgcgccagcgccatcggcgtcgcgtacgcgccgccccggggcacggtagaggtgagcgagggccacggcctcgtcaccgccactgcgcgcgtgcccgcggcaatcggcaccatgcgcgcccaggcggtgtttccggtggagtaccaatgagcgcggtaaccgccgcaggcatcgtcagcgccgtcaccgcgctcgcggtcagcgtcgcgggcatcggtgcgcacgtcgccgattcccaccgcgcgcaggttgccgcggagctcgccgcggttgccggtgcgcaggcctactacgcaggcttcgagccctgcgaggtggcgcggcgcacagccgagctcaactcggcggtgcttcagagctgcacgcttgccgacggccacctcaccacctccacctccgcacgcaccggaagcggccaagcgcgagccggcccggcctaggcctcagcggacgcgtcgcccgcggtcatcgccaccagcgcgcccagcagtttcagcgcggcgtgcttgtccagcggctggttgccgttgccgcacttgggtgactgcacgcacgacgggcagccgtcctcgcagccgcaggagcggactgcctcgtacgtggcggtgatccactcgcggaagcggtgaaagccctcgtcggcaaaccccgcgccgcccgggtggccgtcgtagacgaacacggtgggcagcatcgtgtcggggtgcagcgcggtggacacgccgccgatgtcccaccggtcgcaggtggccaaaagcggcaacagtccgattgcggcgtgctctgcggcgtgcagtgcgccggggacctcgcccgcgctgatccccatcgcgtcaagcgcgagcgggtcgatggtgtaggccaccgcgcgggtgatcaggcgctgctcgggcaggtcgagggggatgtggtcggacacggtgccgtcgctaagccgcacgacgtaccccgtcacccggtcgatcacctccacgtctacgttggccacccacaaccccggcgacgggttcacaatcgcggacggcgagccaaggatcgtgatgtcggtggtcgagcgggcctgggtcgagtaatcgggtgtttccggcgcgacgagggcgacgtggtcgtccaagtcgagggtgtccaccacgaagtgttccccctggtggatgtacaccgcgccgtcgtgcacctggctcattgcccgcacggcgtcgacggtgcccagcagccggccgtcgctcatgtccacgatcgccacttcgttgccggagccgccgcgcagcgagacgtgcgcgtgggcggtctcgggagcgatgtcgccttcgagctggggcacggcgaagaggcgttgcccgcggcgtcgtaaatagcactgcctcaccagctccccgacgactgcttcagcaccgaaggcggcgacgtcggtgtcggtcagcgggcgctccacggccgcgcagtagatgtgcccgcgcagaaggtaggggttcgacgggttgaacacactgttctccaccggccggtcgagcagcgcctccgggtggtggaccaggtaagtgtccatcggctcgtcgcgggcaaccatgaccgccaccgcgtgctggccgcgccggcctgcgcggcccacctgctggcgaaacgacgccaccgtgccaggaaaccccgccatcaccacagcgtcgaggccgccgacgtcgatgccgagttccagcgcgttcgtggaggccagccccagaagatccccgttgtccaaggcgcgctcgagcttgcggcggtcctcggccaggtagccagcccggtaggaggcgacgcggctggcgaaatccggcttgcccagcaggatgagctcctcctgcgcgcgcatcgccacgatctcagcggcgcgccgggagcgcacgaaggtgagcgtgcgcgcgccgtctgcgatgagctgcgccatgatcgcgccggcctcggtcgtggccgcgtagcgcacgggggcgccgttttctccctcagcgccctcgatgaagccgggttcccacagcgcgatggtgcgctcgccggtcggcgcgccgtcgtccgtgaccgcggtgacctcgcggccgcacaggcgcgaggcctggcccgccgggtccgccgctgtcgcagaggcgaagatgaaggtggggtgcgcgccgtaggcctcggcgatgcgggtaagcctgcgcagcaccagcgacacgttggcgccgaagacgccgcggtacgtgtggcactcgtccaccaccacgtacttcaggtggcgcagaaggcgcgcccagcgctggtgtcccgcgaggatgccggcgtggagcatgtccgggttcgtgaacacgaaccgggtgtgctcccgaatgccggcgcgggcctcggcgggggtgtcgccgtcgtacggcgcggcgttgatgccggcggtaacgagcccgtcagcctcccggatcatccaggagaccgcgtgcagctggtctgagccaagcgccttcgtcggcgtgatgtacatggcgcacgcctttgggtccgcggcgagcgcagacagcaccggcagctggtagccgagcgacttgcctgaggaggtgccggtggcgacgatgacgtcgcggcccgcccaggcaagttctgcggtgtgtgcttggtggaggtaaggggaggtgaggtgggcgtcgacaagcagctgcttcaagctgggctcaatccacgcgggccacgccgcgtagcgcgccggagacgaggggaccttggctacgtgcgtgacggtggagctgggcaggcggcgcgtaagcgacccgatcagctcttcaccgaaatcaaccatggacacaaagggtaggtcatacctgaggttaacggcgtgccgggcagcgcgtttcgtggcacactatgggtaggtcacaggttttgtgtgcgccctgctacaaggcgctcgcgaggattgtgcacgcgggcgccaggactttccccgaactaccggcgaaaagccctggtggacggccttccatatctacaacgcaacatctttgaaaggtttcatttacaccatggcaactggcaccgttaagtggttcaacgccgaaaagggctacggcttcatcgcaccggaggacggctccgccgacctgttcgtgcactactccgagatccagggctccggcttccgcaccctggaggagaaccagcaggtcgagttcgaggtcggcgagggctccaagggcccgcaggcgcagcaggtgcacatcatctagtttttgcgctctgctctcaacgagctttgtttgatcccgctggccgcgcgccggcgggatttttcaaatcgcggacacgccgcggctgacatccctccactcgaagaacttcgcctgggcgcgctggatgagcaagcccaccagcgaccccagcaggacgccgaccaccatcgccaaaagcgggaagtccgacaacagcgagccgccgaggtagcccagccccacgcccaaaaacgcccagaggatcacgccgacggtgtcgtaaatgaaaaacgcgaaccagttatagcccaccgaggcaagcacgatcgtggccacccagcgggcccacggcaggaagcgcccgaccaagatcgtgatgcccgcgccgcgcttcatgtttctgcgcacccactgaatcgcctggcccgccttggactcggggtcgaggcgctcgaccacgccgatcagcttgctgccgagggcgaaacacaagttatcgccgatcaccccgccgatgattgccgcgaggatcgtgccccacacattcggcaccccctgggatgcggaaaacgcgccggcgaggttcagaatggtttcgctcggcagcagggggcaaatcgcgtcgccgaccaccaacagcgcgagcagcgggtagaaggcgggggtggccatcaaagtgtggaggaaagcgatgaaggaatcgatcatggggccaagcatcgattgcgtgctcctttcctcccggtccgcttacgtggtctgctcgttgtgcgatatcgatgcgagtctagccgtgcgggggaacgggtggggtgctgtgttgggtggtgtgttgggggagtctgctacaaatgaggaagttttcgcacctatatataaggcgcgctgaaaacggcgcagtatatggtgcgagggacatccctgcgaacgcgaagtgaggtggctcggcattgtcagcaagcggtaaggccgacggcaagactctggtcatcgtggagtctgcgacgaaagcgaagaagatccagaagtacctgggcgacaactacatcgtcgaggcgtctgtgggccatatccgcgatttgcccggtcgcgccgccgacattccggcgaagtacaaaaacgagccgtgggcgaagcttggtgtgaacccggaggacgggttcagcccgatttacgtggtcagccaggacaagaagaagaaagttgcggacctcaaggcgaagctgaaagagtctgacaagctgctgctcgccacagacccagaccgcgaaggcgaggcgatcgcctggcaccttttggagacgctgaagccgaaggtgccggttgagcgcatggtgttcaacgagatcaccgagtccgccatccgcgaggccgcggagaacacccgcgaggtggacatggacctggttgacgcgcaggagacgcgccgcattttggaccgcctctacggctacgaggtctccccggtgttgtggaagaaggtcatgccgcgcctgtccgccggccgcgtgcagtcggtggccacccgcgtgattgtggagcgcgaacgcgagcgcatggcgtttgtcgaagccgagtactgggacctgacggcgacgcttcaacctcagtccgggactgagcgcgtgtccttcgacgcgaagctgacggctatcgacggcacgagggtcgcccaaggccgcgacttcgacgaccgcgggcaggtgaaaaccgcagacgtcaccgtggtggacaaggccgcggccgaggcgctcgccgccgggctcgagggcgccgcgatgcgggttgccggcgtggaggagaagccgtactcgcgcaaaccctacgcaccgttcatgacgtcgacgctgcagcaggaggccggccgcaagctgcacttcacctccgcccgcacgatgcgcatcgcgcagcgcctgtacgaaaacggccacatcacctacatgcgtacggactccacgtccttgtccaagcagggcttggatgccgcccgcgccgccgcgagcgagctctacggcgcgaactacgtcaccacatccccccgcgtgtacgaccgcaaggtgaagaactcacaggaggctcacgaggcgatccgcccagccggtgagcgcttcgccaccccgggccagctcgccggttccttggacgccgaagagttcaagctctacgagctgatctggcagcgcaccgttgcctcccagatggaggacgcgcgcggcaattccaccaaggtcacggctgaggcgaccgcgtccaccggccagctcgcccagttcgcggcgaccggtcgcaccattaccttcccgggctggctgcgcgcgtactccgatcaagacaaggaaacgcacctgccgcaggtcgccgagggcgacgcactggacaccgagaagatcaccgcagaccagcactccaccaacccgccggcgcgctacaccgaggccagcctggtgaagaagatggaggatctgggcatcggccgcccgtcgacctacgccagcatcatcaacaccatccaggaccgcgggtacgtggtcgcgcgcggcaacgcgcttgtgcccacctgggtcgcgttttccgtggtggggctgatggagaacaactttgacgcgctggtggactacgacttcacctcctccatggaggacaacctggacgagatcgcccacggcaacggcgaccgcacccgctggctcaacggcttctactacggcgacgccgacgcgcgagagtcgatggccgaggcgatcgcgcgccgcggcgggctcaagcacatgatcgaggacaacctcgagcacatcgacgcccgcgaggccaactcgctgcgcctgttcaacgacgaccaagaccgtcccgtggtggtgcgcgtcggccgctacggcccgtacatcgagcgccagatcggcacgacagcagacggcgaaccggagtaccagcgcgccaacctgccggaatccgccaccccagacgagatcacgctcgagatggcggagcgcctcttcgccacgccccagtccggccgcgagctgggggccaaccccgccaacggccgcatggtggtggcgaaggagggccgttacggcccgtacgtcacggagctggtgcgtgacgacgagcgctcccacgccgaagcccgcgccgaggagatcgtcgccgaggagcgcgccgcggaagacaagcagcgcgccgaggaaggcaagcgggcgaagaactgggagaccaagaccgcgaccgcgcagaaagaaaagcgcatcgaggagctggtcaccgagcagctcaagcccgccaccgcgtccctgttccagtccatggagccggcgagcgtaaccctggaggaggcgctgcaacttctgagtctcccgcgcgaggtgggcgtcgacccggctgacggcgaagtgatcacagcccagaacggccgctacggcccgtacctgaagaagggcagcgattcccgctccctggcgtcggaggaccagatcttcaccatcagcctggacgaggcgcgccgcatctacgcggagccgaagcgccgcggccgcgccgccgcgaagccgccgctgaagatgcttggcgacaacgacgtgaccggtaagccgatgaccatcaaggacggccgcttcggcccgtacgtcaccgacggtgaaaccaacgcctcgctgcagcgcggcgacacaccggagaccatgaccgaccagcgggctaacgagctgctgtccgcacgccgcgctcgcgaggccgaagacggcggcaagaaagccacgaagaagaaggcggcgaagaagacgacgcggccgaagaagaccaccaagcgggtggttaaggcgcgcaagaagtagcgcttaagcccggtccgccatcgtggagcgcaccgggcgggccagctgcgtcatcttgttgcgtccgcgcagctccaccgacttcatgagcgtccagcgctgctgctcaacctcgttggcggcgcgcagggtcgcggcgttggtcaggaccttgcccggggtgtccttggccagctctgtcaggcgcgcggccgtgtttaccgcgtcgccgatgacggtgtactcgaaacggtcgtggccgccaatgtggcctgcgacgacatgtcccgccgcggcgccgattccggcttggaggtcaagcccgtccagctcatcgctcaattctcgggatgcttggagggcgtgcgacgctgcgtcgtgaagcgaaactggcgcaccgaagactgccagcgctgcatccccctggaacttgttgatgacgcccttgttgcggtgcaccacgtcgaccaccacctcgaagaagttgttgagctctgcaaccacctcttccggggtgtgctcgacggcgaacgtggtcgagccgatgacgtcgatgaacaagacggcgaccttgcggtcctccccgccgagctccggcttctcctccagcgccttctgggcgacctccgtgcccacgtagcggccgaaaatgtcgcggacgcgctggcgttcgttgaggccgcgcatcatttcgttgaacccggcctgcaggacgccgatctcggagccgtcgtaaatatccacctgcgtgtcctgctccccgcggcgcacgcggttgatggcgtcttggagctccgtgatggggtcgaccacgctcatgacgccgaacgctgtgccgatggagccggtgaccagcgccatgatggtcagggcgaagaccgcgggcacgagctcgcccgcggtgtgggtgaaaaagccccgcgactgcgcggcgaacagcagcaggatacccaccagcggtacggcggaggtggtgatccacgtcatgtacaggcgctgcttgatcggcggctcgagcgtggagtcctcgaagcggcgggctagcgcttcggcggcgacggggcggacgaggcgctcggcctgcagatacgtcagcaccgccatgacgaagcaggtcaaaagtgtggcgacgaagatgaccagcgccagctgccacgagatctgcagcgcggcgatcgtgatgatggcgatgccgatcagccacaccgccaccacgatcatggtctgcaggaccggcagccggagcacgaggttgcgcaccatgttcgggtcgtgcttgtcagggttttgctgccactcgaacacggggcggaacatcagaagcgtcgccacaaggcccaccacaacggcgaacagcgcgtagatcacaccgatcacgccgatgcccatgtggtccagggtgagttcctccgcctcctccatgggcacgaggaagcggacgaagaacatcactccgagtgcgccgacgacgttcgtgcccagcacactcgcggcgtacaacggccacgacgtgcgcaagagccacttgagccggcgcaagagtcgttccatgacttatcaccttagcgtcgaacatggggtgttgttccgaccgagtagtctttgcaaatgtgacgaaccgaagcccccgcagtgttgctgagatcctcggcgacgcgcccaaggtgcgagacaccatcctggccgcggctgccgcggcacgaggtgtttctggggctgatccgcgcgcgctcgcgcactcttggctcttcaccggaccgccgggatcggggcgctcgaacgcggcgctggcgttcgctgcggcgctggtgtgcactgaccctgacgtgatcggctgcggcaagtgcaaggcgtgccgcgacgcgctcggcgggacccacaccgacgtcgtccacgtcgtgccgcaggagctggtcatccgagtcaaatatgtgcgcgacgagattgtggccaaagcagcccgcttgccgacggttgcgcgctaccgcattgtcatcatcgaaaatgccgaccgcctccgccaggacgcggcggacaccctcttgaaaaccgtggaggagccgccggagcagacaatcatcatcctgtgcgccccgtccactgacccggaggacatttcccagaccctgcgctcgcgctgccgtcacctctacatccccgccccttcggaagctgaggtggtccgcctgctggtggaggaagagggcgcggccgaggacgacgcgaggctcgccgccgcaacgtcgcttcgccacattggccgcgcccgcaagctggtcaccacccagtcggtgcagtcccgccgcgccaacgccatccagctcgcggagcacgtcttctacggctctcaggccttccgcgcagccaactcgctggtgaagaccgcccagaaggaggctatcgacgactacgccgaggccgacgccctcgagcgggcccggctggagaacgccctcggcgtcggtgcgaagggcaagggcgcggcgaaggcgatgtccggcaccgccgcggagctgaaagcgctcgaggcgcagcagaagttgcgcggcacccgccgcaagcgcgacgccctcgacctggtgctggtggatctggccggtgtgtaccgcgacgcgctggtgttgcagtctggtgccggcgttgccctgacgcaccccgacttcgagggactatcgcgcgaggtgggcaaccgcgtcagcgccgaaggcctcgtcgcctgccaggacgccatctcgcagtgccgcgagcgcctgcaccagaacgtggacccgggcatcgccttcaacggcatgctcggccgcatccgccaagcgtgcggcgtgcgctagggccctcctagctgctggtttacgtaggccgtagcgcgtgatataagctttctaaccggtacgcgcagcgtccggccaccttagctcagtcggtagagcatctcactcgtaatgagaaggtcgcgagttcgattctcgcaggtggctctaacaaaaccccagctaaacaccagttttagctgggctttctttttgtctctaacgtttcgcgttgtcccaagttgtcccaggttgtttcttttattggcgcacacagagcgcacacagagcgcacactcggcgaggggtagcgatttggaacacgggcgcgaaaagcggcgttggattagatagagaacggtaaagtacaagccggaaccaggaaggaggcccccgatggcatatagcccccgtgttgtagcgaataacatcctcgctcgcgcttttgaagaaaagcggctcatcacgccaatgaagctccaaaagattctttacttcgtgacgagccagtactccaagaagacggagggggactaccttcttgaggcgccgtttgagacatgggcttatggcccggtggaatacacggtcttcgacgagtttcgaactttttcgaagaagccgatcaccaaatacgccagagatgcggcggggaacactctcgtcgtgaacgaaagcgaagacccgtatctccgtgaagcgctcgacgaagtatgggaggcaactcgggataaaggtgcggtgttcttatccaagctcacccattcggaagactctgcatgggacaaggcgtatcagaatgactgtggcgtgctggatccacacgatatcttcgaagatgacacttaccaggatgctttaggactgtgagcgaagagggcgagatcaaaccgggacggaagcctgccccggaagtgaacgacaccgaagatgagccgatcggtcagattcgtcccaatcgtgagatacggattgtcaggtcgacaccgcctaaaggtgcaaaggcgacgttaactaaagcgcgagccagtgagccaaaaccgcggaattggagagagcagctggactggacccgccacaagttcgcccaacggctggtggtgggggcgctgatcgccatcttcgcaatggcaatcatgcaatactggtggcccaaagaggaacagtccttcaccagcacaataaacattttccaaatcgtcgcgacaaccgcgctgggttacgttatcgggcgatccgaaggaccccccactcctaaggactaacagaccccgggtatcgcgcgctgccgcgccaggcggggatcgaagtcatgcagcgcatcgagcaagaaattctggccagcaagcgacgtctcagccgctaaccagcgtccggcaccgcgcgcaggccgtcgcgccgggcggtgcgttcttcgcgtcgctttgctcgggcagcgtcgcgttcgcgctcggcggcgaggtaggcatccatggcgctcggcacggcgtccaggccctcgtcccagaggtggccgtagatgttgagggtggtggaggcgtcggcgtggccgcacatgcgttgcaccgcgtatacgtcagcgccggaggcgatggccatggagacgccggtgtgcttgagggtgtaggtgtcgacgccttccagcccggcgtctttgcacatctgtgcccagatgcgccgccagcgggcggtggtccagacgttgccgtgctcgtcggtcagcagaggatcggtgggggctttgcccacgcactcgtcctcaaggtcgagcaggagctcgcctccgacgggaacgtcgcggcagaggtggttcttggtgtcgccctcgtggccgagctggtccacagagcgctgcacgtgcagcctccgccggcggtagtcgagatcctccacatggaaccccttggcctcgcccgggcggacgagagtcaagagcaacacccgcacaaatagcttggcctgcggggtcggtgccgcttccagaagccggtcgacctcggacacgcgcagcgcgcggcgcttccccttctcttgccgaacgaggtcaccggattcgagcgggtggtcgtagatgatcttctgcttcaccgcgagcgtgcaaagggcgttgatcacgatgccgaccttgcgcttctgcccagagccgagcggcttcgcttccttctggtggggccgccgcgactgcaggctgtcgatccaggtggtgatcgtcggaccgtccaactcgcagatcggtgttttgccgaagaccggtttcacgtgggcccaggcggagcggtaagacgccacggttgacttcgccttgccctccttggacttaatccacggatcccagaggtcctcgagggtgatatcgcgcttgtccttggtgatccaggtgccctgctcctggccgacggccaccttcgcgcaccacgcttcggcggcatcctgggtggggaaggtctttgagaccttgcgcccgttctcttcccagacagcgcgccagcggttgcccttgccccaccgcgcggaacgcacgcgggttttgcggctggttttgtcagggtttggctttgtccagtcgtcgcggacgtgtgccatgtattcttctccttgtctgatcacccacccccaccccccgggtggttggacacctcataagtcgccccgcggttgtagctagccggctcccgcggggcgcatctagttctttttgatgtcgcgtacggcggcttccagggccgccatgtctttggcgtttacctcatcgtcgagcctctttttataggcgatccactgcgccttggcatgcttgtcggcctgcgccttgctgcggctgcccgcgccggagagcacctcgcgctcgttgaagacaagccacttgtcagtgaggtctttccaatcgctaagcagcatcccttgtcgcttctcggctcgatcttcggcgtagtcgagatacatggtggtcaaacgcgccatctcgcggagctcgttgtcgtggaggtagttctttgcgacgatgacgtctttacttccgggcccgtgaatgctgtcccagtttgtaagccccatgttcttcttcgaggcgtccgctcgctcgaggatgagttcggccgcagttttgccgtgcgccgcgaagtgcagtttgttctgtattgaggcgaagaagcgttgtacgtcggtgctttttgggttgtagtcgtcactggaggcggcgatgacatcgcagattttgcggaaaaactggcgttccgataggcggatttcccggatgcgttcgagcagttcgtcgaagtgggtatcgcgaccgtcattcttcagacgctggtcatcaagggcaaaacctttgacgaggtactcgcggagcacgagggtggcccatgctcggaattggcttccgcgaggaccccgtacgcggtagccgactgcgataatcatgtcgaggttgtagtggttcactgaccgggtttgaccaggtactttcaaaagttgtttgaatgtagcttcctcgccaatctcgtgcgatagggtgacgtccttgatgtggtgggagatggcggaggtggtgacgtcaaacagctgcgccatctgcttctgtgttaaccaagcatcgccatcgaccacctggaggcgtacctgtgccttgccgtcatcggtgttgtagatgactacctcgtccggctgagtcatatcatcgatcctcccgtttagatcttctcgtaaaactgctgtgctgcccccgcattgagcctgtccgctcctgtggggcgcgctttttaaaatttgattcggggtgcttggtgaaggttgatgtcgcggatcctcttgttgatgaaaaaggcgtcagcgatccaccagatgccgaatccgccgacggtcaaggtttgtagtagacccattccgatgttgcctaagtagtagcggtgcccacctaacaatcccaggagggcccaccacaaccatgcgatggtcttatttaccggacgggacgcaccgggtgcggagaggcgttgagagtatggatcgtgattatgtgaagccgcatacgatgcgatcggcggttgctcaccgaaaacgtgtgattccgtgatcggactattcgctgaagacggtcgcctaacgtcagaggcgttggattcgaaagccagatcggaatcgtcgtcctcagtgcgaacctcttggtctaaagaatcgccgttatacgcgtcagggtgggtggttttgacaacggattccacctctggcaacgtaacttcctccgcctcgtccccgtgttgccttgtcgaaaatggtgcttcgtcatcttcgggttgataccgaggcactgcgtcatactctcgagggtctgcttggtaatgaactaggcgcggcaacggcttggtgacgtctgtttccaatagttcttctgcaagctcgtgcgctcgagcggcgacgagcacaatttcagctgcgatagatgagcctgagatcgttgcccgcgatatgacagtaagcccctgtgaatcgaaatgccgcactatcggggcgaacttctccgaagataccttcgacagctcgcctactctctcgccgtctagccggatttcaactgcttcccacttcttggtcttgccagcttcaaaaagatggagcgaaacaagcacttggcccaagccagataaggggacaaagtcagcaagatattctgtgtgctccgactctttcgctacttgtgtcttcgggccttcggggagcaggacaaagccatctgtcggggggtcgttaagtggcaggagcaagtctggatcgggtagcgcgagacttagccaaaagtcccgctcgcccttccaaccaacgttggtccaaacgcgcattgttgcgcctgcgtcgtagccgcttgcggctactcgccgtagctgcgaatacttcgcacattcgtctgatgagatgtagccgacgacgttgtcccaccatcgaactgagatcgcattgccagaagtgctaaacggattatctggttctggaaccagcgtgacgtcaacataaaactccttgttgtctcgtccacgttcaatttggaacatgccttccaaggagcggcgatggtagtgtgcccccttcacttcaaccgaaaaattcttccctgtgagtccaagcgggtacaccggtttgctaagcattcgtaaaatccttcgacagaaactgttctcgtcgggttgcttgccagacttccaataggtggatagtgaccccgagctcggcggcgatcgcgccggggtggccgtcatatatcatttcaagttctgcgtattcctgcgggttaatcagcagatttgctgcgtagaggtccgcgcgcatctcgtatctagattggtgccccgcggggtcgtcgctggctgcgtggccgagttcgtgggccagtgtgtggattcggttacgtggcccgaggccagttcggataaggatcaggcgttcatctgggaaccatccaccgaggtggccacgttgaaggtgctggccgatgtcatcttcaacgcgcacgtcgaggtcctccgctaagcggaggagtttaagctccaggtccgtaatcgtcatcaccttcttccggctcaggcacgcgttcgttcgccgcgtatgagagtgggtactcagtcgcccgattagtcgaacgttcgttggccagctcgtcaacgggcacgtcctcgatcagcttcagccgacgcaacagctcgtccgtgagctgctcgtcagtggcccgggcgagcgcggttagcacgcccggttctgtcatccatcgcgccgacatgaagccgagatcaaccaacgcaattactggagactcgtcgtaagcctcggccactctgatgatcagctcaggcttgagttcgccagcccgcatctggttagcaagagtccggtcgtttatcccagaaacctcagcgaccctccgataactgtcccctcgcgtaactctctgcagccattcggtgtgtttcatgtacgcaacattagtgacgttacgcgcattgcgcaacttttacgcacgttttgaactgcggaaacaaatcaggggcgcattcagcttgcgcaatctaagttgggtgcgtaaaacagagttcagcgcgtaaaggttgcgcgcgccactcggaaaggagagcggatggcaacccgattggaccccaccgtgattgatcagctccgggaaaagcacgaactcaccagcttcgagcaggttgctaacaaacttggccgaacggcccacaccgtgcgcaagtggtatcacggtcaatccactccaagcgcaggagatctggtgaagctgcagttcctgaccggccgaccctacggcaccatgctgatcctccccgacaactcggaccatgccgcgtaaaagacctccacggcatcgccgcataagaaaacccgcctgatagcagcaagcgggtctggatccagaaaaggaaaaccatgcagaacaataccacttcaacaccagcggaggggcgaatggcgtctcgtgaagctctgacggaggaccgtcaacggccatcaggggagcgcaagcgcgtcctcgagttgtccccggagcagcgcagctaccacagggccaacatgacaaaaccgcaaagggcacaagcagaaatgcgccgatccttcgagaatttaggcgaagccctcgacctgttccgatggtacgacgtgaccgggcacccagaggattggctaccgcacgccgtcgaagcgatcgatgggttcttcaccgcgctcctcggtttccaacgcgaggttaacgccgtcgtagcacgcgacccgtacttcgccgccgtccgcgagcggcagcacctcgaacggatcgaactgcatgaggacccgaccgccaagtccgtcttggaggacggcttgcgcttctccgaaggggcgtcggtcgaggcggctcgcatagtgcgccgcatgattcatgcggtcgatgatgcggaaggtgacgtcctcgacggaaagcccatcggcaagaacgaatctcgaaccggcgtagtgcaaaacgacgttactcatgccgccgaagctacctcgcgtgcggtcgccccgctggataacaccgcttctggcctggaagaagggcgctgaccgatggcgtggatcagaacagcaggcagcgacggatacctgttttatcgatcacgacggttcttcggggcaggggtcgagctattcgtcgccgggctcggtgtagaggggctcggcaccgccactttgcaggtccaggacccaataaccgtaccgacgacgaccagaaaagatatccataaagccgtcgtactcatcctccgtgaggggctgcagacactcgggttcagcggcatccgggacatcgaaatagatgtcatcggttggcttaagccagagcaccggattgccaggggagtaaagcttcaccggcacaccgtattgctgcgcgttcacctaggcagcgcgaacatacgcgaaatcccgcaaggggattgggtattcacggtcatcttcgaagcaaagagagaaaacgttgttcgccatgtcgtgaagcgtattcgcaaggcgcgagtgatgcgccgcaccaaccgaagtttcccgcttggggacgctgcccgccgccgggaggtgaagaaatgagcacgttcatcaccgtccgtgagttcgcgcagcgcacgggttactcggagaagaccatccgcaagctcgtacgccgcggcgaaatcaggtctggccgtcgacgcggccagaaaccaggcaggggagtgaagatcctcatccccgagcaggaagtccagcggtttgtccgcatggaggaagtcgcctagagggaattgataacgagggagttcgagcgatgcagtatctcgacttggccgaaagcgcaggccgtgagcgtcagcgaatgcttctgcggctgcacaattcgggcgttgcctcagatgtcgaagaggtggcgacggaagaactggacggtctcgtgaaccgtgaattcggcgttggccatccggtcgtccatcgaccacgccccgtaggaggggacggatcgttgaacccactcggggacatcgaactggattgtccagctgacgtctataccgtcgtctctttgaggcgtgaagccgggtttgatggcgattcgggcgagctccaattgctcatcgtcccggatgaacgctgcgaattgatcgcatatacgcgttcgcgaggcgtcgatagcgagagacggaccgttgaccttcagttcgatcacgcgccaagtcagagagcgtccacggcggtgccggtcgagtcgagcaagctcgttgatccaccacagagcgcttccgaggtggccacctgtcgagtggtagggctgcgtggcttcgatgagttcgcgcatccgctcggacaaagcgctgggtatccgctcgtggaaggacgcggggctggtggtcatcgggtacgacagtctgccggcgttcggtgggggatcggtggcggtgtcgtagacgacgagttcatagaacagtccgtcgagcgcggccctcagattgtaaagccactctccaaacagcacagacaaggcaggagggaaggggtgtgtgctttcgaccatgatgatctgctcatctgggcgtcggtcgatgtgtttcaccaccgggtgggcctccagatgttcggacgcgatgtgccacatctcgtctcggtgcgccgtcgcgcgctgaactcgctcaaggaggacatcgaaatgtttgttctgccccataagacctaggccgctttccgtgctcgcaactacctcggacgcacacaagaaatctgaacgaaaggagtgttctcgatggacctgaagtgcagccagaactttagcaccgcacagatggtgtcaaaggaggaacgcatgctcctgcagctgtaaccgcctcgagcccgtccatgccaggtggtctggcacgactcatgtccccctcgcgctgtaggtgcgcaccggttcgagtccggggacgggcaccaggagacgtcgcggaggaatttctgctcctccgaaggacggatccgcgtcgcgaagttcgctactccgtcgttcagacgcggcaaggcgtacttgcgtctcccctcaacctcaacaaccaggagaaaacaatgcaacagctcttcaccgaccccacactcttgaccgtggccatcaactccgcgcttgacgtgtgttggccggtcctcccgcagcccatcctcgaccagctggcgtgggtgtagccatgagcgacctcactgccatcgccaccgccgtcggcgtcctggagagcaacctcgcctgccgtcggcgcccaccactcgaccacatctcgccggcggcagcggcacttcggcacgcccagccggaggaagacctctacatcccaacggggaaggacttcgccgcggccgtcctggccatcttcaccttctggttcttttacgtggccacatgggccgtgtggggagcgtaagaccatgccgcaattcaacgccgaactctacgcccgcaaccacgccgacaaagcggcgccgcaaatcgtggtcaaggtcgtcaccgcttggctcgctggcttcacgactgccagcgtcgcctttgtcttgatcggcctttgggcgctggggacagcatgatggccgcaccaaatccaggtgatgttgccttccaggccagggcgcgcgagatgcgccggcgacttggcgatatcgcggacgccgtcatcgaggtggaagaagtcttcgcccacttccagaaccgcgtcgacacgcaaactgccgcactgctcacgctcgcagcggtccttcaccaccaaccggaggaagaactatgaccacccagcaagaactcattcgccaagcgttccccgacaaagaagagcagcgccccgttgccacccgctcggacatcatccgcgaactattaccgctcgtcggagacctccgggcttcgcacgcccacgtcctcgacgagaacaagcggctgcagaacgaacgcgacaccaagtccgctctcgtggccaccctcgaagcagcactcgccgctacccgcctacaggtcaaggaactcgagaggcaggacaacgccgccgagaacacgcgcctggcgaaggaggtcgtcgcgctcaagaatcagctcgccggtgctaaggccgacgccgccgaagcccgccgcgcccgccaagccattgacgaaaagctgaagcgcaagaccgcagaccacgacatggccactaaaacacttctcgccaacaacgacgagatcagaaaggccctcgagcaacgagatgtcgccaaagccgaggtcgaccggctccaaaaagattacgaggccgcgcgccaagacttcaaggagatccaggccgacaacaacacgctcaccaaagaacgcgacgccgccgaagcagaggcgcgccgggttaacgccgagatgctggacatcgttacccgcgagaggcaagtcatcgaggagaaccaagaactcaagtcacagatcgagcagctccgcgaagcggtggccacgagcgagggtgcccccccgcagagcggccagacggtagccgaggaagggcttcgccggcatctcgagacggccgtcgcccagttcgaggaggccccagacaagtcgctccgcgccatcactcgcgccctctcccttctgaaccacccagccgaaaaggaaacgaccaatgagtgacctctacgcagtgaccttccacaacccgaaccgccactaccgcgtcctccggctaagcgaggacgaggcccaacgctgggcaaacacgcttagccacttctcgatcgacctgccgcagttcccggcccacccgttccagatcgcacccatcgttgaggacccggacggcgaagttcgctacctcggcaagcagtaccgccgcggcgcagccctcaaggaaaaggcggtggccaatgcttagcgccagggaactcgagctggcacgagctacggtcgccacgcttgtggtgtgcctgctcacctttgtggcatcggtggccacgctcgtcatcaacttctccgaagcccgaggttcgcagcgctgcccgtcagatcacgtgtgggtggacaccggggagataccgcaggccggatgtatgcccctcggcaccgcccgcgagctaggagcgtggccatgagcatcaacctcgcagacctcacgcccgagcagcacggcgagcacgtcggccgctggtgcgagctcaaaaccaatccgggcgtcctcgccatctacgaggggccattcctcggcggacgggtgaaggtcccgttagaagtgcacccgctctacgtcgacccggagcaaatcatcatccgaaccgacctcccccgggcctggaacccggacgggtcaccaccgaaggagccgtgatgtactcctcccacgtctacgactgctcaccgcgcttcaccgccagcgacggacaaccgaagagcgttagctccaaagccgacgacctcatgcgactcatgccacgaggtgtccgtaacgcgctggtgcccctggccaagggggagtgtggcctcgacgacgtcccggactacgccctcgaatggctcgaaaagcacgaagcgattgcacctgcccgaaaagcgggcattacctggaagcacggtccgaagttcaagaccttgctccaccgaatatcggagcgacacaaatgaggagggcgtggtgtcaacgatgcggcgccgaagcctgggaagtgcaagggcaatccgggccgatactcgtcgagagtaaaaccggccgcgccggggaccttgtccgggtcaagacagccctcgccgagggcacctcggtctcgaactggtacgtccaccgctgcatagaggttaagtacccgccgaaacgaaacactgccgccatgaaccgagcgctgcaggtcgtcggcctcgatccgatagaggagcggggggacagtgcgtgaacgagacctcgacgactggtgggcagcccttccgcagaagcggaaggcccagatccactcctggctctcaaaagatgaagacccaggcgaactacccaaccaaatcccccttttccagaagggacaggaacaggaaggagaaaaactgtgactgactcaagcttcctctgccgcatggacagcctcgccttcgcactcaaagcagccgtcaaggtagctggcaaagacgagctcgccttcgtccgcctccaccgcctcaacgaggacaccctctcggtctccgcgctaggcaacgacctctcattccgcgccaaggtcaaggtcgacttcatccactggaacgacgaccgcgacgaccgcgtcgagatatccaagcacgccgccaactcactcgccggctaccaagtcaaaacgcccgaggggctagacgtcgaaccgctcgtctcgatccaaatcggccacgagcgcatccgcgtcgaggacgccaccggactcttccaaacagccggcggccgcgacgaacaccggctcaaagacccgatcctccccggcgaccacgagaaaatcttctacgacgccgcaagcgcaccgggcgcaccgttctggataacccccgaggccatcggcaccatcgcaggcgtggccaaggtgctccaccgccgaatcgtcatgctcaaacgctccgaaccggccgagttcgcatcccgctggtacgtcctcggcgacgactggcagatgaccatctccaacaaggagaagctccgccacaccgagccggtggccaccccgcccgccggagacgacccggagcagaccgccctcccgccgcgccgaatgctcgcactacccgtcggaggcatcgcatgacatacccccagaacccagtaacgctgctcatcaagcaccgccatcgggctgatcccgagctgctccgggcaatctcccaaccgatgtttgacgccgcccggttcctccaaccggccttagaacacttcaaggaccgcggcatacacatcccatcaccactggaagaagagtgccagcgagcagtccaggcctatttcaacgagcacgccggtgactttcactcgacatggccattcgtcgccacccgcaccgggcagacaggtcaaagttgatgtcaggcacggtagaacacctttggggcctggagccaggcgacgagaccgcggcactgtgctggtacaaacgccagagcaccggcgtttcgccgtgggacggttcccacccccgcgaatcgaccaaagaagtccttgtacgccacgaggaagcccgcatgcggtgccaccgctgcccgctgctcgaagcgtgcgaacgtgcgctcagcgacatggaaaagcagaacctccgtgtggacggcgtcatggctggccggtactccgacgtcatcgcgtactccagcggagagcgcatgttcgtgcagaccacgtgccgcggctgccgcgcacccctgcggccgcaaggaggtgtgagaaatagtaggacgctccccgccggagcacgcgaccatcggggcgaaggactatgcgaccagtgctacccacggctcgcgcgggcagtgcgcaacccaccgccaccaataccgaaacgctcataccaacagaacaatcccatcgggacaaccccatgactgccactacgagacgaagagaggagttgcgcacatgccctggctacggatcggcgacaacgccaccacccacccactcatggccaaactcctcgtcgccaccaacctcaaccaccaagaaaaaaacgaagcattcggagtcctcgtccaactcgcctccgtctccgcaggacacctcaccgactacctcgtcgaatacggatccctcgcccaagtcgcgccgggccgtgagcgcgaggtgctcaacattctcaaaaaggccagccttgccaccgaggtggaggtggacggaaacaaggtcatccgtcttgttattgatgatgaggaattcgttcatgcgaagcgccgtgaggaagtcgagacagaccggcgtcgtgcgcgcgataagcgcacacccggcctgctcgcccaggtgcgcgtccgtgacggcgatagctgccgctggtgcgcgaagtcggtcagctggaaaaacagatccggtttccgcgccgccacctacgattcgctcaccggtcataaagacagcaccgtcgacacgctcgttgttgcgtgtaatccctgtaacaccaagcgaggcaatggggagaagctgaatctactcccgccaccacccccagaaaggctaatttacggccagcagacagtagatttcgtcaacgaagacaagtggtgccaagaccacggcatccgtatcgagctcacccagccgacgctccccctcgaggaggacccggcagcagcggccactaggcagcagcaggatgagaaggcagcagcgcccgaagcggcagcagcgccagatcaccgagcagcgccacggcaagcagcgccaaccttcgacgaggacgagccagcttggctccgtcagccgatctccgattttctatcccgccccgcccccgcagcagcgcccaaagcggcagcagcgcgacccggcgatgaggcagcagcggccactaggcagcagcaggatgagaaggcagcagcgcccgaagcggcagcagcgcctgaccaccgagcagcgccacggcaagcagcgcccaatacgatgacaggcggcgagggtaacgaaactgtaacggagttagaacgcgtcctaggacgctcgggtgacggacctgggaacgtcgggtcgggtcgggtcgggtcgggtcgggcaggtatggcgcgtaagcgccgaaggcgcggtaggcgaggagggaagaataagtgagccttgatgatttgggtaggcacctgtactggttagagaccgatggagatcttcttgatgatcttcttgttcctcgtcggccgacttccggtgagaatgctgggcgagctcctcagcggggcaagtcgaagcctccggtggtgctgggcatagtggacctcaaggcggacgtggaggaagtgctcgggtactggtgcggtcagttggtggcgtcggttcctgcactaggggcaccgccgacgactcggcgtatcgctgcgcgggcggggtggttgcgtggccacgcccctgaattgttggcgatgccgtgggcggagatgatggccgatgaggtggcgtcgcgggcccgcttggtccgtgacgtggtgtcaccgcctgcaagagcaagcgacccggagccgattgaggagggcaccaccagggaggttgaatcgtggttgcgtctgctcggcgtgcctgcgagtcggacgtcgctgcggcggtggatagatgccggcgaccttgagtgccgcatgctcgatgatgggcgtcgcgttgtgcgtttggctgacgctgttgagctggctaaacgacgtcgattcagtggtggcccacctagcgttgtaagctgacgctcgaaagagctatggccccggtgacgtgaagttccggggcctttgtcatgcccgcgggaggtgagcctttggcgtgggatgaccgggcgacgaaggagcggcgcaagcagttccgggcggagcacgaggctatgcagtcagtgtgctggctgtgccgccagccgattgattacaccgcgccggcgcagtcggtgaacgcgttcgagccggatcacgtcttgccgcgttcgacgcacccggagctggaagatgacccggagaattggcggccgtcgcacgcgtcgtgcaaccggtcgcgcaaggatggtgctccgccgccggacctcggttcgtgctcggagcaatggtgaagggggaggggccttgagatcgctggcgttcgcgcgcggccgcctgcgggcgggtgaggaggcctctctccccgcgaggtatcccccctagggccgaggccggtagcggggtcgagttgtggaaatggaggttgaccgtggacaacgtttccgagcgccctgtgggcgagctagagcaggcgtttctcgattcgcttgcggcgctggacgagcaaccgcccgccgagtacggcggcgtcgtcgccctcggccgggcgtacgcggagaacatcgacgagtcgcgctcgacagacacggagacggcgacgaagtcgctgtaccttggcccgcacctgctgggcgtgatgaagttgcttggcctcgctccgaccgaagcgccggagactgccgggacgaagaagggcggcacaaccagcccggatgtgatcgacattatgcgccgcatgagccgcgagacggccaaggagaatggggcgtaagggctgtaccgagccgcgtttctacaccccgccactgcgggagctcaccccggagacctcgaaaggattcgaggtcattgagttcgccgagctgctcggtattgagctgtacccgtggcagaagtgggtgctgattcacggcctggagctgctgccgtccggcgagttccggttcaagacgatcatcgtggaggtggcccgccagaacggcaagacgctgctgatggtggtgctcggcctgtggcggatgttccagttcggcgcgtcgcgcatcatctcggcagcgcagtcgctcggcgacgccgaggacacgctcgacgaggcgttcgcgatcgcggcgtggaacccggtgctgcgctactttctgccggacaacccgcgcgcggacgaggaggacgacgcctacaacggcgcgtaccgctcccgcgccaacggcaagccggcaatggagctcgcgctcgcgccccggccggaagcgctcgacctggccggcaagatgccgatctggtcgctggcggtgacctcgcgtaagggcggccgctcgaagtcggcagacctggcgctgctcgacgagctgcgcgagcacctggactgggaagcgtggaacgccatcgtgccgacctcgcgtaaccggccgcagtcgcaggtgtggggcttgtccaacgccggtgaccttcgctcggtcgtgctccgctccctccgggaatcggcgatcaagcagattgacgacgggacgtcggacgcgagccgcacggcgttcttttcttactcggcccacccggacgccgacgtcctcgacccggacgcgcacgcccaggcgaacccctcgatgggctactcgaacctcaccgaagaatccatcatggccgaggccaaggacgcggtcgccggcgacaacgaggccggcttccgcgccgagtgcctgtgccagtggcaagacgtgctcacccccggaaagatttccctcaagctctgggaatcgctcacagaccccgcctcggcccgcgcgccgggcgcggaggtgttcgtaggcgtcgacgtggccctggacggccgttgggcgcatgtggccatagcgtcgcagcgtgaggacggcctgtggcacgtcgagatcgtggccagccgcgccgggtaccggtgggtacccgcgtggcttgcggcgcgcaagggccgagggtggttctccgggacggtgggcatgcaggttcgcggctccgcctcggcggcgctgctgccgctactgcaggaggccggcatcgacgtcgcggagtggcagggcacggacatgtcggcgtcggtgctcggctttgtcacggaaatcaagaaccgcggtatccgccaccgcgaccagccggtgctgacggtgtcggtggaaggcgcggtggagaagcgccgcggtgacattttcatctgggatcgcgagaagtcagcgaccgacgcggcgccgaccgtggccgcgaatatcgcgtggtggatggccaccaggcacgaaacgacagtgacctcggcgtacgacgacgaaaactatgacgcttccgcgcaggagctcgaaaacgacgagccacaggacggcgaggactttgacgacggcggactgatgttcgtctaaggaggtggtgcccgtgggtatcttcagcaggttattcgggcgtctcgaagagactgcggccatcgtggccaactccgacgacgagtacatgttctccgccccgatcttcaccgctctcgcccgggacgtggacaagctcggcgctgcggagctctacgcccagcagccgcacctgcgcacggtggtgaccttcatcgccgagcagatcgccgcggtgtcactgcacaccttcgagcgcatgccggacggcggccgtgagcgcgtccgcgtcggcgacgagaccggcgacaattcgctctacgctgaccgcccaggccttgtgccgctgttgatgcagaagcccaacaagcaccagctcatgcaggacttgctgcgcgcgtccatcctggattatctgctcttcgacgagttcatgtgggcgatcgacgaggcacccgacaagctgccggagatcgtccgcatcccggtgtcctggatcatcggccgcaagtgggaagacccgtggacactcaaggcgatccgcatccgcgacaaccgcggctacgtccgcgagtacagcggcgaaaagctgatccacgtccacggctacaacccagagtacgaggaaatcggcgtctctccggtggactccctgaaggagactctccgcgagcagctgcaggccgcgtcctaccgctcggagctgtggcgtaacggcccgcgcctcggcggcgttatcacccgccccccggaaaaggacgtcggcaaatggtcgccggagggtcgccgtcgctttaaggcgtcgctcgcggcgcaatacagcgccggcggctccaacgccggcggcaccatggtcctcgaagatggcatgaagttcgagccgcagcacctcaacgccaaggacgaacaactaccggagatgaccaagctgtcgctctccaccgtcgcgcaggtctaccacgtcaacccaaccatggtcggcctgctggacaacgccaactactccaacgtccaggccttccgccaaagcctctacgttgacagcctcggcccgctgatcaagcagatcgagggcaccatcaactccttcgtcctgcccatgctcaaggtcgacgaaacccgctactacgtcgagttcaacctcgaagagaagctgcgcggcaacttcgaagagcaggcagctatgcagaccgcagccgccggcggcccgtggatgaccatcaacgaggtccgcgccatgcgcaacctcccagccctcgaaggcggcgacgacctcattcgtccgctcaacgtcaccactgccaccgccgaccaaggcgagccgcaagacccgccgccggcactcaaccccgcgccgggaggtgacccgccatgatccacgtcgtaatgggcccgccttgctccggcaagaccaccttcgtcgagaccaccgccgcgccgggcgtggcccgcttcgacctcgaacaggtcgcgtccaccatcgccgcgcaaccagtggcagacaccgcgccgggcaccgtgctcgacgcggtgcttgctatgcgccgcgggctcaccgggtggctcctcgacgtcgagaccccggtcgaggagttctggctaatcaactcccgcccacccgacacccttattgccgctctcgcagctcaaggcgcgcagttccacgtcctcgacccgggcgaggaggagtgcattgcccgggcgatccgcgccgggcggcctgattcaacggtggagcggatcaagcagtggtacctcaacccgccggagataccgggggagaaaggagacaacgtgaagaccaagaccatcactgttgggctcaaggcaacccccgacgacgtcgacatcgtagatgccggcaccttcgagggctacgccagcgtgttcaacaacaccgacacctacggcgacgtgatccgaccgggcgcgttcgccgagaccatcaaggacttccaggagcgcggccgggtgattccggtgctctacggccacgatttcagtgacccgttctcgaacatcggggctgtggaggaggtcattgaggacgaccacgggctccgggtgaaggcaaggcttgacctggacaacccgaaagctgcccaggtctaccggctgatgaaggcaaagcggctcaacgagatgtcgttcgcgttcaacgtccttgacggcagctgggccgagatcgacggcgaggaagtctacgagatcaaacgcgtgaagctcttcgaggtctcggtcgttcctatcggcgcgaatccgcaggccgaaattctcaccgtcaagcaggcaaccgaagcgctggtgaccgctgcgaagcaggccaacccagcagttgccgagtccgtggccaagcacgcgggctccatcgccgcgctcctggaccccgccgccgaaagcggcgcgcaggtcccccaggagccaaaccacgccaaagacggcgacgtcgccgtcttcgaagcaaccgtccgattcctcgaaaggaagcactatgtctaagaccctcatggaaaagcgtgcgacggcgatggacgccgtccgctccgcactggctaactacaaggccaacccgaccgacgacaacctccgtggcgaccttgagtccgcgatcaacaccgtcgacgagatcgacgccgagctgcgcgccgccgaaatcacggtcaacgcggagaagctgctctccggcgccacgttcgaggccacccccggccagaagtcggccgagccgcacacgctcggccaccacttcgccaagcacggcctggacatggtcaagcgccagaagaacggcgaacgtctggacttcgccgtgccggagttcgaagtcaaggccgccaacgacccgatggtccgtcccgccgccgacgccccgctggcggggtggggcaccacttttcagcgctccatcgtcaaccagcgccgcgagcagctggttgtcgcagaccttatgggatctgcctccgtctcccagccggtaatcaagtacctcgtcgagaaggcgaagcgcatcgtcgagggtgcgttcaccaccgtcgccgagggcgcgcagaagccctacatccgctacgactccttcgacgttgtcaccgagtctctgtccaagatcgcggccctgaccaaggtctccgacgagatggcggcagactacggtttcatcgtcgactggatcaacaaccagctcgtctacgacctctccgtcgcagaagagttccagcttatgcagggcgacggccagggctccaacctgcgcggtctgctcaaccgcgagggcatccaggagttcaacatcgacgccgccgaccccatcgagcagctcaagggcctgtacgaggcgtcccgcctgccgggccgcgccacgaacctctccgctgacgcgctggtgctcaacgagctcgactacggccgcatgcgcctcgcccaggacaacaacggccagttcctcgccggcggcccgttcactggccagtacggcaacggcggcgtcctgatcaacccgcctgtctgggggttgaagaccgtcactactaacgccgcggtgccggagggcacctacgtggtgggcaacttccgccagggtgcgaccgtgttgcgcaagggcggtgtccgcgtcgacgccgccaaccagaacgagcgggatttcgaggagaacttgatcacgctgcgcgccgaggagcgcgtcggcctgatggtgccgctgccggcagcgttcgtcaccggcaccctcggcacgcctggggcaggtgcgtaactcatgagcaggctctacccctaccgggtcaacaccgaccagggcccgctcactatccgcctcacggaggagaccgcagccacccgctacccgggcgccgtccgcgtcgccacgggtctgccggagaccaaggaatcccccgacaaggagcgccggccccgcaagcgcaccccgtcgcagtaatagccaaggagggaccacaccatgaacaccaccctggaccatgggctggcccccaacccgtcagccgccgtcccggtcacgcaagcagacattgacctcgccgttgaaacgctgcgcgacctggcgggctggcatatttggcccgtgcggcaggagaccgtcaccgtcgacaccgccggagacaacgtcatcttcctacccacgctgcggcttctccaggtccacgcactcgccctcgacggcaccccggttggcctggacaccatcgagtggtcagaatccggaatggtccgcctcaaacggcgcagcggcaggggattccgccgcgccacagcgaccatcacccatggattcgacaccacccctctcgcgggcgtggccatgcacatggccgcccgcgccacccaacccggaaccaacatgacggtcggcggaatctcggtcggcgcgccgggcgcaatgacgccgcagtcttctgagtggcgtctgctcgaccgctacaagctagggccgatgccatgaccgcctcgctgatcttcaccgagcggatcaccatcatccgcgcccgcatggcccccggcgaatacggcggcctggtcgaggattgggagcaggcagaggaaatcccttacccgcacccggtatcagtccagccggtgacctcaaccgaagacgcggacggacgctcgcacctcgtgaccgaccgctggcgggtcttcaccgaaccgccgcacctgatcgaggaactccggcccaccgaccgcatccgtgtcgacacctggggagaggtcctctgggccgtcgcgcgcccgctgcactggcggacagccatcctgccgcactccgaggtcgacctcgaagtcatccgcggcgctggccaatcctccggcaggaggcgctagtggtccgaatcaacatcgacaccgacgcgatcttcatgcaagtcatgggatccgaaaaagtccaggccaaagtccaggaaaaagcgaccagaatcgcagcactcacccgccgcgaactcggccgcgccggcatcgacgccaccgtcaagatcgaaccacacccgacgcccagcggccgcgccgcgttcaacgtcgtcggaagcgtcacaagacccgaagacgccagaaaagcaggccgcatagcgcgccgggtaggaaggagtctgcggtgattgacgagcttcaagaggtggacatcctcaagatcgcgctcgacgcggtccgcgaggtgctgccggacggtgcgtgggtggctgatcggctcccggaggccgaccggctcaccgagagcttgccggcggtggtgattgatctgctgccgggggaggaaaccgtgccgtggggcggccgggatagcccgtcgctgctcgatgcggtgcctctcgacgtggaggtgtttgccccgtcgcgggcggaggccaccaagatcggcgtgaaagtgcggcaagcgcttcaccagctgccctacatcgagggcactggcgtcaagcacgtcgattgcccgcgcctcgcaacccgcgaggagctgaatccgtatgtgaaagtcctcggggttgtcgccgaccttggcgtcgcaccccactaacccgttccagccctgccgtccggtggggctttacctacgttcctaggaggaattatggctaagcagtccactctgcagggcttcaacgcccgcgctgcccgcgtcggcatgaccggagctatccgccgagccgcactcggcaccccggttgtcccgctgggcatcaagttcgacaccgagacccacaccaacaagggctacacgtccccggacggcctggaaatctccttcgacgaggagaagcaggagtacatcccgtggcaagaggtctccgcaatccgtaccgacatcacgaagtccgtgaagtcgatcaagtacaccctctgggagaccaacctcaagaacatcgccgaccacctcggcgtgcgcgaggatgacatcgtcttcgacaacaacggcaccgcgagcttctacgaggacgccctgccggtgttcccgtacgagcagcaggtgttcgacgtggtcgacggcgatacagcgatgcgcctgacggcgttcaacgcccagctcaccggtcgaggcgcaatggtgttcaagaaggaccagatcttcggcctggaacagaccatcaccacattccccgccggcgccgagtacgaagacgtcgactctgcggcagtaggccggacggcgcactggcagttcaacgatgcgtgggccaagggcaaggacgccacgtcctccaccacggacggcgtgcgcccgctgaccatcgccaccgccgcgactctcggctcctcgaagcccgccgtgtccaagaagatcaccgccaacggcggcacgtcgccctacacctacgaggtctccaacggtgccctgccgaagggtgtgacgctcgacgagaagtccggcgagatcaagggcaccgcaaccgagtcgggaacgaccacgttcaccgtcaaggtgactgacgccgcgggcctggtagccagccgccagttcaccatgaccgtcaccgagtaagcgaccactagcaggggtggggtgcgggaaagcaccgggcaggctcgcccgcacccctgcctacccacccgcactaaagagcctgccccatagctttcgaaaaggagccagccccatgactatcaacttcaacgagatcgtcgagcagcgcagcgaagccaccggcatcgcaggcgatcgaatccccttcgagttcggcaacaagaccttctccttccgcgacccgctcatgctcacggacgatgagaaagatgagctagagctcatcgactacgacgctgacattgccgcctggtacatgggcgacgaagaatacgacgaattcctcctgaccgaggtcgaaatcccggcagaggacggcaagaccatcaagaagaccggctcgtccagcttcttcttcctagtgctgcgcgagcacatgcgcaccgcccgcgcctcggatgcggagggaaaccctacgatgcgcaatcgctcctcgcggcgtgcggaggcgcggaagcggcggaagcagcactagagcaggcctacgggtgggatgtgctcgccgcgtattggcgcggcgaaatcactctccgtaagctccgcgtgcttatcgagtacctgcctgacaactcacccgcacgctggcacaccacggacgggcaaccgttctccactgctgacgccattgggtggcgctccctttgggcgctcgccgctatcgctcagggcatggctggcaaggaccagaacatcttcgacaagatgccgcaattcccgtggaagaagcccaacaacccgaatgcctacggctccttcggcgaccacacgccggaagaagtcctggattacctcgattcactctaaggaggaccagccatgtcgaacgcagtatgggtgcccgtcaacgcggagatgaagggtttcatcggcaccctcgtcaaagaagcctctggcgccgcgcggcaggccgggcagaaggtcaccgatgagatgggcaaggccggtaagaacgccggcgaagccctcgccggcggcctcgcatcgcaagcggcaaaggtcgagcagatcacagccaaggtggccaacgcccgcaaggtcgaagcccgcgcggccgccgacgtgatcagcgcggagcaagagctccagaccctccggggccaggccgacgcctccgcgtcgcaaatcgccgcagccgaggaaaagctggctaccgcgaagaaccgccaccaggacgccaccgtcaccctgtcgcgtaccgagcaagacctcgaatccgtgcgcgccgggggagaggccacttccacggcgttggcgcgtgcggaggacaacctcgcccgggcgaagacgcaggcgcagactgcggcggacaagctgcacacggccgagctcaagcttggcgaggccaaggagcgccaagcggcgcgtgcgcaggctgtccgcgacgccgaaatgaacttgattaacgtgcgcgaccgttacggcgccaatacccgcgaaacggagcgcgcggagcggcagctgcagacggcgaaagatcaggctgcggcttctgatcgacgggtggccaccgagaccggaaacgtcacgaagaagcgcgcggagctcgcctccgcgacggagaacgtggcggcaaagacccgcactcacaaggccacccagcaggatgtggctgccgcagagcgaaacgccggcaacgaggcggagtccgctggtcgcaagattcgtgggcttggcgaggacatggacggcgcgtcgcgctccggtggcgggttcatgtcctcgctcggcggattcgccaagaaggcggctctcgccggcggcgcgttcctgggcgtcgcctccgctagccaggccctcggcggcggctttgagcgactgaacaacctgcagcgcgccgacattatgttccgcaacatcgggctgtcagcagatcagactgccacaaccatggacgacctcaacgacctggtcaccggcactaacgtctcgctcgcagatgcggccggcaccgcctccatgctcatgcaggccggtgtcgaggctggaaagcccctcaacgattcgatcaaggcgctaaccaacatctccgcgattgccggcggctccgccgacgacgtcggcatggtcctcatgcagatcaaggccgccggccgcctcatgggcggcgacgcgatgcagctgcagcagcgcggcgtcaacatctacggctacctcgcggactccctcggcatgagcttcgaggaagtcaagaagctcggcgaggaaggcaagattacctacgagcaagtcatcgacgcgatcaacgcgaaaacgggtgatctggctaaggagatgggtgacaccctgccggccaagatgggcaacttcaagacggcggtgtcttccgcagcagccgagctaatcaagcccttcatggagccgatgacgcgcggagtggagacgctcacccagaaaatcaaggacgcgaagcccgccattaccgagttcgccgaaggcgtcaagaacgtcttcacttggctcggcgaccacccggcggtcatcgccggcatcgccagcggcctggcgtcgctcgcggccggagctgccgcagtcaaagccgtcggcatcgcgaaggaagctgtcgccgccgcgcgtggcattaagaccttcgcggacatgatgaagatattgaacctatcgttcctggcgtcgcccgttgggcttgtggtgaccggcattgccgcacttaccgccgggctgacctacttcttcaccaagaccgagaccggccaggagctgtggtcgacgttcatggacgggcttcgctccgctggcgagtggctgaagggcacttttgctccgatttttgagtacatcggtgacgccgtttccagcgcgttctccgtggtcgcggagaaagtcgatgccgtcgtcgacaccgtcaagggcgtattcgaggtactcttcaacggcaccgttccggacagcgggctcttcggcatcagagacgaatcatcggcgctgttcggaacgctgatcacggtccgcaataccatcatcacgctcaaagacgccgcagttgcagcattcgactggatgggcgcgaagtggcaagagttcacgatcggctttggccagttttacaacacctgggtctcgcccgtagtcaccttcttcaccgaggcattcaatgtgatcaaggaggtcgtgggttcgacagtctccgtcattagcgagaacgcccgcatcttcggcgacatgctcggtctggttttctctggcgtccgcgacgccttctcggtggttggctcggtgatcacctcggtggccaccgctgtgatccaaccggcctggaccttgatacagatgggtgcccagatcatgtggaccgtcctgcagggcgtcttccagatgatccagaccggcttcgagttcgtgggcaccatgatccagtccgtttggacaaatatcatcgcgccgacttggggcttcctaaaggaagccgcgggattgctcgccgacgtgctgacgggcaacttcgagaacatcggcaatcggttctcgtcgatgggtgacttcatctcgcagatcgtccaggggccgatcaacgtggcgatggatcttttccgcggtctcgtgggcttggttggtgatgcttggcgcacgtttcagtccacggtctcggacgtggttgatgtggtcaagaccaagatcaccgagatggtcaacaacgtccaggagatccctggcaagatcaagtcgatctttgcggatgccgggcagtggctgctgtcagccggtcgcgacatcatctcgggtctctggaccggtatgcagcagatgtgggacaacatgaccggatggctcaccagcctgccgggtcgtatccgcaacgctgtcgggtcggtctccttcggcttcggtggcgggtcctcgaacgcgaatgggtcgttcgcgcagtacgtcacaggcggaatcgccgcggcagaagtgtacgcgaacggcggcggcaacctgccgacccaggcagtcatcgaacgcccgcacggcaagcgcggcctagtccagtgggccgaagctgaaaccggcggcgaggcgttcatcccgctggcaccgtcgaagcgtgagcgctctgaagcgatcctcgagcgcgtggccgacaacttcggctacgcgttggtggactccaaaactggtgtgccgtaccagtccaactaccggggctacttgggcccgcaggtcgtcggttccttcgcagatggcggtatcactggcgacgatttgatgaagttcctgcagggtgggtcggtcaacggatatcaggctgcgtacccgctggagggcgcgaagtatctctgggccgggcagcacccgtactggggtgactgctccggcacggtctctagtgtcacctcgctcgcgattggggagaaccccgcaccgcgccgctacgcaactggttcccagggttcgtggctttcttctcacggcttcctccgtggccgcggcggcgagggcgatctgcgcatcggcttcagaaacggcggtcctgcaggtgggcacacgtccggaacgctgccgaacggtgtgaacttcgagatgggcggagccagaggcaacggccagctcggcggtcgcgcggccggtgcatgggactcgtactacaacgagttcttctacttgccgatgcaggagcagaagtggctggacccggaagtcaccggcctgaaggatctatccgccgatgagcgccaggtcgtggtcgccgcggtagacaccgcggagctctccacgtcgacgccggtgcagcaaggcccgcagacaccgtatgaggcgttcgctacgacgttcgccgccgagatgggcaaccgcaccgttggccagattggtttcgacgccgtagcggacttcttcggggtcgacccgaaggcgacccgcaaggtgctgttcacgccgatggacgagctcctcggcgtggccgacgtcaaccagaccgccgcggtgggcaacccgtccaccaacgtggctggtgcacatgctgcacagcttcacgacgaagcactcacgtcgatgaccccggcagagctggcacgcgacccgcagttgtcgcaggttaaggacgcggacgtcgtgaagcagccggacgtgcccgagtggggtccgcagttcttcgcccacgagatagctagccaggcgaagtcgatgggcctggacaagttggccgcacagatcggtatcgccaccgccctggttgagtccggcaaccccatgaagatgtacgcgaaccgggccgtcccggaatccctgtcgttccggcatgacgcgctggggagcgatcacgattcagtgggcctgttccagcagcgaaacaatggtgcgtggggctcggtgaaggaccggatgacgcctgcggagtctgccggcatgttcctccgcaagctgagcagcttcgactaccgggccatggcgcccggcgacgcggcgcagcgtgtccaggtcagtgcgttcccagaccgctacggtcagcagatggccgaggcggccgagctgttgtcgaatactggcgtgttcgaccgtggcgggctcgcgcgaggcctcggattcctgcgcaaggcgaccatcgagccggaggaggttctttctcctgcgatgacgccgttgttccgccggttcatcggcttcttgccgggcatgatggagaccattgacacagcccgggcggagctgcgcatcgcggccgccggcggtgatgccggatatggcgccctggctgagctcttcggggcgcaggtcggctaccagctcgcggattctgcgttctgggcaggcgggctggttgaagagctgcaggaggcgttcgccggcggcgacttcgggtatggctctgctgcccacattttcggcgaggaggccggacgtgccctcgtggatgaagccagctggctcggcaccgccgtcgaggagctcacagcagccgcgcgcggcgaggacttcggtctcgcggccacggcacgctacctcggcgacgaacgccttgccgcagcagctctggacggcgtcggcgctgccggcacaggctttgacaacgcgttccaggcgctctctggagtgcggcaagttgcacagcgcgccgggtcgaccgtggtcatcaacatcgatggccaggaagtcatgcgccgccgcctggaggacgtcgaggaacagctcgacctgaacaccgaggacatcatcgggctgaagacgccccgccgaccgacgccgatgatgacgacacgaggaggtgcgatgtgatggaactcctggaaccgggcctgttggccgagggggactacaagatcaccctcaccggcccgcaagggcagaccttcaacatcgccacccctcaccgccacgagcgggaacaccagcccgtcctactactgaaaggaggcactgacgggttcagagtcaagccggagcgccgagcccgtgcaagcgtcaaccgctacggcgaacgcgagtacggcaagcgcttcccgcccttcggcggcaccctcaaaacgctcgtcggcgcgccgggcttcaagctcggtcacgtcgaccggaactggcgcaagctgtggagcccgttcgaagacaccaaggtgaccgtggcggccacggacggcggtaacgcctttgccaacttccggctcgtggacatgtcggacttgccgcacaatctgcgcggccagccgtcctacccgtgcgacgtcacctggacatgcccggacggcgcctggagcgggcccgcccgcacctactccggagccgcgaccgtgatcgacccatccgacccgggtttctccgcgaagctcacgctcgcgtggaacacggccgaggacctggacgtgacgtttcctgccggcaacaggatcacgttcaaggcgtcgtcgataagcaaaaagctcccggacaccgtcttcttcgacctcgagccgggcatgatgggccggcctaccgatgccgccggcaacgaactggacaccctctggtccgcattcgcgggcaagatgcgcgggctcgagctcgagcctcacattccgacccgctgggcgctctccggctgcgagctgcgcgtaacaccccgctacctacacccgtggaggtgaccgatggaagagagcattatggaagcaatcctcgcgggcctcgccctgcccgactaccgcgaactcaacgagttcgactgggcagccgagaagcgacgtcgcgagaacatcgttgccgcgcgcagccagtacgtcggcctcctgaacaagaacttcatgccggtcatggacatcgaggactgggagggcgcgtcttggggcgagacgttccaggacaccgccaacatgcagatggtcctcccgggcgaggtgaagccgggcgtgcaaaacccgctcgtgcgctatctcctgcagaccggcagcgacgacccggacggcgtcttccacgacgcgctgacggtcatcgtcgaacggccggggcggggtggcacactgcggcgcttctaccgcgtcctcgacatctcgcccgagggtggccgcgactacccggacaaggtcaccatcaccgggctggacggcatcgagtacctcaagcacctgccgttgtgggccgacccgtcgaaccggagcaaagtagtccagctgcagttcgaggacaagcaggcaggctcggccgagttcgtctcgcgaaagctgatcggccgcaacctgatcggctaccagcagccgtcgatgctcgcgcagatcctcgacggcaaggtcggctcgttcaccatgacggacgactacgacgacccgcgccgctggcggccgatgcaatcacagatgcaccgcattatctgctcgccagtggcatccggcctgccgtccgaacactgcattgttaccgcccgatgggacaatgcgtgggatctgctcaagccgacgtgggaggcatccggcatcctgccgatcgtcaccctctggctccccggcgaccgccagccgttcccgaaccacacagaactgaccatgcccaccgtcatcgtcgacttccggccggtctccacggtcaccggcgcgcgcaccatgctcgggcagggcatccagtctttgcgacggaagatcgacgccggcgatcgtttcacctccgttaccgaattttctgacgtggccccgccgacccgcgacggccgcccgccgtgggtcgtattcgactgcgaggacgcgccgcgcgtcaccatccgcaaatcgaccgatagccgcttcctcgtcggcggcaagtcgcccaaagccatcaacaccgtggtcaacgccggcgtgaagggcgtaggagcgacgctgggcttcttctttccccgcctcgcgtcgctcgcgacctacggcgccgacatggttgccgaactatccgccgaccgcttcctcaacctcaacgagcaccacgaccgggaccgctacgtccgccacggccgctccggctacatctccgtggccaaacaaggcgaagccaacagcgtcgactccatccagaaggcatggcaagccaaaacggagaccaacggcgggttgagtgttgagttccgtatcggtgacgcctacccgtaccaacccggcagagacttccagctcggcgacaccgtcggcctgggtgcctggagtgaggtctgggccgcctacgtctccgagatcacctggacctcgacccccggtgaacctgtcggctacgagatcaccctcggcgacctccgccaagtcacctcaccggagaagcttttcgccgccaacgtcgagaccatcaagtcgcgcctcgcgcggctcacatccaccgtcaactaggaggacacgatgcagctctacccctacaacgtcccagacggagcgcacccgctcgcctggaccctctacggccacggcctagacaccgcgaccatcaaccgtctttgccgccatctttacgacaatctcggcgcccgcctccacctcccggagccgcgcgacgtcacaatgggctgggccgtcgactgggcactcgacccaggagaccgcgacgtcgcccacgtcggccacaaactcgacatcggcctcggcttcgacaccgccgtcaccatcatcgacggcgcgctcccgccaggcatccgcctcgaggcccacaccggccgcctcgtcggcgtcttcaagcaagccggcctctactccgccaccttccgcctcgccccgcgcaccaagtacgaccccctcggcggtccgggcggcccggacaccgccggcaaatggattccgcttgaccagccgcgctacacaccacccgccgccgaccccgctcccgcgcgggacctcgcggccatgacaccgcacgagctcgaagctctgatcgttcaggcgcagcaggcccagcgcgccgggttgatccgcgatgccgacaaggagccgagcggtggggattagaccaatcactagcggcgagcagatcatcgtacgcgacgtccgcgaggagcttgccgatgacctcacggccaccgctggcgaggtcgggcagcccatcggcgaggccctggacgagatctacgcgacagcagattccgcgaacacgtcggcaggtgaagtagcggcgacccttgctgacctgcaaagcagagtcgagtctctggaactgaagctcgcgtcactgcaatcgaaagtggacacgctcttatcggctgaagagctgacatccgcagtttccgatctgcgaaagcgggttgaagcgttggaaacgcctcccactacctaaaacgaatttttcaaccgatcaccgcatctactcagtgcatgtataggaggagggacttatggctgaaacaattactttgacgggccgtttgactgatatcacctcgcggccagttgagcgcatcacaaggatttctgttaaatcgcccgtttacgggcccgggccaggtattgacctcaccacttcccagcctgtagcggtcgaggcttcccaaggtggaacgctcaccattcaggtggttgagggcgtgggctggttgttcgttgagggggatggttggtcggactcgatccggtttgttgccgctcctggaatgtccaccttgtgggaggcggtggtgaatgcgctgccgcacacgattgaggtcaaaaacatgcttatcgccttgggtgaagcgtatgaggcgtcgcaggcaggccaggcgctaccgccgtggttgacggaggcggcacttaatggcacttatgcgacgaaacaggagtttttggcagcgttgcaggacaaggtggagccactagtgatggactatcttgcgtccgatagggctgtcactgatgccgcgattgcagctatcgagaagcaagtcccgggcgcggtggatgcgtatgtcaaggggcaggttacttggcgaggcgtggttggcaacactgtcgatttgaatgctgtccgcgatccgggtttttatacggtgccgtcatctgtggtgggccggtctttggacgcctggccggataagtttggtggcgtgctcgctgtgtacgccaataagggcacgagtgtggccattcaggaagctattgtgtcgcagggtgggtcgtttaggcgttacctgcggtattccgcggctctaggcgctgatagctggactccgtgggaagaccagtcagcaacaggtgtgctgccgtccggtacggatcttcagaagtggcgggcgcagggtgcttatcaggtctccctcacggaatccttgaagctgctggatatgccgaaagacgctgatggcaaccctgtggcggggcagggtgtggttgaaactctgactgcggcgggtactggtatggcgatgcagcgcatgacgatcaaccagagatccgggggtcttgccacgtatgttcgcttcacatcgcttacatctgggtggccggagtggcagcgtatcggcggcggtagctctgctggtggtgggcaggtggcgagcccgcaggctacggcacggtcctacacgtcgtcccacgcagcgagggtggagtacgcgaaaacccgccggggcggaagcattggtacaggcgggaagcccgtggttatgttgcgatttgaccactggctcgttgcgttccgtgacaaggtgttgcctatcttggagaagtaccagctgccggcaacgctgaacctgaaccacgacaacctcgagctagagcaaaacggcagcggctcaatcacctgggagcacattcaggactggaaccagtacaagtgcattgagattgctaaccatggctccacccaccgcgaccagtccaccacggagggtatttttcacgagatcgtgaatgggcggcgcaacctggagaaagcgatgccgcgggtagcggtagaggcatggcaagagcatggtgcgtcgtacttctataacggcgacattgacggcgatattggccttgatctcgggcgtaccttggcgaactacaccgattcctacgccggccagctggtgctctcggagcacgctgtggtggagggtaagtctggcggatttttccatccactgaccggcaccccgcagatcgggcagtcgcatttcagttttgaccgttcgacagcggcggagatgatcgcccaggtcgataccgttgaaacggtcggtggtggggtcacgttgtacgcgcacccaggttcgatgcagaacgtgcttgtgggtgggaagaactggccgtgggcaaagctacccgacgggcgagtcacgctcactgaccctaagaacggggcggtgcaaacattcgcgtccgaacaggcgctccgcgactgggcgggggcgaacggcaatatcgtgttcgctagcttcgatgacttcgatgtgttctgtgctgagctggcacgtcgccgtgacgagggccggcttatggtcatgaccgcaaccggcggtggtgtcgctgattcctcccacgcacgccgtcgaaacctgctcgtcaagcccgatttcaccgacgggcataaagactggtggacgtacatgaccggctggacagtcactaaccccggcccggacgtgacactcacctccactgggagcgcgcagcctcttggccagtcgatgctgctgtattcacgtttcgggtgggcgatgggcgcagcccacgaattggttgtgactgcctcggcgaccacaccgaccacgttgacgctgcaaatgcaccagctcggcaagcctgaaaactggaacgcgcagcgtgaatttgaggtgccgggcgacggcaagaaacgcgcctaccgcctcaacctgaccttgccgagggacaaggacatctcccagatgactatccgcatcggcggacccagtctcacaattcacggcgcgccactcctcgccgcgatttagacctaccgatcaccggacaagcgcccgcaggggcgattttttatgtcaaaggagagcgaatatgaccatcaaaccaaacccaaactggcgaggagaccccacgttcctgccggaagtattccgcgccttcggcgtcaaattccgcgaatacccgggctggaaagactggggaatgggggacttcggcgtcatccagggcgtgatgtggcaccacacaggcgccatgaacacgagtccggaatacatccgaaacaacccacgactaagtaacgggctttcctcgcagttccacaccgcgccgaacgggctgcagaccatcctcggtgccggcattgcctggcacgccggtcgcggctggctcgacgggtggcccaccaacgatgcaaaccgtgtctgcctcggtttcgagatgcagcacgacggtatctcgccatggccggaggaacagctcgaatccaccaggctcgcaactgcggccatcctttggttcctcggcaagcgagcaacaaagaagacgatgatcgcgcactgggagtactcgatgcaggcccagggtaaatgggacccgggcgctggcaccgggaaagccggagtcgtgatgaacatggatcggcagcgcgagctcgtgaaccagttgatcgacaacttcacccgaacaggcgacccgtacggaaaacccgccccgccaccgaaacccaaggaggacaccgtgccgctttcaaccaagttcttcactgacttcatcgtcggattcatcggcccgatcatctccgacgtcaaggacattcgacagcagataacgggagggcgcgatgccggaaattacgacggctggtccatctcgtggctgatcgagcagtaccagcgccgtaaaggcgaccatggcaccctgccggaattgatcgccgtaaacctcaaggagaccgagcggctagccgaccaggtcgcccgcctcgcagacgtgatcgagaaaaaggagcagaagtaatggccagcatctttcagacagcagtgagccaagcactcgtagaccaaccttggtatatccgccgcaaagactccctcaccgcggccgcggggctcgtcctgcagatcgctaacgtccttgtcgcctacggatccgacatgccggaatgggccaacgtcgccatcgcggcagttatcggcataagccagatcttcatccacgcgggcaccccaggtgccatcaccccctcgcaggccgcaaagctcgaagctgccgcagagcagagcgttcccgaccgccagtccgtctccggatacgtcatcgaccccggcgagacggtcgagatctccgaccccaacgaagaccacgcgcccgcagtgagcgcctttgccgcagggcggcaggccgcgtaccgggaagggcgtgaggtcccggagggaggaactcacagtgttggctaaacccgctagagaaaacgccaaggaatacctacagcagcaccttcctcggctcctggcggcgatgtgggcactgtggagcatggccaccgcagcggcctacgttgatcgagttccaccccagctcgaagtcgtggacaaagcgaccagtgtgccgctttggacgatttgggcacttgccacgatcgcgctcgcgctcggcgttctcgccccctcaaccgcccctgacaaagttcaggacgtcgctcgttggctgcgcatcggcggcatgatgatcgcctgcgccgcactgatcgtttggacagtggcgttcttctacgacgagccccgcgggtgggtgaccggcaaaaactatgcgctgctcgccgcgatggctgcgttcaccacctggactattgcgcgggacaacgcgcgccgggagcgggtggtggccgtatgacgagtgaacaggtcatcatcgcgatcatttccggtatcggagcgctcctcgtcgccgccattgggtggctggggcgccgcgacgagacgaaggcatccgcctcggagacgttaatcaacggccaggcggcgcgcatcgacaagctcgaaacgagactcgatgcgatcgaagcagaactccgcgagactcgcgcggagctgcagacaatccagtctcacgcgggcgatctgcgagacgccttgcggcgagcgctcgcctggatcgcagaggctcttgagcatctttctgcccctgacacgatcgcagctccgccggctcctgatgtggactcgtggcaggcactcattgactccccgccgagggcgaggaatccgccgcgttgactccgggagccacctctatccgcggcagcggttcaaatgccgataacgcgcacagaacgcgcacgcccatctaacgcgcaggtcaaggccataaagcattgtcctcgtaatgagaaggtcgcgagttcgattctcgcaggtggctcaggtggaaccccagctagattgttcgtctggctggggtttcggcgttctctcccggtgccctcgggagttaatagcgggtaactcgcgggggcggttccggcgacctgcggaaacgcggttgtcgactcgagttacccgctatcaccgagcaagccggccggccaacagcggccaaccgcccctaccgcggccgcttcttgcggtagtacacctgccgccgcacgcgggcgaccacgtctccgccggcatccacgatgtcggtgtcgaaccagtgcaaatacttgtcgccggcggcggtcttttcgcggatgaggttgtaggtggcgtcgtcaatcagcatttctgccgtcagacgcccgcggcccggtttgacgaacgtgatttcggcgccggcgtcccaaatcgagtaccccttgcccagccgggacatggaggcgagcatgtagaacgggtcggtcatcgccatcatggtgccgccgaacgcggtgcccacgccgttttgcgtgagtaggcgcggggtgtgcgcaacgacgacgcgggagccgtcgggcgcgaattccttgacgcggatgcccgcgccgagaaacggcggccacagccacatgaagcgctcaagcgttttcggtgcgagcagattcaccttaggcaaccgcatcactttccaacctccgaaccgtcgccgccaattcccggcaggaagcgcggcacgaccttgccgacggcgttgcgcggtagcgccggcagaaagtgcacgtcgcgcggcacagagtgatctgcaagccggtcgcgcacccacgcctgcacggactccacatcgagcgccttgcccgcgtcgtccttgcccggcacgatccacacggcgatgcgcttgaacatcaccgggtcgtccacgccgtgcgcgtagacctcgtcgacgcccggcatttcgtcgagcacctcggtcacggactgcgggtgcacgttctcgccgccgacgatgatcatgtcgtcgttgcgcgactgcacgtgcaagaacccgcgctcgtcgaagtacccgagatcgccgatctcaatcagcccgtcgatctcgacgacgtccgtgtgcgggttggtgtagcccttcagcgcggtttcgttgtgcaagaagatgcgcccggtctggccggtggggacgggtttgcccgcggcgtcgtaaagccgaagcaccgtgccgggcggaaccttgcccacaatcgtcgggtcagcctgcatctgttcgggggaggcggcggctgcgagcgcgagttcggtggagccgtagatgtttgccaggatggggccgaagcgttccgtggtgcgcctcagcagcgcaggggtgacggcgttgccggcggtggccaggtagcgcagcgtcgaggtgtcgtagtcctcgtccagatccagcatctgcttgaaaaagatgggagaggagatcagcccgtcgcagcggaaatcttggatctgcttgaagcaggcctcggcgtcgaacacgcgccgcatgaccagcgtcgagcgcgtggccagcccaacctgcagcgccgaccaaccccacgtgtggaagatcgacgcggacagctgcaccgtgtcgccgccgcgccacgggatcgcctccaggtacccgctcagcacaaacggcagccgcggctccggccgcacaatgcccttcggaattccggtggtgcccgagctcatcagcacaatgttgccgtggggcgggaaaaggggcagttgcttatcgacgcccccctcaaccaccacatccccaatcgacagcccctcgcgcccctctgccgtatgggcccgcacgacggtgaccgcatctgccgcgccggcggggacgcggtcggcgaactcgtcgtcgatgaacaggacgttgatgttgttctcttcgaagatgcctcgcagctgctccggcgaggagccgatgttgagcaggaagatgtggccgccggcgtaccccttcgcgccgagggggaggatgatgccgcggccgttgcgcgccatcacgccgatgcgcagctcctcgaggccgcgctcctccttcaggctgagcagccactttgccagcgtgcgcgactggtcgcggagttggcggtaagagagcaacccgtcgtcgtcgataatcgccgtgcgctcgggcaccgccgcagcaccctgctcaatctcgcgggcggtggtgaagcggtacctcgccagatttgggatgagctgggcggccgcgcgggggccgccctcggtgctgagaacgccggcgcgcaggactgcggggagaaagcgcgcgaacgacttcatcacgaagatagggttttcggtgggacgcatacttgaaatgtagcgtaaggtgctgatgggattattgtttcagtagtgattgcgtaagaaaggcacctccatgacccgccctacgatccgccgccgcctcagcgccatcgccgcagccgccgccatcgccgtcggcgcgattgcccccgccccgcacgccgaagcgcagcagcgcaacatggtcatcttcggcgattcggtggtctccgacccgtccgggccgaaatggcttggcggcaagctgggactcgacccccgcggctcctccgacgtcaccacgtggtgcccaaccagcccgacgaactggggcaagcagtcggctggacagctcggcctgccggcgtgggattactcctgcaccggtaccgtctccatccaagccggcccgcagttctcctcccaggtcgaccgcgcggtccgcgacggcggcctcaaccgcaacaccgcgcgcgtggtcatcaccaccggtttcaatgacacgtaccacaacgacggacgtgaccgcgcagcgttccggcgcgactgggtcgccgccatgaccccgcaggtcaaccgcatccgcgccgccgccccgaacgcccgcatccagatcgtcggttacccgaagatcacctccaacggcaacgtctgcctcttccacgtcgccccgaacgtctccgacaccacgccgttccagcaagtcgcatattgggaggactccatccagtgggcgcaggtcgatttggcccgcgccaccggcgtcgagttcctcgacctgaagccgtccacttggaacaacaacatgtgcgcccccgacaaccagcgcatgtgggcaggcctggtcgacttctacggcggccccggcaacctccccatccacgtcaaccagcgcggccacgcccacgtcgcacgcgtcatcgcgggctcctagccgccgcggcgcaaatggtcacccgcaaagtgttgcttgcagatggtcattaaccgggtaaccgcaaagaggtgatctttcgcgacggcggttaatgaccttctggtagttaccgggtgggggttaccttttgggaagcgcgtccgcgtgcgggggttcggcgttctggagggcaaccgcgcgcgcgaggcgggcgtagcgcagctcctgttcgcggaaccgggtccacgtggagatcgtggtgaagaagaacgcgatgatcaggatgtagagcatcaggtcggtgccgcggtcgacaccgagccagttcgctagcaccgtcacgtcgtcggggcgcaggatcgcccagatcgcggcgaccatcatcaccacaaacccgatcttcacccacgccttcgcgttggccttcttgcggttggtgaagaagtacgccgcgagcgcgaccgtcgcgatgatcagaagcagctgaatcacttgagcctccgtgccatgattccgtcggcgaggatgttcacaccgttaataagcgactgccccttggccattgagtactcggtgtagaggatgtccaccggttgctcggcgacgcgccagccgcagtcgtcgatcatcgccacgatctcggatgcgtggctcatcccgttcatgcggatgttcatctcttcggcgacgcggcggttgaagacgcgcagcccgttgtgggcgtccgataacccgagacgcttggtgcgcggggagagcatgaccaccgtcttcagcacgaggcgtttgatccacggcacctgcgagttgtcctggccggcgaagcgggtgccgacgacgatgtcgaggggctcggtgcgcaggcgctccaccatcgcgacgacgtctttaacctggtgctggccgtcggcgtcgaaggtgacgaagtactgcgcgccgggctgggcgcgggcgtactccacgccggtctggattgcggcgccttggccgaggttcaccgggtggttgactagatgggcgccggcggcgcggatggcgtcggcggaattatccgcggagccgtcgttgaccgcgacgatgttggggaaggtgcggcgagcttgggtgatcacgtcctggatgacttgaccctcgttgtagcaggggatcaccaaccaagtgtccccgtaaagattcgcctctttggcgcgccgcgattccatcgcgaaacaatttacccgccgcggtggaaaagtacggtgtttacgcgcttgaccacaccgattggcagcaacctgtaaacattgcgcgcgacgaggttgaacgcggcgcgcggacgcgagatcagaccgtagcgcaccaagttgcgctgcatcatgcgctccgctctgcgggtttggttggcagagcggcggcggtgctgggcatcggtgacgcgcagatacgtcagcggctccggcaagttgcgcagttcccaccctccggcgagcatacgggcccagaggtcgtaatcctccatgaacggcacatcctcgtacccgccgacgttcttcgccgcgtccgtgcggaacatcacggatgggttgttgatcggggagttcatcttggcgtactgggcggggttttggggcagcgtgcggatgcgggcggcgtcgccaagcaaatgctcaaattcctcgaccgccgtgccgagcgccgccacctcgggatgcgcctcgaggtacgacagttggcgttcgaagcgctccgggcgcgcggcgtcgtcggagtccaggcgggcggtgtagtccgactcgatcgtttccagaccagcctgggaggcggggcccgagccgcggtttaccggcaggcggatcaggcgggccttctgggtagcggcaaagccggttgctacgtgctcaacatcctccgcgacggggccgtcgaacacgatgaccacctcatccgccgggcgggtctgcgccgccaaggactgcagcgcgacggcgagttctgcggcgttggtgccgtggtaaatggtcataaggacagacagcgtggccatggtgtgctcccggttagtcccttgcagcgtcaatgaggtagcggccgtagccggatttcagcatcggctcggcgaggcgttcgagctgggccgcgtcaatgaatccctcccggtacgcagcgacctcgggcgagccgatgaccgtgccggtgcgtttctggatcacttcgacgtacgcgctggcctcggccatcgagtcgatcgtgccggtgtccagccacacgtcgccgcggtgcaggcggtgcaccttcaggttgccctcgttgaggtaggcctcgttgaccgacgtgatctccagctcgccgcgcgccgacggggtgatgcttttcgctttctccaccacggtgttgtcgtagaagtacagcccgaccacggcgtagttcgacttcgggttcgtgggtttctcctcgatggatagcgccgtgccgtcggcggcgaacgccaccacgccgtagcgctgcggatccgacacctcgtaggcgaagatcgcgccgccgtcgattccggccgtgctgtccgtttcacccagcactgcggtaagcccgttgccgtcgaagatgttgtccccaagcaccagcgcaaccgcgtcgtcgccaatgaagtcctcgccgatgaggaaggcctgcgccagcccgtcgggggagggctgctcggcgtagctcagcatcacgccgaactgcgcgccggtgcctaaaaggcgctcaaacgcggggcggtcctccggggtggtaatgacgaggatctcgcggatgccggcgctgatcagcgtggtgagcgggtagtagatcatcggcttgtcgtaaatcggcatcagctgcttcgagatgccttttgtaatcgggtacaggcgcgtgcccgatccgccagccaggatgatccccttcaccgcgtcagcccgccccgctgcctagcgcggcagctgcgggagctgcgggagctgcggaagctgcggcatttccggcagttgcggcatttccggcaggcggacgtttgccagcatcgcctcgatctggccgttgtcgaactgcatgatgatgttcagcaggccggtgaggacagcgatgacgaacagcgcgatcgaggccggtccgacctcggagaagtcaccggaggacatcgcgcgtacgacgtcgcccgcgcttgcgggcttcggggttgtcggcgcgacggtggtgctggtgaccgtgactgtcggggtggtggtcaccgtggtggaaacggttgcgcccggcgtcggcgtggtggtgaccggggtgccggtcgcagaaaccggcgccaccggcgtaggcggcacctccgtcggctccgcctgagcgtggctaaccagcacagtcgcgcacgtcgcggcggtgactagggcaatcgaggtgcgggtgcgggacatggaggggctccttgagaacatcctgaagcgtgaaaagactgcacacagtctaaacacaactgctagcaggtgggaagatacatcgccagcgccgcgcgccagttggtcggggagaatccggttgccttgatcttggtgagatccagcgtggattccttcggccgcggggcttccgcgccgtaaagctgcgtgtactgctcggtggttacggggtgcacgtcggaggggtcgtggccgagcccgatgaacacggccatggcgatctcgtcgcgtccggcggtgtcgccgtcggaggtgaggttgtacacgccgtactccgcgcccgtgtccaaaaggtgcaggatgcccttggctaagtcctcggcccaggtgggacgccctcgctggtccgccaccacgctgggctgcttcccggcctgggcgagcgccgccatcgtggacatgaagttgccgccgtcgccgaagacccaggaggtgcggatgacgtagtggcgccgcgcgacttgggcggccgtgtcgcctgcggccttcgacgcgccgtacgccgacagcgggctggccggctcgtcttccgcgtgcacctccaccgatccgtcgaagatgtagtcgctggagacgtgcaccagcgtcaggtcgtgttcgttcgcgatctccgcgaggcgcgccggggcgtccgcgttgacccgccacgcctgcgcgcggttggtttcggcgccgttgacgtcgttgaacgcggcgcagttgatgatcgcgcggtacggggagaagtcgaaatctgggtcgatcgcggtgatgtcgaactcgtcgcgaccgacaaagtcggcgtcaccctcgccgaggcgggtgcggagtgcgcggcccagctggccgttcgctcccgtgacaaggatgcgctttggggggactaagggggcgtcggcaagcagcggatgctcctggtcggccttcgatagctttgtgggcgtaagcggccagtcgatctccttgtaggagcagtacgcgtagtcgccgcgcgggttgtatcgctggttgaccaggtaaatgtaggcggtgtcgggttcgagtgtctggaacccgttggccaccccgcgcggcacgaacaccgcggtggacggggtgatctctacgccgaacttcgcaccaaacgtcggcgagccctcgcgcatgtccacccacgcgccgtagacccggcccgtggcaacgctgacccacttgtcccacggctcagcgtgcatgccgcgcgtggtgccgggtgtggcgttaaagctcacgttgttttgccgcggcaccagcgcctgccccgcccagttctccttgaaccagccgcgagagtcctcgtggactgtgaggtggtggatttccaggccgtcgatcggggtgcgcatggtgcccaagttactgtccgctcagggcatattgcttttcgacgccacccttcaccccctcccaccatccacggttatcggtgtaccacgcaatggtctgcgcaagaccgtcgcgcagatcggtgtagcgcggccgccacccgagttcttcgcgcagtttcgtggcgtccatggtgtagcgctggtcgtgcccggggcggtccgccacgtgctcgtaggtgccgcccatgatctggcagatggcctcgatgacctgcttgttcgtcacgtgcgcgtcgccgggcgcgctcgcgccgatgttgtaggtttcgcccggtttgccgcgctcgaggatggtgagcacagcgtcgttgtggtcgtcgacgtggatccagtcgcgcacctgctcgcccgagccgtacagcttcgccggctggccggtgaggatgttggtgatctggcgggggatgaacttctctacgtgctggtatggaccgtagttgttcgagcagttggagatcgtcgcgttgatgtcgaaggagcgcacccacgcgcgcaccaagtggtcggagccggccttggttgcagagtagggcgaggaggggttgtagggggtcgtttccacaaaccgctcatcgccgccgagcgggaggtcgccgaagacctcgtcggtggagatgtggtgcaggcgcgtgccgtgctcgcgcacggcctctaacagagcaaacgtgccgacgacgttggtctgcacgaaggcggacgggtcgcgcagagagttgtcgttgtgcgactccgcggcgaaatgcaccaccgcgtccgcttggcgcacaagctcgctgaccagctcagcatcggcgacatcgccgagcacgaactcgagggccgcgccctcgatgccgtcgaggttcgcctcgttgccggcgtaggtcagcttgtccagcaccacgatgcgctcggcggcgccgcgctgcgccgcgagcctcacgaagttcgaaccgatgaacccggcgccaccggttaccagcaaagttgtcatgcgtggctatgttaccgcccgcgacaacccgaggacgtggacgaacgcgccggcgaggggccccgcgaacagggccacgatcaccgaggtgatcactggccacggcccgatgaacagcaccgcgaacgccaccgccgaggccacgagccacccggcgacgtaccagccgtggcgctccgttgccaggaccgcgacgccggtaatcatcagcatgcccatgatcgctgacgcgagcgtcaggaaccccagcgtcaccccgccgacaaacaactccggcttgaacgccacgcgcagaatccacggcccgaccgcccacgcggcggcgaacccgatcgcgccgacgcctaacaccgccgccgccgggccagcgagcgcgcggtagatctggtccttcttttccacgaagcggaccaccagcgcggattggaagcgctgcagcggcaccagcaccggcgcgcgggtgagcatgacagcgttgttgaccgcggcgacgatggtggagacgcgctcgtcgccgtcagcgaacgcggcggaaaccgccgtcgggaacccggtgatcagcgccgctgatgcgcccgaggccaccatggcggagacgacgcggccgatgaacgcgccccggtccacgtcgagcgcgatcctgatgttgctgcgcgccgacgtcgacgcgcccaagacaacgagccagctagctgcgccgatgacggtgatgaacaaaaacgcgtccagcccccagccgagcccccacgcggcgagcgcgatcagcagccggatgccggagtcgagggcgacaagcccggcgtactggtcccacaggccggcgccggacaagatcccggcgagcaccgcctggaagatgtagctgaccagcccgaagaccagtagcgaggtggctagcgtcggcgacatcggcacgatcgcgcgcatcgcccagtagccggcagcgatgaccaccaccacgacaaacgccgcaaccatggaggcgaaacgccacgggttggcgctcccgcggactttcgtttcccgcgcgtgcgcgacggcgcgcgtggtttcgttggtcacaccgtcgataagtcctgttgaagcgaagaacagcccccagtacgcctggaagtagcggtactccgtgccgacgtttaaagcccagctcgccacccacatgaggatgaacccggcgagcgctgagaacaccgttgcgagcgagaggttgcgcatagcggtttacccgagcgggggaagggcggtggtgcggagccacgcgttccacacggcgtcgatctggggcttcatgcttggcgacgcagcgcccaacgcccgcgcgaaatccccctgctccaccacaccgtgagctgacttggcggtgtaattgcgcactgcagagaagaacgcctcgctaccaagcgccatgtgcaacgcgtgcaaggtcaacgcgccgcgtttgtacacccggtcatcgaacatttccttcgggcccgggtttgccagcgggaattccagcggccgcagagaggcgaggatgttgtagtgggtggtcaccgacgagtccagagtggtccggcccttgaagtccagccacagccactcggcgtagcaggcgaaaccttcgttgagccagatatcgccccagtcggcgatactcaaggagttgccgaaccactggtgcgcgagctcgtgtgcgatgaggcgctcctctcccgaggtgtggttgcggccgaagattgactggcccgctgcctccagcgggatctcgaggttgtcttcgtggacgatcgcgtcgtagcgctcgaacgggtaggggccgaagcgcgtttcgaagaagtccaacatctcctgctgcagcgcgaagtcgcccatctcgacgctgcgcggcagccatgtgccggtgttgcggcccgaacggacgtggcggaactggccaatgttgacgctggccaggtacgcggggacagggcgggtggtgctggtggtgatggcctggtagccgcggtccgtgcgcactgcgatggtgtaggtcgccttttcgccgggggcgtcgtcacaggggaaccagctcggcgcgccgttgggttggttcgctgtcagcgcgccgttggtcagctcttcccacccgaggtggccccatgtcgtgcggcgcgggtgcgggttgccgacatagcgaaccgcaagccggaactcagtgtccacctcaaccggttccgcaaacgtgatgcgcagcttgttgcccgactgccggaaccgcttcaccggcgcagcgctcgcctccacgctgcgcactcgcatcccgtcaacgagatccagcgtcatggtttccaagtcgcgccacggcgtcagcgtaagcgtcgcggtggcgtctaaccggttcggacctacccggtaatcgaagtccaggttgtagtgcgagacgtgaaaaccgaggttgaaatccacacccgtgtacgcatcgcgcgtggcgggtttcgacgtggaagccggcgacccagcgggctcgttgttcagacggtgcatgatcatatcgaggggaagtctactgcgggccagctctcgcgttgctgccgggattatgcgcggcgtaattgcctaagggaatgcggcagtctgcgccgctgtcgacccaccgcagctatgttgcggatgtggcgggtggtgcgagattctgccgcgcataatcccaacagggccttgacctgcgggtgtggcgcgtggggccggtggggcgaaattatgcctcgcataatgtcctggggaaatgcggcaacaaaaacgccgcgatccgaaaggactcggtggtcgcggcgtcgtgcggctctgtgagttacaggccgaaggccggtgcgaaggtggtgaaccaagccttctcaacatcctcgcgccagtacggccaagagtgtgtgccgacgttgcggaactcgtagtgggccgggatgccgagggagtccagcttcacacgcatgtcgtggttgcactggttgatggcggcctcgatcgcgccgcccgacacctgcaggcgggcagacgcgaactgggcgatgccttgcggtgcgccctggccgaggaggtagccgacttggtcctggcggcctgcgaggcccgtggctgtggagaggtagagccgtgtgccgcggagattctccgcgttgacgagtgcgtcgttccagcggttgtacgggccgcccatcgggccccacatcatctccggagtgatggtctggaaatcagagccgccggcgcgattcaccgtcaggcgcgcaaagttgtacgcgtggggtgagctcgtggccgggcatcccgagaacgacgcggcggcgtcgtagaacccggggttgtgctcgggcagtacgagcgcagacgtgccagacatggagaaaccggcgatgccgcggcggttgtcggcgttcagcatgcgctcgattggacccggcagctccttagttaggaaggtctcccacttctgggggccgcgcatgtacggggtgttcatcgactcgtcgagccagtcggtgtagtacgagaacgcgccagcctgggggatgaccacgttcacgcccttgccagcgaaaaagtccttgactggggccatgttcagccagtcctggttctgctctgcgccgccggcgccgttgagcaggtacagggttggtgcctttgccacgcgctggccctgcgcattggtggcagggatgaccgcaaccgggacgtcgcggcgcatggagggggagtagaccatgtaggacagcacggtcttgtggtcgacctgcttgacccactcctgcggaaggcccgaactcacgatcagtggcgggttacccggcgcgttccaagccttgacagtgccgaccggggtctgacctgcgacctgcgcggggttgaccggggcagcagtagctgcgggtgtgatgccgagggcaatggcggctgccgcgactgcggccgtgacggtacgctttaggctcataaccggccatattacggtcacagtaaacaaattgtgcaacaataacccacaactgcttcctcacccgtaaaggaattcacatgattgagaacgtgcagctgcagatcaacgaggtcctcggccagctaatccacttcggctcgtccacttcgtcccagatcgcgttcggcatcgggttgttctaagaagagccagaaagcgtaagaggagccgcggcacgcgccgcggctcctcttcttcgttcgggggccgtaactaaccgagcagcgccggcttaatcaccttgtcccaggacaccttgaggtcgtcttgccagatcggccacgagtgggtgcctaccgcgcggcggttgaagtacacgtctgcgcccacgctgcgcgccttggtgttgaagtcgtgggtgcacgcgttcatagcagcctcgatcgcgccgccctcaacccacagggtgagcgcctgctgcagggccacggaagaggtttggttctccttcaggtaacccagcatgtcggtttgtcccggaaggccggtgccggcggagacgtagaacttcgtcttggagtccttgagattgtctgccattaccagcgcgtcgttgtaccggttgtactcggacccgcgcgggccccagaggttttccggggtgaccctgccggtgccggcagagccgcggttgacggtcaggccgacgaagaagttgggcagcggggtcgaggtggcggcacagccggagaacgagcccaccgcgtcgaacatgtccgggttgtgctccgccagaagcaggacggacgtcgcagccatcgagaacccggagaccgcgcgcttgtcgctggcctttgtgtagtcctcgatggaggggcgcagttcgtgagccaagaacgtcgaccacttctgctcgcccttgaagtacttgttctcctcgggcttagtcagccagtcgacgtagtaggagaacgcgccttccatcgggatgacaacgttgaccggctcgttctccagcacgtcctgcacggtggtggcggcctgggagatccagtcggtgttctgctcggagccaccggcgccgttgagcaggtagtaggtcggtgcgtcctcgaccggcttgccttcctggtcggtcgcgcggatcaacgcgacgggaatgtagcggtccatggcctgggagtagacctccacggcctcgccgccacggtaccgcctgatctggctgaaccaatactggtcctcaccgttgtagtccttcggtgccgcggtcagctcgcgcacttcgccgagcgaatcagcggcgtcctgcgccgtcaccgcttcaggcatgttgtcggcgtcctcgccggttgcctcgggctgcagcgccgtctccaccacgttggtcaagccctgcccgtcgccgtcggggacggatgcgccgttcacaaccggagcctcggccacctcctgcgcttcaacgacctcaaccgtctcagcttccacgacggtcgtgtcagccgtggtctcgtccgtgtcacccgcgtcccccgcgtcacccgccgcgccgctctccgcggcggcgttggcaatctcgtctaaatcagcaggctccgaggcttcagcaaccacctcgacttgctcgtcggccggctggatgcgtgcaattgtttgcaagccctgcgcgtcctccgcagcgcggtggtggacagcggctggagcggcgcctgccacaagcgcgatcgcggcgacggtggtgagaacgcggcgggtgtgtttcatgctctgtgagctctcttcctgtgagttggcgggcacgaggcgtatatgttccttatcttgccagactgcgcgagcattaccgtccggtaatctgccaactcgccgcccctcgtgtgcctaagcgacgtattctgtagggcgtgactaccgaacattttgacgttgttgtcctcggcgcgggccccggtggctacgttgccgcaattcgtgcagctcaacttggcaaaaaggttgccgttgttgagaagaagtactggggtggtgtctgcctcaacgtgggctgcatcccgtcgaagtccctgatcaagaacgccgaggtggcggagatcttcaaccacgaggcgaagaccttcggcatcaagggtgacgtggagttcgactacacggacgcccaaaagcgctcccgcaaggtctccgagaagattgtcggcggcgtgcactacctgatgaagaagaacaagatccaggaaatcaacggcctgggcatcttcaaggacgccaagaccatcgagatcacagagggtgacgacaagggcaagaccatcaccttcgacgactgcatcatcgcaaccggcgcagttgtgcgcaccctgccgggcatcgagctgtccgagaacgtcgtctcctacgaggagcagatcctcaacccggaggctccgaagaagatggtcatcgtcggcgccggcgcgattggcatggagttcgcgtacgtgctgtccaactacggcgttgacgtcaccgtcatcgagtacatggaccgcgtcctgccgaacgaggacaaggacgtgtccaaggagatcgccaaggcgtacaagaagctcggcgtgaagctgctcaccggccacgccaccaccgaggtgcgcgacaacggcgattccgtcgaggtcgacgtgaagaagaacggctccgacgacgttgagaccctcaccgccgaccgcgtcatgatctccgtcggcttcgccccgcgcaccgagggctacggcctggagaacaccggcgtggagctcaccgaccgcggcgccatcgccatcgacgagcgcatgcgcaccaacgtcgagcacatctacgccatcggcgacgtcaccgcgaagctccagctcgcccacgtggcggaggcccagggcatcatcgccgccgagaccatcgcggacgcggagaccctcgagatcgaggactacatgatgaccccgcgcgccaccttctgcaacccgcaggtcgcctccatgggctacaccgaggagcaggccaaggagaagtggccggaccgcgacatcaaggtcgccaccttcccgttcagcgcgaacggcaaggcagtcggcctggcggagaccgctggctttggcaagctcgtcgcggatgccgagttcggcgagatcctcggctgccacctcgtcggcgccaacgtctccgagctcctgccggaggtcgtcctggctcagcgcttcgacctcaccgcaggcgagatcgcccgctcgatccacattcacccgaccctgcccgaggtgatcaaggagatcgcgcacggcgtcgaaggccacatgatcaacctctaaggggcaggtgcttggcgacggggcgagcgtcgccaagcaaagcccaaaaaagctcccgcacagcgtcgcgccgtgcgggagctttttgggctctctagttgtcggtgccggcaacagccgcagcgagggagtcgagcgacttcgccaggaagtcgtcgtcgaacttctcgctcatcttgcggacctcgtcggactcgatctcgtcgcgctggtaggtcagggtgacctcggtgtggtccgggtcgaccggctcgagctcgtagagccacttggcgccgaccttcacctcggcggtggtgttctcgacgttcttccatccgataacacggtcctcctggaaagcgaagacctcgttcttggtctggtagtcgccgtcctccttggtcatgttcatggtgaaggtgtcaccgacagccttcaggcgctcagcctggtctgcggagaccaccatgccggagtcgtctgtttccttgtggcgctccgggttggaaaggatgtcgaagatgtcctttgccggtgcgtcgatggtgcgggttgcggagttctgattcgttgcttcagtcatgtgcccaagggtaccgcgtttcgccataacgcgaggtaagataatacttaccaaccaaaggttgacgctgaaaggggtggcagcagtactttgtgcgcaatatcacaattggcgcgatttgcgggaaaatggcgcgactaccggctctgagtggcgtccgatgattgaagctgtaaggagccggggagatgcctgaagaaaagcgccggccaaaaatgtgtgggggcgcggcgccttccttaaagtgaaaccgacactggaggtgccatgactgtacaaaacgcagaccgtgaggccattcgtcacggaaaaattaccgaagcgccgctgcgcgagcggccatctttcccaacttgggctgtcaaactcaccatggccatcaccggcctgatcttcgggctgtttgtgctcggccacatggtgggcaacctgaaaatcttcatgccgcttaacgccaacggtgttgcgccgatcgacgagtacggcgagtggctgcgcacgctgggtgagccgctgttcccgcgggagggcttcctgtggattgtccgcattgtgctgctcgcctgcctggtgctgcacgtgtggggcgcgttcgcgctgcgcgcgcgttcgtccaagtcgcgcggaaagttccgccgcaccaacctcatgggcggctggcagtccaccgcgacccgcgcgatgctgaccaccggcgtcatcttgttgctcttcatcatcttccacctgctggacctgaccatcggtgaggtcgtcgcgtctgacgagttcgtccacggcgctgtccgcgacaacctgctggccaccttcgcgcctgcgcgttggccggtcaccctgttctacgtcctcgccatggttgcgctcgcgctgcacctgacccacggcgtctacctcgcggtgtccgacctgggctggctcggcgagcgcggtcgcgggctgatggtgctgctcgcctacgttcttccgctcatcgttgtcattggcaacatcgtcatgccgatcgccatcgcattcggctgggtaccgggatttaccaggtaacggctgtttaggagaaaaactatgactacctcaatcaacgcggcgcagggcgcttccggcgaccagctgaccgcttctgccccgcagggcgcagacgtcaccggcggcttccgccagccagagtccgcagtttccggtgtgaccatcggcgaggtgctggcgagcaacgagccgaaccgcgacgaagttcggatgcgcgacatgtgggagtaccagaaggaccacatgaacttggtctccccgctgaaccgccgcaagttcaccgtcctcgttgtcggcaccggcctctccggcggcgccgccgccgccgcgctcggcgagctgggctacaacgtgaaggtcttcacctaccacgacgctccccgccgcgcccactccatcgcagcgcagggtggcgtgaactccgcccgcggcaagaaggtggacaacgacggcgcgtaccgccacaccaaggacaccgtcaagggcggcgactaccgctgccgcgagtccgactgctggcgcctggccatcgagtcggtccgcgtgatcgaccacatgaacgccatcggcgcaccgttcgcccgcgagtacggcggcaccctggccacccgttcattcggaggtgtgcaggtgtcccgcacctactacacccgcggccaaacagggcagcagctgcagctgtcgaccgcgtccgcgctgcagcgccagatccacctgggcaacgtggagatcttcacccacaacgacctgatggatctgatcattacggaagaggacggcaagaaggcttgccgcggtattgtcacccgcaacctgatcacgggcacgatcactccgttcaccggccacgccgttattctcgccaccggcgggtacggcaacgtgtaccacaagaccaccctggcgaagaactccaacgcgtccgccatgatgcgcgcgtacgagcgtggcgcctacctcgcgtccccgtgcttcgtgcagttccacccgactggtcttccggtcaacgccaagtggcaggcaaagacgacgctgatgtcggagtcgctgcgcaacgacggtcgcatctggaccccgaaggagaagggcgacgaccgcgacccgaaggacatcccggaggacgagcgcgattacttcctcgagcgccgttacccggcgttcggtaacctcgtgccgcgcgacgtggcgtcccgcgccatttcccagcagctgaacgccggctacggcgtgggcccgctgcacaactccgcgtacctggacttctccgacgcgattgagcgcctcggtgaggacaccatccgcgagcgctactccaacctgttcgaaatgtacgaggactccactggcgaggacccgtacaaggccccgatgcgcattgcaccgaccgtccacttcaccatgggtggcctgtggaccgacttcaacgagatgacctcgattgacggcctcttcgctgccggcgagtgctcgtggacctaccacggcgccaaccgactgggcgcgaactcgctgctgtcggcgtccgttgacggctggttcacgctgccgttcaccatcccgaactacctggcgaaccacctgggcgaggaagtgctctctctcgaggcgccggaggtggccgaagccgtcacccgcacccaggaccgcatcgaatccctgatgcgcatccaggcggttgagccacacggcccggaatacttccacgagcagctcggcgccatcctctacgagttctgcggtgtgtcccgcaccgtcgagggcctggaggaaggcatccgccgtatccgtgcactgcgcgaggacttctggcgcaacctgcacattccgggtaacccgaacgacatgaaccagaccctcgaggcggcgctccgccttgtggactacatcaacctcggcgagcttatgtgcgtggacgcgttggaccgcgacgagtcgtgcggtgctcactaccgcatggaccacctcaccgacgacggtgaggccgagcgtgacgacgacaactggtgcttcgtctccgcgtgggagccggccggcgaaggccagttcatccgccacgctgaacccctgttcttcgattcgatcccgctgatggcaaggaactacaagtaaatgaaactgacacttgagatctggcgtcaggccggacccgataccgacggcagcttcgaaaccgtccaggtcgacgacgctgtcgagcagatgtccatcctggagttgctggaccacgtgaacaaccgctacgtggaggagggcaaggagcccttcaccttcgcgcacgactgccgcgagggcatctgtggcacctgcggcctcacggtgaacggtcgcccgcacggcgccggccagaacaccactgcgtgtctgcagcgcctgttcaactacaaagacggcgacaccctgaagatcgagccgttccgctccggcgcgttcccggtgatcaaggacctcgctgtggaccgctccgcactggaccgcgtgatgcagcagggcggttacgtgtccgtcaacgccggcaccgcaccggacgccgacaccctgcacgtcaaccaccacgacgccgagctcgcactcgactacgccgcctgcatcggctgcggcgcctgcgttgcggcgtgcccgaacggcgcagctcacctgttcaccggcgcgaagctgaagcacctcaagctgcttccgctgggccagcaggagcgcgcccgccgcgcccgcaagatggttgacgagctggagaccaacttcggccactgctcgctctacggcgagtgcgcggatgtgtgcccggcaggcatcccgctcgacgctgtcggcgccatcaacgcggagcgcgcacgtgctgctttccgtggcggcgacgactagagcatgccgtatagtggctaactaggtacaagatccggatctttccaggaaacgtaaggacatagacatggcttcccagcacgcggttgcagacatccagtcggagtcgttcccgggctaccagacccagctgcacgactcgtacatcgagggctacgacccggtttcgctgggcgcgccgcactcctccctgtcccgctactccacgtgggtgtcgatgggcctgatcctggccaccctgttcggcctgggcatcctggtgtggggcgctggcgcgcacttcgtgggctggggcgctcagagcgaggacttctccagccgcctgatgatcctcggcggcatcgagatggccgtgtgcattgtggctgccgcggtgctgctgtccatgggccgcaaggactacaagaactaccgcaagaccacgggccgcgtgaactaacgcaccgcgcgtcgtaagcgaaggcgcttccctcccaaagccgggtagggaagcgcctttttcgctggtttcaggtgatgttgggcagggctgctttaatcgacagcatggaatcgctacccctaatgccggcgccgtccaacgaggtagagcgccggcgcgtgttgcgcaaccacaagatcttcgtcaccagtctgcttgcaatggctgcggtgatcttcctcgcgtgctcgtggtggcagtcgcgcggcggagcaccggggtgggttgggtacgtccgcgccgcggcggaggccgggatggtcggcgggttggcggactggttcgccgtgacagccctgttcaagtacccgatggggatccccattccgcatacggcgatcatcccgaacaagaaggaccaggtcgccgaggcactgagtgagttcgtcagcgaaaacttcctcaatgcgcgcaccatcacggacaaggtgatgcaggcgggtatcccggagaaagccggccgctggctggcgcaggaggacaacgctgcgcgggtgagcgcggaggcgggaacgttcgcggcgaacattgtcaagggcattgacccagcagacgccgaggcgctgatcgacacccaagtcgtagaacgggtctcggaacctgtttggggcccgccgcttggccgcatgctggagggcttcatcgccgacggcaaggtggagcccgtagtcgacgacatcgtcgcatggggcaggcgcaagcttgacggcatggaagacacgatcgtcaccgcgatcgacgagcggatgccgaagtgggcgccaaagtttgcgaaggaactggtaggggaccgcgtctaccgggagatgacggagttcatggaggacgtcgactctcagcccgagcacgaggcgcgccgcgcgattcgccgcaccatcaaccagttcgcgcaggacctgcagttcgacggcgacatgatcacccgcgtggaggaactcaagcacgacatcatgggctcgagcgcggtcgcgtccgcggcgggcggaatttgggagcaggtgtcggccgcgctggtagcggcattgacggatggggattcgacgttgcgtcgaaaagcgcaaagctccatccaggattggggcgcgctgttggccaccgacccgcaggtgcgctcccaggccgaaaagcggctggagaaagccgtgcactacgcggcggagaacggcgcgggacagatcgtcggcatcatcgcggagacgatccaacggtgggacggcgccgaggccgcggacaaaatcgagctcatggtgggcaaggacctgcagttcatccgcctgaacggcacaatcgtcggtgcgctggccggcttagttatttacactgtgtctcaactgctgttttttacgtaaggagcaccccatgaccgagcacaacaacatcaacgacaacatcaacgagaacctcgaggccgctgcagagtccacgaccgaggagacttcctccgaggtgcgcgacaacctccgcgaggcgggcgacgcgctcttggcagccggttccgcgatcggcgccgcattcggcaagttcgctgagggcctgccggagcgtttcaagatcgcatcggattccgcgcgcgagaccctcaactcggcgaacaccgagggtgaggtccgctcctgggccgccaacgtgaccaacgaggcggagaaggcttttaactcgctgcgcgagcgcgacctgaagttcaccgacgacgcgaaggcatctttgagcaagtcggtcgccgacatccgccagtccttcaacgagcgcctcgaccgcgtcgacgcgtccggctccgagaccgcggagagcaccctgaaggatctgcgcacccgcttcgacgacttggtcgagcgcattcaggaccagttcaccagcagcgaggacgctgctggccgccacgaggccggtgatatcatcgacggcgaaatcgtcgacaacgagggtggcagcaccgccgccgacctgaacaagtaacggagatccgcctgcatggatgcatcagccctcgatcaaatcaccacgatcatgcgaatccccgtggtggctgagcgcatcctcttcgtcgctgtgggcgtcgccggcatcgcgggtgtcatcttcgcatccatcacgcgggccgacgcgttcgaggcagcgggccgccagccgaagatgacgtgggtcgcgattttggctctgtccacgttggcgctgctgttgcggctgccgttcatcgcgtggttcgcggccgtagcggtgggtatttactacttcgatgtccgcccgcaggtcagagagatcgagggcaacagcggcggcgcttggtaacccgctgcgaccagcccacttttagccggcgtaggccggcttttcttgttgctgggtgccctgcggcgatggcaccaaggactgctgcagctcgttgaagttcacgttctcgccgctcagctgcatctgtaagccgtccggggtgacggcgacgtcgctgaggtgcatctgcgagttcccgaaggacgccatcccttcttcgagcgagttgttgatcacgcctgcgacctcgctgggcaggttgaagccgaagagctgggtgctctcggcttcgaacgagaccccgccgcccgtctgcgccgggcgcagctcgataccggccacaccgctggtgaacagcacggtgaaggtgccgtttgctggatcggtggtcacctcggagacggtgatcaggctgtccagccagcggttgtcgcccagctgttcgtgcagcgactggtttagcgtggcgcgcaggaagtcgttcggcagctcggtggtaagtgtgaaggcctgcgccaccggctcgccgtcgacaatgttgaccttgtccattttgatggtggcgccgggctcgccggagatcgtgtcgccgctgactgtgagcgttgaaggggtcgtcaccgtcaggtgcggtagcgacccggtgagcaggcccagcgtgaccggctgcgagccgaaggacacctccggttggccggctgcgaccgcctggccggcagattgctgctcgacgcctttggtgatctggttggtgaggaacatgcgcaccccgatctcggcgacgatcaggagcaccagcagcgccgcgagaattccgacgatgaccttccacgctgttttcatgcggttcagtctacggatggcgcgacagcggcccaatcgactgtgagcgcgttgtctctcagtcggcgccgctgcggcgtgacgggccagccgcggcggatcagctccgcttgcgcttcgcgccagcgcacgcgcgggccgtggggtgcccatccggcggcgttggcccaagcggcgtcggcgtcggcaagcagcgcgtggatggcctctccctccacgttgcggtggatgagcaccttgggcagccgctcggcgacgtcgctgggggaggcgacgtcgtgggggtcccaggccagggtgagggttttgggccccgcggcgtcgagaagcacccaagccccccggcgaccgagctcgtcgcaggtgccctcgatgaacaacccgccgggcgcgaggcgcgagcagacttcctcccacacgtcggcgacatccgccacgtcgtactggcgcagcacgttgaaggcgcgcacgagctgcgggcggtacccggcgagctcgaacccgccaagctcgaagcgcacgcgatcgcgcggcggcagaactcgctgggggtcgatctcgaggccgaccacctctacccgcgggttgatctggcgcaaccacccggcccactccaccgtggtggtgtgggaggcgccgtagcccacatcgagcgccagcggctgcggaaccgagcgcagaagcgattgcacctgcgggttgaacctggtccaacgatcacagcggcgcaggcggtttaccccggtggtgccgcgcgtgatcacgccgtacggctttccggggcccgcctgcgcccgcaggttgtggtagtgcgccatcagcgcttttcgttggaaagtgtgaacagggttagaggttttcggagatccactgctcggtgagcttggcctcgttgcccacgatctcctccagcgcctcggccaccttcggctcgagcgccgcgcccatgaaggggatgtccaccttgacctcgttgtcgtacgccagggtggtggtgtcgccttcgccggtcatctcgatctcgccggaaaagtccaccggggtgcctttcacgtcgccggtgaaggtgtgggtggcgcggccgccgtcgagctcgccgatgttcactacgcgcttgagcttcaggtcctgggaaatcatggcctgcgcggcggccggcatgatggacttcggcaggatctcgaacagcacggcctggttgcccgtgaactcgttgagcgagcccggctccggggagagcttctctgcgatgaactcccagtacgccttggacgcgtacgcctcggcgaccttctgtgccgggtggttgatggtaacggaggtttcgctacgtacagtcatggtcaacagactaccgtgagataggtgcaggacttatctttcgcccatctgaccacactgcgcgtcggcggcacgcccgtggaggtgaccgcgtgcacctccgccgcagaaatcgcggagacggtcgcccggctcgacgccgacggccgcccgcttttggtggtcggcgggggatcgaacttggtagtggctgacggtccgctggatcttacggcggtgctggtgcgcaacgagggcatttcgcttgtcgacgccaccaccatctccatccaagccggcaccccgtgggacgacgtggtcgctttcgccgtcgatcacggcctcggcggcatcgaggcgctttccggcatccccggctccgcgggcgcgaccccggtgcaaaacgtcggcgcttacggctccgagatctcggacgtgctcacgcgcgtgcgcctgcacaaccgggagaccgggcgcgacgagtgggtcgacgcgtccgcgctggacttggcctaccgctactccaacttgaaattcactaaccgtgccgtggtgctggagatcgagctgaagcttaaccccacggaccgctctatcccgctccgccacttgggcgggcgcgaggtcccgctcgctgaagcccgccagtctgtccttcagacccgccgatcaaagggcatggtgctcgacgccgccgaccacgacacgtggtccgctggctcgtttttcaccaacccggtcgtgccggccgcgctcgccgaagagatcgagcgcagcgtgggcgaggccgccatgccgcgctacgcggcggccgacggcaccgagaaactgtcggccgcgtggctgattgagcgcgccgggttcccgcgcggctacccgggtgagggcgcgccggctcgcctgtccaccaagcacaccctggcgctgaccaaccgcggcggcgccgccgccgacgacatcgttgcgctcgcgcgggatgtgcaggcgggcgtgaaagaccggttcggtgtggagctccaccccgaaccggtctggatcggtttctagcgctggtcttccgccagcagttcgagcagtgaatcgcgcacctcgcggcggcggaccttccccatctggtccttgttcagctcctcgaagtggtagaaggtgcgcggcaccttgtagcgggtgaggttttcgcgcgcgaaatcctttaagccctccgggtcgagcgccgcgccgtcttccagcacgacacaggcgacgacgtcctccgaaccgtccttgcgcgggcggccgaccacggcgacgtccttgacgtcgcggtggcggcgcatgacttcctccacctccgccgggtagacgttgaagccgccggtgatgatgagttctttgatgcgggagacgaggcggacgaaaccgtcctcctccatcactcccatgtcgccggtgcggaaccagccgttgtggaaagccttctccgtggcttctgggttgttgaggtagccgccgaaaacctggggtcctttcgccagaatctcgcccgcctcgccgtagggcatcagctcgtccgggttgtccgggttcacaattcgaatttcggtgtcggggaaggggatgccgatgtagccggggcggcggtctgcgcttcgcgggttgccgatcaggatcgggcctgtctcggtcagtccgtagccctcgaccaggtagccgccggtgagcgcctcccagtcctcaatcacctgagccggcagcgaggacgcacccgagaagccgatctgcaccttggaaaggtcaatcttcttttcctttgccgtgctaatgatgcgctcgaacacggtgggcacgcccggcacgaaggtcggggtgtgcttcttcatcgcatccatgatcagttccatcttcggggccgggatcaggatgagctcggagccgaccaggatcggcagcgtgagcgagaacgcgaggccgtaggcgtggaagaagggcaaggtggcaagcatgcgctggcccggttcctgcagctctttcgcccacgcgcggccctgctgcgggttagccagcaagttggtgtgggtgagtaccgcacccttgggcgcgccggtggtgccggaggtgtaaagcaccagtgcgggggattcggcggtaacgctttccgggatttccaagtcggcgccttccccgccgatagcagagctgaccagcgcttcccacggcacggtgttggtggaggggccggtcagcgatgcgcgggcttcgcgcagcttcggcagcgggaggcgcagggcgaagcgctgcagcttcggcatcgccttcgtcatatccacgctgaccacggtctccagcggggtgtccacgcgcagctgctcaagcgtgtccgccgccttatcccagacaatggccacacgggcgccgtggtcgttgaactgcgggcgcagctcgttagcggtgtagagcgggttgtgctcaacgaccacgccgccgatcaggtgcaccgcgtagaacgcggcgacgtgctgcgggcagttcggcagcatgatggccacgcggtcgccggggcgcacgccgaaagctttgaggcccgccgcggcgcggcgcacctcccggtcaagctcggcgaacgtgtgcgtgcggccgaagaagcgcgtcgccggtttgtgggcgttgcgctcgagattgtccaggtagatctccggcagtgtcttgttgctgtactcgagcgtgtggtccgtccactcggggtagtactgcagccacggctgcgtctcgttggggtccacgccgggtgcgtcgttgttcaggggcgtactcatgcggacaacaatacgccaaacctacgcaaccgtaaggtacgagcccgtaactttcttcgggagcgctacgctagctgcatgcgcgtcgccatgatctccatgcacacttccccgcttgagcagccgggcaccggagacgccgggggcatgaacgtctacatccacaacatcgcgacccagctttcgcgccagggtgtggaggtcgacgtgttcacgcgcgccacgcgccccagcctcggtgagatcgtcgaggccgcccccgggtaccgggtgatccacatcgtggctgggccgtacgaagggttggagaaggacgagctgcccacccaactcgcggccttcgcgggcgggatcatccagttcctgcgcaccaacggccacggcggtcacgcgctcgagtacgacctcatccactctcactactggctttccggtcaggtggggtggttgctggcagatctcatcggcgtgccgctggtccacaccgggcacacgtgggctgcggtgaagaacgcctctggcgttgatggcgcagaaagtgaggctcggcgcatctgcgagcagcagctggtggacaacgccgatgtcgtggtggtcaacaccgccgacgagaccgagcagctcgcccgcttctacgacgtcgacacggagaagatcgccgtggtcagccccggcgccgatacggaacttttcacccccggcaccgaccgcaacacggagcgcgcccgtcgcgcgctgggcatcccgctgcacgcgaaagtcgtcgcttttgtgggccggttgcaggatttcaagggtccgcaggtgctcctgcgcgcggtgggggaggtggtgcgccgcgaccagttggacgcccccttacggttggtgatgtgcggcggcgcgtccggcgcgggctcgtcggtggagcactaccgcgccatcgcccaggaagagggcatcgcgtcgatcactcgcttcctcggcccgcgtcccccgcaggagctggcgagcgtgtaccaagccgccgacatcgtggcggtacccagctacaacgaaagcttcgggctggtcgccgtcgaggcgcaggccacaggaacacccgtggtggcagcgcgagtgggcggcctgccgctcgcggtggcggacggcgagtcgggggtgctggtggcaggccacgaccctgccgattgggcgacggcgctggagcagttgcttatcgacgaccacctgcgcatcaccatggccaccaccgcagtggcgcacgcgaagaaattttcgtggcgcgcgtcagcaagcgagctctacaaggtgtaccaaaccgtgctcgacgggttcgacccgcaggccgccacccgccagccggccggggtttagccgagcagcttctgctggagggcgagctcgcccagctgggtgagcttgccggcgtggtagcccgcggtgtgttgcgcctccgcgatgtcgaggttgccgcggagcgcttcgtccacaatgcgctgggcatcctgctgtgcaccggcgatcgccttgtccagctccgccttcgggtcggtttgcgcgagatccgggttcatcgcctcgatttgctcgcccatgtcagcgaactcctcagccgcagtcggaagcgcagcgtgcggggcggtggactcggtcagtgtgaagtggtcgttgaccgcgccgtccgggataccgtaggcctcctcaataatgcggtcggcggcctgcgccttacccagcgggccgagcaccatggagctcacgccgatcacggagttgtctcgcgggtcgtagttcacgccgccggagtcgcccaccacgtagttcaagtcccaggagaagacgccgtcgcggttccggaacagctgcgtgccgcaggtgcggccggtggtggatccgtccttgcagatcggctggccggcgttgtcgaaggagatcgcgccgggggctagcgtgcggtagtccttgatcgaggtcagcaccaccggttcagacggttgcgcctggccgttgccgcgggactgggcggtgcgtgtgtcggtcaccccatcgtcgatcagcacgacgccccagtccgccgtgttgtaagtggccaccgggtccgacaggtcgagtgccgccggcggcacgtggttggagtggccgcgggtgccgatgcgctggtactccccgtcgacgttgacactgacggcgtcgtccatcgcaggcatgcccggcatcgggttgatgcagtgcgaagcggtgagcatgacgtgctgcgtcgtgccatcgagggtgcggatcgtgccaatcgggccctgggaacacaactggacgaacgcctccggcggcaccttcacctggtccccgtagacgttggtgatggtcgctggcgggttgaccggcagcatgcgcatcggcgcgccgggagcggcgagcgccggctctgctgcatgtgcggcgggaacggcagaaaacgacagtgcggctgcgatcatgcccgcagccgctcgtgaaaacctcaagttcatgccggtcagtctaaagcatggcatgctttattacatgggtaacggaaagctgatcctggtccgtcacggccagagcgagtggaataaatccaaccagttcaccggctgggttgacgtcgatctgaccgagcagggcgaggccgaggccgtcaacgccggcaagctcatggtggacaagggcgtgctgccggatgtggtgttcacctcgcttttgcgccgcgcgatccgcaccgccaacatcgcgctgaacgccgccgaccggcactggattccggtcgagcgcaactggcgcctcaacgagcgccactacggcaagctgcagggcctgaacaaggccgagatccgcgaggaattcggcgaagagcagttcatggagtggcgccgctcctacgacaccccgcctccggagatcgacaccgacaaccagtacgcgcagaccgatgacccgcgctacgcgtttctgcccgaggtgccccgcaccgagtgcttgaaggacgtggtggaacgcttcctgccgtactacatcgaccgcatcctgcccgaggtgctcgcgggtaagaccgtcatggtcgcagcccacggcaactcgcttcgcgcgttggtgaagtacctggataacatctccgacgacgacatcgccgggctcaacattccgaccggtatgccgttggtctacgagttcgatgaaaccggccgtgttaccaacccgggcggcacctacttggaccccgaggcggccgaggctggcgctgcggctgtggcgaaccagggccagaagtaaaccgatagggaggtagcgacaccgtgggtgtagcacccattgtcgcgttcctgctcggcgcggcgctcgccgtattggcgtgctggatgtactcctccgtgcgtagctggcgcgaccgcaacagctcggcggagtccagcaacgacgacgagatccagaccgtcagccagcttctgaatttggcggtccagggctcgccgacgggcatcgcaatcttcaaccgctccggtcgcgtcatcatgtcgaacccgcgggcgcacgacatgtcgatcgtgcacgaccgcaccatcaaccccgaggtgtgggacgcggcgctcgtggcgttcgtcgactccgagacgcacacgctggatcttgacctgccaaggcgggcgaccggcagccgcatccgcaacgtgtcggtggtggtgaagccgctcgcgctgacccagagtgcctacgtgatcgcgtacgccaccgacgagagcgagaacgtgcgcatggagtccgcccgccgcgacttcgtcgccaacgtctcacacgagctcaaaacaccggtcggtggcatggccctgttggcggaggccctgctgcaggacccgggcgacgaggagatggtggagcacttcggccagaagctggtgaaagaatcccaccgcatgggcgagatgatcacggatttgatcagcctgtccaagctgcagggcgccgaagcactgccggagatggtgcccgtgagcatcgacgacgtgatcgacgacgccatcgagcgcaaccacgtcaacgccgaaagccgcgagatcgacataacccgtggtccgcacaccggcatccgggtgatgggggaccgcccgcttttgacggcggcggtgtccaacttggtctcgaacgcgatcaattactcgccgaacgggcagccggtgagtatctcgcagaaggtggtgcgcgagaacgtcgtgctggtccgggtgaccgaccgcggcatcggcattgcgccggaagaccagaagcgcgtcttcgagcgtttctaccgcgtggacaaggcgcgttcgcgctcgaccgggggcactggtttgggtttggccattgtcaagcatgtggtggcaaaccacggcggtaatatcaagttgtggtcccgtcttgggacgggctctacgttcaccatcgagctgccgatttaccagcctgacagccggccggagaacacgaagggtaaccaagagaagtgacgacaattctcatcgttgaagacgaagaatcgctcgcggaaccgctcgcgtacctcctcaacaaggaggggttcgagacgatcatggccgccgacggcccgagcgcgctggagcagtttagcgacgacggcgtggacctcgtcttgctcgacctgatgctgcccggcatgagcgggaccgacgtgtgccgcaagctgcgcgccgagtccgacgtgccgatcatcatggtcaccgcccgcgactctgaaatagataaggtcgtcggcctcgagcttggcgccgacgattacgtgaccaagccctactccacccgcgagctggttgcccgcatccgcgcggtgctacgccgcggcccggagatcgaagaagttgaggagttcgacgaccagattatcgagggcggtcgagtgcgcatggacgtcgagcgtcacacggtgtttgtcgacggggcgcccgtcgccatgcctctgaaagagttcgacctcctcgagtacctgatgcgcaacgccggccgggtcctcacccgcgcccagttgatcgaccggatttggggagccgattacgtcggcgacacaaagactctggacgtgcacgtcaagcgcctgcgcaccaagattgagaaagagccctcgcgcccgacccagctggttacagtgcgaggcttgggctacaagttcgaggcctaagccccctcgcgctcgtcggcggcgcgcgttgctgggtgcaccgccttgacttcggcgggaagcgctcggcgtgcccggcagtgcgccgccaacaccgcgtagggttcctcgccgatcaatccgattaactcatctttcatcgtgacccacaccggctcgcgtgtgccgtcggaggtttgggtgtggcacgtcgggtcggccgtgcaccaccaatcgaagtcctcgcccccgccgccccactgacgacggtcgtactcgccgatggtggtgcgcagaatttcctggccatccgggcgctcctcccactcgtcgactcgggagaatggcacctgccagcacacctctggcttcgatccgacgaggttcttacccgcagccaccgcccattgatgcagcgcgcagcccggccccgtctcggcgtcgcttcggttggcgaagatgcacgcgccgtcgataaccttcgtttttactgacggttcttcatcatcgtcgtcccactccagccacggttccagctgggttgggtcggggttggccaggtactcgtcgacacccgcggggcgaagctgccagaagtgtgccggcaagtcgccgacagcggcgtagagatcgtcgcggtcggtttcgtcggcaaggtacgccccgtgcgtgcagcaaccaacaaccggcaagtcagcgttcacgccgtggcactgcggtgtgccgaagcggcaggaccacgtcgattcggcccatgttaagtcaatggagaacgagtgcagcggatcttccggatgtacgaactcgaaccactcgcgggggaaatccgggggcagctcccgcccagcggcaatagacctcccagcgggggaattcacaggaaatccaaggaaaactggttgagaggctggttgattcacaccttggtaccgtagacccgttacgctggctgtgtgcgtttaggtgtattggacgtaggcagcaacactgtccatctcgtggcagtggatgcctacagcggcggccggccaaccccgatgtcggactggaagcaaccgcttcggttggtggagctgattgataaagacggcaacatcgaagacaagggcgtggacaagctcgtcggcgctgtccaagaagcctccgacctcgcggacaacctccgctgcgaggagtttttggcgtttgctacttctgctgtgcgctccgcctcgaactctgacgcggtgcttaagcgcgtggagaaaaaaaccggcgttcgcctgcgcgtgctcagcggggaagaagaagcgcggctgacgttcctcgcggcgcgccgctggtacggctggtcagcaggtcgcatcaccaacttagatatcggcggcggctcactagagatgtctaccggcaccgaagagatccccgacctcgcggtgtcgctcgacctcggtgcgggccggctcacccacgagtggtttgacaccgatccgccggagcgcaaaaagatcaacctgctgcgcgactacatcgacgcagagcttgctggccccgctgagcagttccgcgccatgggcgaagccggcctagcagtcggcacgtcgaagaccttccgctcgcttgcccgcctgactggtgccgcgccgtcatctgccgggccgtacgttaagcggacgttgaccgcgccgggcctgcgccagctcatcgcgttcatctcccgcatgaccgctgcggaccgcgcggaactcgagggcatcaactcggatcgttcccaccaaattgttgccggcgcgctggtcgcggaagccgcgatgcgcgcgctaaacattgataagttggaaatctgtccgtgggcgctgcgcgagggtgtcatcctgaagtggatcgaccaggacaccgcagccggtgccggaggaatggatgaaggagcggacgactgatgtctgagcagaagcaactcaccgtcgcggagatcctggccaaggcgcaacaggagaaccccgaggcagggacgcgccggcgtcgtcgtcgcagcttggaagacggcggtgtgtccgtcgcagaactcaccgggtccttgaagaaggtcgaggccaagccggtcgagtcgcgccactcttccgtgccaatcgacgcgccagagccgaaggttgaaaagccgaagacggaagtgccaaaggtgccgggctccactcgatactctgcgcctgcgccgaaggaggcgacgccgaaggctgctgcgcccaaggctgaggcaccgaaagctgcagcgccaaaggttgaggcgccgaaggctgaggctgcgaaaccggcgcgtgaagagcagacaggcgaagagacgacggttctgcgcaaggttgccgcaccggagccggagcgtgtcgatcgcgtcgagcctgtggcagaggcgaaggaacccgcgccgtcgatggcggagacgtcgccgaatgcagtgccggtggtggaagttcccgtcgaggacaccgatccggttgaggttactgaacctgcggatgaactcgacgagttcctcgagcctgagactgttcccgccgatgagatcgtggttgaggaggagggcgtcaacccgatccttctggtcctactggttttcctcggcgtgcttgtcggtgtcgccggcttcctgctcttccagtggctctgggcgaacacctcggccatcctcgcggcggtgctgggcatcgctgctgtcgccggcgcgatcttcggagcacgcgcgttgggtaccggccgcgattggctcaccaccgcgctggcgggtatcgccgcgatcgttgtcgcattcggccccgcactgctatagatctctccccttaccgttcaccccgcctctaggccgccgcctagaccggcggggtgaacgtgtttaggcttggccggtatggacacaccagaggagactgtggagcaaaccgcggtggagcaggcgaagggcgttcgcaagatcgcagtcatcggagccggcaacatcggcgaggcgctgatcgctggcttgatcgacgcggacgtagacccgaagacaatcaccgcgacaaaccgctcggcgcagcactcggatgagttggccgcgcgctaccaggtccacactgagaccgacaaccgcgaagccgttcaggaagctgaagccgtctttttgtgcgtcaagcccgcccagatcggggaggtgctcgaggagatcggcgaggttgtcgaaggcaacgacgtcgcgaccgtgctggtgtcgatggcggcgggtgtgaccctaagcgcgatggaggcggcggtccccaccgccggtgcgccgctcgtccgcgttatgccgaacaccccgatgctggtgggcaagggagtcttcgcagtgtcgtgggggcgctacgtcaccgaagagcagcgccgggtggtgcgctgcctgctcgcctccgctggcgaggttgtcgaggtcgccgaagcgaagatggacgcggtgacggcgatttccggctcaggtcccgcgtactacttcctgttcacagaggcgctaatcgacgccggcgtttccctcggcctaagccgcgacttggctacccagctggcgacatccacggcggagggggcaggtgtgatgctttcaggcccagtctcgccggctcagctgcgcgcggcggtgtcgtctcccgcgggcacaacggtgcgcgcaatccgcgagctggaggaatcgggtttgcgcggcgcggtctaccgagcaactgaagcgtgtgccgcgcgctctgccgagcttggtctgtagcccgcccgcttcgtcccgtgaatcacacgagcgatctcacagcactttgaaaaatttttagatcataagtcgcgcgtggcacaaggttcacggtaggctcgcgtgagcacgtgcgtgtccgtcctgtgggaggggaagcctacagcgcgcctaccgtgcggaaggttaataacatggcaaatgaagagaagggtaagttccttaccgtcgcggaagtcgcggagattatgcgcgtttccaaaatgaccgtctaccgcctcgtgcactccggtgagctgccggctgtgcgcgtgggtcgctcgttccgcgtgaacgagaccgcggtcagcgagtacctcgagtcctcggtgtacgacgtgggaacggatgcggtctaagcctttgcgcttagctccgcaccccaaagcccgtccggcgccgccctttgggtgaggcgtcggacgtttctctttttgtctccagcgaggggcactgggtaagctgttacccattccaaccggcctggcctgccggtgaacgagtacatgtaccgatttgtagaaacgaggcaaacccaatgggttctgtaattaagaagcgccgcaagcgtatgtccaagaagaagcaccgcaagatgctgcgccgcacgcgcgttcagcgtcgcaagcttggcaagtaagtcttctgggcttcacaccgtctccgcagcagaaactgtctgcagcgggggcggttttttatgcctgacggtggacagtgctcgatctggtggacccgtggctgtgacaggtgttgcgaaattctgccacgcataatccgcggcagcttctcaacctgcgggtgtggcccgtggggctggtggggcgaaattatgcctcgcataatgtcctggggaaacgcggtgggtgacggtcaactcggcggggaagtgtcctcgcggggttgatgctgctgttgcaggtggggtgaaattctgccgcgcataatccgcggcgggcttctaacttagagaagcctcacccctcggctctggcctagcggcggcggttcagtgcgaaggcacccgcgccgagggcggcgacggcaagagctggaagcgcgtacgagcgggtgacgcggcgcatggagcggtagtcgcggatggcccacccgcgggccttcgcgtgctggcgtagttttctgtcagggttgacggcgatgggctcgccgaccatctcgagcatcggcagatcgttgaccgagtccgagtatgcagtgcacttgcctaagtccagctgctggattgcagcgagcgcggcgacggcgtgcttcttgcccggtccgtgcaggatgtcgccgacgaggcggccggtgaacaccccgtcttcttcctccgcgacggtgcccagcgcgccggtgaatccaaggcgctccgccagcgcctgaccaatctgcacaggagtagcagagacaagccacacctgttggccagctgcgatgtgcatcgcgccgagctcgatggtgtcctggtacgccttggtcagcatgtgccggtcgacgatgtcgcggcacagctcctgaagttcggcgacagacttgccgcggacgatggcgagagcttgctcgcgaccctcagcaatgtcgtcggcgttttcggagccggagatgcggtagcgcagctgcttgaccacggcgggcaggagttcgcgaattgagatgaaacggcgcttggccagctcttcggcgagcaggattaacgacgagccctggatgagtgtgttgtcgacgtcgaaaaaggcggcggcgccgacatcgactgggatgtccgggtcgggctgggtcagatgcgggcgaccggcagtcgcgaacgcgccgccgacggagtgcacgccgagggagaagtcctcgatgctgataccgaacgtctcctcgatagcggctgcggctgcggcctcgccggcggtgcgctgggatgcttcgtcgatcgggggcagagcgcggtcctcgaaaaaacggcgcaagttaccgtgcgagacgctccactgcgaaagcagctcactgggctcagccatggctttccttaaagcccgcctttctgctgttagcgtgaacggattagttcatggtaccggatggtggcgctgaggaagacgaggaggaacgggtgtgaagacggtcgagattatggtgcgcgaaggctgcggttcgtgtgtgagggtggctggggaggtgcagggcgtcgtcgataagcatgatgccctgatgcggaccgtggatgtggacaccgaccccgagctggctgcggaattcggcgaccgagtgccggtggtggtgatcgacggagaggaattcgcgtgctgggaagtggaccttcacgagctggaaacagagctcgaatcctaaggcattatactttcggttgattcgcagctgaggaggaattgcgtgagcgtattggtcgtggggatgtcccaccgctcggctccagtcgcgctgcttgagcggttgagtatggacgccgcggtgcaaaaccagaccggggcggcgttggtggatcaggcgtcgctgagcgaagcgatgatcatctcgacgtgcaaccgtttagagatctacaccgtgaccaacgcgttccacgccggggtggaggacgtgctggaggtgctggcggacgtctcaggtgtctccgaggcggagctgcgcacctatctctacgtgcgttacgccgacgcggccgcggagcacatgttctccgtcgccgccggcctcgactcgatggtggttggagagcagcagatcatcggccaagtgcgcacggcgtatctcgacgccgccgagcgcggcaccgtgggcccgacgctgcactcgctcgcccaaacagccctgcacaccggcaagcgcgtgcactccgagaccagcatcgacggcgagggcgtgtcgatggtctccttcgctttggacgaggccgcggcagccatggatgcgtccgggttcgagggcaaaacagcgctggtgctcggcgccggggcgatgagctcgctcgcggcgacgcagttgggcaagcgcggggtgagcaaactgatcattgccaaccgcacgcgctcgcgcgccgagcgcctcgccgagcacgcgcgcgaggcgggcgtgagcgccgaggttgtggacttcaacgcgcgcgccggagcgatttcgcgggcggacatcaccgtctctgcaactgcgtcggacgggttcaccatcaccgcggaggacctttcggggcccgccacgctgatcgacctgtcgctgccccgcgatatcgccgacgacgtcgtctcccgcgagggtgtgcgcctcatcaacattgagtacctgcacaaacgccgcggggatgcgtcgcgtgaggacgcgaccgcgctgcgactcgcccagagcattgtggctgaagaggtcgaggcgttctcctcggagcagcgcgtccgcgaggttgccccggccgtggcgcagctgcgccggaccgcgaacgagattcaggaactcgaactggagaagctgcgcgcgaagctacccgagatggcggacgacgacttcgaacaggtctcgcgcaccgtgcgccgcgttgtggacaagttgctccacacgccgacggtgaagatcaaggagctcgcggcgtcctcgaacaccgtcagcattgacaccgtgttcgaggagttgttcggcatcggcaggtcgagcatcgccgtcgacgcgcagaatctgccgcgcccagaggacatgaacccaaaggagcacgcatgaagcgcatcggtacccgaggatcgcacctcgcgaccacccagtccggacacgtcagggacgctctcggggagttaggccaccccgccgagctgcacattgtgaccacgcccggcgatgtgtcgacggccccagtcgagcgcatcggcgtgggtgtgttcacctccgcgctgcgcgacgcgctgttcgccggcgaggtggacattgccgtgcactcgttcaaggacctgccgacggcggacgagccgcgggcgcacctgatcgtgcccgcgcgagaagacaaccgggaggcactgattgcccgcgacgggctgactctcgaccaactgccgcaaggcgcgcgggtgggcacgtcagcgccgcggcgcgtctcgcagctgcgcagtttgcgcccggacctggagatccgcccgctgcggggcaacatcgagactcgcatggggtacgtcacctccggcgagctggacgcgatcgttttggcgtacgcggggctgtcccgcggcggctacgccgagcgggccacccaaatcttcgagccgcacgtgcttatgccggcgcctgcccagggcgcactggcggtggagtgccgcagtggcgacgacaaaacgcgcagcgcgatcgatgcgctgtccgaccgggttgcgacggtgcaggcgcgcgcagagcgccaggtgctggcgacgctggaggctggctgcaccgcaccggtcgcggcgtacgccacctacggcggggagaccggcggtgaggacgtgctcactttgagcgccggcgtgttcgctctcgacggctcgaaaaaaatcgtcgaaacactggcgggcccggcggattcggctgaggaactggggaagcgggttgccgcggcgctgttggagcgcggcgcggcggttgtgatgggcgacgcctaagacgcgtttttgtttcgagacgcgtccaccttaaggtggacctagcaaacacacccaagtctcggtgctatcgggtcccttaaacggggcctttttgccgagacgactacttgtgccttagaaaagttcacttatgacaaagatcatcttcgtcggtgcaggcccgggaaaccccgatctgctgaccatccgcgctcgcgaggtgttggaatccaatgctatcgcgctggtggatccgcaggtttctcagggggtccaaaacgtcatcgccgctgggttgccagtgccgaaatccaagctcgaggccgccgacgccgcgtacgagcagatggtcgctgaggccaaagaggccggcgcgcgccgcaaacccgcccgccccgaggacccgaccgcagcggaggtcgttgaggttgagtgtggggttgaagggatcgtcgacaagctaaaagctgccctcgcggacgctgaggagttggccgagcgcggcgaaggcggcgagggcgacgtgatccgcctggtgtgcggtaacccgctgacccgcgattcggtcatggcggaggtctccgcagcggcggctgccgggctcgaattccaggtggtgccgggcatgagcctgccgtcgacggtgccgagtttcgccggcatcgcgctgggctcgacctacaccgaaaccgacctggcaaacgagtcggtggactgggaccagctggccaccgcgccgcagcccctggtgttccaggccgcgcaggagcacctcgcggtcatggttgctgagctcacgcagcgcggattcacgggctcgactccggtctcggtcaccacgaacggcacgacgcggctgcagcgcaccttcgacgccacgcttgagaccctggcgaagttggatgccgacctgtctggctcgctggtggtcaccctcggcaccgtgccggatgagcgcgcgaaatactcctggtgggagaaccgcccgctctacggctggcgcgtgctcgtgccccgcgcgaaggaacaggcgggtcctatgaacacccgcctgagctcctacggcgcgatcccgcagtccgtgcccacgatctccatggagccgccccgcaaccccgcgcagatggaccgcgcgatcaagggcatcgttgagggccgctaccagtgggtcgtgttcacctcgaccaacgcggtggacgcggtgtgggacaagttcgaggaactcggcctcgacgcgcgctcgttcgctggagtgcacctcgccgcggtgggggagaagaccgccgacgccgtgcgcgcccgcggcatgtttccggaggtgctgccgcaccgcacgaagcagaacgccgccggcctggtggaagtcttccccgagtacgtcgaagacatcgatccagtctcccgcgtgctgttgccgcgagcggaccttggaacggacgtgctggtggacggcctggtggagaagggctgggaggttgacgacgtggtggcgtaccgcaccgtgcgcgccgccccgccggcgcctgaggtgcgcgacatgatcaagtccggcggcttcgacgcggtgtgcttcacgtccgcgtccacggtcaagaacctggtcggcatcgccggcaaaccgcacccgcgcacgatcatcgcctgcatcggtccgatggccgctgcggaggcgcgggagcagggcttgcgcgtcgacgtcgtccccgaggtggcagacgtgccttcgcttgtcgacgccctcgcggcccatgttgccgacctgcgcgccgccggccagctgccgccgccgcgcaagaagcgccgcgcgcgccgcaaggcgagcgaggacaccgccgctgctgccggccaggacgtcgcggataccgcgagctagcacgataatttgcccctcgtcctaagatggggcacatgtcgcaagatcgcaacgcccactccctgccgctgctgcgccgcccgcgccgcctgcggcagaacccgcaaatccgcactttgacggccgaaacgcggctgaccccggcggacttcatcctcccgctcttcgtggccgacggcatcgatgctccccgcgagatcacttcgatgccgggtgtgtaccagcacaccaccgacagcttgaaggcgatctgccacgaagcgctcgacgccggggtgacctgtgtcgacctgttcggggtcccggtggacgaggacaaggacgcagaaggctcggtggcctgggacgccgacggcgtgctcaaccgcaacctccgggagctgcgcgccgagtttggcgacgacctgctgatcatggctgacacctgcttggacgagttcacggaccacggtcactgcggcgtgctcaccaccgaccgctggggccgcgaagtggtggacaacgacgcaacggtcgatctctacaccaagatggcggtagcgcaggctgaggcgggcgcccacattgtcagcccgtcggggatgatggatggccaaattgaggcgatccgcactgcgctggacgaggccggcttcaccgacgtggcgattatggcgtactccgccaagtacgcgtcgaagttcttcggcccgttccgcgacgccgtgggatcgtcgctcaagggcgaccggcgcacttaccagcaggacccggccaatatccgcgagtccatcttggagacgcagctggatatcgacgaaggcgcagacttcgtcatggtcaagcccgcgatgccgtacctcgacgtgctggccgaggtggccgcgatgtcgccggttccggtcgccgcgtaccaggtctctggcgagtacgcgatgctggtagctgccgggcagaacggctggatcgacttcgaagagacgatgatggagtccctcatcggcatcaagcgcgcaggcgccgaccagattctgacctactacgccatcgaggcggccaagcgtctgggcggcggccgtggctaacatccccgcgcctccggggccttctgcgccagccgggccgccggtcaacccggagaccggatcgcacgtcgacccggctgctgtggaccgcaagaaaggcccgtcgaagaacccgaagcagccggaggctgtgcgattgatgctgttgagctgggcggtcatgatcgccggcgagctgctccaccagatcctcacggttgtcgccatcgttatcgacccgagcgagctcatcgccgccgcaaagcaggcggcgaagaccaagggcgaagaggttcccgaatcggtggtttcggccagcatgtggggttccattgctatcgccgcgttgatccagttagctatcatcgcgctgtttgtaaccgcactggttgccctgcagaagcagaagaagtgggctccgaccgctcgccgtctgctgcaagtgttctcagttttcttcgctgtgcgcgtgctcgccgtgtttgtggcgaagcccgccgcctccgccgtgccgctggcgttctacgcgttcgacggcgtcgtgcagatcattatcggcgtggcgggtgcgctcggcctgttttacgcttcccagaaggaagcgactgactgggcggaagctggtgcaccgcccaccaaggggcgcggcggaagcgcgggccccggtgataaaggagcgtaagaacacatggccgggatgtttccttcgatggtcgcagaccccgacgaccgcaaccgccgctattcggggccggtgggtgataagtggcccgcaccgctgcgcgcggggtactggtgcttcctgctcgcagctgtgctgatgctggtgtctagcttcctcatgctgcgcgccggcgcgcctgcggagctagagcaggacgtcgcgatgtcgttccgccgcaacatgcgcatcgtcgctgccggaaacatcatcctcgcgctgtgcctgaccgcgtgcgcggcgttcttcgagcgcgggtccaagcgcgcccgccgctccgcgtcgctgtttatcttcctcaccatcttcctcaacttcgccggtttcttcgtcggtgtcgctggctgggtggtgttcgccattgtggcgctcctcgccgtgggcgcgttttttatcttccgcccgtcagcaaacgcgttcgtggacgagcgcagcggcgatctgtggcgcaatgtcagctaacgaagcttacgaagacggtggtgcgttgatctctgaggaactgtccgagtccattgagcaggcccgacgcgcagccaagttggcgggcatcgacccggatgccgtgcacggtgtctccgacgacgaggacgcgccgcgccaggcgaacgcgtcgtacgcgttcgagctcgacgggctgaaagacgggccgcagctcggtgacatcgaggaagcgcttgaagctatccccggtgtggatgcccagctggtgtactccacttccatggcttgggtgaccgcgccgacgacgatcgacccgttgaagctcgcggaggtgatcgagtccttcgacgtcacggccgagatgacggattccacgctgcgtcgccgggcgctcatgcacgagccggtcgaccgccgctcgccgcgcttgagcacgcgtgggatgtcggggcagatccggaagcgccgcaaggatgcgcaggcgacgctcacagcagcgcgcgaggctgggtttgtgcgccgcacgcgcgggaagactgactccggcgacgtgctctttaccgcccgcgacttggtcacccctgcccgtctgatcaccgccatcgtgctggccatccccgtggttgtcctcagctacatcccggagatccagttccgcggctggcagtgggtctgcttcgcgctggccaccccggttgccctgtggtgcgccctgccgttccaccgcgcgatggcagggggcgtgcgccgcgggctctcggctctcgacggcgcgagctccgtcgcggtgctggcagcctacatctggtccgccgcggcgctggtgttcacttccgccggtgagatcggctgggtctcctcaggtgggtggctgcccaccaggcgcggtaacgaggttgagatcttcctcgacgttgcctgtggggtgaccgcgctgctgctcatcggccgctactactccaaacgcattggccgctcgctggtggaccagatgcgccgcttcgccccggatcccgagaccaaatatgaagtggcccgccgcggcagcggtcagagccagtggctcacgctctccgaaatcaaccgcggcgacgacgtggtggttggaagcgggtcgatcgtcccggtcgacggggaggtcgtcggcggttctgcgagcttgaggcatgtgcttaccaacgtcgacctcaaagactccgtcggcgtgggcgacgatgtggcggcaggcgccgtggtccaacgcggctccgtgaagatccgcgcgcagcgcaccgggcacgccacccgctggtcctcggtgagccgctgggtggaggaagcgtcgcgccgggaaaacgccgcgacgatggtctccacccgctccgccagtctcctcatcccggcagcctacgtgctggcagtggtggatttcggcatgtggtggctgatcactggggacttgaacgccgccttttccaccgcgctcgccattctcgcggtcgtggcgccggtggcgttggcgatttccccggcgctcgccacgcgccacggcatcgaggcggcggcgcgcaacgccgtgctcgtgcgcgacggcatcaccctgcgccggctggctgacgtagacacggtggtcttcaaccgcgtcggcacattggttgaaccggagatgaacgtcgaaacggtcactgccgcgcgcggggaagactccgagatggtcctgcttatcgccggggcgctgctggtggagtcgaaccacccggcagcccgcgccatcgtcgccgccgcccgcgaggcgaaaggccgcggcgcaccgtggcgcgtcgatctggaagaagtcgagctaggtgccgacggcaccacgaaggggcgcgtcacgctgcgcccggttgttgacggccgcgtggccgacgacgacgcctccacccacctcgacgcactgctgtggcgcccgctcaacatgtcccgcttgtccggccggctcgcactcgcggcgacgtccggcggcgccccgatcgtggtgcgctggaagggcaaagaccgcggagtgatcacgctccacgacccggagaagcaggacgctgcggaggcagtggaccgtctcgaagcaatgggcaccaccaccgtcatgttgacgcgcgacacctataccgtgggccgccgtttcgccaacatgctcggtatcacgtccgtgctcgccggcatcacggcccaggacaaggcggctgcggtgcgccagctccacacgcgtggcgcgaacgtggccatggtcggctccaccagcgtgcttgacgtgatcgaggtcggcgacgtgggcatcctctacgccgaggacgagttcttcgagggccactttaaggcccgggaggaaggcgtggatgccgtcatcatgcgcgacgacgtgatggcggtgccgcagctgatcgagcacggccgccgcgtgtcccgcattatcgactccaacatggcgttcgccctgatctacaacgccgcggcggtgggcttagccatgttcggtgtgctgcccccgatgggtgcgacgctgttcatgctcgggtcgtcgctgatcatcgagcaacgctcgctacgcgctgggcgcttccccgtctaggcttacacagcatgaccagacgcgacctcgaccacgccccgcttatcgacgccgcctgtggccgcaccccaacccgcactcctgtgtggttcatgcgccaagccggccgctcgctcccggagtaccggaaggtccgcgagggcatccccatgctggactcgtgcttcatgccggagctgctcgccgagatcacgctgcagccggtgcgccgccacgacatggacgcggcgatcttgttctccgatatcgtggtgccgctgaaagctgcgggcgtcgacgtcgagatcgtgccgggcaagggcccggtgatgggcaagccgatacggacgaaagaggacgtcgcggccctgccggagctcgaccaccacgttgacgaggtcgccgagggtatccgcatcatcctcgaggagctgaacagcacccaggcgctcatcggttttgtcggtgcgccgttcaccctcgccagctacctggttgagggcgggccgagcaagaaccacgagaagaccaaagccatgatgcacgccgacccggagacgtggcacgcgctcatgcgcaagctggtgcccaccatcacggcgttcctctgcacccaggtggaagcagggatcgacgcgatgcagctgttcgactcgtgggcaggctttttgacggagcgggattaccgcacccacgtccttccgtactccgtggagattttggagtccgtcgcgggagagattccgcgcatccacttcggggtggctaccggcgagctgctcggcgcgatgagcgaggccggcagcgaggtcatgggtgtggactggcgggtcccgctcgacaccgctgcgcgccgcttcgcctcgccgagggtgctgcagggcaacttggaccccgccatcttgttcgcaggcgacgaggtaatcaagagcgaagtgcgccgcatcaaggccgaggccgccgccgcgatcgaggaaggcaccgccaccggccacatcttcaaccttggacacggcgtgctgcccaccactgacccggacgccatcacgcacgcggtgcgcgtgatccacgaggcgtaacaagaggagcaacgaagaacatgaaggtagcaatcatcggcgccggcctagccgggctcacctgcgcgtacgagctgggcaccgccgagggcggcggcatcgaggtggacgtgtacgaagccaccgaccgcatcggcggcaaactcttcaccgtccccttcgaggccggccccaccgacatgggcgccgaggcgttcatggcgcgccggaaagacgccgtggagctcttccaccagttgggactagccgatgcgctggtcgagccctcggggctggggtcgctggtgtacgtggacggccgcactgagccgctgccgcgcgcaggcatcatgggtatcccgtccacgtcggagccggtagcgcacctcgtgtccgccgaaaccgccgcccgcatcgacgccgagggcagcaccgacggattcgcgtgggagatcggcggggatcagaacgtgggcaagctggtgcgcgagcgctacggcgacgaggtggtggacaacgtggtcacctccctgctcggcggagtctactcgtgcgcggcggacgacttgggcgttcgcgccaccatcccgcagctggcggcggagttcgaccgccttgccgccgcgagcgacaacggcaccgtccacctgtccgaggcggtgcgcaacctcgaggacgcgcgcaaggagctgcccaccggccaaggcgcggtgttcaacgcgttccgcgacggctaccaggagctctacgaaacgctggcggaggaatctggcgccgacatctatatcgacgcgttcatctccgccatcacccgcgagggcgaggggttccgcttgaaaggcggcgaggacacggtctacgaccacgtggtgttggccacccccgccccaacagcggcgctgctgctcaagcaggtcgcaccggaggtggcggcgacgctgaagacggtgcagctcgcgaactcggtggtggtgggcatgcggtttgccactgatgagggcctgccggagaactctggtgtgctggtggccgcaggcgcggacgacgtcggcgctaaggcgttcaccctttcgtcgcgcaagtggccgcacttggcagagcgcggcggtgcgctggtgcgcgccagcttcggccgcttcggcgacgacgtcccgctgcgcgccgacgaggacgatcttgtggattgggcgctggacgacctgcagacgatcaccgggttcgacggccgcgctgccggcttggaagagatctacgtccagcgctggttcggcgggctgccgcgcttcgacgagcagcacctcgccaccgtcgccaccgcccgcgagcagctcgccagcgtcgtcggcatctccgccaccggcgcgtgggccggaggagtgggcgtgcctgccgtgatcgcagacgcccgcgccgctgcgcaggaaatcctgaagcagaggtgacacgaatggaaccgcaggaaaaggagtggtgggaggaagaaggcctgccgtggaacggcaaacccaccaaggctgactactggtgcctcggctggttcgggttcgtggggctctttggcctcgccatgatcccgctccgggcgtggctgctgggtctcgatccgccgatcatgctcgcgctcacgggttcacgccttggtgcggcgtccacaggggcgcttgcggcggttgggcaagcgccccactggctggtctacctgctcatcggatcgatcgtcgcgatcaaattcgactggatctactggtgggcgggcaagctgtggggccgcggcatcttggaggtccaaggcgcgaactccaagcgcgcggcaaagaatattgagcgcgtcgagcactgggcggtcaagctcggatggctgggcatcttcctggcgtacgtgccgatcccgctgcccatcgcctttgtggtgttcgtgctgatgggcatgaccgggatgccgctgtggaagttcatggtgctggacttcgtgtccaaaaccatctggtcgttcctctatttcggccttggctggtggatcggcgaacccgtggtcaccgtcctcgaccagtacgccaaggtagcgaactggatcgcgatcggcctgatcgtggtggtcttcttcgggatcttccgcaagcagtcgaagtcagccaaccgccccgctgaggtggtcggcaacgagatcgaggctggccactagcaagcaagggctagttgtcgcggtagacaaccaccgacgacagatcctcgtcgccgtggcctgcgcgctgctgcgcctcaagggagcgcagcgccgcagcgacggcgggcagttcgtggtcggcggaagcaatcatcaaccgcgcgtctttggcgatggcgtcgacggagaagtcgcccgggtccgtggagcgctcgccgcgcacgaacggcgccttcatgttgacgatgaactcgagccccgttgacccaagcatcgaaatgacctcgtcctcggtcagcccctgcgactcgcccatgtcgagggcttcgcggaagccttcgatgctcacggcaagcgccaggttggccaagagcttgcccaccgcggccttggaggcgctgtcgacttcgcgcaggcgatccgggttggcggctgcccagggggcgacggtggaggcgacaagggagcgtcgtgaagcatctgctcctcccacgtagaccccgagcttgccctcgcgcgcaggcggcagcgaaccgacaaccggggtgtggatgaagccgggcaccgcggcggcgaactcggcggcgtccgtgggggagatggtggtggcgtccgcccaggtcaccccgtcggggatgagcgcgggttcgatgacaacctcgcgcacctccgccgggccgaacagggaggtgatgaccagctcggcgccgtccaccgcctcggcaggggagtctgcagcgcgcgcaccacgcgcaaccagcggctcggttttggagtgagtgcggttccacaccgtgagatcgtgatcgtcgacaagcttgagcgccagctcggtgcccatgcggccgaggcctaaaaatgcaatgttcatatggcctagaataggcaaccatgactgcccaaaaaccgacttcagcaaacacgacacgctccgccgaactgttcgctcgcgcgcagcagctcactcccggcggcgtgaactcgccggtgcgcgcgttcgggtccgtcggcgggcagacgcggtttatcgacagcgcgcacggttccacgctgattgacgcggacggcaacgcgtacgtcgacctggtgtgctcctggggtccgatgattcacggcaacgcgcacccggacatcatcgccgcggtggaaaacgcgctgagcaagggcttgagcttcggcgcgccgacggaggccgaggtggagatcgccgagcacctggtcaaccgcaccagcgtggaagaggtccgcatggtcaactccggcacggaggccacgatgagcgcggtgcgcctcgcccgcggcttcaccggacggccgaaggtgatcaagttcgacggctgctaccacggtcacgtggacgcgctgctcgcgtctgcgggctccggcttggcgacgttttcgttgcccgattcccccggcgtcaccggtgcccaagccgccgacaccatcgtggtgccctacaacgatatcgacgccgtccggaaggctttcgaggacaaccccgaccagatcgcctgcgtgatcgcggaggccgcggcgggcaacatgggcaccgttgcgccgaaggataacttcaaccagaagctcaaagacgtctgccacgagcacggcgcgctgctcatcttggacgaggtcatgactggcttccgcacctcgtataagggctggtacggcgtcgacggcgtggcgggcgacctgaccacctttggcaaggtgatctccggcgggctcccggcagcagcattcggcgggcgccgtgacattatggagcgcctcgcgccgaacgggccggtctaccaagcgggcacgctctccggtaacccggtcgccatggcagcggggctggccagccttcgcttggcctccgaggacatctaccccgtgctcaaccgcaacgcggacaccttggctggtctgatctcgactgcgctgacgcgcgagggggttgcgcacaacatccagcgcgccgcgacgatgctgtcggtccgcttcgctgaagggcagggccacaatttcgacgacatgaaggcggcgcagacgtggcgctacccggcgttcttccacgcgttgctcgacgcgggcgtctacgccccgccgagcccgtttgagacctggttcgtctccacggcgctgacggacgaggatttcggccgcatcgaagaggcccttgtgccggcggcgaaggcggcagcggccgcggagccgcgctgatgacgcaagacgcgccgcgcaccaccgtgcacctggtccgccacggggaagtgttcaacccgaagcgggtgctctacgggcgcatgcccgactaccacttaagttcccggggccagtcaatggcggcggccaccgcccgcttcttcgaaggctgcgacgtgacctacctcgcggccagcccgctcgagcgggcccaggagacggcgcagccgatcgcggaacttaccggcctggccattgacacaatcccggacgtcatcgaggcggccaacaccttcgaggggctccgcaccaaaggtgtgcgctcccagctgtggaacccgattcgctggcgccacatgaccaacccgctcaagcccagctggggcgagccgtacacggagatcctcgcccggatggagaccgccatcgaggccgcgcgggtgcacgccgagggccacgaggcagtgctggtgagccaccagctgccgattgtcatggtgcagcgccacgtgcagggcaaacctctctaccacgcctcgcgcgagtgcgacctggccagcgtgacctcacttgtgttcgacgacgacgttgttattgactggtcgtacaacacccctgccgcccacatttagaaagccacgccatgcactccaggtttgccgcaccgtttttaagcgccgccctctgcctgaccgtcttcggcgtggcgggctgcgcgagcgataccaccgacggtggcggcacgttctcgttccactcgccgggtgggcaggtggagatcttctacgacgaggctgagcgcaaacccctggcagatttcggcggggaatcgctcaccgacccgggccaggagatccgcctgtcggatttcgacggccagatcgtggtggtcaacgcgtggggccagtggtgcgcgccgtgccgggcggaggtggacgacctgcaggaggtccacgagaccctccaggcgcacaaccaaggcacggtgctcggcatcaacgtccgcgacttcaaccccgagatctcccgcgacttcgtcgccgacaacggggtgacctacccgtcgatctacgacccgccgttcaagaccgccgcgttcctcggcggcgtgcccagctccgtcatcccaaccacggtgatcctggacaagcagcaccgcccggcggcggtgttcctgcgcgagataagcgccgacgacatcctcgaggtcaccgccaagctggaaacggaatagcgtacgtgggcgatctcttttccaaccttgccgccgagggcccgctgctgctcggcatgctggcggcgatgctcgccgggctggtgtcgtttgcctccccgtgtgtcatcccgctggtgcccggctacctgtcgtacttaaccggcgtcgtcggcggcgagatggagttcgacgaccacggcccgcgcgtgacctccaagcaggcccgcgtggcgggggcggccctgctgttcatcctcgggtttaccgtagtcttcctcctagccacggtctcggtctttggtgcgatctcgctgatccagctcaacgccgacaccctgatgcgcatcggcggggtgatcaccatcgtgatgggcgtggtgttcatgggcgcggtgccgctactccagcgcgacacccgcatgcagccgaagcgctgggccaccatcctcggcgcgccgctgctcggcggggtgttcgccctcggttggacgccctgcctcgggcccacgctcgccgcgatcatctccgtgtccgtcggcaccgccggtgtcaccgcggcgcgcggtgtggtgctggtgatcatgtactgcctggggctcggtctgccgtttctcctgctcgccctcggctcggctcgcgcggtgcgaagcgtcgatttcctgcgccgccactcgcgccagatccaggtgatcggcggcgtggccatgatcgtggtcggtgtgctgctgatcaccggcgcgtggaatcatttcatcggctgggcgcggcagcttacggttggtttcggaacgacggtgatttgaggtgacggcaatgcgcacggtgtggctctacctgcggaaggcgtggcactggctgaccagcatgagcaccgcgctgattctgttgttcctgctcgcgctcgccgcgatccccggcgcgctattgccgcagcgccaggtgagcacatcgcttgtcgacgactacctcaacgccaaccccaccctcggtccgatttacgaccgacttcagttcttcgacgtgttctcctcgacctggttcgtggcgattgtcacgctgttgatggtctccctcgtcggctgcatcatcccccgctccgtcgaccactggcgcgcctaccgcgccacgcccacgcgcgccccgaagtacttggcgcgcatgccgatgtacaaaagcgccaccctcgacgagtcggtggaggagatcgccgaccgctccaaaggcgcgctgaagcgctggcacgtcgcggactacgcgccgggtgaagaccgcgcgggcgcgttctccatctcagccgagcgcggctacgcccgcgagctgatgaacctgatcttccacatcggcttggtcggcatgatcgtcacgttcgccgccggccgtatggtcttctacgaaggccaggtcatcgtggtcacggattccgaatccgagtacgcggtgccggtggagcgctcccgcgagttctgcaacaccagccccgccaacttcgacgtcttccgcgccgggccgctgttcgacggcacggggcttacccccttctgcatcgaatcggagaacttccgcgcggcgtacctgaacaacggccaagccaacgggttctggtccgacatcacctacacggatgacctggctaccccgaaggatcagtggcagccctacacccttcaggtgaacaacccgctgcgcatcaacggcgaccgtgtctacctccagggccacgggttcgccccgcaggtgacaatcacctggccgaacggcgaatcccgcacccagatggtgcagtttaggcccaccgacgtgcagaccttcctctcctccggcgtgatgcgctttgacccgccggcgggcatgtacccggatttgaacgaccgccgccagcaccaaatcgcgatcgagggcgtcttcgcccccaccgcgtcctgggtcgggccgaacgccgacatgctgcagtccgctttccccgcgatggaggacccggcgatggtggttgaggtgtactccggcgacgccgggctcgacaccggtcgcccgcagaacattttcgtgctggatcaggcattgcttgccgacggccgcctgcaaaaagtcgaccgcctccaactcgagccgggccaggaggccttggtggacgtcggcgaccccgccggaccggtgagtgtgcgcttcgacggcgccgccgagtttgccaactaccaaatttcccgcgacccgttccagccctggatcctcgtcaccacggtgaccatgctgctcgcgctcgccgcgtcgctgacgattcgccgccgccgcatttgggtcaggctttcgcttgccgacgccacgaacccctcctccggcaccctcgtcgaaatcgcggggctatcgcgcacggaccgcgcgggttggggtagcgagttcgacgacatcgccgcgcatgtgctcgggcgcgccgattcaaagctcgtcggcgacttggatgagctggacgaggacgaacccgacctcttggaacgcgcttgacgggtgcggtagtttaagcacatgctcgtggattcttcaatggccgccctgtcggacctgacgttccgcacggcgtttgtcatctacatcgctgcgctcgtgatgtcgtgcatctactacggccggctgatcagcgtgatcgacctgcgccgtgagcgcgccgcggtcacaaccgccgtcgcggtgacggccggcggcggcaaccacgaggtggtggtcgaggagccggtatcccgcggcgagaactccatcccgccgggcgagtacgaccagcgcgtggccaacgcgcgcaagtgggcgaacatgacccaggccctggtctggttcggcgtcaccctgcacatcgtcgcctttgtcacccgcggtattgccacgcagcggttcccgctgggcaacctgtacgagtacatcctgttcatgaccgcggtgatcatggtcgtcgccgccaccgtgatccagcgcaagagctggcactccctgtggccgtggctgctgttccccatggtcgtgaccatgttcttgaactccaccgtgttccacctgagggcggccccggtggtgccggcgctgcagtcgtactggctgccggtgcacgtctccacggtgtccgttggcgcgtcgatcggcatcgtctccggcgtcttcgctgcgctgtacctgctgcgtatgtggcagcccaagggtcaggagcagggcttctttggcgcgatcgccaagccgctgccaagcgcgaagacgctcgaccgcatcacctacaagtccgcgattgttacgctgccgctgttcggcatcggcatcgttttcggtgcgatctgggcggaggtcgcctggggccgcccgtggaactgggacgcgaaggaaaccgtgtccatgattacgtgggtgctctacgccgcctacctccacgcccgcgccaccgccggctggaagaactcgaaggccgcgtggattaatgtcttcgccatgctgatgacggtgttcaacatgacctacgtcaacttcgtttccgcgtccctgcactcctacgcgggcttgaactaactcccggtgacagcaatgaaggtccttatcaccggcggggccggctacatcggctcgaccatcactagctgctgcgcagacaacgggatcaccccggtgattcttgatgattactccacggggttgcgcgttttcgcccgccgcttcgaccactacgaaggcgacatcgcggacgccgcgctggtggatcgcatcttcgccgaccacccggacatcgacgccgtggtgcactgcgcggcgaagatcatcgtcccggaaagcgtggccaacccgcttgcgtactacagcaacaacgtggccaagtctatcgagctgctgcgcacacttgagcgccacggcatcacccggttcatcctgagctccaccgcgtcgatgtacgagcccggtcccgactacatggtggacgagcaaagctcgattaacccgttgagcccctacgcggcgtccaaacgcatggtggagcgggtgctcgaggacacccagtcgatccagtcgctgagcctgcgctacttcaacccgatcggcgcggatccttccatgcgcaccgggctgcagaacccgcatccaacccacgcgctgggcaagatgattgaggcgcaccagcgccgcgcgccgttcaccgtcacgggcgtggactggccgacccgcgacggctctggcttgcgcgactacgtccatgtctgggacctcgcccgcgcccacgtccgcgcgctgcagctggacccgtccgcgctgggtgctcacaccacgatcaacctcggcaccggccagggcacgaccgtcttcgagctcgcgaaagcgttcggcgaagcaacgggcgaaccgctcgaggtgacaacagcgccgccgcgcgacggtgacgtcgtgggctgcgcgacgcgcaccgcgcttgccgaggagatcctcggctggcgcgcagaactcaccgttgccgacggagttcgggactcgctcgcgtgggctgcgaagctcccggacgtgttagacaaggagggcacaatccgtgactaggcatctaccccggcacaaagagggcaagcccgccagcgataacgagacgctgatcaagctgggggaacagatcgccacgacgcgccgcgacagcggccgcctccagcaagaggtcgctgacgctgccggggtctcgcgctccacgctgcacaccatcgaacacgggggtgccggcgtgcgctgggagaaagtggtcgcggtggcggacgcgttggggcttgaggtggggtttaacggggcgtcgtcaagctaaagcccctcttcgcggcgcctgcgccgctcttcctcctcgcgccgcttgcgctcttcttcctcttttgcccggcgctctttgaagcggttcttttcgatgttccagaggaactcctcgtcatcgtccggacccttgatttccggccgcggttgctgcgcggcgccgccgtagcgctcgtttgagccggggccgaaggcgcgccacatgaggtacgcggcggcaaggaccaagatgacaagcagaacacgtcccatgactaccaactttacccggcgggtcgttagggttaggaaccgtgactgacaacgcaaccgccgcacaaccgccagccgtcgacccgcaggcccgctcgcgcgcgaacaaggccgctgccaagtacgggctgttgcggctgttgctgtttatcgtgctgacggtggttatccagctgctcgcggtgctgatcggtgcgccggtgcccctggtgatgtcggcgctgctcgcgctgattgtggcgttcccgctgtccatgttcatcttcaccaaacagcgcgttgaggccacccaggccatcgcgcagtggaaagggcagcgcgccgcgcgcaaggagtggatcgcctcggagctcgccgagcgctagcgttctacccgcgttctacccgccgaagatgaacgcgatgagcagcatcgcgggcagcgagaggaacgtggtgaggaagaccgtgtcgcgcgccaccgtctgcccgacctggtaggtggcggtgtagttgtacacgttctgcgcggtcggcagcgcggcgagaatcaccgcggcgtagagcaggtccccgctcaaacccatcgccgcgcccacacctgctgcgacggcgggcatgccgacgagcttcagcgcggtcgcggtcatcgtgggtgcgcgctcgtcttggaggacgcgatcgcccttgagagaggcgccgaaactcatcagaatcagcgggatagaggccccgccgaggatttccagcggcgccatgaccggctcgggcacggtccaccccgcatacgagatgacaaacccgatcaccgccgcaaccaccatcggcgcggtgagccccgcaacgatcgccttgcgcgtgtcggccctgccggatccgccgtagttcagcccggtgatgatgatcggggtgaggatcgccacctgcagcaccagcgccggcacaacatacgtcggatcgccgatgacgtaggtggcaatcggcagcccgatgttgacagagttgtagtagcttgccgacgccgcgcccgccatcgtctccgccacactccgcttaaacagcgccgcactgatcacccagtagagcaccatggtgcttaccgacgccaccgcaatcaccaacaccaccggcgacaaaaacgcgctggtatccgacgtggcaacggaagagaagattaacgacggggtggccacataaaaagcgatctgattcagcatcagccggttgttgcttcggatgatgcctttctgcgccaaaaagaaaccggccccgatcaccgcaaagatgatggaaaagccggttagtacgtcgagcattttttaaagcttaaaacatcggcgcgaccgattgctcaactgcatcgtcgccagggaactcgtcgccagggaactggtcgtcgatgtacatcgaccagccaaagtcagattcaccgacgtacggcactggctggccccagaaggtggacccgaaccaggacagggcgagagcggtcatgaccgcccaaatcagcattgcccacccgttcataccgagcactgggatgaggtccgtgccggtggcgccgcgacgaaccgtgaggatggcggcgatggcgaacgggagtgccgcgaacgcgaggagcgccggggtgaacgtgatggcgagcaggatcgtggcagcaaacggcaccagcgtgagcgcggtgaatagcgcgcgtgcgctttggtcgccgatccgcacggccagggtgtgcttgcccgcggcctcatcagtctcgatgtcgcggatgttgttcgccaggttcaccgccgcggagatgcaaccaatggcgatcgcgcacccgaacccttggccggagacgaacccggactgaacgaactcggttcccatcacggcgacgaggccgaagaagacgaacaccgccagctcgccgaaccccgcgtaaccgtacgggcgtggcccgccggtgtagaaccacgcggcggcgatgcacagcgcgccgacaagaatcagccaccacgacgacgtcgcagcgaggataaagccgagcaccccagccacgccaaacgcgatgaacgcggcgagcttgacatcctcggggcgcgcgataccggatgctgtcagccgcgtcgggccggtgcgcttgttgtcggtgccgcgcaccccgtcggagtagtcgttggcgtagttcacgccgatgatgagcgcgagggcgacacccagcgcgagtagcgccttacccaggtgcgcgctgccccagtaggcggcggcgccagtgccggcgatgacaggggcgatggcgtttggccaggtgtgcgggcgggcggcttcccaccacgcgcgccacgcaatatcggcgcgctcagatttcggggtgtcagcgttcgggtgcatggcacccatcatgcctgcattgcggttggacggctagcgatcgcgggtggccgtttcctcaggcgtgccactaatgcgtgctgtctgtcgtgtctttatagcgtgcgaacaaaggggcggcgttgtttgtaacggtagcgcgtcggttgatggtactggcgagcggcgacttgggttgcagtgtgggtggtaagggtcgtggcgtacttcggattcagtgtctgatttttcgagtggagcgtctcggtcctcacaccccgtgattgtcacatgaattacacgcatgtgctttgcggctttgggtcactggaggtgaatgtctggtgaacattgagccggtgtctgcaccgaccgcggatttgccggggggcggatcttggatggcggatataccgctttttgaccgcatatccgccatccttcatccgcccccctggatgaggtgcggtccactttggtcgccgtgaagggctagagagcctgaagatacccctcttggaatggcgcattcatcgaaccggatgtcaatagaaaggctttcggatccgtagcttcgcttatctgtgctgccattggttcgagtgccgctaccagctgggctagttgaagatgcgcgatgcgccgaccacgggcctggggatgccggggaaccccgatccagtgcaaccccgcagatctgcacgcggctcgttcatgcttccggtccaacccctgaatctggagcagatcagctgtgataactgccttggcgtcgagcgatgcagcgatgctgaatagctcgacatcgctgatcccagttgggtagtcgcggcccggtttcaggaaagtgtgtcgtgatttggccagccgttgtagaggatcaattgtgttccccggaaagttctcatcaatgaggaatctcacgcagaccactctttaaccgctgactcgaagtcgagcgcgtggttgatggcgtcttgatctagcgaggggtacgcatccttaagttcgtccacatccatagcctcgtcaccactgcaaagatctatgactaagtcgaacggaacccgagttcctgcaagcacaggagtcccatgcattttctggggatcaatttcaattccctcgtgcggctgcagaaggggaggcacaatcctgttcttccagttcgggaactctccgtagatatcttcgaaggtgtaaagctcccactggcccgggttggaaaccaaatccagccagccctcgtctgtccacagtttcacggactcaccgtcggtagcgaatctgtacgtggagagatgctcgttgaaatcctggtcgtgcaaggtggccagagcggcgcggatcctctgaagcgacactttcgaacgcaatctggcgatggtccgtagagccacgacatcgcgaaacgaatatcgtcttgggcgggaagagatttcgggtcgcaacacgccgctcttcgcccatccgtctaattgggaacgggtggcaccactgaggaatgacgcgagtttggagtcataggacactgtggacctccttcttcgcagcttcgggcatcagggttttggtgaagtttagccagaaaacgatgctattggctggtcgaacctgcacatttccgtggacaattggaccgaaacgcattatcgataggaaagtgattacagctgggcttagatgaaccatgaaacccgcggtcatatcactgatcctctggttaacatcgctgtatgcagctgcctaaggggaggaccatcgatgtgcgcgatctttcgtcactcgcgcccgcatttaagaagggtgattcgaagtgtggtgtctatcgccttcacttcgaaaacggagaggcgtacccgggtaagtccaagaatgtcgtgagtagattcgcgagccaccggcggcgctggccggacatcgtcgccgttgacttcttcccgttaccggaagaccaaatcaccgcagcggagcagttcctaatcaccgagactgaagctcagtattcagtgcgaaacgtcatgctaaccaatcgaccacggggaaatgacaccgcggagatcgtgactctacaaggttcaaccgtcgcattgccgtgggagcgtgagcgagccaaaggcgccactcagtcctacgcggacgaggtatacgctaagctcgctcagcttcttaggcatcccgtattcccagagatccgggcgcttcttgggtggtacatcgccaacaccatgcctgacccggcagcgaccgccggccagttgtggacggtgacatgcatgccgtccacaaaccgcactccaagggagcaccgcctgctcactctgtcgtgcggaaacctggagacgttgttcattgttgcaagcaagtcggtggattacgcaaacgacccgaacgcattcgtagcggtacggatcaatacctcgcccctggatgacccgaagcggtatgaaagtcaagatggtttttggagggtctacggcaacgtctcataccgcggggagcgggtgtccagcttcgagttcagcctcggcgtgatactcgccattatcgatggccacatcactttcccaaatctcgatcggatgcttgaggaggcatacacgctcaacacccgcctcatgcgccggggctccacgatgtactcgcgcttccacaatgcgaaacttgcggacctactcctagctgaagcggtgacttgggaggagtagccgctcgaaactcctcgaaaagggtgaagatgaacgaacaacagttggaccaactgcggaatttttacgacagcacggatgtctctgacctcatggcggaagcagagcgtgtggacttgggtgatctgacagattctgaagccatggtttcctatacggtcagcatgcctcgaggggtgcttgacgcggcacgtgaaatcgccgctgcccgaggagtttccactgccgacgtcctgcgccgtttaattgacgaaggcgtcactcggcatactactggcgaagcctctgttcccatcagcaagctgatgaggcttatcgacgaggcgcggggagcctagcccgcccgtctgagcggcgcgggtgcaaagggcgggtctcacccgacgggtcggatcagaacggatttggttcactcgaggtgaatgtgtgttgaacagttggagagtccctttccgtcgaaggataagcactcaggatgcatcgctacgacgcaagtgggatcgacgggatatctacgttggttacatcggaaaacatctactgagccgtctgaccgattagccgcgtagaagaaccgtcccacatgtttggcttagcctgtttccatgagcctcggtgatcgtgaatcagccccatcccacgtagaaaaccaactagcgtccatctccatcggcaggcgcgtgcgtggtctcgtacccaaccaggtggtggagataaccgcagtggcaccaatgggcccgtccatggtgcaggtcgcgttccggggccaagacggaatcattcgggaacaggtgctcgagaaggacatcgatatcgagatcgtgatggaagacgagcccgcgtacaccttcgacggcaatcccgatacgttcaaacttgcgtcagaggcgatgcgcattaagtacgctgccctctacgacccactggctgcggtgaattcatctgatgtggatccgctgccgcaccagatccgcgcggtatacgaagagctgctcccgcgcgttccgcttcgcttcttgcttgccgacgacccaggggcgggcaagacgatcatggccggcctatacatcaaagaactgacgttgcgttctgcatgtgaccgggcgatcatcgtcgcgccgggtggcttggtcgaacagtggcgggaggagctggaggagaagttcggcctgcactttgagattttccaccgcgccatgatcgaggccagcgcgggcggcaacgcatttgcggaccatccatatctgatcgtcaggatggaccaggtcgcaagaaacgaagatctattcaacgacctgggtgccgtaacctgggatgtcgcggttgtggacgaggcgcaccgaatgtccgcgcatcacaggtcatgggcgggggaagtggataaaacagccaggtttgagctgggcaggttgctatctcagacggcccaacatttcctcctgatgacagcaacaccgcacgcaggcaaggatgaagattttcagctattcatgtcgctgcttgatccggacaggttcgagggcgagtaccgcccgggtgcgcaccgcacggacaccgacggactcatgcgcaggatggtgaaggaggacctgctcacgtttgaaggcaagccgctgttcccagagcggcgcgcctacaccgtgacgtacgacctgagcccagcggagcggaacttgtatgagcaagtgaccacgtacgtgcgtgaagagatgggtcgagcggaaaggatgttggataagaagcgcggcaacacaattggctttgctctgacagtcctgcagcgccgcttagcatccagccccgaagctatcctccgatcgctggaacgccgccgggcacgtctacagaaccggctcgaggagatcgaaaatctcagcgttgcggagcggaaggcgctgcgaatgatcgaggcggtttcaactgtaggcgccgataaacaatcgaagtgggatgaccctgatgagctcagcatcggtgaattcgaggagctcgaacgagagatcgacgacgtcgtagacctcgctaccgcggcgcaaacggtgccggagctacaggcggagattgccacgctggacgaactggtgcgggtggctatgaacgttcgcagccgagaagaggacacgaaatgggtacaactgcgcacgatcctcgataaggaggtgctgggcaaatctaccgacgacatagcacgcaagatcatcatattcacggagcaccgggatacgttgaactacctggaacgacagattgccacccagctgggcagagacgacgcggtaataaccatccatggtggcacggggcgtgaggagcgtaagcgagcgcaggaaagcttcacgaacgatcccagcgccatggtgctcctggccaccgacgccgcgggtgaaggcctcaacctgcagcgcgctcacctcatggtgaattacgacttgccgtggaatccaaaccgcattgagcagcgtttcggccgcatccaccgaattggtcagcgcgaggtgtgccatctgtggaacctcgtagcggctgacactcgcgaaggcgacgtgtttaccaggctgctcaccaagattgatgcaatgtcgaccgcctacaacggcaaccttttcaacgtactgggtgagggtgacgcgttcgagcaaaggtctttgcgcgatttgttgctagatgcaatccgctacggagaccagccggaggtaaagaagaaactcgaccagatcatcgactcatccgtctcccagggtctcgacgaattaatgcagaaccacggcctcgagcgaagcatccaatcgcagctggacatcgaggagctacgtcgccaaatggaggaagccaaggaacgccgcctgcagccgggcttcattgccgcgtttttcattcccgccttcgagcgcctaggcggacgcatcaaagaccgccgcgatggcacgtacgagatccggcacgtaccaagctcgctaattcacgccgcgcgggccatcaacccctggaacccggtaacgcaacgctatgagcgcgtcacgtttgacctcgacagggtatcgctcgaaggaggcacaaaacccacgttgttggcgccgggccatccgctcctcggtgtcgtgatcgaagaaactataaagcgcgaccacgccgatctgaccaggggaacggttcttgtagaccgccgcgatgccccaatcgccggaaccaccctcatcttcatcgtggaacagcggatcgttactgggaacgacaccagtgtctcgcaccatttcgattacgttctactcgaacaagacggctcgatgacactaacgaagactccgccgttccttgatttcgacgctccaaccgatgaggagttgtcgcaagtacagcaactgtttaaggaaggcttcgttcccgcccaccatgagaacaccatcaaatcctttgccctgagagaaggcgcggtacctcgcaagcgggaggtcgcagtgcggagggatgcagagctcggccacactcggagcgaggtggaagaacggctgaaaactgagatcaaccactgggcgaccgaaatgctccgtttgcaggaggaggagcgagcaggtaggtttagcaggctcactgcgcgtagagcggaagagaaagtcgccgacctccaagaccgtttggaccggcgactcgttgaaatcgatgcatctcgacagctcgctatccgccccgccattgtggttggagccgccctggtggtgccggcttcgctagtggcaccgcccgagaaagtgccagatacgtttgtgttgaatacggaggagacagagcgccgagcagtagacgcggtcatcgctgcagagcgcgctctaggcaggctcccggaggaacaagaccactacaatccgggttttgacatccgctcatatgacgatagaggaattggcttcttcattgaggtcaagggccgcgtagaaggcgcggacacgtttacaatcacctcgatggaggtcaacacagcgaacacacaaaaggcacagcatcgcttggcgctggtgcgagtgtccccgcttggaccggatcacgacgaggtccgctacgtggacaacgctttctcgcacattcagctgtctgccaccacccagtccatgaacgaaaaatggcgtgattattggtcgcgcggatcggcgccacactaaaaagcaacgggataagctcactgaggttatcaatgtagaacctggcatggctgctggtagcttccgccggcagaaccgaatctctgtcctccttgtacagttacccgcatggccgatcccgtgaagaaaaagctcatcgaagtctccctcccattggagaaaatcaacgcagaagcgtcgcgggagaaatcgatccgccacgggcacccatccacgttgcacctctactgggctcgccgcccgctcgccgccgctcgcgcagtgctctttgcgcagcttgtcgacgacccttcggcccaccccgaaaaattccccaccattgaggagcaggacgcggagcgtgaccgcctacacaagctcatcgaggagttggtggtgtgggagaactccaacgacgaacggctgctcgaacaggcccgcaaggagatccgcgacagcaatggcggtgagctccccgccgtcctcgacccgttcgccggcggcggtgccatcccgctcgaggcacaacgacttggtctcgaggcccacgccagcgacctcaacccgctcgcagtgctgatcaacaaagccctcatcgaaatccctccgaagttcaaggacatgcccccggtcttccctggcgcagcggaaactcgcacagagtggaagggcgccgagggccttgcagaagacgtgcgcctttacggcgagtggatgcgcgacgaggccgaaaagcgcatcggccacctctacccaaaggtgaaggccccgggcggcacggaacacaccgtcatcgcctggatctgggcgcgcaccgtccgcaacccgaacccggcaaacccgatcgaggttccgctcgtccgttcctggtggctgagcaagaagaagggcaaggaagcctgggtcgaggcgaaggtcgtcgacggtgaggtccgctacgaggtccgccacgatgcgaatgggccgacgggagatgcagacgggacagtgaagcgtaccggggcagtgtcgattgctgacggcactcccatcgatttcaagtacatccgcgaagaaggccgcgcgggtcgcatcgggactcatctgattgcgatcgttggccaagataaacgggggcgcatctatgcctcccctaacaagctgcatattgagacagcagctatcgatcgaccgcgcgagctccctgttgggcagatcttcgactggccaggacgtatcaacgtttacaggtacggcatgaccgagttcagtgacctgttttcgaatagacagttggtggcaatgaacgagctgacggcactggtggcggaagtgcgaagcttggttgaaagccactgcaccacccaaggtcgaaatacctatcctgaagcggtggcaacttacctttcgtttgcagtgagtcgccaaagtgatcgactttcaaccttggccagctggcagaatggcccagagaagatccgaaatgtgtttgggcgtcaagccatgcctatggtttgggatttcgctgaagcaaatattttttcccaatcttcagggggcttccacggcaatattggctgggttgaggaagtcatacagcgagtgccaacgagtccgcccggatttgccgcgcaagcagatgcggggacgcgaagctacagtaacgcggtaatttcgactgatcctccgtactacgacaatatcggttattccgatctatccgattatttttacgtttggctccgccagtcactcgaatccttctatccagacttgactgcaacgatcctcaccccgaaggaaagagagcttgttgcgaacccccaccgattgggtggtagagcagcagcagaggaattcttcatcgacggttttaataccgtatttgaaaggattagacggggtgccgaggtcacgatacccatgaccgtttactacgcctataagcaacaagatacgcgcgatacgggaacttcctcgacgggctggcatacgttgcttgacggtctaatgaacactggctgggagatcactgctacgtggcccatgcggagcgagcgaggaggccggatgattagcgtgggcactaacgccctagcatcttccatcgtcctcgcgtgccggccgcgacccgagggcgcgccttcgactacgcgccgcgagttcacccgggcgttgaaaaaagaacttccagaagcactccgcacgatgctgcagggatcgatcgcgccggtggacttggcgcaggcggctatcgggccgggcatcgcgatttactcccgctactcgcgggtgcgcgatgccgacggcacagacatgggcgtgcgggaggcgctcattctgatcaaccaggtgctggatgaggtgctgggggagcaagagtcggacttcgatccggagacacgattcgcaagccggtggttccgctcgtatgggtggaacaaggagagctcgggactcgctgaccagctcgcgcggtcctcggatacgtcgctgggtgcgctcgagcgtggggggatcctgcaaacaggcggcggcaaggcgcgcttgctccctccggaggagatgtcgggggagtggaacgcgctcgctgacgacgcgttgagcatctgggaagctacggtgcgactggccggagtgttgcagagcgacggtgcggatggtgccgcgcggatgcttgtcggggtgcagcagcgggtgcagctcgacgcggtgaaggacttgggcttcctcctttttcacgaggcagagaagcgtagcgacagtaggactgctgggtacttcaacgcgctggtcacctcatggcccgacattgttgcgatggcgaacgatatggcagcccagggtccggaggcggtgcagggtacgttcgatctctaaggctggcccgtcgccgatgtgatgggtttagaaagtgtgtgcgctggggccggaggaacgacgacaagcgaagtagtgtgaagaacaaagagaacaaagatcactactggagcgaccatggccataagtaatagtcagcggctcgatgccgcgatgacgttgctgtctgagggtctcggcgactttgtcgacgaggttatgaccgaagcccacggcacggactggaacaagcgcgcggcgcgcgagtacgcgttgaagaacgggcaagaagagcgcgtacaggataagggggatccgcagacgcagctctacgcgatcgtaaacaataggtacctattcaaggatcgcttgtcgtacatgcaggtgggttgggtctccgaactcattgaggcccggaacaattgggctcacagaatgccggtcagctcggaggacacggctcgcacgttggacacagtcgagcgtctcttacgtgcggtggatgcaaacgactccgcagacgacgcgcaaaggatccgcgccgagctgcagcgaagtgtgtacgaggatcagacgcgccgcaaggtaaactcgttgaaggtgctcactgagcaatctgccggactcaagccgtggcgtgaggtgatccgcccgcatgaggacgtgctcagcggtaatttcaacgcggcggagtttgccgcagatctccacctcgtgcacacaggcgagctaaccagcccagagtacgcggaccctgttgagttcttcaaccgcacctacatcaccgagggcttgcgcgacctgctcactcgtgcgctcaagcggctgtctggcgacgaaaacgcgagcccagtggtcaacctgcagactaacttcggcggcggtaagacccactccatgctcgcgctgtaccacttgttctccggaacgccgatcacccggttcccgcaggagctacaggagctcatcggcgataccggggtagacctggaatccctcgatgtgaagcgggttgctctggttggcacgcacatctcgcccgctcaggcgatgcttaaggatgacggcactgagatcaacaccctgtggggcgagctcgcatggcagctcggtggccgcgaggggtacgaggttgtccgcgcagcggacgagaaaggcgtgagcccgggggatgggctacgcgatctgttcctgaagtacggcccagcaatcatcctcatcgacgagtgggtggcgtacgcccgtcagttggctaccgacaagtctctgcccgcaggttcctttgacacgcagttcacgttcgcgcagatccttacggaagcagcgcagtcggtgcccggcacgatggtcgtcatctccatcccagcgtccgaccacggcgatgagaagacctccaacatcgaagttggtggcgagaacggccagcaggcactcgaagcgctgaagaacgtcatcggccgcaaagccgatcagtggcggccatcttcgaaagacgagtcgttcgagatcgttcgtcgccgtctgttccagtccgccgacgcggagggcctgaaggcgatcgcagccacggcgcgcagcttcgtcaacttctaccgggacaacctgcagcagttcccgcgcgcggtttccgagccggggttagagtatgaaaatcgcatcaaggcgtcctacccgctgcacccggaactgctggaccggttgtacgaggactggtctacgctcgagcggttccagcgcacccgcggtgtgctcaagctcgtgtccgtgatcgtttacgagctttggaagtcgcccgaccaatcgccgatgatccttccaggtaacgtcccgcttgatgcgacgacggtctccacagacctcacccagtacctggaggagcaatggacgccgatcatccaccgcgatattgacggcccgggatccacagctgcgcggattgacatcgagcggccgagcctcggctcgcgacacctcacccagcgcgtcgcccgcacaatttttatgggtgcggcgccacggacgaagagcactcgcaagggtctggacaagcagaatgtgtacctggggaccgcgatcccgggcgacacccttggtaacttcggcactgcgctcgatttgcttgcgcaggggtcgacgtacttttacgaggaacagggccactactggttcgatacccagccatcagttgcgaaggctgcgaaagactacgcggagcagctgcgggaggatgaggaaaccgtttggaacgagatcacctcccgcttgcagaagcactcccgtggccagttcgaacgcgtccatgtcgcgcccgagtcgactggtgacatccccgaaaccgaggaacttcgcttggtgattgtgcacccgcggtactccactaacaataggagcagcggcaaggctaacgagtgggtcagaagtgcggtggagatgaagggagcatcccagcgcatcaaccgcaacacgctggtgttcctcgccgctgacagggcagaattggagcaactcgaggccgcagccaggacttacctcggctggaagatggtgcaggacacgagcgaatccctcaatctcacgccgcagcaactcaagcagacgaacgatcgtgtgcggcagaccgatctcgcggtgcagtcgcgtctcgcagacaccttcatttggtgcatgtaccccgagcagccggaccccgagcagggattcgagattgcacaggagcggttgtcgggctctagcagcgcctcgctcgcggagcgcgtctgggagcgcctcaagcgcagcgatgtcatcatcccgctcttggcccccgaaatgctcggtggcaccttgcgccgcgagctgggcgaaatgtggcgggagcgcaaggagatctcagtgggaacactttggacgtattttctcaagtacccgtatatgccgcgtcttgccagccgcggaacgttagacgacgccgtagccgcagccgcaaccaccttcttctcgcaagaggatgagttcgccgtcgctgcgggtaagagcctcgtaaccggctcataccgaggccttttcatgccccccgcagacaccgaagtgagcgtcacagacagtacgttgcttgtcgacgcggacctcgcccgcgaacagctctcccaacggcctgcccctgagccggagcctggccccggccctggtccgggcactgggggaggcagtggcaccggcaccgggggaggcccaagtccgacacctacaccgccgcctccgtcgctagtcccgcctcagattgataaaaagactcgctactacggcagcgtccgcatctcagccggcgaatacggaaggcgccagagcaacatttggaataccatcgtggagcacttgattaagtcgggtgctgaagtgaacctcacactcgatatcgaagccaaacttcccactggctttagtgaagatacgatgcgcaccgtgaaggagaatgcacgaacaaacggcttcagtgataacgagttcgacgattaggggcgggattctggttagattgcccgcagatttttccgtgagcgtcatgcagtaattgagaagccgcgagcggaagcgcctgaatgtgagagggcattggcgatgaaggcgttcattgcgactgcggagcgtggtgcgagcggcacttgagtgctggagtgcgacgaactgggggtggtctcgcagactcggaggcccgacagtgcggaggatgacgtcgcggaggcgatcgcatttcaatcggggtttcagccgggcgagtacgggatcgaggttgtgcccattctcctcactgaggttgagtggttgcggctgcgtgccgacgacctcggcgtgaaggtgaaagctgcgtcggatgaggctgtcgccccaaggtttgcgctggcgcgcaagtcgaaggacgaggggtttacgctccgcgagaaggggcaggtgctcggggtgtcgtactagcgggcgtcggagttggcggcgggttagagcggcgaagatatggtgaagctacaaggaaatccagtctttagacggactgcgcctcattaagcagatcaaggaagggaagcgcccgggcgaagagatcacgccgtttctgcgatgggtggctgactacggctcgccgggctttcaggtcgcgcccctggtaattgagaacccgaacgactagggcgtgagcgcatcaattatcccaatctgggattgggtctagagggagctctgcgggctcgtctaacttgtcagcccacccatcaggtaggtcacttgtaatcgagtcgagcacttccgcggctgactttcgggcatcggcggggtctttcatggccgtcaccctaaaacaactctttgacggctgcgcggtccaccttgcccggcccgagttgcggcagcgccgcgaccaccttgagttctttcggtatctgccagtgcgcgatgcggcccgcgtcctccgcatctgccagcgcgtctaggacgtcgggcactgacgcggagccggtgtaggcggcgcagatgcgttgacccaggcggtcgtcgtctttgctgatgacggtggcggcggtgacgccgtcgataagcaagagctccttttccaacacctcggggtggagtttgaggccgccggaggagatgacgttgtcggtgcggccgaggacagtgagcacgccaccctccagcgaaccggcgtctgaggtgcggaaccagccgtccttgaggtcgggggagtcgagcagatggtagccgcgggcgaccatgggaccgccgaggtggatgcggccaccgacgattttcacacgggcgccggcgatcgggcggccattgtagacgcagccgccggaggtttcggaggagccgtaggtggtgaccacgttgatgcgcagcttcgccgccgattcgagcaggcgcgggttggtggcggcgccaccaatgaggaccgcgctgaaggttcgcagcgcgtcgatgccttgcagtgtggaggtggccttggccagctgcatcggggtcagtgcggtgtaggtgcgctcaccggtgcgggccagctcgtgggcgcgggcggcgaattcggccacgttgaagccgtgtgagaggtcgacaaatgcgggttccacgccggcaaccatgctgcgcaccagcacttggatccccgcgatgtaggcggcgggcatagctagcagccactggccctcgccgccgagcgcttggtgggtagcgtcggcgctggagatcaggtttgcaggggtgagcatcgcgcctttgggtgtgccggtggaaccggaggtggacacgactagtgcgatgtcgtcgtcaacaggcgcgccgggcttcagggtgttgcgcagcacgttggtgcgcgccgggtcatcagctggcaccggtagaagcgtgcggctgccggtgagcgcctcctcgagcgcgggcatgatagccagggggttagccgggtcgacgggggtcaattcgaggaggtgtgacacgggggataagggtagcaacctgtgaggtctcctaacagagcaagctgttgctggaggtgtggaaccatgggcgggtttgctgggtctaaatcggtatgaggaattccggagctgttgcgtggttgtttacggggttggcgtcggccgtggcgcttgcttacgcggtggtgttagcgctcggcccaccaaacatgacagcaccggtcctggatttctccgcgaagttgatcgggccgttaggtgcggcgcttatcgcttgggcaggtgtgtcgcacacggtgttgaactcacggctgcaggacaaagtgaaagagtggcaccaggatttacggtgggcgacggagctgtgtgcctcatctgactcattccaggtagccgtcgggatagcggtgctggatgagctcgatgggcagccgtttctagaacctgagcaggttaagatggtgaacagaatcgccgatgttgcaatgcagaaactattcagtggggtagcagaggaacgagaaaggcgggacagtgatgcggtttagctacaaagagaacacgaccctcgagggcgttcgcttggcgcgcccgccgcatgttggcgagatcgcggcggcgaacctcattattaagcagatcaacgagggcaagcgtccgggcgagaaagttacgccgtttctccagtgggttgctgattacggaacaccgggttttcaggtcgcgcccgtggttatcgagaacccgcggggctaggccatctgtgaacgggtccacaggcagatccgcagaagacgtcaggagccgcgctttcctaagcccggcaaaccgccgctgacggtgcggctgtggaagtcggggtcatacgtgttgatcttggctaggtctaacgatcgctgaagctccatcttggaatccacggcttcctcggcctgcctgcgtaagtcggttcgctgcgattgggtgagtttggcgtcgcgacgcgcccgcttcgcgcacagtgtttcggcatcggcgacttgatggcgggcgataatctcggcgacgcgttcctgtttttccttgcccggcgggcgcgggtatttccgcgcgaactgcacgaagctgccgctgcacattctcccgtcggagtcgtggccgtgctcgtgcaccatgttcttgtccagatcggcgcgaacccacactttgcagaccgggcactcaacgcgcccgtctttgcggacgtttgccaccggcttcggttttctacgctgggggtgcgacagggccacgattgatcctccgtacggtcttgaaagaagtatggcggatcccgtggcccggcggctgggttttgattccgtactagacccacctagtagtagtacggaaactcctcccagttcggagggcgcttctccaggaaggagtcgcggccttccaccgcctcgtcggtcatgtaggccaggcgggtcgcctcaccggcgaagacctgttggcccatgagcccgtcatcggtcaggttgaacgcaaacttcagcatgcgctgcgcggtgggggacttggtgttgatttcgcgcgcggcctggatcgcctccgcctccaactcggcgtgcggggcgacgatgttcaccgcacccatgcgctgcatctcttcggccgtgtacgtgcggccgaggaagaaaatctcgcgggcgaacttctgcccgaccatcttcgccaagtatgccgagccgtagcccgcgtcgaaggaacccacgtcggcgtcggtctgcttgaaacgggcctcttcgcgcgaggcgatcgtcaagtcgcacacgacgtgtagcgagtgcccgccgccggcggcccagccgttgaccaccgcgatgaccaccttgggcatcgtgcggatcaggcgctgcacctccaggatgtgcaagcgcccgccctcggccttcacgcgcgcggtgtcgatctcgccagagtcgctgccgtactggtacccggagcggccgcggatgcgctggtcgccgccggaacaaaacgcccagccgccgtccttttcgctcggcccgttgccggtgagcagcacggtgcccacggtcgggtcttggcgggcgtggtcgagcgcgcggtagagctcgtcgaccgtgtgggggcgaaacgcgttgcgcacctctgggcggtcgaacgcgatgcgcacgatgccgtccgctcgcgtcgtgcccacgtggcggtggtaggtgatgtccgtgaaatcgaaaccctcaaccgcgcgccactggctcgggtcgaagggattctcggtgctgtactgcatgggggtaatcgtactcaccaccccttccaagttaggacagccttgctttattatcaggtgcatgcaggagcatgtgcttatcgacgtccccgtcggccaccaagccaccatcacccacgtgggctgccccacggctcgtcgcctccgcgagctgggtttgcgcgccggggcgaacgtcactgtcatgcagaaaaccgccggcggcggccgcgtggtgaaggttggcggctcccactacgcactcggcgcagccgccttgcggttgatcacgatcgccccggccggtaaggccgcgtaatggctgactgccacggcgccccagttgccgaatatgccccggtcggcaccccgacaatcgcgctggtcggcgcgccgaacgccggcaagtccacgctcttcaacgccctgaccggtgcgagcgcgacgatgggcaactaccccgggaccacggtggaggtctcgcgcggtgtgtggcgcccgcagggtgcgacgtacaacattctcgatttccccggcgcgtactcgctcgacccggccagccccgacgaagcgctgaccagggagctgctgttcgacagcgctaccggcaccgaccgccccgacctcgtgcttgccgccgtggacacctccaacctggcgcgcggcctctacctggtcgcacagcttgcggagcacccttaccgcgttgtggtggtgctgaccaagagcgacgtggcggcgaagcaggggctcgaggtggacccggtggtgctcgagcgggagctgggcttgccggtggtgacgttggatcctcggaggagggatgtgagtggggtggcgggggtcgtcgctaagcaattgctccttcctgccgcagcggcgagaacccctgtagccggcgacgagttcgagcaggcagatgagcgcttcgagtggattgatgcggccgtggctgcggcgaccgtgcgcgatgagcaccgcgacacgctgaccgagcgcgtggacaaggtcgtgctgcacccggtggccgggccgatcatcttccttttcgcgatgtttctggttttccagatcacgaccaccgtcgcagcgcccctgcaggacgggctcgacgcgttttttaccggccccctgtcggactgggcgcgcgccgggctggagcgtatcggcttgggctacccgtttgtggaggggttgattgtcaacggggtgatcggcggcgtgggcatggtgctgacgtttgtgccgctgatggcgctgatgtttctgtgcctggcggtgctcgaggattccgggtacatggcgcgcgctgccgttgtggcggaccgcctcatgcacacgatcgggctgccgggtaaggcgtttatcccgctgatcgtgggtttcggttgcaacgttccggcgatctccgccacccgcgtgctggcgactccggagcagcggcggctgacggcgctgctcgtgccgttcacctcgtgctcggcgcgtctgacggtctacgtcatgctcgcgcagacgttcttcccggaccatgcggggctggttgtgtttgcgatgtacgtgatttcgatcgcgctggtcgtgctcgccgggctgctgcttcgctcgacactgtggcgcaccatgggctcggaccctctcgtgatcgacttgcccacctaccagctgcccaccgcgcgcctgacgctgtcggtgatgtggtcgcggctcaaaggcttccttcacaccgccggcggcatcatcgtggccacggtggtggtgatctgggcgctgcagtccacgcccgcggtcggcggctacagctggggcgacgaggacctgccacccgcggactccgtctacggggtggcctccggtgcggtggccccggtcttcgaaccggctggcttcggctcgtggtcgctcaccgggcctttggtgaccgggttcctagccaaggaggcggtgatctccacgtgggcgcagacctacgcgctggaggatccgtctgatctggacccggctgagcggggccagtccgatctggcggcggccgtgcgcgccgactttgaccaggcttccggcgggcacatgatcgccgcggtgtgggcctacatgatcttcctcatggcgtacaccccgtgcgtggccacgctcgccgcgcagcgccgggagatcgggtggaagtggacggtgttcggcctcgtcggccagcttgcgctcgcgtggacgctggccgtggccacgttccagatcctgcaggtgtttttctgatgcgccccatgcaagcggtcgtcgccgccattgataaaggtgcccgctcccgcgccgacatccgccgcgagaccgggttgaccgattcgaccgtcgacgccgtcatccaccacctcgagcgcaccggccatctcagcctggaagagctcggctcgtcctgcgccggcggcaactgcgggtcctgcatcgccgccgcggccaacggcggcatgacgtgcgccgaccggccgaaggtcaagggcccggtcgcgcttgtgctgacgaagcgacctagttaaccaagcgcccggggcgacctactgcgcgagcaccagcgcgatcgaccccaccccgagcaggatcacagaggcagtcagcacgagcacccggtgcatgttcggctgcacccgctcgtcctccaggccggccacttcgcgcttgtaatcggcgtggttggaaagcacaacgaagcccgcgctcaacgccaaaagcgcaatcaacagcagcaccgcgggcccgtacacgtctgcccagcgcagcagcaccagcgcgacgaccaccatggccaccgccgtgcgcgtccacgacatggacgtgcgctccggctgcagcccgggatccgcgtgtgcgtggaggtcggaccgcaccggctacaccacgatcagcacggcggtgacgacgagcgccaccaccacaactagggacagcaccggcacgatcgctggcaccggcagcgggcggccagtgcgcatcgcgcgctccacacgcacccaccgcacggccgcaccaccggcaatgaggatgcctgcggcaatgatcagtaccgccactgccttctgccgcgagtggtcgagccccgcgatgtcgaacgccgccagcgccaccccgccggccagaaacgcaagcgccgttcgagtccaagcgaggaaagtgcgctcgttagcaagggtgaagcgcgggtctggctcggtgccgtcggggaacagccggcgcgcaagcgcgctgcgatcgggtgcgctcatgtgccccaacgctacgctggctgccatgcacctgcccaccgtcgatgagatcctcgagcgctcacacgtggtcgcactgcccatggccgtgcgcttccgcggaatcaccaccagggaggcattgcttattgacggccccttcggctggggagagttctccccgttcgtggagtacgagccgggcgaggcgaagcactggctgcgcgccgggatcgaggcggcgttcgagggactgcccgaagtcgagggcgacgtggaggttaacggcaccgtgcccgcggtgagaccggaagaggtcgaagcggtcctcgagcgtttcccgggtgtgggaaccttcaaggtcaaggttgcggaaaaggggcacgcattgcttgacgacgttgcccgtgtcgcagccgtccgccgcctccgacccggtgcagcgatccgagtcgacgccaacggcgggtggagcgttgccgaggccgtcgaggcggagcgccaactcaccgccgagggtcagctggagtacatcgagcagccgtgcaaaaccgtcgaagagttagcccaagttcgcgcgcgggtgacgacaccgatcgccgcggacgagtccatcaggagggcggcggacccgtacaaggtggtggcgctgggggcggcgcaggtgggcgtcgttaagcaagccccccttggtggggtacggcgcaccgttgcgcttgcccgggagctgaaccttcagctgaccgttgctagcgccttggacactgcggttgggatcaacgcggggttggtggcggcgaaacttgcgggctcgcgcgcggccgggcttgccacccagcggctgtttgtggaggacatagcggaaaagcgacagcttagcaacggcgcgctgtccactgcgccgctgatcccggacccggagcgtctccacggcttgcgcgcccccgctgaccggcgcgaatggtggtaccaacgggtggctgactgtctccccctgctcgggggtgaaacttcttaggcgggcaaaatttctcctgtttgggttccgtttccgggggtgatggcggttaagttttaagccatgtcaactcccgtcatgctcgattccaccgcccagtcggacggtgaccttgccaagagcccggaaccgggcgagtggcgccgccaacttatcggcctgatcgccggcattgtgctcgccgcgatcgtttactggatcttcccaaccggcgcggctgacaccgtcagccagtcctccggtgcgaaggaaggcgtggagtactccgcgcaatccatgcgcgtcgtcgccaccaccaccgtgctgatggccgcgtggtggatgaccgaggcgatcccgctggcagcgactgcactcctgccgatcgcggtcttcccgatcatgggcgtcgccccgttcaaggaggtctcgtcgccgtacgcgtcggcgacaatcttcctgttcatgggcggcttcctcatggcgctgggcctgcagcgctggaacctgcaccgccgtcttgcgctgatggtggtcaagctggtgggcaccagccccaagcgcatcatcctgggcttcatgctcgccacaggcttcatgtcgatgtgggtgtccaacaccgccaccgccgtggtgatgctcccgatcggcacctcggtgctcatgctcaccgctgattccgtcggcggcatgcagaaccagaagcgcttcgccactgcgctcatgctcgccattgcctactccgcgtccatcggctcgctgggcacgctgatcggtaccccgccgaacgcgcttttgaagggctacatggaggaggcgcacggcatcaccatcggcttcggtgagtggatgcttgtgggtatgccgattgccgtcgtcttcaccttcgtcgcctggtggcttttgatcaccgtgttcaagccggagatcgaccagatcccgggcggcaaggagctcatcgacgacgagctgaagaagctcggggcctggactgccccgcagatcatggtcggcctgatcttcctggtcgccgcgctggcatggatcttcatcccgctgggccgcaacgcgttcggctgggacttcccgtacgacgacgccattgtcggcatcatcgccggcctgctcatgttcaccattccggcgaagggcgacggcaagcgcctgttggactgggagaccgcgaaccagatgccgtgggacgtcctgctgctcttcggcggcggcctcagcctgtcggccatgttcaccgccacgggcctgagcctgtggatcggtgagaaggcgaagggtctggcgtccctgccgatcttcctgctgctcgcggccgtcgcggcgctcgtgctcttcctcaccgagctgacctccaacaccgcgaccgcggccaccttcctgccgatcatgggtggtgtcgcagtgggcatcgggcttaccgacgccaccgacatgaacgtcatgctactcgccatcccagtcgccctcgccgcaacctgcgcgttcatgctgcctgtcgcgaccccgccgaacgcgatcgcgtactcctccggctacgtcaccatgggcgagatggtcaagggcggtatctggctcaacctgatcggcctcgtgctgatctccgtggcgacctacttcatcgccgtcccggtcttcggtctggtgctataggttttcacccccgcttggcgcgttaggcttatccgcatggataaccaaacgcgccaatttggtttcggggacccgacacctcagcgcccgggccgcccgcagcagtatttccccgacccgcaagcgcagtcggggtactacgaggagcccgagtacgccgcccccgagtactccgctccggagccgccgcagcgctccaacaccgccgcggtggtgctgggcttgctgtccgcaatcctcgccgtcgcgtccgtcgtgttgttcttcctctggcgctccgcggcggaggaggcgaacaagcccccggtgaccatcacccagaccaccaccgccacaacgacggagactacgacgcgccgcccgttcgacttcgggcagcgccagaacgagtcgcccagcgcggatcccggcgcgaacccgaacccggcggagccgcagccgaccgcggtacagcccccggcgccggagcttccagaagtcgacatcgaggatttcctgaaccgtctcgacggcttcattgagcaccctgagtcggtgttgccgcaatgacgtactacgcgcaacagttagccaacgccgtcgtcgacgtgctcagccgcaacgtcaccgacgtggtgatgagcccgggctcgcgcaactcgccgctcgcgtacgcgcttctggccaggcgcgacatccgggtgcacatgcgtatcgacgagcgctccgccgcgttcaccgccctcggcatggcgcgcgtgcagaagcgtcacgtggccgttgtgatgacctccggcaccgctgtggcgaacgcgtaccccgccgtgatcgaggcgcacatgtcgcacaccccgatcgcggtggtgagcgcagaccgcccgcaccgcctcgtgggtacgggcgcgccccaaaccatttggcagcaggggatcttcggccgctacgccgaaacgcagcgggtggatacggagcaggacgtcgccaagctgtcgttcgacgccgaccaggtccacatcaacatcgccctcgacacgccgctggtgcctgagaccttgccggcttctgcggggaaggcgaagagggttggcccggggcgtctacaagcaaagccctcctgggtcgaccacggcgcggtcgacgtcgacctgaccaaggacaccctggtgatcgcgggcgacgaggcgtgggaggtgccggggctcgagcacgtgccgacgatcgctgagcccaccgcgccaaccccgttccaccaggtgcacccgcttgccgcgcggtttttcctgcagtccgaggtgtcgatctcgcacgacggtggggatttcgcggcgtcgacgaagccggagcaggtcattgtggtggggcacccgacgctgcaccgcggcgtgatggcgctgatggccgacccggacattgaggtcatcggcctgtcgcgcaccgaaattttcaccggcaacccaatgaggcgcggctcgcgcgtgaatgtaaccggccagccgaccgacacgtggctgaagatctgcgaggcggccggcgaggtcggtgcggagaccgtgcgcaccacgcttgaagacgccgcctttggcttcaccggcctccacgtcgcagcagccgtgtgcgacaccctcgcagtcggcgacacgtttgtcgtcggctcatcgaacccggtgcgcgacgccagcctggtcggcatgccgttcgacggtgtggacacctactgcccgcggggagcagcgggtatcgacggcaccgtgtcccaggcagtcggcgtcgcgctggccacccaggcgctgcgccccgacgaaatccgcgcgccgcgcacggtcgctctcatgggcgacctgacattcctgcacgacgtcaacggcctgctcatcggccccggcgagccgcggccgggcaaccttaccatcgtggtggccaacgacgacggcggcgggatctttgaaacactcgaggttggggctgaggccgtgcgcgagccgttcgagcgggcattcggtaccccccacggcaccgacctggcggctatcgcggacgcgtacggctgcgcgtactaccgcgcggagaacatccccgaactgcaggagatcctcctcgagctggaggcgaaccccgcgccgatcgcggtcgtggaagcggtcaccacccggggcacccggcgggagatggcgcgaaagttcacgtgaacttcacgtttcgttgacggctagtttcagcggctgtgtcaggctcgactgttatgcgtgtaggaattgtggccgagtcgtttctgccgaacatcaacggcgtgaccaattccgtgctccgggtcctcgagcacctcaaggaggagggccacgaggccatcgtgatcgccccaggcgcccgcgattttcaagaggaggtgcccgactacctcggattcgagatagttcgcgtgccgacggtgcgcatcccactggtggactcgctgccggtgggcgtgccgacgaccacggtgaccgcggcgctcgccgagttcaagcccgacgtgatccacctggccagcccgttcgtcctcggcggagcgggcgcgttttccgcgagccagctcgatgttcccgcagtcgcgctgtaccaaacggacgtggccggcttcgccacgaagtaccacgctgcgatgatcgcgaacgtggcgtgggactggacccgcaccgtgcacaacatgtgccagatgacgcttgcgccgtcttccgaggcgatccgcgagctggaggaccgcggcatcaagaacgtgcgacactggggccgcggcgtggacgcggagctgttccacccctcgcgccgaagcggagagctgcgccgcgagtgggatccgacgggggagaagaaggtggtcgggttcgtcggccgccttgccgccgagaagagcgtgcaccgcctggcgccgttgaacagcgacgactcgatccagctcgtcatcgtcggcgacggtcccgagcgccccgcgctggaggaggcgctgccgggggcggtgttcaccggctcgttgtcgggcgaggacctcgcccgcgcttacgccagcttggacctgttcgtccacaccggcgagttcgagacgttctgccaggccatccaagaagcgcaggcctcgggcgtgcccaccatcggtcccagggcaggcgggccgatcgacctgatacaagaggacgtcaacggccggctcctcgacgtggacacgttcgaagaggatctcccggaggcggcggcctggatcctcgacgacacccggttggacgagctgaaggccaacgcccgtgagtccgtcgcggacaagacgtgggacgcgctgtgccggcagctgatgggctactatgaggaagtggtgtccaagcacgaccgcaagcatgtgcgtatcttcggcaaggacgttgttgtgccgcggtggatgcgcctgccgcggcggcgcaagaatgcttagggggcagtcgtgagtaagcgtgcatctcaggcagcggccgcgtgcctggccgcttccgtggcgctcgcggcgaccggctgcagcgttgtgaacaacgtgaaaaccgtgggtaacgcgctcgagggcgctgcaagccccgcgaccgtgacgctgggggagttgctgccgccaatccagcgggccgcgatcgcgtgcccctacagcggtgagggcgtcaacgagctgttcggtgagacggtgttccgaaacgaggacttggacgattcggtgaactggatcgtggccaagctcgagcgcggcgcgctggtcaaggagcgcctcaacagagcagaaatcgacgtgtgcacctcgggcgaaagcgtgcgcgagatcggcgaggacgagccgctgcgctttgaaaaagccgacgggtcctccacctgggtgctggccaactaagcgggcgcgtaaactttcccaccatggccaaggcagacctggacaagcaaccttttgacgtcgcgggcatgttcgacgacgtcggggagaagtacgacatcaccaacacggtgctctcgttcggcctggacagaaagtggcgcacccgaacccgcaggcgcctcgacctgaaacccggcgagcgggtgctggacttggcggcgggtaccgcagtgtccaccgtcgagctggctaagtccggcgcttgggtcgtggcatgcgacttctcccagggcatgctcgcagccgggcgggagcgcaacgtgccgaaggtcgccggcgacgccatgcacctgccgttcgccgacaacaccttcgacgcggtgactatctcctacgggctgcgcaacgtccacgacttcgaagcgggtctgcgcgagatggctcgcgtgaccaagccgggcgggcgcctagcggtcaacgagttctccacgccggtgatcccggggttccgcaccgtgtacaaggaatatcttccggtcgcgctgccccgggtggccaaggtgttttcctccaacccggaggcttacgagtacctcgccgactccatccgcgcctggccgagccaggaggagctcgcccgcgcgatcaaccgaaacggctggcaggacgcgggctggcaaaacctcaccggcgggatcgtggcgatccacagcgctgtcaaacccggatagggtctgcccactgaagtgtgcggccgcggggctgctttccccaggtagtgcttttaggctctgccggtatggggaacacaactttttacgcggaggctgagacctctggaacttacggaacgcagctgcggggaacggtgatgatctccgcacgggggaaagacgtcagcgatttcggctacgagatcggggacgcgatagtcgaggccattgaggccgcagtcttcgagtacgaacctgtcgacgactcgcaaccgctctccggcgaaacgctggaggagctcacccagatcaccattgtggcccgaaccctggtgagtgtgccgccacgcaagcgcgacgcagcgagtgcggcggaggaagcagactccataattgctttttgcggggagggcttaaagcgggagccgcggtttgtgcaagcgtatgcctacgcgctggcgatgcgtagccaagataccgagcggcgcctcgcgcagatgcgcgccgcggttgccgacgttctgcccaagccgattaaacccaccgggaacgaagcgcgcgtcatgcgcgtggaaatacacgatttcaagtccgaaaaactcaaggacagctctgggcgcgtacgggtcgggatgaccaccaagcacaccccgatgacgggcaaacaggcgaagaagcaggttggccaggcggtgttcttcccgctgccgctgttcgacgacaagcggctggggtcacgtgtcgagactcagttctccgtgcacggcatgctagtcgccgtcgtcattgagaccgcgaaaccggcgtatggcctgctgcgcgcggtgctacttgctgttgaagaggtcgtcgaggactacaagctactcgacgcggcctagtccatttcctacgcaacatcccacagcggggcgttgcgcggggcgacgcggccggcggtgcgccacgcgcgggcgatcaggtcgcggtccccgtcgtcgatcaggttgcccatcaggcgggcggccgccggcatcagcttcgcgccgaccggcccgcgcatccccaaggggccgacgagcgggaggaactgcgggtaggtcagtagcctcgccgcggagcgcgccagggtgaaggcttcgccgtaggactggcgcagcgcgtgtggccaggcaagtgtcaggtcgcgggtgccgcttgcgatgagttccacggacatcgccgcggtttccatgccgtaatcgatgccctcgccgtttaaggggttgacgcacgcggcggcgtcaccgatgagcgcccagttcgggcccgccacgttcgagaccgcaccgcccatcggcagcagcgccgaggtgacgtgttcctccggccccagctgccaatcgtcgcgctgctgtgccgcgtagtggctgagcagcttcttcgtgttcaccttggccggccgcgcgtcggtggacagcgcgccgcagccgaggttcacctgcccgttgccaagcgggaaaatccagccgtacccgggttggatcgcgtcgccgtcgcgcagttcaacgtgggagtgcatccacggctcgtcggcaagcggcgaggtgcagtagctgcgggcggcgatcccgtagacctcgccgcggtgccacacccggccgagcgttttgccgaaagaggagcgcaccccgtccgcgacgatcacccacttcggctcgacgtcgccgcgcggggtggtgacaacgctgatcgcgccgccggaaaactccgcgccggtggcggggcagtcgcgccacacggtagcgccggcggcctcggcttcgcgaaccagcgccgcgtcgaactccatgcgcgggctcgcagacccttcggtgccgtagacgccatccggccaggcggcggtgacgtcgccgccgtagccgtgcagcttcaggccgcggttgcggtaggccggcagcacatgctccaagtcgaaagctatgagggtgtgcactgctctcggtgtcaggccgtcgccgcaggttttgtcccggggggttggggctgcgtcgataagcaatgtgctccaacccgccctctgcgcggcgatcgccgccgtcgacccagagggacccgcaccaaccacgaggcagtcgaacctttgcgcactcacggtgagccattgtgccagctcggccctgctgcattgtggacggggattggtggactacggttaagggcagtcattcgcccgttttcaacttttcaaggacatcaccgatgaccaacggcatcacaccgccaccgcggggcgggttccccctcgatctcggcgatgaggggctcaccgagcgcatcgctcgagatttggctgctgtggaggagatgctgaaagaccggctgaacgacggtgaggatttcatcactgagaaggtcaaccacctcgcgttcgccggcgggaagcggttccgccccatcatcacgctgctgtgctccgaattcggaccgcacccggaagcgatcaacgtgatccgcggcgccgtgctcaccgagatggtgcacttggcaacgctctaccacgacgacgtgatggacgaggctgagaggcgccgcggcgtggagtccgccaacgctcgctgggacaactcggtggcgatcctcgcgggcgacattctgctcgcgcagagcgcgcggctgatgagcgagatcgacacccacaccgtcaagcacttcgccgacacgttccagacgctggtcaccggccagatgcgtgaaacggaagggctgcgcggcgcggaccctgtggaccactacctcaaagtgatcgaggaaaagaccggcgtgctgatcgccttggcggcgtacctcggcgcgctgcattccggcgcggacgaggagacggtggcgcgttgccaacgcctcggtgccgcgatcggcatggtcttccagattgtggacgacatcatcgacatcttctccgaccccgagcagtccgggaagaccccgggcaccgacctgcgcgagggggtgttcaccctcccggtgctctacgcgctggaagaggattcgccggcaggtgaggagctgcgcggcatgctgacaggcccgctggagagcgatgcggaggttgcgcgggcgctcgagctgatcggtcagactgacggcagggagcgctccttgacgacggtgcggggctacctcgacgctgtagaaacggagctggcgggccttcctgcctcgcccgcaaaggacgccctgctgcgtttgtcgcggtacacagtctcgcgcgtcggctaggctcacctgccggtttgcgtctgcacgggcgcagtgttgtagagtgatctacgcacttcaaacgtgctcgccaggttgcccgagcggccaaagggagcggactgtaaatccgccggcattgccttcagaagttcgaatcttctacctggcacagtttgaatcggtatcacccgtcacctgcaaggtggcgggttttgtcgttcgcgggtgccgtgccggggtgaggcctaaggggcagccctacgggggttaagggtcaaaaagtgtgtccgtgagacatgtgtttcggtgccaaaaaccggggaataaccagccgatttgtgcaacattgcagtggcgggttaatctttccaaggcttcaacagagagggccgagcgaaacgaaagaatcgcggagttcacgaagaagaggctgtgcccccttagctcagtcggcagagcgtttccatggtaaggaaaaggtcgacagttcgattctgtcagggggctctgttgtttgtctgccaacggtacgacgagcacgatggcggtgtagctcagtggtagagcaagcgactcataatcgctgtgtcgagagttcaattctctccatcgctacttcccaagcacgggagccggcaggcgcccgtggtagggtctaggtgcattgcgcgttttgccgcgattgccctaggggcgtggcgcaattggtagcgcaacggtctccaaaaccgtaggttgcaggttcgagtcctgtcgcccctgccagaacttttaagttggaggagttctcttgactaatccgaacggccagaccccggcgcagcccaccggcaagcgccagctgcgcggagtaactcctgtgtcctctgctgactacgaggacaagcgcgccccggcgaaggacaccaccgccgactccgaccgcgaaagctacggcggtaaaggtgtagcggcgttcccgggcgaagttgccgaggagatgaagaaggtcatctggccgaccggtcgccagatggtcaactacaccctcatcgtgttcgccttcctcatcgtcctgaccgttttgatgtggggcacagactggattgccgccaaccttgttgagtgggtattgatccgttaggtatactccggagttgtacgtttcccgccacctcgagcaccgaggtaggcgggataatttgtctctcaccttcaaaggagcccaccatgacggagaacaacaaggacgttgaaagcaccgttgagaacaacgagctggagatgatcgacgagggtgcgccggttgagccggagacggacccggagaccggcgcccagcacgagcacgacaaggatggcgagtaaatggctacagacaacgacaacgtggaactcgaggccgctgctgaggcggggtacgtggaagacagcgcggcgcaggcaggcaacgcctccgacgaccaacccgaagccttggttgagttcgccgaagaggtcgaagacaaccaggagatgatcgacgagggtgcgccggttgagccggagaccgagccgctgctcgaggagaccgtcgacgagactaccccggaagaggagcccatccaggagggcgacctcgccgcagctgtatccgcgctgggcggcgacgctgctgacgacgactccgagtaccgccgccgtctgcgcgagtacaccagggagctgaagaaactccccggcgagtggtacatcatccagtcctactccggctacgagaacaaggtgaagaccaacctcgatatgcgtatccagacgctcgaggtggaggactcgatttacgacgtcgtcgtgcccatcgagcaggcgctcgagaccaaggacggcaagaagaagctggtcaagcgcaagctgttgccgggctacgtgctcgtccgcatggacatgaacgacgctgcgtggtccgtggtccgcgaaacgccgggcgtgacctccttcgttggcaacgagggcaacgcaacgccggtgaagcaccgcgacgtggcgaagttccttatgccgaaggtcgaggacgccagcaagcaggcggcgaacgaggacggcgagaccgtcattgccatgccggaggaggagaccccgtcgaaggtggcgcacgactaccaggtcggcgaagctgtcaccatcctctccggtgccttggcttctgtctcggcgaccatcaacgcgatcgacccggaaaccggcaagatccaggcgctcgtctccatcttcggccgcgagaccccggtggagctcaccgccgaccagatcgagcgcattatctagcttcccgcagatcacttttggtgattcggtagctggccgatacactcaaacgtcgcacccgaatgcggtgcggcgttttttcattcgttctccccggtggctgggccggccgatgaaggctagacccggcatccggaagggcgcggctatgcatcgtgaccgcgccccgtacctaggaattgaggtaattcgatggcaaagaagaaagtcaccggcctgatcaagctgcagatcgaagctggcatggcgaacccggctccgccggttggtccggcacttggtgcccacggcgtgaacatcgtcgagttcaccaaggcctacaacgctgcgaccgagtccatgcgcggcaacatcatcccggtcgagatcacggtctacgaagaccgctccttcgacttcgtcctgaagtccccgccagctgcgaagctcctgctcaaggctgccggcctgcagaagggctctggcgtcccgcactcccagaaggttggcaaggtcacctgggagcagtgcaaggagatcgcagagaccaagaaggaagacctcaacgcccgcgacatcgaggctggcgctgcgatcatcgctggtactgcccgctccatgggcatcgaggtcgaaaagtaaatccccatttgtggcagggccggccaggcccgcaccaaccacaactccttaaccggaaggaactagaacatggctaacaagtccaagcactacaacgagcagtttgcaaaggtcgaccgcgaccacctgtacaccccgctcgaggctgtgaagctcgctcaggagacctcctccaagaactacgacgcgaccatcgacgtggcaatgcgcctctccgtcgacccgcgcaaggctgatcagctcgtccgcggcactgtgaacctgccgcacggcaccggtaagaccgtccgcgtcgccgtcttcgccgagggcgagaacgctaccaaggctgaggaagcaggtgctgacatcgttggtaccgacgcgctgatcgagcagatcaacgctggccagatcgacttcgacgtcgccatcgctaccccggaccagatggcaaaggtgggccgcgtcgcccgcgtcctcggtccgcgcggcctgatgccgaacccgaagaccggcaccgtcaccccggacgttgcaaaggctgtccaggagtccaagggcggcaagattgccttccgcgtggacaaggcctccaacctccacgccctgatcggcaaggcgtcgttcaccccggagcagctcgctgagaactacggtgcgctgctggacgaggtcatccgtctgaagccggcttccgccaagggcatttacctgaagaagatcaccgtctccgcgactcagggtccgggcgtgccggttgatccgtcggtgcagaagaactacaccgagcaggcgtaagcgccgtatagctagctgccgctagctggctgctgaaagcggcgaggctcccatgtcgcgggaggcctcgccgctttcgtgttatgcgggggtgcggagtggccgatttggtgattcgcacctgtgcccgttagtatccctacctgaagtttgaacggctgctttgcggccgagctcaagtttcaccgaagaccgtcggttgcttcccccgcggaggcttaaagtgtctcgcaagagaccgacccacgcaggagaaacgtggcacacctttttggctgcctcgtgcttctgcacggggcagcttttcgttgtcccgggcggataacagaaccaagaagtaattggaaggaggcgtgtgtcatggcaaacccgaagaacgttgcggagttggctgaactgaaggaaaagttcgctggctcctcggctgtgttcctcaccgagtaccgcggtctgaccgtgggtcagctccagcagctgcgtggtgacctcggatttgacgttgaactgcacgtcgccaagaacaccctcgtcaagatcgctgctaacg

SEQ ID NO: 11 - DNA, 146011 bp, Corynebacterium cassirii
  source 1..146011: mol_type = genomic DNA
cgcccggccgccagcaaccggtgcaccgcccgcgatcaccgggcggattcccccgttcgcgcccgctgcgtgagcgccaccggcagcggagccagctgtaccagcgccgccgtaggtgccgtgggtgccgtgaggggtagcgccggctcccccgcccggcgcgccgggcacccccatggaccccatcggcgcggctgcccctgaagccgaacccggcgcggcgtgtacgcctagctctcccacgtgtgcccccgcaccggccggaaccgcgccgctgcggttcaccccgttcggcctcggcaccgcgcccccgccgaaaccaactgcgttcgccggcgcggacgcgatgttcgcgagctgagctgcagcgtcagccgagcggccaagcgctcctgcggtgcgcgcccctcgcgacaacgcgtcggtgtgcgcgaccacgcgtcccggagcgcccgggaccgcggggccgaagcctgccggtaacggcccggcagccccgccgccgagtagtgcgggcgcaggaagcgccttagtcctcgctcccgccgttcccggggcgccggccaccgccggcggcgctgccgtctgcccaccgtgcgtggccactgccgcgctcggatttcccgcggcgccagccggggacaaggcgcttggcgcacgctggcccggcgcgttgtgcgcccgcggggcggccagcgccggcagagccaaccctgcggatgcggcgctgcttacaactccagccgcggcggtgccgatgcctgacacacgcagcgccgcagcgcccgagttcagtcccgggtgcaggctcgggggcatggtgggcgaggcggccgacgccacctgcgtctgggttgcgcccgccctgatcgcctccacgacgtccggcgtcacttggccgtaggcgtgcaccacgtcgtccggggtcacggcgtgcgccaaatcggcgtgtccgatggccacgaaggaatcgcggaccatctccggcagcggcgagcgctcgaaggagggcgcagcaggctgcggcatctcgccgatgcggaatgggttgcccgaaatgcggtccaaatccgggtagagcttgctgaacgccggcaccgttgttgtcagcgacgcgctcgcgcgcgggccgaaggcggaaagaaacgtcgcctcgtagacggggcggatgtgcagcggcagcgctgccgccaccgccgctgctgccgcggccagggccgtttccgccgaagtggtggtagccagcgaggtgttgtgcgcggacatggcgcgggctcgcatggcgtacatgctcgccgcgcgctggatcttatttacccgctcatccgcgcggcgcacccacgccgtgtcaagcgacgtcgcgagcttctgccgcaccccgaaaagggaatggacggcagcgtcgagccgacccgcgacgtggccccagtaagcggcttcgcttgaggcggcggaaactcgggaggttgacatcaggcgctcgagcagccgcagatttgggggcgcgacggcgactggcggaagtgcggtgatcggggtagacgcggcgtgggcgggaaggtgggcgggttggagggaacccgtagcgccgccaagcgcatgctgccctcccgcttcaatgctgcgaaacgcccctgccaacgtgccgtcggttcgctccatgttggcgaggttgacttcggcggcgtgcgccgtgtcgttgagctgcgccgccatcacgcggaacgcctcgggcgcgtgaaagctggaaaccttgcctagggatcggccggcttcgcgaaaacccgacgcctgggagtaccccgccaggcctgggcggaagccgccgaggttgtcggcgagcaacgaacgcgcttcggcgcgcaagagcttggtcgcgatgtggagtgcgtcggtgtcgatcgaaacgtttgagcccatgaattcccccgggtgacttttaacaggtgagcggtctgggcgaaacgttaaccgccgcgcgcaggcagaaacaggggctgcgcgcacacttcagtggtcgttgcagatcaggggtcgccgccgcttaccggccttccgccgcgtaagccatgacgctgcgtatccaaaacgtaaacgccgcgataaacggggcgaccagccagaccactggctccgtcaccggcggggcaacccgggacgggtcgctgcggtggagcagaccggcggccacgtccccggtggcgagcgctgcgaacgtggccgcaacaccgcacaccgccagccacaggagatacagcgggcccccgcgagccttgccgcggcgcacctgcgcccacgcaaccgcggcgagcaccgccccgatcaccgcggcagcgagacagaaccaaccaacaccagcaaacgcggcgttgggggagctggcgtcttggtcgacgatgggcacgccgtcgaccacctcaatgacaaacgcggggcgggcgaacccccacactgcgccgccgacaatgccgaggaggagcgcggcggccaaaagccctgccccggcgccgattgcgcggggcagtcgtcggcgcaccggggtcggggcttgaatgagttgtggctcggtcacagccggcgagtttagctgttgcagaccttccagcggccatcctccttggcaaacagctggacgttttcggaggtgttgcccgcagccttcgaggtcacggtggcggaggcgcgatcaccatcgacgcgcacgtccgctactgacacctcggtcttcggcatctcgatcgcggagccttgctcctcttgggccgccatgatctgctcgaccatgtcgagggtcaagccctgcttctcaaactcctcgagcgccggttcgcgcaccgcggcgcaggagttgtcgaggatgacgcgggtccactttgcgaaggactcggggttggtgaccttccgcacgacctcctcgatctcgcggcgctccgccgccgtgccttcgcgcccgccggcaaccggctcgtaggtcggcacctcgaagccctcctccagcgggttgatgatggttgggatggcctggtcgccctgctggttcggcgcaggagccgcggcgtcatccgccggcttctccccatcgttcggcttgccgtcccccggcctggccgcgtcgccgttgtcccccggcgtcgctggctcggccgccgcggatgtggcagcgtcctgcgctgcgtcagcaaccgtggcctcgcccggcgccgtcgccgcggtggacaacccgccgccggtcgtttcggtgtcggagccgcacgacaccagggtgagcgaaagcgcggcggcggcgattgcacccgccgcggacttcgctgccgacattgaggcggtggaaagggtcactgcaacatctcctcgcggttgaaagttctttgagcattctaccaacgggtttctggcgcatccgtgcatcgaactagccaaggctctgaacgttgtctgtgagtactgtgtacgaccatgcaactcagccaggacgcaattacgcaggccgcgatgaatatattgcgccagtacggcctggcggatgtgtcgatgcgcagactcgccacctccctcggcgtggcccccggcgcgctgtactggcacatcgaaagcaagcaggagctcatctccaacatggccgcggagatagtccgcccggtgctcgagcacggcgctccaggggaccctgcagagctcagcgcgcttttgcgccggtcgctgttgagcgtgcgcgacggtgcggaagttgcggtcgccgcgatcgggcagccgggcaccgccctgcgggggaaattggtggacgcgttcgcggctgctgtggcggggtgggtaggtgggactaggcgggcgtcggcaagcgagcagctcgccgcagccaacgggctgctgcacctgacccttggtgctgcgtccgtggagcagtctggcgctcagcttgctgcggcgaccgggagcgagacagcggcggagctctcccccgtcgaggcggaggctcaacaccgaaccgctgtgcagctgctcctgcgcggcctgggcgcggttggcgaaggcgtgtagggggtctcgactacgatcagtcggcatgactgaagccactcacgagcagcccgccgcgactcccgcaccggaaacgtggccgggtaccgcctaccccctcggctccacctacgacggcgcaggaaccaacttcgcgttgttctcgaacgccgccgacaaggtcgagctctgcctgatcgacgaggacatgaacgagacccgggtcgagctcgacgaagtggacaactacgtctggcacgcgtacctgccgggtgtcgcccccgggcagcgctacggctaccgcgttcacggcccgtgggacccggccaacggcaagcgctgcgacccgaacaaacttctcgtcgacccgtacgcgcgcgcgttcgacggcgacttcgaccagcactcctcgctgttctcctacgacatccacgccgaggagccgggcaccggccgcaacgaggaggattcgctgggacacaccatgctcagcgtggtgatcaacccgttcttcgactggggtgacgaccgcagcccgaatatcccggacgaggagagcgtgatctacgagtgccacgtcaaaggcatgacgatgacgcacccggacatcccggagaacctccgcggcacctacgccggcatggcgcacccggtgatgatcgactacctgcaggacctcggcgtgacgtccatcgagctgctgcccgtccaccagttcctgcaggacgaccgcctgcgcgacttggggctgcgcaactactggggctacaacaccttcggtttcttcgccccggagaacaactacgcctccaccgaccgccccggcgacgcggtggcggagttcaagcagatggtgcgcgcctaccacgaggcgggcatggaggtcatcctcgatgtggtgtacaaccacacggccgagggcaaccacatgggcccgactattgcgttccgcggcatcgacaacgaggcgtactaccgtctagttgacggcgacaagttccactacatggactacaccggcaccggcaactcgctgaacgtgcgcgaccctcactcgctgcagctgatcatggactcgcttcgttactgggtcaccgagatgcacgtcgacggcttccgcttcgacctcgcctccaccctggcgcgcgagttttccgacgtggaccgtttggcgaccttcttcgatctcgtgcagcaggacccgatcgtctcacaggtcaagctgatcgccgagccgtgggacgtgggcgagaacggttaccaggtgggcaacttcccctcgctgtggagcgagtggaacggcaagtaccgcgacaccatgcgcgacttctggcgcggcgaagcctccaccctcggcgagttcgcgtcccgcctgaccggctcgtcggacctctaccagcacaacggccgccgcccttcgcactcgatcaacttcatcaccgcccacgacgggttcacgctgaacgacctggtgagctacaacgagaagcacaacgaggaaaacggcgaggacaaccgcgacggcgagagccacaaccgctcctggaactgcggtgaggaaggcccgaccgacaacccggagatccagcagctccgcgcgcagcagcgccgcaacttcctgaccaccctgcttttgtcccagggcacgccgatgatcgcccacggcgacgagttcgcgcgcacccagggcggcaacaacaacgtgtactgccaggacaacgagatcgcgtggatgaactgggaccggctggaagaggccgaggatctccacgggttcaccaaacgcctcatcgccatccgaaaagcgcacccggtgttccgccgccggcgcttcctctctggcggcgcgctgggcgaggacgtggtggaccgcgaaatcgcctggctggtgccggacggcaaactgatgacgcaggacgactgggactacgccttcggcaagtcgctgatggtctacctcaacggcgacggcatcaccgagcaggaccgccgcggccgcaaggtcagcgacgactctttcgtgctcatgttcaacgcgcactacgaggccatcgacttcacagccccgccggagcagtacggtgcgagctgggaggtgctgatcgacaccaccgagccgctcggctacccggcggagaagtcggtgctcaaggccggcgacaccaccacggtgcctgcgcgctccacgctggttctgaagcaggtcgagccgccggtacgctagacgctttcaccggattggtatctcaaggagggccagaatgattaccgctaagcgcgcgcggatttctgtcacggcgagtgaagtggtggtgacccccaccgccctggcggcgtcgttgcaggcgagctcctccgacaccctggtggagctggccgctatcacaaacgtcaccgtccaccccggcgacgcgtgggatgaaggccgcgtggagcttgccacggcccgcgggaccgaggtaatcgagttcagccccggcgacagcgacggcccggacgcgttgaaagcgatggtggacaaggcgctgcgcggcgacgccccggacgcggccgcggcggacgggcaggctggtatccccgggttcgacttcgtcgcgttcgacgtggagacggcgaaccagaactggggttccatctgccagatcggcatggtgaagatcgtcgacggcgaggaagtcgaccgcgtgatgtggaagtgctgcccgccgaagggcatcgacgccttcgacccgttcaacgtgggcatccacggcatcacccaggaatcggtggccgattgcccgggcgtgggcgagctcatcgcgtcggttgaagagttcgtcggcgatttgcccctagttgcgcacaacgcccagttcgacgcatccgcgctgcgcgacgcggccgttgcctccggtgttgcggtgccgaagctgatgttcgcctgcaccctggcgcaggcccgtgccaccaagctcgacgtggtgaaccacaaactgccgacgctcgccgagcacttcggcgtggcgctggataaccaccacgacgctggtgcagacgccttcgcgtgcgccggcatcatggtcggtctcgcgcgccaagctgcgtacgaggggtcgctgatgggcttcgtccacgacgcgggtttcgcgctcggttccatcgacgccgaccgcgtcaccccggtgctgcgggaccgttccggtgccatgcgcgcgctgcaggtgcagaaggtgcaaggcggcggcatgtctgctgcggtcgacgcggtctcgcagccgcagggcaacaaccagggcgacggcccatcgcgcggggcggagcaggcttcggataccgctccggccgcgtccgagccggcgagcgggggtaaggcgaagcgcagcgccccgccgtggcaggctgtcgcgaccccggacaccatcccggacccgaacccgaaggctgacccggattccgcgctctacggtgagaacgtcacgttgaccggcgatttcgagccctacgacaagggcgagctatgggcgggtatcgcgcaccacggcggccaggtgggcaagaacgtgacgaagaagaccaccatcctcgtcaccggcgagtgggccactatgacgtccaaggagaaacgcgcccgcgagctgcaggacaagggccaggagatccagatctggaccgcggagcagctgctcgacgccctcggctacgagcggtagggcaaaaagatttttgcttggcgacggaaccgccgccctcccccgcgcgtctaatacacatgacgcacgccctcgcttaccccgtttcgccctttgctccggcgccgtttccgcaccagcagcttcacccccgcctcgctcgccgcgaggagatcaccgcgggcggtgcaaaagcgtggattaccccggggtttagcgcttccacggcgtttatctccttatcgcccgggctggtctgcgtgttcgacgggattgccgcggccggtcacggcgaggccttaacccaccagcagatcggctccctggggctcacggcgcaccaggcgtggaacgcggccgccgagacgctgcgcgctaccgctgtgacggagggagacgtggagttttggtcgcgccccgccaccgttgcgctgggcgacggcgcgccgcccggggtcgagatccgcggcgggacgcacacggcggcggcgtggctcgcccacccgagaacctttgaagtcatccacagacatttctccaccgtgctggcccccacgggcgaacttagctacttctcgcgcgaccagcgggagctgttcattttcgacgcgcaccgcgacgacatcacgcgcgcgttgggcccggttgcgctcatgcgctactcgctgggtttcccgctgctcttgcgctagcgccggcgggcgcggccaatcactatggttgaacacgtctgccgcaacctcaacgcggctgcaagccaagaagaaagttgaaccatgcgccggcccatcacgtccacctaccgcctccagctgcgcggacccaacgctgacccgtccggccgcaagttcgggttcgcagaagctgcagagcaggtgctttatctgcgcgatctcggggtcagccatatctacctctcccccatcttcgccgcggtacgcgagtcgaaccacaactacgacgtgatcgacccgaccgagatcaacccggagctgggaggcatcgaaggtttgcgggagctcgcgcgggtggcgcacgacgcgggcatgggtctcgtgctggacattgtcccgaaccacctcggtgtggagaccccgcgcacgaacgcttggtggtgggatgtgctcaaacacgggcgcgattccgagttcgagccctacttcgacatcgactggcacgaggacaacggcgccggcggcaagctcggtctgcccgtccttgcggttgagggcgacgaggaaaagcttgagctcgtccagctcgggcccgaggagttccccgccggcgccgcccccggcggcgaggtggtgctgaagtacttcgactcttacttcccggtgcgcccgggcaccttcggctcgcttgccgacgaccccgtggaggtctacgccaaacagtcctacaagctgatgtactggcgcgacggcgtgatctcctaccgccgcttcttctctgtcaacgggctcgccggcatccgccaggaggacgaggcagtgttcgagcacagccaccgagccctgcggcagctggtcgacgaagacttgatcgacggcatccgcgtcgaccacccagacggcctcaccgacccgttcggctacctcacccgcctgcgcaaactcatcggccaggaccggtggctagttatcgagaagatcctcgccgtcaacgagccgctggacccgcgcctcaacgtcgacggcaccaccggctacgacgccctgcgagaactcgacggcatcttcatcaaccccgacgccgaggacacgatgtccatgctcgcgttgcagcaatgcggctccacctgggacgaggccgcgattgaggcggcggagcaccagctcaaacgcgacgtcgcacaaaatgagctcggcgccgagctgcagcgcctcgtgcgcgccatgcgccgggacaacttttccaccgcgggccaagacgtgagtgagggcgacctcacagacacgatggtcgagctgttggcctcgatacctgtctaccgcgccgactaccgttctttgtcccgcatcacctcgacggtggttgcggaaatggcgcggaagcagccggcgaggcgcgacgctttggacctcatcgccgcggcaatgctcgccgagggcgaggccaagatgcgctttgcccaggtttgcggcgcggtgatggcgaagggcgtggaagacacgctgttttaccgggcgaaccgcctcgtttcgctgcaggaggtcggcggcgcgccggggcgtttcggtgtcggcgcagccgagttccatctcctccagcaggagcgcgcgcagttgtggccgcacgcgatgacctcgctcacaacgcacgacacgaagcgcaccgaggacacgcgcgcccgcatcggcgagatcgccgaggttgccgacgagtacgctgagctgacccgccagatcttcgccattgttgcgccgccggacacggccaccgggcatttcctgctgcagaacatcgttggtgtgtggcccgccgacggcgaggtgaccgagaccctgcaggagcgcctccacgcctacgcgatcaaggcggtgcgcgaggccggtgtgaacacgacctggttccaccaggaaccggagtacgaggctgcggtgacggactggatcgacgcggtgttgttcggccctgtggctggaccgatcacgcagtttgtggcccgcctgcaccgcggcgcagtgactgtttcgcttggcaggaagctgatgcagatcgccggcgccggtgtccccgacacgtaccagggccaggagtacttcgacctctccctggtcgaccccgataaccgccgatttgtcgattacaccgcccgcgctcagacattggcgcagtaccgcgaacgcgatgtcgaggagaggctcaccggttatctcggtggcgatctcaccggcgcaggcgccagcgtggccaaacagatcgtagttagcgagggcctcaacgcccggcgcgagcaccccgaggtcttcctcgaaggcagccaccaggcggtgttcgctgtcggagaggcgaaggaccatttggtcggcatcgcccgcgccgaccaagcaattgcgctcgccacccgcctgccgctggggttggaagcccgcgggggctggggcgcgacaacggtgcagctgcccgacggcgcgtggcgcgaccggtttagcggccgaaccttttccggcaccgtgaaggtggcggacgtgctcaccgagctaccttgtgctttgctgctgaaaacgagcgagaggtagccggtgggcaaacagaagaaggtttctgacgagacgatctcgcgcctcggctccacctacgcggagtgggtccgtgcaaacgagggcgttgcggcggtgttccgcgacgcgctcaacgagctgatgcgcgacgccggcgtgaacttcgaccgggtcgaagtgcgggtgaaaacgtggccgtcgttaaaagcgaaggcccgcaagctgggggcggacggcgagccgctctaccccgatccgtggaacgacatccgcgacatcatcggcgcgcgcatcacggtgctgcactcgacggagatcccggccgtgcagcggctgctggcggaccagtttgaggtgctgcgcagcgtagacaaggcgcaggagacgcgggtggccggcggattcggctacggctcccaccacctgcaggtgcgcgtcaccgaagaatcggaaggcctcgagcgctacgtcggcaccgtcttcgaggtgcaggtgcgcaccgtgctccagcacgcgtgggcggagtttgagcacgacatccgctacaaacggtccgcgggcgtgcgcctcgatcccgagattgaccgcgccttcaccctcgccgccgggttgattgagttagctgaccagcagtttgaccagatcgcaggcatcgcagggccacagaaggctcacaccgtgggcgccgaggacgctgagatctcaccggagacgctccccggattgctgactatcatgctcggttcgcacttcccgctctcgcgggcgaacgattaccgcttcctcaacgagctgctgcgcacccacggcatcgagcaggtggggcagttgtctgagctcaccaatccagcggacgtcgaggcggtcaagaacgctctcgcccacccgttcgtcccgggccaggtgcgtatcgtggacgacctgctactcaaccgcttcggatcggagcacatcgataaaacctgggacgccggaaaccggccgaaggagcgcagggaacgtctcacgcggcgcctcgccctgctgcgaggcgcctagcgcctaacccccaacaaccactagcgctctcgccccagcaaccggtcggtctggcggcgctccttctttgtcgggcgacccgctccccggtcgcgcttcggcaacgtggcgaagatgtccatcgggggcggcggcggggagatgtcgatgtagcactggcgggcgaccggagcaccgacgcgcctgcgcaccgtagccgtgacctcgaactcgaggtaacggtggtccttccacacgcggacgtgatcgcccgggacaacctgggtcgcggccttcacggtctcctcgttcagcttcacgtggccggcgcgcactgcttcggcggcctggctgcgcgttttaaagatccgcaccgcccacagccatgcgtcgatgcggacggcggaaccatcgggttgggtcataaacggcaggtcttagtactcgtcgacgtggttgacaatcttttgggccttgttccagttcacgtacccgcccacgacggcgacgacgaaaccgaggacaagcaggctccactggccggtcagaagcagcagcaccacgccgccggctacgccgccgccggtccaggcagcggccgcgttcatgtgcttgcgcatggcctgcttgcgctgctcgatggggttgttgggtcgcggctgcattgtcatggggttaattctacccacgtctgccctgctgctttgacggtggcggtgccttgggtgagggaggctaggtgggcgtcgataagcgagcgctcccccggcgcaaagccgagcgtgtagcgcgccagcgagccgtactccacccccaccacctcggtgccggcgttgcgcagctcggcctcgatgcgtcccgcctccgcgtgcggcaggtcgacggtgaccagctccttgaccgcccgagtggtgcgggtgacctgctccagcgcctcggacacggagttcgtgtacgcgctgaccagcccgccggtgccaagcttcaccccgccgaagtagcggatcaccaccgcggcgacgtcgagcatgccggagcctttcagcacctccagcatgggtttgccagcagtgcccgagggctcgccgtcgtccgaggagcgctcgatgggctgcgcgccgtcgacgtggacgatgaacgcggagcagtggtggcgcgcgtccgggtacgcctcgcgcgccttagcaatcagctcacgtgcttcgtcctcggtggctgcgcggttgacccacgtgatgaaccgggagcgtttgatctcgaactcgtgggtcaccagccttgtcgctgggcgttcgtaggaggtacgcatcgtttccaagatagtacggtggcggtatgtctggttttgaggtttgggctccgtacgcacgagacgtgaaagtggtgatcgacggatccgagcaccccatggccgagcgcgggcgcggctggtgggactccgacgaagaaccgcgcgaggggcagcgctacgctttttcgcttttcgacggcacatcatggtccaaacccctccccgacccgcgcacccgcctccaacccgacggcgtgcacggcccctccgaggtcgtgccggcggacttcgagtggaccgacagcgactggtcgggcctgcatctgaaggaccaggtgctctacgagcttcacgtgggtactttcacgcctgagggaaccttcgacggggtgatcagcaagctggactacctcgccgacctgggtgtgaactcgattgagctgctccccgtccagccgttcgccggcgagcgcaactggggatacgacggcgtcgactggttcgccgtgcagcagtcctacggcggcccgcaggggctgaagaagcttgtcgacgcggcccacaaccgcggcatcgccgtcatcatggacgtggtctacaaccacttcggccccgagggcaactacaacccgtgcttcggcccctacatcaccgcgggccacacgagctggggcgacgtagtcaacatctccggcccgggctcagacgaagtgcgcgcttacatcctggacgcggtgcgccagtggctgggcgagttccacgtcgacggtttgcgcctcgacgctgtgcaggcgtacgacgaccgtcgcgcgtactccatcatggaggaaatccgttgggtggcagacgacatcgccgagcgcaccgggatcccccgcaccatcatcggcgagactgaccagaacgacccgcgcattgtcaacgacgaaacccgcggcggctacggtctgtcggcccagtggtgcgacgacctccaccactgcgtgcactcgctgattaccggcgagcgccagggctactacgtggactacggctcgatcgagcagctcgccgccacgctcagcaacgcctaccgcttccgcgacacttggtccgagtaccgccagcgcacccacggccgcccgctggatctagcgcacgtggccccgtggcggatgatcacctacaccaccaaccacgaccagaccggcaaccgcgccgccggcgaccgcccgaccgcaacccacacgccccagcagcttgtgctgcgcgcggcgacgatccttatgtccccgttcaccccgatgctgttcatgggcgaggagttcggcgctgacacgccgttcgcattttttgtctcgcactccgaccccgagctggtgcgcatgacgcgcgagggccgcatgcaggaattctcccgccagggctggaaccaggccgaggtgccggaccccgcggagcagtcgacgttcgactcggcgcgcctcgagtgggatcacaccgcccagcaggcggagatcttggccgcgtacaagcagcttcttgctttccggcgcacccacgcccccgcgcgcgacgatctccgcgaactctccgtcgaacacggcagggccggcgacggcgaaacgagcggcggctggctgctcatgggcgagcgcggcggcgacgtcatcttcgccgcgaacttcagcgccgagcccgccaccgtcccagccggcggcgagctgctctactcgtttacctcgcctgaggtgggtgagaacgagaccgtgctcgacccgtggggcttcgccctgatcaagcagcggtaagtcgacgccgaggcacggccgtctacccggagacgatgtattcgtactccggggtccccggctcgaggcggcggcactcaatcggcgagtccgccatccgctcgagcaacggatcaagatcgctggcgcgcgtgagctccaaaccgaccagcgccgcgccagtttcgcggttgttcttctttaagtactcgaacagcacgatgtcgtcgtccgggcccaagatctctgtgaggaacgtccgcagctgtcccggctcctgcgggaagttcaccaggaagtagtggcgcagaccccggtgcaccagggagcgctccatcacctcggcgtagcgcagcacatcgttgttgccgccggagataatgcacaccacggtcgagcccggctggatcgtcatcgcgttcaggccggtcacggcgagcgcgccggcgggttccgcaatgatgccctcattctggtacagcgccagcatttcggtgcacacagcgccctcgtccacggcaagcaggtgcgtgcggccctggtttcgctcaacgacctcgaacgggaacgccccgatgcgcttcaccgccgcgccgtcgacgaacgggtcgatgtcggtgagcgtcaccggctcaccctgtttcagggcttcgcttaacgacgccgcgcccctcggctccacccccaccacagcagtgcgcggcgacatgtctgcgaagtaggacgtcacacccgcgatcaggccgccgccgccgactggaaccacaatcgtgtccacctcatgccccagtcctgtcagctgcgcgagtacctctgctgcaactgtgccctgcccaatgaccgtgtcgcgggagtcgaacggctcaatcatcttcgcgccgcgggcggaagcgtcctcgcgcgcggcttgcgccgcctcgtcgaaggtgtttccggtgaccacgagctcgatggcgtccccgccgtgcacccggatgcgatcgcgcttctgcttcggcgtcggcttcggcacaaagatcttgccttggatgccaagcgtgcggcacgcgtacgccacaccctgcgcgtggttgccagccgacgccgcgaccacacctttggcccggtcctcgtggctgagccctgagataccgaagtaggcgccgcggatcttgtacgagcgcacgtcttgaagatcttcgcgcttcagataaatattcgccgaatactgctccgacaggcgcgggcagtactgcagcggcgtcggatcaatcaccgacgagatgcgggcctgcgcggcctgaatatcggcggcgtgcacgggctggaacttcgcggaagtcatggtgttacatcctatcccccgccggggcgcgctctgcgttccgtgtgggcgcaggctgatcacgggctgtcatttgcaggcaaacctgctaggtttttacccggtattttccctttccttcgctttcttaggagacctcagatgaagcgcatttctaccgctcttgttgcggccaccgttgccaccggcctcgccctgaccccggccggcgccgagaccgccgcaccgcagccggagaccggagtcaccgccaccaccaacggcgctgccgagggccagcctactggcgaagacaagaccggcaccgacaaggctgatagccagaacccaggcgacaagaaaccttccaagccggcgaagaacagcggttcctccacgggcaagctggtcgccgcagcgactggcatcacctccgcagtgctcaccaccgcgatcatcgtgttctccaacccggccggcatcaacaaggcggtcgacctgctgaacgcgaacttcggcctgggccttcctcacttcaccctgttttaatcacgcgtaaccgagtgcttccgatagccggcccagtggagtagaaactacagttatgaaatctcgtaccgccatcgcgctgctcactgcggcgggcctcggcctgaccggtgtcgcctcggccaacgcggccaacgcggccaacggcagctccagctcgaacggggttgcgtccgccaccgtcaccgcaaccccaaccacgacccccatcgccacgccgacgacaacctacccggtcacggcgacgtccacggtggtgggctctgacggcgtcaccacggtcgtcgagtcggtgacagccgagcccaccaccgtcacctacaccccgccgaagcccacagacgcgagctccaagatgatggagctgagcacgctttctgagcgcggccagaccatcttcatggtcatcaacgccgtgctcactgtcctcggcatcgcgatccaggtggcgacggccgtgctggcgtcgaaccccgagatggtcgaccaactgcgcgcctggctggagagcctagatatttaaccggctccagcagctcagccgcagaagactgaaagcccccgcttccccggccgccgacggcgccggagaagcgggggcttcgcctttcgccttctagccgaacagctcctcggaagcgatgcgggcgccctcaacgagggactcgagcttcgcccaggcaatctggcggttcaggcggccgcccagaccacagtcggaggacgcgatgacgtgctcaggacctgccgcctcagcgaacttcaggatgcggtctgccaccaggcgcgggtgctcgaccgcgttggtgttgtgggaaatcacacccgggtagatgaaggtgttctccggcagctcgcggttctcccacacgcgccactcgtgggcgtggcgcggcgacgcaccctcgaaggagtagccgccgacctcggcgcgcaggatctcgtcgatgatgtcctcgaacggcacatcggtgacgtgcgggccgtgccaagagccccagcaaatgtgcaggcgagtctgctccttcggcaggccttcaagcgcggagttgatcgcgtcgatgcggatgcgcagccatgcgcggtagtcctcgatagacggctcggggttgatctggtcccacgactcggccaggtccggcgcgtcgagctgcacggtgaaaccggcgtcggtgatcgccttgtactcgtgcgccatcgcgtcggcgcacgcctgcaccagctctgcgtcgctgccgtagtgctcgtccttcaggcgcgcggcggagcccggggacagcgcggcgacgaagccgtcggtcgcgccggccttctccatcgcggcacgcatcagctttacgtcggtctccacctggtcctggccgatgtaggtgatcggtccggtgaacttcgggttacccaccttggcgcggccggtgaagatgccggagttggggtcgttgtaggcgtcagcgaacagggcgcggtcgcggcggtccgggaagctcgtcagctggatgttgcccggggtcgagcgcttgacctcctggctcgcccaacggtcctcgtccgtcatggtcaggccgccgaggcgggagaaggagtagttccaccacgcgccgtagtccacggcacccgaggtgatgtggccgtactcgccctcgttgacaatgtcgatgcccatatcgacctggcgcttcaccacctcgtcgacggcggtctcgagaacaccgaaaaattcctcgtcgctgatctcgttgttcgcgcgtcgctcgttcgcctcaagcagagcgtcggtgcgcggcagggagccgacgtgtgtggtgcggatcttctgggttgccatgtgggcattcactccaatgcgtatgtaggtgatacgtccaacacaaagggtacgcccccgctccgccagcgaaacctccggctacccgagaatgccgggccccattgaggctttgaggtcgcccatcaggttggcggagcggtcaacgcgcaggtggtcgccgagcaccagcagctggctctgatccccgttgacgaggttcaagtagacgtccgtgtcgccggggttgttcactaggacgcctttgagtttggcaatgttgtcgatggtgcactggtcggtgcgcatcgtcagcctcagcggcaagccggcgccgttgccgggtccgagttctggcaccttcacgtcgtcgccgaacaggctcatccgttcgtcccgaatcgagatgtgcgccttgaccaagatgatattgtcctcgacgatctgcggagcaacgagggcgtagaccttgttgaacagcagcacctcgacctgcgcgccgtggtggtcctcgagtgtcacgatcgcccagggcgagccgtccttcttggagaagcggcggtccaccgacgagatcaacccgccaatggtcacctccgcaccgtggcgcagctcgcctccgaggatggtggtcagctccgtgtccgtttgggcgtcgatggcctcctcgaacccgtcgagcgggtgcccagaaacgtagagaccgagcatctcccgctcgagcgcgaggcggtgcttgcgctcccactcgtcgtccggcacctcgatcgcgaacgccgcggccgccgcctcgtcctccccgccgagcgcagcgaagaggtcgaactgccccttgtcggcggccttttttgtggaaagcactgagtcgaccgcgtcctcctgaatcagcatgagccccttgcgcgggtggcccagcgagtcgaacgcgccagccttgatcaaggattcggtgatgcgcttgttgcacgccacaaggtcaatcttgtccaggtagtccgagaagctggtgaaattgcccttggtgcgccgtgtttccttgatcgattccaccacctccacaccgacgttgcggatcgcggcgaggccgtagcggacgtcctcgcccacagcgatgaagttctcctccgactcgttaatgtccggctgcagcacggacacacccatgtggcggcagtcggcgaggtagatagccgacttgtcctttttgtcgcccaccgaggtcagaagcgcggccatgtactcggcggtgtagttcgccttcatgtacgcggtccagtacgacacgagcgcgtagcccgcggcatgcgacttgttgaacgcgtaggaggcgaacggctcgatcgtgccccacagcgcgtcgactgctgacttggagtagccgttggcgaacatgcccgccgagaacgtctcgtactccttggccagcacctcgggcttcttcttacccatggctttgcggaagccgtccgcttggcctgctgagtagttggccaccttctgggagatgttcatgatctgctcttggtagacaatcagaccgtatgtctcgtccaggatctccttgagcggttcttcgagctccgggtggatcggggtgattggcttgcgcccgtttttgcggtcagcgtagtcccagtgcgcgttcacacccatcggaccggggcggtagagcgcgagcgacgcgacaatgtcgttgaacccggtcggcttcatgcgcttcagcagctcttgcatgccgccggagtccagctggaacacacccagggtgtcgccgcgtccgagcagctcgtacacagccgggtcgtcggtctccaacccctcgaggtcgatggtttccccgcggttcttctccacgttctccagcgcgtcgccgagcaccgtgaggtttcgcaggcccagaaagtccattttcaacagcccgatggcctcgcatgccgggtagtcccagccggtgatcagcgcgccgtcggcgggccgtttccacatcgggatgtggtccatcagtggcaccgacgccataatcacggcgcaggcgtgcacacctgcttgacgcaccacaccctcgagaccccgggccgtctcgtagatcttggccacatccgggtcggtctcgatcagcgatcgcacttccgcagcctcggcgtagcgggcgtgcccagggtcggtgatgccggccagcgggatgtccttcgccatgatggcgggcggcagggccgcgttgatgcggtccgccatctggaagccgggctggccgaagttcaccttcgccgagtccttgatcgcctgtttcgtcttcaccgtgccgaaggtgatcacctgggcgatcttgtcctcgccccagcgctgggcggcgtaggtgatcatctcgccgcggcggcggtcgtcgaagtcgatatcgatatcgggggcggacgggcgctccgggttcaggaatcgctcgaagagcaggccgtgttccatcgggtcgatgttggtgatcgtcagcgcgtacgccacgagcgagccggcggctgagccgcggccgggtccgacgcggatgccgatctcgcgcgcatgcttaatcagctccgcgacgatcaggaagtacgacgggtagcccttcatgtcgatgacctcgacctcgtagcgcgcgcgctcgaggtactcttccggcacttctgccccgtcgaaccggtcgctcaagccccgcaggacttcctccatcaaccacgaggtcggtgtgtgcccctccggcacatcggcgatcggcatacggtcgtgcgggtgctcctcccacagctccccgtaatcgccgacgcgctcggcgatccacagcgtgttatcgcacccgtccggcacagtggaatcccacagctcgcgcatctgctcggccgacttgatgtagtaccccgtgccgtcgaatttgaaccggtcagggtcaagcagggtcttaccggtctgcacgcacagcatcgcctcgtgcgacggcgcctgcgactcgaggacgtagtggcagtcgttagtcaccagcggcggcagatccagcgcctggccgatccgcagcagatcgtcgcgcacccggcgctcgatgtgcagaccgtggtccatcaactccaggaagtagttgtcgcggccgtagatgtcctgccacattgccgcggcctccagcgccgcgtcgtactgtccgaggcgcaggcgcgtctgcacgtcgcccgacgggcaccccgtcgtcgcgatgatgccgtccgcgtgctcggcgatgagttccgcgtccatgcgcggccacttgcccagctggccctcgtatgacgcgagcgacgacagcttgaacaggttgcgcagccccgtcgcattctccgccaacatggtctggtgcagataggcgccggaggctgacacgtcgtctgacttctggtccggtgttccccacagctggcgtttcttgtcgaagcgcgatcccggcgccatgtacgcctcgatgccgataatcggcttgatcccggcgtccaccatgcggcggtagaacgcgttggagccgaacatgttgccgtggtctgtcatgcctacggccggcatcccttggcgcgccacttcctcggccagcaagtccaccttggccatgccgtcgagcatggagaactccgtgtggttatgcaggtgcacgaacgaggaatgcttggccatgccgatcatcatatccgcggccgcaactcgaattacaagtgtgaagctcgcccggcctactcgtagcgcagcgcgtccacaggctgcatcttcgccgcccgcgacgcggggtaagcgccgaaaaacacgcctgtggccagggagaacagcaacgcaaacagcacggcgctgagcggcggccacgtgaacgcgtcgaaggctgcggtgccgatcatgccggcgatgccgcccagaatcacgccgatcacgccgccgagcaggcagaccatcatcgcctcgacaataaactgcacacggatatcagcctgcgtcgcgccaagggccttacgcacgccgatctcgcgggtgcgctcggtaacggtgatcagcatgatgttcatcacgccaatgccgccgaccagcagcgaaatgccgccaatcgcggacagcacactcgacatgattcggaacacgccggtcagctgttcaagggacgacgacaggtcgagcacctcggcgacgaactcgtcgttgcccgcgtagagccggtcgaggtacttctgcaagtcggcttggaacactgcggagtcctcgtcgggggctgattgcacgctaaacgacgacacccagttcgactcctgccccaacctatccatcgacgtggacgggacgtagatctcggcgaaggattgcaggccgcccagcgcgccgcccgcgttgtgcggttccaacacgccaacgacggtgtagacggcaggagtgccgcctacggtgacgtcgaaacgctgcccgagcgccttggccggatccgaatcgaagagcgcctcgacgaactccggagacacgaccgcgacggggcgctcgccgtccatgtctgcctgcgtgatcccgcgcccgtactgcacgttcaacccgcgcatatcgagtgagccagcaagcaccgcgttcacgctggtgcttgcggtggtgtcgccgcgggtgacctcgccctcgccgctgttatcaatgtcgacggcgcggacccggcctccgaagtgctcctgcagctcgcgcaagtcgtcgagcgtcatgccgtcttcctcgtcggtcggcggcatgtatgaaaacgccgcgaacgggtcgtccgattccgcttcctcgtccggccgctcgtggatcatcacggggtgggttgtggtgcccacaccttcaaggcctttgagcacctggttttccaggccccggccgagggtcatgatgacgatcacggccatgatgccgatgatgatgccgagcagggtcaacagggagcgcagcttgttggtgttcaggctcgacgcggcgagcctgattgattcgctgatgttcacggtgtgcggacccccgcgatgcggccatccatgatttcgacgatgcgctgggtttcctcggccagttccgggttgtgtgtaatgaacacgatggccttgcccatctcctcatgcagctggtggaacaggtccatgacaaggcggcccgtcttggagtcgagggcgccggtcggctcgtcggcgagcagcaggtcagggtcgttcgccaaggcgcgcgcgatggcgacacgctgcttctggccgccggacagctcgttcgggttgtggtggatgcggtcccccatccccatcatgcccagcagctcctcggcgcgggcctcccgggctttcttgtcgacgcccgcgtacatcatcggcatcgccacattctgcagcgcgtccatgcgcccgatgaggttgaagttctggaagatgaagccgatgttgcggctgcggtagccggcaagctcgcggtcggtcttggcgtagaccggttccccgttgaacgcgtaggcgccctcggtgggccggtccagcatgccgatgatgttcatcagcgtcgacttgccgccgccggaggggccgacgatggacacgaactcgttgtggtcggcgtagaagtccacgccgtggagcaccgtcagctcgctgggttcgccgaggttgtacgtcttgaccacgttgcggatgtcaatcaggcgcccggaatcagcgaggcccgcaggctccgcgggagctggttgcttgacgacgggctcttcaacctgcggctgctcatccgtcgcgggctcggcgccgaagaaaaacgggtcgtcgttaagctgttgtgcctctgcctccggctcggcggcgtgcttgccgcggcggaagcgcgaaaacggggtactcacgacgccggagcctcttccggggcctcctcaggggcgtgggttcgcgtactggtcacggtcaccgtggcggtggtgcggcccttttcttccttctcgccgccctcgcgggccgcgacgacatcctcggggtcgaagccggagtcggtgatcttcactgtctcgccgatgcggtcggtgtactcctccggccagttcacaacgatgtcgccggcctgcaggtcgccgccggtaatcgcgatgtccacgtcgttggacgcgccggtttccacggtgcgctcctcgatgcgcccggagcgagcaccgtcgccatcggtggcgaggacgaggactttcttcgcaccctcgttgtcgtacacggcgtccaacggcacgttgagcgcgtcgtcctcctgctgcgtgatgatctcggcgcgcacgctgccgccgagcagcaggccctccgtgtcgccggtgacctcgatttcaaccgggaacacaacgctggatgcgtcgccgccgccttggagggcagcctgcgggtcagttggctgcgccgcggccggcgagatacgaaccacgcggccggtgtactccttcttccccgtcgccgtggacgtgaacgtcaccttgttgcccttggcgatgctgggcacgtccgcctcgcgcacgtcggcgcggatgagcaggctggaatcgtcggcaaggctgagcacgcggccctggggaatgtcgccctcctggacgtcgacgctggtgacaatgccgttgatcggcgagtagatcgtcgcctcctgcacctggtactccagggtgccgtcggacgaatcgagcttggcggcctcagcggagcgccacgcagaatccacctgcgcctgcagctggctgcgctcctgcgcgacctgcgcctgcgccgccgcgaggttcgccttcgcgtcctgcagcgcggcgtacgcctcgtcgacgctcacacccgcgccagccccggcaccggtcagctgcgcgatgtcggcttcgctcacgccgggcgcggccgggttcgcgggttgcgccgggttgggggccgggttggctggtgccggcgcggccgggtccgcgggctgcgccgggttcgccggctggaacgggttcgcgggcagttgcggctcgttgtagccgcccaccacactgtggaccttggaagagatttggccagccatctcgttggccacgcgcaccgcgcgggcgccgccgttcgcggccaccgcggcgttgtaggccgcctgcgcctggttcacctgggactgcgcggagcggatcgtcgggtgggtgccgttgttgaccatctcgttgagcgaattcagctgggcctgggcctgctcaacgcccgccatggcctccgcctgcgcgttcgcctgctgctgctcttggacggcgagctggcgctcgagctggtcggtgtccatcgcggcgaggagctgctcgacctgcacccggtcgcccggcgccacagcgaccgtgcgcacctcggattgcagcggcgtggtgatcgacacggcgcgcaccggggcgatcttgccgttgaccaccacactgctggacaccccgtcggcgttcacgatggtgtagtcgcccggagcgaggccgtcgccgtcggcgttgtctccgccgccgagcccgccggcgctgcacgatgcggcgaagaggctggcggcgacgatgacggcggcggcggtgcgcttgggatcgcggcgcttgaccaaggtgattcctccatgaacgggtgcgttgaactcacggtgactatacaccgcgggcagggtgatccccctgccaagcggtgacggcgaaggacccccacgaggcgtcggcgggcagcacctcgacagcggcgactgcatcgtctgcggcgatggcgcgcagggtttcagcctggtcgtggacaacggcggcggcgattctctgcggatccacctccacgccgtttgcgcgcgcccgcgccgccagccgctcgagctcgcgcgcgaagacgtcggcgcgggtcgtggttgaggttggttcgggggtgggttggaggggggcgtcgataagcagcagcccgttgaccctgcctgcgggagccaccgcacgcgcagcttctgccggggtgagcgggtgggtgaagctcaccagcgcgaacgcggcaccggagctcatgcttaacgacgccgcgcttctctccccgtactccccccacgtttccccgcgctgcgggcccagcgtgtcgccctggatagcgggcggggcggccggcgtagcgagcccgacggcgtagacaccggcgcaggcgaccgccagcccaaccacccccgcgagcgcgtgcgtgcgacgcatgtcacatctgccgaatcgtgtcgagcgcgtgctccagatccgccgggtacggggaatgcacctccatgtagtcgccggtgcgcgggtgcgtgaatcccagcgaggtggcgtgcagccactggcggttgagcttgagagccttggccaggtttgggtcgcagccgtacattgggtcgcccacgcacgggtgaccgagcgccgacatgtgcacgcggatctggtgggtgcggccggtttctaggtggacgtccagcaggctcgcgtggcggaaggcttccatcacctcgtagtgggtgacgctggcgcgtccgtcctcagtcaccgcgaacttccaccccgacgacgggtggcgcccaatcggcgcgtcgatggtgcccacgatgggatccggcagcccctgcaccagcgcgtggtaggtcttgtccacggtgcgctccttgaacgcgcgtttgagcaccgagtacccggggatgctcgcggcgacgaccatcacgccggaggtgccgacatccaaacgctgaacgatgcctttgcgttcgggcgggccggcgtcgggaagcgtgaagcccatcgcctttagacccccgaccaccgtcggaccgtcccaacccagggtggggtgtgcagccacgccgaccggcttgtccacggcgatgacgtcgtcatcttggtagaggatggtcaacccgtcgacgatttcggcgaccggctccggcgccttcttcggctcgggcagggtcgcctcgagcatcgcgccggcggtgacgcggtgggatttggggactggggtggcgtcgataagcacatcgcccgattccaccatctctgcggccgtggctcgggagacgccgaagagcttggccagcgcggcgtcgacgcgcatgcctgcaagcccctcgggtaccggcagcgagcggaacttgccgctcattgcttcgcctccgcgggggtttcgtggtccgggtggaggagcatggacgcgatgaagaccacaacgcccacggtgatgcaggcgtcggcgatgttgaacacggcgaagttgcccacggagatgtagtccaccacgtggccgaaccaaaagccgggatcgcggaacagccggtcgcacaggttacccagcgcaccgcccgcgatgagcgcaatgcctacaagttcccaccggttagcgatccgtggcgcgtagatcagtgcgccaaccacgaacgcgagttggaacgcggtgaacaaccaagtcatgttctggcccatggaaaacgccgcgcccgggttgaacaggaggtagaagcggaaccagtccccgatcaccggctgcggctggcccggctcgagccacgacagcatgagctgcttcacaccctggtcaaccgccgccaccaacaccatgatcgcggcaaccgctttcaggtaaccgcgcccgtccatctccttcatcaccgcaacatgctagtcgctgtggtctgggggtgtgtgaggcgtggggtaggttcgaggagtgcacgaaacgtctgctggttatcgttctttcccctcccggcgcgcgggccgttcgtttgctgcggtcgcggcggcggcgctggcgctcggcttaagcgcctgcgcgggtgagccagacccgctggagggcatcccctcattcccggtggatgccgcgcgcgtgcgggtggttgaggcgggcgaggatccgcaggtgctcgcctaccgcgatgagggttctggttcgggctcgggttccggtggtgaggcctgggagaccggcgtcgaggtcgccgggggcattgcccagtcggtggccgacggggccgaggatgtcgaccctattgccccggctggcggcgacgttatgaccaccaccctgcctctaactgtggttgttgacgccgccggcgaaccgggcgaaggtgaaggggtggcggcccgcgcagtctcgctgactacccgcggcggcgagcactccgagctacagctggggctcgaggtcgcggacaacgaaggcttcatcatgcgctggcgggcggcggattcgggccaggtgcagacggtcaagatgttgccgccggtggactctccggaggccggccgcgaggtggtcgagcgctccctgctgcagctgatgtcgaccgtggtggtcttcccgtccgagccggtcggcgtcggcggatcttggaccgtggagtcgcgcgtgaccggcgacgccaccatgctgcgcacaaccacctacacggttgcttcgatggacggcgatgtggtggagctcgacgtggatgttgaggaacggcccacgcaggcgtcgctgcgcatcgacaactcggccgcgggcgagctcgacggccagagcctgaacgttgcgtccacctccaccacttcggacggccgcctcaccgtggatttgacgaagccgctgcccaccgcagggcgtgtagcggccacgacccgcctcgtctacgaaggcgatgcggcgaagttcagcgtggtgcaggacgtgacctccgccgtcacgttcggaaaggagtagccccgtggtcgcaccgctgcacatcgggctcgacggcatctcgttttcctaccccggcggcaaccgggtgctcaccgacatctcatttgcggtgccgtcgggctcggtcacaggcttgatcggcgaaaacggcgccggcaaatccacgctgttgggcgtcatctcgggcgagctcacccccgacgccgggcggctgatcaccccggaggtcaccggcttcatcgcgcaggaaacctcactgccgtttagcgagccggcgcaggtgcttgtcgacgcagccgtttccgaactccgcgccatcgaagagaccatcgccaccgtctccgaacgcatggcggaagaacccgacaacgtggcgctcgcgaataccttcgaccgcgcgctcgcccgcgcagagaattccggggtgtgggagctcgacgcccgcatcagcaccgtgctcgcgggccttggtctagccaacgtgccgcttaccacccgcctcggcgacatgtcgggcggccaacgccgccgctttgcgctcgccacgctgtttttgcgccccgtggacgcgatggtgctggatgagccgaccaaccacctcgacgacgaagccgtcgacttcctcatcagcgaggtggagtcgttcaaaggcccggtgctggccgcctcccacgaccgttacttcctcgacaccgcctgcgacagcatcgttgacctcgacccgggcctcggccccgagggcggctacggggaggagacccggcaagggtcgcggttcagcggcgccttctccgactacctcgccgcccgcgaggcgcgccggcgacgctgggaaaccgacttcgccgcccaagagcacgagcgggctcggttggagaaggccgcggcggtgggcgaggcggacgtcttccactcccacgagaacaagactgagactcgagcagcggcgaagttctacgccgaccgcgccgccaagaccgtcggtgctaggcgccgcggggcggagcagcgcctggatgccctcgagcgcgccgccatcccagccccgccagagcgcttgcggttcagcgggctgccgccgcacgtcaccacctcaatcggtgtgcccgcggtcacggcgcgcaacttgcgcgttactgacaggctgcagccgctctcgatcaaggtgcagcctggtcagcagctgttggtggaggggccgaacggctccgggaaatcaacgcttctgaaaatcatcgacggggagctgaccggatacgagggcgagctcatcatcccggaggagctcagcgttgcccgcctcgcccaagacgacgattggcgcgatctggctcgcactgcggaggaggtctttgcggagcggactcccgctggcgcgcccacgctctctgagatgggactgctttcaaaagagcaggtagcgaagccgctcagcgacctctcgctggggcagcgccggcgcgtctccctcggcatcatcctcgccgctcccccggacctgctgctgctcgacgagcccacaaaccacctctcgctcgccctcgccgaggagctcgagcaagcactgaccgatttcgccggcacggtgatcatcaccagccacgaccgttggatcaggcgccagtggcgccgccgcatccagcagggcgacacccgcgctcgcgtggtgaccctcgccaccttgtggacgaacgaggtgtggcgcgagggcgagatctagggctttcgcctcgttacaggcccggtgccggctggtagttctcggccggggcctcaactggcgcgtccgccggcggctgcgccgggtcgaccggggccggggcgaccggcgcgttcgccgtgcacatctgcggtacctgctccggcggcagcgtggacgagaccaggttgcaggcccactgctgggacagcttccactggccgtcctcaaagacaaaggtgacgtcgttaatcagcgtcggctcggtgtccggcgcggtgaggttcacggacgcgagcacctggttcggctcgaagtccggcagcaccggcttgaccacctggaagttcgcgccggactcggcctgggactgcgacatgacgtcgaacagctccggcaccgtttcgccgccctggacggtgtgcatgcgctcctcgatcggcaggttcgggtccgcggcgcgctgcagcacctcgttgagttcctcggcggtgggcagctgcgcggcgggagcggcctgcgtctcgacgggggctgcggaggtagcggcggtggtctcctccaccgcagcgtcttcgtttccgcatcccgcaaggccgagggcgaggccgagcgagacggaggcggcgacaatcttggatgcgttcatacatgtcagcgtacccatgaaccatctggcactctaatcacatgcgcaacgaagtcatcgtcgtaggcaccggcggcacgatcgcctcaaccacgaattcccagggcgcgcgggtgccaacactcaccaccgccgagcttgtcgcccgctgcggcaccggcgtcggcgtgcgagcggtggacgcggccagcctcgactcctcctcgatgacgctcgccgacatcgacgcactcgcttcgctcgtggagcagctgcttgattgcgcccccgccatcaccatcacccacggcaccgactccctggccgaaaccgccctcgccctcgaccttatgcacgcgtcagcgaaacccgtcgtgctgaccggagcccagctgcctgccgaccacgaccgcgccgacggccccggcaacctccgcggtgcaatcgaggcagctgccgacccagccaactcctcccagggagtcttagtccacttcggcgggaaaacattgcccgcccgcgggttgtacaagtcttccacaacctccttgactcccttcggcctcaccaccggtgagccctcgccgcgccccgcgcccgtgccccgcgcgcccctggccggtgtcaacgtccccatcctccgcgcgtggcccggcgcggacggcgctttggtggattacgtggcgtcaacggggcccgacggcattgtggtggaggcgctcggctcgggcaacgtctcggatcggatgggtggggctttgcggcgcgcggtcgacgctgggatcccggtcgtggtagccacttctgtcccggacggaggcgtcgagttcgcgtacggcggcgcgggcggcggtgccaccctcggtgccgctggcgctatcgcgtcaggggcactgtctccggggcaggcgcgcatcgcgctcgccaccgccatcgcgacgggaacggacccgtcccacttcttttaagcgcgcccctacagccgcctcgccctatcagaagggtgggcatggatcttgtcctggtggtgggtcggtgttggtcgcgcgccgttgcttgagccggttggcagcagattccgtggcaccggtggaggtattgaactctagcgcggcgccggggcttcgtcttaaacccatccgcccggtttcggggtcgggttctatgtgtgatgtgttgtgtttgtggtcccagaagtcgttgttgtgccggtggtggtgcctgcacaacccggccaggttgccgatgtcggtgttgccgccgcggagccagctcaccacgtggtgggcctcgcactcggtcagcggcgcgttgcagccggcccacgcgcacaccccctgcagcgcgagcagggtgatgcgctggtcaatcgacgcgatacgtgccccgcgacccaagtgcagcgggcgggtacacatctcatcgacggtgaggatgtagtccggcgtgccgccaagacccaggcgcaccaagtcgatcgggccgagctcgaccccggtgttggtctggaagaggctgtcggcgtccgcgtcggctaggtcgtccacggtaacggtcacgaccacggatgcgcagccgtcgtcgctcgggtgcttctcgcagtgctcgacgtgcttcagaaggcgcatcagctggtcgtaccggcgctgggcaggggtgcggtattcctccacgccttccggcaggttcatgttcggcgccatgcccttatccaaaagcgcctttacaagcgccatcccgtcgggcgtgagcactgcatggaagtcgtagttaccgtcagagcggcgcttgccttcgtgcacggcgcggtgctccatgcccgcattggggttcttacggcgcaccttcctgttttcgatgtcgacccatttgcgcacgaggcgtcgcaaatccttgacgtcgcggtccggtgcttccttcatggctgctgcgaggaggcgggggcgctgggaagcggcggcgtcgacaagcctgtccagctcctgtcggatggcttcctgctttgcagtattgacggcggcggcatgtttgcgggcggcttcctgatccctacgtgcctgctcccgcgcggcagcagcatcggcagcagcggcagcatcagcgccagtatcaaacagtccctcctcaccaccggcgccgtcagaaccggaatccgggcccggagcggggttatccacgggcggctcgccgaacaggtcgcgtccgcgcgcgaggcggtcgaaagcctcgcgcggggtgcagcccaggtgctgcttcaagtaggtgctggcgtgcggggagccggcgaggcggccggcgtcgtcgcggtcgcagatgtgggcgaacgaggcgtcgatcagcgctttggcttcgatgaaaccttcgagcttttccatcgactcgtgcacgtccataaacgccacgttctcaggggtggtgaacatgtcgcggatttgcagcatggcgtggccgatcgtgtcgacaagcttggccagttccgcggtcatgatccctccttttcgatccccatcgaacgtttgagccaaactatagaaaccgcacccaacacgcccggaccaaaacaaggccaaaaccagaccggccaggcccgaaagcaccccactaagaacaaaaccccaggtcaacgcctcacaaaaagtggcgcaaatcacacttaaggtacgatcttaacaccctaaccagtcgtcccacgcgagggaatccagggggtcggcgggggtgagcaacgggtcgtcgctacgcaagctcttgatgcgccccggccctgtcgcgcgcgtctcaaaacgcacggtgacccagcccttgcccgcgccctgcacccagccgtggccatagtcggggtgaaacacgtcctgggtcgcctgccactgccccgcctgcggggcggcctccgccaccacctcgaccggcgggccacccgcgtggtcgctcacccccgattcgtactcggaactgatccgcggcggctttacaatcgcctggtccagctccggaaacagcacgtcctgcagcgactcctccaaaccggaataactcacacccaccagccggatcgggcccacctcctccgggtagcgaaccagcttgaaggcggtggccaccagcgtgtccaggtcgtcggtggcgtagggcagcgttgctgagcgcgactcgatgtggaagtcggccatctttaacttgacggttacggtgcgggcgccgcggccgtcggcaagcagcctgcgatgcgaatcccctgccgcccggcgcagcgccgcgtcgacctcctcgggcgtgatcaggtccgtcgggtaggtgtgctcggaggagacctgtttcgactcggcgcgcggcgccaccggccggtcgtcgatgccgcgggcgagctgccacaactgcttgcccaccaccccgccgagggcgatctcgacctccttctcgctcagcgccgcgagatcgccaatggtcgcaattcccgccgccgacaactttgcgccggtcacggggccaacaccccagagctcgctgaccggcagcgggtgcaagatctccagctgctcgtcgtgcgggatgacgaacacgccgtccggtttcgcgaggccggagccgatcttggcgtactgcttgccgctgcctgccccgatcgagctcggcagcccagtctcctttttgatctcggcgcgcagttcgttggcgaaggcggtgatggtgtttacggtggcgtcggcaagcgaagcatgctccaaaaacgcctcgtcgatcgacagctgctccaccacgtcggcgtggcgggcgatgatctcgaacacccggcgcgacgccgccgaatacaccgggcgccttggagcgaccagcaccgcctgcgggccaaccaagcgcgccgccctgtgcgtcggcattgcggaacgcgcgccgtacttccgcgcctcgtagctcgcgccggccaccaccccgcggccggatacccccgccaccaggaccgggcggcccttcagcgtgggccgggtgagctgctcacaggaggcgtagaacgcatccatgtcaatgtgcagcacccagcgaggcatgccccatacgctaccttgggccccatggatcccattctcgcgctggcagacattcaccttggacgcaaacagcacggcgacaagaaagtcgggcccggcatcgactgggccctcgcagcgctcgagcgcggcgcggacgccggcgcggggcacatgatcatgctcggcgacatcatcgaccgcaaacgcttcaccgacgccacctacgacgaggtggaccgcttcttcacccgcgggctcgagctgttcgacacggtcctgttcaccgccggcaaccacgacacccaccacacgctggatctaccggcgggtgtcactcacgcgagcaccaccccggccacctacaacctcggccactgggcggtgcacaccgcggccgtcgaggtggacaaggacccccggaagctcgtgcctgcgttccccgccgcggtggacagccgccccaacctgggcgtgctccacacctccgtcaccggcgagtggtccaacaacccctgcctgccgtgcaccgtgaacgagctggatgcccgaggctacggcgcgtggctgctcggccacgtccaccagccggtcacgctgcgccactcgccccacatcggctgggtaggcatgggccgggcgctcatcgccaccagcaccggtgcgtcggtgcaggtggcagagctggagctggcttgacgacgcccccctaaaccccgcttacgcgttcttcgccaccgtggcgcgcacgccctccaccacgtcgacagcgccgtctacagcacccgcctcacctgcgggcaccacggcgaagtcggtcgccagcacctcgccggcgatgtgaccggcgtggcgctcggcccactcaactcgctccgccggcaccacgaggcgcaccgcgatgcggtcggagacctcgaagcccgcctgcttgcgggcgtcctgcaggccgcggatgacgtccgcggcccagccctcggcctccagctcctcggtgacgttggtgtccagcaccacgagaccgaccacgccgtctgcctctacgcgggcggtggaatccgggttctcggccaccaggcgctcggtgtagagatccggcgtgagcacgatgtcgccgtcgacgaccacgttgtcaccgtcgtggacgtagttgccggccttaacgttcttgatcgcgcgctgcacgtccttgcccagtgtcgggcccgcaaccttcgcgttcaccacgacctcgaagctgcccgcggagtccacgtcgctggtcagcacgaggtccttgacgttgacctcatcgcggatgaccggagcgaactcctcgagcgcctcagcgttcggcatcgcaacggtcaaagacggcagcggcaggcggttgcgcagcttgcgcgccttgcggattgacgacgccgcggagcacaccccgcgggtagcgtccatcgtcgccaccagcgaatcatccgacggcagttcgtccgcgcgcgggaagtccgtcaggtgcacggagcgctcaccggtgagccctcgccagatcacctcggtgatgtacggcagaagcggcgccgccgcgcggcaggtgatctccagaaccgtgtacagggtgttgaacgcctccgggtgcgcctcctggccctcccagaaacggtcgcgggagcggcgcacgtaccagttcgtcaacgtgtcggcgaagcggcgcagctcatcgcaggcgtcagcgatgcgggtgtcgtcaagcgcggcaccgacctcggcgaccatgtcgtgcgtcttggccaggatgtagcggtcgagcacgtcggtggaatccaccgaccacaccgcatcttcagacgagtagagctgcaggaacgtgtacgcgttccagatcggcaggatcgcctggcgcacgccctctcggatgccctgctcggtcacgatcaggttgccgccgcgcaggatcggcgaggacatcaggaaccagcgcatcgcgtcggagccgtcgcggtcgaagacctcgttcacgttcgggtagttacccttcgacttcgacatcttcagcccgtcgctgccgaggacaatgccgtgcgcgacgaccttcttgaaggcgacgcggtcgaacaacgcggtggagagcacgtgctgcacgtagaaccagccgcgcgactggcccgagtactccacgatgaagtccgccggctggcgggcgtcgtgttcctcaacgttttcaaacgggtagtggtactgcgcgaacggcattgagccggactcgaaccagcagtccagcacgtccggcacgcgtcgcatggtcgacttgcccgtcgggtcgtccgggttggggcgcgtcagttcgtcgatgtgcgggcggtgtagcgacaccgggcgcacgccgaagtcgcgctccagctcgtcgagggagccgtagacgtccacgcgcgggtactccgggttgtcggagacccacgccggcaccggcgaaccccagtagcgggtgcgcgagatgttccagtcgcgcgcaccctcgagccacttgccaaactggccgtcgcgcatgtgggacgggatccagtcgatctcctggttcagctcgaccatgcggtcgcggatgtcggtgaccttcacaaaccacgccggcagcgccatgtagatcagcggctcgccggagcgccacgagtgcgggtaggagtggacgatgaccttgtcctgcaccacgcgcccgcgcgccttcaggtcgcggatgatgtcgcggttggcgtcgaagaccagcttgccctggtagtccggcacttgcgcggtgaacttgccgtccgcgtcgaccgggatgaccaggccgataccgtacttctcgcaggtgaacatatcgtcctcaccgaaggcaggggcctggtgcaccacgccggtaccgtcttcggcggtgacatagtccgcgttcaggatcatgaacgcgttctcggtgtcgcggaaatagtcgaagaccggctcgtactccaagccttccagctgcgcgccggtaaacgtcgccacaacctccggcgattcgcccagctccttcgcgtacgcgccgatcagctgcgatgcaaggagcagttgcttgccgacgaggccctcaaccccatcctcgcccaccttcaccagcgcgtactccatctctgggtgaacggccagcgccaagttcgacggcagggtccacggtgtggtggtccaggcgatagcggcagcgtcgtgcagctccgggtgctcggcccacgctgcttccgcggcgaagccggcgcgcgcaccggtcaacggcattgtcaccgtcaccgtcgggtcttggcgctcgcggtaggaatcgtccaggcgggtctcctggttcgacagcggggtgtgctccgcccacgagtacggcaaaacgcggaagccctggtagatcaggcccttgtcgtagagggtcttgaacgcccacataacggactccatgtactccgggtccatcgtcttgtagccgttttcaaaatccacccagcgggcctggcgggtgacgtagtcctcccactcgtccgcgtagtgcatgaccgagcttgcgcagtactcgttgaacttctccaggcccatgtcctcgatctgggccttgtcggtgatgccgagctgcttctccgcctccagctctgccggcaagccgtggcagtcccagccgaacacacgcggcacgtggtagccggcctgtgtgcggtagcgcgggacgatatccttgacgtagccggtgagaaggtgaccgtagtgtggcaagccgttggcgaacggcgggccgtcgttgaacacgtactcttgggcaccctgccggttctgaagcgatgccttgaacgtttcgtcttcgttccaatacgccagcacgtgttgttccatatccgggaacttgctgctgccgccggtcatgtcgaccttggggtacacgccgcctaccatgaaatctcctccacatatccagtgcagggacgcggctttcagccccgcggtaccaccctgcttgagccccgtagaggaaccccgcttcattgtggaggaagtgacgtcttccatgaacgtccggttctaatgagcccgcgtgcgcggaaccgttcttccggaacactccccggtgatggccggatcaacgcgtgtaagcgctaactatagcgcattgaacacgcgaaaactccaccggccagatttcatccggcaggtggagttcgcagtaggaccttcgaaagcctacttctcagcgttcggcgcgaaggagtcgcgggactccaactcctccagctgggaggtcagcatcgtcttcaggcgggtgcggtactcgcgctcgaaggtgcgcagctcggcgatgcgggattcgagagcggtctgctgctgcttcaccgtgttcatgatctcggtgtgcttgcgctcagcttccgcctgcagctgcttggcctgctcctcagccttgcgcacctgctcagtggcgcgggtgttggcctcgttggtggtctgctcggcgttcttctcagcttcggagaccaagcgggtcgcgcgctgctgcgcgtcctcgagctgcttcttggacttggtgtccgcctcggtgagctggcgctctgcagcggccttggcctcctgcagcatggtctgcgcctcgttctgcgcgtcggaggtgaggcgctctgccatctcctgagccaagccgaggaccttggctgcctgcacgtgggtgtccggggtggcgacaccggcgggggctgcggccggcttctgctccaccaggcgagactggttcgcgtccgccttcggcgcgttctgcgaagccttggcggccttctccgcgtttgcggcttgctccttagcgcgcttggcgtcctcgcgagcggcggcagcttcagcctgcgcctgctcctgagcctgcttcgcgttgcggaggcgctcctcgtactcgcggcgcagctcctcctcgacgcggcggcgcaccgctgcctcatcgacattgttgttggcggccgcagccggcgcagcggcagccggggcagactggcccttgccctcgccaagctcctctacgcgggcgcgcagctcgtcgttctcgtcctgcagctgggcgagggtatcctcgacgagatccaggaactgatcaacctcgtcctcgttgtaaccacgctttccaatcggcggcttgctaaaagccacattgtgcacgtctgctggagtcagcggcatgaacgttcccttcgatgtcgaataaggtcaggaatagaagatactgtaatcgttataccctcagtttgcactacaggttgaccttttaggccaaacgctatccgcgcaaacccggggcgatcagcaacacttgaatgaggctctggacgatcacaagcgcgatgaacagcacaataacgctcatgtcgaggcccactcccccgcccaggcgtagcggcggaatcatccggcgcagcgctttgaccggcgggtccgtcaccacgaacagcggctcagccaccaccgagaaccacgacggcgggtcgaaccgcttggaaaaagactgcaccatttcgatgatgatgcggatgatcaccacgagcatgtacagcccgacaagggcgtaaagaatcgctccgaaataagccacgggtcacaccctacccatctcgccgcagcacaccggcgaccaggcagctgccgaaagcacttagatgcgagcggcgcgcttgagctcgtcggtggtgatgcgcgcgttctctggcacgatggcgaagacgcggcggcggctgccggtgccgcgggtcaggttcagcatgctgccccgcagcgcgaagcacagcccggcagcgaagtcgacgacgcgcttcgcgtcggcggcctcgaggtcgcttaagtccatcacgaccgcgtcgccgtcgcggaacggctcgccaatctccttcgcgtcgttgtaggagcgcggcgctgtggtcacgatctccggggtgaacgcccgcgagatcggctcgcggcgctcaacgcgttccggacgctcaaggcgctcggctcgctgcggagcggcaacctcgcgggtctcgcgcggctcgcggtactggggatcgtcgtagtaggcgtcttcagcatcgtcgaacgggccgaatccgaagaactctttggcggtgccgataaaagacatatgtgctgctcctagggtgtaaacgaggtgtgagatcagcctacgggccggggtccgaagacagcggttccgacacgcacgatatcggagccgcacgcaattgctgcttcgaaatcgccgctcatgcccgcggaaagttgcaaggggcggccgagggatacggcgtgggcgtcggtaagcagccgaagctctgtgaacacctcgcgcgggtcggtgtgaagcgggggcaccaccatgaatcctttgaggtggaggtgctcggcctcctccacagcggcgacgagtacgtcgaccccctcgcgcgccaccccgccgcgggaggtgtcgccatcgtaggacacctgcagcatgcacggcagcacgctcgacgtgcggtcgtcgcgctcgagcgccagcgccatgccccggtcaagccccgccgcgagtttgaccgagtcgagcgagtgcacctcgcgagcccagcgcgcaacggcgttggcctttttcgattggatttggccgatcatggcgatcccgcaggtcccgcccagctcggccgccttgtcgcgcgcctcctgctcgcggttctcgcccaccagcgtgatgccgcaggccgcaacctcgcggatcgcttcggctgggtggaatttgctcaccggcaacagcgccacgctgccttccggccgcccggcgcgcgcctcagcctcgcggatctgcgcccgcacctgctcaaggttttccgaaatcatctacttcgcccccgtcaaccagatcacgccggcctggcggcccgtggttccttcgcggcggtaggagaagaagtcggtgtcggtgacggtgtcgcgcgggtctgcgtcgattgcggtcacacccaacgacatcagctgccgcacgagacccgcgcgcaggtccagcccgcttgtgcccttcgcagtggtggtgcgcgagccgggcaggtgcttttcgacgtccgcggccatctccgccggcacctcgtacgacgctccagccgcagccgggcccagaagcgcctggatgtttgccggggtggcacccagcgacaccatcgtctccaccgtcttcttcacgatcccgttgcgcgcgcccaggcgcccggcgtgggcggctgctattacgccagccgcgtgatcagccaaaaggactggcacgcagtcggccaccagcacggtaagcgcaaggcccacctcgcgggtcaccacggcgtcggttgcctcgaccggttccgcctgcggaccgtcgacgacggtgacggtgttggtgtgcagctgctccatccacacaaactgctccggcgcaatgcccaacacccgggcaaggcgctcgcggttggctgccacactcgcggcatcgtcgccgacgtgggcaccgaggttgaacgagtcgtacggggacgacgacgccccgcctgctctggtggtgaacaccatgcggacggggcgtgaagaaagatctgccatgcggccaaactagcgcatgaagtccggcacgtcgacgtcgaagtcgtcgtcgaaaccgccgcggcgggtctcggtgcggtactcctcgcgcggcacctcgcggcgctcggtctcggggttggtaaacaggcccggacggtccgcctcgtagcggtggcgagcctggtactcgtcgccggaggagcggtcgtcgaacagcgagccgcgcgccggcgccggggtcgcgggctcggcgggcttggcggactgctcgacgttgaccgcggtggagccgccggcgttgtccgcgcccggggcctgcgccgcctgctggccgtgatgtgccggctcgttcggctgcggcagcttgttggcgacctcgtcgaagccggtggcaatgatggtcacccggacctcgtcgcccaagttgtcgtcaatgatggtgccgaagatgatgttggcgtcgtcgtcggccttctcctcgacgatggaggcggcggtgtgaacttcctgcaatcccaagtcggaaccgccggcgatggagatcagcacgcccttcgcgccctccatcgtggtctccagcagcggggagttaatcgcctgctcggtcgcggtcatcacgcggttgtcgccgcgcgcggagccgacgcccatgagcgcggagcctgcgtcggccatcacggagcgcacgtcggcgaagtccacgttgatcatgcccgggatggtgatcaggttggtgatgccctgaacaccgttgtagagcacctcgtcagctgcgcggaacgcgtccatcatggacagctcagcgtcgccgagctggagcaagcggtcgttcgggatgacgatgacggtgtcgcagacctctttcaggttctcaatgccctcgagcgcctggcgggtgcggcgcttgccttcgaacgagaacgggcgggtgacaacaccgatggtcagcgcgcccatcttcttggcaatgccggcaacaaccggcgccgcaccggtgccggtgccgccgccctcgccggcggtgacgaagaccatgtcggagcccttgagcgactcctcgatctcctgcttgtggtcctccgcggaggtgcggcccacctccgggttagcgccggcgcccaagccccgggtggcctcgcggccaatgtcgagcttggtgtccgcatcggtgaacagcagcgcctgagagtcggtgttgatggcgacgaattcgacgcccttcaaaccctcctcaatcatgcggttgacagcgttgacgccgccgccaccgacaccgacaacgcggatcatggcgaggtagttcgcgggagaggtcatgagaggattctcgcctttcaacgtagtgaggggaagcaagtagttaacgtggttcccatcattaaggaaaaggcgcggattttcgtgttcccagtcggcgtgtctcgaccctcaacctctactttagggttgtgacctggggttttgcggaactatttcacgccgacgagctgagggttcacgatgttgaactcggtgccctccatctgcagcacggcctcgagggcgtacgacttgttctcgttgtcctcggacgcgccccacgtgatccgtttgccgtccaccgtgcgcagcacgtagttgttcggttgcacttcgattgcggctaccgcagctcgagcacggttgcttatcgacgcggcgatagccaccacatccgccatcgcttccggatcctgcacaggtgcgttgaccagctcgatggcctccggcggcgggtcggcgatgaggaagtctgccccctcctcgtcgatcaggtgcgtgccgtcggattccgccacgaacgccaccgcagcgcgctctgagagggcaacgtcaatggttgacggccagttgcgcgacaccgtcaccgtcttcacccaggggtcggaggcgacgccgttcgccgcgtcctttaggttgaccttgcccatgggggtctccggcgggatagcggcgagctcttccacgcgctcgctgctcaagatgtggtttccgtccactgccactgtgcgcaccggcatcaccggggtgaacggcgccaccgccgcgaggccgccgagcaccgccgcggaagcggcgagcgagatcagcgcgcgccgcttgccgcgcttcggggcttcctgcggcgcttcgatcacctttgtcgacatcggcgcgcccttatccctgcgcgagttcggcgaggatctcgtcgccgagcagggtcacgctgcccgcgcccatggtgaacaccatgtcgcccgggcgggtcaacgatcgaacggttgccggcgccgcagagaagtccggctcgaggcggacctcggtcgcggcgtccatccgctccgcaataatgcgggagctgacgccctcgacaggggtttcgcgggcgccgtagatgtcgaggagcacgcaggcgtcggcgagcgagagcgcctcggcgaactcgacggcgaattcctgagtgcgggagtacagatggggctggaagcaaacgacgacgcgcgcgccctcgtcctcggcctcaacctgagcgcgggcagcgttgagcacggccgcgacttccgtcgggtggtgcgcgtagtcgtcgtatacgcgggtgccggcgaacgcgcccccggtgacctcgcccttgagctcgaagcggcggcgcacgccggtgaactcgctcaagcccgcggcgaggcgctccgagtccgcgccagtcagggcgccggcgagcagggcggcgagcgagttgagcaccatgtggcggcccgggatagcgagcgtgtagcgcagctggcgcggcgtctcgctctcccccgcgcgcagctgcaccgtgacggcgacggcggcggtgtccaaggcttcgtcgacaagcactgcccccggggcaatctccgggtggcgcgccgcggcctccgaggtgccgtaaccgacaacctgcaccccgcgctccgcggcgagcttgccgcatgcggccgcgttgtcgtcgtcgaggcacaccacgagatggccgccgggtgccacgcggtccgcgaaatcgttgaaaacttcgaagtacgcctcgcgggagccgaagtagtcgaggtggtcgggctcgatgttggtgatcacggcgacatcgggcttgtagcgcaacagcgacgcgtccgactcgtcggcctcggcgacgaagacatcgccctggccgtggtgcgcgttcgtgcctgcccggttgagctgaccgccgatggcgaacgacgggtcagcgcccgcggcctgcagggcgaccaccgtcatcgacgtcgtcgacgtcttgccgtgggtacccgcgagcagcacctgggtgcggccttccatcagctcgcccaaaaggtcggagcggcggatgacagggatgccctcctccgcggcgcgcagcagctcggggttgtccttcggaattgccgcaaagctggtcacaaccacggtgggcagctcgccggccagctcaaggttttcgcgagcgtgccccaccgcgacgtgcgccccttggctgcgcaacgtgcgcactgggcgggagtccttcacgtcggacccggtcaccaccgcgccgcggtctagaagaatgtgcgcgacgccggacatgccggagccgccgatgccgatgaggtggacgcgggagagatcaacaggggtgtcgttcgtgctcataaggtttcggtctccttcttccgcttacttcgccgccgcttcggcgatgcggcgggcgatttcttctgccacgttgccggcgccggtttctttcagcgcggcgcgcatccgggcaagctccgcatcgtccccaagcgtgcgcgacaccgcctggtacagcgtgtcggggttaaggtcggcgtcgtcgatgcgcagcgcggcgccggtggcgacgaggtgcgcagaattcagcccctgctcgccgttgccgtgcggcagcggcacatagatcgcgggcagcgaggccgcggagttttccgccaccgtcatcgcgcccgagcggcacaaaacaacatctgccacggcgtacgccgcctccatatcgtcgatgtagggcacggcggtgtagccgtctaccgctgccggcgcatcgttcttgcggccgtaggcgtgcaggacttggtacccgtcggcggtgaggcgttcaatcgcaccagcaagcgcgtcgttgatgcgtaccgcgccctgggaaccgccggtgaccagcagggtcttcttgccctcctcgaggtgccacatcttacggccgcgctcggccttcacaccgtcggggtcaacacctacacccggtcgcaccgggatgcccaccacgtcgcccggcatgcctgagttcggcacggcgttcaggcccacgccgccgagtttgacgccaagcttgttggccattcccgccagcgcgtttgtctccagcacgtaaaacggcagacccaggctgcgcgccgcgaggtacgccgaggccgcaacgtagccgccggtgccgaacacagcctgcgcgccggcgttcttcagcacccggcgcgtctggttgaccgacttggccagcttcaccggcacgccgggcaagagccacggcttgcggcgcgggatcggtaccgggtcaatcagctgcaactcgaacccgcgggccggcacgatgctggtttccaggccgcgctcagtgccgagcgccaccacgttagcttggtacatatcgcgcaacacttcgccgacggcaagcgcaggctcgatgtggcccgcggtgccgccgccggcgacgacaacgcttaggtgcttctcgctcatacttcttttctagcccctctcgcggctcgcccgggcgccgcgggcgccgctagccccgtgggcaccgtaggcggtggtgcggcggcgctggttcgggcgcgcggttgcctgccgggccggctgcggcggccgcggcgggcgggcgcctgttaccggggtaccgtagcgggcttggcgctgctgcgcctgcggcgcacgcgccgggcgcgacgcccgcggggtggccgaggttcgcttggggcgagcaccgcgcagctggtccaaggtcatcggttcgcggatgccaagcatgcggtcgaaggcggggcggccgtggttctgcatagaggagatagcgtcgggctcgtggcgcgcgatcgaggcgagcacgcccatggcggcgagggtgataatggcggaggtgccgccggcggacagcatcggcagctggatgccggtgaccggcagcaggccgaccacgtagccgatgttgatgaacgcctgcgagaccacgccagcggtcaacgccgccgccatcagcgattggaactggctctgcgcgcggcgcgccgcgcgcagaccgaagtagccgagaagagcgaacagggagatcaccagtgcgccgccccacaggccaagttcctcgccgatgaccgcgaaaatgaaatcgttgcgggcttccggcaggtagaaccatttcgcccgggactggccgaggccgacgccgaacagggagccgtcggcaagcgacaaaaagccctggtgcgactggaatgccacgccccgggtgtcctcgaagtggccgaacagcgcgtcgaagtaaacgtggaagcggtgcgagcggaagcccccggagaggaacgcgatggtcaacgcgacaagcccggcggccgcgatcatgccgatcgccttccaggacactccagcgaaaaggaggatgaagccgacgacgatggcaaaagacatcgccatgcccaggtcgccctgcatggcgatcaggaacacgcagatcagcgagacgacgatgaactgcgggaagccgttgttggccttgaacagccaacgcgggtcgcgcccggcgagcacctgcgcgccccagatcgcgatggcgacgcgggcaacctccgacggctggaggcgcagcgggccgacgacgatccacgactgggagcccacctcttccctgcccgtgccgatgccggggatgagcacggcgatcaaaagcgccaccgcggcgagcatgatccacgacgaccacttgtacagccgttccgggtgcgtcttcaacgccacccagaacgcgaacaggccggcgcagaccatcatggtctggcgcgcggcgagcgcccacggcgactccgacagcgcgaacgaggtggccatggaggagctcatcaccatcaccacgccaaggcccgcgagcacgagcacaatagtgcggatcatggtgtagtccagctgcgggtaggactccatgacctggtgcagcttgcggtttcggcgggccacgccggactgcggggccggtgtgctggcggggttgcggaccgtcacgggtgcatctggcctttcgctcgagatcgctacgttaggggtcagtgtaaacctctagttgaggttgctgcctagcagtgtctcattgcggcggcggcaaacgcgtcgccacgcgcagacattcccggatacatatccaggctcgccgccgccggcgccaaaagcaccgtgtccccgggcagagctttcgccgcggcgtagcccacgacctcctccatcgccgcatccgggtcggtggagtccgtgacaaagacgtcgacctcgggcgcgatgcgcgcaagcgcctcgcgcagcacctcccggtcggcgccaaggagcgcaactgcgcgcagctggtccttgtgggcggcaacgagctcatccaccgcggcacctttaagctgcccgccggcgatccacaccacgtcgcccgcaccggagagcgcggagtctgccgcgtgcgggttcgtcgccttggagttgtccacccactgcacgccgcgggccgagtgcacgaccgcaccgcggtgcccgctgacgcggtagccttccagcgcagtctggatgtgctccggcgccgcgccctgggtccacgccacagcggccgcggccagcgcgtcgagcacgcccgcggccccggctggctcgatcccttcggcggacgcgaggtcggtggcggaagcattgcgcttaacgacgatgcgcccgtccaccacaccaacctgcccttggccaggctcgcccagggtgaagccgatgatgtcgtcgcgccccgagcgggcgacaagttcgcggacatgctcgttgtcgatgccggccaccgcgtgcggcgcttgcagcacgcgcgctttcgccagcgcgtagtgctcgaaggagccgtgccagtcgatatggtcgtccgccaggttcaacagcacgcccgcatccgggacaagctggtcggaccagaagagctggaagctggacagctcggcaacaagcacgtcgactcggggggtggccatgagtgcttcagcgacggccaccccgatgttgccgcacgcggcggcgcgcttgccggttgccttgccggcctcggccatcatcgccgccagcatgccggtcgtggtggtcttcccgttggtcccggtgaccacgagccactggcgcggttcgccgaaacagccggcgcggtcgagcctgtagcacgcctcgacatcgcctacgacggggagggaggcaaacgcggcgtcgacaagcagcgggctttcggggcgccaacctggggacgtgaccaccacaccgacatccgcaaaacgctcgcgagcggcgtctgtggtgaccgcctcagcccccagcgcctcagcgcgggcgcggccttcggcgtggtcgtcggcgacgatcaccggcacgccgaggtgctgaaagagctttgtcatgccgatgccggaaaccccggcgccggcgacgatgaccccgcggtcgaactcggccggaatcacaggtgcaccccgatctggaagagccactcggagtagaacacggcgaggcccagcgccacggccatcgacgcgatcagccagaagcggatgaccaccgtggtttccggccagcccttgcgctcgaagtggtggtggaacggcgccatcttgaacacgcgcttgccggtggtcttgaacgacgcgacctggatgactacggacgtagcctcgatcacgaacagcgcgccgatgatgaccatcaaaagctctgtgcgcgagcagacggacaggccggcgaccaggccgccaagcgcgagcgagcccgtgtcgcccatgaaaatcttggccggtgcggcgttccaccacaaaaagcccatgcacgcgccgaagccggcggcggcgagcaccgcaagctccagcgggtcgcgcaccgtgtagcagcctggggccgcggcggtctcgcacgagttccggaactgccagaatgtgacgaaggtgtacgcggccatcaccagcgcggtggtgcccgcggcaagcccgtcgagcccgtcagtgaggttcaccgcgttcgaccaggcggccaaaagaatgtagatgaacagcaaaaagaccacggtgccgatcacgccgccggtggcaccgatgccgagcgtttcaatgtcgcgcgtgaagctcaagaaggtcgagccgggagtcacgccgctgctgtcggggaaacgggtaatcagcaacccgaacacaatcgcaatgaggaactgtgcgaccaacttcgcggttttgttcaagccgaggttgcgcttgaagaagattttgatgccgtcgtcggcgaagcccaccagccctagtgccagggtcaacccgagcacaatcaacccggaggcggtgaatcccgcgtgcccgcccgcgactgcgtaggtggcgctggctagatacccaagcgtgatgccgagcaaaatcgcgatgccacccatcgtcggggtgccgcgcttcttggcgtgccactgcgggccgtcctcgcggatctcctgccccatctcgcggcggtggaaataccggatgagcgcgggcgtggtgaagatagcggtgaggaagctgaccacgccggcgatgatgagctgaatcatgtctctcctatcgttcgccctcaagggtatgcgcaggcatgagccgctccgccactgcccacaggcccagcgagttcgacgccttcaccagcaccacatcgcggtgttcgcgctcgtgccagccggcgacgccgctcggcgcggcggcgagaatggcctccaccgcctcggccgcggccgcggcgttcgaaacttcctcgaccgcgatgccgtgctcgcgcgcgctcgacgcaagcgccccgacagcgtcgttgtcgccgacggtgacaaggtgggagacgcggtagcgggcgagctcctcggccatggctgcgtgcgcctgggcggcgtcttggcccagctccgccatctcgccgagcaccgcgatggagcgcaccccggggcgcgcggcggcggtgaagccgagcgcggcaatcgcggcgcgcatggactccgggttggcgttgtaggcgtcgttgatcaccgtcacgccgtcggggcgcgtgttgacatccatgcgggccaccgacaccgagtaggcgttgctcagcgcgtccgccaccgtggccgcgtcaatgccacactcgatgcccaccgccgcggccgccaaggcgttggaaacctggtgcgcgccgaagacgttcaggcggaccggctgcggcttcgcgccggggctgtggagggtaaaggttgcgcgggccagctcgtccagttcgacgtctgtggcgtagtagtccgcgggcttgccggaggcgatgtcgttgttgccgtcggcggagaaagtgaccacgcgggcgctggtgcgcgagcgcatcgcggagacgaggtcgtcgtcggcgttgagcactgccactccgccgtccgcggcgctgggcagcgactccaccagctctccctttgccagggcgatgttctcgcgggagccgaactcgccgaggtgggcggagccgacgttgagcaccacgccgatcttcgggggcgcgatctgcgctaagtgcgcaatgtggccgatgccgcgggcggacatctccgcgactaagaagcgcgtgtcttcggtgcatcgcagcaccgtgtacgggtggccgatctcgttgttgaaggatccgggcggggccaccgtctccccgccccgcgagagcaccgcggccaacaggtccttggtggaggttttgcccgcggagccggtgacaccggcaatgacaaggccgctgtttgcggccaactcgcgcgcaacatgggcggccagcgcgctcatcccgcgcacaacacctgccgccgaaccgtccgggtcgttcgtggcgaggtcgctgttgtcgccgtcggcgcgtttcaccttctgaagcactacggccggctggcccacctcgcgcgtggtcaacgccgcggcggctccctgctcaaccgccttcgggacgaagtcgtggccgtccaccctcgaaccgggaagcgcgacgaacaggccgcccggggtgatcttccgcgagtcgaactcgacgaagctggtcacccttgcgccgggctgcgcttccgggctcaactgcccgccggtgatctccgcgatctgcgcaagcgtcagcggaatcatgccttttcctccttggatgcagcgagcgcttcgcgcatcgcttccctgtcgtcgaagtggtgtgtggtggtgccgatgatctggcccacttcatggcccttgcctaccgcgatcaccgcgtcgcccgggcgcgcccacgccacgagctgcgcaatcgcctcgccgcggccgccgacttcgcggatctcggtgtccgggccagctgcctcgcgggcgcctttaagcaccgcgccgcggatcgtggccgggtcctcggtgcgcgggttgtcgtcggtcacaatcaccaaatccgcgcggcgcgcggcttcggcccccatgatggggcgcttggaggcgtcgcggtcgccgccggcgcccacaaccaccccgacgcgcccggcgacctggctgcgcagcgtgtccagcaccgcggcgattgccgcaggcttgtgagcgtaatccactaccgctacgaacccttggccctcgtcgacgcgctccatgcggcctgggacggcggcgttttccagcccccggatgaacgcttcgacgtccgcgcccaccgcgttcgccaggcccacggcaagcgccgcgttcgccacgttgaactcccccggcattggcagccgcaggtcgtacgcggcgccgtcgacggtgagcctgatgtcttgggcgccgttcgcgtgcgtgccgcgctgctcggcggccacggtcagcccggactgtccacgtgtgccaacaaggtctggcgtttgggccacgcccgccatccgctcgccccactcgtcgtccacgcagatcacgcttcgccgggcggcgaggtccgacgctgggtcgaagaacagcgccttcgccgcgaagtagtcctccatcgtagggtggaaatcgaggtggtcctgcgaaaggttggtgaacccggcgacgtcgaagtctgtgcccccgacgcgccccagcattagcgcgtgggaggagacctccatcactacgtgcgtgaccccgctggcgagcatctgcccgaacagctcctgcagcttcggcgcctcgggggtggtcagctgggaggggacgtcgcggccgtcgatacgcgtgcctgtggtgccgatcagccccaccttgcacccggcggccgcaagcccccgctcaagcatgtacgtggttgtggttttgcccgacgttccggtgacgccaatgagcttcatgcttttcgacgcccacccgtacacctcagccgccaccaccccaaggaccgcgcgcacgtcgtccaccaccagcaccgggcgcgtatcgcccgcagcctcgatgatgcgaaggccctcgcggtctgtcaggatcgaccccgccggggacgcggcggcgaactccgccccgtggacccgcgtgccgggaagtgccgcgaacatcccgcccggctccaccgccttcgagtccagggttatctgcgtcacggtcagcggcgccgccggcgggttgacggtctccgcgccagcgattgttgcaagcacctgcaatgtggtctgcatgcttctctccttactgcgcctgaagtacgtacggctcggctggcgggctgggcggcacattctcgcggttgagcagccacgacgcgatctcggtgaacaccggtgcggcggactggccgccggcgcccccgcggagcgggccgcgctgcggctcgtccagcatcacagccaccacgaaccgcgggtcgtccgctggtgccacgcccgcgaatgtgatccagaactggctctgcgagtacgcgccggtatcggggttcaccttctgcgcggtgcccgtcttgccggccagctggtagccctcgagcccgctgccctgggctgtgccggactgcagccccgaggggtccgactggaacacagagcggaacatgtcgacggtggtccgcgccgtttcctcgctgaccaccctggtgcgcgccggctccggctgctccacagtctccccgtcagggccggtcacgctggcgatgatgcgcggctcgatgcgctcgccgccgttagccagcgcctggtacacccccgccatctgcagcgccgtccagctcatgccctgcccaatgggcaggttggcgaaggtgccgcccgaccactgctcgcgcacgggcagaagccccggcgactcgttgggcagctcgatgccggtagtggtgccgatgccgaatcgctgcaagtactcccagtacttgtcctctccgagtcgctgcgccagctgcagggtgccaacgttagaggacttaccaaagatgcccgccgtggtgtacggcgcaacatcgtgactccacgcgtcgttcacggtaacgcctgccatgtcgatagagccgggcacttggtggacctcggtcgggtcggttaacccctcctcgatcgccgccgcagcggtgatcactttcgccactgaacccggctcaaaggggtgggaaatcgagttgttgtcgaaatcgcgcccctccttgagctgcttttccaagtcgccgttcgggtcgatggtgtccgtgttcgccatcgcgagcacctcaccggtgcgcgcgtccaggacgaccgcttgcccctccttggccagcgagttctccttcgcttgctgcagcgtctgctgaacaaacgtctgcaggtcgaggtcgatagtcagctcgatgcgggagccgtcgacggcgggcaccacgtcacgcagcgaaccggggatggccaacccgtccgcggagacgtcttcggtggagcgtccgttgatgccggtgagcatcgcgtcgctggacgcttcgaggccgaactgcccgtggccgtccatggacaccttgcccaagatgttctcgccgatcgcgccgttcgggtactggcggatgtcttggtgatcggccgcgacaccgtggaagttggaggcaactttcgccgccacgtccgggtcgacgttgcgcaccagcacctcgtagtccgtctcggcgtgcagcttgtccaagatctcgcgggcggagacgttgcccaccttcacgttctcggtcgcacgggcgtcgcgcgaggtggtctccttggcggcctgctccccgatcatggctggaatctcgttggccatggtgcgcagcacgtcctcgacgcgggcgtctatttgggcgtcgatggagtcctgcgaaaggccgtcgacacgcatctggagctcctgctgctcctggatttccttgcgcagcgtcaccggcgaaacagtgagcgagcgcgcctgcatggtgtaggcgagccggttgccctcgcggtcaacgatctcgccgcggcgcgccgggtccacgtaggtgcgggtgcgttgcgcgctggcctgctcgcgcaggtccggcccccacaccacttgcacccagaacaaccggccgatgagcagtgcagccacggcaaggaacgcaactgccagccacgtggcgcggcggttcgtgatctgcgactgcgtcatcggttgctcgcgcctggccacgtgcgttctcacctaccttgcttcgtttgcggagacgggttgcgtaacgacccttatattgcacgcagcgcgctcgtttcagggcgcgccacacgctagaacgctgcgggaacgttgggctggtacggcgcgaggttgtccgtgcgcgcggccgcgggcgggttcatcatgttgccgccgggcagctgggtcaggttgtcgcccagctcatcggttgcgcgctggtcgctggtggcgcggcctgcgcgggtgggctggccgttgacgtccagaaccggggcgacggattcggggttgaactcgcgccgctcctcgacccggccgtcggcgtcgacctccacgatgccgggctgattcgccaccaccatgttggcctccgcggcgcgctgcgcgagctccgccgaggaacgcaggtcctccaggtcgcggctgagcgactccacctcgttctctaacgcgcgctcctgggactgtagttgctgcaccgtgaacgtctgggccgtggacaggcccgacaggaccatggccacggcgacgccgataaccaagagggtcaccgccaagccgccgaccttgccgagcgcggttttctgtttggcaggagttgctactcgacgcccgcggaccgacaccacctgctgcgaccccaaccggccgccgcgagacttctggtgcgggacgtgcgggcgcacatcgggacgggtggccggggtgcgcttcggcgccggtgcgtaagtggcctggtccgtgcgagtcatcactgccatggtgaatctgtccttaagtcggaaagtttttcaatgccacgcacccgcaccggtgtagcgcgggggttgagttcgatttcgtccttcgaagccttctccgccccgttggtgatcggggcgaacttcgccgccgtgccaggcagatccatcggcaaccccggcggggtcttcgacgttgtcaggtccgcgaacgcggttttgatgattttgtcttccaagctctggtagctcatgaacaccactcggccgccaggccccagcagctccgtgatgaccgggacagcgttctcgactgcctccagctcgcggttgacctcgacgcgcagcgcttgaaaggtgcgcttggcggggtggcctccggtgcgccgcgacgccgccggaatcgtctcgtacaaaagctccacgaggcggccgcttcgcgcgaacggctcgcgctcgcgctccttcaccaccgcagaggcgatctttcccgcgaagcgctcatcgccgtacgtcttgaggatgcgggcgatgtcgccgtgcgagtaggtgttgaggatgtccgccgcggtaatgccctgcgtcgggtccatgcgcatgtccagcggcgcgtcaactttgtacgcgaatccgcgctcttcttggtccagctgcatcgacgacacgccaaggtcgtacagggcgcccgcgacaccgtgctcgcgcaccgtgtcgaaaacgcggccctccccctccccgatcggccccgcgatgtcgtcgaaccgcgcctggagcgggacgaagcggtcgccgaacggcgcaagccgctccgtcgcctgcgcgagcgcgatggggtcgcggtcgacgccgatcacgctggcaccggggaaaacagtgagaaaatgctcggtgtggccaccggcacccaaggtgccgtcgacgatcaccgcgttgctgccgaagcgctcaaccgcaggggcgagcagctgccccatccggtcgcgcatgacagggacgtggccgtggttcgctgcagttgtgaattccacgggtgccacccccaatccctgtccgatgtaagtctctgaagttcttgcttcccttggtgagggggagcgagtagagccctgcccggggcggccggtctgatgtcggggaagtacaccagaaaagctcacgccccggacagagtccgtacacgctctccgtcagtagtcgtttgcctgctgcgcgggtagtcagtccttacagcagaccggagagaatgtcgtcgtcgtccgccgccgagaaggcggcttccgtctgttcctgatagtcggcccaggacttcgcgtcccagatctccagaaaatcaaccgagccgataaccacgcactccttggacaggtttgcgtactcgcggtgcgccggcgacaacgtaatgcgaccagaaccgtcgagcgtctgctcatccgcgctggcagccaggttgcggatgaaggcgcgcgccttcgggttcgtgcgggaggccgccgccgccttgcgagcgcgctgcgcgaactcctcccggggatagaccgctagcgagtggtcctgccccttggtcaccattagcccgtccgccaagtcctcccggaacttcgcgggcagcgtcaggcgccccttgtcgtcgagcttgggagtgtaggttcccaggaacatcgggcgacctacctttcctttcgccgtctgacttcggcttgtgaagtttttctgccgcttcgatgtgccgcacccacgtagtcagatgggcgccacacttctccgctgcgccccactttaacccacttctccccacgatggctacaccacagccgaaaatgcccgattatttcggtgttactgcaggttgtagcggtggagacaaggtggagattctgtgccccaggagcgtaaagctgccacattggacctcaagatgcacatggattcgcgtgtccggtgaactcccaacattgcatcgacggccgaaaagccctgctcgcgtggtggcgcgccaccctggtgggcaggagtggggcgcgtaggtgggggaaggtgggagacggcggtgatagcgggtaactcgggacagacgccgcgtttccgcaggtcgctacgggtggcgcgaggagttacccgctatcaccgggtttccagccgccggaaagacgaaaaagcgccccacacggggcgcttccaaaggtcgggaccgtcttaggcttgcggatcctcgaaacggcggcggaagttctcttccatactcacgcttcgggccgatcgctgcttcggcgcactcgcgctaatgcgtgggcccgcagaaggagtggtggccggggtgcgcagcgccatcacgccaccgagcatcatgacgccgaaaccgacgatgctgatgacaactgcccacatgctggcggacgcgagtgcgacgccgccgagcaagaggacgatccccagcacaatcagcgcaacgctgcgcattgtgagacgccccctccgcggggtctcgctgaatccagcgttgtgcgcgacgctgctggcgaactttgggtcctcagcaaagagggactgctcgatctcgcggagcgcgcgctgttcttgctcagaaagggacactgaaatttctctccacgttgacgggaacgatatttcttaaccaacggacatcgtagccgttttgttccccgcacccactacgctgccgcgagcggcgcctccccagggtggatctcgtggtagaactcttccgcgtcggcgagcagccgaacgacaatcgcgggatctgggtgcatctccagcccagatacaacccggccccggaggcgggagtaggagcggaatcgggcagcccagagtttcccgctatcgccgacaagcgccagcttctcccacgcgctagtgggcaaccgtttccttttccgcagcgcttccgaatcggcgacaacggcaccggcgacccgaagcgccgcccggtaggcgctttccatggccaggtctgcccggccgtcttcaaattcctcgtgcgccgcaacaagaagagactccgccgaggcgaggaacgcgtcgcggcgcgagaccttcgcgggggcaccgtaggctcgggacgtggtggcggaaatgacgctttgcattgtgtttccccttctcttccagtggtgtttacaacgattgcgctcactgtaaaacacgcgttcgacaccacaccgccgacattagaacacgcgttcgattagcgggcatcgaaaaccacccgccggcatactcccgcgtggttaggtagtggtgtgccagttgaaatccgccgcttaactcctggggagttcaccctgcttgtcccccagctcgtggacatctacctcgccgcaatggagtacaacccgcaaatccgcgaccagcgaatccgcgtgtggaaagacgaggtgacctggcccggattcaccgcggttgccgcggttgacggggacgaggtggtcggcgtcgcgtacgggttcctcggcagcagggagcggtggtgggaccgccagctcgtgcgcgccatgcgcggttccggccagctgaccgagcagcaccgagcgatccttgacagctacttcgaggtcactgaggtccacgtggctcccggccggcagggcgcgggcatcggcgcagctctgcttcaggagcttcttcgcaacgcctccgccgagtgggcgctgctttcgacgcctgaggtggataacgaggccaaccacgccttccacctgtaccgccgcttcggctttacagatatcgcgcgcggctaccgctaccccggcgaccacaggccgttcgctatcctgggccgcccgctgccgctttaaaagtgggggcacgtgaaccaggtagggtggggagccaccgcacgattgctgcaaggagttcgcacgtggacgcaaacgcgcttgatttgtcacgggtgccagaagaagtcggccaccagctgcaacgattcttcgctgagcgctcggcggagatcggccgcttaggcgcgccggtgcaaagcgcagtgctccacctcgagcgcttcgttctcggcggcggcaaacgcatccgcccgctttacggctgggccggattcgtcggcggcggcggcatcgagcgcgcagccgaggacccggaagcggtgatgcgcgcggtcagctcgctcgaactcatccaggcctgcgccctcatccacgacgacatcattgacgcctccgacacccgccgcggcaacccaacggtacaccgggcaattgaggcggagcacaacaaggagcagctgcttggcgacgcagccttgttcggccagaacaccgccattttgatcggcgacctcgcactcgcttgggccgaggacatgtggcgctcctccggtgtgaccgcggaagcgctcgcgcgcgctgagggcgcgtggcgcggtatgcgcaccgaggtcatcggcggccagatcctcgacatttctctcgaggcagcgggcagcgagtcggtcgagatggcagaccaagtcaaccgcttcaaaactgccgcgtacacaattgaacgcccgcttcacttgggtgccgcgctcgccggcgcggacgaggcgacgatcgaggcgttccgcggctacggccgcgacatcggcattgccttccagctgcgcgacgatcttctcggcgtgttcggcgactccgccgtcaccggcaagcccgccggcgacgacatccgggaaggcaagcgcaccgtgctttacgccgaggcactttcgcttctcgacgccgccggcaacccctccgcgcgcaccctccgagagggcatcggcgcgacttccgacccagaggcgttggacgcgcttgccggggtgattcgggaaagtggggctgtggaggccgtcgaaaagcggattgcttccctcaccgaatcgggacttgcgcacctcgaaaccgcgaacatcaacgccgcggtggcgaagaccctgcgcgatctcgcgatccgctcgaccgagcgccgaagctaaaacgccatagcctgcgcgcggcggataacttcgcgcgcgccgtggccgtgaagcgcgtcgatcggccggcccgggagggaatcgtccggcgtgtagagaaagtggaggatctcgtcggggtcgtagccgccgtccgccagcacggtaatagccccgccgacaaacttggacaactcgccgtcgccgagcagcgacgccggaatgtagcgcacgccgtccttgcggtacacggccagcttcccagagttgacgatgtcgtggaccttcgtcacgggaacgccgaggatctccgcgacgtcaggaaccgggaggagctcctcgcctaccagcagttcgtccagggttggctgttgcggtgtagtcacaagcccacattctactgcccttgtcgcgggcgctgttggccaacaccgcggcgggtgatcatactggttgcatgcgtttggcagtgggcgattccttggagggccggtacatcatcgaccgccccatcgcgcgcggcgggatggccacggtgtaccgctgcgttgacaccaggctgggccgcgaggtggcggcgaaggtgatgcacgagcagtacgtgcacgacccggtgttctcggagcggttccggcgcgaagcacgggcaatggcgcaactcagtcaccccaacctggtcaacgtctacgacttttccgccgacggcgacacgatctttctcatcatggagttgattaccgggggcacgctgcgcgagcttctcgacgagcgcggccccatgcctgcgcacgccgccgcctccgtgatgcgcggcatgctcacgggcctgtctgtggcgcacgcgaagggcctgattcaccgggacatcaagccggacaacgtgctaatcaacgccgaccaccgggtcaagctcgccgacttcggcctggtgcgcgccgcctccgacgcgacgcactccaccgaccagatcgtgggcacggtggcctacctctcccccgagcaagtcgacgggacgcacctgacggccgcatccgacgtctactccgccggcatcgtcttcttcgaactgctgaccggccgcacgccgttccacggcgactccccgctcgcccacgcctacgctcgcctccaccacgacgtagcggcgccgtcgtcgctgattgctggggtgccgaagcttttcgacgagctcgtagccacagccaccgcgcgccgcccggaagaccgcttccgcgacgcccgcgagttcctcggcgcgctcgacgatgtcgctgatgcgctccagctgcccgcctacaccgtcccggtgccgcgcaactccgcggcgaaccgcgccgcggccgtgccgacgagcttcggcaccctgaacgggccgtcccgcaaggtggagccgcgggtggagccgcgcgcaagccagcagcggctcttccccgatcagacacaggaggtgcggtatgagccagcgccacctgcgcgcaggcaacctcagcctgcgccgcgcccccaactcgaggcccccgcttcgccgggcgctgtgcctgcggaacgcccgcgcatcaacccggtgacgaaccggggtggcatcgggctggcgctgtttgtcgccgtttccatcgcagcactcgccgcggtgctcgtgggcgcctggtggttcggctccgggctgtacgggatgttcccgccgatcctcgccggctaggttcaccccgaagcgttagtagcggagcatctccgcgacgaggaacgcgagttccagcgcttgttcggtgttcaggcgcgggtcaacagcagactcgtagcggcccggcaggtcgacgtcggtgatgtcctgcgcgccgccgaggcactcagtgacgttctcgccggtcgcctcaacgtggatgccgcccgggtgggtgcccaactcgcggtgcacttcgaagaagccctgcacctcgtcgatgatcttgtcgaagtggcgggtcttgtacccgttggaggcggtgaaggtgttgccgtgcatcgggtcggactgccagaccaccttgtggcccgacgcttcgacggccttgacaatgcccggcagcaccgagcggatgttgtcgtggcccatgcgggtgatcatggtcaaccggcccggctcgcggttcgggtcgatcttgtcggcgtacgccaccgcctcttccggcgtggtggaggggccgagcttgatgcccaccgggttgtcgatgagcgccgcgaagttgacgtggaagtcgtcgatgccgcgggtgcgctcgccgatccacagctggtgcgcggagaggtcgtagagcttggtctcgccgcgctcgttctcagcgagacgcagcatcgcgcgctcgtagtccaccaaaagcgcctcgtgggaggcgtagaactcggagctgcgcaggttctcgtcgttcacgccgcaggcgtccatgaacgcgagcgagcgcgaaatctcgcggccgagcgcttcgtagcgcgcgcctgccggggagttggcgacgaactcgcggttccagtcgttgatatggtgcaggtcggcggtgccggaggagacgagcgcacgcaccaagttcatcgcggccgaagagttcgcgtacgcgcggaccatgcgggccgggtcgtggcggcgggactcctcggtcggctccacgccgttgacgatgtcgccgcggtagttcagaagaccgttggagtcgcggtcggaagaacgcggtttcgcgtactggccggcgatgcggccgatcttgaccaccggcagggatgcgccgtaggtcagcaccgcggccatctgcagcagggtgcggatgttggcgcggatgtgcggttcggtgttggactcgaacgtctccgcgcagtcgcctccctggaggaggaaggctttgcccagcgcgacgtcggcaagcttggctttgagctcctcaacctccggcgccagcacgaccggcgggacagactcgaggatcttgcggaccgcgttcgccgcgtcctggtcccaggacggctgctgcttcgcgtcgcgggccagcacgtcgagccagcgctgattcaggtcccccggcatcggcgggagatcgggcagcacgtctttggggatgtcgattgtccaactcacagctctattcctaccacacaattcatcgggcggaatggttgttccgcatagtggacaccttgccgttgcggtcaagcggcaaagcttcagcgcaggcgcggtacttcttgaggttgtggcgcgcatccaccagcgcgtcgtggttgccgtctggcagtcgcggcaagcgcgggcggcccgccatgatccagtattgcttgagctcgcgggtgtaccgcggcaactcgcgcggcaagccctgcatgtcgccccaaagctgggcgaaaacgacgtggtcgtaggcgccgacccacgcccacagctcaggttcggggcgggaggtgaggaaggcgaagagctcgtcgcggatgaccccaagtgacttccacgccgggttgtgcgccggcggcagcttgtcgagcacgttctcgcgcacccactcgttcgccgcagctgcgtcgaactcggtggagacggcgtagtactccctgccgtcctcggccacgacgccgatggagatcaactcaatagtggagccgtcctcgatgaactcagtgtcgtagaagtacttcactgcccttaccgcttctgctcttcccggatttccttgatctccgcgcgggtcgaaggagtatgctcgccgcggcgcggccagaacatgacaacagccaccgcgaccacggcgagcggggccgcgatctcgttgtggaactcgagccgcgacgccacaaggtaggccgcaacgataactacaacagcagcgatgcgggtaaccagatccctatccacgggtgccctccttcccgaccggcgcggtttccaggtcaccgcccggctcagcgccttcggggtacgtgcccgtcttatccagcgacttcttcacgtcggtggcgtacatgtcgacgtaggggtagccggacagctcggacagcttgcgcatgcagtagtcggtgaaggggcgcgcgacctcgcgcgagtgcgggtcgtagccgttgtcgcgggcccactggtgcgggtcaatctgctcgctcaagtggatcttcaccttggcggggcgcggaacggtcgtcccgatcgggttcgcgtcgcgcgagccgaccatggcgaccaagacaacaggcgcaccagtggccatggcgatgcgcgccatgccggtgcggcctttgtaaatgcgaccgtccggcgagcgggtgccctcgggatagatgccgaacacgtcgccgtcagcaagcaccttctccgcggcttcctgcagcgcgtcgccagctgtggagctggagcggtccaccgggatctgacccaccgaggagaagaagaacttctgaatgcgcccgcttatccccggagaggtgaagtactccttcttcgccgggaactggatttgcctgcgcatcatcaacggcaggtagaaggaatccatcaccgcttggtggttggacaccaagatcaccggcccctcgtccggcacgtgctcgcttccggtgatcgtcgggcggttgtacaccagaagcggcgggccgaggatcgctttgaagaaggagtaccacttgttctgcattggaaacgctccttgtgcctttctttcgcgacccctaggccagcagggtgcgggccaaatcagctacgccgatcatacctgcctggggtcccagctccgcccgcagcacctcgggcacgggccggtagccggagcccaccatgttcgccgccatctccgcgcgggcctggtctaaatagaggtctgcgtcggcactgactcccccgccgagcacgatcagcgcggggtccaacacgtcggcgacgatggaaagtcccctgcctagccaggtggcgaagctgtcgagggcggccacacctaacttgtctccgcggcgcgcagcctccatcacgtcgtgaccgtccgctcgcttgtccaccaccttgcggtagagcgcgcagtcggtgaacgcaccgtgggtggctttctcaatcgcgcagtcgatcagtgacgtgccggaggcgtagcgctcgaggcagcccttcttgccgcacgagcacacgcgcccgccggggacgacggtgatgtgcccgaactccggcgcggtgccgaaagagccgcggtagatctccccgcggtgcatcaaggtggctccgatgcccgtgcccacggcgaagaacacccacgtctcggcgtcgcgcgccgccccgtaccggtactcgccccaggcggcggcgttcgcgtcgtgctcaagccgcaccggcagcccgatcgcgtcctcaagctccgtgcgcaccggccggtcgtcgcgccacggcaagtgcggagcaaaccggacaatctcgcactccgggtcgaggaaacccgcaatggccaggcccactgcctcgaccgggtagtcggcccgcagattctcgaccgtctccacgatcgcgcggtctaagtcgtccgccgcgtgaggtgtttctgtggagcgcacgtgcacaacagtgccgtccgcgtcgaccaccgcggcgcgcatattcgtgccgccgatatcgaagcctacggtcaatggcgaaggtgacggcgtggatggcagggtcatagcagaacacattacgcacggagcgcgtcgacgaggcgatcgcccagcaccgaccacgagtagttcgaagcgacgtgggcgcggccggcggagcccatgcggtttgagggggcgtgatcaagcaacctgctcaacgcgtccgccagccctgctgtgtccctccccccgaccaccacaccggtttccggcgtgaccgtctcgggtgcgccgccagaggtgcctgcgatgaccggcacctcgcaggcctgcgcttcgaggtagacaatacccaagccctcgacgtcgagcccgccgccgcgggtgcgcgcgggcatggcaaagacgtccgctgaggcgacaatgtcgcgcagcagatcgcgctcgaccttgcccgtgaagtgcaccccgtcgaccccacgcgccatgcgctgaagtctgccgcggtacggtccgtcgccgacaatgaccagctgcgcacccggcacccgctcgcgcaccgtcggcagcgcgcgaatcagctggtcttgacccttccgggccaccaggcgcgaggcgcacaccacaagcggcgcttcgcctacccccaaaagatcgcgggtagcactgcgcctttgcttgtcgacggggcgaaaataccccacatccacccccgacggcagcgccacatactcaggccccgcaccgaacgccggccgcagcctcctcaaagtgtattcggagatgtacgtcaccacgtcggcgctgttgccgatgcggcgcagcgcctgccgagcccccggcagcatcgaccaccccacttcgtggccgtgggtcgtagcgacaacgcggcgcgcgcccgcccttttcgccgccgcgcccagaagcccgagcggcgccgccgcaccgaaccagaccgtgtcgatgccgtagtcggcgatcaactcgctcatccggcgcgctgtcgctggcgtgggcagcatgacgttgcgtggccagcggacaacggtgtacggctgctcggcgtcgaaggcggcggcctcacgggcgtcttgcgtggaggcgaacacgacgatcgagtccgcgccctcgcgggcgaccacctcagcggcgaagtcgcgcagatacgattgaatcccgcccacggtgggcgggaaatcgttcgtgaccagaagcgttgtcatcggccggctagtagcgcaccgccccagtgatcggcatcgagttgtacggcaccacctgaattggaatcccgtagtcggaggagtgaacaatcatgccgtctccgatgtacatgcccacgtgtgtggtgcccgggaagtagccgataatgtcgcccggctgcaggtcgcccagggacaccggtgtgccgccggcaagctgcgcctgtgaggtgcgcggaatggcaacaccgttctgggcgtacgcgtacaccatcagccccgagcagtcgaactggttcgggccggtcgctccccagccgtagggtttgcccagctgtgccagcgccgcggagaccacgccggtgccagtgccggagagcaccatccctgcggtgtcgaccggattgtctttgttcacccatcgggcgcgggcttcaggcgcaagcccgtcaacgcgagcctcgatgtcgtgcacccgcttgtccaagtcctcgcgctcacgctcgagcacactgcgcttcttatctagttcctcgcgctggcggcgggcctcatcggcggcgcggttagcggcgtcggaccgctcggacgcgtcgcggctcgcagcgttgaggttgtcgatcgtgcggccagcgttacgcgacagcgctcccaagtatgccgcgcggtcaattgcagcctgcgggctaccggactcaagcgtgttgaggaggagctccgactgcgtgttgcggtagcgcgactgggcaatcccgttgacgttctgctggaacccctggcgagcgccgctagcgcgctccacgtcgccgcgcgcaaggtccgcctggtggttcagatcgtcgacgcggtgctgcgccgccgcgatctcgtcctccagcttcttgatctcctcgaccttggcggtcgcgtcgtgcgagatggagtcgagctccgcgatgaggtcgtccacctcatccgcgcccgcaggcgggctcactaccggtgcccaaacagccgctgcagccgcaattgctgccgtgtaccggaggcccgaaaccgccctgcgccgcgaatgctttcccacgcccataactcccgttgttactgcgcctttacaaaaccgttaccactatagcgctggccgcaacccccgccaacccgccttcggcacccaagaaaacctggtgaactgcagtgatagcagagaagggtgggacaaacgggaaactacgcgcggggcggcaaaagtgaaaggcccagccccagtgggctaggcctatcgtgcccgcgtcagcgggaaagctactctagtagaagcggaaagcggagtgaaccggcatcatgtgcagcgagcggtagcccaccggaatgccagagttcaacgcgtcgatgatctggccgttgccgacgtagatcgccacgtgggaagcgccgccgtagtaggcgacaatgtcgcccggctgcaactggtcaagcggaacgcggtagccggctgcagcctgcgcctgggaggtgcgcgggatggagatacctgcctgggagtagacccaggaggtgaagccggagcagtcgaacgcgttcgggccggcagcgccgtagacgtacggagcgccaaccttggagcgtgcaatgtcagcgatctgctgacccttgttcactgcaggcgccggggccggcgcggcgtaagcctgagcctgggcagctgccggtgcgggagcctgctgcgcctcgacgttgttcaggaagttgttgaagctcgggacgttggcgacacccggcagggcgcgggcagcctggacagctgcgttgacgtcagcgttcgaggtctggcctgcgagagagggaacccactgctcgatgcccgggatagcggcgatgcccggaacggactcgatgccaggaacctcaactgcgatcggggtgttcggaacgcgaacctcggccgcctcagcggtcggggccatcatggttgcgcctgcaacgacggcggttgctgctgcgacggtgcgtgcagcggtgttgttgtcctggcgacggtgcttagccacgaaagtgttctccatatcaatctctgcgcctaccgggttagctgacgggttgggctcgagacagccctagcgcgctccgcagcgcgattaccatcgcgccgtcctcgcggccattcaccccaggggcgaaacggtatcgaccgtttccgtatgggcccccggctcccctctttctctccgctgcggtgttgcacctcgagcgagtgggactcggcgtcatatgttgttgtttcgtaccttgcgtcaacgttcgttatcgcaatgtctcgagaagattacaaaacggcaacagcgatgtccatttcccacgccgttatcttttcgttacaagacaaagttaccccaattcggggtgcgcggcatgtggccacttcaccaccgggcgatacggacgcggtctaaaaatggccgctacctggacacactcagatgctcgcgcccagtcccccgccacggtggttgagactggcaccgaaatcgtcctccggcgtgatctccatctcttaaccgttttgtgacataacgaaagcccctcccgcgaaggaaggggcttgtcgctggactaggaaagcctagtcgcgcggagttgcgtcacgatcggtgaggtgcttcgtctcctcgagacggcgcagggtctcaatctcctcgtggtggtactcgtccgcaacgtcgcgcacgcgctcggtaacaccgatctcagccggggagaaggcgccgatcgtctcggcgtccgcgaaaccgagctggttgagctgcttcggcaccggagcgcctgcgtactcgagcggcaccgggtgaccgtgctcgtccaccgggccgagcggctggtggatctcgacgaaggcgccgttcggcagcttcttgatcacaccggtctcgataccgtgctccaggacctcgcggtcggagcgctggaggccaacgcagatgcggtaggtgatgaagtacgccagcggcggcaggacaatcagaccgatgcggccgaaccaggtcatcgcgttcagcgagatctggaagaagtgcgccacgtggtcgttaccgccggagatggtcagcagcatgaagaacacgatgcccatgacacccagacccgtgcgggccggaacgtcgcgtggtcgctgcagcaggttgtggtgagcatcgtcgccggtgaccttcttttcaatgaacgggtaggtcagcaagacgatcaccatgaccagcgccatcagggcgacccagaaggcgcccggaatggtgtagcggccgaggtagagctcccacgccggcatgacacgggcggcaccgtcagtccagagcatgtagacgtccggctgggaaccagcagaaacctgcgacgggttgtaggggccaaggttccagatcgcgttgatcgaggttaggcccgccatgcccgcgaggactgcgaagacgatcagcatgaagccgatagccttcactgcgaagaccgggaggatgcggatgccgatgacgttgttctcggtgcggcccgggcccgggaactgggtgtgcttctggaaccagaccatgagcaggtggccggcgatcagcgcgaggatgatgcccggcagcacaagcacgtgcaggatgtagaagcggtccagcatcaggtcggacgggaagtcgccgccgaagatggcccagtggatccaggtgccgatgataggcacggacagaataatcgcggacatgattcgcaggccgacgccggagagcaggtcgtccggcagcgagtagcccatgaagccctcgatcatgccgagcaggatcagggtgacaccgataacccagttcgcctcgcgcgggcggcggaatgcgccggtgaagaagatgcgcatcatgtgggcgaacatggacatcatgaacatcagcgcggcccagtggtgcatctgacgaacgaacaggccgccgcggacgtcgaaggagaggtccagcgcggtggcgtaggcgcgagacatctcgacgccgttgagaggcaggtacgcaccgtcgtaaatcaccttggtgatcgacgggtcgaaaaacagtgccaagtacacaccggtaagaagcaggatgatgaagctgtacagcgccatttcacccagcatgaacgaccagtggctcgggaatactttgttcagctgcgggcggaggaagcctgcgcccgagtagcgcgaatcagcgttgtccgcggcttttgcgagtctcgtgctcattaggattgacgctcccagaatgccgggccaacgggttcgatgaagttgccgttggcgatgaggtaaccttcttcgtcaattgacaccggcagctgcggaagcgcgcgggcggcggggccgaagatcggcttaccgtgctgcagcgcgtcgaactgcgactggtggcaaggacacaggattcggttggtctgcgcctcgtacagcgaggtcgggcaaccaatgtgggtacaaatcttcgagtaggcgtagtagtcgccgtagtggaagtcctcctgaccctcgcgctcgatgacgcgcttggcgtcctgcgagcgcaggcgaatcagcatgaccgcgttgcgcggaccgtggatggagtgcatgtggtgctcgtagacgtcgcgcttcggatcgtagaggttgccgtcgttgacgtcctcttcgtaaagcgggaacacggtctccatggcagcagccgccaggtcctccgggcgcatgcggacgagtcgggacacgccggcggtggtgtagtgctcgccggtgacgccggagtggcgctcagcgatcgcgccggtgtcgcggccgaggtaaaccttcacgcccttgtcctggatggtccagccgtgagtccacagagtgccgtcgccgtggtagtcaagctcgtggcgcggacgccacgggttcttgatcaaaccaccgagcggagcaatgacgaccaaaccggagagcacagcagcggtgccgaggaggccctttatcgcggagcggcgccccagtgtcgaggtctcccaagcgtcgttcaaaagcgctgtggtagtacggcggtcgagctcggaggagcggccgtcgtggcggcgctgcaccgaaatctcttccgggatgaacttcttcacgtactggatgacggcgatacccagagcgccaaagctcagcatcgcggtcaggccgagaagcggggtgtacagggtgtacgtccacaagccctcgtcaccgtggaacttcggctcccacggccagaacaggtaaatgccaaggaaggcgagcgcggcgatgaccgagacaaccagccaagtgatgacgccggcggcagctgccttctcgtggggatcaccctcgaccgggaagcgctccttgcggtaggcgacggtaacgtcgtcgagctcggtgccgagtgcggcgagctccgcattgttcatgcggtcgagctcttctgtcgtgtaattcttcttcacttcactcatgaacgggatccaatccaaatagcagcggcggccacgagggtcacaccgatcatccacatcgccataccctcagagaccgggccgagaccgccgaggctccagccgcccgggctcggggtttccttggaggacttgatgaaggcgatgatgtccttcttctcgtcagcggacagctggcggtcggagaacttcggcatgttctgcgggccggtcagcatcgcctggtagatctcctgctcattggcgggatccagcacgggcgcgtacttaccggaagaaagtgcgccgccgcggccggtaaagctgtggcaggacgcgcagttcagccggaacagctcgccgccgcgcgcgacatcggcagcctggatctggccgtcgtagttcttgccgcgcagctcctccatcgcaatagagccgtcttcgttgtacaccagcgccgggccgccgccgttggctgcgacgtacgcggccagagcgagagcctgggactcggtgtagcgcgggcgcttacgctctgcctgcgcgtcgttggacatcatcggcattcggccggagttcacctggaagtacacggcgccttcgccggtaccgatcagggacgggccgcggtcctcaacgccctgcaggttcgcgccgtggcaggtgatgcaagcaacgtcgtagatgtccttgccttcctggatcatcgcctgctcgtcgcgctgggcgttggcgacctgagcgttcggcgcgagagcggaggcgaggaaacctgcaccggtcagacccaaggtaagcgctgcggcaccggcgacggtgcgctgcgtcttgcgacggctgcgcatctttttaggtgtgttttccatcttgtttccttaatagaaaagtttcagattcagttccggatcagccggtgttactggacgatgtacagcgtgatgaacacgccaacccagatgacgtcaacgaagtgccagtagtaggacgtcgccatggcggccgttgcctgcgccggggtgaacttcgacttggccacgcgcagcatcaccacaacgaacgcgatgatgccggcggtcacgtgcgccatgtggaagccggtgatgatgtagaacatcgagccgtagacgctggcctgaatggtcacgccggcgtggatcatctcggaccactcgaacgcgacgagacccaagaagatcacgccgagcagaatggtcacgccgaaccacttgcgcagcccgaacacgtctccccgctcagcggcgaaaacgcccatctgcgaagtcacagaggacgtcagcagcacgaccgtaatgatcgtgccaaagagaacattgaggtgcgcggtctggttgtcccagtcacctgcggtcaggccgttcgctcgcgacacgaagtacatcgcgaacaagccggcgaagaacatcaactcttgggcgaggaacgcaatcgtgccaacgctgacgatgtttggtcggttcagcgctgcgacgcgatcttgcggtgtcgccataccttggttagaaattgcggtcgtcacgggtgtgattatcccccctcgcgcccgtaaagtcacctcgtatacccccgaaagttttctgggtagaggggcacaacctgccactttcggcgccgccgcggtgcttgcgaaatttttcgaaactaacgggaacttttcttaccccgtttccgaccgctatcgctgcaggtcagttggcggcgcttccgcgagccgcggagaattcccgggtccaagcatccggcgcgaaggctcttcgctgcttatcgacgcccccgccagttcccaaacgtgaccaaactcacacctcagtcgcgccgtgcgcgcgctgcccccaactttcggttgacccccgcggcgccaacgggcacagacagcaaaaccccgccacctcccgcattgttgcggggaggtgacggggtgtgtccgtcggcggaggcgggccggcgggtcacggtgccgtcgaaaagcttagtgcttctcgcgcgggataccgtactgcaggttcagctgcgtggtggtccagatcaggaagaccgcaccgaaggcgatcagccacagctggtagaaggcgataccgaggcccaggaagaagaccgcgccggacatcgcgaacggccagatggagctcggggagaagaagccgagcacgccagcgccgtcctcgatctccgcctcttcccagtcctccgggacgatgtccatgcggcgctcggtgaagtccaagtagacgccgagcatgaaggacatagccgtggcaagcaccaaggcgacagcaccgatccactcgatgccgtagagccacgcgtcctcgccgacccacgaggtggcgagaatgtagaacaccgccatcagggccaagaaggtgccgattgcgtagaaaactcttgcgccagttcccattgtcgttccttctttctaaacgttcgcgttcgggtcggtggtgttctcgccgtcgcgggtgccggtgcggtcagacacgaacgggcgggtggaggttgcgtacggggcctcgccgatcgcctcgagcgcttcggagttcggcgcctgagggttagcggtgcggaaggcaacgtagtcgcggaacttctccgggctcacagcgcgaacctcgaagttcatcattgcgtggtaggtaccgcacatctcagcgcagcggccgacgaacgcgccctcgcggtcgatgcgctcaatctggaacgcgcgctgctgctggttgttctccgggtgcgcgtacacgtcgcgcttgaacaggaactccggaacccagaacgcgtggttcacgtcgccggacgcgaggcggaactcgatcgcggtctcggtcggcagcacgagaaccggaacctcttcagtggtgccgagggtttcgatctcgttgaagttcaggtaggagatgtcgccggcggaggtcccgtgaatcgggttcgcgttgtgcatgtcctccgggtcgtacttggtcgcgtcggcgattgcctggcgctcctcgtcgcggccgtcgtactgctgaccgtttgcagtgaactcgccgtcgatctctgcgtagccaaacttccagttccactggtacgcggtgacgtcgaccgcaaccttcgggtccttgttcagggccgtggtgcgcgtctgcgcctggacggtgaagaagaacagcaccatcacgatgacgatcggcacaatcgtcaggccgagctcgagtggcacgttgtactgcagctgcttcggaaactccgaggcgccctgcttctcgcgcttcttgttgttccacgcgaagatcgccacgaggaacaggccccacatgatgatgccgatgatccacgccgcgagccagacccagacccagaagttgtgcaactgcacgccctccggggtgaccggatccggccagcccataccgagtacgcgggacatcgcttccggaggagcgacctcgcagcccgtaagcgcgagccccccgaaaatgagcgaagccgcgacgccagccttcttggcaaagctgcggttcgtttgcttttccacgtgtgtttgccttcctgtccacactcttaaccatgaatgcccatggaaatacctgaacattcctacccagtcagaatagttcaaatggaatacgccgttggaattcaacagttcccccgcgacgtttgcttccgcgttgcagagtttgcgatcgcccggcaaggaaatctgggcctgaacttggatttatcccctcccccacgcttgatccgcaagtggcgctgcggccaccctggggtagttcctccgaaagttggccccctttcggggcacggcaaaaggtggacgcagcggcgacgcgcccagcgctcacgcgatgcacgagacgcggccgggcgactctattcttgagggagcaattcggcgcgtcggccgctttcgtttcagcgtcgacgcgcaccttatatataggagaggattcataccgacatgtgtggcctgttagcaatgctcaccgcgggtgcggatgcccaacgctacgcccaatccgtcgagcaagcgctcccctgcatgtaccaccgcggccccgacgcggcgggcacctggcacgacgagaacgccgtgttcgggttcaatcgcttggcaattatcgacattgagcactcgcaccaaccgctgcgctggggaccggagggcaacccggatcgctacgcgctgacgtttaacggcgagatctacaactacctcgagctgcgcgacgagctgacgaaggagggctacacgttcgccacctccggcgacggcgagcccatcgtcgtgggttaccaccactggggcgcggatgtggtcaaccacctgcgcggcatgttcgccttcgtcatttgggacacggagacgaacacgatgtttgctgcgcgcgaccagttcggcatcaagccgctgtactacgccaccacggcggccggtacggtgttcgcctcggagaagaagtcgatcctggacatggctgagcatattggtctcggcctggagcttgaccgccgagctatcgaacactacgtcgacctgcagtacgtgccggagccggagagcttgcacactgagatccggcgcgtcgagtccggctgcacggtttcgctgacgcccggcggcgaggtcgtgtccgagcgctacttcaaaccgcacttcactccgcagccggtggtaaagggcaaagagcaggacctctacgaccgcatcgcgcgcgcgctggaggacagtgtggagaagcacatgcgtgccgacgtcaccgtgggatctttcctctccggcggcatcgactccaccgcgatcgcggcgctggcgaagcgccacaacccgaacctgctcaccttcaccaccggcttcgagcgcgagggctactccgaggtcgacgtggcggcggagtccgccgctgcgatcggtgtggagcacatcgtgaagatcgtctcccccgaagagtacgcggacgcgatcccgaagatcatgtggtacctcgacgacccggtcgcggacccctccctcgtcccgctgttcttcgtcgcccaggaggcgcgcaagcacgtcaaagtcgtgctctccggcgagggcgccgacgaactcttcggtggctacaccatctacaaggagccgttgtcgctcgcgccgtttgagaagctcccctcgccgctggcaagggggctcaaccgcctcagccgggtcctgccggaaggtgtcaagggcaagagcctgcttgagcgcggcaccaccccgatcgaggaccgctactacggcaacgcgcgctcgttcaacttcgcgcagctggaacgtgtgctgccgtgggcgaagcgcgagtgggaccacagggaggtgacggcgccgatttacgcggcgtcgacaagcatggaccctgtggcgcggatgcagaacctcgacctgttcacctggatgcgcggcgacatcttggtcaaggccgacaagatgaacatggcgaactcccttgagctgcgcgtgccgttcctggataaagaggtcttcgaggtggcgcaaaccattccgttcgaccagaagatcgccggcggcaccaccaagtacgcgctgcgcaaggcgatggagcagatcgtgccgccgcacgtgctgcaccgcaagaagctcggcttcccagtgccgatgcgccactggctggccggcgacgagctctacggctgggcgcaggacacgatcaacgagtccgaaaccgacgacatcttcaacaagccgcaggtgctggagatgctgaaggagcaccgcgacggcgtgtccgaccactccaggcgcttgtggacggtgctcgcgttcatggtctggcacggcatctttgtggaagagcgcatcgatccgcagatcgagcacaaggactacccggtgaagctgtaaagagacacagaaaagcccgagcgcaatgctcgggcttttctgtgtttcgtcgctatcgcgtttagttaaacgagtcgccgcaggcgcaggcgctaccggcgttcgggttgtcgatagtgaagccctgctgctcgatcgtgtcggcgaaatcgatggtcgcgcccatcaggtacggcacgctcatgcggtcgacaacgaggcgcacgccgcccacgacgtcggccttgtcgccgtcgagctcgcggtcgtcgaagtaaagctggtagcgcaggcccgcgcagccgccgggctgcacagcgatgcgcagggagaggtcgtcgcggccctcctggtcgagcagcgccttggccttcgctgctgctgcctcggtcaagataacgccggttgcggacgtaggtgcagtcattaggttctcctcacttagctgtcgtggagttcggccccaccttactccacgtctggtagatcgtcggaaagatccaagccatgcaaccggacgaaggcgggcgatattccatctgttgaggtcgccttgtagccttgagggcgtgaaaaaaccctggcagaaatccgaacagaccacatccgggtcgaccaaggtggagctcccgtcggcaagtgagccgaagaagggggctggggtggttgaggggggcgtcgacaagcgtgatgcccctgagcttccgaagggctacacgccgccgaagggccgcccgacgccgaagcgccacgaccaggaggtcaagcgcggcgtggtgcgcgacccgaacgccaagactccggagcaggcgcggcagcagcgcaaagagctcaagaagaccatgagcaaggacgagtggaaggcgtacaagaagactgagcgcgacgagcggcgcgaaagcaaccgcaaaattcaggagcgcatcgacgctggcgacgagcgctacctgcagcagcgcgaccaaggcgaggtgcgccgctacgtgcgcgactgggtcgatgcccgccgcttcttcaacaactacgcgttcccgttcgcgatggtgctgctcgcggtcatgttcttcggtacgttcttgccccgcgtcgcagcggtgttgagtgtggtggcgatgctgttcattctcaccatcctgattgagatgttcatcatcggtcgtcgcgccaatgctgcggtacgcaagcgtttcccagacaccaccgacaccggcttcggcctcggcatgtacgcgttcagccgcgcttcccagccgcgcagctggcgatcgcccaagccgcaggtcgccgtcggcgccaaggtgtaggagtgcgaccgtgtccgtgacgtttccgcccgttgcctcccccaacgagtcgctgcggcgcgaggtgatcgacatgctcgactcctcaaccgccggccgcgcgctcggcaggctcgggtccatcggcgcgtgggtcgccggcgtgcaggactcaccgcagccgcagccgttcggccgcgcgcgtgctgtggttgtcgcaggcaatcacggcgttgctcagcggggggtgtccgcgtggaccacggacgcggcccgcgcgcaggtcgaagagatagaggcgggcggcggcgcggtcaacgcggcggcgcgcctcgcgggcgcgggtgtacgcctcatcacggactacctggactcccccaccggattcatcgacgtcgagcccgctatgacccccgaggcgtgcgaagctgcgttcgaagctggcatcgcggtcgccgaccaggaaatcgacgcgggcacagacctcatcgtcccaggcgacatcggggtggccagcaccacggtggccgcagcgctgtacggcgtattcacccgcaccgagccggtcagcgccatcggccgcggctccggcatcaacgacgaggtgtggaaagtcaaggtcgaagcgatccgcgacgccatgttccgcgtccgcaccttccgagacgatgaagcgcgcgtcatcgcggagatcggcggccccgacgtcgcgttcctcgtggggctcatcgcgcagtcggccgcgcgtaggacgccgctgcttatcgacggagcgttgaccaccaccgccgccctcaccgccgagcgcatggcccctggcacgcgccagtggcttatcgcaggccaggtcaccccggaaccctgccacgtgggcagcgcccaagcgctgggccttacccccgttttggcgctcgacgccaccgcaggccaaggcgtcggagcgctcgcagcgctaccgacgatcaacctggccgcggaactcgtggcggacctggccagctagcggctacaccaggcggtagttccagccgtgggtgtcttccacggcgccgttttggatgccgcgcagacgctcgcgcagctccatcgacaccggtccggcctcgttgccgttcacagtgaactcgccctcagccgacagcacacgcccgaccggcgtgatcacggccgccgtgccgcaggccagggtctcactgaagcggccgctctctgcaccgtcgcgccactcgtccacggtgatgcggcgctcctcggtggcgtaaccgagatcctcggcgacctgcagcaacgacttgcgggtgatgcctgcgagcagcgagccggacagcgccggggtgaccagcttgacctcgtcggcgagcttctcaacgaacatgaggttcatgccgcccatttcctcgatgtacttgcgctcgatcgcgtccagccacacaacttggtcgcagcctttctgctccgcttccttctgagcgagcaggctggccgcgtagttgccggcgaacttcgcgtcgccggtgccgccgggagccgcgcggacatactcctcggagatccacacactcaccggcttcacgccgcccttgaagtaggcgccggccggcgaggcgatgacgtagtacgtgtaggagctgctcggcttcacaccgagggtctcctcggtggaaatcatgaacgggcgcaggtacagcgccgcctcgccgccggcttcggggacccagtcctggtcgatctccaccagctggcgcagcgactcgatgaacagctcctcgggcagctccggcatagccaggcggtgcgccgagtgctggaagcgcgcggcgttctggtcggggcggaacgtggtgatagtgccgtcttcgtggcggtacgccttcaagccctcgaagatcgcttgcccgtagtgcacaacgctggtggccgggcccagctcaatcggtccgaacgggcgcacctgcgcgttgtgccagccttccccctcggtccattcgatggagaccatgtggtcggtgaacttctggccgaacgccgggtcggcgaggatctcgcggcgctcctcgtcggacgccgggtgctcgttgcgggttacgttgaattccgttgctgccatggtttcaccctactcggtagcgccgagagccatatgtaggctcggagcatggctatcaacactttgctccccgctcgcggcgcgtccgcgacggtggatttctccgacaccgcccccgaaaacgcgacgctgatcgtgcccgtctcccggggcgaggacgggctcgaggtcccggtcacccgcttcgcggctggaggcctgctcgaggctctttcagctgtcggcgccaccggcagtgcgggggaaacggtgcggctgcttgtcgacggccgcgtgtacctcaccaccggcctcggcaaagacatcaccgacgaagccgtgcgccgcgcgtacggtgccgcggcgcgctcgctcaaggcaggcgcagtggcggcagcctcctgcgagttcggtgtcgccgccgttgctgagggccttcttctcggctcctacgcctaccaggggctgaagtcgaaagacgaggacgacgctgaggaaggctcccccgccatcacagtcgtgggcgacgcggagcaccgcgccgagtttgagcgcgccgcaatcatcgccgactcggttaacctcgcgcgcgacctggtcaacacccccggcaacttcctcgctccagccgcctacgcggacgcgatcaagcacgcggccgcgccgtttgggcttgaagtcgaggacttcggcgttgacgagctgcgcgcccagggcttcgggggcatcctcgcggttggggctggctccgcaaacgctccccacttggtgcacgttgggtggcgcccggagggcgcgcagaagcgtgttgccctggtcggtaaaggcatcaccttcgacacaggcggcatttcgctcaagcccgccgcaaagatggaggagatgatttcggacatgggcggctccgcggcgcagctcggcgccgtgatcgcggcggctcgcctgaacctgccggtcgcggtggacgcgtggctgccgctggcggagaacatgccgtccggctcggcaacgcgcccgggcgacgtgatcacccactacggcggtaccacctccgaggtgctcaacaccgacgccgagggccgcctcgtgcttgccgacgccatcgcccgtgcctgcgaggacaccggcgaaggacaacccgactacctcattgaaaccgcgactctgaccggcgcgcagctggtggcgctgggcacccgcactgcgggtgtgatgggcaccgacgagttccgcgacagcgtcgccgcgaccggccgcgaggtcggcgagccggcctgggcgatgccgttgctcgaggagcagaacgacgagctcaaatccccggtcgccgacatccgcaacacgcacaacgcgcgaaccggcggcatgctgttcgcgggcctctacctttcgcgcttcgtgccggaaggcacccagtgggtacacatcgacatcgccgggcccgcctggaacggcggcaaggcctacggctacacgccggcgcgggcgacgggtgcgccggtgcgcacaattgtggcgacgctgacccagctcgccgaagcgtaaagagcttctactcgtacgggttttcgccgcgctcgaacttggcgcggcgttccttctgctcggctcgcttgcgcaggatgcgctcttgctcgatgcgtttgcgcatgcggtccgggtacccggtctcctcaacgtcgtaaagcgcaatgcccaactgcgaccgaaccgcatcgatgcccttcggtcccccgatacgccggcgggtgtagttgcccttctcgtccaccagcacgaccgacatctcgttgaccatcgtctctggctccacgaacccctcaacaaacacccgaccctgcacccattggcgcaggtaagcggcatcgtcatcgcggatggtctcccctggggcgcgcggaggggcgaactgcgaattccgtttgcctttgccgaagagattgaacacggcagacatattacttcagccccgtattcaaacaacgggcgcgagcgttagcgggtattctcgggggacgtataaccaatcaattttgatgaggagacttgagaaaacatggcgcactcagttgagatgcccgagctgggcgagtcggtaaccgaaggcacgatcaccacctggctgaaggaagtcggcgacaccgtcgaggtcgacgagccgctgctcgaggtctccaccgacaaggtcgacaccgaaattccgtcccctgtcgcaggcgtcatccttgagatcaaggctgaggaagacgacaccgtcgaggttggcgacgtgatcgtcattatcggcgaggaaggcgaagaggccgcttcctcctcctcggacgacgaggacaccgcagacgctgaggaaaaggctgacgctgaggagtccaagaaggtcgaggacaccgacgaggacaccaagaagaaggtggagaagtccgccaagggttcctcctccgcttccgccaccgacgttgagatgcctgagctcggcgaatccgtcaccgagggcacgatcaccacatggctgaaggaagtcggcgacaccgtcgaggtcgacgagccgctgctcgaggtctccaccgacaaggtcgacaccgagatcccatccccggttgccggcacgctcatcgaaatcctcgctgaagaggacgacaccgtcgaggttggcgacgttatcgcccgcattggcgacgccgatgcagctgcgtccggcgacgaggacgacagcgacgacgaagagaaccgcggcgaggacaacgtcgccgacgaggacgaggaagtcaccgagtccaactccgctgagggtgagggcaccaacccagaggacgccccgaagaagtccgaggagaagtcctcctccaagaacaagaagggctccggcgagtccaccaccgtcgagatgccggagctcggcgagtctgtcaccgagggcaccatcaccacctggctgaagtcggtcggcgacatggtcgaggttgatgagccgctgctcgaggtctccaccgataaggtcgacaccgagatcccgtccccggtcgagggcaccatcctcgagatcctcgccgaagaggacgacaccgtcgaggtcggccaggcaatcgtggtgatcggcgacgctgaggcggccgccgcagacgacgctgacactgccgacgaggcggaagaggctgaggagccgaagaaggaagaggctccgaaggagaaggagaccgaggaagctgaggagccgaaggctgagaagggctccgcagcgaacgagcgttccgagaaggacgccaagaagtccgaggacgacaccaagccgggttccaacgcttccgagaagctggagaaccgcggcgacaaggtaccgtacgtcaccccgctggtgcgcaagctggccgagaagcacggcgttgacctgaactccatcgagggcaccggcgttggtggccgcatccgcaagcaggacgtgctcgcagccgctgagggcaccggcgctgagggcggcaaggctgcagacgccactgaggccaagaccgagagccaggcgccgaagggcgagcgcgccaactggtccaccaagtccgtggacccggcgaagcaggagctgatcggcaccacccagaaggtcaaccgcatccgcgagatcaccgccgcgaagatggtcgagtcgctgcagaccactgcccagctgacccacgtgcaagaagtcgacgtcacccgcgtcgccgagctgcgcaagaaggtcaagccggccttcgtggacaagcacggcgcgaacatcacttacctggcgttctttatcaaggccaccgctgaggcgctcgtttcccacccgaacgtcaacgcgtcctacaacgcggacgagaagacgatcacctaccacgaggacgtcaacatcggcatcgccgtggacaccccgcagggcctgcttgtgccggtgattaagaaggttcaggacatgaacctagcggacattgccaaggcgatcgccgacctggctgagcgcgcgcgcaacaagaagctgcgcccggacgacctttccggcgcaaccttcacggtgaccaacatcggttccgagggcgccctgctggataccccggtgctcaccccgccgcaggccggcatcctgggcaccgccgcgattgagaagcgcccggtcatcgtgaccgaggacggcatcgactcgatcgcaatccgccagatgtgctacctgccgttcacctacgatcaccagttgatcgacggtgcagatgcaggacgtttcgtcaccacgatcaaggaccgcatcgaggcgggcaacttcgaggacgacttgggcctctaaccccccacttgtagccggttaacccggcgccggatgcttccggcgccgggtttttcgtgcgcaaatgccgcttggtgaccgagctgaagcgttacactgatccgtggtcactcgcctctatggataaggagcttcagttggattacatctcccgtcatgtcggcccaaaccaggacgagcggcagaaaatgctcgacattttggggtacgagagcatcgatgcgctgattgcggctgcggtgccaggcgggatcttgatggacggcgcgctcgacttgccggaagccttgacggagtacgaggcgcaggcccggttgcgtgagctcgcggataagaaccgcgtcctgcgcgccttccacggccaggggttcaactccacactcaccccgccggtgatccgccgcggcgtggtggaggacgctggctggtacaccgcttacaccccgtaccaagctgaaatctcccaaggccgccttgaggcgctgttgaacttccagacaatggtgcaggacctcaccggtctcgacatcgcgaacgcctcgttgctcgacgaggcttccgccgcagcggaggcagtcggcctgatgtcgcgggtggtgaagaagggccgccgcgtgctactggattcgcgcctgcacccccaagtggtcaacgtcgccgcggagcgcgcccgcgccatcgatctggaggtggaggtcaccgaccttacccaaagcgttgtcggcgaagacttggtcggcgctgtgttcgcgtacccgggtaccgagggcgacatcgctgatccccgccccgtcatcgaggcgattcacgagcgcggcggtctcgtcgcaatcgacgccgacatcctcgcgctgacgctgcttgaatcgccgggtgagctcggcgccgatatcgccatcggcactacccagcgcttcggtgtgccgttgttctacggcggcccgcacgcggcatacatggcagtcaaagagaagctgcagcgccagctgccgggccgtcttgtcggcgtgtccaaggacgccgaaggctaccccgcctaccgcctcgccctgcagacgcgtgagcagcacatccgccgcgagcgcgccacctccaacatctgcaccgcgcaggcgctgctcgcggtcacggcgtcgatgtacgccgtctaccacggcccgcaagggctgaccgagatcgcccgcgcagtgcaccagcgcgcgaccgattttgctgcggcgcttgagaaggcgggtgtgaaggtcaagcactccgagttcttcgacactgtggcggttgaagttggggatgttgaagggtgcgtcggcaagcttgctcaagccggctacttggtgcgcgccatcgatgcgcagaccgtgggtgtttccttcggcgaggacaccacggacgccgatgttgccacattgctcgagggcttcggcgcgtctgccggggcgaccggcgacagccgcattccggaggagcttgcccgcaccaccgatttcctcacccacgagacgttcaaccgcatccactccgagacgcagatgatgcgctacatccgggagctcggcgacaaggacctcgcgctggaccgcaccatgatcccgctgggctcctgcaccatgaagctcaaccccaccgcggggctcgaggcgatcacctggccggggttcgccaacgtgcacccgttcaccccggacgagtacaccgagggctggcgcgagctgattgaggagatccgctcctggctagttgaggtcaccggctacgccgaggtgtcggtacagccgaactcgggcgcgaccggcgagctggcgggccttctggccatccgccgctaccacgtggcaaacggtgacacggagcgcgatatctgcctgatcccggcttccgcccacggcaccaacgcggcgtctgccaccctggcgaacctgcgcgtagtggtggtgaaaaccgccgacgacggatcgatcgacatcgcggacctggacgagaagctggccaagcacgccgatcacgtcgccgcgatcatgctcacttacccctccacgcacggcgtgtacgagaccgatgtgcgcacggtgtgcgagaaggtgcacgcggcgggcggccaggtctacatcgacggcgcgaacatgaacgcgctgaccggcatcgcccggccgggcgacttcggcggcgacgtgagccacctcaacctgcacaagaccttcaccatcccgcacggcggcggcggcccgggtgtgggcccgatcggcgtggcggagcacttgattcccttcctgccgtcgaacccgaacgtgccgctcgagcaggccgcgggcgagatcgacattcgcgaaggcgtgccggtagcctccacgctgtacggctcggcgggtgtgctgccgatctcctggtcctacatcgcgatgtcgggcgctgccgggctgcgcgcagcaaccgagcacgctgtgctgaacgccaactacatcgcgcgttcgctgcgcgactcgttcccgattctctacaccggcaacgaggagctggtgggccacgagtgcatcctggacttgcgcggcatcaccgagcagtccggcgtgaccgcggccgatgtggccaagcgcctgatcgactacggcttccacgcccccacgctggctttccccgtggcgggcacgcttatggtggagccgaccgagtcggaggacttggaggagttggaccgcttcatcgaggcgatgcgctccatccgcgccgagattcaggagattatcgacggccgcgtggactacgagtcctccgtcgtccacaacgcgccgttcaccgcgcagagcgtgatccgcaacgagtggccgtacgagttcacccgcgagcaagcggcctaccccgtcgacacgcttgtgcaccgcaagtacttcccgccggtgcgccgcattgacgaggcgttcggcgaccgcaacctgcagtgcgcctgcccgccgccggaggcgttcgacatcacccccgaagtagtcgaggacgtcgacgtcgagatctcagagaagaacgcgaagtactagataagcgaaggagcacccatgccacagaccccacttcaccaaacacacgaggcgctcggcgcccagttcaccgacttcggcggctggacgatgccgctgaagtacggctccgagctggaggaacaccgcgccgtgcgaaccggcgtcggtattttcgacctctcccacatgggcgagatcgacgtgatgggccccgacgccgccgcgtttttggactacgcgctgatctccaacttctcctcgctcaaggagggcaaggcgaagtactccatgatcgttggcgaggacggcggcatcctggacgacctgatcacctaccgcttcggcgagcaccacttcatggtcgtgcccaacgctgccaacaccgacacagtgtgggaagcgttccaggcgcgcaagggcgacttcaacgtcgagctgcgcaacgattcgcagaccgtggcgctcgttgcggtccagggtccaggttcgctcgaggtgttggggcagttgcttgccgacgacccgtcgaacctctcctactattccggagcatggaacacgcttcgctccggcggcgaggacatcgaggtcttcgtcgcccgcacgggctacaccggcgaggacggcttcgagctgttctgcatgttcgatgacgcccagaaggtgtgggacgccgtgattgaccacggcaccccgtgtgggttggctgcgcgtgattcgctgcgtcttgaagcatcaatgcccctctacggccacgagctgaccaccggaatcacccccgtcgaggcggggatgggacgcgcgtacgcgaagaaggaggcggacttcgtgggcaagcaagccctcacgggccgcgagccgtcgatagtcatcgcgggcctgacttctaccgcgcgccgcgcagcccgcgagggcgcggagattttcctgcccggctcggacgacaagatcggcgtggtcacctccggccagccctcgcctaccctgggccacccggtggcgctggcgcacctcgatcccgcacacgcggagatcggaactgacgtagagattgacatccgcgggcgccgctacccgtttaccattactgcaaccccgttttacaagcgaaaggacgcgtaacgcaccatggcactgaaccaggactacttctactccgaggaccacgagtggatcaacgcgaccccggacaccgctgtcggccagaaggtccgcgtgggcatcaccaacgtggcagctgaccgcctgggcgaggttgtcttcgctgagctgccggccgtcggcgacaccgtgactgcgggcgagacctgcggcgagatcgagtccacgaagagcgtctccgacctctactccccagtcaccggcactgtcaccgcggtgaacgaggacatcgacggcgcctacgaggcgatcaacaacgacccgttcggcgccggctggctcttcgaggtcgaggttgaggaggtcggcccgctgctcagcgccggcgagtacgccgaagcgaacggcatcgaggcgtaaggctctcgcaaaacatcatgaccgctccccgcgacccgttcttccccgccgacaagtccatccgcgcctccgcggacccagttgacgtgcgcaacttgggtgtcgtggactaccaacaggcgtgggacatgcaggcggaactcgcggcgaagcgggcagccggcgagatcggcgacaccatcttagtgctcgagcacccgagcacgttcacggccggcaaacgcacccagccggaggacatgccagacgagtcctacccggtccccgtggtcgccgtcgaccgcggcggccgcatcacctggcacggcgagggccagctggtggtctacccgattatcaaactcgccgagccggtggacgtcgtcgactacgtccgccgcctcgaagaggcgctgattgaggcggttcgcatcgcaggagtggaaaccgccgggcgcattgacggccgctccggcgtgtgggtgcccgctcaaacccgcgcggccgacccgtccgcctccacgcgcgaccgcaaggtcgcggctcttggcatccgcatcacccgcggcgtgaccatgcacgggctcagcctcaactgcaacaacaccctcgagcactactcccacatcgtcgcctgcggcatcgacgacgccgatgtgaccacgatgagcttggagctcggccgcgacgtcaccccaagcgacatggagcagttgcttatcgacgccctcctgcgcgccctaagcggcgagctcgtcgtcgcagaccattccttcggctccgcccccgatccgtccaagggcctgcgcaagcgccgtccctgacgtgtcgcttgacacatccactacggtgaaggtgtgactgttgcacctgaaggccgcaagatgttgcgcattgagaagcgaaatgcgcagaccccaatcgagtcgaaaccgcggtggatccgcaacgcggtgaaaacaggtcccgagtacgaggacatgaagcaaaaggtcaagggtgcgtccctgcacaccgtgtgccaggaggcaggctgccccaacatccacgagtgctgggagtcccgcgaggccacgttcctgatcggcggggcgaactgctcccgccgctgcgacttctgccagatcaactccgcgaagccggagccgctcgaccgtgaggagccgcagcgcgtggccgagtcggtccgcgagatgaacctgaactactccaccatcaccggtgtgacccgcgacgacctcgaggacgagggcgcgtggctctacgccgaggtggtgcgcaaaatccacgaactcaacccgcacaccggcgtggagaacctgaccccggacttctccggcaagccggatcttttggccgaggtctttgaggctcgccccgaggtgttcgcccacaacgtggaaactgtgccgcgcattttcaagcgcatccgtccggccttccgctacgagcgctcgctcgatgtgatccgccaggcccgcgatttcggactcatcaccaagtcgaacctgatcctcggcatgggcgagacccaggacgaggtcatggaggccctccacgacctcgtcgacgccggcaccgacatcatcacgatcacccagtacctgcgcccgggcccgatgtaccacccgatcgagcgctgggtgaagccggaagagttcatcgagtaccgcgacgccgcgtacgagatgggcttcggcgccgtcatgtctggcccgctggtccgctcctcctaccgcgcaggcaagctttacgtcgaggcgatggagcaccgcggtctcgaactcccggaaaacctgaagcacttggcgcagacgtcgcaaggcgatactgcccaagaggcctccaccctgctggcaaagtacggcgagagcgccgaccacccggttaccactcgttagctttggcagccggcgcgctgtgacctagagtatttcccatggccaaggacgcgaaggcacaagcccagaagtcagcagcgaaggcggcgcagaaggctgccaagaaggagcagcgacaagcgaagcgcgagaaggggaaggccacccgcggccagatccgccaggcgttttccctgcagcgcaagcgcgacaagaagctcatcccgcttatggtggcctctgttctcgggttgggtctgctgttcttcctcatcggcctgcttttcaacggccagtggttcatgctggtgctgggcctgctcgcgggcgcggttttggcgatgttcatcttctcccgccgcctcgaaggctcgatgtacgacgaggtgggcgatacccccggcgccgcgggatggacgctggagaacatgcgcaacaccatgggcatcgtgtggctgacgaagaccgccgttcaggcgaccccgcagatggacacagtccaccgagtcgtgggcaacccgggtgtcgtgctcgtcggcgaaggcgatccgaagcgcctcaagcaactcatgaacaaggagcacaagcgcactgaacgcctgctcgccggcgtgccggtctacgaggtctacgccggtgagggcgaaggccaggtacgcgtccgcgacctgcagaagcaccttctgaagctgccgaagaactaccagaaggaccaggtctacgggatgtcggcaaagcttgaggccatggacaaccgaacccgcggcggcaacatgccgggcctgcccggcggtccgatgccacggcaggcgcagaacatggcgggcatgaaccgcaagatgcgccgcatgcagcagcgccagggcggcaagtagcgcctcctcccccaccgcgcccgtggctgaccagacagatttcgccgccgaagcaaacacgacgcttcgattcggcatgatgctgctcgccgcaggtgcgtccggttaccgggtgatccgcggcatgaaacgctgcgcgcgctcgctcgggttcgacgaagcggacgtgctcgtcgggttcaactccatcagcgctaccttccaccacggagcggatttccgcaccgtggtagccgacgttccgctgccgggtgttaacgccagccgcatcgaggcactcgagactgtagcccactccatgatgcagagcccgcactcggcgcaggagatcaacgctgccctcgatgacatcgagcgcatccccaccccccgctggcccctgtggttagccatgatcgccgccgggctcgcgtgcgccgggttcgccgtgattaaccagttcggctacgacgcggcgtgcctcgtgtttatcgccgccgccgtcggccactacgtgcgtgtgaagttgcaccacacgcacttgaacgtcctcggggtcatcggatgcagcgcgtttaccacctcggtgctctacctcatcttggcgcattttgcgcccaccgcgacggatctttccgccggattcatcgccgcagtgctctttctcatccccggttttccgctcttctcgtcgttcgtggatctggcccgcttcgacttcacctcaggcatcccccggctgtttttcgccctcgagatcatcaccgtcatcatgctcaccgtcgtcgtggtggcgatgctctccggcaccccgcagccggtgcccgcgtcgcgcgagccgagtttggagtacttcgtctcggggggcatcgcctccttcgtggccgtcgggtgcttcgcgctgctgttcaactcctcgcgccgcatggcgctcatcgccgcgtccgtcggtttcatggcgaacttgggccgcctcgccctgctgacacaggacatcgcgccgtttttggcggccttcgtcgcggcgctgttcatcggcctcttcggttcccagctcggtcgcctcgccaccatcccgcgtgtgaccgtgaccatcccggcgtctgtggtgatgattccgggaaccacgatctacacggctgtgcacgggttcgcgcagggcaacacgccggacgcgctctacgcgtttaccgacgttgccctcaccgtcttgttcatcgccgcagggctgactatcgcccggatgctgactgaccaggcttgggctttcaaccggcacatcgactttcacaagcccctcgacggggaggcagtgccgattaaccgttgatgacggtggtgttcgttgcccggtcgtgcatgccgcggccgtccgcgtccaccatcgcggcgggcaaaatgaacccggtcaagatcgtgcgcaccgcggcccgccaaaagcccaccggtgcttccgcgtctacgcgagccacgcccatgcgcagcagcgccatgccgggggtgcgcgcaaacagccagccagtgaggatgcccatcgcgacccagatcaggtaggtcagcgtcgccgtgtcgccgaggcggtcggtgttcgcggtcagaagcgtcgcaacagcgaggcagagaagccagtcaatcaacacagctgccatgcggcgcgcgacagacgcctgcgatccaggaccagttctgggcataccaaagaattcgcccgggtactccggcagaccgggctccccgctgaattggttcggaatttccggtccttcgcgccagcttcccctcttttcagccatgcgatgtagcgtagctggctgcatcgattccgatagaatcggtgacgttcaattttcgttctaaggagaggcacgtggccttcgagtccatcgacgacgtacagaaattcatcaccgacgaagacgtggaattcattgatgtgaggttcaccgacgtaccgggtattgaacaccacttctctattccggcgtccgagttcggtgaggaagagatggaagaaggcctggcgttcgacggctcctccatccgcggctttaccaccatcgaggaatccgacatggtgcttatgccggacttggcgacggccaagctagacctgttccgctccacgaagacgctgaacctcaagttcttcgtcaacgacccgttcacccacgagccgttcagccgcgacccgcgcaacgtcgcccgcaaggcagagcagtacctcgcctccaccggcatcgccgacacctgcagcttcggcgcggaagcggagttctacctcttcgactccatccgctacgaggtcgaaccccaccgctccttcttcgagatcgatgccgaggaaggctggtggaaccgcggcaaagagaccgacatcgacggcggcccgaacttgggctacaagaaccgcgagaagggcggctacttccccgtcgcgccgcacgacaagacggtcgaggtgcgcgacgcgatggtgcacaacctggcccgctccggcttcacggttgagcgcttccaccgcgaagtgggtaacggtggccagcaggagatcaactaccgcttcaacacgctgctgcacgccgcagatgacctgcaggacttcaagtacatcgtgaagaacaccgccctgcagttcggcaaaaccgccacgtttatgccgaaaccgctcgccggtgacaacggctccggcatgcacgcccaccagtcgctgtggaaggacggcgagccactgttttacgacgagtccggctacggcggtctttccgacatcgcccgctggtacatcggcggcatcctcgagcacgccggcgccgtgctggcgttcacgaacccgacgctcaactcctaccaccgcctggtaccgggcttcgaggccccgatcaacctcgtctactcgcagcgcaaccgctccgcagccatccgcatcccgatcaccggtacgaacccgaaggccaagcgcatcgagttccgcgctccggatccgtcgggcaacccgtacttcggcttcgccgcgatgatgatggctggtctcgacggcgtgaagaaccgcatcgagccgcacgccccggtggacaaggacctttacgagctgccgccggaagaggccaaggaaatcccgcaggcaccgacgtccctcgaggcatccctcgcggctctggaagcggaccacgacttcctgaccgaaggcgacgtcttcaccgacgacctgatcgagacctacgtgcgcctcaagtacgacaacgagatcgccccggcgcgcctgcgcccgacgccgctcgagttcgagatgtacttcgactgctaaaacgcgcggagctcggcgtgtcggcgtggctgggccgctcgcaacgcggctcagacgccgagcgccgtcgagttgacgagcctattatcgggttatgcatgaagaagtcgtcagttcttccccagggaaccacccaaacgaaagcgctgagaatgcggaaacccggcacagtgctgagcgacctggcagcgaaagcgccgacgtcgacaatgatgtcgtttctcaccccactgggttgagttggaaagacgccgtgcgttacgtgctgaaggtgagcggcggcccgatgagcaccaccgcaatctccgaccgcattagcgagtggaacctacgcagcagccagatttccaacccggtgcaagcggtcaacaacgcgctgcgtattcagctcaaggctgaggtagagcaggaccaggatagtaagtaccgccttacggacgaggctgcggccgcagtgcgtctagaggagttctacaacaccccgtcgacgaacactgccattgcggaagacgcggaggtctcgcgcgagatcgccaaagagaacagcgaccgtatcatccgctcattcgggatcttctggagccgatccgacgtaatttggaaagcgagccagggcagctcgcgcaccgctacccgaatgctgggcagatcgaacgacagggcaccggagatcgattttggtgatcagcccggtatctacattctgtacaacggcgagaagccgatctacgtgggacaagcgaaagacgggcgacttagcgacaggatcggcgaccacacgcgcgaccgcttgaagtcccgctgggatcggttctcgtggtttggtctgaagtcagtggacccgaacgcatcaaggcttgaaccgttgctcggctacgaaagcgacccgacggttatggtgaaacagctcatcgacgcgttcgaggcgctgcttatcgagggcatggaaccagcacagaaccgacgtggcggcaaccagcttaaagacatcgaatatctgcaggttcgcgacccaaacctcgatcagtttcaagatcaagcggaggccttcgcccgcttcatgcgattagtgatcgattaggacgacctagactcgccacgttgccccacactccaaagggcgtccgtaggagggcgtcagccggagggcggaagtgcgggttcttgaacgtatatccgccctcctacggacgccctttgggtgacttgcactctgcgggcgcgtgtgggcgggtggtgtggaggtgggttgaggggttgaaggggcgtcgtgaagcaaaagaaactaccatattcgccgtgactgaacgttttcgcggattgcctgcgccgggtcctgcgtggggcggcagcctcatgggtacctccatcgttgcccgtctgttggtcgaggaagacatgatggtggcggccggggtgttcgccgtcatctcctgcgccatcatggtggcgctaacagttgggtttttgagataccgggagccgtcgttcgagcgcgccaccgttgcggagtggtcaatgtacttcatcggcatcttggcgcttggtgcggcgctgtccgggttgacggacaacagcgtgtaccgcctcgttggtttttggattggcgctccagtcaccgttatcacgtgggtgatccagctgacgcgctttgagggcgacccgaaattcacgtggggtctgccacttgtcgggccgatgatctcagcctcggttgctgggtggctctcgcgcgactacggccacatctatcacgtgatgggcacgacactgttcttcatgtcgctgctcaccgcagtgccaacgtttatccgcgtgtactgggctgcttggcacggcagggtcgatttgtcgggtccgaagtctgcgacagcgtgggtgcctctgggcgttatcgggcaatccaccaccgcgctgcagattttattcccgggccgcgtttccatctactacggctatgtggcgctcatcctggcgattccgcttgcgatctacgcgatgatcacgttctacccgaacgtggcgcgctgggtggactactcccccgcgtggtggtcgtgcacgttcccgccgggaacggtgagcatgggcggccaccaagtggcgctggtcaacggttctaagtggcttgatgcggtcgcgctgagcatcccggtcctgctgattatccactggacgctgtgctcgagccggttcgtcacctgggtgctggaagagcggaaaacgggtgccgcgagttagttaggtaaggctagaaaaaggtaccttaccctgcgcaaagttaccctcggcttgcttgctcggggtcgcgttggccgtcacaatgtgcggcatggaaactcgacagtcggcgccatccggcactgcgagcgtcggcgagaagctcaaccgcctccgcgccgcggtgctgggcgcgaacgacggcattgtctccaccgcggcggtgctcgtcggtgtcgcaggcgccacgaacgacacgaaggcgatcgccacggcgggcctggcggcggtagtcggcggtgcggtgtcgatggcgcttggtgagtatgtgtcggtgtcgtcgcaaagagactccgaggaaacaatgggcgtggaagcccacgagcgggtgaacccgtggtcggcaggagtcgcttcgttcttcgcgttcctgctgggggcaatgctgcctttcggcgcggcgatgctcgcccccgcctcgtggcggattggcgcaatctttgcgctgaccttggtttcgctcgcgctcacgggtgcgctcagcgccaagctcggcaacgcgaagatgggtcgcagcgttatgcgaatcgtcatcggtggatcgctcgccttggcggcgacgttcatcgttgggtcgctcttcggccaaagcgtgtgacacacagctgggttagactcactttcgttcctgtccgcgctgactacagcaactgcgccccgcgaaaggtagccatgacctcgcccaacttcggtggcccgcacggccccggtcccagcggaaacaactacagcaacccccaattcggcggttccacagcctggaatggcggcgggcaaccgggtcagccggggcagccacagtggggcgtaaacttccagcacccgcagcagccgcagcaggcgcctgcagcgaagcgcaacctagatctcgggtggcccgcgtgggcgtacctcggcctgacgctgcttacttttgtcggcagcttcttcaccgtggtgacgtgggcggccggcctcgagggcatcggctccgccggcgtgagctggaactggtggggcgccttctcatacgagggcaccgggctcggatcgatggccaccgagtacatccccgccgagctcggttacgacagcggcatggtggtttccaccgtcgccgtcctgctccttcttgccgctacgtgcgttctgatgttcctcggacgcatccgcccgggcgcgattctaggcatcgtcgcctccgcggcgcagctggtgattgtgatcgtctccttcgccgagatcgacaccaacttcggcatgcacatgggtctgggctggttcatctggctggtcgcggcgctggctggcctggcgatctccatttacctcctcgccaccggccgcggcaagaagatcgctgctccgcagaacccgtacgcgaacccgggcgcaccggcccaaccggcgccacagcagtggggtcagcagtacccgaaccagcagggccagcagggccagtggggccaggggcattagggcagtgaagcactccaaaataggcgcggccgcggtggtcgccctcgcactaagcacgggcgcctgcggcggcggggcgggcagcgccggacagaccgcgcttgaggcgccgacgtttgtcacgctggataaccttcacggagctgacgtggagatcacgaagcgccaaccgctggtgatcccggtcggctacgaccaggacgcctcggcgtggacgagcggcggggtggacgacgagacagtggctacgttcgtgccgggatcgaaagacgggaacacggaaacgaacccggggtttcacgccgtgggcagcggcacgacgggcgcgcacctgactaacccggcgaccggcgaggacatcgagttcactatcacggtgaagtaggccgacagtaacccagagctaccgcgcgagattcagatccacctcgacgccgccgacgcgtcctcgcgaggtgaattgccagaccgcgggctcgggcatgccgagcttcttcggccagtcggatgaagacggcagctggtctcgaaacgggtcggttgtggggttggtgccccagtgggcaagccagagtttgccgaaggcgtgggcgtcggcaagcaacatgtgcccccgccagtaccgtgcggtggtgtagatcccctcgaccgcaacccccgcggtggtcaaggcgcggtgggctgcgctgacgtctgcgagcgtgagccccgcgggcgattcgacgtcgatccagacaggcaggcgcgcgtcccccatcacctcaagcgctgcgctgatttgcttgtcgacgccctccccctcccccggagccctcaaatagtggtacgcggcgacctcgaccctggccgcccgcgcgttggccaggtgcgcggcgaaggcgtggtcgcggtaagttccgtcggtcgtgcgcaggatggcgaagtcgaagccggtgaagtcgaattcgcgctggtgctcggagacgtcgacgccgagcctcatcgtttagtgaaacccatccgcggtgcgaaaccggcggggtgcttgcgctgggcggcggcgtcgccgatgaccaagcgccacttcgggtccgtgaccggcatggtggagatcgggaaccacccgacgtcggtggattcgtcatcgccgacaactggtgccgcggccgggtccaccggctccatgcgcagctgaatggacatgtagctggctttatcgccgttgctgtgggtgacggggccgaccgcgccgacgcccaagatcgccgctgggacgacctccacaccggtctcctcgcgcacctcgcgcacggccgcttcgtgggcctcttcgcccgggtcggcgatgccggtcaccggtgtccactcgccgttgtcggtgcgcttgaccagcagcacctccggcacggcccaggcggaattgtccgtggagtcgcgcaaaacgacggccgcaacgctgggcagccacatgaggtcggtgccgatcttctcccgcgtcgccgcgatgaattctgggattggcatgctgcgtccttcctggtccttcctgcgccgggtgcgtgtggtgttcgagtgtagacttccatgcatcatgagcaccctgcacaccccaacgagcgaaccggagctgcccgcggagaccgcgcctggcaccgcacccgcagcgcccaagcgcagcttgatcgcccggctgcccggtccggtgtttgtggtcgggtacggggcgctgctcatcgccgtggtggtcgcggtagcgatgttcgcaagctacgagtccggctcgggcaccgggccgctcacgtcggccgccgcgaaagagcaggaaccgatgcaaccgtggaacccggcaccgcgcgacgaggacaacgtccgcgaaagcatccgcagctacctgatcaccgacgtcgagacaggcgtgacggacaccggcgtgatgctacgcggagagattacggacttcgcggtggcgaacctcgccgagttcaccggccacctctcccgcctcatgcagcaaaactgcctggacaccgtggtgctgaccacccccgacaacttccgcatggaaattctcggttactgtttcgcctcgccggacctcgaaccgttaacggagttcaccagctacgcgcttgaagaagacgcggattcaatcgcgttcgtggattactacggcaaagacggcaaagaaatcgggataaactggttgaacctcgcgtctgacgccaagctcgagcagctggataagcagtgggacaaaaccgagcgccccgccgggttcaaccagctgcggttcaccgcctacacgccgaacgaagcgtacgtgcgcgacgatgtgaaggacgtgggcgtccgcgtggcccgcggcccgcggttcaccgcggtcgacgagaccgccgagcgcaccaccacgccgcagccgaccgcgtacatgctcagcaccgcgccctcggctaccacgactggctcacccacgccggatcaggaaccgcggcgtgaatcgcactcataacctgctcgacgttggagtagctcatccgcttcgggttctccatgccctcgaagcattcctcgtcggagcggccggcctcggtgccggacaccacgccaacgatcacggcgcgcccgttcacctcgctgaacactgggccgcctgagtcgcccggcgagacacacacctctgcaatatcgccgaacgtggagcgcgggatgtcgacgtcggtgtcggtgatctgcacgcgctgcgtctccaagaacggcccgcacgtgtagccggtggtgctgccggtcttgcacacacggccgagctccgggatgtcctcgccgatgccggtcgggattggcgcgccgatgacatccataaaccgctgcgggtcggtgatctcgataatgcccacgtccacaccgtcgccgtcctcagcaaacaggccggagtacacaaacctgcccgcctcgacctggtagtcggtggcgtactcggcgttcgtcggccacaccaagtcgcccaccttgccgcagtggctggcggtgacggcgaaattccggccggacgtgtcggagaaagaaaacgcaacggtgcaggcctgcgcggtgaagctctcccccggctgcggatagtggtctgtggtctggatctttgttcccggcgcccacagcgcgtactcgggaacgaggatccggttgcccggcaccgcatcacccgcaggcgcacccgctggcgcacctgccggcgcctcgcttggcggggtgcgcacctcttcttgcgcttgacgctcagccactgtgccggtcggcgcctgcgacatggtgacccccatccaggtcacagcggcgaccagcatcaacaccgcgacgacggcgaaaacccagaatgcgcccaggcctttgcggcgcgtcggcggcgcaccggcgggcgcggcttcgggccacgtcttgtccggatacgtccactgcggcccgtccgcggtttggtacttcttcgccgcgtcgtagccgttcggctcgttcgagtacgtgctactcgcccgcctcgtccgccgccttgtccgaggcggcggcgtcggtctccgcggcctggatcttcaagtcgcggatgaacttctcggggtcgaactcggtgaagtaatccggtccggcaaattgctcctgcgccacggctttcgctccttagacctcggtgttctcgatcgcgtctgcgatgaactgcttcaccgcgtccacgtcgttcggcaggtcagccacgtgccggcccgcgttcataatctccgcaaaccgctccgggacctcgggtgcggccccgaccgcctccacgatcgtgtcggcgaacttcaccggcagggcggtctcaagaacaatgattggcgtgtcaagggcatgttgcttagcgacgcccaccccatccgccgtatgcggatccaccagcaccccgtactcgtccttcactgccttgatcgtggcgagtcggtccgcgtgcgtcgacgtgccggagaggaacccgtattcgtttcggatgcgctcgaggacctcctcactcacgtcgaatccgccctctttgaccttggtgccgaagtactcggcggtgaggctggggtcgcgcaacgttgcgtcgaaaagcatccgctcgaagttgctcgccttggagatgtccatcgacggcgaggaggtcgcgtgcgtctccgccgcggagcgcgggcggtactggcccgtttggaaaaactcgtgcagcacgtcgttctcgttggttgcgacgatgagcttgtcaatcggcaggcccatttgcttggcaatgtggcccgcgcacacgtcgccgaagttgccggtgggcacgcagaagctcaccttctcgtcgttcgactccgtgaccttgaggtaactcgaaatgtagtagacgatctgggccatcaggcgcgcccagttgatggagttcaccgcgccgatggagtacttcgacttgaagccggcgtcagcgctgacctccttgaccacgtcctggcagtcgtcgaagacgccgtcgagcgcgatgttgaagatgttcgggtcgtcgagaccgaacatctgcgcctgctggaacggcgtcatgcggcccgccggggtgagcatgaaaacgcggatgttgtcgcgaccgcgcatcgcgtactcggctgaggaaccggtgtcgccggaggtggcgcccaagatgttgatctcttcgccgcggcggccgagctcgaactcgaacagctcgcccaaaagctgcatcgccatatccttgaacgcggcggtggggccctcggagaggtgcgcgatgtagagctcgtcgcccagcttggtcaccggcacgatctcttcatcggcgaacttgccgccctcggtggtgtaggcgttcgccgtgagctcctcgaccttcgccggcgggatgtcgtcggcaaaaagcttgaccacctcggcggccagcgcagcgtagccagacgacgccagcagctcgcgccactgcgtgagcgtctcatccgtgatctgcgggtacacagcaggcatgtaaagcccgccgtcggggcttaagccacccagcaggatgtcggtgaaggtctgcctagtcgcctgcgtatcgcgcgtcgagatgtaatccacgggtgtctagcttaccttggcactgcttaccgacgcggcggttcctgcctccccgtgaggatatccaccaccgagcgaatcgccgcgtcgcccaactgcggcagcgggcggtgggacgtgtccgcggactccgcgggggcgctggtgcgcgccggcttggcctggcttgcgcgcgccgaggtgtctacctcgatcgaaagcgccgcgccgtcgagtttcaccggcgcggcgtcggccacgccggcaacgcgcgccgcgtccacaagcgccacgaggtcggcgaaggtcgcgttgtcgaggtcaatactcatgttcactgccataccccacttctactcgaactcaagcgaaggcgcctcaccccagaacactccctccaccacgccgtgggcccggcgagtgatgcgcaggtagtcctcgagaaactcctgctggttgtccgggtcgtagccggcggagccggcaacctgggccaggtgcgggcccggcgcgggcagctggtcggtgcgcttgccggcgacgagcacgagcgcgttgcgcgcgcgggtggcggtgagccacgcgctgcgcagaacgcgcgcgtcggaaccgctgatcacgtccggatcgtctaactcggcgaggtagtccagcgcggccagggtggacgtggtgtgcagctcggcgtgctcgtgggcgtgcatcatggttaaaagctggacggtccactccacgtccgcgagcgcgccgcggcccagcttggtgtgcacggagcggtcagccccgcgcggcaggcgctcgttgtccacgcgcgccttgatgcggcggatctcgcgcacatcgctcttgttcgcgccgccggccgggtagcggaactcgtcgatcatgtggaggaacttcagccccacctcctcgtcgccggcgacggtggtggcgcgcagcagcgcctgcttttcccagacttcgccccactcgcggtagtagcgctcgtaggaggcggtggtgcgcaccaccgccccggagcgcccctccggccgaaggcccaggtcgacctcgagcggcgggtcgccggacggcttggacaggcgggtgcgcatctggtcgacgattcgcgacgcccacgcgagcgcctccgactcgtcctcgccagcgaccggctcggcgacgaccatcacgtctgcatcggagccgtagcccagctccgccccgccgaggcggcccatgccgatgatcgcgatgcgcgccggcgcgtcgtcaacgccgcgctcttgaaggtcggagcggatctcggcgaccagcgccgcctgcagcaccgcctcccacacgatggtcagctccaagcagacctggcgcacgtccatcatctgcaaaagatcggcggaggcgattcgggccagttccgcgcgccgaagcgaacgcgcaacactgacagccttgtccgcgtcgtcctggtagcgcttcgacgcggagatgatcgccttcgacacctggtccggcgctggctcgagcaagcgcggtccgttagaaccgtctccgagcagcttcaccacttccggcgcggcgatgatcaggtcggatgtgtacggcgagttgcccaggattttcatgagccgcatgccgacaacgccttcgtcgcgaagcatgcgcaaaaaccagctcttgtcctcggctgcctcggacagcttgcggtagttcagaaggcccgcgccggggtcggcggtgccggcaagccacgtcatcagcgtgggcagcaagattgcttgcagcttcgctttgcgagaggtgcccttgaccagcgcggtcaggtggtcgtacgcgcgggccgggtggcggtagcccagcgccgccaggcgcgccttcacggcgtcggcgctgagctccgcttcgccgacgctcagatccacaacggcgccaagcagcgggcggtagaagaggcgctcgtgcagcgtcgagacggtgccgcgcacccgcttgagctctgcttccatctcgtcgattgaggtcttcgccttgctgggggtgaacccgctcgcgcgcgcgagccaccgcttgcgcttctcgtcgtcgtccgccggcagctggtgggtgcggcggaagcgctgcagctggagccggtgctcgagcaggcggaggaactcgtaggcctcgatgagctggctggcgtcgtcgcggccgacgtaaccgccgtctttgagcgcctcgagcgcgtcgatggtgttcggggtgcgcagcgtttcatcgatacgaccgtgcacgagctggaggagctggacggcgaactccacatcccgcagccccccgttgcccagtttgagctcgcgggcgcgctcatctttcggcacattcgccagcacgcgccgacgcatcgcttggacgtcctcgacgaagctttcgcgttgcgacgcctcccacaccatcggcgacaccgcctcgaggtacgcctcgccgagctccatgtcgccggccatcgggcgggccttcagcagcgcctggaactcccaggtctcggcccatcgtttgtagtacgcgcggtgggaatcgacggtgcgcaccagcgccccggacttgccttcggggcgcaggttggcgtcgacttcgaagaacgcggcggagccgactttcatgaactcggcggccgcgcgcgtgatcttcggcgtgacgggttcggcgacgaagatgacgtcgacgtcggagatgtagttcagctcgcgggcgccgcacttgcccatcgcgatcaccgcgagacggctgtccggctcctcgtcgccgtagacgcgcgcgagcgccatgtcgagggctgcagtcagcgccgcgtccgcgattgaagtcagcgtctccgtcaccgcgaggtagcccaagtgttcgccctcgccgtggcctttcaccttggcaaacgtgccggccaagtcggcggccgccacccgcgtgatcagagtgcggtaggcgcttttcaggctggcctcgtcggcgccgtccgcgctcgcggccgcgcgcatgaacacgagcgactcctccgcgctcggcaccggctgcgccagcgcgggggcgatgtcggggttggcgatgaggtgatccgccagcgccgtcgatccgcccatcagggcgaaaaagcgggtgcggtataaggggtcgtcgataagcaactgcttcacggccggccagctgccgcacgcctgcatgaaccggtgcgtgttgttcagcgccaagtccgggtcgctggagccggcgagggtccacagcagctcatcgctgtcaaagccgagctcttcgaggtcctcggcggcgcgggggctggtgaggccgagctttgcggggctgatcacaggtccagcccggagtcgatctcccacggcgtgatctgggaggtgtagtcgtgccattcgtcccacttcgagcggaggaagaactcgaagacctgctcgccgagcacctcggccatgaactcggacttctccaggtgccgcagcgcctggtcgagcgagttcggcaggtcgcggtagcccatcgcgcggcgctcgcgccgggtcagcgcgaacacgtcgtcgcgggccggttcgtccagctcgtagccgttttcgatgcccttcagccccgcggcgagcacggccgcgaacgccaggtacgggttgcacgcggagtccaaggaccgcacctcaatgcgccgcgactccgccttgtgcaggcggtacgtgggcacgcgcaccatcgcggaacggttggaaatgccccacgtcgcggccgtcggcgcctcggagccgaactgcaggcgcttgtacgagttcacccactggttggtcaccgcggagatctcgttcgcgtgctcgatgatgccggcgatgaactggcggcccaccttggacatgctgatctcatcgtccgggtcgtggaacgcgttcgtctccccctcgaacagggaaaagtgcgtgtgcatcgctgagccgtccaggtccgggaacggcttcggcatgaacgtcgcgtgcacgccgttcgactccgccaccgtcttcacgatgtacttaaacgtcacgatgttgtccgccattgtcagcgcgtccgtgtgccgcaggtcgatctcctgctgccccgggctggcctcgtggtgggagaactccgtggtgatacccatgtattcaagggcagaaattgcttgacgacgcaacttcggcgcctcattacgcttcgcctggtcaaagtacccacctttgtccgcgggtgtgatcccctcaccgtcaggtttgaccacgtagaactcaatttcggggctggcgaagaactcgaagcccatctcgcgggcggcgttcatctggcggcgcagcacttgccgcgggtccgcgtacagcgggtcgccgtccggcatcgtgatgtcgcaaaacatacgggccgtttgcaggccggcgttctcatcgaacggcagcggctggtacgtactcgggtccggccgcagcagcgtgtccgactctgagatgcgggagaagccctcaatcgagctaccgtcgaaccccacgccctcctcgaaggcgctctccagttccgccggcgacatcatcactgttttcagacttccgaagatgtccgtgaaccagagtcggatgaacgcaatgtcctgctgttccaccagtcgcagcacgttatcggtctgagagctcatagggggcagtttagctttcgagcgggtcgctttgcccgcttctggcgcgctggcgcggggggcggatgaaggatggcggaagtacggccaagaaggggcatatccgccatccgccggacgccctccgctagacgcccccttgcacggtgaagaccggccccaagcgatttcgccacgcggctccggggacatgggcagcggcttcagctggctcgggcgtcggctccggctgccccgccacccgcttccatcccaggggggcggatgaaggatggcggaagtaccgccaagaaggggcatatccgccatccgctagacgccctcctccagacgcccccctgcacggtgaagaccggccccaagcgatttcgccacgcggctccggggacatgggcagcggcttcagctggctccggcgtcgactccggctgccccgccacccgcttccatcccaggggggcggatgaaggatggcggaagtacggccaaaaaggggcatatccgccatccgccggacgccatccgctagacgccatccgccggacgccctccgtcaaacgccccctagacgctcaaacccgcccattgccgagcgcccagcccgcaagtgggttaatctgccaccggagagagccgatacgcatcgacctcgcaggggaacgcactcgggggaacacactcggggaaacacaagtggggaactatttcgggggaaatgggaaatgggaaatatggacaaggctgcgctgatcaacctgttggtccgccctggcgacgctgataagcaaccgtgcaagaaactttccagaaacaaattcatcgccctatctgactgggaggcgctgaagcgccacgaagcggagtttctccgcgcgtacgcgatgggcgcaggctcccccacatccgcgctagtactgcgctcggccgcggcggtgcacaacatgtggacgatgccagtctcaggggcggcggaaacaccggtctatcttgcgaacccgaagagccgtccacggggcaaaaagtcctggccaaccggtgtcgagtatgtgcggatgagcatcccagagatagacctgtacgagttcaatcccaaaggcaccgaggacacgctgcgtctcaccactaccgtgcgaacggccgtcgatatcgcgcggctacacggggtgcgcgctggcgtcgtcgccatggattcgctcttcaccaccgcgcaaaccaaaaaggagcgcaaccaaatcaaggcaaagctcgagacaaccattgacaggatgagcgggaagatggggatcgatgacgctcgccaagcgctggagtggagctccaccctttccgagtcgccgtacgaaacgcttgtgcgcctcttcctccaggagcgcgacatcgtcgtccaggagcagatgtggataggccagtttgcgcgcgccgacctactctggggccaggtcatcatagagatcgacggccaggtcaaactcgacgacaacccaaaacaaactgcgattgaccagcttgagcgcgagaactggcttcgctcgcagaactacgaggtggtgcgcctgaccacgcacctcatcaagaccgacgaggaagagtgcgtgcgccgcatcgtcgagatgcacgagcgctcgctcaaacttcctcccccactcaccgaagcgactcaccgccgcccgacccgcggcgtcgactggcgaagcagcagctacataacccagccgtgactatggttgtggtgaaccaacgaattaggagggtaactatgggtgagaaagccaaagccgagcgccacctcgaggtggagatcaagctggccgtggacgagtcgacctctgtcccggacctgacgcagctgccgggcgtggaatccctcttgggcaccacgcagcacaacctctccgccgtgtattacgacaccgccgacctgcgcctgacgcgctccaagatcacgcttcgccgccgcaccggcggggaggatgacggttggcacatgaagcttccgcttgacgacggtcgccaagaactccgtgccccactcggagagcccggcgcgatcccggaggagctcatcgagccggtgcgcatcatcgtgcgcaacgagccgctcgagcctgtggcgcaggtggataaccgccgcgtcgagtcgaagctcgccggcgaggacggcaaccagatcgcggagttttgcgacgaccacgtcaccgcctggtctctgctgcccggcggcgagcgcacgtcgtggcgcgagtgggagctcgagttggctgagtcggtggcggagaccgacgagggtgactccatcattaggcaagccacgtcgtttctgatcaactccggcgcccgcaagtcctcgtcgccgtcgaagctggccaccgccctgggcgagacgatcaacaccgcgcccctgccgccgcacctggtggaggcggagctggagaaggactcgcccgccgccgcggtcatcgacgcccttcgcgcgcagcgcaacgcgatcgtcgactgggagccgcgcgtgcgcgccgacgagttcgattcggtgcaccagctccgcgtggccacgcgcgagatgcgctcgctgctcgagaccttcgagggcatcctcgagggcgacacgctggaggaacttgagggcgagctgaaggaaaccgccgccgtgctcggcgtggcgcgcgacgccgaggtggtcgaggagcggttcttagagctgctagagagcgacgagagcggtcttatcgacgccaccgcgtcctcccacatcgaacaggacatgcgacgcgactacgaaaaagcccacggcgagatcgtggagatgctgaactcggagcggttcctgaacctgctcgacgcgatcgacaacctcttggccgagccgccggtggccaaggccgacggcgactccgaagacgaggacgaggacagcgacaacaaggacctcagcgagaaagaatcgcgcgagatcatggtggagcacctggagaaggcgtttaagaaggtgcgcaagcgcgacgcaaaggtccaggagcactaccacgacaccgagcttccgttgcacgagcgcgaggagtacgtccacgacgtgcgcaaggctgtgaaaaaactgcgctacgcgacggccgcggcggagtctgccggcatcaagacgaagcgcctagccaaggcgaccaagcagctgcagacggtgctgggcgacttccaggacgcggtcacctcgcgcgaccgcatcatgcggctcgccgaagaggcgcgcgagcgcggcgaggacacgttcgcctacggcatgctctacgagcgcgagctcgcccgcggcaacaaggcgctcgccgggtacgacgaggcaatgcgcgaagtgaagaaagccttcaagaagctttcctagaacgctttagcgctcccaggaggccggctcgccccagtcatcgtcggcctcctcggcctcatctgcgtcgtcggcgcgcttggtgcgctcggcggcgatagcaagcgcctgctccgcctcctcgcgggtggcgtaggggcccatgcggttgtcccacgaggcaactttgccctgggtcacttcgccggtggcggggttgtagtaaaactgctcgtcgctcatggccgcttactctaccctcgccggttggtagtgtggtgcgcatgccgatgtggaatccccctgctcattcccccgccgagcgcgccgcggcggcgcatcagaaccgcaccaagaaggccccggcgcacactgcgtccgcgccggggacgtgggtgctcatcggggaaaacgtcgaccatttcggcggcgtgaccatcatggggctgtccagccttcgcgccgcggcgagcgtgagcccgcgcgaggacggcacgatcgcgctgcacgccgaggcgccctacgcggcgacgattgagcgcgaggccacactcgcccagctcggcgccggggagatcgaagacccgctgatgcgccgcatcacggggcttgtccagacgctgatccaccgccaggtgctctcccgcgacacggccggactcgacatcacggtggtctcggacgtgccgatgggcgcaggccttggtgcgctctacgccgccgacgccgcgatcgcgctggcgcttgcgggcgcgaacccggagctcaacgagccgccgatgcgcgcgcgcttggccgagatctgctcccacgccgccgccacctactcgtcgctcgcggtgttgcgcgcgcgccacacggtcgcgctgcgcggcgccgaggggcaggtcagcgtcgtcgattacgcggacggctcggttgcgccggctccgcacccgggcaagctgggcgtgcgcatcttctcggtgtcggaaaagctgggcctcccccacggcgagcagagggagcagattgctttacgacgcgacttcatcgacgctgcggtggcgaattttggggtggcgtcgttaagagagctccccgacaacgtggagcgggtcgtcgattgggtccaagcgcggcgcgatacgggggatgcggacgcgccggagccggcgaccgcgcgccagtgggtgcagttctgcgagtctgagacgctgcgcagcatggccactgccaaggcgctgcgctcgcgccgcggaaacgagctgtttacgctgctgaactcgccgaacgaagcgcacgatatcgccacccccgatgcgctcgtcgccttggcactcgagcgcggcgcggtggcggcgcgccccgcggccgccggcacgtcgcaggccgtgatcgcgtttgtgccggtgcgcgaggcggacggctttgcccaccagttcgccgaggacttcgaggtggtggaggtcgtgcccggcgcgccggcgcgcgtggaagaacccaccagctagtcagccggccaggcgaactccacctcgcgctctttcgcgtcggcgcggatcagcgagaacatcgcctcgatgccctcggccggcgcgccaatggacggcgccaaaagcggcggctgcgtgacaaagatgcgggcaggatcgctcggttcggcgccacgtttgagcacgatcccgccgaagttgtggccgacccacggcgcgagcacggtcgcctcggtaaggttcagcgccgccttttccaccatgttcgccagttggctggtgcgcgccatggtctgcaggacggttggcgcgccgtcgcggacccaagacggcacctcgtagccgccgcagatggcgaggcagacttcggttgcgtagcgatcaatcagcctgcgcagcggcgcggtgacgtggctgtagtacccgccgataccggcgtgcacctcgggagccttctcgcttaggtccacgtacccggagccgcgcagcagcttcttcgcctcccgcatcacggcggcgccgcgcggcgtgtccgcgtccaccccggcgaggaactcgccgatgccgccggtcacctcgtagcccaggttgcgcgcctcgcgccgaaactcggcttccgcctcggccggcgccggcccgagcgtgcgcaaaaacccctcgcctgcctcgaccatcatccgccccgccaccatgcctgtgagcagcgaaatctccgagttgtagtccatcacagcgtgccgcggctcgatcatcagctcaaaggcgccgtcggcggtttcgaccacgcggatcgacggcagccgcaggttgatcgcggcgcgacgcagggaggattgctgccgcagctggccgacgtggggcaggttgcttatcgacggatgctcatcccccctttccaacgcctcctgcacaccgtcgtagtccagccgcgccaccgagtgcaccagcgcgcgctgaacgtgggcgtgttccacctcgccggcgccgtccaggtcaaacgtccagagcacagccggacgatccacgttgggaagtagcgacgccgagccttcggaaagcactgccgggtgcaggcgggccggctcgtctggcaggtagatggtctggccgcggataagcgactcgcccttcaccagcgagctgggttcgacgaaggcggcgacgtctgcaatcgcgtactgcacccggtacccgtcgccgcgcggggcgatatgcaccgcttggtctaagtctttggagcccggcgggtcgatggtgacgagtgggatatcgcgggcgtcggtgcggtggttggcgtgggcgtcggcaagcatgcctgcctctgcgacaacctctggatcgaacgccgtgcgcacgttgaactcctcggccagcgggcggaagttcaagggcgcggcgtagagcttcatacgttgccatggtgccagaagtgtggcgaatgagttggtctatgagccggattctgtctccctcggggtttgcccctcgggcggcgatcatccatctgggccacccattgctgggcgcctcaagcagctaccttcggactgggcgggcagcctcatcgcgtccgacgacctccgccgtgttgcaggcgggggctcttgccttgctcccggtggggtttacctggccgcctgtgtcaccacaaacgccggtgcgctcttaccgcaccctttcacccttacccgcacgcaaaacgcgcgggcggtttgctctctgttgcactttcccgcggatcgctccgggttgccgttagcaaccaccgtgccctacggagtccggactttcctcgacctgtgccttttcgcttgagcgacggttcacagcgccgcgatcacccgaccaactcattcgcgccctgaaatgttacgccgagcgtaaccggatgcaaagcgctagcggtggtgggcgacgtcattgaacgtgcgcaccacgccgtagtcgccgtagaactccaccacgctgacactcgcaaggtccaagaacatgtgcttgaagctctccgcgttggagccgagcgcctggcggataacggacttgatcggcatcatgtgcgtgaccaccaggatggtctggccctcatgcgcctcgagcgttttcaggcgcgcgcgggtgacacggcggtggagcgcggcgacggtctcgccgcccggcgcgtccgcgtgcggtccctcccactcggcgccgaggcgcgcggcggcctcgtccttggtcaggccctcgaggtcgccgaagtcgatctcgcggaagccgtcgacggtctcgataccgtcatggtcgatgccgagcgcgtcggcacagtagcgcgcggtttccagcgcgcgctttttcggcgaggagacgatcgcgtcgatcgtgcccatggccgcgatcgcctcggcggcgcgcttagcctgggcgcggccgacctcggtgagctcgggatccgaggagccggagaaacgcttctgggcggagtgctcggtttggccgtggcgcagcagcacgaagcgggtgcgcggggcgtcggtgccggaccagtgcgcgggcgaggctgtctggtgtgcggcgggcttggccgatgcggaagcggcgggcgcggccgacggggtgtccaggatgcggggcgtgccgtccttcgcggcggcgtccatagccacgttcgacagctcgtcggccttcttgttcttcgcgcgcggcacccaggtgtaggtgacgcgctcaaatcctttggccagctcgcgggcctcgagggcgagctgcttcatgtccgggtgcttgatcttccagcgcccgttcatctgctcgacgaccaacttggagtccatcgagacgcggacctcggtggcccccagatccttcgcggcctcgaggccgcggacaaggccgtagtactcggcgacgttgtttgaggccttggcgccgacgacgtaggcgatctccgcgagcgttgcgccggagtcgtcgtagatcacggagccggagccggcgacgccggggttcccgcgagaaccgccgtcgcagaagagcgagacgcgcattacgcctccggggaagacgcgtccggggaaacgcgcacgagcagggtgccgcagttcgggcaggtgggtagctcgtcgtcttcggctgccatcacttcggcgcgctcggagggcgggagctggatgtagcaggagttgcaggtgcggccgttgaaggaggcggcgccgacgcggtcgtagacgtccagcacgtccgccggcagctgggtgcgcagctcctcggtgtccacaacctcgggctccggcagtgcgtcgacggtgcgctgggccgcctcgaccttgcgggtcgcctcatcaagctgggcgccgtggacgtcgcggttgttgcgcagcgccgcgatctcgttgtgggcctctttgagctcgtagcgaaggtcggtcaggcgcgcctcggtggcagacagatcgtgctgcaggtccttgcggcgctcgttgtcggtctctgcacccagctgcgcgacgtcgtccttcttgcgccgctcgagtttgcgcgagtcctcctggatgcggcggatctcaagctccatgtcgtcgacggcgagttgggcggacgaggaggcgagctggaggcggtcgcgggcgtcgataagcttggaaagctcctgctcctccggacggtgcacgggcctgcggcgcgcgcggtcggcgttggccagctcaagcaggaccggttgaaggtttgggcttaagtgcacgtgactactcctttacggacgggtgcgcggagatggtccacggatcagtgcggatcgggatgatctcggtttcaacgtctaggcctgccacgatacccgcggcctgctgggtccacggaaactcgctggcccagtgggcggtgtcgatcacagccggtccgccggcgcgcaggtgctcgtccaccgggtggtggcgcaggtcggaggtgacgtacacgtccacgcccaggcgggcgacgtcggcgaggaacgagtcgcccgcgcccgaagagaccgccaccttcttcacttttctgtccgggtcgccggcggcgcgcacgccccacgcggtctcgggaagcgcgtcggcgacttgctgggtgaactggcgaagcgtcatggcctcaggcagctcgccgatgcggcccaggcccgtggcgttggacaagtcgcgcgtctcctccatctggaccacgtcgaacgccggctcttcgtaggggtggcaagcgcgaagcgtctcaaccagcgtgcggcgcaagcgcgtcggcgcgacgaactcgacgcgggtctcggtcgcgctgtgcgccttcccaatctcgccctcggtggggttcgcgccgtcgacgggcgtgaacgtgccgcggccgtcggtgtggaacgcgcactcgcggtaatcgccgatctcgccagcgccggcgtcgaatagcgggcgcatcacgcgctccacgtcggccggcgggatgtgcacgccccagtggtcgatgcctccggtaaacaccggtttgatcggccggcccggggtgatgccgaccagctcagccaagcggtcgctcacgccggggcgggcggaatcggcgttggtgtgcgcggcgaacagcgccaccccgccgcttaagagcgtgtggatgaccttgcccttcggcgtgttcgcagcgacggagtgcacgcccttgagcagcagcgggtggtgcacgaccagcatctgcgcgccgcgggccaccgcctcctcggcgacggccagcgtgcagtcgagggcgaacgccacgcgggtcacctcagcctcagggtcgccgcagatcagcccgacgtggtcccagctttcagccaggtgcggcgggtaggcggcttccagcttgtcagcgatatcctgaactgtgtgcatgacctcaaccataaagcgacgttgctttttgacgtcgacggcaccctgatcgactcctaccccggtatccgcgaaggcttcgtccgggcgcttaacgcgatcggccacccggtgcccgacgagagctttctcaagcgcatccccggcccgccgatgcgcgagtccatgacaaacgccgggttggacggcgatcaggtagagcgcgccatggaggtctactccgacttcatgagcggcgaggggtggcaggatttcaccgtctacaagggcatggctgatcttgtggcgaagcttcgcggtgaggggtttggggtggtgacggcgacgtccaaaagcgaaaagtttgcttccctggccttggagcgcgcaggcattctcaagcacgtggagttcttgggcgccgcgaatgccgacgtgggccgcgtgaccaaaatcgacgtcatccgccacgtgctggataacgtggaggtagtcaacccgctgatgatcggcgatcggatgcacgactacgaaggcgccgccgagttcggcctcgattccgtggccgtcacctggggctacggtgacgaggacgagtggtcgcgcgccacccacgtggcccgcgacgcaagcgagctggaagggattgtgagaaaccatgcgcattgatttcgtttgcaccggcaacatctgccgctcccccatggccgaggtgatcgtgcgccagaagttggaagaggcgggccttggcggcgaggtccaagtcacctccagcggcatcggcgactggcacgtcggccgcccggcggacacacgcgcgctggctgagcttgccgcgcacggctacgacggctccgcccaccgcgcgcagcagttcggcttcgagcaggagtcggcggacctcatcgtggcgctggacaccaaccacgtctcggagctggtcgcacgcggcgtgccggagcacaaggtacgccttttgcgctccttcgacccggacccggcagcggccgaggaaggggtcaaagacccgtactacggcgggcccgaaggcttcacgctcacccgcgagcagatcgaggcggcgtccgccggcattattgcctgggtgcgcgagcaactagactaggcacccgtggcagcgaaaaacggcaaatcatgggcgcggacgttcctcacgcccggctgggtcatcgccgcgctgctgatcatcacgttctcctatttcgcgttcacgttcctcgctccctggcagctcggcaaaaacgagcgcctcgagcagcgaaacgagcacatcgtcgaggccttcgagcacgacccggtgccggtggcgaccaaactcggccccggcggcacgctcgaggcggacaacgagtggtcgcgcgtcaccgccaccggccgcttcctccccgaaggtgaggtgctgctgcgcctgcgcccggtcgaccgcgtgcccgcgttccaagtcctgaccccgtttcagctcacctccggcgaaaccgtcgtggtcaaccgcgggtgggtgcccgcagtcgactccacaaaggtgccggagtacgacgccgcgccaaccggtgatgtgacggttcagggcatgctgcttgccgacgaaggcgtccaccccaccacccccaacatcgaccaaggccaccagatggtctactccatcagcccccaccagatcggggagctgaccgggatcgacgttgtcagcccctacatccagctcaccagcgactcggccgcggtgctgaacgcaatcccgctaccgcagctggagacgggcaaccacctctcctacggcctgcagtggatcgcgttcggcctcctcgcgccggctggcctgatctacttcatcgccgcggagaccaaggagcgccgccgctaccgcgacgagcaggacgagctcgcggcgctgaccgcagagaccgcgccggccgagcccgctgagcccacggccgccccagcgcgttcgcgctacggccacgcgcggcgcaaccactgggccgaggacgacgaccagcgcgtctagctcgggtttagctgaagcgcagccccgcgtacgagccctccgcccgccacgcatccagcagctttcggaacaccgtgatgccctcggggaagagctggtttgtgtaggcgccgtcgccgtgctcgtagccggtgtagtagccgggcacgcaggtctcgaatgcggcgcgcacgccttcgcccctctcgcgcacggttgtagcccacgtctcggtcgcctcggcggtcggctcgacggtgatggcgccgcgccgcttcgtttccgcgatgatgtctaggatgtgctcggcctgcgtggtcaggcccgaggtgttgttcgccgtcagcgcgttttggccggtgccgatctggaagtggttgggaaagccgtcggccatggcgccgtggagggtttgcaggccgttggcgtagtggtcggtaagacgctcgtcgccgcggccgcgcacgtcgaaaccggtgcgcgtcaacgggttgccggtggtgtcgaagccggtggcgaagatgatgcagtccgcgtcgaaggtgcggtcgcccgcgtggagggttgtcccttggatgtggctcaggccggttgagggggcgtcgataagcgtgatgctctcgtcgttgaatgcctcgtagtagccgttatcaaaggtcacgcgcttgcagcggcggctgtagaagggcttgagggcgtcggcggtggcgggatcggtgacttgtgcgtcaatcaggtcgcggatctcgcccatgatcgcggcgtcctcgtcctgcgggttgtcggcggtgagcaggcggcgggcgtggacggtgaagttgtcctgcacctcgtcgtgcggctggaggaagccggaggtgttgaggtcgtaggtgaggatgcgctcgcgctgccaccccgcgggctgggcggtgaaccactcggggtctgtcggcgtcgtgtcacgctcgcccaccgcgggccccggcgtgcgctgcaccgcgtagacgtgcttggcctggccgacgagcgcggggatgatctgcaccgcgctcgctccggagccgacgaccgcgaccgtcttgtccacgagcttgtccaaaaccggattctccggcgagccgccggtgtagttgtagtcccagcgcgaggagtggaaagcggtcccggtaaaggtgtccatgccgctgatctgcggcaatgccggcgcgccgaacgcgccgttggagcggatgaggaagcgcgcacggatctcatctccgcggttagtctcaacgacccactcttcgttcttatcgtcccacgccgcacggatcgcgccggtgtggaagaccgcgcggtcgtagaggctgaagtggcgcccgaagtggcggcagtagtcgagggtctcgtgcgccatcgggtagcgcgaggacggcacgtagccggtctcctccagaagcgggtagtagatgtagctctccacatcacactgcgcgcccgggtagcgattccagtaccaggtgccgccgaagtcgccggcttggtcgacgatcatgaaatcgctgtggcccacctgcgtgagctgcgcgcctaggatcatgcccgcgaacccggcaccaacgacgaggatctcggtgctgcgggaaaacggctcgcgcggcttgatcggctcccacgggtcgtccgtgatcggggtggtaatactcggggctttcgcgcccgcgcgcttgtccagctcttcgcggtagcggtggtcaatcatggttcacagactctatcggccccgtgattccgccgctaggattgtcacccgtggagcacattttgactaacgacgaccacgccaaactcgaccacgccttctcccttttaacgcgcgccggcgtccgcctcgccgaggatatcgagccggacgacatcgaggacgcgattgccgacgaccccgcgggcttccgcaccgccccactgaccacgcttgccgggctttgcgaccccgacgcccaccccctcatccacaacgccgtcatctcgggcggcgacgccggtatccccgccgtggtcgagcgcttcgcccgcgccgccggcgtgtccgcccacgacatcgccgtcatgtccgacccgggttccgacggcgcttccggttccgtccgcatccgcttcgacgagtgggacgtcgccgacatcgactacgacttctccggttctggccaggacttcgagctggacgtcgtcgccgccgccctgccggtgggtgcgatggcggcaaccttccccaccccggacggccgcgacgtcacccttttcctccccgccggcgccgacgaggacgcggtcgacgcgctcatcgacgcgatcgaggcagagttcgcctagcggcgcgccggcgacccacgttgatagcgggtaactccgggctgcttccccgtttccgcaggtcgccgtcggcgggtccgcgagttacccgctattaccgacccggcccttttgttgacgccgctggcggtctgctacgatgaaacaactcgcgccgttagctcagctggaagagcaactggtttacacccagtaggtcgggggttcgatcccctcatggcgcacaaaactgcgaaggcgctctcggaaaacccgggagcgcctttcgcatgcggctgctcggtcctacttcttggtttgtggggcggcgagcagggagccctgccactcgccgaagcggtcggccttcgtctgcacgaggccggccaactgcgcggattcagcgatctcaccgggtgccacgccgccggaggtacctgctgccggggtcagcagccatacgcggccgccgtcggagaggttgcggatggcgtcgacaagcgaatcgaccaggtccccgtcatcgtcgcggtgccagagcaggacgaagtcgcacagctcgtcagagtcttcgtcgaggagcggctccccgatggcgtcttcgatcgcctcggagatggtcgaatcggcgtcgttgtcccagccgatctcctggacgatgtcgccctctttcactccgaagcgggcggcgtacgtgtctcccccggtggcaaccaaggtcggcatcctccttgttcgtggcaataaatcgacttccagtttaccgccggatgcgcgccgccacaggtgaacgctgcggaggtagtatttatcagccaactccgtgcgccgcggaactcgaaacgttctagaattgaaaggtgaaacgataccgactcttagggaggatttcccgtggctgataacgccaacaagaacgagcacctcgaaggaacggacgccgcaggcgtgtcagcggaaaccaacattccgctgctgcgtgacggcgtcgcctcctacctgcatgacgccgatccggaggaaacgcaggagtggatggattccctcgacggcctcctggaagcctccgacccggagcgcgcccgctacctcatgctgcgcctgattgagcgcgccaacgccaagcgcgtgccgctgccggcgctgtccgagaccgacttcgtcaacaccatcccgacgaagctggagccggaattcccgggcgacgagaagattgagaagcgctaccgccgctggatccgctggaacgcagccgtgatggtgcaccgcgcgcagcgcccgggcattaaggtcggcggccacatctccacctacgcctccgccgctgctctttacgaggtcggcttcaaccacttcttccacggcaaggacgccgagcagcgcggcgaccagatcttcttccagggccacgcgtcgccgggcatgtacgcccgcgcgttcatggagggccgccttagcgaggacgacctcgacggcttccgccaggaagtgtcccgcccgcagggcggcctgccgtcctacccgcacccgtacggcatgccggagttctgggaattcccgaccgtgtccatgggccttggcccgatgaacgcgatctaccaggcccgcttcaacaagtacctgcaggaccgcggcatcaaggacaccgacaagcagcacgtgtgggccttcctcggcgacggcgagatggacgagccggaatcccgcggcctgatccagatggcctcgctgtacggcctggacaacctcacctttgtcatcaactgcaacctgcagcgtctcgacggcccggtgcgcggcaacggccagatcatccaggagctggaggcgttcttcatcggcgccggctggaacgtgatcaaggtggtctggggtcgcgagtgggacgagctgcttgaaaaggatgaggacggcgcgctcgtccacatcatgaacaccaccccggacggcgactaccagacgttcaaggcaaacgacggcgcgtacgtccgcgagcacttcttcggccgcgacccgcgcaccgcgaagctggttgaggacatgtccgacgaagagctgtgggcgctgcgccgcggcggccacgactaccgcaaagtctacgccgcctacaagaaggcgctggagaccaagggcaagccaacggtcattctcgcgcacacagtgaagggctacggcctgggccacaacttcgagggccgcaacgcgacccaccagatgaagaagctgacgctggacgatctgaagctgttccgcgacaagcagggcatcccgattaccgacgaggagctggagaaggatccgtacctgccgccgtactaccacccgggcgaggacgcggaggagatcaagtacctcaaggagcgccgcaaggagctcggcggcaaccttccggagcgccgcgtggacttcacgccgctcgagcagccggacttcgagaagacctacaaggccctgttcaaggactccggctcccaggaagtcgcaaccacgatggcgctcgtgcgcaccttcaaggcgctcatgcgagatcaggagattggcaagcgcgtcgtgccgatcatcccggacgaggcccgcaccttcggcctggactcctggttcccgacgctgaagatctacaacccgaacggccagaactacgtgccggtcgaccacgacctgcagctgtcctaccgcgaggcgaaggacggccagatcctgcacgagggcatcaacgaggctggttcgtccgcgtccttcctggctgcggccaccagctacgccacccacggcgagccgatgatcccgatgtacatcttctattccatgttcggtttccagcgcaccggcgacaacttctgggcagccggcgaccagatgggccgcggcttcatcgttggcgcaaccgctggccgcaccaccctgttcggtgagggcctgcagcacatggacggccactccccgatcctggccagcacgaacccggccatggtgatctacgatccggcgttcgcgtacgagatgccgtacatcatctccaagggtatcgagcgcatgtacggctccaacccgggcgagaacgtcatgtactacctcaccgtgtacaaccagcccacgcaccagccggcgcgcccggagaacctcgacgtggagggcctgcacaagggcatctacctcttcgacgagggcgacacctccaaggagcaccgcgtatccctgctggcttccggtgtgggcatgcaggccgcgatgcaggcgcagaagatcctgcaggaggactacaacgtcggcgcagcgctgtactcggtgacttcctgggtcgagctggcccgcgacggtgcgcacattgcgaacgagcagctgctgcacccgggcgaggacttcggcgagccgtttgcgaccaagcagctcaagcagaccgagggcccgtacatcgccaccagcgattttgcctccgacctgcaggagcagatccgcccgtacgttccgggccagtacatcgtgctcggtgcggacggcttcggtttcgcggacacccgcgaggcagcccgccgcttcttccacatcgacggcgagtccatggccgtcgccgccctgatgggtctggcgcgcgagggcaagatcgacatgtcggtcgcagccaaggccgccgaggacctgaagatcggcgacccgactgcagctgcgcccgaccaggacggtgaagaggtaggccctgagaacgcggccgagtaggagcgatgcacgctgtgggcgcacgctgtcggcaggcggtgcgcgttaatagcgggtaacttccggaacgccgaatcgcgacctgcggaaacgcgaaaggcggcccgagttacccgctattaacgccaggttgcctgcgctaacaccagcccgcctgcgctaacgcccggccggcccgccgaccagccgcacaatcgccgccgacaccgcccccggggcgtccagcggcggcatgtggcccgagtctgggaggacttgcacgtacgcccgtggccagatctcagccaagcgctgggactgcgacacgggcgttacgtaatctttgtcgccgaccaggatgaagccggggatgccggcgagcacgtctgccgcgcccagctcggagtgcaggtgcaggtcgtcgaagaatcccgcgtaggtggccaacggcgtctgctggatcatctccgcgtggaagcggatggtggcgtagtccatcggccggaagtagaacccgagcgcgagcaccggcgcgagcgtgcgcgtgatcgcgcggcgcatgccctcggcgaagcgcggtgtgtggttaacgatccactcgagcacgcggccgaaggggccggcgagcatgcgcggcatcccctgcacggtgaacggctccacggccgaggaaatctgtacgctgccggcccagtcgaaggcgtctgggtggcggcgcatcatggacagcgacaccggccctccgagagaatgccccaccacgtacaccgggccggagacggcgaggtactcaaggacggtgatgatgtcgttggcggcggcgtcgatagtcagctgctccggcgcgcattttttggattgcccgtgcccgcgcaggtcaaccagcacttggcgcacgccgagcggccgtaaagcgtcgacctggaggtagaactcggcagacgagatgttgaagccgtgcacgtagaccactgtcgggccgtcggccgggccgacctcgtagtagtggatgccgccgacggtgccttcgcggtcggggttcaagcgggcttcgggcggttgcatgtccccaagcttaaagcctcgtcctgccgtctccacatgggcgttcgccagggaccgtacatgaaagcgcttccaataattctctttgacttcaaatgatggtaaccaaaacttcaccgccatggtggaaagtacgttaatgaaagcgcgttcacgctctacgtccaagccattggctcggcggaacctctttcgcaatcccgatcagttcccaaaccggaaaggcacttccgtgaatcgcccatccttgttcaaatcggctgccgctgtcctcacttctgctactgccgcactgactcttgtttcatgcagctcctcagagagcggttcggatgagccgcttgtaatctactccaactccacctccgatggtcgcggcgagtggctgaccgagcaagctgctgaagccggctttgacatcgaattcgtgaacctcggcggcgcggacatccaagaccggcttgtggccgagcaggccaaccccattgctgacgtcgtctttggtctcaacaacgtcttcttcgagcatctcaaggctgacggcgtcctcgaaccgtacaaaccatcttggtccgacaaggtggagacgggcgtcggggacgacgaacagtactggccgatcgttcgcgaacccatcatgctcgtctacaacaacggtgcattcaccgaagcggacgcaccgaaggactggccggacctgtgggaagaggatcgtttccacaacaggtacgaggttccgaccggcctcggcggcgcgactacgcaaatggtgctctccggcatcctgtcccgctacttagatgagaacggcgacttgggcgtatcggacgaaggctggaaagccgtagaagcttacttcgataacggaaataaggctatcaagggcactgacctctacgcccgtatgaaggagggggaggtcgacgcaggccagatgtggctggccggcaaggcaaaccgcgagaaagaatacgggatccagactaccgcggttcacccggccgtcggcgtgcctatggcaacgcagcacattgcaaaggttgccggcaccgacaacgagaaggcggaggacttcattgactggttcggctccggcgaggtccaggctgcatggtcgcgtgaattctttactgcgccggtaaacaccgatgcgctggctgatgccgaccaaaccgccgtggaagaaacggattccttcaaggcgcaagatattgactgggaggctgtggcaaagaacctcccgtcttgggtcgagaagattgagctgcagtacctctaggtcgcgtgaattaacctcgcacagtctcgtttgataccaaacgagactgcagttgtgcaccccctcttcgtcctcggaggcctcatgatcactttcgaccgcatcaaggtcgtgtacggcgacttcgtcgcaattccggatttcaacctcagcgtcaatgaaggcgagttcttcacgttcctcggcccatctggttgcggaaagtccacagctctgcgcacgctcgcaggattcatttccccagcatcggggactattcaaatcgacggcaaggatgtcacgtacgcgcacccctcaaagcgcggcatcggcatggtgttccagaactacgccctgttcccctcgatgaacgtacgagaaaacatcgaattcggcctcaagatggccaagctgccgaaagcccaaatttcggaacgcgcattaagagccgccaatcaggtttcgctcactgatgagcagctggaaaagcaggtttcggagttgtccggcggccagcagcagcgtgtggccatcgctcgcgcacttgtgatggagccaagcatcttgcttctcgacgaaccgttgtccaaccttgatgcccgcctccgcaagcagctgcgtgtgcaattgaaagagattcaaaccgacgtcgggatcaccactgtatatgtcactcacgaccaggaagaggccctgtcaatgtcggaccgcattgcggtgctgaatgaaggcaggattgagcaagttggcaccccgcgcgaactctacgaagatgccgcgaccgaattcgtctgcaacttcctcggacaggtgaataagctcagcgagggacaggttgcagaactgaacaaccaaggcgcccacctctccccctccaatgcgcactacatcaggcccgagcgcctgctcgtacaacgcggcagcacaacatcattacccgcaggctctgagcttcgcctgcccgcggccgttattggtgaaagctacctaggcgatcactcagtggtggaggtagatgccatcgggtcttcgctccgcgtcaacgtaccgggtccgaaccctctacatacagaagacgggacgttgactttggtgcttgatgaagactccatctatagcttcgatgtaaacgggcgacgcgtcaccgcgtgaggggcagctatgaaaaagaaccgactctcgattcgcgcgatgctcaagtcgcccctaaacatcgtcattttgaccgtgatgacctatttcctcatcacgtttcttatctggcccaatctttctctcctgttgagcgtcttccgacccagcggcgagtggagcctagacgtgttcccggagcttttcgcatccgatcgagcgatgaagtcgttgcgaaactccatcattctcgctttcgcgctgtgtatcacggtcaacgccgtcggtatcttcatcgtcttggtgacgcgttacttcgacatcaagggatcaagaattttgttcttgggattcgcgactcccctgttgtacggcggtgtcgtgctggtctccgcgtacaaactgatttacggtcccagtgggtacctgacaaatgcggccacgcgaatcttccccggaatggatacgcattggttcgaaggcgccctcgctgtgattttggtgatgacgttatctggcaccggaagccacctgctcttccttaccgactcgatttccaaaatcgactaccaaaccatcgaagcctcaaagcagatgggcgcgtccacactccagacgttccgggcggtcgttttgccggtcctgcgcccgatgatcttcgcgatcacgattttgacgtttctcggtgggctcggcgcgctgacagcaccactgatcttgggaggtgagaatttccaaaccatttcgccgatgatcctgacgttctccagaactgtcagctcccgagatctagcagcgaccttggccatgttccttggcttgatgaccatcctcatgctcgcgctgttgaactgggcggaaaaaggcggcacctacttctcggtatcgaaggttccagtcgcgttgcagaaacagaagatcgacaaccccgttgccaacgtcatcgtgcacattttggcgtgggggttgtggctgatttacatcttgccgccagtgctcattgtgatcttctcgtttaccaacgcatctgcaatcagcagcggccggatcaattttgaggatttcacgctgcgcaactacgggcgcatcttcaccgatccgtcggcaatcaagccgttcgcaatctctatcgcctactccgcagtggcatcggttgtagtggtctttgcgatgctattcgtggcgcgacttatccagcgacaccgcaacgcgatcaccatctggctcgagtacttactgcacatcccgtggctgctccccggcacaatgattgctcttggccttctgttgacattcagcacccctcagccgctggtcttcgggcgagtcctgtcgggcaccgtagtgctgctcgctatcggttacgtcatcgaaaagattccgtttaccctgcgcatgctgaaagcttcatacactggggtccccgacaacctcgaggaagcagcctcgctgctcggcgcgagtgattttcagatattccggaagattctgctgcccatcgtgttgccggtggctgcggcgattaccgcccgcaactttaacgcgctgctggataactatgacacagcgatcttccttgctcaccccttctatcaaccgctgggcatcttcatctacaacgcaacagagtccgacaccttaaacgacaccaccgcgttgacctttgtctacacggtgttgctgatgatcatctctgccgtggtcttgtacttggtctacggccggaacagcaagccttcccgctcacctaagcacggctggctgcgtaacctcttccgccgacgcgcggttccgacagaaaccaaggaggctgtcaccgcatgacacaagaagtattagggcggcaagagtacgccgctgtgaaccgccgtttccttgccgcatgtaatgtcaagcggccgctgatagctgtccaccgcggtcagaatgctggaagcattgttgaaaacacggcacgtgcagtccgggcggctattgtctcgggtgcggatatcgtagagattgatgtgatcgaatctactgacggcgacttttttacattccacaacgggttcgaaggtgtctacttcgggcttgatcgtgacattcgaacactcagtactaaggagcttgaacgactgcagtttgatctctacgtctcggcgaaggcagaaaagtacggtctagaaaggctggaaaccattgtttgcggtttcccggacactttgctcaacattgatcgatcgtgggagtactgggaccacctcctcccgttcttggatgacctcggttgcgtcgaccgtgtgctcttcaagtcgccagtagcgcaagagtggttgcagaaactcgccgatcatcctgtgaaatacccgtacatgcctattgtgaagtcgaaggacgaagttgaactagttctcaattgtgccgatgtcaacacaattgcagtcgagattctcgcagcttccgaagatgaggagctggcttcccaagagtttgtgcaggagatgcacgatttaaatttgttggtgcagaccaacgctctcaacctcccgaatcgtgtcccgctgttcctcggttgggacgatgaaatctcggtgctggatgaacctgagaagggttggggccgccttgtagatcacggcgccgacatcattcagaccgactggccgatgttgcttgatcgtttcctctcaaccagggggtgaaacgttcaggcagcaccggtgggggccggcagctaaaatgagcgcgcaagtcattttcctctgagcatcgaggccctcgtgaactctccccgacacacagtgcgcgtgaccatggacgatgtggcgcgcgctgctggagtgtcccgcgccaccgtttctcgagtgatgacgggcaattcctccgtcagccaagaaacgatcgccagagtcaacgaagccatagcggctttgggttatgttccgaatgccgccgcacaatcgctcgccgggcgcaagagcgacgtacccacggtcggcttgctgctaagggatccggcgagcacctactacgggttcttcttctctcaaatgcagcgtcaagccgaggaatcgggcctgcagttggtcgcatcgatacctacgatccgcgggagggcagcagacgagctgtccgcgctcgatcgtttggtacgacttggggtcaacggcatctatctcgctacgggatcgatcaagcccgcagatgtggagtcactgttggatgcagtcccaatgatttcggtgggacgcccagagttccacgatgagattacggccatctcatacgacgaggaggctcacggcgagattatggcatcgaacgtggtttaccacgggcatcagtccgtgtgcgtcgttcacgtagccgcagaggtttcttcgtccgaatcccaccgctcgcaagcgatgatccgcacgctgaaacaggctggcgtcgaggtcgctgtcgtggacgaaaacgagaaccagcagcgcatgaccacaatcaaccaggtgctccagctggtgtgggaaaaggaggtaacctgcgttatgttcccagcggattacagggcgctccagttcatcgattattgcaccatggcggggctgcaaatccccgaagctgtaagcgtcaccggcgttgatggcgtatttcctcggtggcagcatcttgggttggcgacacttcgcctgcccgtcgaatcagttgccgcgcgtgcggcacaggttatgagtgcgcggttggaaaaccctcgccaacctgtcacccatgaaacgttcgtcggctcctttgtccccggccgcaccttgaatacggctcataacttttcgcggtagtcgtcagttcgggtccctatgatgaagactatgctctcggaacttctcgcgctgcttagcacccgcttcgacgcaaccccggagcccgagaccgcgctcgcggattcgggcctgacgtcgctcgacttaatcgaactggcggtgcgaatcgaggacgaattcggcgtgcgcatcagcgaggacgtgtaccagcagcacgcaaccgtgggcgagctcgccgcctacatcgaggagcaccagccgtgatttcctatctgaccgacatggacggtgtcctgcaccgcgagggagacctgattcccggcgcggacgcgttcatccgcacgctgggcgacgaggacatcgagttcatggtgctgaccaacaactcgatccagaccccgcgggatctgtcggcgaagctgcagcgcctcggcctagacatcccggaggagcgcatctggacctccgcgacggccaccgcgcgcttcctctctcagcaggcaggtgaggcctccgcgtacgtcatcggcgaggcggggctgaccaccgcactccacgagattggctggattcttaccgacgccgacccggatttcgtcgtgctgggcgagacgcgcacctactcgctcgaggccgtaaccaccgcgtgcaacctgatcatgaacggctcacgattcatcgccacgaacccggatctgaccggcccgggcccaagcggcgtgatcccggcaacgggtgcggtcgcggccatgatcaccgcggtgaccggcatggagccgtactacgtgggcaaacccaacccggtgatgatgcgcacggcgctgaacaacatcggcgcgcactcggagcacacggtgatgatcggcgaccgcatggacaccgacgtcaaggccgggctggaggcgggcatgcgcacgatcctggtccgcaccggcatcgcggacgacaaggagatcgcccgctacccctaccgccccaccaaggtgctcgattcggtcgccgcactcgcggacacggagcgcatccatgaccccttccgcgacggcgcgtacagggattagaggaaggcctcgatcaggtcgttgacggggccaggcttatcgacgttcgcgttatgcccagcaccggcaaccgtcgttaagctgatgccctcttccgccgcccaccgctggttcatcgccttgatcccgcccatggtgtcgtgctcccccacgatgagcgctgccgggcacagcagggcgggcgcgttattggacacggcgtctgctatggcgcggaagatgcggctggcgagggcgacgtactcgtccttggtgtagtcgcgaagcatttcgcgcgtgagctcttgggcgtgctcggtgtggcacgtttccttcggcgcctcggcgaggatggtcggccacgacctcatgcgcagcagtgggccggcgtgtttcaggcccgcgagcatgagcgggttccagtacgcgcggttcagcggcatggtgtcgatgcctacgaacccgtccgctagatccgcgcggagaccaagtactgcctgccccacgatcccgccgaaggactggccgaccagcgtcacggggccgtcgatcgccagcgagtccaggatggcgatgagctggcgggcaatgccgtccaccgtcagcgcctcgaggtcgtacgggcgggacgcgccgtgcgcgggcgggtcccacacgaacgtgttcaccttgccgtgcaacgcgccacgcgtgaagtgctccagctgcggcgaaaagaggcggtggtcggtgagcatgcccggcaagaacaccagccacggcgcgttcgctacctccgcccgtgtgacggagtagcggatcgggccgtggggtgtgccgaccgagtcgaacgagctagtcagcaatgaagaaacgctgcttgttcacaaactcgtccatgcccagcgggccgagctcgcggccgaggccggagttcttcacgccgccgaacggcagctcggcgccgcgggcctgcgggatgttgacgtgaatcataccggtgtcgatcttgtcggcaacgcgcttggcgcgctcctcgtcggtcgacatcacggcgccgccgaggccgtagcgggaatcgttggccacctcgacggcctcctcgtcggacgacaccttgtacacggtagcgacggggccgaagagctcctcgtagtagatgtcggagccgaccgggatgccggtgactacggcgggcgcgaagtaggcgccgtcgccgtcgatggtgccgccgacatggatggtggcgccggcctcctccgccagtttcagctgctggaccaggttctcggcggcgtcgcgggacgacagcgggtagtattcgttctcgcctgcctctcctggcttgagcgggtcgcccttgacgtaggaagaggcgatgttcaccagctcctcgacgaactcatcgtaaatgtcctccatgacaatcatgtgcttgttggaggtgcaggcctggcccacgttgccgatacgcttggtccacgcggtcttcgcggcttctttcgggtcctcggcgtcgagcaccacgtaggcgtcggtgccgccgagctccagcacgcacttctttaagttctcgccggcctgcttggcaatggagcggccagcgcgctcggaaccggtcagtgaaatgcccttcacgcgcgggtccgcgatcagggtcgtgatgtcgtcgtgggaagcgtagatgttggtgtacacacccttgggcagacccgcctcttccaggatgtcctggatcttctgcgcggagcgcgggcagatctcggcgtgcttgaccagcaccacgttgccggccatgatcgcgggcgctgcgaagcgggcgacctggtagtacgggaagttccacggcatcacgccaacgatcacgccgagcggcaccttgcgcatgatggccttgccgcccttgttagtcggaatctcctcatcggcgccgaactcggcaccgtggtcggcgtagtagttgaagatctcaacgacgtcgtcaacctcgccgtcgccctccttcacagacttgcccatctcctctgcgatgatgcgggcaagttcgtcacgctgggcgtcgaaaagcgaagctgccttgtgcagcagctcggcgcgctcctcgtagctggtgtcgcgccaggttgtaaacgcctcgtcggcagttgcgagcacgttctcgagctcgtcggcggtgaggcggtcgaacgtctcaactacttcgttcgttgcggggttctgtacgcggtacggattagtcatagatgccagcgtacggacgctgcgccagccgtgccacgaacccgcgctgagctgccagctcctcaagtgcggcggcgaattccaccgcgtcggcatacggcgcgacgatgcgctcgcggcacgagtaggtgccgtccggcgcgcggtgccagcgggtgaaccacacctcgccgggttccccgtcgggcaaaaggagcatcagcttttcgacgtccccccgcacccccctatccatcccatcaatagcgagcacgaacgtgacattgtttgcggtagcggcgagcgtttcgggggcagcaagtgtggctgtcacagcggggagacctttcctgtgcgtggcgcggaacgcgcatgtgtacaacgcacccagcgcgcgccgagtggcgacagcacgcaggtgcgagacgagaggttcgtcttccccaacggcctcttgacgtagctgaagcgatcatgcgccacaaccgccacagcaacaaccctcaaggcttgcttaatccccctgtttactgaagctgaacttcagccttaggtcgcccgcgcagtgggatcagttagagcaggcggaccgccaccacgccggcgaagatcagcgccagcccggctacgcgcgcagcgtccatccgcgccttgcgcgccccgaacgcgccgaacgactccagcacttggccgccgacgatggtgcccgcgttaaacgcgatgaccgtcgtcgccgtgcccagaatcggcgcgagggttgcgccgccgatgacgaacaaagcgcccacgaaaccgccgagccacatccaccacggccccggctcgggcttggtggcgagctggcgcgggctggtgacaagcgctgcgatcaaaagcagcgtcacgccgacggtgaggttgatctccgcggcgtggagcgaggagcccgcgatggtgcccaggtagccgttgattgcggtctgcatggccgatcccataccaatacccacgccaagggcgcggtagagccagacggaggcgccggtgtcgtccgcggccgagcttgccgcagcgccggtccccttcttctgcagcacgagcgcgatgccgagcaccaccacggccgcgcccaggatgcgcagcagcgacacgtccacctgcttcgcgttgaacagcccccactggtcgatgaccagacccatcgtgacctggcccaggatgggcagcaccaccgtctgcacggccccgagcttggggaagagcaagatgttgccgatcacgaacgcgaccccgaagaacccgccgagccagacccaccagctggccggtgcacctgcctcagcgaactgcggcagcgggttgccctgcagcaccacggtggccgcgacggcaacagtgagcgccacggcaaaggacacgagcgcggagaccaccgggcggttgcccacagcaaggcgcaggcgcgaattcgccgccgtttggacgggcacgagcgcgccgatcagcagcgcggcgggtaagtagaacatggtgcttaagccatcaccggagaaacgtgcggtgccggagttgcttgtgtgggtgcgaatctagcggtcatcttccatttctcctctctgtgagtgtgagtgctcgttgaattctaatgaccgctgccgcacggggccggacagcggcacgcaggggggcggatgaaggatggcggacgaaggagggcggacgaaggatggcggaagtacggccaagagggggcatatccgccatccgccggacgccctccgccggacgccctccgccagacgcccccgacggtagtggccgcgacgatcgcgacggtcgttaccgcagcccggagcgacccgcctacgccttcgcctcggagcgctccttgacttcgttgcgcagcagcacgcgcaccgcctgcagaagttgctcgtcggaggcgctatccagcgcggcaaccacgttctccgcggacgcgtgcggctcgtctgggtcgtcctccacgccgagcgcttggccgatgcgggcctccagcgggcgctccggcatccggccgcggcgcaggtagttgccgccgaagtagaccaccatcgccaggatcggggccgccgccgcggaggcgagcatgccgtggtagagcatgccgaagtggttgaaccccaacagcagcaggctcgaaacgatcgcgggcaggacgtacatcttctgctcggtgaacaaggacgggatgcggcgcagcaccacgtcgcgcattaacgtgccgccgacagcggtgataatcgccagcagcacgcaggcgacccagccgagcccgttcgacaggcccttgatcgtgccggcgacggcccacacgccgatggtgatcacgtcggcgtagaagcggaacttgtcccacaccctcccgcccaggttcacggtgtaggcgacggcggcgccgatcgtggcggtgattaagtagccggggttggtgagggcggctgcgggggcgtcgttaagcaatgcgtccctcaacattcccccggacagcgaggaaatcatggcgatgaacgcgaaaccgatgacgtcgaaatgcatgcgcttcgccacggtgcctccgaccgtggcggcgagggcgacgccggtgtattcgaggacgaagaagagattttgtacgttttcggacagctccatgcgcacggatattagtgccgggcgctacaaaagcgcctgccagatcgcggtgttggtctcctgccacaggggtttggcccagtcgccgaactcgcggtccgtcagcgccaccatggcgtgatcccccgccacccacaggtacgtgccggccatgccgaagtggccgaaggtggttgccggcataccgtcgccggtccagtgcggcgatttgtcgcccttcagctcgaaaccgagaccccacgggcacggcttctgcatgccgtagcccggcaccacgccgcgcacaccaccgaactggttggaggtggcctcccccaggctggtgatcagttgcggttcaaggagttcctgggcgaagaggagcaggttgctcgccgacgccacgcccccatgcccagctcccccctccaacctcgcgccttccatcccaagcggggcaaacacgccctcgtagaggtaatccgggaacgcaatcccggtggtttcctccacgtgctcagcgagaatctcgtagcccgccgaggagtagatgcgccgctgacccgccggcttctgctgctcccgggtgtcaaaccccacacccgaggtgtgcgcgagcaggtgccgcacggtggagccttcgggcccgcaggcgtcatcgagctcgaaagccccctcctccaccgcgagcagcacgccgtaggccgaaagcagcttcgtcacgctcgccagctcgtaggcgcggtcgagatcgccgtaggcgtcgatcaccccgtccgggccgatcagccccgccgagacgttgtccaccggccagttgcctaggtgctgctgcaaaatatccgcgctcatgcgcccgatcctagcggcgcagctggttccagcggcgcacgagcaaccaggtggccagcactagcgcgcccgcgagcagacccggccagatcgccgggtccggcgagaagacgttgataacggcctgcaccacggcgaggaacgcgaagaagccgacgaagccgatcaccgtctgccagacgaggtccctgcgttggtccatgtgtgttttgcgagtgctagtcgatctcgttgggcttgcagatcagcacggcgtcgataagctgctgcggcgcgccctgctcccgcagcgtcaggccgttgtaacaaccgaagccggtgtaggtggtgccccgcttcggcacgcgctgccacgcgccgccggtgaagcggaaggtctccgtccagtcggtctggttggcgccggccgtagcccacagcccgtcgcagtaggtgactgtggtgccggtaaagttcggccaccccggcacaagcttgtcaaactcctccggcgcgcacgaccccttcgccggagttgccgcggcgcggttgttcgcgcgccccggcaatgcaggcaaggtgggtagcgccggaaacagcgcgttgatctgggccatgtccacacccgggatttggatccagccctgctgcaccgcaagcgcggtgccggcactgacaagcgcgagcacaccgagggtgataccggcgatggcggcgggacttaaagactcctcgctgcttgtgccggctgaggcggcaggctcggctgcgggttcatctgcctcgtctgcggcccacgcctgcggcaccgccaccggtgctacggccaccgaggcagcaacggttgctgccaggatcgatttcttcatgtttacagtgtagctaaccggcttaaaaccctcgccttacctgccgattttgtgaagtaggacctacggggttagtgttactactcgttgcttcgagcaacggaaacattcctccatagctcagttggcagagcattcgactgttaatcgaagggtcactggttcgagcccagttggaggagcaggttgaatagcccgcttcggcgggcttttttctattgccgtacatctcgagcccaaggtacggttctgttatgcacatcacattttctcgctttgcccctgccgcagcgtccgccgtcattgcggccttcgtcctcgccgcccccgcccacgccgccgattcccaggtcttcggcaacgcgaaaaacaccgtccgttgcagccttactaccgagggcggcaacaccttcgccctgtgcaccagcgacatcggccgcggcgcccagcccgagtgcaacccgccgaatgaacttgttccgtcggtggccattgagcccgagtatgtcggcacctcgtgctggaaccagggcttcgaccgggttacccgtttgcagccgctgcaaatccgctcgtttggtaccgccaccgtcatccccgggttcaccggcagcctctacgtcctcgacttggcgcagcgagccctggttcgtgcgggcaccgcgaacaaggtcattttcggggccaaatagccacctagcgagtacggctgtgtcatacttgccggcatgagaaaacctgtcatttgcctagcaaccgcccttgcactcactgtcagccccatcgctacgccgtcgtacgcccaggcaacgcccgcgaccgaggaacgggaagacagcaagacaggtctgatcatcggtggcgtgatcagcaccctcgcgctcctcggcgctggcgctggcgcggcgtgctgggcgatgcagcagggcatgatctcgaacccggctccgcagttcatcccgtgccacccgccggcaccggctcctgcacccgcgccggcccccgcccctgcaccggcgcgggtgcagga

SEQ ID NO: 12 - DNA, 114813 bp, Corynebacterium cassirii
  source 1..114813: mol_type = genomic DNA
gggctggggtgccgccggttgaggaacgctccacccgccgcccggcgcggaggtcggcccccatccgccaccggttgctggcggttgctgtgctggcccggtacccggctggggtgctccccaaccacctccggattgccagccgttgttcggcgtggacatgggcatttctccattcctagcgggcaaaataagccctgcccgagatgcgtaagtatgtacttctcggcggggccataacgggcgtcatgttagcaaagctcgtcgtggttggcccgagttagatgctgccgccgacctgcttgcgcaccagtttggcggcgaaatgcggcaagtcgacgccttcttcttcggcgcgcgccgccagtgcctctgggtccgcgggaagtcccagcgactgcgcgccggcaagcgcctttttgtcaaagaccggtgcaagctccggccacacgccctgggcctcgcgggcgaacatcgtcgcgcaggccggcccgacgccgtcgaagacctcgagcgacgccggcgcgccgtcccgcagttcgcgcaggtctccgccgtactcgtcgatcagtttcgccgcgaaggcgtgcaggcgggtggcggtggattcgtcgtagcgcttgtagccgttttgtccgaagatcctgatcagcgtgctgcgcggcgcgtcgcgcatcgcctccggggtggtgaggcccgcgtcgaagagcgcgcgggcggcggcggtggccacgtccgcgcggattggcttcgcctgcagcaggcacagggtgagcagctggaagaggggcgcgggggcgctatcaaggctaatgcccgcttcttctgcgaaggtctgcaccatggctaccgctgcgccgccggcgccggttcgagctcggagatcatcgtgatcccttcggccgccgaggccttcttggagttcgcccgcgccttcaccacgccgcgccaggacaggatggcgccgatggcgagcagcagcacgcgcacgatccagagtttctggtcgaggccgagagcggcaaggaccaccggcaggttcagcgtcaagatgatggtgccgacgaacccgccgagcaggatcgggttgaggcgggtgaccagccacgcagcgagcggtgccgcgattacgccgccgatcagcagcgccacaaccgccgcgaggttctgcagcagctggtcacgcatgccgaccaagaatccggctgtagctgccgcggtgaccagaaactccgcggtgttcacggtgcccacgatgcggcgcggctcgctgcggcccgcggccatcaaggtggaggtggttacaggcccccaaccgcctccgcccgcggcgtcgatgaagccgccgaacgcgccgagcggaatgaggaagcgtttcgagtgcggctcctgctgcgcgggcttggtgcgggtcaggccgcgggcgaaccggagcatcaggttcagaccgatcacggcgaggatcgctgacatcagcggccgcgccgactccatcgacagcttcgacagcacggttgcgccgaggaacgcgccgacggcgcccgggatgccgatggccgcgacggtgcgccagtccacgttgccgaaacgggtgtgcgccacgccggagaccagcgtggtgcccagctccgcggtgtgcaccacggcggacgcggtggccggcgtgagcccggccagcatgatcagcatggtggtagaggtgacgccgaatcccatgcccaggccgccgtccacaagctgggccgccaggccggctactgcgatcaaaagcagtgtcgtcaggtttcgcatgtcacacctccagtgtggttcggtagcggtcggcgacgatgccggccaagtctgtggtcagcggcccggagcacgtcacgcgcgccccggtagccgcctcaatgcgcgggatcgcatcccgagctttgtcgagcaggagcccatcagtaacgaacaggggcaggatgtgcaggtcgccgcgggttcgcgccagctcggtgaggtgctcctcgcccccgcgggtcgcggcaaccacgtcgacggttgaagcagttcgcttgccgacgctgcccgcaacctccacgtaccttctcgcctgaacctcgtccgaggtgccgaccgggtaaaggacggggtgggcgtgcttcggtgcgtcggcaagcaagcgctccgacagcacctccgcgacgtcctcgccgagccccagccccttggtcaggcgaagcggcgcgtgtgcgcgcgcggctttcaggtgcgcgggcacgtcgtgtttcgcgtgaaacgcctccgtgaacagcagcggcaccacgacggcaggcccgttcagcgcctgcgccgcgccttcaagcgacggctcattgaactccaagtgcgcgtccgcgctctcggcttcggcaagcgccgcggcggcgcgggtgagcgccttgatgccgtcgacggcccgcgggtgccgcgacccgtgggagagcgtgatcagcgcggtcatggagaactccgggtacctagcgcaggcggttgcctacgaatccggcggcaagcgtgttgccggaagcctggtcgacgagcaggaagctgccaaccgcaccgcgcgccgcgtactcctccaccggcagctcgtcggcggtttggatggtcacatgcgcgatgtcgttgagcttgaccgcctcgacgttggtgacgtcgcccgccggcgaatcgatgtcgaggacgcggtcaacgcttgccacccgcgcgcgcaccagcgaggtgccgtagcgcagcttcacggccttgcccggggtgagctgggtctccgtcaggcccaccacggtggtggcgaactcgcggacgtcctccgggcggtccgtgcccgccagcaggtcgccgcgggtgaggtcgatttcgtcagcgagccggagcgcgaccgaatcgcccgcctgggccttttccacctcgccgtcggcggtgtcgatgcccgcgactgtggtggtgcggccgtggggcgcggtgacggtgtcgcccaccgagatcgtgccggcagtaacgcggcccgcgtaggcgcggtagtcgctcgcgtgctcgcgcagcacgtactggatggggaagcggaagtcgagctcgagggcgcggccggagttcaccgggatggtctccagcacctcgagaaccgtcgggccctggtaccagtcggtgtgggtgccgcgctcgaccacgttgtcgcccttgagcgccgagatcggcaccgcgatcggctcttcgatacccagttcgcgcgccttcttttcgaaggtgtcgcggatcccgtcgaagatctcctgggagtagtccaccaggtcgatcttgttcacgcccaagatcaccgtcttgacacccaagaggtgggcgacggtgaggtggcgcacggtctgctcgacgacgccgtttcgcgcgtccaccagcaacaccaccacctgcgaggtggacatgccggtcacggtgttgcgcgtgtactgcacatgccccggggtgtccgcgaggatgaaggtgcgcttatcggtggcgaagtagcggtaggccacgtcgatggtgatgccctgctcgcgctcggcgcggaggccgtcgacaagcaagctcaaatccaacccctcgaacccgcggtcggcggaggtgcgctccaccgaggccagctggtccgcgagcaccgacttcgtgtcgtgcagcaggcggccgacgaaggtggacttgccgtcgtcgacgctgccggcggtgcagaggcgcagcgtggcgcggtctgccaaagcgtctgtggtcgtggtcatcagaagtagccctccttcttgcggtcctccatggcggactcgctcaaacggtcatccgcgcgggtggcgccgcgctcggtcaaagtcgacgtcgcgatctcagcgagcacctcgtcgatggtggaggcgtccgagtccaccgctccggtgcaggacatgtcgcccacggtgcggtagcgaacccggcgcgtctggatttcctcgccctcgcgcggcccgccccactcgcctgccgtgagccacatgccgccgcggttgaacacctcgcggtcgtgggcgaagtagatgctgggcagctcgatgccgcgcgcgccgatgtactcccacacgtcggactcggtccagttggagatggggaacacgcggatgttctcgcccggcagcttgccgccgttgtagaggtcccacagctccgggcgttggcggcgcgggtcccagccgccgaacgagtcgcgcaccgagaagatgcgctccttggcgcgggcgcgctcctcgtcgcggcgcgcgccgccgagcactgcgtcgtagccggcctcggcgatggtctccaccagcgggacggtctgcaaggggttgcgggtgccgtcggggcgctcgaccaggtcgccgcggtcgatccagtcctggacgtgggcgacgcgcaggcgcgcgccggtctctgccaccaggcggtcgcggaactcgatgacctccgggaagttgtggccggtgtccacgtggagcagctcgatcggcatcgcggccggggcgaacgcgcggcgcgccagctcgaagaccacacaggagtccttgccgccggagaacaacaggccgatcttgtcgaactgtcctgccacctcgcgcaggatgtgaatcgactcgttttccaagtccttcaggtgcggggagagcgcaccggttggtgtctgtgtcacaggtgttcctttactactcgtgcagttctactcgtgcaggccgcactcggtcttcgcggcgaacgcccagcgcccggcgcgcgggtcctcgccctcggcgacgggcatggtgcaggtcgcgcagccgatcgacgggtacccttggcgggtcagcgggtggatgatcaggttgttatcgcgctcgaaggtctcggtgtcttccagcgaccacgtcaccagcggggaaattttcagccggccggtggcgtccagcgacagtgcgggggcctcggcgcgggtggggccgtcggcgcggcgcagccccgtgatccagccggcgtacgggctcatgtgcaccgccagcggctcgaccttgcgcatccggcagcacgcggacggcgcgcgcaggtataggttcggaccgtacgtcttgtcctgctccggccggctcagttgcgccttcgcccgcaccagccggtgcgccgggtagcgggcctccacctcgtcggccacctcgagcgtttccgggaagtggtactcggtgtcgaggaacaggaaatccgcgtccggcaagtggcgctcggcgagctccgcgagcacggtgttttccatcgacagcgtcacaaccaacggtcccggcgcgtgctcgtgcgcccacgcgaggatctcttcggcggtggcgttgtacagcgcaccggcgtactgctccaccagctcggcgttgcgggccgcgacttccgggtcaaggggctgtgtggtcttgggtccgtcagggcttacctccgggtcgcggaagcccgcgcccgacgtttgcaaaaagtttgtcatttcagtcttgctcatccttgccagtatccctgccgcgcataagcaccgcagtgtggccgccgcgcttcagcgattcctgcaacgcttcgggggtggacagcgctttggcgtggccgcccaccggatcgtcttggccgtggaacttcacctcgaacacgcgcaggcactcgccgcacttccaggcgaaatccgtctcctcgttcggccacaggtcctcgcccccgcagtacgggcagtacgtggggtggttgcggttcgggttcggagcgcggcgaaagctcatcgcaggtcgtcctcctcggcgcgctgcacccacgcgcggaacgtctcaccgtcttcgcgctggtccacgtagttgcccaccacgcggctgacgtagtcggtcagctcggtggaaagcaccttgtggccgcgcagtttgcgcccgaagttcgcgccctcgccgatggtgccgccgaggtgcacctggaagccttcgaccttctccccgtcgggtccggccaccatctggcccttcagcccgatgtcggagacgtggtggcgcgcgcacgcgttcgggcagccgttcagcgaaatcgagatcggggaatccaggtcgccgaagcgctcctccagctcgtccgccagctcaatcgcgcgcgacttcgtggtcacgtgggccagcttgcagtactccaggccggtgcaggagatcaggccacgccggaactcgctcggctcgctggtgagaccgagcttgtccagctcgagcttcagcttgtccacgtctgcctcctccacatccagcaacagcaactccttgaacggggtgaatcgcagctgggttacgccgaaacgctccgccaactccgccacctcgatgagctgctcgccggacatgtggcccagcgtaggtttgaccccgatgtagaagttgccgtctctttgctcgtgaacgccgatgtgatcccggtcgacgaggttgttgggggccttcgggccgtcggcaagcgcgtagcccaggtagtcttcctccagcacctgccggaacttctctacgccccactcggcgaccaggaacttcaggcgagcgcggttgcgcaggcggcggtagccgtagtcgcggaagatgcgcaccacgcccgcccacacgtccggcacctgctcgagggtgacaaacgcgccaagcgactgcgcgagcatcgggttggtagataagcccccgccgacgtagcactcgaatccgggtcccagctccgggtgctcgacgccgatgaaggcgaggtcgttgatctcgtgcaccacgtcctggcgcgcgttgccggagatcgcggttttgaacttgcgcggcaggttctggaactcgtcgtcggtgacgatctgctggatcttttcaatcgcgggcgtggcgtcgatgatttcgtccttggcaatgccggccaccggcgaaccgaggatcacgcgcggcacatcgccgcaggcgtcccacgtgttgaggccgtgcgcctcgagcttgtcccagatcgcgggcacgtcctcgatcgccacccagtgcagctggatgttctggcggtccgtcaggtccacggtggagcgggcgtagtcgcgcgagatctcgccgacagcgcgggcctgggcggtggagcagatgccgccatcgaagcgcacgcgcatcatgaagtacttgtcttccagctctttgttgtccgccccggtgtgctcaccgcccaggttctgcttgcgctgggtgtacaggccgagccacttgaaccgcgggtagaggtcttcgcggtcgatggagtcgaagccctgcttggagtaggtgtcaatcacccgctgcttgacgtcccagatcgcggattcctgcttgatctcttcgtcgtggttgaggggcgcggggccgtcgacaagccactgcccctctggcttctttgtccgcttcaccgttggtgcgctcacgggcaactccttaaacctagaccgctctgtcttttgcgccattacttaacgacgtcctccgggtagcctgccgtaccgtgcggtctatcgcaaggccgcgtcaagaaaaggcgtgctgatctgggtattagcaggtgaatagaatgcgccgtcggggacgggtgaagttaatttggcagcgggtggaagacagcttggtctatagactatattggcttggagaaaagagcacccacacgaaaggaacgtgtaaccaatgagcttgcgtgtcgccgttgtcggcgccggcccggccggaatttacgcctctgacctgctgatccgcaacgaggagctcgacgtgcacgtcgacctgttcgagcagatgcccgcccccttcggcctgattcgctacggcgttgcgcccgaccacccgcgcatcaagggcattgtcaagagcctccacaacgtgctggacaaggacaagctgcgcctgatcgccaacgtcacagtcggccgcgacgtcaccgtcgaggaactgacggactactacgacgcagtggtgttctccaccggcgcagtgcgcgaccgcgaactgctggtcccgggcggcgacaagtccatcggcgccggcgagttcgtcggcttctacgacggcaacccgcgcttcgagcgcaactggaagctcgacgcgaaagaagttgccgtcatcggcgtgggcaacgtggccctcgacatctcccgcgtgctggccaagaccggcgacgagcttttggtcaccgagatcccggacaacgtctacgagtcgctgaagcagaacaaggccgagaccgtccacatgttcggccgccgcggccccgcccaggcgaagttcacgccgaaggagctgcgcgagctcgatgagtccgacaccatccaggtgctcgtcgaccccgaggacatcgactacgaccagctttcggaggaagtccgccgcgccgacaagtccgtggacctcgtgtgccaggtgctcgagcagtacgccatgcgcgagccggacgacagcccgcacaagatctacatccacttcttcgaggaaccggtcgaggtgctcactgacgacgccggcgagatcgtgggcttgcgcaccgagcgtcaggagctcgacggccagggtggcattaccggtaccggcaagttcaccgactggccggtccagcaggtctaccatgccgtcggctaccgctcggaaccggtcgagggtgtgccgttcgacttcgaccgccacgtcatccccaatgacggcggccacgtccttgctgaggccggctcatccgagatcgtgcccgacctctacaccaccggctggatcaagcgcggtccaatcggcctgatcggcaacacaaagtccgatgccaaggagacgaccgacatgctcatcgccgacgctgtcgccggtcgcctcatcgcgccgacccacacgggtgccgacgacatcttcgaccttttgcgggagcgcggcgtggactacgccacctgggaaggctggtacaagctcgacgaggctgagcgcgcgctcggcgccgccgaccccacgaacccgcgcgagcgcaagaagatcgttgagtggaacgagatgctctcccactcccgcgccggccagtaaggccccgtggcgggagcgggtgtctgaccgccgctgggccacccgggaggacctatcctggttcgcatgcaatggctggccacgacgcagcggttcttgaacccgacttggcggcgggcgacggtgctcgtgctcatcgcaatcctgacggcgcttttcgtattcgactgggtcacggtgcagtcaccttacggttcggccggcaccgcagccggcgccacgctcatcgccgtgtgcggcgcctgctgcgcggcgcacggcgtccgccccgtcacagccgtcgccgggatcgccgcgtgcgccagcttcgcgctgtttctcaacgcgctgagcgtccccctctactgggagccagcgctcgccttcggcgcggtcgtcaccacctcccgggtgccccggcgcgaccgcacctggctgaccgtctggctcctcgcgatacccaccgtcgcgcttttcacccacagcatgttcacgccggactggccgggcagtcagtcggcgggtcgtgccgccgccgtcgcggcccgcgcggtggcgctgtcatgggtcgtcctcggcttctttttccttctcggtgctcagcttcgcaaccggcgggaaaagatctccgagctggagcagcagatcgaattcgctcacgtccgcgagcgcactcagatcgcgcgagagatgcacgacatcgtcgcccacacgctcgccgggatcaccgccctggcggacggcgcgcgatacgcatccaaacacaacccggaggtggccagggacgcccttgaaacaatcagcgccgaatcacgtaccgcgctgtcgcagatgcgcgggctactcagcgtgttacgcgacgacgacgccgcagcacccaccggcactgccccgggccgacgtgacttcaccgctctgttcaacgaagcccgcgcccgtggcctcgacttaagcgtcgcgggcttcgacgagcttccagaggatgtgccgccactcacgcttttcaccctctaccgtgtctgtcaggaggccatcacaaacatgctgcgacacgcgtccgcaccggaaggtgcgctcaccttttccgccgacgcgaagtcggtgcgtgtggaggcggtcaacgctgcgccgaaaagcaagcacggccccgacggtttcgggctggtgggcatccgcgagcgcgtcgcggcgcacggcgggcgcgtgaacgtgaccgacgacggcggcgagttcgttctgaccgcggaggtgccgcgatgatcagcgtcgcgcttgtggacgaccagccgctcgtgcgcgccggcttctccatgctcgtcacctcccaggacgacatggacgtggtctggcaggcgggcgacggcgcgggggtggccgggcagccggcggcggacattgtgctcatggacatccagatgcccggcacggacggcatcgaggcctgccgcgcgttgctcgccgagcaccccgacacccgcgtgatcatgctgacaacctttgacgagcgcgacctcgtcctcggcgcgctcgacgccggggcctccgggttcctgctcaaagacgccgaccctgacgagctgctcgacgcgctgcgcactgtccacggcggcgacgcggtactcgcgccgaaggtgacgcgccacgtcatcggcgccgcgcaagcccccgagcagcgggaggcggcacgcaacgaggcgatgctcgagcgcctcaccccgcgcgaggtggaggtccttcgcttggtggcgctcggctactcaaacgaggagatcgccgaggccgagacgctctcccccgcgacggtgaagacgcacgtgcaccgcattctgttcaagaccgagtcccgcgaccgcgtccacgccgtcctcttcgcgttccgcgcgggcctggtgggcaccagcgagttgctgggccactagccgcgtacacccgagggtgtacgcgccgatttacacccgcgggcggacgatttctcccgcaccacgcgcgattgtgggaaccatgatcgacgttcacaacctgaccaaacggtattcaagctccaccgccgtagacgcgctgtcgttcaccgcgccggacggtgccgtcaccggtttcttgggcccgaacggctccggcaagtccacgaccatgcgcatgatcgtcgggctagaaaccccaaacgagggcgaggcgcttatcgacggctccactttccgatccctcgaccaacccgcacgcgtcgtcggggcgctgctcaacccggaatggatcgccccgcacacgactgggcgcggccacctgaagatggtcgccgactacgccggcgttcctgaatcccgcgccgacgaggcgctcgaggcgttcgggctcgcggaggcgtcaaaacggaaagtgaaaaactactccctcggcatgcgccaacgcctcggcgtggccagcgcgctgatcgcggacccatccaacgtcatcctggacgagccggtcaacggcctcgacccgcagggcgtggcctggatgcgggggcgcatccgcgagatggccgccgagggccgtgcggtagtcgtctcttcgcacctgatgagcgagatgcagctcactgcggaccgccttgtggtgatcaaccgcggccgcctcgccggcgagggcccgctcgaggacttcctgggctccaaccgggttgaggcgacctgcagcgacccggcgcggctggccgaggccgtcggcggccaggtcattggcgactccgttgtcgtcgacgacgccaccgcccgagacgtcggcgaggccgcccagcgcgccggggtgacggtttactcccttcaggaatcccgccgcagcctcgaagaagtgttcctggaatcaacgaaataagacgtaggaggttttccatgcatacgttgaaagcaaccctgcgggaggtcttctcccgccccgcgacgcgcatcctgctcgcattcgtcgcggtcgccctcattctcggtcccataaccgtagcgatgctccttggccccaacggaacaaacgtcgcagacccggcgatgctgctcatccccgccaacttgatgctccccgtggcgctcgccgcaggcgccttccccgccggcggcgcacactcgcgcggcacgatcggctacgcctacctcgcgtcgaaccaccgcggctgggagcttgcctgccgcgttggcgtcgcagctctcgcctgcacactgacggcgtttgctgcctcggcgatcgggctcggcggcgcgcacgcgttcgtcgacagcgtcgcgctgggcggtgccgacagcgcgggtgcggtgcgctaccaggccgagctgtggatcgcctacccactgcttgcggccctgacagccgtgctgctcggctcgggcaccgcgtccttcttcgtctgggtcgtcgagttgctcatcgtggagactgccctcagtgcgatcaaccagccgtgggccgcggtcctggagaagctcctgccaggcggcgctgccgggaacggcacggccggagtagctaccctcgtggtgtgggtcgtggccctcgccgccgccacgtatgcggccgttcagcggagggcagtgaagtgaccgcaacagagaccacaacacacaccggtgagcgcaccgcggcccaccagcggttcgtggcccccgacctcgcccgcgggttcgctctcgtcggcatcgcgatggccaacatggtcactgactgggaccctgccgagggcgtcgaccacgcggcgggcctcggcggctacaacggcgacggcaccgtgttggagaagctgctcgtcttcttcgagacgctcttcgtgcacgtgcgcggtttgcccatgtttgccaccctgctcggtgttggcgtcggcatgatctttgccagcctcgagcggcgcggctacccgctgcgcgcccggcgcatggttctcgcgcgccgctatgggttcctgttcctgttcggcctagtgcacaagacgctgtttttcaccaacgacatcatgaccgcgtacggcatcgcggcgcttatcctgtgcctgttcatcgggtggagcgaccgagcactctacgcgctcgcaggtgcagcgttcgccctgaacgcggtacttcgtgcccctggtatattcgccgcgttttcgtcggcagcggaaccgataggcggcagccccgcgcgcatcgttgacctcggccagcgcatagccgtcggcctggccaacttctgggtgtacccggcaatgggcgtaatcgagatgctcgccttcttcccgcttgtcgtggtcgggtttgtctggggccggcgcggcgtctttggcgacgtaaacggcaattcccggatgctccgcgggtgggcaattcttgcggccatagtcatggcggccatcggcatcccgtggggctacggggaaatcggcgcgctcggacccgggtgggctacagggctcactgccgccaacgggcttgtcggcatgctgaccggccccggtatcctcgccgcaatcaccctcgcgtgccggccgttgcaatcgcgtatcaacgcctccggcactctcccacacctagcccgacccctcgtggcgctggggaaacgttccatgagcggctaccttgcgcaaacgattctcttcaccctgacaacccagcccgcgttctggtgggtaactcgcgacgcgacgatctccggcaaactcggctgggcgctgattacgtggctggccacggtagctggtgcgtgggcgcttgagagggccggcaagccggggccgttcgaatggctgcaccgtcgcctgtcgtacggcaaaaacggcctgcccgagcactaccacggctaggcgcccagagcagacgcgcccggacggtaccgtgcccacgctcgagccgtgcgcgatgcgacggaagtataggattgcccgggcaacgagaagaaggggcatacgtggatctcatccgactcaccgcgcgcttcggcaaaccctacgccggccaattcgcattcgtcatcgcgttacagctggtcactaccctggcaacgctgtatctgccggacttgaacgcggacatcatcaacaacggcgtcgcgcaagcggatgtgccgtacatctggagcgtcggccgcaccatgcttctcgtcgcattcatccaggtcatcgccgccatcgcggcggtgtggttcgcctccaaggcggcgatgcaaaccggacgagacctgcgccgcgccgtctacgaccaggtcgcaggcttcagctccgaggacatgagccacttcggcacgcccaccctgatcacccgcggcacgaacgacgtgcagcaggtgcagatgacgctgctgctcttcctcaacttcatggtcaccgcgccgatcatggccatcggcggcatcatcatggcactgcgccaggacgcgggcatgtcgtggctggtcatcgtggcagtggtgacacttgccgtcgtggtgagcatcatcgcggcgatcctcatgccgctgttcaaacagatgcagaacaagctggacaccatcaacggcctgctcagagagcagatcgccggcatccgtgtagtgcgagcgttcggccgcgaggagcacgaagccgaacgcttcaccgacgcgaactcccagctaacgcggctgagtctcaacatcggccgggtattcgtcaccatgttccccgtcatcatgctgatcctgaacatggccaccgccgcggtgctgtggttcggcggccaccgcgtggatcagggcttggtcgaggtcgggtcactcaccgcgttcatgcagtacctgatgcagatcctgatggccgtgatgatgggcgtgttcatgttgatgatgttgccgcgcgcggtggtgtgtagccgtcgcatagcggaggtactctcgcacgagcctcggcaagctgagccgaccaacgggggcgaacttcccggccgcggggtgctcgagttccgcgacgtgtcctacgcttacccgggcgcgtcggaacccgtgctcaaggacacttccttcaccgcccaccccggcaccaccacggcgatcatcggttcgacgggttccggcaagtccactttgttgggcctcattccgcgcctctacctccccaccgaggggcaagtgcttatcgacggcgccgacaccgccaccatcccccgccaaaatctcgtcaacgccgtttccatggtgccgcagaaaccgtggctcttcggcggcacggtggcgtcgaacctgcgcgtgggcaaccccgatgccacggacgaggaactctgggaagcgctccgcgtagcccaggcaagcttcgtcgaggacctagagatgccgatctctcaaggcggcgcgaacgtttccggcggtcagcgccaacgcctgtgcatcgcgcggatgctagtggcgaagccagacatctacctgttcgacgactcgttttccgccctcgacgcgctgacggagaagaacctgcgcgaggcgatggaggagtacacgagggagaagacggttgtggttgtggcgcagcgggtggcgtcgataagcaatgcccaccagatcctggtgatggaggccggcgagatcgtagcgcgcggcacccacgaagaacttatggagacaagcgagacgtaccgcgagatcgcgcgcagtcaagaggcggtggaggcgtgagcgagcagatgaacgagcacgaggcgaacgcgccgcgcaaggcgaagcacttttggccgtcggcgaagcggctcatcgggcttttggcgccgttcaaggcagcgctgactgcggtctttgtcatgaacgcgctgtcggtggtgttaagcgtctacgcgccgcgcgtgatggggcgcgcgatggacgtgatcttctccggcgtggtgtcgaagcaaatgccgcccggcacgacgaaggagcaggcggttgagggcttgcgcgcggcgggtgaggaccggttcgccgacatggcggaagcgatggacctcaacccgggcgtgggcatcgacttcacgcagctcggtgagctcatcgtcgtggtgctcgcgctgtacctcgccgcctcgctgttgatgtgggcccagggcgcgatcctgaaccggctgaccatgcgcgcggtgctcgacctgcgcgagcgcgtcgaggcgaagctgcaccgcttgccgctgtcgtacttcgacgcccgcgagcgcggggatgtgatgagccgcaccaccaacgacgtcgacaacgttcagcaggctctgcagcagtccctgtccagcctgttcaacgcgattttgacgctcgtcggcatcatcgtgatgatgttcgcgatctccccgcagctggccctggtggcgctgctcgctatccctctgacgggtctggtgatgggcctggtgggcacacggagccagaaacagttcgtcacccagtggaaggccaccggcgaggtcaacggccacgtcgaagaggcgttctccggccacgacgtggcggtgatcttcggacgcacagacgagatggcgcgcgagttcgaccgccgcaacaacgaacttgcgggtgccgcgcagaaggcgcagttcctctcgaactcgatgcacccgatcatgcagttcatctcgtatctgtcctacgtcgcgatcgcggtgctcggcggggtgaaggtggcctcgggcaagctcacgcttggtagcgccaccgcgttcatccagtactcccgccagttcaaccagccgctcggtgagatcgccggcatgatgcagatgcttcaatccggcgtcgcctccgccgagcgcgtcttcgaactcctcgacgccgaggaggaaccgcaggacctggccgcagccagcctcgacactccggcgcaggggcttgtcctgcttgacgacgtcgccttttcctacaccgacgaccccttgatccaaaacctgaacctgcgggttgagcccggtcagacagcggcgatcgtcggtccgacgggcgcgggcaagactaccctggtgaacctgatcatgcgcttctacgacgtggacgccggctcgatcacgctcgacggcgtggacatccgcgaccttagccgcgccgagcttcgctcccagatcgggatggtgctccaggacgcggtcctgttcaagggcacgatcatggacaacatccgctacggccgcctcgacgccaccgacgaggaggtcatcgccgcggcgaaggcgacctacgtcgaccgcttcgttcgcacgctgcccgacggctacgacaccgaggtagaccaggacggcggctcgatctcccagggcgagcgtcagctgatcaccatcgctcgggcgtttctagcgcagccggcgctgctgatcctggatgaggcgacctcgtctgtcgacacccgcaccgaagtgctggtgcagcaggcgatgaacgccctgcgcgccaaccgcacctcgtttgtcatcgcgcaccgcctctccaccatccgcgacgcggacgtgatcatcgtgatgcgtgacggccagattgtggagcagggggcgcacgcggagctcatcgcagcccgcggcgtgtactacgagatgagcaagacccagttcagcgaggacgtgtaaggacgggtaagttcctccaacgttcaccttgcgttcattgatcaaacacccaggttccgtagtgtcaggcgagtaagtctgccgaaatgaacataagagattgggttgcaatgagcaggaagaacgacgagggcctttacaccggcgatgccggtgagccccagcgcggcgccggtcacggcaccgagcacgccgccgaggacggctccggtgtgcaggtcctcgatgaggccggccagtacgaccagaacgcccgctggaacgaggaagcggaggccaaggatgacgagaaccgcaacctttccgacaacgaggtcgatgacgacgacgaaaagaaggacccgctcggattcctcccgttcgagggcaccgcgaagcaggtagcgaactggatcgccgtcatcctcggcatctggctgctgctcaacggtgtgggcatgattggcgacggcttccagctcatcgccggcgaccgcgccgaggagctcttctcgtttgccgagaacccgttcgtgggtctggccatcggtatcgtggccaccgccatcatccaatcctcctccaccaccacctcgatcgtggtgggcatgatcgccggtggtctgccactgaacatcgcgatcccgatgctcttcggcgcgaacatgggtacctcggtcacctcgaccctggtggctctgggcttggccggtaacaagaagcagttccagtccggtttctccatggcgaccgtgcacgacttcttcaacgtgatcgccatcctgatcttcttcccgctggagatgctcaccggcttcctgggcaagaccgcaaccgcgatcgccccggcgctgtccggtacgggcgaaggcgtcgtcgctggcatcttcgagtccatcggcgacttcatcgacatgctcaccgagccgttggtgggccttgcttccaacctggttgagccgctcagcgacgtgtgggccggcatcatcctcgcgctggttggtatcgggctgatcctgttctccatccagttcattggcaagatcctgaacgcgctgctggtgggtaaggcgcaggagatcctctacaacaccctgggcaagaatgcgttcctcggcgtcctctcgggtgcggccatcaccacgctggtgcagtcctcctccaccaccacctcgctcacggtgccgctggcagcgtccggcaagttcaaggtgcgcgacctgttcccgttcgtggtcggcgccaacatcggtaccaccgtcaccggcctgatcgcggccttctccgcctccggcgccgaggccgaagccgccatggccggtgcgttggtgcacaccctgttcaacacgtttgcagccatcctgatcctgagtgtgccgttcctgcgcaagctgcctccggccggctccgattggctggcgggcctcgcaacgaagaacaaggtctacgtcttcatctggatcggtggcgtgttcttcctgatcccgatcttggccgtgttcatctcgaacgccgtgtcctaacaacaacgcgatacaaggagcgcacccatgactgagaacgagaacatccagacccccgatctgacgccgatggcccatgacctgatccagaacgaggccccggacaacgccctcgtggcgctactcaacgagctggaagaaaccgccgctgagctgcgcaccgagctcgaggcgcgccacggacatcgccagcaggcggcagctgaagctcacgaggcgggcgccaccggcgccgccaccgaggtcgccgcagcccccaagacggccgagcgccacgtgaagaagaacccgaacgtgaccccggagcaggaagccgagctgaacgagaacttcgaggagtactggaccaactcccagggctcctggaagaacctcttccgcctgctgcgtgagttccgcaccgaaatgaaggagcacaagcagcatggctaagttcccccgccgcgccaccgccgtggcgctgaccgccaccacccttttggccgccgcctgctcgtcggacaacaccccgggcgaggacgcgatccaggtcaccggctcctccacggttgagccgatcacccgctacatggccaaccgctacgactttgacgtcaacatcgagggcattggctccaccgacggttttgagaaattctgcgccggcgaggccgacatcaacgacgcctccgtgtccatcccgggcgaaggtgagccggtggactaccagaagcagtgcgccgacaacaacgtggagtacgtcgagctgcccatcgcactcgacgccatcacgattgtgaagaacaccaagaacgactgggcgaaggacctttccatcgagcagctgcacgacatctggtcgaaggagtcctccgtgaccaagtggtcggacattgacccgtcgtggccggacgaggagatcaagctctacggccgccccgccggctccggcaccttgggggtgttcgagacgctcgtgctcgacggcgacaccatccgcgaggattacgagtccaccgacgacatccaagagctctcctcctgggtcgcggacgacgtgaacgcgctgtcgtttatgggcatcggcaactacctcgccaccgaggacccgacccgcagccgcatcgacaacgtgctggtggacggcgtcgccccgtctgccgaggaggcgaagagcggcaactacccgctggcccgcccgctgttcatctacgtcaacgaggcctccgccaagcgcgaggacgtggacaacttcgtcaccacctacctggacaaggtggaggcggtactgccgcgcgtgtacttctaccagttgcctgaggaggagtacggggcgtcgcaaagccggtacgcagaccgcgtcaccggtatcgacgagcgttggcactaagccccgagggggtgcttcgcatatacgatgtgaagggtgagtaccccttacggcaacttcagaatcggtgacgccgagcgcatggaggccatggatgtccttggccgcgcgctcggcgaaggccgtctgaccatggctgagttcgacgagcgctgcgcgttcctggcaaaggcgcagacgcacgcggacctcggaccgatcttgtcggatctgccgactggccctcccccgtcggcgcaagcgcagccttcgcacgatgtcacgctgtactcccaggccgagatcatgcaggcccgccgcgccggcaagcgcacccgcgccggcgtcttctggctcggcaccatcggctctatgggcctgaccgcagtggccggcgccgcggggttggacgccctggcgggcctgtcgctactgctgatccccaccctgttcatcctgctgtacgtgatgaaggtcggcccggactcctggtacatgccgagcctgcggcagctggagatgcagcgccgccaggagttgaaggcccgccagctggagatcgaggccgccaaggcgcagcagcaagcgctggtgcgggcgcagcgccaggaccagttcaaccagatcaccaccgacgcgctcgacgtcgcccaccaaaccgtgaaccgcttcaggaggaagccatgaatcaccggcacttcgaccaagccgacaagctgaaaaacgtcttctacgacatccgcggcccggtgagcgcgaccgccgagaagatggagcgcgacggccacacgattctgaagctcaacaccggcaacccggccatcttcgggttcgaggcaccggacgtgatcatgcgcgacatgatcgcgaacctgcccacctcgcagggctacaccacctccaagggcatcatttccgcccgccgcgccattgtcacccgctacgagatgatcgacgcattcccgcacttcgacgtcgacgacgtctacatcggcaacggcgtgagcgagctgatcagcatggtcacgcaagcactgcttaacgacggcgacgagatcctcatccccgcccccgactaccccctgtggactgcggcatcgacgctggccggcggcaaggtcgtgcactacctgtgcgacgaggaggacaactggaacccgtcgctggaggatatccgggagaagatcaccccgcgcacgaaggcgatcgtggtgatcaacccgaacaaccccaccggcgcggtctactcccgtgacgtgctcgagggcattgcgaacattgcgcgcgaacacgagctgatggtgctcgcagacgagatttacgaccgcgtgctgtacgacggcgcgcagcacatctccatggccgaagtcgcccccgacctagtcaccgtcaccttcaacggcctgtccaaggcataccgcgtgtgcggctaccgcgccggctggatgatcatcaccggcccgcgccgccgcgctaccggtttcatcgagggcttggacctgctctcaggcacgcgcctgtgcgcgaacgtgccaggccagcacgcgatccaggtcgcgctcggcggccgccagtcaatctacgagcttaccgccgaaggcggccgcctgcacaagcagcgcgacgtcgcggtgcgcaagctccgcgagatcccgggtgtttccgtggttgagccgaagggcgcgctgtattgcttccccaagatcgacgccgagatgtacaacatccacgacgacgagaagttcatgctcgacctgctcaaggcggagaaaatcctcatggtgcagggcacgggctttaactacccgaccccggaccacttccgcgtcgtgttcttgccgtgggcgtcgcagctagaaaacgctatcgataggttgggcaacttcctcgccgactaccaccagcactaagtttcgcggtttccgaaaattgccaaactttagcccagaagtttggtggtaggctttctcggcatggcgtggcaccaccgcatccgtggcggcagcgtcagcaggcctggcgctcccctgacgtcctttcgcttctcgacgacttcgccgccgcagctggccgtcggcttactagtgactagggcgggagggcgtctcggcctgcgccaaagccgacttcactgagctggccaaaagcaccatcgaaagaaggaagaggatgacgtaggtgcgaccgaacgccacgataaaggccacagagatgaacaccgcgagggtggtgatgccgatcgcaaacttggggttctgcagtttcatggtggcctcctagcagaaggtggcggcgccgaccataccgccaccgagcgcaccccagcccccactgaccgccccggccacaagcgcggagccaccagtgccgacggcacacttaccccagtcgctccaccacccgtaggtgacggcaccgttagcgccagtctgggtgacctgcagctgattgccgttcttcacggtgtagtagaagccgatcgtgtcgcgttccttgttcaccgcggcctcgggcagggtctcgacaacattgccggttgcgtccttgaccaccacgtctttaccctgttcggcgaaagtcgcaccgtgtttgagggaaatgaggaggtcgcggccgttattcgcggtggagaatacagcggtgtcgttctcccgggtttcgacggtggaagcggcagtactagcggtggccaccatcgccggtgccacggctgcagcggtcagggccagggtgaaagcgggagcgacaaccgccttgcggaaggaaattgagcggtacatgggtaaaccttgcaacagtcgagggacgcatcgtacgaggaggactgtatgcgcactgctgcaggatgaacatggctagcgctggctttcggaccttcgtccccgaatccggcactttcgatccctctcgacggtgcggggcaccggttggttgctgtgtgggaaggggagggcgtcgataagcaaaatgctctgcttacggccccaacaaagacacgggcgctacaacaattccgtcggggcgggtgtacgcgggaccgcccccggtcaccacgagcaggataggatccgcttccagttggtcggcgaagcggagaagcgtactcgccgccgcatcgatcacctgcgggtagtggcccaacttgacctccaccagaatcggacggccattgataggcacaaccgcgtccacctcgaggtttgtgttcaaccgcgcgtggtagacctgctcgtcgctgtaggcgcggagttcgtggacaacgaaagactcgaacagctggcccgcgtattcgtagtcgttggcgatatcgcgcggctgccgcttcagcgcagcgacagccaacgctgggtcgacgaggtgccgcttcggagatttgcggagtgtcgccttcgaccggagatgggcagaccaggcgggttgatccaccgaaatgaagatccgcgagagcgcgtctaggtaatcggacaccgtttctcgcgcgaccccagcatccttggcaagggtttgcacgtcggcctcagtgcccacgttgcgcgcgatcgaggcgaggaggcgctccaccttctccgggcttcgctgggcaccgtccggagtccggatatctacgtgtgcaacttgctcgacgtattctcggttggagcggagcgcatccggtgtagaaagcccgacgttatcaggccagccaccgcggcacatcctttccacaagcgcgtccaagctcatcgcgctgtcgatgtagcttggccgctccgcctccgcaagagcgctgagcgacacctctccagacgactcgccagtctcgaacatggtgagcgtagacatggtcacatgcgcaaaccgcccggccccggaatggcgtgtgagctcctcggtcggaaccgtcgaccccgtgaagatgaactgccctttcgtttgccgccggtcaatcgcgtgacgagccaaatcccaaagctgcggttggaactgccattcatcgatcagccgcggggtgtcgccttcgagcaggcttgctgggtcacttcccattaaaaattgcacccggggatccgtgtccacattgagcacgctgcttgattgctgcagcgatgtctcggtcttgccacaccctttcgggccgcggacgaggactccaccctttcgcctgagcgcgttttctaagcgttgatccgcgatccgcggaatgtacataagctgctactatacgcgcaacccgtcagattgtaaggcgaagactcgtcagattggaacgctgggactcgacagattgtaatgttctacaagctgcggcccagcgcgcgcagttcccagccggcttgttgccaggaggtgacggggaggacgttgcgggcgtcgataagcaactgcttttcgaccagccctgcagcccacaccgggtccatctccttgaactcctgccactcggtggcgaggatggtcagctccgcgccgcgcagggcgtcctcgagggaggcggcgtaatcgagggtggggaacaccttgcgggcgttgtccatgccctgggggtcgtacacgcgcaccgcggcgccggcgagggaaagctggccggcgacggcaagcgccggcgaatcgcgcacgtcatccgagttcggcttaaacgcggcaccgagcacggtgatgcgtttgccgatcagcgaaccgagcatctcgcgggagagatccaccacgcgctggcggcggcgcatgttgatcgcgtcgacctcgcgaaggaacgtcaacgcctggtcggcgccgagctcgccggcgcgagccatgaacgcgcggatgtctttcggcaagcagccgccgccgaaaccaaggcccgcgcccaagaacttgcggccgatgcggtcgtcgtagccgatcgcgtccgccagctgggtcacgtccgcgccgacgatctcgcagacctcgctgacggcgttgatgaaggagatcttcgtggccaagaacgcgtttgcagagactttcaccagctccgcggtctgcaggtcggtgacgataaacggggtgttgttagccagtggcgtggcgtagacctcgcgggcgatttcctcagctcggctctctccgtgcggggcgctcgcgccccgcacgccgaggacgatgcggtcgggttcgatggtgtctttcaccgcgtagccttcgcgcaggaattccgggttccacgcgatctcgacggtggcgttgttgccgtgcttagcgatcagctcgtcggcttgctgctgcagctgagccgcggtaccgaccgggacggtcgacttgccgaagatgacgtggtggccctcaagcttcggcaccaagtcggcgatcacggcctcgacgtagcgggtgtcggcggcgtacgagccgcgctgctgcggggtgcccaccccgatgaagtgaacgttggcaaagtctgctgcctcgtcgtagtcggtggtgaagtcgaggcggccggcggccatgttgcgctcgagcacctcgggcaggcccggctcataaaacggcaccttcgacgccttcagctggttgatcttgttttcatcaacatcaacaccaagcacctcgtgccccagctccgccatacacgccgcgtgggtcgcaccaaggtagccagtaccgatcacagtcatacgcattagaaagaccccttctcaggaaaatggtgaagcagcgcgtttaccctgcacctagagcacgtgttgatcgcagatttcacgccctacagagactcgtgcgggcacattgcgagcaaacagggcgaccagtttgtcctgctcatcaatcgttcacatcttgcacgatcttaatggtcttcagcgctctacgcagtgctgatttccgacaaacgaggagacttcagcaggcggatgcttcgtttactagtttctaggcatctagatacgtagtttctttcgcttgaaagtcttgatgcgcttcttcccaagaaacgccaaagtagtcctcccaagagtccataccgaattgcacatcgccacgagcatcttcaagactcacgatgtgcatttcttgcaccacatcctcagttgcaagcgcttctatctgctccactgccgcatcatctgtacgcgcttccaccgtatatgtgccgcattcaatgaagacctcgaagtgcttcctgcttgttttgaagaggacgatatccgggttctttgcgtacatcatcatcgggaagctcttctgcgggtgctctagagcattcgtaagggcctcttcgacgtatgcattagcaagaagcgcgtagagcgttgatgcggcaagcgatagagcagggtccaagccctcatcagcaagttcgccatctacttcatctgggtcaaggcttaagacttctacatagcgctccagcgcatcggagagctgctccgccttctcctccggcttaagtgaagagtccttgttgatatccgcgatctctgctgcataacggaggattttggatttcctggccgtgaagaaaaagttgagcgctgcgtccacgtcgatacggcgcgcaagctcccaaatctcatctttgttgatctggttgttcgactcgttggtggggaaaaacagttgtttcgccattttgattctcctagcggcacggcggagcaacagcccctcgcctaccaacccgtacgcaaggggcaggttgcttgtcgacgcccttacctagttcacattgcccttctcagcactgccctgcccacttccagtagcgtcaccgcccgcagccgggacattgccgtcgttccagcgggtgccatcaacgtgggtctcagcaccatcgaccgtgcgaacctcgccgtcgatgtcagcagtgttctcgcggccgttgtcgtgtccgtgaccgtgaccgtgtccgccgcagcagctggacttgggggtctcgttcgcgccgtggcccttgccgcattggcactcgccctcagcgcagccgcaagcagaaccctcggccggcgcgacagttgcgtctaccgagccctcagcgggaacgatcttgatctcttcacgcacgtgggcgtgatcggggttgaccggcttgtcggcgtggttgccgcagccgcaggagtggtgctcgttcggagtagtcatggtctcaaggttacgcgcttcgccaacatgcgggcgcgcgttaacggaagtttaggtacgccttcgacggcgtcgggccgcgctgaccttggtacttcgaccccagcgcagaagatccgtacggagtctcagccgccgaggtcatggcgaacagtgcgagctggccaaccttcatccccggccacagcgtgatcggcagatttgccacgttcgatagctccagggtgatgtgtccggtgaaacccgggtcgatgaagcctgcggttgagtgcgtcaaaagccccaggcggcctaacgacgacttaccctccaaccgccccgccagatccgccggaagcgtgaattgctccaacgtcgcggccaacacaaactcacccgggtgcagcacaaaaggctcaccttcgggcacctcaacaagcgtggtcagctccggctgctcctgctttggatcgatgtgcgtgtacttcgagttgttgaagacgcggaacaggttgtccatgcgcacgtcgatcgagctgggctggatcaggtcggcgtcgaacgggtcgataccgagccggcccgattcaatggcgtcgcggatgtcatggtctgaaagcagcacggcatataagtgtatcggcccgacccccaagttttttgggctcccccgtgccagtgctaaagtaaccctcaccgcaagatgccggcgtagtttagtggtagaacatcagcttcccaagctgagagtgcgagttcgattctcgtcgccggctcaaatttgaccagggttttaccctggtccttttgttttggcgacccctacccacgagacaatcgccgcacccggacattggcaaagtgttgcttgcaaagtgttgcttgcagatggtcattagccgagaaaacgacgactcggcggggaccagctactcggttaatgaccatctgccggtcaccatttaggggttaccatttgcaattgccctggtagcgaacgtggcgcgttgcgggggcaccgaccgcaccgaccgcaccgaccgcaccgaccggccgtcaaacgcaaaccaccctcacgcgatacacggcccgatcggcgccgtcgaatacatgaagcacgcccggcgctgccgcccatccgcatcctcctcccccgcgccgcgcagtatgcggaattcttggtggacttcggtggcgtcgcgaagccggtcgggcgcgtggtggtaaacggtgaggatcccagcgggcgtggccagagaaactttctggccctccgcgctgaggaactcaacgggttcccactcctcggcgggacggtgagccgccttcaaggctgggatgtgatgcgggcggtggccgtcgagaatcagggtgcattcggtgtggtcgacgaaccgctgcggggcctccagaacaggcagatcaagaacctgaccggcggagttgcgcacggcgttcttctcggcggaaaactcaaacgacatgccggcttcggcgacgaagccaacggcgccggcagccgaagagaacgtgcgcagaaccgggatgtcgccggcaacgaaaacgatggtggcgctgcttaaggcgcgcagcatggcgggggtccaatcggacatgggaaaactccaaagaaatactcgctacttccggcgcgcgggtcgcttacgccggccgatcttcccccgggagcaccgtgcgcggtgggcgcggttgctagttgacgagccgggggtctttcaaccgtcaggacttctggatcgcttacccgacgatactagacagcttggtctatgggcaacgtcgtcaagcacaatgctccctatgcgacttcttgtggcggcgctgtgggccgaaggtgcgcggcgggcggctgagacccgccccccgcttccgttcaacgaccccgatttcgtgcccgcgcacccgacgccggtggtgtacctgcacggcatcaccgcgcgcgtgcgcagcttccggcagaacgcggagcttctgaaaagccgcgggtactgggtgtggggccacgactacggcgacatgttcgcgccgggttttcgcggcgtgggcgacctcgacctgattgtcgacgacgtcgcggagaacgtcgaacgcgtgctgaaagcgacgggtgcgaagcaggtggacttggtggcgcactcccagggcggtttgatggccaagctgtacatcgccgacggcggcgccgagcgcgtgcgccgcgtggtggcgatgggcgcgaatttccacggcacggacctcgccgggcgcgcccgctggtttgagccggtgattgcgaagcacccgcgcttttcgtcgttcgtggcccctggcggggtgcagcagttggtcagctcggagtggaacgcggcgcacgtcggggtgccggacaccgatccgcgcgtggtctacacctcgctgtactcgccggcagaccgcattgtcacgcccaacaccgcatcaaaactggtcgcggtcgacggcgcggacgtagcgaacatcgacgtggcgcagtggtacgacggctacgcgccgcgccacccgatgatgccgcgcgacccgttgatggctgagctcaccgcttggggtttggagcgcggccccggcgaaacgcacccgccggcgcttgattggttggcgtagcgttgccaccatggcacgcaacgacgaactgatcagcttcatcctgctcggcggcacgagcgacctggcgatgcgtcttctgcttcccggcctcggcgagtacgcgcgcgcaagcggccgccgcttcgaggtcatcggctccggccgcgacgaggtggatagctaccaggcgatggttgacgaggccactggcggcggcatcccggcgcgctacacccccggcgacgccaccgagcaggcgtatttggagcagttgcttaattgcgcccacggcaaccacaccatcctctacttcgccctcgcgccagccgtgaccatgcgcgccgtcgaggcgctgcgcggcgttgagctgcctcctcgatccgcttcgccatggagaagccgtacggcgtgagtgccgcggacgcggacgatttggaccgggcgctgcacgcgctggttggtgaggacgcgatctaccgcgtcgaccacttcctctccgagccgggtgtgaacacggccgccgcccgcgtcgccgccgagggcgcgccggagacgctgtcgctcgtctttgaggagtcgctcggcctggagggacgcgccgagttctacgactccaccggcgccgccgaggacatggtgcagtcgcacctgatccagtccgcggcgcgcatcttggccggcgggccgaatcccacccgcgtgcgcgaggtgcttgactccttcgagctggcgccgggatcggtcaagcgcggccgctacgccggctacgcggaggaagcaggtgtggacccctcgcgcgaaaccgagacgcttatcgaagtcgagcttgaagcaccggagacgcgcgtgacgctgcgcaccggcaagggtttccgcgaggacgtcaaagagatccagggcgtgccgctggccaacggcccgctatcgccctacggcaacgttatccgcggcgtggtcgagcgcgaccacaccgcctttgttcccgagggtgcggcgcaggctgcctggcgcctgatggacgacatcaaggccgccatggcgcaagccccgctcgaggagtactaggcgctggccagcagttagccgcacttcacaatcggctgcggggtgtagaccgtggtctgggtttcgcgggagagctcgttgcccgcgaggtcgtagatcacgcgggtgtccgaggtggtgaagccgggcgcgccgccggacgggatacagctctcaccggtcacgcgctgctcctgcggctgcgtggtggcccaccgcccgccgttgatcgattcaacgttggtggtcttgacccccatcaggctgacggtgagctggccgccgcctgcggaggtggtgatcttcaccgggtacggcgagtcgtttctgaactgcaggtcgatcgcgccctcgaagaccgtggcctcgcggcccgccgggtagcgggagatgtagtacgagtgcggcgtgtgcgcgatgtccgtcatgcccgcgaagtaggcggcgttgtagagcgtggtcgcgaactgggagatgccgccgccgacggcggtgtccgcgcgaccgttcaaaatgatgccggattccacgtagccctgcgcggtgccgcggggaccggtgtaaccgttgagcgagaacgtctcgccagggttgacgatcgcgccgttgaccgtctgcgcaaccagcgcgatgttctggccggaagccgccgagtagccgctggtggtgaagctgcccaccacctcgttgaaggtggcgttggccgcctgctcggaggtgaacgccgcgggcaccgcctcgtacgccgcgtcccactcgcgcggggtggtgcccagcaagcggtcgtcgaagctctccatcgtcttcgcccagtccacctgggagccgtcgacagagtcggtgtagccgccgccggcgagtacgcgcgcgttctgcatctcggtctcggtgactgcgagctgctcgccgaggatcgcctgcgccgcttcgtggttgatctcgggggtgagcgcgccgtcgcgaaccgggaactggaccacttcgccgaggcggtcctgcgggatcacagcgtcaaccggcgcgccgtcgggctcgcccgcggccgggcggccgtgcaccgtcagcggcccgcgcagcgcggcgcgcaccgggccgtcttgggcggcgcggatcgcggcgtcgtccaccgcgggttgcagcacgtccgggtcaacctcgataccgccggggcgcagccagttgtccaccaccgcggggcgcagcgagtctgcggtcacgttctgccccggcttcggcgccgtcacctcggctgcgccgccgttgatgtggatcgcgccgtcggcaggctcgcggtgcagttcttccgaggctttctgcaacgcaggtgccagcttcgcctcgtcgaccgcggtcactgccggcacctcgtgctcggtgaacatgccgcgaaggcggctgaccgggttcgccgactcgatgcctgcggcgtccaccgtctgttgccagtccacggtgaggccggctttcgctgggaggaactcggctcgctcggaacccgccgcgatctcgaccgggttgttctccaccccgcccagctcgcgctccagcgcttgcttcgcgtcctcggggctcatgccgccgatggccaccccgccgaccgtggtgccgcgggggacgttgccgcggttcatagccaggtcggccaggtacagcgccaccagcacggcgaggatgccgaaaaggacaccgagggtgatctttttgcctctcacgcggttaagcgtactggttgtttacagccccacgctcatcagcatctgctgggtgcgaagcgccgcctcatcaatgcgctccaccgggatctcgccggtgttcactgccgcgaccacgtggtcgatgatgtgcggcaggtcagcgccggacgaccacagggcctggtcggcgccggccatgatggcgtacttcaccgcgtcgggcgtcggcgcgtagtccaaaatgccgcgcatcccggaaaggtcgtcggtgaccaccacaccgtcgtatggtacgccgccggggtagtcgccctcgcgcagcacccggtacgcctccgggttcaacgagctgggaacaccgtcgtttcccaaacccggcacgatcatgtggcccatcatcacgctcgccgttgggaagcggttcagcagcggcccgtacggcgccatgtccaaaccgcgcacctcgtccactggcggggtcaccgccaactggtggtgggtgtcgccggaggcccggccgtggccggggaagtgcttgaaggtcggcgtcacgccggcgtccaccaacccctgggagaacaggcccgccacgcgcacaacctcctcgggcgaggcgttaaacgagcggtcgccgacgatgtttaagtcggtcacgtccaaatccagaagcggcgcgtagtccacgttgatgccatggtgtcgaagggagacgccgatgtcgtagccggtgccctggatcacctcgtcggggtgggcggacagcatccgcggcggcatgaaatcgcccagcacgtgggtgtggcgctgcacgcggccgccctcgaagtcgatggcgacgctgaacggccgggcgtactcggcgcgcagcgcgttgatgttgcgcccctcctccaccaacagcgccgggtcggcccagctgggaatgatcagtccgcccgcgccctggtcgagggcaaaccgcgcctggtcgtagttggacacgccgacaaccatcagagatgcgactttggcgcgcaagtcttccgggacgcggctgtgggggctgacaggggcgctgtcaagcaactcaagctccggtgcggcgggaggggccaccaccggcgcttctgatgtctcggcagtctcgggcatgtgagggtcttgaggctcgtcaggctccccagacgcgcagccggccatgagcaacgcggccgtcgccacagccagcaccccgttgcgcaccccggtcctcctcgcgaattgctgttttgaaacgccatacactctacgcactgccggcacctgcccactggtaggctccaacccatgtcaacgacaacccagccagagcagcggcgcgcagcgtcgtccgtgctggcgagcgccgtcgtcggtgcggtgctgggcattgtcggcgtgctgggggtgggcgcgttcagcgggcaatccaccgtgcccaccggtggcgcggtcccagcggatgaggccgtgctcggcgggccggagtacggctcgcgcgggtagcgggcccgtgcgtcagcgggaaggtgccgcggcgcacctcatcggctggctcgcactcgccctgaccgcgtttctgcagccgcccggccaggtcgcggcggacacaaagtttgacctggtggccaaccccgcgggctttctcgcgcgcgccacgcacgtgtggaccgacgagttcccactcggccagatgcagaaccaggcctacggctacctctttccacaggggctgttcttcctgctcgcggacgccttccgcctgcccgactgggtcgcccagcgtctctggtggacactccttctcggcttggccttttccggaatgctggtgctggctcgccgcgcgggcgtgcgaggaaccgccggccccgtcatcgccgcggtgctgtacgcgctcagcccccgcatcttgacgacgctcacggccatctcctcggaggcgtggccagtcgcgctggttccgtggacgcttatcccgctggtgggcaagcgccccaacccgtgggccgcggttatcgcggtggcgttgatgggcgcggtcaacgccgccgccaccatcgccgcgtgcctgcccgcgttcatctacctgctagcccggcgcgccttcgcggacgcgggcaggtttctcgccggcagcgtcgccgtgtccgcgtggtggctcggcccgcttgtgattctcggccgctactctccgccatttacggagttcatcgagtcggccaccgtcaccaccgcgtggctcaacccggtggaaatcctgcgcggtgccacgtcgtggtcgccgttcgtggacaccgaacgcgtcgccggccacctgctcgtcgcagaacccgcgttcgtcatcgccaccgccctcgtcgcggcgctcggccttgcggggcttacccgcgccccgcgcgagttcgtcctcatgttcgcggtggggtttacgctcctcggtgcggcgcgctggggcattccgcttttcgacggccccttatcccccttccgcaacctccacaagttcgacccactcgtccgcctcccgatgtgcctgggggtgggcgtggtggccagcgcggccgccgctggagccaagcggtgctcgcctcagctcgtcggggtggtgctggtcagcgccttagctaccgcccccgcgtggtcgcttcgcctgctgccgcagggcacgtgggaggagatctcgcccgactgggttgcggcgggcgagtacctcgacgggcacgccgccggcacccgcacccttgtcgtgccgccggtgcagttcgctcgccaggagtggggttggacgcgcgacgagccgatccagggcttaaccacttcccgcttcgcgttccgcgacgcggtcccgctggttgcgccggaggccatccggggcctcgacgggcagacggacgtggtggatgctgaggcgctgcgctccatcggcgtgggcgcggtagtggtacgccgcgacctcgccgaccagcagcccacgcccccgctgggcgtgccggataagagcttcggcgacgtggatgtgtttctcatcgatcctgcccgcgacatgatggtcacctccgacacgccgcttctcatcgacggcggcggggaggtgctgccgctgctgtggcgcgagctcggctacttcccggcgcagctggtgtctgcgtctgccggggagagggtggatgtggtgacagacgcgccgtcgttaagcaagcgcaactacggcgccctgcggggccagtccgcccagctcgcggacctttcggaggacgacacggtgtccaaccggcaagcggactacccctccgccggcacgcgcgtcggcgtggcggtcaccggcggcagcgcttccgcctcgtcctcggccgccgacgcaggtgccttcggcggccccgacccggccaagtcgctgacctccgccttcgacgggctggacgacaccgcctggtggcccgcaccgggcgaccgcgcgccgtccatcacgctcgcgcccgagaccccaaccggcaccatcgcgattaccgccaccgacaccacccgcgtcgttgttgaagatggcggctcctcgcgcaccgtcacgctcgtcggcggcgaaccgcgcaccgtcaccgtgccggaagggccaatcacggtccgcctcaccgagcgcgtcggcatcaccggcatcgacgccggcatccgccgcatcgtcgacgtccccggcgtaggcgacgcctacttcttccagcgccacttccccgccaccgaccacatcacgcgccgcttcaccaccgccgccgacgccgagtgggaactgtccgcccccgccgacatcgacggccagccccgcgagggcacggtgttccttcccgccggcacccacgagctgaccacgcgcgcagatacgatcctgctcaccaaccgcccgcttgacctgcccgaatgggctcccttcgacccctcgcacgtcgcacccgcaggcaccgaccgcatcatcaccaccacccgcggctacaacccaggcttgcgcgcgcgggtcggctccaccgagttggagcccacgcttatcgacgccgccgcccaatcattccgcctcccctcccacgtccacggcgagttccacatgtggcacactgccgagcgcgcttaccgcgcggccctcttcttcggcggcgcgttctccctgctcgccaccgccgcgtgcttgtgggtgccgtggcgccgcttcgaaccgcgccggcctgaggtcagccggggctctcccgccgccgcggccgccgctgttgcagtgaacccgctcgccggcatccccgccctcgccatcgcctttgctgtgcgccgctacacgctcatccccgcgtcgtggcttgccggcggcgcgatgaccgcggccgggttgtggctggcccgcgccccgtggcccgccgccaattacgccggcgacagctacctcctcgcctttgccggttgcctcgccgtcgccgcgctgctgccggcaggtaccggcaaacggtaatagcgggtaactcgcggctgcccgagatgcgacctgggcaaacgccgaaaccgtctggagttacccgctatcaccggcccagcggcgggtgatgacgcgggcggcggggacctcgacgagctcgtaggagatgtaggcgacggctgtgctgaccaccgcggtgaacagccataccggcacaaaatggccgctgaacaggggcacaccgaggacggggaaggcgaagtaaaggactgcgacgtgccagaggaagacggagtaggaccagcggccgagcgcgaccacgggcggccaggacaacacggtgccgcgggtgcgggggccacgggcatcgcgtccaagcgcgaacgggaccagcagcagcgcagcgaaggcggtgcccaagatgacgcgcgcgttgaactcggcgggcgtcgggtgggtgaggccggcgggaccgatctggcccgcgaaccaggccacggcgagcgcggcgaggggaaacggccagcggggaccgcggtagctcacaccctcgcgctcgagttcggcgcagatgaggccgacggcgaaccacgggatgtaggacgggggccagatttgcaggttgaccgcttcgtggatgtcggcgtcgagggaaccgatgaggtgggggtaggtgagggcggcgggcgtcaataagcacaatgccccccaacgccccttcttcccgagcgacatgtagaccggaagaaccaggtaaaacgcgacttcgacgcacagcgaccacatttgggtgagtccgtcgataagcccgtgcgggacgtagatttggatgagcaggaggttggccagcgcctgcgcgggggtcaccgcagtcagcgggggcagggcgaggagaacgacaacaacgcaggtgaggtacgccggggcgaggcgggcgacgcggcggcggaagtaaccgccgcgtcgccactcgccgcgcgccagcaggaacgcggagagcgcgaagaagacggcgacaaagtagtcgagtcgctccgccaagccggaggtgacgccggtttggaacgcaacgtgcgtggtcaggatgccaaaggcggcgacggcgcgcaggccgtcgagctcgggcagtacgttattgtttcggatgtggccattgtaaagactcggcttgacccagtagtggtgtacggtgccgcgctggttatcgccgtgacgtggccatttttcgtcccgggcgaggcgttcgcgctgcgcgacatggtggtgttcgaccagatggcgctgacccgggcgtcgctgggctacggggatcttcccgcccgcaacgtcccgcaggacgcgctcttgggcattctgccgcacccggtgctcgcgttgcgcgtcatcatggtggccgccgccgtcgccgcggcaacgagcgcgtaccggctggggcgcacgcgactgggccaggcagcagcgatgaccgtgatcctgtggaacccgttcgtggtcgaaaggctgctgcaggggcactggtccgtggtggccgcggcgtggctgctgccggcggttgcaatggctgcgcctccggtagcgacgctttcgcactggttggcgtcgctcacccccaccggcgcggtcgccgcggcgctgttcgcgcgcgggaagcggggcgcgctggtcaccgcgatgacgtgcgcgccgtgggtagttgctggggcggttggcgctgcggggggtgctgccgagtcaacgggtagcgccgcctcggcggcggcgttcgcgccgcgggcggagaccttcgccggcacgctgggggcgcttatgggcctgggagggatctggaacgcggaggcggtgccggcgtcgcggcatgccgggttcgccgtgttcggcgtggtgctgctgccggtgctggcggccgggtggcgggcggtgccgcggcgctggctggccgccgcggcgctcggtttcgccgtcccgctcgcgtcgtgggcgggacttctgacgccgctcatagagcacgttccgggagggggcttgcttcgcgacgcccacaagttcctcatcctcaccctccccgcgctgaccgcagccgccggcgcgctcaacgcaaaactcgcgggcgcggcgcttgcgctcgcgatcctgcaggtccccgacgcgccgcttgcgctcgcccagctgtcacccaccgcggtcacggtgccgccggtggaccatcgcgggcgcgacgtcttcatccccgggcacgcgacgctggaggttgtcggcggccgcccggtcgtctcccccgctccgaaagcgatgaacgtggttgaacaaggggcgctcgtggtcgacggcgttgtggtggacgagccctcgccgcggtgggtggcggcgcagcgcgcgtacgaggcaggtgacctgggtgcgttgcgggagctcggggtggggctggtgcttgccgacgccgcgcccatcgacaccggcgcccccgccagagggtggccttggctgggggtttgggccttttgtgtgtggtgcgcggtgccggtggtggggtgcgtcgacaagcaatgtgctcgacgtcacactttcaaactataatccattgacctgctgttttatgaacattagttggcggtaacccattaatggcgcccgccaacgataggaacccttgcattattatcgccagctccctaaggtgaactccagatgaactaaaggttacgaaaggaggccccgatgccaccaaggcagacaacaactgaaacttcggccccaacctttgacaccgacacgaacaccgctacggaaggacaaacgacaatgcgcacctacaccgacatcaacaacatcgacttctccatcatccgcgaaaaggctctgaacaacatccgcgaggacctgatcaacgactgggccggccgcttcaacgcagccgacatcaacgcagcgttcaacgctgtcgtcgaggcgcaccgcgccaacgccgtgatcgaggacttcctcccggtgctggttgaaaacgagatgaagaaccggctgctggaaggcgaccttgccgtcgcagccgcgtaagccggagcacgtttcaggccgaccccttcaccggggccggcctgtttgctattgtcggggcgaacattgtcggtagcgggcaagccgccgacgtcgcgtcagcgaacaccagccccctccgcccggggttcgaaagggcggaattgcatggcgccccgtggccgtatcggggctaaaggcggttcgagtccgtcgttcgcacacactgcggcctgcacaacgcacacgtgcaccgccttcaccaaggccgcaccgcgcacaatttaccaccacggtgttggggcgaggcgaaggtttcgggctgcccgcgagggttgggtacggggacataaacgttggaggtagaaccatgctgcttgcagaagctctcgcgcgccgcgccgaggccgacgaacgcctgcgcgcgctcacgcagcgcctcacccagggcgcgctgatccaagagggcgacaccccggccgaggacccggccgagctgctcgccgaaaccgcgcaccttctcaccgagatcgagacgctggtgcggcgcatcaaccacaccaactcgcagacgccgtttgagggggccacgcttacggacgccctcgcccgccgcgacgccaccctccgagcgcggcgactctactcccaggtggcggacgccgcagctgcccgccaagaccgctactcgcgctccgaggtgcgcttcgtccccaccgtcgacgtagcgcagctgcgcaagatggcggacgacgcagcgaaggcctaccgggagctggacaccaagatccagcaggcgaactggtccacgcagctgctctagctcggctccgggcccgccggccacatgttcaccagcaaatggttactaccaaaaggtcattaaccgccgacgccgattttcggctcgacccagttactcggttaatgaccatctgccggcaacactttgccagtgaccatctgcagcacccgctcaaaccgccgcccggtctcctcccacgagaagcggctagcccactcccgcgcggcgccagcgtagtcctcccccgcaacctcggacaccacctgaggaaacgactcgccctcacgcaccagccggccagtaaccccgtcgaggacggattcggtgacgccgccggcgtcggcaaacgcgaccgtcggcacgccgtgctgcgccgcctcgatcaccgcaataccccacccttccttccgcgagggcaacaggtgcaccgccgcgcggctcagtagcgcgtgtttatgcgcctccgacacatgcccgtggaagacgaccttgtcgggtccgagccccttcgccgcggcgtattcgcgcaggttgtcctcccaccacccggagccgacaacgtccagcaccgcgccgtcgattgcggccgccgcgtcgatcgcgagctcgatccgcttgtgcggcaccagccgcgacagcgttaccaggcgcgtctggcgaccgtccggcagcgccggcaccccctccggcacggggtccacaccgttttccacgatgtcgaccggctcccgcacgcccaacgagagcaggtcgcttttcgacgcccccgacaccgtcacatacctcgacccgcggtagacccgcggcgcaacctgggattcaaggaaccaaccgagccggccgatcaccgggcccgccaccggccactgctccttgtggcagtggtgtgtgagcagcacaaccggccggcgggtgaacagccgcgcgaagaacgggatcccgttttgggtgtccacgacgacgtcggggcggttgcgccagatggatagcggcgcgagcacgtacacgccgtacttgccgccggcgcgctcgtagcgcacgccgttccgggtcgaacgtcgcggcgcgccggtgtgctttgccgtccggtagaccacctcgtgaccgcgggatgcgagatactccccgacgcgctcgaggtagatctccgagccgccgccctgcgggtgggtcgaatcgcgccagcacatcagcagtatcttcatcggtatgtaccgtacccgccgcatgagcacgctgaagcgctcagtgcgcctgctgcgcctgttccgctacgagcagttccggccgcgcatcttctacaccgcgctcgcgcgggacacgtacgcgttggtcgacgcgctcgcccgcgatctcacgggcgaggcggtaactggcaaggcggtgctggacgtcggcggtgggcccgggtacttcgccgaggcgttcgcggacacgttctacgtcggcctcgagccggatgtctccgagatgtcggcggccggcatcaccggctacggcgcggtgcgcggcgacgcgaaggcgctgcccttcgctaacggcgccttcgacgtggtgtactcctccaacgtcgccgagcacatccccaactggcaggagatggtcggcgagatgcggcgggtgaccaagcccggcgggatcaccgtggtcagctacacggtgtggctcggccctttcggcgggcacgagacgggcctgtggcagcactacgttggcggggcgttcgcccgcaggcggtacgcgcgcgttcacggccgcgagccgaagaacaaatggggcgagtccctctttgccgtctctgcgaaagagggactcgccctaaacccggacgccgcgtttccccgctaccacccgcggtgggcctggtggctcacccgggtgccggttgtcagagagttcgcggtgtccaacctggtgctggtctggcgcggctagttgcccgcgttcgactccagccactcgcgtgtggccttgttcgcggccttcacgcggttgcccagcttctccagctcgtcgaaaagctccttcggcacgcgggaaccgagctcctcgaagtactcgtaggcgtcctcgacgtcgttcttccacaggtccgggcctgcgtagagcgcctcctgcacgtcctcgaacgggatgtccaagccggtcaggtcgaggtcctcagcacgcgcggtggagccgaccaccgtctcgttggcgccgacttcgccctcaatacgctggacgatccacttcagcacgcgcgagttgtcgccgaagcccggccacaggaagcggccgtcgtcgccgcggcggaaccagttgaccaggaacacctttggcatgcggtcgccgccgcgctcgcccatgtcgatccagtgctgcaagtagtcgcccacgttgtagccgatgaacggcagcatcgccatcgggtcgtgacgcaggctgcccacggtagcttcgacggacgcagcggtctggccggacgagagcatcgcgccgatcagcgtgccgtggttccagtcgtgcgcctcggtgaccagcggaacggtgtccgggcggcgaccgccgaagaggatcgcgtcgatcttgacgccctccgggttgttgaactccggagacgccgacgggcactgctcaatcggcacgcagtagcgggagttcgggtgcgcggccttgcgctcgtcgtccggcgtccagtcgttgccgcgccagtcaatgaggtggctaggagcgtcgccgtccatgccctcccaccacacgtcgccgtcatcagtcagcgcaacgttggtgaacagcgtgttacccggctccatggagcgcatcgccatcgggttggacgcgtagttggtgccaggcgccacgccgaagaagccattctccgggttcacggcgtagaggccgtcctccttcagcttcagccacgcgatgtcgtcgccgacgacctctgcggtccagccttccagtgtcggggtgatcatggcgaggttggtcttgccgcaagctgacgggaacgcgcccgtgacgtggtaaacgcggccttccgggctggtcagcttcagaatgagcatgtgctcggccatccagccctcttccttcgccatcaccgaggcgatgcgcagggcgtagcacttcttggccaagatggcgttgccgccgtagccggagccgaaggaccagatctccttggtctccgggaagtgggagatgtacttcgtgtcgttgcacggccacgccacatcctcctggccctcggcgagcgggtagcccacggagtgcaggcagggcacgaagttgtcgcccgtgatcttctccagcgccgcggtacccatgcgcgtcatgatgcgcatggacatcaccacgtacgccgagtccgtcagctgcacgcccagcttcgggtccgggtcggtgatcgggcccatgcagaacggcacgacgtacatggtgcgcccgcgcatggatccgtcgaagtgctcgcgcatctcagtcttcagcgcctccgggcgcatccagttgttggtcgggccggcgtcggcttccttgacggtggagatgaacgtgcgcgattccacgcgcgccacgtcagacgggtgggagcgggcgaggaacgagttcgggcgcttctcctcgttgagcttgatcagcgtgcccttctcaaccagctccgcggccaagcggtcccactcctcctgggaaccgtcggcgaagaccacgcggtccgggtcaaagagttcaacagcgtcgttgatccaggtaatcagcgcttcgttgtcggtgggctgcggaccttccagtcgctgcacggcggtagtcatagttactccttgccattagatacgtatcgcgtcctccagcgtacgcaacgggggtggccgcgtcagcgagttcggagcagctgtgactaggcaaacacgctccggcgcgcccccagcggaaaatccacccccacacggggccagcgcgccgcccaatgcccacgggccggcccggcgcccatacccggtttccacccccgcgttctcccggcgcggttagttgcatcatcccacgtcatgtggacaattaatgcgatgcatactactgattcttctgataacaccggcgccgccgagcgcgaaggtgtcggcgagctcccccacggccgcccgatgcagaccgagttcgacaccgggcttgattacccgcgcttgggttcggtcacgttccgccgcggcacgctgacggacaaccaggaggcgctgttcgagaagcactggccgcggttgggcatgatgcttaacgacgcccacgtggacgtcgcctcctggttcggccgctcgggccaccccaccatcttggagatcggctccggcaccggcacatcgacagccgcaatggctccgctggagcaggacaccaacatcatcgccgtggagctgtacaaacccggcctggccaagcttttgggctcggtggtgcgcggcgacatcgacaacatccgcatgatccgcggcgacggcgtcgaagtgctcgcgcgcatgttcggcgaagagtcgctcgacggggtgcgcatctttttccccgatccgtggccgaaggcccgccaccacaagcgccgcatcattcagtccggcaccttgaacctcatcgccacgcgtttgaagcccggcggcgtgctccacgtcgccaccgaccacgccgactacgccgagtggatcgacgagctggtcaacgtcgagcccgcgctggagtacaaggggtggccgtggactgaggcgccgcttctgaccgaccgccaagtcatcaccaagttcgagggcaagggcctggacaaggaccacgtcatccgcgagtacctctgggtaaagaagtaaggggcgagaaaccgcaatggatctgcacgagatgacccacccgtacacaccgggcgccgccccgggcccggccagctacctcttggtgtgggacgcgccgaacctggacatgggcctcggcgccattcttggcggccgccccagcaaggaccaccgcccccgcttcgacgctgtcggccgctggctgatcggccaagctaccgagctttccgccgagacgcacgagcgcatagagcccgaggcgacggtattcaccaacgtctccgcctcctccgccgacgccgtgcggccctgggtggaggcgctgcgcaacgtcggtttcgcggtgtttgccaagccgaagaccgacgaggactccgatgtggataaggacatgctcgcccacatcgagcgccgccaggccgagggcgtgctgcgcggcgtcgccgtggcgtccgcggacgggcagaacttcctcgagccgatcgaggagctggtcgcccagggcattccggtgacggtgctcggtttccacgagcacgcctcctgggcggtgaactccccgctggtcacgtttgtggacctcgaggacatccccggggtgttccgcgagccgctgccgcgcgtcagcctcgaccacctgcccgagggcggcgcgtggcttcagccgttccgtccgctcgcatccttgctgggcgacacgcactagggaaagggaaacgagacgtgttttaccgctgggggcagtttgcttatgagcgccgccgtgtcatcccaatcctgatcatcctggtcatcatcgcgctgcacgtgctgttcggatccaaactgggcgagcgcctctcccaggagggctgggaagacccccgcgcagcctccaccaccgccgccgcgatcgagcaggagaccttcggccgcgataactccggcgacgtcatcatcatggtcgaagcgccgggcggcgtgaacgacccggccgttttcgaagccgccgacgcgcagatcagggcgctgaaaactgagcacccgggcgaggtggcgagcctgcgcagctacttcgccaaccccaacgaccagcaggtcagcgccgacggtacgaaggcgttcgccgccctcggcttggccggcgacggcgagaagacgctgcaggatttccgcgccattaagcccgccctcgaggccattgagctgccgaacgacgccaccgtctccatcgccggggccaccgccgtcgccgacgcgctggacgccggcatggcgaacgacatcgcccgcgccgagcgcttggggcttgtcttcgtcgctgtcatcctgctcttcgtcttcggcggcgtggtcgccgccgcgatgccgctgatcgtcggcatcctctccatcgtgggctcgctgtcgctgttgtccgtgctcgcgcagtaccagcaggtcaacatcttctcccagtccgtcatcacgcttctgggccttggcctagccatcgactacggcctgttcatggtctctcgcttccgcgaagaactcgaccgaggcgcggacgtgccggaggcggtcgccgccaccaccgccaccgcaggcaagacggtgttcttctccgcgttgatggtgggcgtggcgctctccggcctgctcatgttcccccaggccttcctgaagtcggtggcctacggcgcgataagcgcagtgctgctcgccgcggttatctcggtgacggtgctgccgtcgctgttcggcatgctgggccaccgcatcgacatgtggtcggtgcgccgcacctcgcggcgcggccgcgagctcgaggacaccatctggtaccgcatccccagctgggcgatgaaaaacgccaagaaggtcgccatcggtgtcagcgccctgctgcttctgatcaccgcgccgatggcgggcatcaccttcggcggcatcaacgagacctacctgccccccacccaggaaactcgccaggctcaagacgacttcaacgagacattcccggcgtttcgcaccgacccgatcaagttcgtggtcaccggcgccaacgaggagcagatcggtcagatcgtctacgacacctaccaggttgaagggctcgcccgcccgctcaagcccgtccaccccaccgcaggcgacgtcacagtgctctccgcgccgcttgcggacagaaccggcggccaagcggtcgtcgaccagctgcgcgcgctcgacactccaaacggcgtgaccacctacgttggcggcaccccggccatggaggtcgaatccatcgaagcgctgctcgagcgcctgccgtggatggcgctctacatggtgctcgccacgttcctgctcatggcgctggtgttcggctcgatcatcctgccggccaaggcggtgatcatgaacgtgctcggcatcggcgcgaccctgggcttcctcaccctggtcttcgttcacggcgcgggttccgggctgctcaacttcaccccgggcccgttgatgagtccggtgctggtgctcatcatcgccatcctctacggcctgtccacggactacgaggtgttcctggtttcgcgcatggtggaggcgcgtcaaaagggcgccagcaccgacagggcgattaaggacggcaccgcccgcaccggcggcatcatcaccgcggcggccgccatcatgatcgtcgtcgccgcagcctttgcgatgagcgacatcgtgatgatgaagtacatcgcctacggcatgatcttctcgctcgcgctcgacgcaaccgttatccgcctgctgttggtgccggccgtgatgcacctgcttcgtgaggacaactggtgggcaccggcctttatcaagcgcgccgcagccggtctggaaggtgcgcagcgagctcccgaaatcgagcgcccggcgggcgaggtggccatcgacgatgtggtggttgacacccagccgtaccgcagcggcgtgagcgtggacgacgacaagaacctcgtccccttcgaggatctggtcaggcgcctggagcagcgtgaccggtagacgcgcgtgggtgcgctggctcgcgccggtcgtcctcatcgcgctcgcgctgctggtcttccgcgaccagctgccctttctcgccgaggcccgagcccagatcgcgcacgcgcaggtggggccgctgctcgcttcggtggtgaccgcgctgcttgccatcgtcgcgatgagcggcgtcatgcagatcctcctcaacgtcgagcggacaatcgccaaccccgccaacacaaacgcgatcgtcttggcatccaacgcgtggtccaccacggtcccaggtgggcccgccctgtcggcgtggttgaccttccgcgtgcaccgctcgtggggtgcctcagtaggtctctgcgggtggttcttcgtggtcagcggcgcgctgtccacggtgtggatggcgctgatcggcgttggcgcagtggtcatgctgggcgcggagctgtccatctggtcgctcggcggcaccgtcgttgctggagccgtcacgatgtgggtggtgttctgggcgacgcgcaacccggaggcgatcaaacggtggttccgcttccttcccaccggtgcgcgcgcccgcgtcggcgacgtcatcgaccaggtcggcgcgctgcacatttccggacccgcgtttatcggcgccgccgtgctcagtttgtgcaaccagctgtttgacgtcgcgaccatgaccttcgccgtctgggcggcgaccggcgccgccccggacaaccccgtcggtatttttctggcctacatcatgaccaagctcgcgggagccgcgcagattacgccgggtggggtgggcaccgtggagccggtagcagttggcatgctcgtcgcgtctgggatgccacttgctagcgccaccgcggcaaccgtcctgtaccgcgccgtgtccttcctgttcgtcagcgcgatcggctgggtgatctacgccgcggtgtacgcgggccgcgggtatttagtaggaattcgccaagcagatgctgagagaaaggactacgctgcggggcatgaacgtaccaccgatgattggacgcagcgttgactgggagccgattgcgtgtgtgggctgggaggggcatcagcggggcgtcgacaagctaaaagcttcttttcctgagaccggaagggtccggctgaagaagaacacctccaacctgttccgcaagcgcgaaagcggcggcgcggggctggacgtcagcgggctcggcggtgtgattgcggtggatccggtggcgaaaacggctgacgtgcagggcatgtgcacctacgaggatcttgtcgacgcgacgttgcccttcggccttgcgcccctggtggtgccgcagctgaagacgatcacactcggcggcgccgtaagcggcatgggggtcgaatcgacgtcgttccgcaacgggctgccgcacgaatctgttatcgagatggacgtgctggttggcaccggcgagatcgtcacctgctcgcgcagcgagaacgtggagctcttccgcgcgttcccgaactcgtacggttcgctcggctacgcggtgcgcctgaccatcgagctggaggccgtgcccgaattcatcgagctcaaccacgcgcggttttcggatttgggcgagtacgaggaagccttggcccgcgctgccgccagcggcgagtgggagggccgcgagatctacgggctcgacggcgtggcgtttggcaaagacgagcagtacctggcgctggcgtttcgcgctgaatcggtggctggggtgtccgactacacgcggcagcagatctactaccgctcgatccagcacccgcgcgggataaagcacgactacctgacgattcgggactacatctggcgctgggacaccgactggttctggtgctcgcgcgcactcggcgcgcagcagcccaccgcgcgcaagctgtggccgcgcgagctgcgccgcagctccttctactggaagctggttgggctggataaaaagtacgacctggagtaccgcttcttgaagaagccgaaggggctggcccgcaccgagcgcgtggtccaagacatcgaggtcaccgacgaccggctcgcagagttcctcgactggttcttcgacgcaagttcgattcagccggtgtggctgtgccccatccggctccgcagcggtgtcgaggagctggccggggtgggtatcgacgcggccgagccgtggccgctctaccccttgaagccaggcacgacgtgggtcaacgcgggattctggtcgggagtacccgccgaccacgtctcgcccgcgcaagaactcggcgcgtttaacaaggtcatcgaggcgaaggtttccgagctcggcgggcacaagtccctgtactcggaggcgttctactcgcgcgagcagttcgccgcgctgtacggcggcgacctacctgagcagatgaagcgcacctacgacccggacggcaggttcccgggcctctacgaaaaggcggtggagaatgcttgattttgaaccgatgacggtggccgacatcgtcgacacactctttccctccaacaacccgtttaggtgggtcgccttcgacggctcggaaaccgggcccgaggacgcggagcacaccgttcgcgtgaccagcccagaggggctgtcctacattgtgaccgcacccggcgacgtggggcttgcccgcgcgtgggtgaccgggggtcttgcggtcgagggcgagcacctggcgtacccgtacggcgtcttcgacaacctgcgcacgctctacgactcgtttgagcggccggacgcgggggcgtcgatacgcatcatgcgctccctgcgctcgatgggtgcgatccagatccagccaatccccgaggcggagcaggcgagctggctcgagcggcgcgtgcgccaaggcctgtccatccactccaaacagcgcgacgccgaagtcatttcgtcgcactacgacgtgggcaacgacttctacgagctgttcctcggcgattcaatggcctacacctgcgcctactaccccaccccggacgcgagcctcgacgaggcgcaagagaacaagttccggctcgtgtttgagaaactgcgcttaaagcccggcgacaggcacctcgacgtgggctgcggctggggatcgatggtgcgctacgccgcgcgccaaggcgtgcactcgctcggcgtcaccctgtccaaggagcaggccgagtgggcgcaacaacagatcgaggaagaaggtctcgaagagttcgccgaggtacgccacctggactaccgcgacgtttccgagaccgatttcgatgccatctcctccatcggtctgctcgagcacatcggcgtggacaactacgccagctacttccagttcctctcggacaagctgcgcccgggcggtgtcatggtcaaccactgcatcacgtacccggacaaccacaagacagacaaaggcgcgtttatgaaccgctacatcttccccgatggggagctgaccggttccggcacgattatcaggaagatgcaggacaacgggttcgaggtgttccacgaggagaacatccgcctcgactacgcgcgcacgcttcgcgactggtgcctcaacctcaaagacaactgggacgaagcggtggcgcttgccggtgagaacaccgccaagctgtgggggatgtacatggccgggtcgcagtggggcttcgagcacgacgtggttgagctgcaccaggtgctgggcatcaaactggatagcgacggctcgcgcgcggggacaccggagcgccggtggtggaacgactcggtgttctagctgcggggttggtgggctagttgggatgggctgcggcgattatgcgcggcggaattatgccccaccaaccacacccgccacatggtaactaccaaaaggtcattaaccgccgtcggccgaaacagacggggcccggctactcggttaatgaccatctgcaagcaacactctgcaagcaacactctgccggtgaccatttactgagatcacgggcggcagacttatgcgcggcggaattatgccccaccaaccacaccggccacatggtaactaccaaaaggtcattaaccgccgtcggccgaaacagacggggctcggctactcggttaatgaccatctgcaagcaacactttgccggtgaccatttattgggcggcgggcctagagtgggtggcatgaagcgaacgatttcgaagccgtcggcgatcgccgcggactacgtggcccttgctgtcttcgcgctgctggcgcgggcggcgcaccgcagcgacgacatgccgttcacgttcaccgggtggttgtctaccctgtggccgttcgcgctgggcgcgacgctcggctggttgatcgtgcgcgagaacaagggcggcgccatctgggccgtcacagtgatcacgggcttggtgatctgggggatccgcaaccaggcggtgccgcactggtcgttcgtgattgtcgctaccgttatgagcgccctgctcatgctcggttggcgcttggtcgcccggaaggtttagaaggatgagccccaagcgtagagcgggtcgccggaagcgaggccgttagcgaaccaaacgatggcgttgatcaggtcgccgagaagatcgagagtgctggaaagcatgggatacctttcgagttggcttccccggaggtgccggggacggatcggtagttaagaatagcctggaaaagccgcaatctacagcggggagatcgtgtgcttcttaggcagatcgaaatcttgcttggtgcggagttggcgaagcgcccgccttaaagcaaggcgcgtctcggagggctgaatcatggagtcgatgtagccgcgctcggcggcaacgtacggcgaggtcatgttctcgtcgtagaaatccatgaacatcttcttcatcgcctcgcgctgggcagggtcctcgatggcgttgagctgcttgccctggagggtaaccgcggcggcggccgcgcccatcaccgcgatctgcgcggtgggccaggcgaggtttaaatcgccgctcaagttcttcgaacccatcaccgcgtaggcgccgccgtaggccttgcgcacgatcagcgcgaccttcggcaccgtcgcctccacgccggcgaaggcgaacttcgcgccgcggtggatgaggccctggcgctcctggtccacacctggcatgtagcccggggtgtccacgacgtagacgatcgggatgttgtacgcgtcgcaggtgcggatgaagcgcgcgcctttgtcggcggcgtcggcgtcgatgcagcccgcgaggtacatggggttgtttgccacgaaaccgacgggttggccgtcgatgcggccgaaggcgcagatgaggttttcggcgtatccggattggatttcgacgagggcgtcgtcgtcgccaagctgcaccaaaagctccatcatgtcgtagccggcgttggtgtcgtccggcaggaacgtgtcgagcgcggtgtcgtcgagctcgtcgtcctccggcgcccacgcggtgggcagcgggtcgaaggtggaggtaggcaggtggtcgagcaggtcgcgcacgaagtcgaaggcctcgtcctcgctggcgacgacagcggagatgttgcccgcctgctcctgcacgcgcgccccgcccaactcggcggaggtgatgtcttcgccggtgacctcgcggataacgttcgggccggtgacgtacatttcggactggccgtcgaccgccacgatgaagtcggtggtcaccggggcgtagacggcgccgccggcggacttgcccagcatgatggagatctgcgggcagcggccgctcaacggcagctggcgcctggcgatctcggagtacatggccagcgacgtcaccgcgtcctggatgcgggcgccgccggaatcctggataccgatcacggggcagccgatcttgatggcgaactccatgacctcgaccaccttgcggccgaaggtgacgccgacggacccgccgtagacggtcttgtcgtgggcgtagatggccacggggcggccgtcgatgcggccgtagccggtgatcacgccgtcggagtacaccgcgttctcgtcgcccggagtgcgggcgagtgcgccgatctcgacaaaagagtcctcgtcgagcagcgcggcgatgcgctggcgcggggtggtcaaaccggcgtcgtcgcgcttcttgcgcgaacgctcggaacccgggtcctgcgctttctcgaggcgctcgcgcagatccgcgagcttgtcagcggtagtcatttacacgcccatccattcgttcatgtgcttgccaacgatgcccaccgccggttcatcaacgacagcgagatggtcgcccggcaggtgcacgatggtcaaatcatccacgatcttcgcccagccgccgtcctcgtcgatgtgggcgtagttcggctccagcgtgatcgcgccgtcgtgcatcttctcggagcggaagagcagcaccggcacgtccacatccgcccagcgggtgaagtcgaggcggttgaggatctggttgtccacaaacgatgcgcgctggtgctcgagcacaccggcggcgagcccgtgctccgaggcgtcggtctccgcgaggaagtcgcgcagcatgtccatcagcgcctcctccccggcgctctccagcagctcgtaggggacctcgaagtccaggccgtaggtgtccttcgcaaacgcggcgtagcgctcccagcgcgcccgggtttcctccggggtgttcgggataggttcggacggctgcgtggtgtccaaaagcgcaatgaacttgatccggtcgttgccgagctggtgggccacctcgtaggcgagcgcgccaccgaaggaccagccggcgaggatcacttgccgctcccccgcgatctgctcgatgtccttcacgtacgccgccgcgcgctcctgaagcgagccctcgaggcgctccacgccgtagaccggcaccgattcatccaggcgccgggccagcggcgcgtagaccgccgaggacccgccggccgggtggaacacgaacacgggctcgcgggtgtcggcgccgtcgcggaagacgcggatgttgccctctacctcggtctccagcccctcgcgcaccatgttcgccagcggctccagggtggcagcaccccgcacgtcgtcggcggtgatctcgatgccggaacggttggtcaggtgctcagcaatctgcttggcgacgccctctgaaacctccggcagctcactcgtcacaccagccggcgctgcgccggagtatttcgcccaggcgccgaagaccatgcgctccgaggcgtcgcgcggggcgacgccgacgcccttcgcccttgtcacctcggcggccgggtcgcgggtctcggcgttctcggccatcttaagcggggcgtcggtgttgccggcgacggcttcctcgacgatggcgatgacgtcggcgacggaggcgtcgcgaagcgtctgcacctgcagcggcgggatctggaagtcgttctcaatgcggttcttaatgcgcatgcccatcagcgagtcgagacccagatcgatcagcggcagctcgtcggggaggtcttccgcctcgaagcccatggattcggaaacgattgagcgcaggcgctcggccacggtttcggttgcgggatcccagcggacggtgtccacggtgtcgtcgataagcgagggctccacctcagcaacccctgcgatctgcggtgcttcgggggccgcgagcgccgaggcgaagccttctgcaatgagcgtgtcgccgtcgaagacgcggacgctggcgccgccgagggagcgggtgacgatcgtggtcacctcgccgtcggcgggcaggtagccgtgctcctcggtggcgacgacctgcgcctcggggagaacctccccggcggcggcctcgatgagctggtacgggctgtagacggcgtccgccggggtggcgaaagcggtctggccgtccggcagcgaaacgcgggcgccgagcaccgagcttgtcgacgcgttcggccgcgcgctcgtccacaagtggttgcgctggaacgtcacacccggcgcggccacccgcggttcggcgccgtagaaaccggtgaagtcgaccttcacgcctgcgacgtagagcttcgtcgcgaggtcgagcaacgtctccgcctcgtcgagcttgcgtttggtggtgaacaacagctgcgcgtccggcctgccggaggcgaacgccgtgttcatcatgcccatcagcgcgaccgggttcggggtgacctccacaagcgtggtgtggccggcgttgaacgcggcgcgggtggcgtcctcgaagtagaccggctggcgggtcatgcgcaggaagtactggtcgtcgtgcaccaccgcgcccgcggggtagacctcgccgcggtcgacggaggtaaacagcgggatcttcagcggcgagggcgcaatgccggcgatctcggccgcgaggtccgccatgatcggatccagcatggaggtgtggccggcgccgcgaacgttgagcttgcgggcgaacttctcctgtccctccagctcggcgacgatgtagtcgacagccttacccggcccgccgacagtggtcatgccgggcccggcgtacacggccggctcaacaccttccgcctccgggtgggcggcgacgaactcggccaagtcctcggcgccgagctcgaccacggccatcgccccctcgccgtcagtaccggcgatcattgcttcgccctcgcccatcaggcgcgcgcgatggcaggcgatgagcatcgcgtcgcgatctgtgatgccaccagctgcgtaggcggcggcgatctcgcccatggacatacccatggtggcggcggggaccatgcccatcgacgccatcaggtcggtctgcgcaatctggatcgcggtgatggtgacctgcccggtctgggtgtcgtaagtctgctcgtcgtccaggatgatgtccaccatggaccagccgccctcgaaggcgaccatctcgtccagctcgcgcatgcgggcggcgaagaactcgctggtttccatcagccgcttcgccatcttgcggtgctgcgagccgaaaccggagtagacgaaaaccggccccatcgggttcggcgcgtcggccgcaacaatgccggggccgatcttgccgtcggcgacggcgcgcaggcgcgagaccgcctcctcggtcgtcgcggcctgcaccaccgcggcggaacggccgtggttgcgcttcgccagggagcgcgccaccgggatcagatccgcgtcggggcggttttcaaggaagtcagccagggttgcggcttcagcttttcttctcgacggcagcaaccccgacaccggcagcgccgccacatcaagcgccgcaaacccggtctgcgcagcctcggaagccgcgtcgtactcgccggcgtcgaaatcagtcagcacaacgtgcgcgttcgtgccgccgaagccgaagccggatacaccggcgacgcggcggccggagtagcgcggccactcgcgcgggtcggcgacaacctcaatgtgctccgcgtcgaagtccacgaagtggttgggggcggagaagttcgcgctcgcggggatcgtgtcgtgcttcagcgcctcgagcaccttgatcagcgcgacggcgccggcagccgactcggaatggccgatgttggacttcgccgagcctaaaagcagcgggttcgcgttcgtgcggtcgcggccgagcaccgtgcccagcgcggtggcctcgatcgggtcacccaagatggtgccggtgccgtgggcttcgaccaggtcgacctcggccgggtcgatgcccgcatccgcgtaggcgcgctcgagcacgtcaacctgcgcctgcgggttgggggcggtcagaccgttggagtggccgtcggagttggtggcggatcccttgatcacggcgaggatctcgtcgccgtcagcgatcgcgtcgcccacgcgcttcagcacaagcatgccggcagcctcggagcggacgatgccgtcggcgtcgtcggaaaaggcgcggatcgcgcccgtgggcgagatcacgcccagctcggagaacataagcgacgcgaacgggttggccagcacgttcacgccgccggcgagcgcgatgtcgcactcgcggtcgcgcagcgcgcgcaccgcgtggtgcaccgacaccagcgacgacgagcacgcggtgtccacgttcatggacggcccgcggaagtcgaaggtgtaggagatgcggttcggaatgatcgagctcgacgaaccggtcagggcgtacgggtgcgcctgcgccgggtcggcgcccatgagcatgccgtagtcgttcgagctggagccgacgaagacaccgaccgcctcgccgcgcaagctgtcggccggaatgtgggcgttctccagcgcctcccacgccacctcgagcatgatgcgctgctgcgggtccatgtgctgcgcttccagcggggacaggccgaagaactcgttgtcgaagctggcgatgtcgtccaagtagccgccgtcggtggattcctcggcgatcttggtcttcaggtacgggtcgcccaggtactcggaccagcgtccggggggcaggggtgaggtggtcacgcggccgtcgataagcagtgcccaaaactcgtcggtgttgcgggcccccgggaacttgcctgcggaacccacgacggcgatgtcgcgctcggcgggcgagcttgcagcgacgacgcgctcgcggcgcacccgagtctcggccgcggtcagcgcgtgcgccagcgcggcgatcgtggggtgctggtacgcgatggtcgggtccaccttgcggcccagcaggcgctcgagctcgcccgagagcaccaccgcgtcgcgggacgaaagaccgtacgattcgagcgacgcggccgggttgaccgcctccgcccccgtgtgggaggccacccattgctcgagccagctgatcagttcgttttctgtcataacaaaagaccttatcgcccgcaggcttctattcgttatccctttcgcgcggggtgcgcgcgtttaagcgccgcggttgcggtagttgttggcgttcacgcggcgggcaattttgcctgacgacgtccgcgcgatcccgttcggctcgtagaactcaatgacctccggggagatgccgtggttgttggtcaccgccgcgcggatggcgtcctcggcggccttgtcgtcggccgggtccttctcttctgcccgctcaacgaggatgatgagctgctccacgtcctcgcccggcaccgcgaacgccgccaccgagtcgcggcgcacgtggtcggaggcctccatgacggtggcctcgatgtcctgcgggtagtggttgcggcccgcgaccaccacaaggtctttcacgcggccggtgatgtagaggtggccgccgaccagcgttccgaggtcgcccgtgttcaaccagccgtcggccggcaggttctcctggcgggtggcgccgatggtgttgcggaaggtggcgttggtctcctcctcgcggccgaggtaaccggcggcctggttcgggccgcgcagccagatctcgccgatcacgccctcctcgacctcgtccttggtctccgtgtccacgatggcaaagtgcatccacggcaccggctggccgttggaggcgaacgaaacgccatcctcggcctccaccgcgcggccctgtgcgagcgcttcgcggtcgaaagtggcgaacttcggccgctgatcggtctgcggggtggacacgatgagcgtcgcctccgccaggccgtaggagggccgcaccgcgcggcggtcgagctgcatcggctcgaacgcttccaagaagctcgacacgctggattcggtgaccggctcggagccgacgatcagcgcgcttacgtgcgagaagtcgtagtcgccggcggcgtagcgcgccgccagctcgagcgagaagttcggcgccacggtaaagatgtgcatgtcgtccgggtcctcgccgcggcgcgagaggcgctccagccagcgcgtgggctgctgcacgaagtcgcgcggggcgaagacctcgaactcgttgcccaggatgacagccaagatcgccagcaccatgcccatgtcgtggtgcagcggcagccaggagacgatgcgcagcggctgctccgcgcccacgcccttgtacatctgcagcacgttggccacgatcgagcggttggtcagctcaacgccggccgggttgcgggtggaaccggaggtgtactgcaaaaacgctatctggtcggcggtgtcggcggtcggcgggagcggctcccacgcgcccgcgagcgaatccggcagcgagtccaccgcgaggatgcgggggcgctcggtggccggcagctcagcaaagtacgcccgcaccgccggcgcgccctggcggttagtgagcacgatcttcgcgcccgcgtcttccagcacggcgcgcaggtggtgctcgtggcccggctcgttcgggtcgtagagcgggatcggcacttggcccgcgtagagcgcgcccatgaacgcgtagatgtactcgggcgaattaccggccaagatggccacgcggtcgcccgggttgcccacctgcatcaggcgcgccgcgacagccttcatgcgggtgttaacgtcgcggcgcgaaagcgggacgttgacgccgtcggtgtcggacgagtagtcccagaaacggatgttcacgtcctcggccaagccctgggcttcagcgccggtaaacatcagctccgccagcgccgggatggtgaacccttccggaagcgcgatgttgccgtcctcatccaagaagcgctggatgatcatcttcagatccatagggggcttcctttcgcttaactggtgctttctactggtgctgcagaacagcgtcgatggttgtcgccgcccaatctagcgtccaattcgtcgcggtagtgccgggaatcacgtcggggttggaggcgtagagggcgtggtttccgtttgctaacaaaagatcggccgcgcggtcgatggcgttacccaccgcgtacggggcgtcgcacaccgagtcgttcggcgcgcagatttcaaaagcgcggtcagccacctcgccgaactttccgggtcgcgcgccggtcatggtcgcgcctggggttgccaggtccaccacgcgctgcagcggctgcatggtgatctcggcgccttggcctgtgacctccacgcccgggttcacgcccacgccgttctcgcggcgtccgtccgcaatcatcaccgcaccgagcaggcgctccggctcgatcgcgcctgcgcgcgtgccgatcgcgtccgccgcgtcgcccacgatcaccgcgccctgggagaagccggcgatgatgaactgcgtggagcggcagtgctcggcgacaaacttcagctcgccgttgagctttgccaggccctcggcgcgagattcgtcgtacggcatctcctcgcgcccgcgctgggtctggatgttgcggaactgcgcggtgtacgggacggtgaacacgcggacatcgtcaatgctgtagcgctcctgcagcgggcgcgtgactgagagcatgaggctcgccgggttggcctgcgggttgaacgggtcgtcgtcgggcgccgattcccacgtgcccggcactgagacgacctcgacggcggggcaccactccggctcggcggggcgctcaggcgtctgctcgctggtagcgggcgcggtggcctcctccccgagcggcggcagcggatccccgtccgagcccgcgcgccactggtagatgcccagcccaatcaacgccaggatgacgatgacggcggcgacgatgaagacgttgcgcgatcggcgcatgcaggtgctccttcccgtgcgcggcttaggagcacaggttgtcgcgggcggcggcggtgatcagctcgccgagcgcctccggcgtcatgtcggtgcgccgctgctccacaagctgacccgccaccgcgtcgcgggtgatcatgtcattcgcgcacacattaaggcccgttgctgtgagttgatcctcaacaccctcgatgttgagtccattgttgctgagctgatccagaaacgcgcgctcctgcgggctaaagtcgctggtgacggccggaacttcctcgacgtctcgcgccggctggtcctccggcccgcctgcccgtgcgggtgcttgggcggaggagcttttgcttgtcgacgtctctgtcaccgtcgccgtacccccactcgaggtggtcggcgcagtcgtcgcaggggtcgtcgcgtcggaggcgtcgacggtggcggagccgccgccgcacgccgcgagcgtcagggccgtgccgacgacagctgcggcggggaggatgcgggctctactcatcgcttcctctcaatcaccacgccgttaatctggtccagccggcccttctggaagtcgatggtcaagccgccggccgggatctgcttcatgtccgaagtcggccagcccagcgagccctgctcgtagccgcgcttgccccactcgttgaagatgtcgccgtagtagatcacgtgggcgccggttgccggcgaccagtagatgttgcccttctcgaactcctggaagaagccgccgcggatggcgatctcgttgcccttcgggaagcccagattactggtcgcaccgcccatctggccgtacttctcgccgatggcgccgtagaccatgaagttcttgccgtccgggttgcgcgtgaggtagccgccctggaacttctgcacgtaaccctcgccgaccttggtggcctcggccgccgggtacttcagcgttccggtttcgtaacccttagcgccccacgccttgaacatgtcgcccgggatcgcgtacgcgccggtgttcggtgtccagtagatggagccgttctggaagtgcacgaagcggccgaccccgtccggcgtcttcgtctcgccggtggttgggaaaccgagccagccggccgggccctgcagcgcgttgtacttcgccaggatggcgccgtagatcgcgtgcgccccggtctccggcgaccagtaggcggtgccgccgcgaaagtcctgcgcgcggcccttgccgttctcaccggccgcgtactcctcgttgacgcactcgccgatgatgccggacttggtggcctcggcgatcgcgccgatcggtgcgcacttcgcgccccggtcgccctccggcacgttcagcgcgttggcgatgtacggccacgcctgcgccatctcgaactgccagtattcccaggagtgcacgccggacgggcggaagcgcacgatcggcttcacgttggtgcgggatgcgtagtccacgaacgtttgggtagacaggcgcgaaatcacttccaggcccttgccggccgggttcgcggcgccgcgggcgacggagtccgggctgccgaagtcgtcgcggccggagcccgcagagacgtacaccgtcatgccttcgaggttctcaatacccagcttcgggtcgtggtcaacccacgcctgggagccggccgggccccacatggcttcagagttgtacccgccagcgtcgagctgcgccgccttgatcgcggtcggcatgccggacgtggtggtgtctaggtagccggagaaggagccgacgaagttgaacagatgcgggttgcgctcagccaggttgaccgcggcggtgccgcccatggaaatacccgtgacggcgcgcttgccgttggagcggaagttgttgttcaaaaccggcacgagctccttggtcaaaaacgtctcccacttgtagttcttgccgttgttgggctgctgccagtcggcgtagaaggaggattcgccgccgaccgggaggatcacgttgacgttcttgtcggcgtagaactgctcgatgttggtctcgatggtccagccgttctcgtcgtcgcgggcgcgcaggccgtcgagcgcccacacctcagggaacttcgcacccgggttggagtgccagtcgcgcgcgagcaggatctggacctggatgagctgctccggcatggcctgggatttaataaacaccgcgacgcggcgctgggtgagccactcgatacggtcgacggaaacaccctccggcaggttcgggatctgcgggtggcggtccacctcgatcggtgtgcgcggcagcgggtcggagggtcggatcgcgtcggagagcccgttggaagaaccgaacgtgctggaaagatccgaggactgcgcggctgcctgctgcgccggcgcgacgacggacgcgagtgtggcggcggccacggcgacctgaaggaaacgggggcgggaaacgcgcattagggatcagcctcttctatcgatgacggggtcaacggcggtcaagtactcaaatgttaagtttcacttgagactttacccgcgcgacacgccggtgacagatgaggttattgatccccgtgtgaacctctaccaggcgttcatgacgttcagcacgcgcggcctcgtcgcctcgagctggctgccgaactggtcccagttgtgcaggcccgtcggcgtgaacacggcggtgtgctgcacgccggtggccgtcgccttcgccgaccacaggcgggtggtgaagttcgccacggtctccagtgcgatgccggcggcgcggtgctccgggaggtacttcgcgtcagccggtcccggcgtgccggaaccagcggaaacgtacacgtccttgccgcgcaggttacccatgttcaggaacgggtcgttctcgtagcggcgcgggttaaaaatagagccccacatcgcgttgaggttgtacaaaccgccgtcaagcagcgcgatgcgcaggcccgtctgggcgcccgggatagtggtggtcaggtagccggagtacgacagcacctggcggaactggtcggggtgcagcgccgcgaggttcaccgcggcggtgccgcccatagacaggccgaggatagagttgttcgtcggcgagacaccgaagtggtgctgcaggtacggcggcagctccttggttaagaaggtgtcccacttgtaggtgaccgggttgttgaaatcgtaggtcgccggcgcgttccagtcggtgtagaaggaggattcgccgccgaccggcatcacgagcgtgatgttgtcgttgacgtaggtgcgcgccgcgttgacgtcgacgagccacgcgttactggtctcctgcgcgcgcaggccgtcaagcaggtacaggcccgcgttgccgccgtttttcgccggctggatctggaccgtgacgtggcggttcatcgccggggaccacacggtgcagcgctgcacccagtagccgatcccgtcccactcgcatgcgccggtggagtctgggcgcagccagtcgcggtttgccgcagacgcctgcggggcggcggcgaagctgccgacaaacgccagcagagtagtcagcattgccacgaggccgcgacgagcgcgcgaggaaaaagcgtgcatagtgaaaagccctctcaagaacagcaaagttatcaatcagttatcaaaccacggacggtggggcgattcaatcggtcagctagtcgcggggccaagcaatttgcttgccgacgggctttaatcccacgtcagcgccgtttcggatctggcgcttcgtctgcgcatccaggtagccagacgggtcctcattcagctccaaggtccgccccgggccgagcgagaagcgcacatttttccagaaacgctcccagctcatcggctcccgggaggtggccaacagctccccaatctcttcggtgcgcagcgccgcccgcgcctgcttcgcctcctccgcgtcgaaccagtccggcagcgcgtttaagtcaacagcagagtcggcaacctgccactcagctttcaactgcttgtcgtggccgacgcggccgtcagggtcgcgcggcatgcgcgccgccagcgggtcggcgagccccaccgtgtccaagatgcgcgcgtccagcgggctgttcatgctggtcattcccaggttgatccagtacgcggtgggagccaggtactgcaaatccgagttctggtactcctcgcgcgggcgcgagtaccacttatacagcagcggttccccggagatgtaggcgatagcgatctccccgtcgttgtcgcgcagcgccttttccatggtggtgtcgaaggtgcgcatcaacggcgacgacatgaagtcctccgcatacttcggcggatccccctgcttgcgccccaccgccatggtccagaaatcccgctcgtcgacgatcccaagctcaccgtcttcgttcagaaagcggtctgggtcgtcgctgggctgctgcacaagcacgaagaatgcccacaccgcgaccgcggcgcctaacacccctaccaggcggttgtacggcacggccatgacgggcatgagcagcgcgaacaggggcaggagcagcatgcgcccgtgcatgaagtcgccgccgacgcgcagcacgtagagggtgtgcgcaagcgcgcaaccgacgatgatcaggcccacggtgcggcgcctcccctcagcgcggcgcactacggcgacaagcgggaggagtgcgatgacaagcgggatccacagcaggtacgggtcgttgaagtcgcgcaagtaggcccacccgcttgcccactcagcatcggaagcggacttcgccaccgcggtgtgcggggtgagcaggccgtagtaccccatgcgaaagagctggtaggccgccggcaacggtagcgccgcagccaaaatacccggcgtcttgcgcggggtaaacgcgatcagcgcgatgccggtcaccccgccgtagagcgcgaactcggggcgcaccagccacgacagaccacaccagaacgcgagcaggtagcccgcggaaggcttggcccggcgcgccggcgaggcccagtccacgagcagtgcgaaccacaccgccagccagaacagcgccagcccccactccaggccggaggtggcgaagtcgcgcgccggtggcagcgcgaagtagatgaggatgccgaacgggatgacgggcgctgcctttttcagcacaccctgccagtacacactggacgcgtaggtggcgatcgcggcggccagcacggtgcaggtcaaggcgagggtggtggcgacgtcttcaagcctgccccccgtcacccaggcgaacgcggtgatcatgtactgccacagcgtcgacgtgttggcctcgatgcgctccccgatgttgaacacgggaccgttgccggcgagcaggttgcgcaccgtgcgcaggacgatcaggccgtcgtcgctgatccagcggcgcgaccacccgccccagaacgcgataacgcccgctagaactgtcgcggtggcggcagagatgcgggcgtgttgttgcattcgtcagaccttacccagtgaaagccggaacgatgtacaccgccatgccgatgcacaccaaccacgcgacagcgagcagctgcagcacacggtcctccagcgcgatctcgtccggcgcgccgccgcgcccaccgtcgacctccgcggcgtagcgcaggatcgcgatcacgaacggaaccatggagatctgataccagatcgcggcggggccctcggtggcgtcggaaagctcgaagccccacagcgcgtagaagatcaccacggcggttgccgacagggtccacacaaagcgcaggtacgtcgcggtgtaaccctcgagcgccttgcggatcttcgcgccggtttctttcgccaggatcagctcggcgtagcgcttgccggaggccatgaacagcgagccgaacgcggcaaccaggaggaaccactgcgacagcgcgatgccggcggccacgccgcccgccatcgtgcgcagcatgaagcccgaggacaccagcgcgatatccaccaccgggatgtgcttccagccgaagcagtagcccagctgcagcccaatgtagatggcgatgaccgtggccaacgccgccccgtccgtggcgaggaacgacaatcccagcgccagcgcgatcaggaccagcgccatcgcgtacgccaggttgatcggcagcatgccggaggcgatcgggcggaagcgcttggtgggatgctcgcggtcagactcgacatcgcgggcgtcgttaatcaggtagatcgaggacgcgccgaagcagaacacgatgaacgcgagggcgatgtccagcaccgtgcgggcggtaaacgcgtcgaggccggcggcgagcggcgccgcgagaacaaggacgtttttcacccactgcttcgggcgcaggcctttcaccatcgcgtcgggcaggttcttcggcggggtctttgtcaccaacacgtcgaccccggcggtgtgcggctcgggccggatcaggggctctttgtataccgcgtcgttcgcgtcgctcatcgggttcgcctttccgcttcgagcgcggccttgcccacggcggcgccgagcgctgcgccggcaagcgtgtcggtgggatagtgcacgccaagcacgttgcgcgaggccatcatgaccggcaccagcgcccacggccactttttccccgcgatctcgctgagcaccaccgcggccgcgccggtgttggtggcgtgcgaggagggaaacgacagctgcgacggtgttttcacgccgattgcaatgcgctcatccgtcgggcgcgggcggcgcacgatgcgcttgagcaccaccgacgccgcgtgggcagcaaaggtgccggcgcccagcgccacccacaggcggcggcgctttgtgtcagcagctgcgccggcggcggcaaccgccatccagcccaagtcgtgctcgccgaagtggctcaaggtgcgcgccgctttgagcgcggcgggcgagccgaccgcgtcctgcagggcgaccaggaggtcggcttctctactgctcattaaagatcttcccccagttctcctggctggtcagctcgccgcgcgcgtcgcggtaggagcgcttcagctccggccagcggcgcttgatctccgcttggaggtccttggtttcttgcagcaggtcgctcgcaagctgcttgtccctcttgcggaacgccacgcccgtgccgccggcggtggacactgtggccgaatcaacgcgggcgagtgtgaaccagcgggcctcatccgcggtcaggttcagctgcggcgcttcccagtgggtgcggtcctcggccttacgctggtgcagcagtgccttcgcggcccaggggagtttcttgatcttggccaggcggccaccgatgttgcgggtgggcacgcccggcgcgccggtgggtgcgggcagctcggtggcgctgggcagcacctgcgcgtcggcgtactgcttccgaatctcctggatgcgcggcagcgaggattcgaggatgtcgaagagctggtccgggccggcgaggaagtccttcatggcctcgacctggatcgccatggtggagtactccatgcacatgatgtgcttgtgggtggacttcatcatgttcttcagcatcgcgtccgggttgtcgggcccgtagatcgcggcgacaatcagacggttgcgcatgtggaagtacgcctgccagtcaatcgcgtcgtccttgtccgcccaggccatgtgccagatcgcaacccccggccaggtcacggtggggaaccccgcctccttggcgcgcagggcgtactcgttgtcgtcccacttgataaacagcggcaggggcaaccccatgcgctcagcgacgacgcgcgggaagaggttcatccaccagccgttgtaatccacgtcgacgcggcggtgcagtgcacgcgaggtggtcttgcgcgggtccatctgctcctcgggcgtgcccacgtaccccagcgggtacttggcaaagtcgtggtcgtacacggcgtgctcggcagcgcggaacatgaagatgtcggggtcaacggcctcaccggtggtgcgcagctggctgcggtcttgcaggttcagcatctgcccgccgaccaaaatcggctgcttggcgtagcgcgccgcctgcaccgcgcgcacgatcgagtccggctcgatggcaatgtcgtcgtccatgtagagaatgaacggcgcatcagtcgagttcagcgcttcgtacatgatgcgggagtagccgccggagccaccgaggttgccctggctgaagatccgcagtttgccgccgagtgcggcttcggctgcagcaaagtccggttcgtcggccgggtgctggttgccttggtccggcatgagcacatggcttatcgacgccaccacaaacccatcctccgccaacgcgtgcaacgcgttgactgcatcccgcgggcggttaaacgtcgggatgcccacggcaacttctttgggttggggtgggataacggtgccgtcggcaagcacctgctccttcggctcctgcgcggcgcaccacgcggcgtttgagatgcgcgtgtcctcttccgcggtgacgtcgaaccagagccagccgccgtcttcgaagttggcgagcttcagctcgatctctgtgcggccggtcgcctcgacgttggtcacggcgatgcgcgtgccgtcgtgcttggagcggtagaccgagatcgtggcgcggccctcgacgtccatggcgaggaccacgctgtccagctgcgaccagcggcgccagtagctcgccgggaacgcgttgaagtaggtctcgaagctgacctcgttgcccgccggcacctcgaagctggtgcggtcggaccagcgcagccgctgcttgttctgctcctgctcgatgaggtacagcatgcgcacgtcgtgcggctcgccctttttcggcataagcacgcgcgcgagggtgtccaccgcgagggtcttcgttgtctccacagctctcactttctgttgtgggcagtcggaatccaagcgtaatcgctctgcaggtgtttccttggtgtggctcgcggctcagcgggggttagccggcgaagaggaggcgcaggccctcacggaggtcggccaggatgcggtcgacctccgcttcgggaacccgcaggttgtccagagtgagaccgttgatcagcgcggtaactaggcgcgccttgggctttgcatcctcgtcagcgccgagcgcagcgacaacgctgctctgaaagtcttcgaggacctcggtatagagcttcgcaatccagtcccgggtcgcagaggcggagccgtacgtgacccagattgcggcgtcttcggaacgcacccctccgatcgggagaagctccgcaagcctcgccacccaggtttcgagctcgtctcccctttcaggaactgccgctacccgttcgctctgacgctggatggagcggataaacgcgtgcgcaagcaaggtgtccttgttcggagcatgatattgcaccgaaccggcggcgaacccggattccttcgccacctcccgcacgctcaccgcatcgaggccgcgcgacgcaatgatgcggatagtggcgtcggcaattgccgcggccgattctgaaaactgatggtccagggaaaagtcattcatggttgcaccccagtctagattctcgtacgttcgtaagtcgtagtacgttcgtacgagagatccggagatccccatgagttcggtcatccccgttgttggcttggcgctgctcgacagcctgagcctgggcacccttgttatccctctcgcgctcatcgtccactggcgcgccgttaaagtgccggcacttaccgcgtatttgatcaccgtcgcggcggtctacttcctcctcgggctggggatactcctcgggttcgcaggactgggctcggtcgccgaacgggtcacgcagaccgatgtcttcccctggatcacgttgatactgggcgcggcccttgcgatcttcggcatcttcgcccccaaccccaagaagcccgaacccgggcagctgccgaaacgcgcagccggagccacaagcagtctgccaagtatggtcgccttaggcctcggcgcatcacttaccgaggcggcgacgatgctgccgtacatcgcagcgatgggcatcatcggcagctgggaaatcccctccgcggcaaaggctgggtccgtgggcatttactgcctcattatgatcatgccaaccgtcatcctcgctaccttcgcgctgctcttcggccaaaaggttttcccgcggctcgagcgcctcatcccccgcctcgagtacgagacaaaaagtgacgcttctctggatcgccgccatcgtcggcatctacatggtggcgaacagcgtggcgacgatccgcggcgacctccccgcctcgtaatgaggactgttttcgcgcggcggctgcattggcgctcgcctccccggagccgttacggtagctacggtttccacccctcacctcctcgaggggaaatcatctaacgcattgaaaacggtatacatatggctacccctcacactgagaccactcgcgaaccgctcgccccgacgggcgttgtggaatccttccgctacgcattttcgtccccggcgcggcttcgtcgtgaagtactcgccgggctcaccgtcgcactggcacttatccccgaggccattgcgttttcgatcctcgccggggtcgacccggccctcggcctgttcgcctccgtgatcatggccatcgccatcgcgttcaccggcggtcgccccgctatgatcactgccgccactggagccgtcgcgctcgttattgccccggtcgcccgggaatacggtcttgactatttcatcgccacggtcatcctcgccggcgtgtttcagatcgtgctcggagccctcggcgtggccaaactgcagcgcttcatcccgcgctcggtgatgatcggctttgtcaatgcgcttggcatcctcatcttctccgcgcagcttgagcacctgatcaacgttccatggccggtctacccgctcgtcgcagccggcatcgcgatcattatcttctggccgaaaatcaccggcgcgatcccagcaccgctgatcacgatcatcttgcttaccggcgtcgtcgtcgctggaggcatcagcgtgccgacggtctccgacatgggggaactgccgacatcgctgcccggcctcttcatccccgacgtgccgctgacgctggaaaccctgcgcatcattggcccgtacgcgctcggcatggcagtcgtgggcctcatggagtcgctcatgaccgcaaagcttgtcgacgacatcaccgactcccactccaacaaaacccgcgaatcctggggccaaggggtggccaacatcgcctccggcctgttcggcggcatgggcggatgcgcgatgatcgggcaaaccatgatcaacgtgaaggagtccggcgcccgcacccgcctgtcgaccctgctcgccggcgtgtttctgctcgtgttgatcctgctcctcggcgacatcgtcggcatcatcccgatggccgcgctcgtggcgatcatgatcatggtttccgtgggcaccatagattggcactccgtccacccgcggaccctgaaactcatgccggcatccgagaccattgtcatgttggtcacggtcgtcgccacgcttgcaacgagcaacctcgctgtcggcgtggtcctcggtgtcctcacggcgatgatcgcatttgcccgccgagttgcgcacatcactcacgttgagcgtatcgaggggcccggccccgctaccaacacctaccgcatccacggccaactgttctgggcgtccagcaacgacttggtctacgccttcgactacgccgatagcgccgaccacatcatcattgacctttccaccgccgagatctgggatgcttcgacggtggcgacgctggatgccatcacccacaaattcgaggaacggggcaagacggtcaccattagcggattgcacgggccgagcaaggatagagtcgaccgtcttacgggccagctctcgtaggttctggctgctagtagatctgggttggcgttttaaaagccctctgcttggcgttttgaaaacggattgcttggcgtttgggaaattggctgaaggcggagagtgaaggaacacatcgacaccgtcgaaaatggcgtgaaagatgtccgtcgtcgcctcggcggacttgtccacgcaccgtcactcgctgatctctcccaggtcgatcgaacttttctcgtcgcaatgtcccaagatgatgggccatcacgcatcggggatgtggctgagcgcctcggtgtggacgcccagtacgccggtaagtaccggcgccgcctcatcgacgcggaaatgatccagccggcaggctacgggttcatcgacttcgagcttccctacatgcgcgagtacttacgttcccaccccgcatcggacacaatggagcaattttcgatgtggcccgaggaagaatcctagggacctaaacagcaacctcgaacggcgcctcggtggcctcgcgaacggtgtcgaccgtctcacccggcgcgacctctacaagcgtgaggccttgcttctcatccaccgtgaacacggcgaggttggtgatgatgaggtcgacacacttggcgccggtgagcgggaggcggcactcggacagcaccttggagtcgccgtgcttgttcacgtgctccatgagcaggatgaccttcttcgcgccgtgaaccaagtccatcgcgccgcccatgcccttgaccatcttgccggggatcatccagttggccaggtcgccgaactgggagacttccatcgcgccgaggacggcgacgtcgatcgcacgggagcggatcatgccgaagctggtggaggaggagaagaacgaaccgcccggggcgaccgtgatggtctccttgccggcgttgatcagctcggggtcgaccgcgtcgtctttcgggtaggggccgacacccaggatgccgttctcggagtggaggaccacctcaatatcgtccgggaggaagcccgggatgagcgtcggcatgccgatacccaggttgacgtactggccgttctccagctcctgtgcggcgcgcgccgccatttcttcgcgtgtccaagccattactcgctcaccgtcctgaattcgataccggtctcctgcgggccaacttccaccacgcggtcgacgtaaatgccgggcaggtccacctcgtgcgccgggatctcgtccacgacttcctcggcttggacgatggtgaccttgccgcacaccgcggcgtccgggttgaagttctgcgcagtcttggaaaagaccaggttgccgaagcggtccgcgcggtgcgcgtgcacgaacgcgaagtccggcgtcagcgcggtttccatcacgtactgctcgccgtcgaactcgcgcagctctttcggcttggagtactccgcgatcgtgccgtccgggttgtagcgggtggggatctcgccggtggccagcggggtgcctacgccggccttggtgtagaacgccgggatgcccgcgccgccggcgcgcatgcgctcggccagggtgccctgcggggtgaactccacggtcagctcgccctcgaggtactggcgcgcgtactccttgttcgtgcccaggtaggagccgatggagcgggagatgcgcttgtcttgaaggagcagacccagaccgaaaccgtcggtgcccaagttgttcgaaatgatcgtgaggtcgccggcaccttgggcgcgcagcgcttcgatgagccgggccgggatgccgacaaggccgaatccgccgacggcgatggatgcaccgtcgtggatatcggcgacagcctcatccgccgttgaaaccaccttgttaatcatgtgtgcatggtaactgccgttcggatattgcacaagggttcacaaagcgaacattgatgagctaggctcacacgcatgggagaaagtgacgtgcaactcgttcagagtttaagccggggactcgcggttatccgcgcgttcgacgctgagcgcccacgtcaaacgttggcgcaggtggcggacgccaccgggctggcccgcgccactacccgcaggttcctccacacattggttgcggagggcttcgcgcttaccgacggcacgttgttctggctcacccccaaaaccctcgaactgggctactcgtacctgtccagcctggggctgccggcgatcgcgcaaccccacctcgtgcggctgtcgagcgaactcaacgaatcgtgctcggtgtgcgtcctggacgaaggcgacgtggtctacgtcgcgcgcgccgccaccaacagcatcatgagcgtgaacatcaccatcggcacccgcttccccgcctacgccacggcgatgggccgcgtgatgctcgccggcttgagcgaagtggagctggacgcgtacctcgcagcggcaacgttgcacccgcgaacgccgctgacgatcacggacgcatccaagctgcgcgaggtggtggacaccgtccgcgagcagggctacagcgtggtcgaccaggagctcgagatggggctccgctcgattgcgtgccccatctacaacgccgccggagaagtgaccgcggcggtgaacgtgcccgcgcacgcggcgaggtaccagcccgcccaggtggtggggcggctcttaccgccgctgcgagacaccgccgccgcgatcacccgcgacgtcgtgacaaccgatatgacaacgaaggagacattgtgactactgcaaaccccgccgacatcgtcatctgcaacccgaagcgcaccgcggtgggccgctacggcggcgccttcgtcggtgtaccggtgcaggaactcgccgcaaccgtggtcaaggcggtgattgaggaggccggcatttccggagatgcgatcgacgacgtcattttgggccaggcctccccgaacggcgccgcccccgctttgggccgcgtggtcgcacttgacgcggagatcggcctcaacgtgccgggcatgcagctcgaccgccgctgcggttccggcctgcaggccgttgccacagcggcggcgcacgtcgcctcgggcgcggcggacctgatcatcgccggcggcgccgagtccatgtccaacacggagtacaccgtggacggcaagatccgctggggcgcgaagggcggcacgatggagttcgtcgaccgcctccaggagggccgcgagaaggccggcggcaagcaccacccgatcccgggcggcatgattgaaacagccgagaacttgcgcgaggagtactcggtttcccgcgagcggcaggacaagctggccgcggagtcgcaccgccgcgcggccgccgcgcaggaggccggcgacttcgacgcggaaatcgtgccggtgagtgtcccgcagcgcaagggcgacccggtcgtcgtggacaaggacgagcacatccgtcccggcaccacggaggagtccctggccaagctgaagccggtgatgggcaagaagctcgacggcgccaccgtcaccgccggcaacgcgtccggccagaacgacggcgccgccgcaatgatcgtgaccacccgcgcaaaggccgaagagctgggcctgactccggcagttgtgctgcgcggctggtcggtggccggcgtgccgccggagaccatgggcatcggccccgtcgcggctaccgaaaagctcttcggccgcctgggcctgacgttcgacgacattgacctcatcgaactcaacgaggcgttcgccgctcaggcgctggcggtgctggacgcgtggggcatctccgaggacgatccgcgtgtcaacccggtcggctccggcatctcgctcggccaccctgtcggcgccaccggcgcgcgcatgctggtcaccgcggctcaccgcatggagcgcaccggcgcccagcgcgcgctggtgaccatgtgcatcggcggtggccagggtctggccgccgtgatcgagaaggcgtagcgggcataatcgggcgcatggacactcccggcaagaactacgccctcggcgccgtactcatcgtggtgtgcgccgcctcgttcgcgttcctctccggctccaccgcggtgttcgtgggcatcgccggagcgatcggcggcgccgtgctgatccttcgcggcatacagctcgcggacgcacagtcagacccgagcttgcaggacccgatgttgcaggatccgctcaacttcgacgacggctacgactgggacgccgagttccgccgcaacaccgagggcggccgctaactgccgtcgctcatccgcatcatcttgctggggtttgctaacgcactgcgctggctcgccatgatgaggttgtctaggtcggcgagcaccgcgtcgacgtcggcagggttgtaacgccgttcccggcgcgccttctgcagctcgtggctggcagccttgaacgccacttgctgcatctcgagtgcaccctcgcgggcgcgcaggaacgcttccttgcgctccttcgacccctcgggatccatcacgcggcgctccgcgacggagtcgagccagtcctgcacgatcgtgtacgcctccggcgcgaactcgtcgttgtgctcctggatcgccttgcgcgccgcggcgtaggcgcgctcgttgagctcgccgtacgccttgtccgcgtccgcgtccgggccgtgctcgaagtccatcttgctcaccaaccacggcagcagcatgcccgggatcaccatggtgcaggtcagcaccgtcagcgcaataacagacagctcgtggtggtattgggttgccgacgcgggcatcgacaggaccagcgccaaggtgaccagtcctcgcatgccggaccacgccatgaggagtacttcctgcatgcgcagcggggacacattggtcctcccctttcgctgattcgccttgcacagcacccacatccacgcgaagcgaaccaagaacgcaaccagggagagcaccacgccgatcaggatggcctgcgtgatgttcgtgcccgcggtgtcgatcgcgtcgcgcacgctcatgccgatcagcccgaacgcgacgcccgtgaagagcagctccacggtctcccagaagaagtggccggtgaggcggtcctccgccgtcatcgcggaacgcgacgacatctccaccgcggcgatcacgatcgcaatcacgccggatgcgtggatagcttcggcgccggcgtagatcgcgaacggtaagacccaggtaaacgcggtgcggatcaccgaatccggcaccgagttcgcgaatttcgccgccaagcgccccacgatcaggccgattaccacggccgccaccgcggcgtacaggaaggacaagaacccgcggccgaaattcacctcgtcgtgggcgacggcagctgcaagcgcgacgttgaatgcgacgatggacgcggcgtcgttaaacaagccctctgtctgcagcgtgccggtgatgcgcttcggaatgccggcgggacccgccaccgcatccacagcgaccgggtccggcggcgcgatcgccgcggcgagcaccatcgccgccgcaagcccgatacccggcatcatccacatggcggtcgccgtcagagcggcgatggtgaggaaaaccagcaccaccgacatggtgagcacaacgttgagctgtgaggcgatttgcccccagctggtgcgccgcgccaaagaccacaacagcggcggcaggaagatcggcaggatcaggtgcggatcgactgtgatcgtttcaatgcccgggatgaacagcaccggcgccaccacaatggtcagcagcgccggccacggcaggccggtgcgctcaccgatggcggcgacgagaacggtagcgagcagaagaccaacgagcgcaagaaagattgacacgcggccagtgtaatcggcgcggcgttcgctagtgcccgcgcggctggctcagcggctggccggactcgaagtacgggcgcagctggttctcgaagagggtcagcgccgcagcgatcgccatgtgcatgtccaggtactggtaggtgcccaggcggccgccgaaaaggacgcccttttcggactccttggcggcgagctcgcggtaacgccccagcttctcgcggtcctcgggggtgttgatcgggtagtagacctcgtcctcgtcgccggcgaagcgggagtactccttcacaatcaccgttttgtcgtccgggtactcggagcgctccgggtggaagtggcggaactcgtggatacgggtgtacggcacgtcggcgtcgttgtagttcatgaccggggtgccctggaagtcgccggtttccagcacttcctgctcgaagtcgagggtgcgccaacccaggcggcccttcgagtactcgaagtagcggtcgagggggccggtgtagacaatcggcgcgtccgggttctcagcgcgcagctcgtcccggagctcgaagtaatcggtgttgaggcggacgtcgataagcttgtgctccgccatgcgctcgagccacgccgcgtacccgtcgaccggcaggccttcgtgcgtgtcgttgaagtagcggttgttgaaggtgtagcgcactggcaggcgagagatgatttccggcggcaggtcggtggggtcggtttgccactgcttggcggtgtagtgcttcacaaacgcgtcgtacaagggcttgccaatcagggcgatgccgcgctcctccaggttggtggcggcggccgggtcgagtccctcagtctgctcggcgatcagcgcgcgcgcctcgtccggcgagtagtagcggccgaagaactggttaatcaggccgagccccatcgggaactggtacgccgtgccgtcgtgcatggcgaagacgcggtgctggtagtcggtgaaatccgtgaaacggttgacgtactcccacacgcgctcgttggaggtgtggaacaggtgcgcgccgtacttgtgcacctcgatgccggtttccgggtccttctcgctgtaggcgttgccgccgatgtggtcgcgggcctccaccaccagcacccgcttgcccagctcgctcgcggcctgctctgcgatggtgaggccgaaaaagcccgatccgacaacgatgaggtcataagtcatgccacgtattttcgcatagttgcttgtcgacggggcgccccacgacacgctcaccctcaagtcttacttgagacttgatattggtgtagggtgcaacgtgaatcactatcgtcacatcggccacaggagtaatacagtgaaacaacgccgccgactgaatagtgccgccacccgcgtgcacccgatgctcgccgcgatcctgaccgtggctgtggtcgccaccgccgcggtcggcggccagcagatcctgcaggtccaatccgtcgcgccggctagcgtagaggtgtacagcgattccgcctccttcgacggcggcgccaacatcaccgtcaacgacgcagccgtgcgcacccagtccggcgagcaggaggaagtccaccgcgtggtcaaggagttcacgcgcgaccgcgagttctccctcttcgcgctgacctggtccggcgagcgcgacatcgtcgccttcgcccgctcccagcgcgcggacggcacgtggaccccgtggtacgagatggagatcgccgactcccccaacggcatcgccaccttcggcaccgagccgatttacgtggagcgcaccaagagggtgcaagtctccaccggcggcgtcgacctgctcgagggcggccgcaccgcctccgccgcgccgaccaccgcccgcgacctgcaggcagtgtttatcgacggcggcgtaggcaccaccgccggcgacatcaccccggttgccgactcctactcgcgctacatgcccaaggtggtcacccgcgcgcagtggggcgcgaagagcactaagaagccgtactacaccgaaccggtcaccgccgtgacagtgcaccacacggcagggtccaacaactacacggccgccgaggccccggggctggtccgaggcatcgagcactaccacgctgtgacccgcggctggggcgacatcggctacaacgcgctggtggacaagtacggcaacatctacgagggccgcgccggcgggttagaccgcgctgtacagggcgcgcatgtcggcggctttaacaccaacacctggggcgtgtccgtcatgggcgactactccgtcgctcgcccgaccacggaatccattaaggcgctgggcgagctcatcggctggaaggccgcagtttccggcttcgatccgacgggctctagccgccactacgccgacttcacgttcgccggctcgcgctacgcggctggccagggtgccgtgttccccaacgtgaacgcgcaccgcgacttccacttcaacgactgcccgggcgacaacctctacgcccgcatgggcgacatccgccgcgcggcgaaggtgaagtacgacgccacccgcgcctcgcgcgtgattgcaaacccggccctgccgtcgcagccgagcaccaccgagaccgtccgcaaccccgacgggacaaccaccacggtcatccgcaccgacggttccggttcttccaccggcacgaacaccaccgacaccgcgaacctgctccagggtgtggcggacggcgacgcggtcgccatcgccacggtggtcggcaccgtggcaggcgcggcgctcatttgggccctgcagaacggcaagctggacaaccaggtcaagaacgtcgcgggcaccgagctgatcgcggggctcaccgtgcaagacgttgccccggtgcttggcccggttctgagcctggccggcagctccaacaccgccgacgtgtggaagaagttcgaacccgagctgggcaaggtggtcggctccgtgtccggcgtcggcggccagcagatggtcttctacgccaacggcatcggcgtgcgcgactccaagggcgagatcttcaccctcgccggccagatcgccaacgcgtggctgcagcagggcctcgacgccggccctctgggcatgccgaagtcgaaggcgcgcaacgtcaacaccgacgaggtgcgcatggacttcgaaggcggctcggtggtctactcgatctcgaagcgcaagatcgacatcaccaccagctaaatcacgcctggttgtaggcgcgcaacaccgcgtcttcccactgcgcaacgagccgatcccgctcggggtcggccattgtgtttttgaaggtggtggcgctggtgaggttgaagggggcgtcgataagcgaaatgcccatggcagccgctgacgccgcacccatcaccgtcgtttcgatgttggccgggcgcaccacgtcgatgccgaggatgtccgcctgcatttgcataagcaggttgttgctggtcatgccgccgtcgacacgcagctgctccgggtgcgcccccatcgcgcgcaccacctcgagcgtctggaggcaggtcgcttcgagtgcggcgcgggcaatgtgccgcttatcgacgtagcgcgtcaaccccacaatcaccccacgggcatccgggcgccacctgggggcgaacagcccggagaacgccggcacgatggtgaccccgcccgaatccgagacctgggcggccagcgtttcgctctccgcggcggtgtcgatgatgcccagctggtcgcgcagccactgaatcaggctgccgccgacggccacgctgccctcctgagcgtagaccggggcctcgccctcgatctggtaggcgacggtggtgagcatgcccgagtcgctgatcctcggcgtcgcacccgtgttgaccagcatgaacaggccggtgccgtaggtgactttcgcgtcgttctctctcaggcagttctggccgaacagggcggcttgctggtcgccgagcacgcccgtgatcggcacgccgccgagcgggccgcgcgaacggacgtggccgaacgtgccgatcgacggcttaatctccggcagcatcctcctcggcacccgcagctgttcacaaagctcgtcgtcccagtccatggtggcgagatccatcaggagcgtgcggctggcgttggtcacgtcggtcaagtggagcgagtttgcggtgtcgcgcgcaccgccggtgaggttccaaatcagccacgtgtcgatagtcccggcgagcagttcaccgttctcggcccgctcgcgcgcgccttcgacgttgtcgaggatccacgcccacttcggacccgccgggtacgagttgtggagcaggcccgtttgctgcaggtactgcgtttggtcctgctggtcggtggggttcgtgcgcgtgtcctgccagacgatcgcgttgtagatcgggcggcccgtatccttctcccagatcaccgcagtttcgcgctggttagagatgccgagcgccgccacgtcctcgtcggcgatatcctggctggccagcgcctcgaccaccgcgcggcgcgtgttgcgccagatctcgatcgggtcgtgttccacccacccctgccgcggcataaactgcttgtgctcgaactgcgcctccgagacgacgttgccgccagcgtcagtaatgaacactcgagtcgatgtcgtgccctggtcgatcgcggcgatgtacggcatggcaacgagtgtatgtgggcaggtgtgtggaaattttcgggggtgtagctcccagcgaaaaccggccccttttccgccgcgtttccgcaggtgggttgtctagccaaatccttgggagctacagggcaggtgggccgggccaggttgggcccgggttttgggccaggttggggccgggccggctcggggccgccggacgcccgccggcaggcctggggtgaactacacgggtcggccagcaagcacaaggcgctatccacaggcgagctacccaacacgggcctgcaccaggaagctatccacaatccgcggatcgggcttcccccgcggccgaaagtccgagatgatcgggtcatggatggggaatcgagggtggaacggaagcgtcgccaagagctcgagctcatatcggcggtggcgaaagacacgaagaacgcggtgatcaccggaccggccgccgccagagtgttgggggtgagcaacctggggtgggtggagcaagtgcacctcatcatgccgggcaggtcgcaccagtggggaaagaagcggcagtatccggaccgggtgtacgtcagcgccggcatcaccgacgaggattggtacgttaaccaggggtttcgtgtcaccacactggtgcgcgcaatgttcgacacctaccgctactgcgggaggatgcctgcactggtgcagatcgaatccgcgaggaacaagtggaacgcgtatacccaaaagaccctgctcgagcagtcggcctcgctgccccgggctcatggtctccgggggtttcgggagcttatttgcttatcgacgcaccaagcagaaagcccactcgaaacacttgcgcgacaccagatccttcaagcggtggagagaggggagctgagcgaggtgagaacggtcgaggtgcaggtcaacttcgtcgtcaaggacctcgacggcgcgatcgtttacgcgcgggttgacctgttggttaacggctacatcgcaatcgagttggacggccgcgtcaaaaccgacgggacatacggagacccggttgccgtgacgttacaagagcggcaccgggagaaggagctgcaaaaccttgggatcatcgtgctgcgtttcgggtggaaagcagtgatgacaggcgaatttctcaaggtcatcgaggcggtgctgcgaatgtatccgaagccgaagacgcttccgctgagagcggcgtagctagaaccactgctcgaggaccatggcgacgccgtcctcgtcgttggaagcggtgacgtggtcggcaacctccaaaagcaccggcgaggcgttggccatggcgacgccggtgccggcccaggcgagcatctcgacgtcgttgggcatgtcgccgaaggcgatgacgtcggcaggggcaactccgtagcgctcggcgagcgcggcaacgccggcggccttgttcacgccgggggacgagatctcgatcagcccctcatccattgagtacgtcacgtgggcgatacccgggtcgacgacgggggcgatcagcgcgtgcatctgcgccgacgacagctccgcgcttctcaccagcagtttcgcggcgggaacggcgacaagatcggtgatggggacgatgccgaagcgagcgtcccaggcatcggggttgtattccggcgtgatcagaaaaacttcgtgctcggggtcgagggcgctggagccgacgcgctctacgccgtagccgtgaggcacgccgtcgagtacgcggctgacgtcggccgcgatctcggacatcgtggcgggagcgagttcggcggcgtgcagcacggtgtcggaggcggggtcgtagaccaccgcgccgttggcgcagacgcagatcggggatacggtgatttggtcgaggacggggataagccagcggtgggggcgccccgtcgccaagcagaaaaatgcccctccgcctaccgcgcgggcgacgacctcccgaaggcgcggcgtgacgcggccgtccgagtttaagaaggtgccgtcgatgtcagaggcgatgagtttcggggccatggcgtctagcgcttcttctgcgccctcgcctccttctccaggcggtagatctccgcggcctcatcgatcgtcggcgcggtgccgcccatcgatttcggcatccacgcctcgccggtgaacgggccgaaagtggcgtcgtactcccggcgcgactgctcaagcatggcctgcatcgcggacttcagcgcagccgtgtcggcctccgcgtcgccggtgaggtggatcggttcgccgtagcgcacgatcacaggcacgtggtggagcttcttcggcaaatccttcgtccagattcgctgcgagccccaaatcacgcacgggatcagcggcacgtcggcggcgtgggcgatgcgggcggcaccggttttgaagtcggcgagctcgaaggagcgcgagatcgtcgcctcggggaagatgcccaccagattgccgctgcgcagcatggcggcggcggtggagatggaggccgcgcccttggagcggtcgaccggcacgtggttcatgcggcgcagcaccgcgccgaggacggggacctcgaagacggacttcttcgccatgaagcgcacgagacgctcgccgcgcaggtaagggccggtgcccagcaggacgaagtcggcgtagccggtgtggttgccggcgatcatcgcgccgccctcagcggggatgtgctcggcgccgacgacggtcacctcgatcttcagcaggttcagcacgcggcgcgcggttttcaccgtgcgctggtagaagcgctcggcggcttcctcctggttgaccccgatctccctgaacaagcgggggacgcggaaaccgcggtacttccgggtatctacaagcgcagccattagggggtgagcacgtccttgcccacccacgggcgcagcgccttcggcacgacgacagagccgtcggcctgctggtggttctccaaaatcgcgaccagccagcgggtggtggccagcgtgccgttcagggtggcggcggtctgcgtcttgccgtcctcgtcgcggtagcgcgtgttcaggcggcgggcctggaacgtggtgcagttcgacgtggacgtcagctcgcggtaggtgtcctgcgacggcacccacgcctcggtgtcgaacttgcgggcggcggaggaaccgaggtcgccggcggcgacgtcgatgacgcggtacggcacctccacaagacccagcatctcgcgctcgaggccgagcagcttctggtgcatctcctcggcatcctcgggcttgcagtaaacaaacatctcaagtttgtcgaactggtggacgcgcaggatgcccttcgtgtccttgccgtaggagccggcttcgcggcggaagcagctcgaccagccggcgtagagcaggggtccgtcggagaggtcgatgatctcgtcgcggtggtagccggccagcgccacctcggaggtaccgaccaggtacatttcgtcgcgctcgaggtagtagatctcctcgtcgtgctggtccaagaagccggtgccggccatgatttcggggcgcaccagcaccggcgggaccatcaccttgaagccagcttcgcgcgccttttgcgcggcgagcatgagcatgcccagctgcatccaggcgccgtcgccgacgaggtagtagaagcgggcgccgccgaccttggtgccgcgcttcatgtcgataatccccaggctctcgcccaggtcgaggtggtctttcacctcgaaatcgaactcgggcacctcgccgacgtgctcgaggaccacgaagtcctcctcgccgccggcgggcgcgccctcgatcgggttcgggatcgccacctgcaggcgcgcaacctcggcctcggccgcgtcctgcgcagcctccgcgtctttcacccgcgccttgagttcgttcgagccctcgagcagcgccgggcggtcctccggcgctgcttggccgatcttcttgccaaatgctttctgctcgccgcgcagctcatccgccttctggatggcgctgcggcgggtctcgtccgctgccagcagctggtccaccagcgagggatcctccccgcgggcgacctgggagttgcggacgtggtccggattttcgcgcacttgtttgagatcgatcacgccttcatactttagccgctgaacacacaggcgcaggccgaggtctaagctatccgccatggccaccaagtccacagccgcgcgttcgttcgtcatcgccgcgctcgccggcgcggtcgggatcggctccttcgatcttgcgcgccagcaaccggagggtgatcaggtggaggacaacggggcgcaagtaagcaaaagctccttcaccaccgccgacgcgggctcctgcctgacctgggacatcgggccggacggcgcgattaccgggttcgaccagactgattgcgcgggcccgcaccgcttcgaggtggcgctgcgcgaggatctgggcacctaccccacttccgagtttgggccggaggcgccgatgccgagctcgacgcggcaagcgcagctgcgcgaggagctgtgcggcgcggcgacggtgcgctacctcgacggcacgtacgaccccgccgggcgctactccatcgcccccatcctgccgccggcgagcgcgtgggccgagggcgaccgcacgatgctgtgcggcctgcaggagacggacttggagggcgaacccgttttgaccagcggccgcgttgccgaccaggaccaggcgcgcgtgttcgaggcggggcagtgcgtggccatcgacccgtcgaattcgctttcggtggttgactgcggcgaggtccaccagatggagatcacctccacggtcgagctggccagcgtgttcccagaccacacgccgagcgtcgaggagcaggaccaccacctcggcgacgtgtgcaccgcggccgcgcaggactacctcggcggcgaagagaacctctatcaaatcacgctgcagccgttctggaccacgcagaagccggtctcctgggacggcggctcgcgcagcgtcaactgcgcactcgtcttctcgcggccggagggcggcttcgcagacctcaccggttccgcaacgggcggcagggagcagttgcttatcgacgcagcgccccccgcccaaaagccccaacgccgacccttgcgcaccgacgcctccaccgcgcccgccaccgaaccggctgtggaaccgcaatgatgacgccggtgacgcaggaggagttcgaggagatgatcaacgacgccctcgatgccatccccgacgagttcgccgagcacatgaccaacatggtcgtcctcgcccgcgacttcaactacgacgacccgacgcttctgggcctgttcgagggtgtcccgctccccgagcagcactccaaccacaccgggttcctccccgacgccgtcttcgtgtacaaaaacgcgctggaggcgatgtgctcggatgttgacgagctgcgcgaagaggtcaaggtcaccgtactgcacgaggtcggccactacttcggcctccaggagcacgagctgcacgagcttggttggggctagatcgccgttacaaccggctgttccaaatggtcaccgccaaagtgttgcttgcacatggtcatcaaccgagtaaccggcccgagcccaaaacctgcgacggcgactaatgaccttctgctaacaacactttgcaagcaacactttgtgggcggctacggcagcgggtaatccgcccactgcacaacccgccagctgccgaattccctcgccggctcacccggatccaacacaacgtactggcagttggccaggtgggactgctcggcgtactcgggcgtgatcccggtttcgtgggtggcgttggcagcgtaggcgcggatggcgccgccgtgggagacaacgaccgtggtgccacccatctcaacgtacggctggatcgcgccgtggtagcgggtgaggaacgtatctaaggtgtcgccgtcttcgatgaacgcggcgaggtcgcggcggtaaaagccccggaaagcggcgaaataggcggtgtgggcggaacgggagttgtgcatctcccaccgcccggcgttgacctcctgcaggccggcaacagccgggatgtcgccgaacctacccccggactcggggccgaaggcgaggtgggcggtttggcgggctcggagcgcctccgacgagatcacccggtccacgtcgaaattcgcgaggatctcgtggccagcggcgcgcgcctgctcctcacccagctccgtgagctgggctccgggcagcgcggtgtccagcttgcggtcgacgttggaaaacgtctgtccgtgacgaagcaggatcagcatggtgcaccgtcacctaagtccgcaccctcgacgaaccgcggccatgagcccaagaagcgcagttggctggcgcgcgcctcgatcccccgcagcgcctcagcgacgggcgcgtcgtcgcggtggccgacgagctcgacaaagaagtggtacgtgtttgccacctcgcgggtcggccgcgactcgatgcgcgacatgtcaacaccgcgcgcggctagttcttgcagcgccgaggccaacgcgcccggcttgttagcggtctggaaaatgatgaacgtgcggtcgttcccggtcggcccgccgccaaccgccccacgaccggccgctcccccagctggacccacgaggatgaaacgcgtgcgcgccgtcgacaggtctgccacaccgcgggcgtgcacctcgaggtcaaacagctccgcggcgcgctcgggagcggcggcaacatcggcagcgccctcggccaccatgctggcggcggccgcattcgaggtcgcgggcaaaaactgcacgtccccgaggtgctcggcgatccacgacttcacctgttgctgggcaacagggtgggtggaaaacaggcgggcgcgatcaagcgcaaagcctctccgcgtcatgatggcgaacgcgatagccagctcggtctcggcgtagatctccacgcccggggcgacgagagcgtcggcggttgaggtcacggccccatccacggagttttccaccgcgaccaccgcgtagtcaaccttgcccgcgcgtaccgcgtcgagagcctgggcgggcgaatccaccggcacgtactcggggtctggaaggtcgaagcggcgcgcggcctcctcggtgaaggtgccggccggtccgagatacgcgatgcgggtcacggcgctaaagttaccgcatgcgccagcgccttatcaccgaagtgctgcttgtcctcgccgtcaccttcggcgcgtcaggggtgcgcgcagtgctgcggctgatcgaatcgctcattgccgcgccgctgaacgagcagtcgacggtgctggtcaaccagcagtccaccacgacgtggattgatctcgcgctgcagctcacctccgtcggcgtactcatcgcgtggggcgggctggcctggtacctactgaacgagagatggcgctggccgaggtggcgcgacctcggtgccggtgccgggctcgctgccctcatcggcctgccgggactcgcgttctacatcgccgcggtgcacctgggtttcagcaaggttgtcgtgccggccaccgatgcggtgcagatccccacctcgcttctgtgggcgttcgcgaacggcttcggcgaggaggtcgtagtcgtgatgtacctgctcacgcgccttgcgcagctggggtggaaaccgtggcaggcggtggcggcatcagcagggctgcgcggctcctaccacctctaccagggcctctccgcgggcctcggcaacgtggtgatgggcgtcatcttcgcctggttcttccacagaacaggccgcgtgtggccgcttatccttgcgcacttccttatcgacgccatcgcgttcaccgcctacccactcctggacctttcctggctcggcatctaagcccgcgggtttagactgtccgacatgtcaacgacgccgcactccaacgaccccagggacaacctgggcgattacgtgctgggcaaagacggcaagccgctggtggaccgctacggccgcccagtgcaccgccgcacggattaccagccgcgccgcacgccgcacgagcagcgcaatcaggagcagcgcgcccaagagcgcccccgcccgcggcagcagatgccagcgccgcaacccaaaccccaacccaggcctcaaccgcggcccgtgcccaaaccgcagcctcggcccgagccaaggcccgagccccgccagaagtcgcgcaggcagcgcaggcagcgcaaggccccggggtgcttggggtgcttcacggttgttgcggcagtactggtcctcaccctcgtagggcttttgcttgccgacgcccgcctcacccgcacccaagcgctcccgccatcacaggtcgagaacacctccggaaccaactggttgctggtcggctccgattcccgaaccggcctgtcccaagctgagattgatcgcctcggcaccggcggcgatatcggctcgacgcgcaccgacacgatcatgcttttgcatattccgcgaacggggcagcccacgctggtgtccatcccgcgcgattcctacctcgcgattcctggttacggctacgacaaggtcaacgccgccttttcctacggcggggcgccgctactcgtccagaccgttgaacaggcgacggggcttaggatcgaccgctacgccgaggtgggcatgggcgggctcgcaaacgtcgtcgacgccatcggcggcgtagagatctgcgtggcggagccgattgatgacccgctggcgaacctgaacgtccaacccgggtgccagaaaatggacggtgcaacaggcttgggttacgtccgcacccgtgcaacagcgctgggcgatctcgaccgcgtcgcccgccagcgagaattcttgaccgccgtggtgtcgcgaaccctctcccccgcggtgctgctgaaccccttccgattggtcccgctcatgtggacggcgccgacgatgttcacggtcaaccagtccgaccacgtgtggaacctcgcgcgcatcgcgctcgctatgcgctcgggcttggtcacggaaaccatcccgctgggcggtttcgccgacaccgaggtgggcaacgtgatgctgtgggacgaggctggggcgcaggagttgtttaaccggctgcggtagggggcgcggtggtgggccaggtgccgtcggcaagcatctgcttcttccgctccacccagaagtcggcgtttctgataccgagggcttccgggtcgaactgcgggtcaaggcccgccttcttctggcggcggtaatcccacaggcatttgagcgccggggcctggatcaccaggaccgctacgatgttgagccacgcggtggtgcccacgccgatgtcaccgagcgcccacgccgtgcccggggtggacgttgcgccgacgacaactgcggcaatgatcagcgcccgcagcacccaaatcagcgcggtgcgcgcgctctcgcttttcacccagcggttcaggtacgcgaagttcacctcggccatgtagtagtaggccagcaccgtggtgaaggcgaagaacaagatcgccagcgccacgaacgaggagccgaggccgccgctgagcgtgttcaggccctcttgcacgaaacccgggcccacggccacgccgtccggaagcgagccttggtagatcacgccgccgtcctcggactggtcttcgaagaccttgtacatgtcggtcgagatgatgatgaacgcggttgcggagcagacaaacagggtgtcgatatagacggcgaacgcctggacaaaaccctgcttcgccgggtgggacacctcagccgccgccgccgactgcgggccggtgccctggccggcctcgttggagtagatgccgcgcttgacaccccacgcgattgccgcgcccagcatgccgctgaacatcgcctcctggtcgaaggcggagcggaagatgagcccgaacacattcgggatctcggaggcgttcgcgatcatgatcacggccgcgacgacgatgtagatcacggccatgaacggcacgaccatcgatgcgaaggtagcgatgcgcttgacgccgccgatgatgatgaagccgagaagcgccgccatcgccgcagcggtgacccaggtggagatgccccacgcgttgttcaccgcggccgccacgccgttggcctggatgcctggcaggaagtaggaggtggccaggatcatgcagatagcgaagaagatggcgtacgccttggcaacgccgcgggcgccggtgtgggcgtaggccttctcgatgtagaaggccgggccgccgcggtattcgccggtgtcgcggtccttctccttgtagatctgcgccagggtgcattcgacgtacgacgttgccgagccgaggaacgccacgacccacatccaaaagaccgcgccaggaccgccaaaggcgatggcggtggcgacacctgcgatgttgcccacgccgacgcggcccgcaagcgagaccatcagcgattggaacgaggagatccccgcttcagagctctcgccggtggacagctgcttaatcatgtcgggcaggcagcggacctgcaggaacaaggtcacggcggtgaagtacacacccgcgccgagacagagatacaccagccactgggaccaaatgatcccgtcgagggtgttgatgaacgtctccatgttgccctccacaaacccggttttatgcacagatatccaagtgatacaaaagatagaccacgaaccctgtgtcccgggtcacttttacgggggcaaaattctcgcgcgccgctagatcgtcacctggcgcgacttgatgttgtcgagctgcttgcgctcgtcggcgttgagctgcgcgtcggaggcgtactccgccacaattttctcgttcagcgcggtgagcgcctcggcgtacgcggcagccggcgcctcatcggcgatcgggtccacggccgggtccaaatcccacaccggcacaacaaccccgtgggtgcggaacgcgccggcgaacttggtgccctcgcccaggttgagctcgccgcgggccgcgatgcgcgcgagcgcggccagcatcttgtcctcgttgtcctcgccgcgcacccagcggatgtgggccttgccgccgccggggttgacccaccacgccgagcccgggatcgcgtcgccggatgctgccttgatctgggtggacggcatcactgcgtcgttggcgcgggcgagagcctggcgcacctcggcgggaagcgcggagccgtcggcgaaccaccagtcgaagtcttggtgctcggtgatggcaggtagcgcggacgcgccgacaagcgaggtcagctccggctgcgtaccgtcggcgaccgtcgacgcgagcgactcgcccggcttggcctcaagcacccacgccagcgcgtaggccaggtcgcgccccgggttctgggagtgcgactgcacctgcagcgcgacgaagcgctcgccgccttcctcttccggacgcaccatcgcggcgccggcgcccggcagcacggtgacgatgttgaccggggtgccgttcacctcgaacgcggcgacggcggaggggacaaactcctgcagcgcgatcaggtcggcctcggcggccaagccgccgaacgggcgggggtccttggcaaactgctcgcgctcggcggcgcgcgccgccagtttcgcctcgcggcgggtcatgccctcgggcagctgctctttagtcttctgcttcttcggtttccttggtgccatgggcactcatcgtagccagcgcgaggtccggcaggtccgtagccatgacgtccaccccgtggtcggcgcaccactgcatctcaatcggcttgttcaccgtccacgtgtacgttttcaaaccccggtagcccagaagctccggcttggccatcaggtgcgagatcccgggccccacaccgtagggcttcgaccacatcacgttcttcgggttccagcgccgctcgcggaggttgaacaggtagaacgtctccagctgcggggcgaactcggtgaagtagcgcaccgcgcggtgggaaaaggagatgaggtggatgcgctccgagtcgtgcagccggtggtagcgaagggcccgcaaggtctgttcctccacctccggcccgaatcggctcgggtgtttagtctctatgtagaggtgtttgtcggggtgggcggtgatgaggtctaacaggtcgtcgataagcatcaagccctcagcgctttgcaccgggtcgtgcgcaaccaccagctcgcccttcggcgtgaggcgcacgtcgcactcgataccgtggatgggcagcgcgagcgcctcctcgaacgcctgcggcgtgtgctcgggaaagcggccggagaagccgcggtgcgccacaatctcagtcacgcgccccaccgtagtcgttgtttgacacaatgcttgcatgcaacgtccccgccttgaccagatgctggagtccgtccgcaacgcgcgcaaccgctactcggtgagcaaagacggcctgctcgcggcgccggttgcggcggtgcaggtgttcacggacctttcccccgcgctgcggctgcgcgggttccagcggctgcccaggagcttccgcgcaggcgccttgggcgccgaggtggccacgtggggcgcgctcgcaccgtcgctccttccgcacaagtgggccaccaccgcggcgaacacggcggtgctccagggcatcgggcacggggtggccaccgcggcggtgcgggtgttcttccccggcgagtaccgcaacgtgcgccagctcgccggcccgacccgcctggccatgacgggggtgaccaccggcgtgatcaccatggcgcttttgcgccgccgggagcaggagcacctggtggaggtcgagggcgactactccgtgtgggacaccatcggcgggctgaccctgggcaccatcggttacggtgcgctgctgggcgtcggggaggtcatccagacgcttatcgacgccctgaacgcactcctcggccgcaaactcccgcccgtgacctcgtggccgatcgcgatcctcggcggcggcgggctgatcttcctgttcacggaccggttggtgctgcgccgcttcgtctcgtcggtgatgcgcgaggcccaggagctcgaccgcgatttcatgcgcggcgccgaccgccccaccgagcccgagcgctccggctcgcccgcctccaccgtgtcctgggagtccatgggccgccagggccgcgccacggtggccgggggtccacgcaagcgccagatcgagcgcgtgctcggcttaagcgacggcgtggcgaaggaaccgatccgcatcttcatcggcctgcacgggctcgacgcgaagaagtcgcccgactacgcggcgatggccgaggaagcggttgcggagatgcaccgcaccggcgcgtttgagcgcggccacatcgcgctcatggccggcgccggcacgggctgggtgaacgacttccacacctccggcttcgagttcgtcacccgcggcgactccgcgatcgtgtccatgcagtactcgtttttgccctcggcgtactcctacctggcggaccacgaatcccccgtgcgctcgacgcgcctgctggccaaggcgatcctgcaggagatggagaagatcgacgaggacgcgcgccccaagctctacttcggtggcgaatcgctcggcgcctacggcgtgtccgacgtgttcgaatcggtggaggagttcatgcacggcacctccggcggcgtgttcaccggcgtgcccggcttcgcccgcaaccactccgagctcacccgccgcagggaagaaggaagtccgcagcgcctgccgcttatcgacggcggccgcaacacccgcttcgccgcccaccccgaccacctcgcccacgatttcaagggcgacccgtacgacaacgagtgggaggagccgcgctacgtcttcgcccagcacgcctccgaccccgtggtctggtgggagccgcacctgatctggcgcgccccggactggttgaaggaaccgggatcgcgcggccgcaaggcgcctgaggcgcagcacctcgacgtgctggacaccctgcactggttgccgctggtcacgttctggcaggtcgcgatcgaccaactggtctcccaagacgtgccgtcgccgcacgggcacaactaccacgacgagacggtggcctactggaacgctgtcgtccacggcgagggcgggagcgacggcgcgggtctaaccgaggcggaaatcgcccgcgccagcgcctggattcaccgcgacgcggtgaagctgcgcaagcccccgggtggcttcccttccaagcacgggtactgacatgaagatgcgctccgaagtattccgcaacgccgtctccgccgtcgccgcgtgggcggtgggcacggcgtcgctcctcgccggctacgcgtcgggaatcttggactaccaagacttcgacttctggggcaccgccctcgtcggctggctgctgatgtgggtgctcttcgttggcatctacagcacgtggaccgaccggatgctgcgcggccgcagccaggagcatctgcgggagtacgccgcgcgcgagcgcgccaccgcccgcaagccgtgggcgcagcagctcgggttcaagggcgccacgcagcttgccgtcaccgccggcttcgcctccctgttcctggtcatcatgagcacccagcttccccagacgatcaaccacctggcgctgctggtgctcaacgtcctcgccaccgctctgtcctggcactacatggtggtcgtcttcgccaccgattacctcgagctcgacctcggggaggacggcgcgcgccacttcgaattcgcgcacgtggaacgccgcggcgaggagccgatttacgacgactacttcaccctcgccgccttcacctccgtcatgggcgcgctggcacctgcgcaggcgctgacccgtaagggctggaagcggctgcgcgccaacgccatggtggcgttcgcgttcaacacgatggtgattgccgtggtggtcgcgatcgtgaccgccggcatcaccaccgagtagcctccgctagataccgcaggccacgcccgtggagtggtgcgggcagtacccgttgggcaccttgtgcaggtactgctggtgttcctcttcggcgaggtagtactccacgccgtctgactccacggatttgacctcggtggtgatctcgccgaagcccgcgtccgcgagcgcctgctggtactccgcgatccacccgcggatctgctccgcctcctcttcggtgtcggtgtagaacgccgagcggtactgggtgcccacgtcgttgccctggcggtagccctgcgtcgggtcgtgcgcctcaagcgcggccttcaccaactccttcaggctcaccacctgcgggtcatagaccacctcgaccagctccacgtggttggtcgcacccgagcacacttcgcgatacgtcgggtttggggtcacaccgccgccgtatccaacggacgtcgactccaccccgtccatctgccagtacatcttctccgcaccccagaagcagccgatgccgatcagcaggcgcttctgtccctcgcgccacgggccggtgatcggcgtggccagcaccgcatgcgtgcgcgggatggccagcacgggctcgcttcgcccggccagcgcctgatccttgtccaccaattgcggagttctaccaaagaggaatcccatagcgccccaatttacctcggcgccccaacaaagaaattttcattaccatggggcacgcaattgattttcaacgaaaggaatcaccatggctgtttacgagcttccggaactcccgtacgcgtacgacgcgctcgagccgcacatctctgccgagatcatggagctgcaccacgataagcaccacgcgaactacgtcaagggcgcgaacgcagcccttgaggcgcttgaggctgagcgcaacggcgaggcagacgccgacaagatccgcgcgctgaccaagaacctcgcatttaacctcggtggccacaccaaccactccatcttctggaagaacatggcaccgaacgccggcggcaacccgaccggcgctatcgctgaggccatcgaccgcgacttcggttccttcgaggcctttaagaagcagttctccgcagtggcgaacggcctgcagggctccggctgggccgtggctggttacgaccacatcgctggccgcctgatcatccagcagatgaccgaccagcagggcaacatctccgtggacttcaccccggtgctcatgctcgacatgtgggagcacgcgttctacctgcagtacaagaacgtcaaggctgactacgtcaccgcttggtggaacgttgttaactgggacgacgtcaacgagcgctacaccaaggctgcggcgtaaacgcctagcgtctcgctgcacctgccaacggcatcgggttgttaccggtgccgttttttggttgcgccgcagggtgagctgggccaccatgggtacgcatgaggaagggcagcgccgaataccgcagagccacgatcgcgatgctgttcgttggcctcgccgtcttctcctcgctgtacctcacgcaggctctcttgccgacgctcaccgaaaccctccagaccacaccttcgaccgccgcgctcacggtttcagctgcaaccggtgccctcgcggtctgtgtggtgccggcctccatcctttctgaaaagttcggccgcggccgcgtgctcatcatttccgccgtcgtggcgaccgcgctcgggatcgtggtggcgcttagccgcagcatcgagcaaatgatcgcgctgcgcgccctccagggcgtgctgctcgccggtacgccggcggtggcgatgacgtggttaagcgaggaactgcacaacgatgacctgcccggcgcgatgggcctctacatcgccgggaacacggtcggcgggctcatgggccgcctcatcccctccttcgtgctcgaggtggcgtcgtggcggtgggctatcgcggtgagcgcgaccgtgagcctggcgctggcgctgggcgcgtgggcgcttctgccggagcagaagaacttcgtgcccaaggagtcgattcggcccggcgcggagttctggtcggtggttgggcacctgaagaacccgcgcttagtcggccttgcggtgaccgcgtttttgggcatgggcgtattcgtttccatgtacaacttcttcgggttccgcgcgattgcgcagttcagcctaccgcctgcgcttgctgggttgacgttcgtgatgtatctgtcgggcacgtggtcgagcgcccgcgccggcacctttgtcggccgccacggccgcggccgggtggtcgtcgccggcgcggtgctcatgctcgtcggcgcgctcatcggcgcgagctcgaacctgtgggtcacgctcgttggcctgctcatcttcacggcaagcttcttcgccatgcactccaccgcctccgggtgggtgggccagatcgcggagcacgaccgcgccgaggcctccagcctctacgtgttctcctactacatggggtcgtcgctgctcggcgcggcgaccggccgggcgttcgaggcgctttcctggagcgggttcgtgggcgtgctggcggcgctgctggcggcgctcgttgcggtcgcgctcgcgctcgcggcaggcgagcggcgggcgcgctaacggcgcccgcgctaggaaagcggcggcacacccggcgcgcccgcggtgaggaagttgcgcaccgcgcgggtagctcggcagtcgtcttcgttgtagcgcagcagcatgtcgcgggcggccgcgtcgccaagccgggcagccctgcgcagcgcgatggagcgctccccgtccatgtcctcgtcctcccagcggaaccccgcaacgggcgcgagcactttcagccccaagccgtcggtgccgacaagatagcggcgggcgtgggcgaaaacgtccacccactcgtcggaagacgtgaacgcggcgacctcgtcggcatcgatagagccgaaccgcttcgccgaggagcgcatccagtagttctccccgccggcggcgtagcagtaggcgcggaacgtcttgccggccgcgtgcgcatctcggcgctgctgcatcagccacgcccagaaggacgagaagttggcctcttccgcctcgccgccaacttcctcccacgtgacaaaggcgtggtagtccgagccgtcgaaggcgccccagaggtaggcgccctggtcgaggtaggcctccatgtccacatcgatctcgacgtcggcgcgcgggatgtcgatctcgccttcgcggcgcagcactgcaacaccatcgcgccgggcttgagcgatgcgggaaggatcgccgaggttggcgtcgataagctgctgcaccgtgtcgatcccctgctgccgaaacgcgtcgccgcggccgcccggaaaaacgagcgagatgtcgtcgagctcctcgaggcgcggctggcacagcacccaaaaacggcaggtagcgcactgtttcaaccgcttcggctcgtctggaattggcgcgttcagcgcctcgatgagcggcgggatgaaacgggtgacgtccgcgatatacgcgcgcgtgcggtcttggccgatgacgccgccggagccggtgtccaacccctcggcgcgcagaagcagctccgccagacccaagcggtagccgtcggcggtgtggtggcgggccttggcgtgcaccgccagcgggtccgagaggccgaggcggttgacggcgaccatttcaagctccgcttccgggtggggcctggccacgcggtggttggagatcaccaccggcgcgtagccggcgtcggtgcgcacaagcacgtccacgtcgacggccacgcgccagccctcgagctcgccggtgagcgcggcgttggtgatcaggttggcgcccgcgcgcatcgcggcgcgggtctgggagaacgcttgctcgggggtcagcgcggggtcaaggtcgacgcggcggaaaagtttccggcggccgtcgccaaccgcccgcttcaccggcaagctgtccagcacgatcgcccgggccgcgtcgatctgcggctggcgcgacaccgcgtccggcagcggaggaacatccgggtgcgcggcgcgctggcggagccggtaccggcaacccaccaggtccgaggcgcgcacatccggatggttcgtcacaatgccagcgatgttacctgccgggaaaggtaaggtggttcaccgaagcttatttatagatgtagggagcacatttccatgggaatcatcaagtcgatccgcaggtcgcgcaagaagagccgcgccaaggcgcaggcggcggcgaagaaggcgcaggccgaggtgaagcgcgcggaggcgcgcgcacgcaagtacgcccgcgacgaggcgaaggcagacctgcgcaccgccgagctgttagacaaagcggaaaaacgcctgctgaaggaggagaagaagggcctgaagcagaagcgcaagcacgagaagcagctagccgaggcgcacctgaagcgcatcgaggaatccggactgaccaagaagaaggcgaagaagttcaccggcggtgcccgcgccctcatccccgtgctgcttccgctggcttacaaggcgctgacctcgcttcagcagggccagctgaacaaccgcgcagcgtcgatgggcctgacctcccaggacattgcccgccactccggccgcggcgccgagctgaaggcccgcatcgaggcgatccgcgcaaacgttgagcgcgacaacaacctgccgcgcggcttcgccgaagacgcgcgcgtgcgcctcgccgaccttgagcaggccgtccgcaacgcagagaacgcgagcccggtgcagcagcgtcttgcccacaacgcgatcgaggaagacctgaccgatctggcgaacctggtgcacgacaaggcggtcaaaaactagcggctggcttgagcccccgctagagcacgccgagctcgcgcgccgcggcgacggcggaggtgcgcgagcgcacgcccagcttgtcgtagatgtgcacgaggtggctcttcaccgtcgcctcagagagcatgaggtcttggccgatttcgcggttggacgacccagcggccaccagctgcagcacctccagctcgcgcggcgtgagcgaggagcgcggctccgcctcgcgcgtggccaggcgctcgcgcaccaccggcgacatcgggggcacgggcggctgcgcatcctcgccgccgacggagcgcaccgcggcgatgagctcctccggcggggcgtccttcaataggtagcccacggcaccggcctcgatcgcgccgaggatgtcggcatccgtgtcgtagttggtcaccaccatcaccttcggcggggttcccatggtggcgcggatctcggccgtggcctgcgcgcccgtcattacgcgggcaccttccgcgccggcaccgaagcgcaggtccatcagcaccacgtcgatgccgccggcctgggcggtcgcaatcgctgcttccgcggtggccacctcgcccaccaccaaaatgtcgtcggcctgctcgagcaccgagcgcaggcctagtcggacaatctcgtggtcatcggcgagcaagacgcgaatcatggctccatcctatccgccggccccgcagccgaaagcggcaccgcgacactcagcgccgtcggcccgcccggcgcggattcgatcgtgagctccccgccaagctccgcggcgcgggagcgcatcgcatcgagccctaaatgccccaaccccgccggcttgccggcttgcgcggccgcgtcgaagccgcggccgttgtccaccacgtccaggtgcacatcccccggctcgtaggtcatggtgatccgcacccgcgtcgcacccgagtgctgcacggcgttggacaccgcgccctgggcgatgcgcagcaggccggcctcgacgcgcatgggcaggtccaccacctcgccgtgggtttccacctcgattttcatgtcactggccgccacgaagtcggcggcgatgcgctccagcgcctcactgatgcgggcctcccgcagcccggccggggtgagtgccgcaatcatggcgcgcgtctccgcgaggttgttcgacgcggcccggcgcgccgcctccatgcgcttcagcggcatctccagctcgttttcccccacgtcgagggcgcgcaggtcgcgctcggcagcgtgcagcagcatctggatcgaagacaggttctgcgcgacggtgtcgtggatctcgtgggcgagccgctcgcgctcttgcgccacaccggcttcgcgctcggtggtggcgagttgcttgcgggtggccaacagctcgtcgataagcaaaagcctctctttgctcacccggctgatcgtggtgaacgcgtagttgatcgccaccacaaccacagcggacagcgcgggccccatcacgccgccgagggtgagaccggtggggacttggaagccgatggcggtggccaggcccagcgcgacccaggtcaggccgcgccaatcgttgaacgcgcgcagcgagacgaaaaacaggatgaacacccagtagatcgccaccggggaaacgaccatatccgcgatccagacggcgaacagcgcggtaatccagatcgcgcggtgccacccgccccagcgcggcatctccacaatgccgtaaaacagcaggaaggaaaacgccgtgaccagcacaatgtgcagcagcgccgcgttgagcggcatccgcgcaagcgccgcgagcgagaccagcaccagactcacggccagcacggtgatgccggtgtcgagggccttgttgtcggggatgtcggcggggtcccgctccaacatcactagtctggagctcatgcgcatgagactacccatcctggccttggcgatcggcctcgcggggtgctccgcgccgcaggtggttgaggaggcgcccgaggagccggtgcttgccgacgccccgccggtcgccatcctcccccacaccgaccgcgcgagcttcgacgaatgcccgtacctgaacacgcagtgggttgcggacacgaacgggcagcgcgtcaccggtgtgggcgtcgacccgggcccggacggggtgttcgacccgccggcgtgccagttctggtcctacccggaagagccccagctgacggtgtttgtgcgccgcatgccgacgccggagcaagcgatggccgtggtggactgggccgcgccggtggagttcaccgacccggccgaccagccggaggggtggaacgggggccgccacggcggcggcgcggtgccgggccgcatcggcgctgcgtactcggtggccaagggcccggtcgccgtgaccgtgttcaccaaccaggacgaatcggtcaaagcgcagcttgtcgccgaggaagttatcactaacctgggattgtgatgatcaatgttgccgctgttgtgatccgaaacgcgcgcggcgaggtgctgtgcgtgcgcaagaaaaccagcccgcgcttccagctgccgggaggcaagccggaggagggtgagtcggtggtggacaccgcactgcgcgaaacgctggaggagaccgggctcgagctggaccgcctctcactgggctacctcggccgcttctccgcgccggcgtcgaacgagccggggcacaccgtaacctcgaccgtgttcacggcgcccgagccggcagacgcacccgcgccggcggcagagatcgccgaggtggcctggatcgaccccgccgcccccggcgaggtggaactcgcgccgcttttggccacgcaggtcttccccgcgcttgcgccgcgccaattgcgcgccgttgccgtcttcgccggcgcgcgccccggcaccgacccagcgacatcccggctcgcgttcgctttcggtgaggcgctcggccgcgccggcatcacgctggtctacggcggctcgaagctggggctgatgggcgaggtggcgcgcggcgcgcacttgcaaaacggccggacttgcggcgtgctcaccacgcacttggcgggctacgagctgaagtacgacgagctcgaccagcttgaagtggtggacaccatggcgcagcgcaaagctcggatgggcgagctcgccgacgcgttcgtggtcctccccggcggggtcggcacgctcgacgagctttttgatgaatggacgaatcagcaactcggccttcacgccaaaccgattgggctgctcggcgagcagttctggcgcccgatggcggagatggtggaccacatggtcgaccacggtttcgtccgcgccaccgaccgcgaccacctgctcgtcgaagactcgccggagacgatgctggaatcaatgcggacctgggtgccgccggtgccgcggtggatctaaggcgccggcttgccgcggccgggttacacggcgacgtcgttgtacggcatcagtgatgacacccacgggaagacaacttccatgagtaggaagaagaccgccaccaggatgatgatggtaatcagccacttcaccgccggcggaccggggagtttgcgccacagggctgcgtacatggttgctcctttcgcgtatcccgttagctgagcctctaaccgagctccgtcatcgcaggcggcagcgcgccaccgccgcccggcgccttcggcatggattccgacatcaccgcgtggatgatcatgcgctccgcgttcgagaactgcgggtggcacgtggtcaacgtgatgattgacgccatgcccggcaccacctcggtcgagcgggtctccggcatggggttgaccacgttgatgtcgttcggggtcgtgatgtggcggcccatcacctgcgcgtagtcgccgcccgccacgcggtcggtgaggtcctggggcaggcacggagacacggacgcgcggcgcagctcagggtctgcgtccatgggcagcacccggtaggtcacccactgggactgggtctccaccacgatggcgtcgcacgttctcagctggcctaagtcgttgaacggcgcacccttgcccacgcggtggccggcgacagcgaagttgccgggctcgccgggcatctgcgtgccggggtagcgccctggtccggccaaaagcgtttgctcgccgacaccctccagcacggcgaactggtagtcggggccgaaggcggggatgtacatgcgcgcgaacgcgtcgccgtcttgcggcacgcggcgctcgcgcgggttgacccagttctcctcccacacggcctcgagccgcgactgcgcgtcgttctgcatcttggccgaggcgatgttggtccagaacgactcgtaaaacgcgaacaggagcagcagcgcacccacggtgaggaacacctcgccgacgatttggggcaccgtcaccggcttgcgccccgcttctccggccgggacggttttagccgccggagccgtctcaccgggccagtacggttgcggtggtgtggagcccgattgcatggcctaacattaacgcacatgctggaattgctcgtgtacccggtctcggccgtgatgaagttctggcattggctgctcacgggggccttcagcgtcgagtccagcaaagcgtgggcggcgtcggtgttcctcctcgtgctgtcggtgcgctcgatcatcctcccgttcgcgtggcagacgtacaagtccacgcgcacgtcgtttttgatgcgcccccacatggacaagatcaccgagctctacggcgagtccaccgaggtcgccgacctgcgcgccgaggagaaggcccgaaagcagatccagaaggagcacggctacaacccgttcgcggcctgcgtgccggcgatgatccagatccccgtgttcttgggcctctaccgcctccttttgtggatggctgtgccggacgccgccgccggcaaacgcatcggcgtgctttccgactccgagatcgcctccttccgcgactccaccttcttcgacgtgccgctggcagcttacgcgtcgatgacccaggagcagttcgccttcctcggcaccaccgaggacgaggtgattgtcctcgcagcgatcatgattctgctcgccatcgcgttcacctcgacgaacatgctggtcacgcagatccgcaaccgcttcaccctcgagtgggcgaacaccacgtcgcgccgggcctactacttcatttactgggtgatcccgctggtcgcgctcagcctcctcgttgcggggctgaccggccgcgtgccggtcgcgctgttgatgtactgggttgtcaacaacctgttcaccgccgtgcagaacgtctgcctgtggttctttgccgtgcgcacgatgccagcgaccccgctccaccgcgaggcccaggccgcggcgcacgccaaggtgaagcaagagcgcaagcaggtgaaagaggacagggcagctttacgacgccaacgtgtctccatcctcacccacccctccgaagccggccgcatcacccgcgaaatccgcgaagaaaagcgcgcgcgcaaggagaagaaggctgcggagaaggcggacgcgaaggcgctgaagaaggagcgcaacctcgcgcgcaaggagctgaacaagctgctcgccgaggaaaaggcggccaaaaagcgcgcgaaaaacacggaacccggtgccgccgccggcatcactatcgagggcagcacccgctggaccggcgagtagcctgcgctagatcgagtagtccgcaggcggtgcgccgagctcgtttttcgcgagctggcgcgcggttttcagcggcgcgacgctctgggtgaaccgggcgccggcgaggccgccgtcgaggaagatgagcatctggtccgcctggccggaggagtcgtacccgttcttctccgacagcagaccggtcagcgtctcgtgcatccagcgccggtggttcaagctggtctccacaatgcgcttctcggaatcggtttcaggacgcgggtactcgttcgccgcgttgaagaacggggacccgcggaacttcttctctggctcttcgtcaatcgccatgtcgaagaacgcgagcaccctcgcgtcgttgtcggcggcgcgatccgcgcgctcctgccagcgggtgcggtactcctcgtccatgcgctcgaggtaggccacgaccaagttgtccttagagccgagcagcgagtacagcgacgccttggccacgtccgcctcgcgcaggatgcggtcgatgccgatgacgcggatgccttcttcgttgaagagttttgtcgctgcgtcgagaagcctctgcctggggctgggccgattgcggcggcgcgtagccggcttcttcttcgccgggtctgcttgtgtcacactcgtctcctgttctcccactcgccaactagacaaaccggtacgttcatcttagaccctgccccatgcaaatgcccattaaaaaaatcccccggacggatccgggggatgatctaactagcgagttaacgacggctgctagtcaccttgttcacgatccacaggaggataatcgcgccaagcaggcaggtgaggaagctgaagaagaagttgcggccctcaacctggacaccgaagagggtcagcagccaaccgccgatgagaccgccgatgatgccgacgaggatgttcaggccgatgcccatctgcgcgtcgcggttctgcaccatcgacgcgatccagccggcgagaccgccgagcacgagccaaccaaagaagccgagagtaggagtcattgggataatccctttcacattgagttgtgtctatagaccttttgctgggcccattatgccagcctaatcctctggtcgcaccaccatcatcgggcacggcgccgactgcagcagcgcgcgcgaggtggaacccagcagcatgcccttgaatccgccgcggccgtgcgagcccgtgaccagcagctgcgcgccctgcgcggcctcggtcagcgcgcgcaccgggcggtcgcgcgtaatcatcttgcgcatctcaacgttcgggtgggacttggcaaattcgcccaggtactcgtcgagcatcgccgatttctccgcgcgggcctcttcccagcggtcgtccgtgatggtgaacgccgggcccgacattgtcacctgcgagtcgatccacgtgtgcactgccagaagctccgcgccgcgcgcttccgcctcttggaaggccacttcggtggctcgcttagacacctcggaaccgtccacgcccaccacgatcgggccgtacttcgtctcatcggtcaccgcgttgtcttcgcgcaccacgacaaccgggcaatgggcgtgggagaccacggcggccgagacggagcccaaaaccacgccggaaagtccgccgagaccgcgggagccggtaacaatcatgcccgcgtcgcgcgacatctccagcagcatgtcgatcggcgagccttccgccaccgcgtgcccgatgcgcagctcaggcgcgacctcgagtgcgaccccgcgcgcgtcgtcgaccttctgcatcgtctcgcgctgcaggtcgtcgtacagttcctgcggcggcaccatgccctcggcgtagaggaactgcggcatggtgtagctcgacgccaagcgcagcgccacatcgcgtttcgcggcggtgttggccgcccaccgcaccgcgttgtccgatgctgggctgccgtcgacggcgactacaacgtcgttctcgctggtcattacgtgctccttacttctccgggtacgccttcaagcttatcccttggtggcggcttccgcgtttgcagggaagaggaaccgatagagggccgccgcgacgtcataaatcgtcttgcccactccttcgcggaagaaggcgagcacgggttcagtaagagctgcaagatccatggcggataatctactacaccatggcacgtgctaaacgcccgaaagccgccccgctgcccccgcgcgacgggctgacggccacccgcgcgcggtacccgggtccagagccggttactgcgttcgaatttgtctcccacctggttgcgacgcagcggcacaggcaccctgaggacgacgaggctgccgtgttggagcgcttcgcgcaggggcaggttgtgcttgccgacgccacccccctctcccccaccacccccatccacgaaggcaccgacgtcttcttctaccgccgccccgcgcccgagaagccggtgccgtacgaaatcgggattgtgtacgaggacaccgacctgctcgtggtggacaaaccgccgtttctggcgacaatgccgcgggcagcgcacatcaccgaaaccgccactgttcgtcttcggcgagcgaccggcaacgaggaactcgcgccggcccaccgcctcgaccgcatgacctccggcctgctgctattcaccaaacgccgcgaaacccgcggcgcctaccaggagctgttcgcccgccgcgaggtgcacaagcagtacgaggccattgcccgcactcttgatctcgacacccccgttaccttgcgtagccacatcgacaagcaacacggcgagttggcctctaccgagatcccagacgtcgagccaaacgcggtgacaatcgtgcattcggccgctccactcgatccaacacatgccgatcgtttacaccgcctgcacaaagtgactgagcccttggcccgctaccttctcgaacccatcaccggccgcacccaccaactgcgagtgcacatgaattccgccggcgccccgattcttggcgaccccatctaccccacaccccttcccttcggcgacgaggacttcgcagtaccgatgcaactgaagtccgtcacgctcgccttcaccgatccgctcactggagccgaccgccacttctctgccccaggcttgggctagctgttgccggtcatggtgaccgcggcgggcgttggtagcgggcatccctgcgccggtttggtgtttgcactggtcgcggttgattgagccgcgtgttgcccactgtgggtgtgcgcggcctgtagctcccagggttgtgagctggtggcgacctggggttttgcacgtagtgatcgggctgttccgtgttgggagctacaggcctcgttgctgatagcgggtatctcggcgacagttgtgtgtttccgcaggtcgcgttgcgcggtcgtgggagttacccgctatcagtggttgtggcctgtagctcccaaggtttcagtgtgtcagcgacagggggttttgcacctaccgatgaggctgtttgtcgtcgggagctacagggcgcggcgcgtgcgtcgccggtgtcactgccgcctatgtgccgggagcgcgccgatatgtcagtgcagtcggcggcttgtagctcccaaggtttcggggtgtcagcgacctggggttttgtacctaccgatgagcctgtttttcgttgggagctacagggcggagccgtaacgcggccgcgacgacgttgcggccttcaggggggcggatgaagtatggcggatgcacggcgttgctctcgtatatccgccatccgttatccgccccccggtgtgacgctgttcggggggcggggctgggtgtggacatggcaaagcacccagtccaaggactgggtgctttggtgtattgagttgttttgttgttgttgggtcggcggtaacctactctcccacaccctcccgggtgcagtaccatcggcgcgggcgggcttagcttccgggttcggaatgggtccgggcgtttccccgccgctatca

SEQ ID NO: 13 - DNA, 80139 bp, Corynebacterium cassirii
  source 1..80139: mol_type = genomic DNA
ctcccccagcacctccccacccggaccgaagacgaccgcgcccaccggcacatcccccggcggagtcctttgcgcaaccgcaatcgcgcggcgcatgcgcgcttcagcgtcgcgtaacggcttcgatgaactcatccaaaaacccgaggtcctccgcgatcgtctcggccagctcgtgcgggccgggatcgctgtcgagcaggatgctcaagcgctcctccgacaagcccaagtcgccgaagatagcgaagtcgccgtcggcccacgcgtccacgtcgtccagctcgtcggggtcgatgtcggggacgtcaacgcccgcctcgtcgaggatgtccgcggcgaagtcgtcgtcgacggccatggtggcgtcggaaagcaaaagcctcaccttgctggggcccggacgaaccaccaccagatagtcctcctcgacgttgagcagcgcgaacgccgcaccttcgctgcgcagctggcgcaccgcgcggacggaggtgccaaggtcggtgaaatcgtcgcggaaggtgcgcaccacccaaccggcgtcggtgcgcgcgacggtgaccgcgtacccgtcctcgaaatcgtggctcatggggcccaagcgtagttaaactcgggcagcatgaggcaaagtggtgttttacgtccagtctgcgttgtcggcaacggcctgatcggcgggtcgctgatgcgggacttggcggcggagggcgccgaagtgttcgggcacacgcagtccaacgccggtgcgaggcaggcgcttgccgacggcttcgatatgtccaccaacctccccgaagtactttcgcgcgccgaggagctcggggcgttaatcgtggtcgccgtcccgttcgacgctgtcggaggcgtcctggacgcggtggcgcagtacgcgccgagctgcggcgtgaccgacgtagtgtcggtgaaggggccggtgtacgagctggtgcgcgagcgcgggatggaggcgcgctacgtcggcggccacccgatggccggcaccgagtcctccgggtgggctgcctcccacacgggcctgttcacccgcgcggcgtgggtggtgacgtacgactatgcgcttgaggtagatcgcgtgcccgagatgtgggcggagatgttcggtcaggtgtgccgcatggcggcgctggttggcgcggaggcggtgccggtgtcggccgcgaagcacgacgaagcggtcgcgcgcgtgtcccacctgccgcacgtgctggccgaggcgctgtcggttgtcggcgaccgcggccacacgctggcgcaatcgctcgccgccgggtcgttcaagggtgcgacgcgcgtagctggcacgcagccgtcgctggtgcgcaacatgtgcgagaccaacgccgcgtcgctggtgccggtgctcgacgagtacatcgagatcctgcagcgcgcccgcggcgagctcgcctcaggcgagccgtcgatggagtggcttgcggagtccggcttccgcgctcacgagcgcatggccgcccgctccggcgcgcgccgcgagtcggtgtcgccggtggcaatttcgtcgcgccccgtcatgcgcctgcaccccggcgccccggggtgggttaggcagctgcagcagatcgagtcgctgggcggccgcgtcgaggtgttttaagcttcccgacgccgccccatcgccacatacgccccaccaataatcagcgccaaaataccgagcgagatcaccgtctgcatcggggtgccggtatcggcgagatcgtcgtcgcggtcgtcggagctcgagttcgaggtcgagcggaccacggtgctgcccttcgcgttcgtcaccgtggtgcgcgagcccccggagccggcgacgctggtcgtgcggccggtggagaccttgccgttgagcgtggtcgcgcgcgcaccggtggtctcggtcgtggtggtgctggtggtcttggtgccgcccttggccatgcccgcgccgagcgccgccggaccagccagcgcagcaaccagcggctgcacttcttcgatcacgtcgaggatctgctgcggcgtggacttggtcgaggtggtcgacgtcgacgccttcggcagcacgatctccgcaccgtccgactcgcgcgagatcgatttctgcgcggtgcggtagccgttcggcgcggtgcgcacgccgagggtcacctccttgccgttgcccacgttgcccgggatgaagacgtacaccagaccgttctcgtctgtctcgccgcggacctcgacgtcaaggccgtgcacgctgtagacctgcgcgtactgcaccgggtcgccaccgtcggtcttgacggtgatgccgatcgtcgcgtcagcgtacttgggcttttcgttgccggacgctggcgcgctatcgatggtgatgtccagagattcctggtctgccccaatctcccaggtgccgccgcggttgccctcgatctccacgtagaacttgccctcggttacaggcacgtccagcgtcgcgtcgccgaaccggttcgtggtggaggttctaccggtgtagtcgtcgctaacaaccttcagcttcacgttgggttcgacgcggccagcgtcgtccttcacggtcacctctagtttgcgggtctccggctttttcccgtcgccggtgccggcggtgccgcccgcgtttgcatcagctccggtgtcgccgtctccaccgtcggcgaggagcgtgacgtacatgcgcttgtcggtaggggcgagctcgtgggtttcgccctcgaccagcacgtcgacggcgccggtgccggcgggcacgtcaacgaccacctgaccgttgcggtcggtgtcggtggagacgccgaggtcggcgatgttcacggcggcgcccttgacggcgcggcccttgtcgtcggcgacggtgatcggcacgcggcgggcctcggcggagaagacagtagcttcgctgcgcacctcctcggccggagcagccggtgcggcagcagccggggacggggtcggttcgccgcgctcggcgacaacggtcgggacggacacgtcgccgacggcgcgggcgacgtcgttggccgcgtcgcccacgcgggcgaggtcgcgcgcaatttcggccgcgtccgggcgggaagacgcggctgggacggcgtgctcgcccggcagcggggcgggcttgttgaactgggtcaccggcttgtaacccgcgccgagaggcaggtacgcaagctcgcggaagttgtccacgacctcgttggtgccggtagcgacaacctcggtgcccttcagctcgatggtgcgggcttggtcatcggcgaaaacaaaggtgtcgttcggcttggtgtaggcgtagttgaggttggagggtgcgtcaacaagcaggccctggcgaacagcaacctgatcgatggcaacccggccgttggtggtgtccagcgtccacttgtgcacgccgccgcgcttgtcgcgggagatggcgtacagctcgtgctgcttttccgggtcagtgctggacgcccatgcgctggggaaaccgatctcgcccgtgcccgccggcagggtgagcttctgcgacttcacagccagggaggacgcgtccttgatcttgtccgcgaatagggggttcgtcaggtcgtccttggccaggctgagcgtgcggaactccgagcccgagaacagcaccagcacgccggacggagtgattgcggcggaagcgacatccttagtgttgatgccgcgcaggtccaacgcgccgaggtccgcgagctggtccatatccggcttgatacgcaacaggtggcctgccggcttgccgccctcacccgtggagatggcgtagatacggtccgcgcccggatagtacgccacggcggtgtaggtccagccgccggaggagtagcgggcgtcggcggaaccgctgcccggcttcaccgtcttcaccaccgaacccgcaacgcggtcgagattgttgttgatcaccgagttcgcgccgttgatggttcgcgcgatgtccagcgggttgatctcctgcgcctcgaccggggtcaacgcaaacgcgccggcaactgcggcagccagggaaacgccagcgacgcggcgggtgttcttcgggtttttcatgggtacctctcgagtgattttgggcgcacgcgtccgcacacccagaaagccacatctgaatgtacttgcgttataggcctatctcaatacgtggaaggaaaacgtgaaaaccgcttagagcccgaggatcgaggtggcgatcatgaagtaaatgatgagccccgtcgcgtcgcagaacgtggagatgaacgggttggagaacaccgccggatctgcgccgacggttttggcgatgatcggcatcgcaccacccacggtcgccgacatcgtgcagatggaaagcagcgtcaagccaatcaccgccccgagatccatgccgtacaccagcgaggccagcgcgaaaccgaggccgccgagcaccgcacccagcatcaggccgacgcggacctcgcgccacatcacccgcacgatgtcggactttttcacgtcgccgagcgccagcgcgcgcgccaccgtcgtcgccgcctggttgccggtattcccgccggtgccggtgagcagcgggatgaatagcgacaggacgacggcctgctccatcttctcctcgaagacgtcgagaacctgcacggtgaggatcgcggagacggccagcaccagcagccacacgatgcgcgaacgcaccagtttggtcagcggcgtggacaggtacggctgcttcagcgcctccgagccgccctggcgggcgctgtcctcggtgtcctcgctttccacgatgccctgggcctcgtcgaaggtgaagatgccgacgagccggttgcccgaatccaccaccggcagcgcgagcagcgccagcgggaggaaccagcgcgcggtctcctccgcgtcggcggtcgcttccgccgacggtgactcctccagcatgtcggcaacgggagtgtcggcgtccgcaaggaacagccggcgcatcttcacaatgccgagcagctgccggtcgcggtcgatcaccgggagggtgtagagcgtctccaagtcctcttcctgctcgcgcagcatctcgcggacctcgcgcgccgtcatctcgaggtagatctcggggatctcaggtgacatcacgcggcccacagtccccttctcgtagccgagaaccgcgtcggtgttttccttgtccttttcgctcaggtccctcagaaggcgctcggcgacgggtccgggcagctcgtcgagaagcatgactcggtcctccgcccccatgccctcaaagaacgctccgacactgtcgctgcccagcgcgttgaccatttccgcctggtggcgtgggtcgagcgcgtcgaacacaacgcctgcgcgttccggcggcagcaggcggaacagcaccgcggcgcgcttgaccggcgaacgctcaatcagccggatgatatcgctcagcttcgcgtcctggagcagcccggagatctgttccgcgtcatcgccgcgcatccgcgtctcaacgaccttttcaagttcacgcagagcgtcgcgttgctgcatcgatgccataccgaccccattcatccgcacaaaaagccggccagggtggtcctgaccggctagagtttggtgcgcccggagggattcgaacccccaaccttctgatccgtagtcagatgctctatccgttgagctacgggcgcttgcaacgtgggattacattacacggcggcacgtattgctccaaaaccgcagggcatgatgcttttcgaggcccccttccccccgggggcacccactaactgagaacgtcctaagttttacgcaggtggcgttacgtttctgggcagctttgggatactaccaatgattttcccacctccctgccaaaaaggagccctcatggcaacaccaatcaagcaccgccgcgtcgtcgcggccggcgtcctctccttgtccttgatcgcgccgtctgttgccatccctcaggccgccgagctcgtcttgcctgccgccgccgcccagaatgctgacgttttcaacggccgctacaccactgcaaacttctggaacgagaaggaagcagtcgtagagggtctcacgcttgagccggggacgaaggtcgagccgacgacgaacaccatcttcaattggaatttccgcaacgacggcggccagctggtactcatccgcccgcagtcgcaggccgcgtttaaaaccggcgatgttgatattcgcgtgaaggttactcccgccaacggcaacgcctaccgcaccacgttgaaggtgactgttgtcgatgagggccggacgccgcctgcggcggttgaggaggccgtcgacaagcaaagcttcgacgagcgctaccccaccgccaacttctggaatgcgaacgaagcggccgttgaggggctgacccttcagccgggcaccaccgtcaagccggcggcgaacaccatcttcaactggaacttccgcaacgacggcggccagctggtgctgatccgcccgcagtcgcaagccgcattccgcgccggcgaggttgacatcccggtgcgtgtggcggaagggaatggctcgacatacaacaccacgctcaaagtgaacgtcatcgacgcgcgaactccgaaggagtgggagcagcagctggcgaagacttacaccatggacttcgagaagtctgctgagccgaaggcgattgaggacatcacgttgccggagggcgtgaccctgtctaagggaaccgttgcaccaccacctccgggctggggggtatccgttgagggcggcaaggtgaccgtcaagcctgcgtcgacctttaccgaaggcttcatcgagttgcccgtgactgtgaacgacggcaccgatgagttcggcgcgaaactccgaattaacgcgaagaacccgcagacctccacctccgacatcactagcggtgttggtaagacgatcgggtccatcgtcggcggcctgctcggcatcccgaacttgggcaacctcttgggtggcggctcgggcggctccggcggcggcagtggccgactcgtgaacgtggtgatcacgaacaatgccaacaacaacggcagcccgaacatcatcatcacgaacaacgccaacccggtgattaccggcaacgcgaatgacaatggctcgaacaatgggtcccacaacagcgccgtcatcaccaacaacgccaacccggtgatcaccggcaacgcgaatgacaatgcctcgaacaatgggtccaacaacagcgccgtcatcaccaacaacgccaacccggtcataacgggcaacgccaacccgaacgtcgagatcaaggacaacgccaacccggtcataacgggcaacgccaacccgaacgtcgagatcaaggacaacgccaacccgtccgtcgtcatcaccaacaacgccaacccggtgatcaccggcaacgcgaacccgaacgtggagatcaaggacaacgggtccaacaacgcctccaacaacacggcgaatgtctcagacaacgcgaacccaaccgtcgtgatcaccggcaacgccaacccagtgattaccggtaacgccaacccgaacgtggagatcaaggacaacgggtccaacaacgcgtcgaataacaccgcggagatcaaggacaacgccaacccggttgtgaccggtaatgcgaacccgaccgttggcggcggcctcggcagcgcgctgggcggctcgtcgaagcgcgacaagggcaacggcaacggtgacggcaacggcgcagctggcggcggcaatgctggtagctccaaccgcggcggctccagcatcggcgctgacgtcgaggccaccggcggcctcaccgacccgcgctgcgtcgcatcgctggccggtctcggcctcccgctgctgctcgccatcccggtcgccctggctcagggcctgaacacgccgggtctcgaccagctctcggcccaggtcgccggcgcgctcaacgacaccgcgcgcaacttcggcgttgaggcggcgcaggtcaccgcggtcgccggcggtgtggtcggcgcgaccttggccgtggttggtgccctcgcgctcgcgacctgcatccccgacgtgcaaaacgttggcatcaccgtaggcggcccgaagacggtaacagaaacgtcccccacacccgccccggcggccactgtggtgaccaacccgacggagccgaccgccgcggcgtaaaccactgcagagctaagaaaaccccgcgtgagcggggttttccttctgtgcgcccggagggattcgaacccccaaccttctgatccgtagtcagatgctctatccgttgagctacgggcgcgtggcggagacgacaggatttgaacctgcggccctcgtcaagaaggcaactccttagcagggagccccattcggccactctggcacgtctccagacctcgtcacagcttagtccacgccacaccacgggcaaaatacgcactgatttttccgtaacatcaacggtatgaaactcaacacttggctcaactccggcttctgcgcccgcggcgaccacgccgatacctccaactggatcgtctggttccccgcgaacctcgacgctttgaccgctggtccgctcgcaggcgacagcaactcggttcccttctacctcaccccgaagacctcggtacttgcggtcgacaccccgggcgagatcgtccttctcggcgtcccgctcggcgacctcgagggttcctggcgcttcagcgaccgctcgggcgccggctccgacgtcaactccgtcgagtcgttggaagaggtcgcgggtctcatgggcaacgaattcggccaccgcaccgacggcaccgctgtggtgcagctgcgcggcacgttcccgatcgagaaggtccaagtggttgccggccagaaccgcgcggccacgaagcgcgcgatcggcctgctgaacggcgtggaatcggacttcgacggcgagcgccagttccacaccatgccggagctcttccccgacgaggcgtaacccccaaaaaagaaatggcggagacggcgggatttgaacccgcggaggtgtgaccctcgccggttttcaagaccggtgcattcggccgctctgccacgtctccaactccggtaatgctacacgcaggtattctgggcgggcatgaaggccatccagatcacggacccgaataacccccgctcgcttgagctgcaagaagtggctgcaccggagctcgatgaaggctcggtgctcgtcaaagtcacggccgccggggtcaaccgcgccgatcttgtgcaggccgccggcaagtaccccgcgccggagggcgagtcgaacatcatcgggctggagtgctcgggcgtgatcgtggatccgggcaccacggaccgcaaagaaggcgaggaggtcggctgcctgctcgcaggcggcggctacgccgagtacgtcgccgtgcctgaaggtcagctcatgccgcgtccggagaacctcacgatggttgagctcgctggcgtggtcgaagtcgcctgcacggtgtggtcgaacttaggcatggtcgcgggcatccgcgagggctccaaggtgctgattcacggcggctcgggcggcatcggctcgttcgcgatccagctgtgcaaggcgctgggctgcgaggtggccgtcacggcgggctcggaggagaaactcgcgtactgccgcgagctcggcgccgacatcgcgatcaactacaaggagcaggacttcgccgacgagctcaaagggtgggctgacgtgattttggacgtcgtcggcgggccgtacctcgaaccgaacatcaaggcgctggctgtggacggccagctggtggtcatcgcgctgcagggcgggcacaagggtgagatttcgctgggccggatgatgccgcgcaggcaatcgctgcaccctaccaccctgcgcgcgcggccgcgggcaatgaaggcggcaatcgtgcgctcgaccatcgaaaacgtctggccgctcatcgaatccggggagattgtgcccaacgtgagcaggacttttccgcttgtcgacgccgccttagcccacgaccacctcgactccggagaaagcaccggcaagatcgtgctggaagtcggggccggcgggaactaggcgaggctcgcgacggtcctcgtcagctgcacgacgtcagcctgggtgttaaacgggctgaggctgacggtgactgcgccgcccatgtcgtcgacgcccatgtcggtgagcagctgcgtcagcggcgtctcgctggccacgagcccgttggctacgaggcgctggtacaccgtcgccgagggcaccccgttcacgccgaacgtcaggcgcgggatgcggtcggggcgggcgtgctccgcggcctcgccggacacacccacgatgtgcacgccgggcagggtgccgaggaaggtgtagaggtcttcgcgcaggtgctccatgtagtcggcggcctctgccatcgacgccaccaggcggttgcggcgcgacaccttcccctcggctaccgctgccgggacggccagcgaggcgtagtgctcgaccgtcgcggagaccccgccggccaacccgggcgcgaccggcagatcgagcatctggcggtcgaggcggcgcagcatcgcctcgtctcggaacaccagggcggagatgtgcggcccgcccagctcagccacgtcgagggcgacaatgtcggccccgaactcgtcgaaggtgagggggcggtagggggcgtagacggtggcgtcgacaagcagccatgccctcgagcgctcccggagcttctcccccaccgacgcgaccgcaaccaccgtcccgagctcggcgtgcgccgcgggcaccgacaccaagcgggtggaaccgtcgacaagatcggcgaactgccacgcgggaagctcgcccgtcgccaggtctgccgcagcccagcgcacctcagcgccggtgccttgaaggatgctggtcaactgcgggcggtcgaggttgttcagcacgatcgtggagttgtggcgcagcaccgggcgcatcgcgttggccagcgccatgtagagcgacgaaatgtttggccccagcaccacgcgctccggcgtcgcgcccaccaggtccgccaccgccgcctttgcgtccgcgatcaacgttgcgccctcaggtgcgcccggcgcgtggcgggtgtgggtgccgcgcgccggctcgggcggagcgaccgtcggggccgcgcggaagctgcgcgccaccgccgaggccacgcgctccggtacctgcggcgcgtcgtgcgcgttcaggtacgtccacccgcccgaaagggatgtgtagagcccgcgcacactcgccacgtcatacgccatgctgcccacacctcactcgcggtttcattagtccataattatgcacgctgcgttcacacgctgcatcctcgcagcgtggcggcagcggggccgacccaccacgcaggtgcgcgggaaacgcacccgcgggcgctagggtgttgagggtgcaggacattcaacaattgcgctccgacgtggccaggatgaccagtgagccgccgtcggcgacgcctgcgtccaagtccaagaccatggccatgtcgtggcgcgacctggcctacgggtggcgccagaacgagctgtggctgcagctcgggtggcaggacatcaagcagcgctaccgccgctccacgctggggcctttgtggattaccatcgccaccggcgtgatgtcgctcgcgctcggcctgttgtactccatgctgttccagatcgacgtggcggcgtttttgccgcacgtcaccgtcggcttcatcgtgtggggttttatctctggctgcattaaagacggcgcgaacgtcttcattgaaaacgagggcctgatcaagcagctgccgtcggcgttgtcggtgcacgtgtaccgcttggtgtggcgccagctgctgtttttcgcgcacaacatgatcatctggctcttgctgatcatgattttccgcatcccgctcgggtggaacgtgctgtgggcgatcccgggcctgatcttgctggtgatcaacggggtgtgggtgaccatgctgttcggcatcatcgccacgcgcttccgcgacgtcgcgccgctgctggaggcgttggtgcagctgcttttctacgtcaccccgatcgtgtggacgaccgacacgctgaaggagcagggcggcgaggttgcccggcgcgccctgctcgcggagattaacccgctgtaccactacctcgagatcgtgcgcgcgccgctgattggcaagacggtggacccgtaccactggtggattgtcatcggctgcacggtggtggggctgttggtgtccttgttcgccatgcgccagatgcgcttccgcgtgccgtactgggtataggagtttcacatggtttcaatcgacacctacaacgcctgcgtggacttccccatcttcgacgccaaatcgcggtcactgaagaaggcgatgatctcgtccgccggcgggcgcatcggtaaaaacgacgccaacaccgtggtggtggaggcgttgcgggacatcaacctccacctgcgcgagggcgaccgcgtgggcctagtgggccacaacggtgcgggcaagtcgacgcttttgcgccttctgtcgggcatctacgaacccacccgcggctccgctgaggtgcgcgggcgagttgcgccggtgttcgacctcggcgtgggcatggacccggagatctcgggctacgagaacatcatcatccgcggcctcttcctcggccagacgcgtaagcagatgaaggcgaagatggacgagatcgcggagttctccgagctcggcgactacctggacatgccgcttcgcacgtactccaccggcatgcgagtgcgcttggcgctcggcgtggtcacctcgatcgagccggagatcctgctgctcgacgagggcatcggcgccgtcgacgccgcgttcatgtccaaggcccgcgtgcgtctagccgagatggtggagcgctccggcatcctcgtctttgccagccactcgaacgacttcctcgcccagctgtgcacgacagcgttgtgggtggacaagggcgaaatccgcaaagccggcttggtcaacgaggtggttgaggcctacgaaggcccggaggccggcgagtacgtcaccgaactggtcgagcgcttccacggcccagggttcgcccggtagcaactgagcaaggcacaatacacaccatgaccgccacgctaagcagcactggaacgaccgccgccgtcattgtcacccacaagcgggtggagttgctcgccggcagcttggagcaggtggtgaaccagacgcacccggtggactgggtgattgtggtggacaacggggcggagccggaggttgagcagctgctcgccgacatggccggcgagcgcggcgtgtacttggcaagcaagaccaacctcggcggcgcgggcgggttcgcgtacgggttcctgcacgcgctcgcgctaggagccgacgcgatctggtgcgccgacgacgacgggcgcccggcggaccacgcaacgctggcagagctctaccgcgtggcggaagcaaggcgcctgcacgaggtgagccccgtggtggccaacatcagtgacccggcaaaactcgcgttcccgctgcgccagggcacggtgtggcaccgccgggtggacgagctggagggcgactttttgccccgctacgccagcctgttcaacggcgcgttgatctccgcggaggcgatggagcgcatcggcgtgcccgactaccgcctgttcatccgcggcgacgaggtggagtaccaccgccgcttagcgcagtcggggctggactacggaacggcgctgaccgccttttaccttcacccggacggctcaggcgagttccacccgattatgggcggccgcgcgcacgcgcagtggccggacaacgacgcgaagcgctacttcacgtacagaaaccgcggctacatcatcaaccagcagggcatgcggaagatgaagctgcaagaagtggtgcgcttcgggtggttcttcctcgttgagaagaaggacccgcgcgggtttattcagtggctgcggctgctgcggatgggggcgcgggaggatttccgccggccgtaggctcagactgcgaaatgatcttcgtctcctcgcggaagatcacgtggcgctgcaggacgaagttggtcaccgtcgccacaccctgggcgatgacgaaggcgaacaggtcggtgaagaacttgccaaggccgagcgcgcgaagcggcggcgccgcccagcggtagagcagcagctgcaccgcgaacgtagatgcgtacagcagcgtcaccgcgccggccttgcgggcgttgacctcggcttggaaggcgaagcgcgagttgagcaggtacgccgcgagcgtgcccacgcaccagccgattgccttcgacatctcgcgcgacagtggcgtgagctgggtgagcgagtaggtcacgccgaagtcgagcacggcgcagccgatgccgatgatcacgaacggcaccagctgtttcttcagggcggttgaactcacggccggagagtctacccgcgcaaaaggtcgcggtagacatccaggcgcgccggaagcggcaggtcggcgcaaagcgcgtcgagctggcttatcgacaccgcgcacaacccccggatctcccgcacattcatctcgccccaccccagcgagcgcatgatcgattcggtcagatccgcggtaacctcctcgtccacgcagcaggccgacgccaagacgacggaccagaaggcgtcgcgggcgcgcgggtcttcctcgagcggcaggctttggaggatggggctggggtggttcgacggggcgtcggcaagcaatgccctctctaccccgagtgcctggatgagcggaacaaagtcgtgggaggcggcgcggcgcagcacgtcgcgggcgtcggcccgcacaagctcttcgaggccttcggcgcgctcgacgccgagcagccgcgcgttgacctcgcggatgttgaaggcggcgccgccgaagctgccggagcccgcaacgcaaatcgacggcggggtggattcgtcgcgcctgtacacgtcggccagctgcatgccgaaggtccacaggccccacgtgaaccgggtggattcgccggggcgggtcagcacctcgcccagctcaagcgcggcgtcagcctccgcgcgcacccggtcggagcggtcgtcgatgccgaagacggtggccacgacgcttctgcactcgtccacagtcgtgcgctcgtggatgccgacccagcggtacacagtgtcgtccgcaagcagcacgcaccgcaccatcagcgtgtcgccgacggagctctccccggcgagccgcgcccgcgcatcggacagcgatatgacgggcgccaggtagtccgatgtgtagatcgtgctcgacatggcgcccaagatacctatttccgcaggcgcttcgctgccaggtacgccgccccaagggatgcaccaaggagggcttcaggcttgtcgacgccccgtttccccatcccagccgccaccgcgtcaaccgccttggacgcagtccagcacgcggccgccgcacccgcggcaagccccgccagcacgccccacgacagcccgacggagtcctcttccccctgctcctcgtccaccaccgcggtgagatcgttcgttttgtcctcctcgaacgcgttgaacgcggcgatggtggcaacgttgcccaacaccagcggcacgcgcgcggcgggcagcgccgcgaacgcggcgatgaacccggcctggatgcactggccggcaaacgtgttgtcgagcgcgttgtagtcgatgcgctcctcgtgcgcggtgtcctggatggtcatgcccgccgatcgtaccggtacggtttgacgcatggagcaaccgctaaaccacttcatgcagcagttgatggcccaggaactgccggtgctggactcggccagccgggcgcgcgtgatgaaggtgctgaaggaatacgacggccccgtcatcacgagccaggacgagcttcccgcggagatccgcgagatcctcgaactgtaggactacaactttaggatgaaagtcacaccatttgctcacggttttgggcggaccgctgggtaacgtggggagccatgacactgcacaccgatttgaagtccctgcatggctggggcagaacggcgccttcgactgcgcatgtcctttccacccctgacgttgacgtgatcaaggcggccgtcgcgcaggtggcggacgagaactcgtcccttccggagtacgcgcgccgcggtgtgatcgcccgcggcctgggccgctcctacggtgacccggcccagaacggcggcggcttggtcgtggacatgaacccgctgaaccagatccactccatcgacccggacaccggcatcgtggacgtggacgcgggcgtgaacctggaccagctgatgaaggcggccctgccgtacggcctgtgggttccggtgctccccggcacccgccaggtgaccatcggcggcgccatcggcccggacatccacggcaagaaccaccactccgcgggctctttcggtgaccacgtgctgtccatggagcttctggttgcggacggccgcgtgctccacctcgagccggagggctccgcagacgacccggacggcaccctgttctgggccaccgtcggcggcatggggcttaccggcatcattctgcgcgcgcgcatccagatgacgaagacggagacggcctacttcatcgcggacaccgagcgcaccacgaccctcgacgagacgatcgcgctgcactccgacggctccgaggtcaactacacctactcgtctgcctggttcgacgcgatctccgcgccgccgaagaccggccgctcaaccatctcccgcggctccttggccacgctcgcgcagcttgaggagtacgcgccgaagctggcaaaggacccgctgcgcttcaaggccccgcagctgatgacagtgccggacatcttcccgtcctggaccatgaacaagctgacgctttccgccatcggcgaggcgtactacctgatgggcgcgccggcgaagaaccaggtgaagaacctcacgcagttctaccagcccctggatctgatcggcgagtggaaccgcggctacggcgacgccggcttcctgcagtaccagttcgtggtgccgactgacgctgtcgagccgttcaaggacatcatctaccagatccagtcctcgggccactacacggcgctcaacgtgttcaagctgttcggcgagggcaaccgcgcaccgctgtcctacccaatgaagggttggaacgtctgcgtcgacttcccgatccgcgacggcctcaacgagttcctcgaccgcctggacgaccaggtgatggagttcggcggccgcctctacttggccaaggagtcccgcacctccgccgagaagttccacgccatgtacccggggatggcaggctggctggaaacccgccgcgcgatcgacccgaccggcgtgttcgcctccgacatgtcccgccgtttggaactgaactaaggagaaccaatgcttaacgcagtaggccaagcccagaacatcctgctgatcggcggcacgtccgagatcggcctcgccattgtcagcgaacttgtctcccgcggcggtgccccgaccgtcaccctcgccgcgcgcgaggagtccccgcgtatcgacgccgccgttgccaccctccagcgcgccggcgcatccgagatccgcctcgtggacttcgacgcccttgatttcgagtcccaccctgcggtgatcaacgccgccttcgacgccggtgacgtcgacgtcgcggttgtcgccttcggcaccctgggcgaccaggaggagctgtggcaggaccaggcgaaggccgtggattccgcgcaggtgaactacacggcgttcgtctccgtcggcgtgctgttgggccaggccatgaagcgccaaggtcacggcaccatcatcgccatgagctcggtcgccggcaccaaagtccgccgctccaacttcgtctacggctcggcgaaggccggtatggacggcttctacctgcagcttggtgaggcgcttcgcaaggacggcgtgaaggtcaccgtggtccgcccgggccaggtgcgcactaagatgacggccggcttgaaggaagcgccgctgaccgtgaacaaggaagatgtggcgcaggcagctgtcgacgccgcgctgagcggcgagcgcttcgtgttcgtgcacaagctgttctggcccatctcgaccgcgctgcagctcatcccggcgccgatcatgcgccgcctgagcttctaaccgcggatgtgttcacgccccagtgaacacatccctgccgcggcctgtggtgtattcactttcctcaggccgttttcattaccgatcgaatttgttcacattcccgatccacgccagcgaacttttcctagtcgttcgcccggcccatcccgcgcagcactttctcgcgcaaccggccggtccccagcaccgccaggacgcaaccgaccagcgccaccacaacgagcgcgccgaacagcaccaacttgtccatcacattgacgtggaccaagaccatgacggtgcccatcaggctgcccatcccgaacccgagcagcgccaccaccagcatgggcaccccaacctcgcgggcagccaccttggtgtggaaggacgcgggcgcaccgatgaagtagaacgacttggtcagctgcttctgctccaccacgctcagcgcctgggtgagcaaagtggacgacaccatcagcaccgccgcgaagaccacggtgatagccacaccggaggggatatcacccgcgatcatcttcagggcaggggcttcgtcaatttcaggtaccgctgagaaccaaccgccaacaccgccgataaacgccacgaagtagagcgcggtcacgcgcttccatgtggttttggcaccccggcccacccggcgcgtggctacgtagttggcagccccgggcacccggtagctcagccgcgcgagcagctggatgatgccgacggcgatcagcgcgttgacggtgagaatgccgccggcgacgaccagcatcgcggcgtatgccgccgcgtcggcgcccggcgcgatgttcatcgagcccagggcgcggtacagcaccaccgcgccaaccactgacaacaccagcgtgatccagctctgcccctttggcgggatctttttggtcacgccgagtggggtcacggcgactcgtcgcaaagcaagccacacggaacaggcggccaagaccaacaccacgatccacgcggcggggatgacccaccaagtgaacatctcccaggtgccgacacgcttttcctggaacgtcagcaaactccacgcggggcacgtgagcacgtacagcgccgagccgagcaccagtccggcaagggcctggcgcagcgattccaggatcatcatcccgcgcacctcgccagccgtcgcgccgatgaggcgaagcgccgccaggtgctcctcgcgcccgccgaggttcgcccgcgcggcctgggtgagcagccccaacaggctcggcacgagcagcacactggcgaacaaggcaaggaacacgtactccagtgagatcggatcgacctccacgagcgcttcatgcgggtgcatgttgcgcgccacgaacatccaggtgccgcccatgagtgtgcacagcatccacgtcgccaccgtcaccgcgaccagcgacagcgcacgaacccagcgctcgccgatctgccgttgcgagcgcccttcgcttgtctgcgacaccgccgaccgcatcaacgtcaccgcactcatcgcgccacctccgagtggatcaggccgtcgcgaatttcaacgcggcggctgcaccagtcggcgatcttcgggtcgtgcgtgaccaccacgagtgtcacaccgaacttctgacacaccgccacgatctgctgcatgacttcgtggccggtggcctggtctaacgccgcggttggctcgtcggcgaacacgacggacggcggcccggccaaggcacgcgcgatggccacgcgctgcccctgaccgccggagagctgccccggataccggtccacataggcacccaggcccagcctggtgagcatgtccacagcatcattgtgcgcctgcgaccgcgccaccccgcgcatgatctgtggcagggcaacgttttcggtggcggtcagctcgggcaacagttggccgtcctggaagatgaagccgaagtgctcgaggcgcaggcgcgagcgttcggcgtcgctcattgcggccacatcgtggccgtcgaacagcacctcgccctggtcgggcacgagcacgccggacatgcagtgcagcagggtcgatttgccggagcccgaaggtcccatgatggccacggattcgccgtcgcccaccgtcaggctgatgccttcgaggacccgctgctgggggaatgactttgtgatgtctctgagttcaagcatggtttctatttcacaggtggtcgtcgtgaagcactatggccctgactcccgaatatgggtagtgctagctctaccccgctacgctcgcgggcatgcggcaacgaaggaaccacgagcagcgggcttccgccaagatccaccagctcactgcctctcggcgcaagattgcggaggcgtacgaggtggagcgcctgcgtatcgagcgcgacctgcacgacggcgcgcagcagtacttcgtggccgcggcgatgaaactcggcgaggccagactcgacgttgattcgccgcttctcgacgacgccgcccgcgacctccgcaacggcctcgatgcgctcaggagaaccgtgcgcggcatccacccgcgggagttgtcggaccacgggctcatcgccgcgatcgagacagccgccgcgcagtacggcccgcacgtcacggtccgtgcaccacacgaactgccgcgtatcgacgactccgtcaccgcagccgcctacttcttcaccgccgaagcgctcaccaacgccgcgaagcacgcaccacaggcacccgtcagcgtgctcgtgacctgcgaccacaccctgaacatctcggtgaccgaccaaggcggcggcaacgcgcgcatcacccccggtggcgggctcgacggcatgcaggagcggatcgcggcgttcggcgggtcgatggaaatgacctcgcccgacggcgggccgaccaccgtcaccgcccgtattccgttgctgttgttccgaggagaaagtgggattgcgccatgaggattgttatcgcggacgactccgcactgctgcgggaaggcgtcgctggtctactcacccggcgcggccacgaggttgtggcgcaggtggatagtgcggatcgggtgcagggggtcgtcgatacgcatgcgcccgacctggtgatcacggacgtgcgcatgccgcccaacatgcgcgacgacggcctgcaagccgcgctggagctgcgccagcgcggcccggtcaacgtgctggtgctgtcgcagtacgtcgcgcccgcctatgcgcgggaactgttctccggcggcgacggcggcaccggctacctgctgaaagatcgtgtcgcggaggtgaaagacttcatccaggcgtgcgaaaccgtggcgtccggcggggtggtcatcgacccggacgtggccagcgcgctcatggccgcgagctcgcgctggctgaccacgctcacgccgcgcgagatggaggtgctcgaacacatggcggaggggctgtccaacgctcagatctccgagcagctctacctctccggcgcggcggtggcgaagcacgtctccagtatcttctccaaactgggacttacccccgacgaggacaaccggcgcgtgcgcgcaatcctgatgtacctggcagaacgtggagttgggtagcgtacgcggcggtggtggccattttcttgccggcggcggcaatcatggcgtaccgcgcggcgcgcggctcgtgggcgcctccaagatgactgcggacttgaaggaagcgccgctgaccgtgaacaaggaagatgtggcgcaggcagctgtcgacgccgcgcttagcggcgagcgcttcgtgttcgtgcacaagctgttctggcccatctcgaccgcgctgcagctcatcccggcgccgatcatgcgccgcctgagcttctaaccttctcaagcccggcacgcccccgtttccagcaagggggcgcgctgggcatgtgcgaaactaatgggcatgacaaccgcagtttcccgcgaaatgcgggtcatcgagtatgccccggacaagctgtccgccaagcaaacggtgatccgcgcggtcagctatctcgtgctcggcggcgttctggcgcttgcgtcgtggttcgtgctccactcgctgtcgctgccggcgttcaacacctcgatgatgacgaagtcgctggccgcggtgtcgtcgttggtagtgatcgcgctggcggtgtggtgctgcctgctgtgggtccgcgagcaccagaacctcctggttgagagtgtcgtgtcgttggcgccggcggcaattgtggtgacgtcgacaggcatcccgctcactgccacccgcctgtggctggacggtatccaggtcgaccagggcttccgctcgcagttcctcacgcgcatggcgcaggcgccgtcgtacgcggacatgaactacgtcgacctgcccacgttctaccccctcggctggttttggctcggcggccgcatggcgggcgtgctggatatgccgggctgggaggtctaccagccgtgggcgctgacgtcgctggcggcggtggcggccatgctcaccccgatctggcggcggatcactggatccctgccggtggcggcggccatctcgatggtcaccgtcgcggtcgtgctcacagaggtgccggaggagccgtacgccgcgatcgtcgccatgctgttcccggcggccgcgatcgcggcgcagcgcgcgctctacggctcttggttcgccacctgggcgcttgcaggctacctcggcatttcagccacgttctacaccctgttcaccgcgatcatggcgctgacggtggtggtgatggcgatcgtggcttacttctggacgggccactcgctgctgccgatcaagcgcctcatgatcgtcggcttcacctcgatcgcgatcgcgttgaccgcgtggggcccgtacctggtcaaactgctcagcggcaaatacgacgcgcactccaccgcgaaccacttcctgccggttgagggaacgtacttccccatgccgttcttcagcatctcgatcatcggtgcgctgtctttgatcggtttagtgttcatcatcctgcgcatcagcgacatggaagttgcggcgctgagcctcgcgcttctgatgtgctacatctgggcgatgggctcgatggcggccacgcttttgggcacgtcgctgctcggcttccgcgtcgaagtgctggtcatcctcatcttcgccacaaccggtgtcctcggcatcgcggaagcgcagctgaccggcatcgacttgctctacccggggcgtttctccgagcgcagccaccgcggcatcctcaccgcgttcatcgtcctcgtcggcgccgggtccctgtactacgtgcagcagatccccgcggagaaccagaagtacatcgaccaggcgtacgccgacaccgacggttacggcgagcgcgccgaccgcttcccgcctgacgcggcgaggtactacggcgacatcgtcgagtacttgagcgaccacggccgcaagccgaacgaggccgtggtctacaccgacgagattaacttcatggcctacaacccctactacgggttcaacgcgttcaccagccactacgccaacccgctcggcgagttcgacaggcgcaacgaggagctggtgcactgggcgcgtctgtctgagagcgacccggaggagctcacctccgcaatcgacgcgtcgcagtggcgcgccccggaggccttcatcttccgcggcgacctggagaacaagacgccgctgaagacccacgtcgcgcacgacatctacccgagccagccgaacgtgcgctacgagggcttgttcttcaacccagaagccttcggcgccaacgagtgggacatggagcagttcggcccgttcgtcgtcgtcgtccgcaagtgaccgtaaagcgcgcaggacgtaagaaagtagagtgctgtaatcgtgacaatcgtcgaacctcgttctacccccgcaccccgcacgtcgcatggtcgcgcgcccggctccctggtgggcaccgccattgtctccggcatgctgtccttcctgctgctggtgctggtgccgctgctgccggtcaaccaggtgcagtcttcgctcgactggccgcagaacaactcgatccaggcggtcaacgcgccgctgatctcgctcgcgccgcaggaagttgagatcacggtcccggtcgccgcggttgaccacctgcgccccggcgagtctgtcatcctcggcactctgccggaatcctcccaagaggcgttcgaccgcggcctgttcatcaccgcccccggcggcgggctcgtggtctcctcgctcaacgaggtcgtcttcgagctcacccctgccgaggtgcaggcgcttcccgatgacgccaagctcgagttgcaccagacgcacgaggcgatgacggtgcgcatccccggcacctcccacaaggaagaggcggaggacgactaccgggcgcagttcacagggttctacaccgagctggatccggcctcggagcagttgcttatcgacgccggcctcgccgcccacatcgacatcaactcccgcttcacctccactccctccgcggtcaagatgttcgccatgatcgcgggcctgatctccgcgctcgcggggctttgggcgctggggcggttggacagcctcaaccgcaggtcaatcccgttcttcggcgagcagtggcgcaccttccgcccgctggacgccctcgtggtcgctgtgctgctgttctggcacgtcttcggcgcgaacacctcggacgacggattcctgctcaccatggcgcgggtagccaacgactcggactacatggccaactactaccgctggtacggcgtgcccgaggcccccttcggctccccgttctacgacacgttggcgctgttggccaaggtcagcaccgcctcgatgtggatgcgcctgcccacgctcatcgccgggctgttgacctggtggatcctgtccagggagattctgccgaagttgggggaggtcgtcgctaagcggcgcgtggcgtactggactgccgcgttcgtcttcctcgcgttctggctgccgtacaacaacggcacccgcccagagccgatcatcgcttgcggtatcgtcgtcacctgggccctgttcgagcgggcaatcgccaccgaccggctgctgccggcagcggtgggcacgatcaccgcagcactcacgttggcttgcggcccgacaggcttgagcgccgtgggcgtgttcttggtgtgcctgccggcggtgttccgcacgctgcgccggaagaaggctatcgccccagccaccgcgtttatcgctcccttcctgggcgccggcatggcggtcatggtgccggtgttcaaggaccaaacgctcgccgcggtgatcgaggcgacctcagtgcgagccgaggtcgggccggcgctgaactggtacgacgagtgggttcgctacgccacgctgttcgagcagacggtggacgcatcgatggagcgccgcttccccgtcttcgtcctgatcttctcgctggtgctgatcctggccggttttgccaagcacaaaaccatcccgggcacctcgagcgggccgaccaagcgcatggtgatcatcctcgcgctgtcgatgttcttcctcatgttcacaccgacgaagtggacccaccacttcggcatctacgcgggcctcggcggcgcggtggcggcgctcggcgcggtcgtgctctcccagttcgcgctgcagtcgaagcgcaaccgcaccttcgctatagcagccgcgctgtttttgatgtcgctcaccctcgccggctggaacggctggtggtacgtgtcctccttcggcgtgccgtggtgggaccgcaccgtgcagtacaaggcggtggaggcgaacaccatcatgctggcgctcaccctagtggtgctcttgatcggcatcttccagtcgttgagccacaacgccgggcgcgccgaggccgcacaactcggcgctgcggacgagttcgacgcccaagcgcgggtggacgccggccgctggtccggagtgatgggtgcgccgattgccgtcttggcggtactgatggtggcgttttcctgcctcacctttatcaaggcctttgtctcccaggcgccggcgtactcggtcggcatgggcaacgtgcgcaccttcaagggtgactcgtgcgcgctcgccagcgacgtgatgctggagcaggacaccaacgattccttcctcacccccgtcggcggtgtaccgctgggccgttcgctggacgccggcgagaacaccgggttcaccccggacggcgtgcccgcctacatcgcgtccgagaacgcgaacaccactgacgtaatcacctcggcgcagaccgacgcgcaagccgcagagcagcccgagaacgagactgccgacgaggcgcagtccacctcgcgcgtcaacacccagggcaaccgcccgtcgagcatgcgcggcgtcaacggctccacggtgcgcctgccgttcaacctggactaccagcgcatcccggttgccggcacgttcgaggacgatccgacgcacaaggccacgcttgaaaccgtgtggttcgagctgcccgaggcgaacccggacgcgccgcttctggtcgcctcggtggcgggccgcattgcccaccacgacatcaacggcgtcgagcaggaaggcaccgacttagcgctggagtacgggcagctgcttgccgacggcaccgttacctccctcggcgaacgcgagatgctggacccgggccccaccggccagtggcgcaacgtgaacgtgccggtcgcggacttgccggagaaggcgaacgtggtccgcctcgtcgccgaggacgcctccttctccgagcgggactggttggctgtcacaccgctgcgcaaccccaccctgaagcccatgaccgaggtcatcgactccgacaccccgggtcttctggactggacggtcgctttccagtacccctgccagcgcaccttcaaccactacgccggcgtgaccgagatcccgcagttccgcatcatgccggacgctcccggcaagcagcagctttccggcttccaggacttccttggcggcggagccttggctacagccgaagctgtcaactattcttacgacgttcccgggtacttgcggaatgactggcagcgcgactggggctcgatcgccaagtacgagctgcgcaccgattccacgggtgctgctcccgtcgaggcggatgttgactacacaacggtctcaaggtggggctggtggacacctggcccgatgaagatccgcaacccgaatgagtaggcccacatgaaacttgccaagcttgccgccgctgccgcagctgttgccgccgctttgtccgcagtcctcgccccggccgcgagcgcgcagaccatgcctgcgccgatcacctcgtcggacaacaccggtccgctgcttaaccagcagggctgcaagtcgcgttaccttattgcggtgccgggcggggcaaacacggttgccggtgtgccgacgttcttgccgcacggcggccaggtgctcaccaccggccttctggtccagggcgcgaccgccggccagacgcagccgctgtgggtgtcatacaactcgctggcgtttgccaaccgcccgtactacgcggcgtcggcagaggcgtacggggtgacgcgggggaccgtcgaaaagcttgcaaacgcctgcccgaacgccaagttcagcctcaccggctactcgctcggcgctgacgtggcagctcgcctgacgcgcgatatcgcgtacggaaacgggccggtcgccgccgaccgcatcgacggggtcgcgctgatcgccaacccgtaccaggggcacaacggggcgacgttgtcgccgggcacctcccccgattccgtcggcgcgctcggtgagctcgaaggcggctacggccagcttgcagaccgcgtgctggagatctgccgccccgacgacctggtgtgctccatgaaggaggcgcaccgcccgctggtcgcgcccgcgctgcgcacccacgtcagcgccggccgcattccgctgggcgagttccaggccatcttccgcaccctcggcaccgactccgtcagcgtcgtgaccggcatgggcgcccacggcggttactccaccttcgcgccgcagcaggcggcggactggattgtcgcccacgccaaccgctaagcactacgcgaagtggttagagttgggactcatgcatgacctcttcgcactagtcaacggcgcctgggtggaaaaccacgtcatccccgctgatcgcgggatcgacggctcgttttacgccctgcgcgacaaatccgaggcggacgtccacgagctgctgaaggaatccgacagccggggcggcgcgctctaccgctccttcatggacaccgaggcggtcaacgccgcgggcaccgccccactcgaggccgacttggccaagatcgcggccgcggacattgaggagttcgcccgcaacttgggcgagctggagcgcgccggcgtcggcgcgccgctgacctactgggtggagaaagattcccagggtgaaacggccgtcgcctacctctaccagtcgggcctggggttgccggacgaggcgtactaccgcgaggagcagcacgccgagacgcttgcggcctacgaaaagcacgtcgcccgcatgctcaccttcatcgacgcgaagtacctgatggggctcgacccggcggttgccgcgcgccgcatcgtcgcccacgagacgcagctggccgccagccactgggacgtggtgcgcgcccgcgacgcggttgccacctacaacccggtgcagctggatgagctgccggagatcatccaggtgatgcttggggcatcaggcttgtcgacggggcgcctcatcaaccaaatgccctcctacaccgacgcgctcgccgagatgctgcgcccggagacgctcgcggactggcagctgtgggcagtgtggaaggtcctgcgctcgcgcgccggcctgctcaccgaggagatctcgcgcgcgaacttcgagttctacggcacccgcctctccggcgccacggagcagcgcgaccgctggaagcgcggcgtgggcttggcggaatcgttggtgggcgaggagattggccgggagtatgtgggcaagcacttccccgcgccgcacaagagcgcgatgctcgagctggttgcctacttggtgcgggcgtaccgcgagcgcatcaccaaactgccctggatgagcgacggcacgaaggaccgggcgctggagaagctcgcgcagttcagcgcgaagatcggctacccggaccgctggcgcagcttcgaggggctcgaattttttgaaaacggcgccgatcttctggacaacgtgcgcgccggctccgcgttcgagcacgactaccaggtggcgaagatcggcaaacccgccgaccgcgacgagtgggtctccaccccgcagaccgtcaacgcgttctacaacccggtggtcaacgacatcaccttccccgccgctatcctgcagccgccgttcttcgatcccgaggccgacgccgcggagaatttcggcgcaatcggcgcggtgatcggccacgagatcggccacggtttcgacgaccagggctcgcgctacgacggtttgggcaacctgaactcctggtggaccgacgccgaccgcgccgcgttcgaggagctgaccgcgaagctggtcggccagttccaggacctggtgccgagcgtgctcgcgggcgaggaaggtgtcagcggcgtcaacggcgagttcactttgggcgagaacatcggcgatcttggcggcctcggcatcgcggtcgaagcgtacaagctctacctcgccgataacggcctggaagactgcgaggcgaagccgttcggcgacttggacggcacgttcaccgggttccagcgcctcttcttggcctgggcgcgggtgtggcgctccaaggcgcgccccgagatggcggcacagctgctcgcgatcgacccgcactcccccaacgagttccgctgcaacgtgatcgcttccaacgtcgacgagttctacgaggccttcgacgtggaagagggctccgcgatgtggatcgatccgcaggaccgggtgaagatttggtagcgggcgaggtttcgccgcagccgctgcgccagggcggccccgacgagcagtacccggaaaacgagcagctcggtgagcacttccaggtgggaggagtggagcgctcgcttcccgacgctctccagctcgaccagctggtcagctacatcgagtccacctacgactcgtctgccccgaactacctggcgctgttgcccgaccgcatcacgcacgcctcgatgctgatgctgggttcggccgtcgaccacacaatgcctggtgtcgcctacgccggcgctgtggacgtgcagacgagcgaatggggccaggtgttcgtcccgtctgagcccaccggcgcgtgggccgtgacgctctacgctgggccggacactgcccgcgactacgcgtggcgcccggacgtggctgccaccgcggaactttccggtgtgacgatcatcgacgtcgacaacccacttgacgcagctgctgtggaggcggcgttggcgcacgccgccgatgagtcaggtagcgcagcagctgtgtgggcgttcggcgagaccgccccgcttgtgccggaaggcgcgggcgcgtacgcgctgacgtttcccaccggcgtgccagcgcacgctcgccaaggcgcggtgctggtacaggtggcgacacgcgatgaggtggcaacaccgccggagatcagcggtgttgcggagtaccactccacccactacatcgccacgcccgccgagtcgcgccgcagggtgcgggacgtcgccgagttcctgcgcgctacgagcgctccttcttcttcggcgaatcgtcgacttccttgatgccgttgcgcacgtcaaccgtgttttggtaggcgttgccgtaggtcagcgccgaggccacccaggtgtcgccgccagttttgccccacgacacgctgccggtgccgctggtgcggtcgtcggtccagcccattttggagccctccgcgtcctcgatccgtgcggtgccgaagccctgaatgaacccgtccgcggccacgctgtcttggtgctccatgccgctgaacaggggtttggctaccgggtcccaaagaatctcggagataaacgtcgcgatgtcccgagcggacgtctgcgtcttgccccaccccccggcgcgcgcggttgaggtgaggtcgaaatcggaagcaatttcgtcgatcgcctcggggtacgcgcggtccagcttgccggcgatcgcgtcgttcgacgacgcgatcatcttctctacctggtccttctcctcgctcgtaccgtggtagagcacgtagtagcccaggtaaagcttggccagcgacagcgccgggcgcggctcctccccgtccgcggacatggagatccgcccgtcggggtggacgacggcaagcgcggtgcgctcccgcaggtaggaggggtccacgtggacggcctgcgcgggcgctgccccgctggtgatcacaagcgccgcggccgtggcggctgatagtgcggcggtgagtcgcttcatttcaggtccaggttcaggatggaatcggcctcgctgatctcctcgaactgcgggacctccacctcgcacaggtggcaaccagcgccgaccgcgtcttcgatgaacagcgcaacgccgaatgggctatccaccggctcggtgacgtaggtcgccccgaactgctgggtcagctgcagcgcgcgagccatgtcttccacgccgaagaaaatctgccagaacgccacgtcgggctcagcgccaatctccatgccgagaaacggtgcgccgtccttgaaggccacgtagtagttgccctcgttgcgcacttcccagtcgaacagttcgccgtaaaagtccaccgcggtagtgtctggcccgacgtactcgtaccagaccggcacaccgggctcgccggcggcgacgaagttgtcctcgcccgccggctgcatgaggccgaacaccgcgccgtgcgggtcggcgcacaccgtcagccgaccgagcgagacgtcttggctgctcagcacctggccgcccagcttctctacgcggttggcgtcaccgctcaggaagtacgggatccactcctgcagctgttcctcggcagcgacgatgccggcaaccggcaggccgtccttgcgcgctaggcggtactcgtcgcggctgacctcccagccgagcaccttggaatagaagtacgccgccttttgcggctcggtggtgatcaggtcttgccagtacggcatgccgggcacggcttcgaacgcgggcatttacatgttcctccacttttccgggtcgaaatcgtcgtcggcggtcgcctcgtcgaagtagtcgccgccgtcggtgtcggtgacgacggttgcttgggtgtcgccgatggcgaccagcgctgcgtcgtgaagcaaaaagcccctcgacgtgactacctcgccgttgaccgacacctcaccggcctcgatgagttctttggcgtgcccgccggattcaacgaggtttgccagtttgaggaactggccgagtttgatggaatcgccgctgatcggcacctcgagatgcatgccggttagtctaaatcagataggttgcggcgccagttgaagaccggttgaatccttacgtatgcactagcttgccgtgccggcgctgctcacggggctttgcgccgcggcgcttggcctcaccgggtgcgctcccgaccccgcgccggagccggccgccaccctcaccaccacagcggaacccgccgccgagccggtgcacttcaccatccgcaccgtgggcgacatcttgattcacagcgacgtctacaacactgccaaccgctacgccggcggcgagggctacgacttcgggccaatgttcgacgaggtgcgcgactacctgcagaacgccgacatcaccaccgggaacctggaggtcccggtcgccggcgccgagttcgggctctccggctaccccgcgttcaacgccccgccgcagatcgtggacgcgctgcaggacgcgggcgtcgacatcgtgaacaacgccaccaaccacacactggatcgcggtggggacggtgtggtggcgtcggtaagcaacctgcgtgagcgcggcatgctgtacgccggcgggtacgactcgtgggaggacaaggccaccccgcgcgtcatcgacgtcaacggggtgaaggtcggctttctcggctactcctatggcacgaacgggatcccggtgccggagggccgcgagtactcggtcgcgctcatcgacgacgcgatgccggacgagatcacggcgctcgacgacgacgtggatatgacggtggtgatgatccacatgggcgaggagtacgagccgctccccgtgcagttccagcgcgacacagcccagacggcggtcgacgcgggtgctgatctggtgctcggcggacacccgcacgtggtgcagccctttgaacttgtcgcaggcggcacgccggtgtggtggtcgcacggcaacttcctgcacgggcagtgggacgagcgcacgaaggtgggtggcatcggcgagttcgcgttcacccgaagtgctgacggcgctgtcaccctcgaccgcatccggtttatgcccacctacaccgtcggcccgccgatctcgtatgagcacaaggtgctgccgcttgtccgcgcccacgagtacatcgacgtcgccgccaccttcgccgagctgcgcgaacgcttagggccagacgtggagatcgtggaatacctggattaggtaaggccgctgtagaccatccacacaccgatcgccacgaagatgacaccggtgaccatgtcgatggcgtagccgtatcgctggatcggcgcggcgagcgcacgaaccgcgacggcaaagccggtgaaccacgcgagcccggtgacaatgagcgtgaccgcaatcgccaccatccactgccagcccatgtcgggccggacgaactgggcgaagatcgcgccgaagaacagcagcgccttcgggttggagaggttcgtcgccaccccgaggccgaacgcgcgggccggtgtgagggtgcgcgccggcggggcgggcggggtgtctccggcacccccggtgctgcctgcggtggtacgcactgcttcccggcgcgccgccaacccgccgcgcagcgccccgatgcccatgtaggtgaggtacgccccgccaacgacctgcagcacggcgagcacctgcggcgcggattgcacgagggcggacaagcccaaaagcgaggcggtgatccacacggtgttgcccagcgagatgccgagcgcgcacgcgatgccggctgcgcggtcgcgcgcaccgatacggatgatctggaacaagtccgggcccgggctcatgatcgcggcgaaccacacgccgagcagggcggcgaacgcagatgctgtcatggacgtaccgctacctttccgcctggtcggccggcatgatgctcagcgtgtcgatgttgacgtgcgccggcagcgacgccacccagcggatcgcctccgccacgtcctcggcgcttaagttcagcttgccctcgtagaccttggcggcgcgctcggcatccccggcgaaacggttgagcgagaagtccgtcttcacgcgccccgggtcgatctcgcaaacccggatgtcgggcgcctcctcgcggcggaaggcgcgcgtgagcccgcgcagaccgtgcttcgccgcgttgtagccgctgccgccggggtacgcgtcggtgcctgcgatcgaaccgatgttgatcaccagtcccttcgccgccttcagctgcgggtagagcgtctgcgtcacgcgcatcgtgccggccacgttcgtctcgtacatccactcccagtcggccgcgtcggcgtctttcaggtggtcgagctgcttcgccccacccgcgttgttgaccagcaggtccacgcgcggaagggctttcagcttatcgacgctcccctgatccaccacatccaacgcccacgcctgaccaccgatctcgtcggcgatcatctcgcagcgctcgattctgcgcgccgccacgatgacgtgccaaccgtccgccgccaacgcccggcacgcggcctcgccaatgccggcggagccgcccgtgaccacggccactttcttctcgttcacggtttcagaggttaccggagcacctggcgcatcgtgatgttgatccgcccatctttcaggccggtgccctccggcccggtgccgggcctcgcccccttcacgccgtggcgcgcccggcgcgcgggcccgccgaacacgagcgcatcgccggacatcaacagcaggtcgactggcccgtcggggccctcgatgcgaaacaccgtctcctccccgatggagaggctgaccacggcgttatcgctttcctcctccgcgtcgacgtgcaaccccatgccgtcgccaggcgggtagaagttcaccagcgcggtctccaccttcagtgtgaggcctatttgcttatcgacgccccgcgccacatccatcaccgcactcgccagcgcctggaagttctccggcaccggcgggaccgcgtagccgccaacctcctgcacgagccggtacggctgggtttgccagtaccagccgagcgagagcatccacgccttcatctgcccgctcgcgagcacgggcttgcgcatcgccaccggcgtgcccgcgacctgcctcgctatcccacgggcctgcgtaaccagcgccgcctgctgctccagcggcaggaagttcggcaggtgcactaccccagggatggggttggcggggtcgcgcgggagggcgtcgaaaagcatggctttaagcctattcccgcagctttccactagcctggcgggtcacgtcggaccaaggagaagctaatgcaccgaaaccgaaccatcgcggcagccttcgcggctgcatccttggtgctcgcgggttgcgcgggcaccgaaacgtctgcgacggcggcgccggaaacggtgacggaaacaacgtcggcgacgcagacccaggttgagaccaccacggcgacgacgaccgacacggtcaccgagagcccggccgccgatgccgcagccggcgggacccctgccgacggcggtgacgcgtaccgcgccttttccgcggtgctggaccacccgaaccagttcccgttcccgccgcagttccagcaggagaccaacggcacgtacgagtacgcggtcgtggacatcaccggcgacggcgcggacgaagtgctgctcaaggccaacaccgtgaatatcccatcgccggtgaaggtgctgtactgggacggctcggccgtgcaagcgaccgaggacgtgcttcttgatggccccggcggcgaagagggcgtgcgctacatggtgttcgttgacccctacaccacgggtcttaaccagtacgaggcgacgtcgacaacgctgacgcaccaggcgttcgtgcttgacggcggccgtttggtgcccacgacgcagccgcaggagacggtggccggcaactccttggagcaggagaatctggcggcctggcaatcgatcgcggaccgccaggcgctggccaacatgcggggctagctggcctgccggcgcgccggtccgcgcaggtagaacgtgtcgacgacctcgtacttcgggcctccggagcggccctggccaaggtgggattccatgaggtggacttcatcgacggtccagcgcggtccggagtagatggacagggcgtgggcgtggtcgtcgagaagccaaaagtccctggtgcgggtgccggtgcgtgcgacggtgaggtgcgcgcgctggcggccgcgcacgtcgggctcaatgagcgaatcagccatcagctccttcaagcccgccttgtcgccgccgacgccgatccacagggtgcggcggtcgaaacaaccggcgccgcgcagttgcagctccaatgaaggagcccaggccgtggcctgggctagaacgtcggtgacatacgctgcgtcgttcggctgcgaaccgtagaacgcgagcgtgatgtgccagttatccgggtcggtccaccgcgactcggtgccgaagccgtcccggatcggccgcagcgcggtgaccaggtgctcgcgaacctcgacgggtgggacgattgcagcgaacaggcgtctcatgcccctaaaggtaccttggatcgcaatgtttgacttggaacgaatcgggcgtggtttgcccgtcgcccgcgtgatcgaccagctgccgccacgcggcccggtggtggttgaggccccgcccggcacgggtaagaccacgctcgtgccgccggcggtggcgaacgcgcacggcaaaacgctggtgacggcgccacgcagggtggcggtgcgctccgcgcacaagcgcttggcgtcgatgagcgagcccgggcttgccggttacgccatccgcggggagcgcacccgcggctcgctggtcgagtttgtcacccccggcgtgctgctcaaccggttgctggcagaccccgggctggacggggtgaacgcggtggttatcgacgaggtccacgagcgccagctcgacaccgacttagtgctcgccatgtgcatggaagtggcgatcctccgggacgatttctacctcgcggcgatgtcggcgacgttggacgcctcggcggtggcggcgcacatgggtgcgtccgtggtgtccaccaccgcggaggcgcacccggttgcggtgagctacgcgccgcacccgggccggctggagtgcacccgcgagttctaccgccacgtggccgagcttgccgccgcaccgggcgcgcacggcgggcgcaccttggtcttcgtacccggcgtacgcgaggtggagctggtgtgccaggcgacgcccggcgcggtaccgctgcacggcaggctgaccagcgccgagcaggacgaagcgcttgacggcgacgcgccggtggtcgtggccaccgccgtcgccgaatcctcgctgacggtgccgggagtgcgccgcgtggtggacgcgggcctgtctcgtgagccgcgccgcgacgcgcgcgggatgaccggcctgattacggtctccgcgtcgaaggcgagcgccgatcagcgcgcgggccgcgcggggcgcctcggaccgggtgacgtggtgcgggcgtattcccaatccgattaccaacacttccgcgccgacatcgccccggagatcacaaccagcgacctgaccggcgcggcgctgactatcaacgcgtggggctctcccgacctgccgctgctcaccccgccgccggccgcggcgtacgcggaggccgaggacacgctcgccgccctcggcgcgctggatagaaacgacagcggctacgcaatcactccgctcggtgcccgcctggccgcgatgcccgtcgacccgcgcttgggcgctgcgctggtgcacctgggctctggcgcggcacccaccgtggccgcaattgcagaaggcgtaggcggcgatctcgcccgcgcgcaggcgccgaaacggcaggtcgagcgtcttgcgcggctcgcggatccgggtccagcggtggccgcgggcgaggtggtttcggccgcgttcccgcagtgggtggcgaaccgcaccggcgacgagtacctgttggccagcggcacgcgcgcgaagctcgacccggcgcttgctacccaggtgggcgcgcccgagtggttcgcggcagctgaggtgcagcgcacggcgaaaggcgcggtgatccgcgcgggtgcggccaccgtactgcccgccgagcgcgtggaggagacctaccgcgcaagcgttaccggcgacaaacttcaaggtcgcaaagtcaaagccgttggcgccatcgagctgagctccacgccggtgcgcctttccccggaccaggccatggcggcgctcgaggggttcgcgtttgagggcttcgtgcttgacgacgccgccttgcatctcaagcagcggctcgattttgtgcacggtgccgtcggcaagccgtggcccgatgtcgccgaaggcgactactcccccgagctgctgcaacttgctgagggggtgccgctgtccaagctggatatgcgcgcggcgctcatgcggaacttgccttggccggaggcggccgactttgacatgctggcgccggagcgcctgaaggtgccgagcgggtcgcgcccggtcattgactactccaccgggcggcccgtggtgcgggtgaagctgcaagaatgcttcggccttgccgcctcgcctgaaatcgccggggtgaaggtgctcttccacctgctgtcaccagccggcagggaactggccgtgacggacgacttggcaagtttctgggacggtccgtaccacgacgtgcgcaaggaaatgcgcggccgctacccgaaacacccgtggccagaagacccgtggagcgcaaaggcgacttcgaggaccaaacgccagctgttagattaatcagccatgacaactgcacagggcaggcacacagtgaccgtatgggcgctagtgtctctgattatcggctcgacggtgggctccggcatcttcgcgctgccgcaaaacatcggctccgtcgccgggcccggcgcgatgctcaccggttggctcattgccggcgtgggcatgctctccatcgcgttcgttttccagatcctggcgcagcgcaaaccgcacctcgactcgggcgtgtactcctacgtccgcgcgggactcggcgacttcatcgggttcacctccggtctcggctactggatgggttcggtgatggcgcaggttggctacgccacgctgttcttctcgacgctcggctattacttccccgtcttccgcaaccgctgggtgctcgccgtcgcggtctcggtgctgacgtggctgatcttcttcgcgctgacgcgcggcgtgaagcaagccgcggtgatgaacgtggtggtcacggtggccaaggcagtgccgattgtctgcttcatcgtgctggtggcgttcctcgggttctcctgggacacctttaccgcggacttctggggccgcgaatccgagttcaccttctctgagcagctgcagggcatcatgctctacaccgtgtgggtgttcatcggcatcgagggcgcctcggtgtactctaagcaggccagcaagcgcaccgacgtcggccgcgccaccatcatcggcttcctctcggtgctcgccctgctcgtcgccgtgtccaccttgagctacggcgtgctcacccaggaggagctcgcggcgctaccggacaactctatggcggcggtgctcgaggccgtggtcggcccgtggggcggtgtgttcatctcgatcgggctgtgcctgtcggtgctgggcgcgtacgtgtcttggcagatgctgtgcgccgagccgattgtgttgatggcgcgcgacggcctgctgcccgcccgcgtgggccgggtcaacgcggcaggcgcgccgtttaccgcgcagctgatctccacggtggtcattcagttctttgtcatcgtgttcttcgccaacgagacctcgtacaacgcgatggtgcagctggcgacgatcatgtacctgctgccgtacatcttctcctcgctgtatctcgtgctgctcgccctgcgtccggaaaaggacccgacgaagggtgaggtccgccccgacccgcgcaccaactcccgccagctggtcgtcgccgcgatcgccttcgtctactcactgtggctgatctacgctgcggaccccgtctacgtgctcttcggcgcactcgccgtgctgccgggcatggtgccctacatcctgaccaagcgctccaagggcgagcggctgttcaacaccttcgagtgggttgtggtcgcgcttgtcttcctcggctcgatccttgcggtcgctggcttggctaacgggtcgctggtgctggaataacgacgtgaaccgctggctcgttgtcgctcccctgtccgtggcgctggggtggttgctcagcgcggcgcacgtgccggcggcgtggatcctcggcgccatcatcgtctcgggatcggtggcgctcgtgtcggggcgcgaactgcgcctgccgaagcgcctgttcagcctcgcgcgcggcaccatcggcgtgctggcggcggtgccgctgatcggtatccccggacgcgagctggcgacgtttctcatccccggacttgcagccgccgcgttcacgatcgggctcgccttcgtcggtggcctcgtgctggccaaccacggggtttcccgtgaaaccggcgtgctgtcgctgctagccggcggcgcgtcggtgatgccggccatcgccgaagaggtcggcgcagatgtgcgctacgtggccttgtcgcagtacctgcgcctgctcacggtgtcgattacgctgccgctggtcgcctcactcatggcgcccggcagcgcggaggcctcgcctgcggctgctgcagaagcggtggcctcgccgtggatgtggttgctggtgcccgcgctcgttgtcaccggcatcccgctcggtaaagtcctgcacctacccaacgcgtctgtgttcggcccgatgctgctgacagtgctggtgggtacgctcgcggacttctccattaccccgccgatgccgctgacggtggcgtcgctcatcgcgatcggctggctcgccggcggagggctcgacattgacgcgttgaagcgcttcagccggatgcttccggcaacaatgctctacatcgtcgggctcatggccgcgtgcgcgggcgtgggctgggtgatgtcgaagtggctgggcatttccctctacgagggctacctggccaccacgcccggcgcgctggaaacggtcctggcgctgtccgcggaggggggcgccggcccagccgtgatcgcgctacagttgattcgcttgatctgcgtgctggtgttcgccgcgtacctgccgcggattctgagagcgctttagcggccgtggttgagcacttcggcggccagcatgtccatcggcattgagccgaggcgcagcgccttgtcgtggaagcgcttcagcgacatgccctgggcgagcgccttgtctcgcagggtgagccagtcgcggtagccgatcgcgtacgacggcgcctggcccggccagcccatgtagcggtccagctcgaaggtgaggttcgcctccatcatcgcggagttgtcgcgcagaaacgccttcgcgtactgcgcgtcccacacgcctgcgccgtccggaacggtcttgcgcaagtgcacgccgatatccaccatcacgcgggcgagccgcaggcggcgggagtcgagcaggcccatgcggtagcccgggtcgtcgaagtaaccgtgctcgcccatgaggtgctcggcgtaaagggcccaaccctcgccgtggccggagttccagcacatggagcggcgccacaggttgagatcgtggcgctgggtgagtgcagtgccgatctggaggtggtggccgggaatgccctcgtggaagacggtggtcagctcctgccacgtgtggaacacctcttggccttcgggcacggaccaccacatcgtgcctgggcgcagcatgtcgtccgacggagcggtgtagaagatgccgccggagccggcgcggtccaccgcgcactcgaccttgtgcaggtcttccggcacggtgaggtccttgccgtcgatctccgcgagcacctgctcgttgacgctgttcatccactccatcagcgcgtcggtgccgcgcagctgatagcgggggtcctcgttgagcttgcggtaggcgccgagcacgctcgtgtcggagccgtagagcttgtgggcgagctcgacctgctcgctcacagtcgcggccagttcctccttggcccacgagtaggcctcgtcgaggtcgatgctgcggccgaggaagaattcggagaagacctcgtagcggtcgcggcctaccccgtcgtcgtgggtggcctgcggggaaagctcggtggagagccagtcggcaaactcggcgaacgcctccttggcctcctcgaccaccttcgattccgcgggcaggccgaggtgttcgagctgcgagtcgtcgtcggcgagggcctcgcactggttgaccacgttgtctatttggcggtgggaggcgacgtcgccggtagcggcagcctccgcgagcgactcggcgtaaccgcgcagcgcgccgcgcacgtgcgacatgcgcgaggcgatgttgtcgaggtcttcttttgtcaccttcggcatcagctcgaaggagtcgcggatggtctgcaccggcgaatcgatgttgttcagccggcgaaggaactcgccgcggtggtgcagctcgagttccatcgtcacccggtcgcgcaggatggtggcggtgaggcggtcaacgtcatcgaagtcgtcctcgtcgtcggaggcgtccgtgcagtcgttgagcgcctcgacgtcttggatgacgtcgcgcatgcggtcagcgaccgtttcccagaactccgggctgaagttctgcagttctccgtcgtagccctccagcccgatctcggttgccaccgtcggcatcagtgcggccatgtcgtagacgaagttttcgcacgtagcgtcgagaagcgaaggctcgcgcaagggcgaggaagttgacgtcatggcatggcagtctatcccagcccccgaaatgacgggcagctgaactgcacggtctgccaggatgaacaggctgggcccggaaatggacaaagcggtctagaatgtggaagagtaattttatgcctttcctgcgcccgcaaactcccccggcgaagtgcctccacctcgtacgactcggcgagttgaccacgcgcagcgaactgatcgaggcaactgagctgtcccagcccaccatcacccgggccgtcggcgcgctgacccaggcgggctacgtcaccgagcggctcgacttagccaaatccgccggccgcggccgccccgttgtccccttggagcttgcggagacgccggccgtgcacgcaggcatttcaatcggcaccgactccacgtacattgcgctgttcgacatcaaggggcgcacgctgcgcagctcggacgtggatctgccggtggcgacgctgaaccaggacgacttcatccagcacgtgatggcggggctgcaccggcttaccgcagggttggaccgcccgctcgccaccgtgggggtcaccgcctcgggcacagtgactgacgacggctgcgttaccgcccccaacctcggctggaacaaggtgcccttcggcgagcagatgcgcgaacagttctccgtgcccgtgcaggtgacctcggtgagcgctgccattgtcggctccgagatgcagtcgagccgcaacctgaagatgccgaacgtgctcgccctgttcgccgacgactccatcgcctgcgccatcggcaccgacaccggcgtggagccgatcgacgtcgaccgcgacgacctcaccacgcgcgggttgctccagcagatcggcatcgacgagatccgcacgctgaacgacgcggtgacagactccgcgcaccgcgacaccacgcgcccggcgctggataggcgcgcgagggggcttggacagctcgtcggcaagctgtgcctcgagcactcgcccgcaaccgtggtcattgccggcagcgcgttccacgacgacccgctgtcgcacgtcccgttcgcgcaatcggtgcgcgagagcgccgccaaggacgcgtccaagctggacctgcgcatgctgcccggccaccgcgagatggtgcgcgacatcgcgcgcgctgcggcgctagacctcgtgctctgcgatcccctcgcggtggcggcgcgctaggtcgacatacgccgcggcgtggtccacacggtcagcgcgcgtggattcctcgagctcgcgcttgactgcggccggcacgcctgcggcaagtgaaaacgccggaatctcctggccctcgcgcaccacggaacctgcggcgatgacgctgcactggccgatcaccgaccggctcagcacggtagcggacatgccgaccagcgtgccgctgccgacctcgcaggagtgcagcatggccatgtggccgaccgtgacgtcttcgcccaacaccgtttccccgccggtgtcgacgtggaccacggtgccgtcctggatgttggagcgcgcgccgacgacgatgcgcccgacgtcgccacggagcacagcgcccggccagatgttgacgtcctcgcccagcacgacatcgccgatcaccgtcgcccccggggcgacgtaggcgctggggtggatctgcggagtcttgccttcgaagctgtaaatcatggtgcgattctaagcgttttaagacagctcggtacaccgtaagttgcgacataggtgccgcgttggtgtaggttaatcgcgaatattgattgtttctagaccgaattgtctataggagaactcatgcgacttcccaaatgggccacgagcttcggcgcccaggtgatcgcgggccttatcatcggcctcatcctcggcttcgtcgccgccggcatgcccgaagacaacgcgctggccgccacactcggctgggtgggcagcacctacgtcaagctgttgaagcttctgatcccgccgctggtcttcaccgcggtagtcacctcgatcgcgaacctgcgccaggtggccaacgccgcccgcctcgcggtgcagacgctggtgtggttcgccatcaccgcgttcttctccgtggtgatcggcattgtggtgggcctggtggtcaagccgggcgtcaactccaccgtcgacgccgccaacgccgcggacccttccagcaccggatcctggatgggcttcatcaactcggtggtcccggccaacatcctgggcctcggagcgaaggtgaacgacgccggcgccgtcaccttgaacttcaacgtgctgcagatcctggtgatctccctgctcctcggcatcgccgctgtgcgggtgggcaaggccgcagagccgttcatcaacgtctccgagtccctgctcaaagtcatccaggaagtgctgtggtgggtcatccgcctcgcaccgatcggcaccgccgcgctcatcggtaacgcggtggtgtcctacggctgggaagcgctcggatcgctgggcaagttcgtgttcgctatctacctgggcctcgcgctggtgatcttcggcctgtacccggtcgtgctggcgctcaacggcctctccgtcagcggcttcttcaagcgcgtgtggcctgtgaccacgctgggctttgtcacccgctcttccatgggtgtgatgccggtgacgcagcgcacaaccgaggaatccctcggcgtgccgcgcgagtacgcctcgtttgccatcccgctgggcgcgaccacgaagatggacggctgcgcctccatctacccggcaatcgccgcgatcttcgtcgcccagttctacggcgtgccgctgagcttcagcgactacgtgctcatcgcgattgtggcggtgctgggctccgccgccacggccggcaccaccggcgcgacggtgatgctcaccctcaccctctccacgctcggcctgccgctcgccggtgtcggcctgctgctggccgtcgacccgatcatcgacatgggccgcaccgcggtcaacgtcaccggccaagcgctggtcgccgctgtggtggcgaagcgcgagggcatcctgaaccaggacgtctgggacgccgccgaggacggcgtcgaccgcgcaccgcgcgaggagcgcgttaacgcataaactgctgcgcgacacccgccagcacgctgatcagcgtgatcaccgcgctgataatgctgatgatggtcttcacgtcggcagaggaaccggaaacgccggtgccaacggtgttgcccaagttgggcttggctggggcgcggaacggctgctcacccgtcggggtttcgccggaacgggccgggcggtagaggttcagttcctgtttgcctgccgggagggaagccccgcttgcagcggcggaggcggaaataccggcggtgtattcgtaaaaactgccgttcgcgtaaacgctgacgtgcccgaagccgaaggacctattcgctgggttgagcaggttgtgcaggtggccgttgcttagattccactcgccgccagcagattggagggcgcggagctcgccgtgcccccaggcctgcaaaattgcgccctccagatttctccccaacgcaagcgcttcaccgctagcgctcttgccgttaatggcggcaggaaccgcgcggtcgtgggtgagggagccgagcggctgctcagctgcgcgctgcaccgcaatgcgcgtcagatctgggtcgatctggaacgcgtttacgtacgcatccttggtggtcaaaccattcttacgggcgatgtcttgcaggcgggtgcctgtctcttcggagccgtagggcacatacgcggggttgatatcccacatttctgcgcggagtctacgaagagcaggaagaccgacggtctcggcatcgctgaagtcgaagcgggcgttgacggcaacggcgttcgagagcgacgtgccgagctcaaccccggtcacaggcgccggctcagcgttggcggcttgcagggggacgagggtgagggcggttgcggtcgccacggtcgcggcgagaagacgtgtgcgcctgggaaatgacatgtgggaagcgtacctcgcgccacacgtaccagcccatgaaaccgatcgggacgaccgtgaagagcaggttgggcaccacgaacagctcgtgcgaaacgttgtcggcggcgtacggcaacatgaatacaatcagcatgagcgggccccaccagcggtagatcacgcagccaaacagcacgatccacacccagtggtggtgccaggagaacgggctgaccaggcaggacgccatgccgatgagggaaacggcgagggggagctcggagcgcgataaagcgaaatgcgcccctgcggcagccagcagcgtcaccagcaccgtcagcaacaaccacagcggcgtggactcgatgcccagctctcgggagagcacctggcgcatcgcctgggcacccgggttgtcggcgtacccgacgcggtcggagttgaacatggactcggtccagaaccggcttgcgtctgtaacggagttgaaccccgtggcaacggtgcacaaaaacgtcaggcccgcgatgaacaccgcgccccagcggcgctgcagcgcaagcagcagaatgaagtacgcgggggtgagcttcatgcccgcggcaagcccgacgccgatgcctggcaggcggtaacgcggcagaaagtccaggcaaaccaaaagcatgaggaagatgttgatctggccgaagtagagcgttgcgtgcaccggctccgtcgcgagcacgaaaaacgctgtgagcagtaccgcgggcacgagggagcgggtaccccaccagcagatcagggacagggcggttatcgacgccaccgtccacgccacacccagctcgtgcgtcgcctcgccgaaccaggagaagaccacaccggcaaacggcgggtaggtaaacggtaggccgggcagcaggtcaccgctgtacagcggctggccgtgcgccaccttttgcccgccaagcaggtagacctgcaggtcggaaggcacatcgccgtgcgaaaggatggcccacacgctgtgcaggttgtccgcgttctcggcatagcgccaccaactgaacccgatcgccgcgatcagaatcagcgcgcttgcaaccggggccgccacggttacagccccagcccgtcgagaacgtcgtcgagggcggcgccgacgtcggcgcgccacaaggtgtccactttcgcgtcggcgcgccccgggccgccgttgatcaccgcaatcggcttgccctggcggcgggcgtcgaggacgaacttgtagccgctcatgaccgcgagcgacgtcccgaccgcgatgacggaggtggactcgtccagccacccgtccgccagcacccggcgtgccttcggcacgttctcgccgaagtacaccacgttcggcttgaggcgctcggatccgcacaccgggcagccgatcatgcggaagcgctccacgtcggcgtcgtcgagctccacgtcaccgtcggggttgaccgtcagcccgcgcttgttcacgttgccgaagaaggtggggttggcgtggtggaaggcggcgtcgataagcgagcgctcgtgcagcgcgccgcaatcgaggcagaccacctgctccatgtcgccgtgtagcgcgatgacgttcttcgcgcccgcctcggtgtgcaggccgtcgacgttttgggtgacgatgccgcggatcagcccggcgcgctccagctcgaccagcgcgaagtgggcgcggttgggctccgccgcgcgcatgaactggatgcccacgaacgcgcgcgcccagtagcggcgcacctggttcggcgagtgggcgaactcctggaacgtcatcgggcggcccttggtcaggcggccgttcttgctgcggtagtccgggatgcctgaggcggtggagacgcccgcgccggtgatcaccagggccttcgggttgcgcagctgctccacaacgcgcgcgagcgcctcctccggcggtgtcggctccgcggtctcgtgcaccacccgctcgatcgagcgcacggcgctcttgtgcgccatggcaatcgctgggtcggcgaattcggtgacgtcgaagcgctgcatcagcggaacggtacctcgccgatcgtgcggcgcagcttgcgggtgcgcagccggtcggggttcttggctaaccgctccatcgcgcgcacagcgcacatcacgtgcgcttcctttgagttggagtagaacgcctgggcgcctgccggcagcttgggcactgcgtggataggcaggtcggagacggccagaagcgtgccgtagggcacgcggtagcggtacccgttggcggcgacggtgcacgactccatgtccacggccgcggcggtggagccgcgcagccagtcccacagatcgcgcggggatttccattcccagttcctgtcgccggtgcttaagacggtgccggtgcgcatcagcgagctgtcctcaccgtagaccttggccacggccttttctagcgtgcgctggatctccggcacggccgggatcggctggtcggcgcggatgtggtcgtcgagcacgtggtcgtggcgctcgtaggcgttacccaagatgaggtcgccgatgcgcatgcgcgcgtccatgccggcgcagtggccgatcatgatccacgcctccgggcgcaccaccgcaaggcagtcggtgatcgtcttcgcgttggaggggcccaccccgatgttgatcatggtgatgccgtcaccgtccggggtgaccaagtcgtagcgcggcatctggaacttcgagccgagctcgagatcctccagcgccacggtgtcggagacggtctctccgctgggcagcaccaggcgggtgtagcgcgactcttcgcgtgacagctcgcgcacgccgaagcgcacaaactcggtcacgtgcatggcgtagttggtgaacaggatgtacttctgcaacgactccgggctgataccggtgtagtgctgcaagcgcgcaagtgcgagatcgaagcgctgcgggccgaagtggaacagcggcttctcgtcgccgtggaaggcgtcccagtggccgtccacgatcgcgtcgtccacctcgtccaaggacggtcgcgggataaacgagctgttggctgcgcgcacctcgcttaagtcgccgacgccggggatgtactcgggcgggatgcgcacgtccgagtaacccacctccacgtcgcactcgtagttggaggtcagcgcgtcgagctgcgcgcgcaggtagccggccatcaggtcggggcgcgacagcaccgcggagtacacgcccgcctcgtcgacgtagccgaagggctccgatcggttgatcgggtgccacgccttcacggtcacggaaagtttcgggtaacgcacggccgcgtactgctcgtactcgcccgattcgattgtgcggcgggcgaggtttaaggacgcgtcgtaaagcgcgataagctcctccactgtgtccatgaaaccaacactactgattccggcgcttgcggtctggggcctctgcgcgtgtgcggcggaccagccggagccggagccgctcgaggtggtgcgggaggcggaggcaaccccgggagtggacgcggccgcgctggaggcggccatcgcgcgcattgagcaggacactgacacgcgcatggggctttcgctttacgacggatccgtgcacaccacgctcggctccgtcgcctcgctgcccgcgtggtcgacggtgaagatccccatcgcgttcgcttcggagcagcactgcgagtacgacgaggactacctcgagcagctgatcacgtggtctattgagatctccgacaacgacgcgaccaacgaactgtgggcttgtctcaacgcggccggcggcgcggaagagctcgtgcgcgacgagatcggctcgcgggtggacgtggcgtggggccgcaccgcctggccgttcgcctcgcaggccgagtacgcgtacggcttgtcgcagcgcagcgacgtggagacgaacccggttatcaaccacatgcgccacatcgacgaggagcaaagctggggtctcggcgcactcggcatgccgttcaagggcggctggggcgacgtggaggccgacggctcgtggcagtcgcggcagatggccttcggcgagatcaacggcgtgacctacggcattgccgccggcgcgttgagcgaggagggctcgtttcaggccacgacggacgcgctcgacgagctggccgaggtgttggcgagcttctaggccagcagggtgcggcggacctcttccagccgtttgcccacttcctccggggcgagctcctcttggaacgccaggttgaacacgccctgcatcccagccgtgaggaagcgcgaagtggaggctgcgttgcgctcgttggcctcgctggtttcggtaccgtgctcctcgaagcgggtgaagaggtcggcggcgatcggctcctccatgatgttgatgacgaagcggttgagcagcccgcgaaccggcgagttcatcaggttactcaccgtttcccgccgctcgccgagagcgcggaagagcgcggccacgtgctcgccgagctcctcgtcggcggtgatgccgccgtgctcggtcaccgcagccgcgaatgcctcgtacgggtctttgaacacggccttgccagcggcgtagatcaccgcgtcgcggtcggcgaagtgctcgtagaacacctgccggctgacgttcgcttcctggacgatagcggtgaccgagatgtcgctggccccctgcttctccagcatcctgaccgtggcatcgacaagcgcgtggtgcgtgcggaccgctcgggggtcatcgctcaaaccgcggcgtgccatctccggctcctttcaaagcataagctcgttcgcatgacagcccctgactttagcgacgccgcgatcaaactactgaaagacctgatcaaaaatgcctgtgtaaacgacttgagttctgactcgggccaggaggtgcgaaacgccgacacgctggaggcgttcttcgcttccgcgccggacgtgaaggtgcagcgcttcgagccgcacccggggcgcacctctatcgcgttcacactggagggcaccgaccccggcgccgagccgctgaccctgctcggccacaccgacgtggtccccgtcgacggggcgaagtggacccgcgaccccttcggcgcggaggaggttgacggcaagatctacggccgcggcgcgaccgacatgctctacatcaccgctgcgatggcggcggcggtgcgcgacgtggcgcgaagcggcgcccgcccccgcggcaccctcacctttgtcggctgcgctgacgaggaggcccgcggcggcttgggcgcgggctggctggcggagcacgcaccagacgcgttctcgtggaagaactgtctgtccgaggagggcggctcacacctgccggtggccgacggcagcgacgcgcttgtggtggttgtcggcgagaagggcgctgcgcagcggcggttgacggtgcacggcgacgccggccacggctccaccccgtacgagcgcgacctcgccgtggcgaagatcgccgaggtggcccgccgcatcgccgccatcgagccccaagtgaccgacgacgagctgtggcgcggctacgtccgcgcgttccgcttcgaccccgagacggagcaggcgcttattggcggcgccgggtacgactccctcggcccactcgcccgctactcccacgcgatgagccacctgaccatctcccccaccgtgctgcgcgccggcggcgccatcaacgtgctgccgtccaccgcctggctggagatggactgccgcccgctgcccggccagacgcaagaggaaattgacgcattgcttaccgacgccctcggcgacatggccgacgacgtcgaaatcacccacctcatcaccgaagacggcaccgtctcccccacctcggggccgctgtacgacgccatcgtggacaccttcggcgagttcttccccggcgtgccggtcgtgccgacgattgccgctggcggctccgacctgcgtttcggccgtcgcaagggcggggtggggtacggcttcgccctgcaccagcgccaccagacgctcggcagcgtgctggacaacctgcacagccacgacgagtacgtggaggtcgaagacgtgcggctgaccgcgcaggcgtaccgctcgctgatccgccgttttgtgggcgcgtagtcactttcgtcacatccgtgacatactgggtggcatgacgatccgctcacgctccctgaccactgccgccaccgcggcgatcgccggcactttggtgctcgcgcccgccgcgcaggccgacttgatcgatgacgctctggcgaagcttcctgccggccagatcccctgcagccaggcctccaagtactggacgaacgaggcagactacaactccaaggtccgccaagcacagaccgtggcccgcttcgacagccgcggcccgcagatcctcgaggccctcggccgcgtggacgaggccgccaaccgctgcgggctgaagggcggcggcaacgcgccggcgcgccagaacccgcccgctcaaccggcccagcaggctcagcaggctcagcgccagaaccagcaggccgcgcagcaggcgccggcccagcaggaccggcaggctcagcaggcgcagcaggcgccggccccggcccagcaggcgccggccggccagcgcatccagctggcgccggcgggtgtgccgtcgttcgaggtgccggtgggcggtgtcggcaccgtcgtgctgccggacgtgctcacgctgctgcgccaagccctggccgagatcctcaacttcttcaacgtgaaggtgccgggcatcaactagagctctaccccagccattcgtactcgaccccgtctccggagtgcacgcgcaccccgggggcggggtcgagccacgcgtcgagcgtgagcgagtgttcgccctcgtcgccgcttgcaaacgcccgcaacgagatcgtctcgttggtcttatgggtgacctcgatatccgcgttggtcagccaggcgttgcggcgccgcatgctgatcagtttctggtgctccgcgaagatccagcggccgaggtcggagagctcctgaggatccgcgggcagcgcggggcgcacgctgtcgtcggcgctaaatccctcggtgcgaagcccctcgaaaccctgctcgtcgccgtagtagatcgacggcattccgggcacggtcatcaggatcgccagcgcgaggatctccttgtgctggcccaccttggaggcgatgcggtcaacgtcgtggttgccgataaacgtgttggcggtgacgcgggaagaaatttcgcgatggcggccgagggtgtggtcgagttcgaaaaagttggcgtcgttaagcgagctccaaatgcccttccacagctcgtactgcgtcaccgaatccagcgttcctgcttccgcgatggccgcgtaatcgccgtggatcacctcgccgaggaagaacgcgtccgggtggtcttcgcgcacgcggcccagcacgtcgcgccagaattccgccggcacagagtaagcgacgtcgaggcgccaacccacgatcccgcggtcgagccagtagctcatgatgtccgccaccgcctctttcacgcgctcgtcggagtggtggagtgtggccaactcgccgtggccctcccagtcggtgtcgccggcgagcccttccgcaacccacgggtgcgtgcgggcgacgtggttgaacacgccgtcgagcatgacgttgatgccgcgcttattgcactcggcgatcaagtggtcgaagtccgccaagtcgccgaggcgggagtcgatggcgtagtggtcgagggtgtcgtagccgtggccgacggactcaaagatcggaccgagcagcaacccgtttaagcccagctcgatcaggtagtccagccagtgctccaagtcccgcaggcggtggcccgcgtcatcggggtgctcgccgcggtccctgatcggggccccggtcgcgccgagcgggtacacatgccaccaaatgacgtgatcaagcatgcgcccgattatcgcacgggcccagagctctctgcgccctccgcatcttccccgccgttgttgcccagccggctcaacagcggctgcagcccggtggcaatgcgctcgcgcagccccttcgcctcttcctcgtagccctgctcaaaggggcgcctaccgcggtgggtgaaccgcaccttagtctcgccggaaccctcgtcgtcgacgaaatcgatgatcagcgacgtgtcgtcgccttccgtgcggtcctcgtcctcctcgccgtgcggctcgaggtgccacaccacgcggttgccggcgtcggtctcggagacggtcatggccgagtgctcctcgccgccctcgccccaccactcggacggctggctgattgcggagtacacgtcctcgcgcgcggcggggaaggagaacgacgtggtgaagtcccgaatcgcctcggcggaggtgccgtcggagaactcgtagcccgacagggtgccgtccgggtcgtagaaggccacgtccacgccgttgtcgcggtactgcttcaaaccctccttgatcaggttgcgcccggatttgttgaaagaagtcacccgtgatgcgtcgagcaccagccggccggcgatgtggtggcgctggaggtcgaagaggatcttctccgcagcgacgaagttgacgcgtccttgcagctccacaacggtgtcggtgccggagtgctcgatggagcgcacgcccggcgcgacatagaagttcgaggacaccaggtttaagccgagcttgccggagagctcgttgaagatcttcacgccgcgcacggagttgccctgttcatccagccgaggcgagagagaagcgatgcccatttgcgacgggatcgtgccgatcagcccgccagccacgcccgacttcgcggggatacccacgttgaccatccagcggccggacgcgtcgtacatgcctgcggaaatcatcacggcttgggtcacccggcacgcctcggcggtgaggatcttctcgccggtgatcggctgcgtgccgccgttggacagcgtcgccgccatcaccgcgaggtctttcacgttgaccagcaccgagcactgcttgatgtagctggccacagcttcgtgcgcctggtcggtgaccatgtccacctcgcgcaaaaggtgggcgatcgccatgttgcggtcggcgccggccatctcggaggcgtaaatctcctcgtcgatagccagttcgcggccggcgaggcgggagaagtagtcgcggatcttctccacccggtcgccgacctcgatgtcggggccgccgatgagctggttgacggtgatcgcgcccgcgttgatcagggggttggcgggcctgccgttcttgtccagcgacagctggttgaacccctccccgctcggctcgacgccgacgtacttgtgcacctcctccgcaccgtagatgtccagcgcgagcgcgtagacgaacggtttcgagatcgactggatggagaactcgtactcgtcgtcgccggcggagtagacgtgcccgtctgcggtgcacaaggcgagcgcgagcttgtccgagtccgcggtttggagtttctcgatgtagctggcgttctcgccgccgtcgtggtcgcggacgttatccaggatctcttcgaggtagtgctgcacgggcgaaagcatgcgcccgatcttacgggtgcaggtcgcccgatttcgggttgccggcgaagcaccacaggctcaaaaggcccatgcttgccgacgccaccgccaacaccaccatcacgcccccatatgcctccatgtaggtctgggtttcgagccagcgccccatcagcgagcccgtcacagcaaccgagagcagggcgccgagctcgtacgacacctcctcgacgccggcggccatgccggagcggtgcggcggcgctgccccgatgatcgcaatcgacgacacgctcatgatcgccccggcagacacacccatcaccgccaagccggcaaactgcgcgcccgccgcgagcagcagcgtgccagcggcggcgccgaagaacccgccggcgatcagcggcagaaaccccacgcggtgcaagttcgcgccgcccaaggctgaggccggaaaggcggccagcgccatcacgatgatgatgaggccggcttgaaggggcgacagggcgtcgacaagctgcagcttctgcgtcgtgttgagctcgacgccgatgagcacgaacatcgcccccgcggcggcgaccaccccgccgacaaaaaggcgggagcggaagatgtcgaaggtgagcagcggttctgtaaggaggcgctggcggcggccgaacagcgccccggcggtcaccgtgacggcgaccgcggcggcgagcagccaccaccagcgctccgccttcgctgcctccttcaccgcgatggtgaagcccgagagcgcgaccaggacgtacacggaggacaccgcgtcccagtgcttgtccgggttcgggacgttctccggcgcgagcagcagcgtcaggaccagcgcgacgacaacgatcgggacgttgatcaagaagatcgagccccaccagaacgcggagagcagcgccccgccgattaaggggccgaccgccgcgccgacgaccgcgaccgagctccagataccgatggcggtgttgcgctcctgctcgtcggcgaacgttaagcggatcagcgcgagggtggcgggcatcatggctgcggccccgacgccgagtgctgcgcgggcggcgaccagcgcccaggccgacggcgcgaacgccgcagccagcgaggctgcgccgaagaccgcgagcccgacaatgaacatcaggcggtggccgatcttgtcgccgagcgtgcctgcacccagcaacaggccggaaaggacaagcgggtaggcgttgataatccagagcgactccgcgggcgtggtgcccagctgccggttcaattccggcagggcggtgtagagaatcgagttgtccaggctgatcatgaacagcccgagcgagatcacggcgaaaaacgtccaccgctgggacttggaggtcggttcgaaactactcatggtgtgaactactcacggtgtgtatgcaaaatgccccgcatcgctgcggggcattcgttgtgcccggggggggacttgaacccccacgttcttgcgaacactggcacctgaagccagcgcgtctgccaattccgccacccgggcgggtggaacttgaccaatataaatcacggccgcgccaagctccaaatcccgtggtccgcgtcagtctttgtgcaggtagtccgggatgcgctcgaccgggataaccaccacatcatgcagctggtaatccatctcctgaagttgcttgcgcagctgaaccaggttggacagcgtcgctgcgctgtcgcccgcgggcacgacgaagatctcggcgtgcagcacgtggcccatgtcgcggaagcggccggccgcctggcgcacccacggctcgccttctgcagtgttgacggccttgtcgatggcgctgtgcttcttgccgtggatgtcagtcgggcgcgcgtctgttaacccgccgacggcgctgcgcaggttggacacaccgtcgtgaatgatcgacaccgacaccaccatcgcggtcgccgcgtccatccaccagaagccgtagcccacaccgaaaagaccgatgaccgttgccaccgccgtcatccagtctgccttgttcatgtccgcgtcggcgtacagcaccttgtccgggaaatcctcgacgaggcgcagcttcatccggccgaggatgacgggcccgagcgcggagacgaccatcacggccatcatcagccaccccagccaaatgctgcggccgaagaggaccacggtgccgatcggcggccggtcgcccgcaatcaggctcatggtgctgtcaatcagcaggtagacacccatggcgaacaaggcggtggcggcgactaagtggccaacgccgatggagcggtggtgtccgtacgggtgcttcgcgctcggctcgcggcggatctggcgcgcggcaatgaggaacgcgatcggcggcagcagctccaagatgtcttcgtaccaggcggtgcgcatcgcctgcgactgcccggccacgagacccaccagcgggatggtaaccaccttgaacattagcgtgatccactccaggcggaccgcctttttcatcagctcccgctgcttttcgggcagtgcctcgctgccgcggccggtgctggcctcagttttcgcgctcactagatctccccggttttcttgctcaagaaccgttcgagctccaccagcatcctgttctcaccgaggccgaccgccatgaccttcttgtcgtccttgccgtcggcgccggtgaccgtctcgtacgggcgggtgaacgccatcttgtcgtcccaaccggtgtcgtggcttaaccccccgatcactacgtccaagtcgtaattggacatcatctcggccagcacgctctccggagcgatgcggaagtcaacgtctgcgcccatctcctcggcgaactcgcgcacgaggtctgcttccgtgccactgacctcacccgtgagggagtcaacgaccgtccacggcgcgtgaggtgaaacaccgacgcgcaaggcgccgccggcggcctggttgtaggaatccgcggcgtcgcgcggcagggagctgcacccgccgagcgcgacgatgcaggcagcggctaaaacgccaggtaagagtcttttcatcggggtttcgctttcgttggccgccggtcgctcgcgcgcgggcagaactcatctgtccaccttggacacagtgcccgcaaatcgtagtccacgcctccggcgcaggcctttgagaccgcgttggcaggggctttcacgcttgtggcgtctaggttggtgtgaattgggcacttatactggctcgcatgtaatagcgaccccgcaaggaaaggaggtgtgcgggaaatgtccgtgatggaccggttagccaagttggacagctcgattcagcgcggcctggacaactccatggccgcagtcttcggcggcaaagttgtgccggcggagatcgaggagctgatcaagcaggaggcgcaggattccgtcgtggtcaccgaccaagacgagtttgtcgccccgaacgtctacgccgtcggcgtgtcgtcgaaagatctggaaaacctgtcccagcagcgcgaccttcccgtggacctcgccgagcagatcacgcggtttgtccgcaaccaagggtggttcctcgacggccccgccgtcgtgcggatcgccgaggagtctggtctgcgcaccgggcaactgcgggtgtcgtcgtacattgattccgtgcccgatgtggccagcggcttcgacgcaattttcgccgagccgcagtaccaggaggatgctatgtccgaaccaaatgttgaaccgatgaacgcggccgcgggaggcgcccagccgaccgtgagcttgctgctgcaggacgggtcgtcgaggacctacctcgtccacgaggggtcgaacatcctcggccgctctaacgacgcggacttccgcctgccggacacgggggtgtcacgccagcacgcggagatcacgtgggacggcgaggtggcggtgctggtggacctgcagtcgaccaacggcaccaccgtcaacgacgagccggttgagaactggatgctcgcggacggcgacgtgatcaccgtcggccactcgcacatcgaggtccgcatcgtcggcccgaacgctggccaaccggttggccagccggccgcgcagcagcccgagccgtacccgagcgacgctgccgcgtaccccggcaccgagtttttccgcgcctaggaaggattaaggcaagcacatggattccacggtgatcttgagcgcccgcttcgggctgctcgccctgctgtggctgttcattttgctcgtgctctgggtgcagcgccgcgacgtttcgcgggccgccggccaagtgcgcaagcagacggccgcgcaggcgccggtgaagcgggagaaaccgcgccacctcacggtggtggagggcccactcgtcggctcgcacatggagatcgccagcgtggaagacctcactatcgggcgcggccccgacaacgacttccagcttggggacgattttgcgtcctcgcgccacgcccggctcttccgccgcggcagcgagtggttcatcgaggacctcgattcgcgcaacggcacgtttgtgcagggcatgcgcatcgaccaaccggaacgggtgtccgttggcaccgacatcaaaatgggacgcacgattgtgaggcttgtgccctaaatggataccactaagaacttgcacctggatttcgtcgcgtcgtcggaccgcggcctggtgcgcggcaacaacgaggattccgcgtacgccggcccgcacttgatcgcgctggctgacggcatgggcggtcacgccgctggcgaggtcgcctcccagctgatgatcgagcacctcgagcacctggacaaggatccgaaagacgcggacctgctcgctctgctcggcgccgctgccgacgatgccaacgcggcgatcgcgcggtcggtgcgcgatcacccggagcaggaaggcatgggcaccacgctcacggcgctgatgttcaacggcgccgagttcggcctgatccacgtcggcgattcaaggggctatctgcttcgcgacggagcgctgacccaaatcaccgtcgacgacaccttcgtgcagtcgctggtggacgaaggcaagctaaacgccgaggacgtgtcctcgcatccgcagaaatccctgattctgaaggcgtacaccggccgccccgtagagccgcaccttgaaatggtcgaggcgcgcgagggcgaccgcttcctgttgtgctccgacgggttatccgacccggtgaccgcggagacgatcgcggtggcactcggccagggcaccacccaggacgcggcggaccgcctcatcgaactcgcgctgcgctccggcggcccggacaacatcacggttgttgtcgcagaggtgaagggaggaggcagcggggcgtcggcaagcaaccctgcccctgtgaaagccggtgccctagcgccgaacatcgaaccgacgcaccccgactcttctgccagccgggccgcggcgctgctgcgcaaatccgagacgatcgagccggaccacaaccgcgcgaagctgcagccttccgagggtgacggcagcgctgacgatgcggagggtcccctacaactaaccccgccgcagaccgagcgcaagcgcagcgcgtggccgtgggtgatcggcgcgctgctgctcgcgctaattctggtgttcgcgggcgtgatgtgggtgcagcagaaaacccctgacacctactcgctcacgaccgacgacgacggcgtgtttgtcatcgagcgcggcagcagctccaagcgcgaagcagtgcagaacgcctgcatcgacgcgaagaacacgctgcgcacccagccggtggactcgcagagcgactgccacctgttcaccgcctccgacctgccggaaagccagcagcaggcggccgaacggctgccaaccggcacctacgacgaggtgctggcgatgctcaacaggctcgccggcgaagcgctgcccgtctgcgtggacggcaagcaggacaagtgccgggaggtgaagtaaatgtcgcggatcttcggccgctcgaaggagctgtttttgctgctgtgctcggcaggccttttgctgctcatgctgtttagcctcgaactgagccagggccgcatactcaccgctgagctgctctacctcgtcggcggcttcatcttggtctacggcatcgcgcacgtggcgatcgggctgctcgccccgcacgcggaccaaacgatgctgccggtggtctcgctgctcaacgccatggggctggtcatgctgtaccgcctcggcttcgccgacggcgtgagcctagccaaccgccagatgatctggtcgctcgtcggcgtggtgctcatggtgttgaccttggctatcgtgcgcgaccacaaatccctgtcgcgctactcctacctgctgggcatcctggggctcatcctgctggcgctgccgctggtgtggccgcagccgccagaggtgaacgagcggatctggatctggatcggcccgttttctctccagcccggcgagttttccaagatcctgctgctgattttcttcgcccaactgctcacgcagaagcgcgcgctgttcaccgtggccggcaagcggttcatgggcctgactttcccccgcctgcgcgacctggctccgatcctgatcgtctgggctattgcgatcctgatcatggcggtctccgacgacttcggccccgccctgatcctgttcgccaccgtgctggccatgctgtacttcgccaccggccgcacctcgtggctgctcatcggcggcggtctcctcgccatcggcgggtacgcggtctacaccgtgagctcgaagattcaggaccgcgtggccaacttcctcgacccgctggcaaacttcgagagcttcggctaccagccctcccaggcgctgttcggcctgagctggggcgggctgaccggcacgggcttaggctacggccaccccgatctgatcccggtggcggaatccgactacatcctcgccgccctcggcgaggagctggggctcgtcggtgtggctgctgtgctcagcctgttcgcgatcctggtcacctgcgggttccgagcgtcgctccaggtgcgcgacacctacggcaagctgctcgctgcaggtctggccaccaccatcgcgatccaaatcttcgtggtcgccggcggcgtgtccgccatgctgcccatgacgggcctgaccaccccgttcatgtcggccggcggttcctccgtcatggctaactacatcctgctgggactgctgctgcgcgtgtccaactcagcgaaccgcccggctgagtacgacgagggcgtgatgcgcaaggcaccgggcagtgcgcgccgcgtgagcgcccagcctgcgggggtgggtgcgtaaatgaacaagtccatccgcgtgggcgcaaccttcgccctgatcatgatcatcgcgctgctggccaacttcaccgtggtgcagggcttccgcgaagacgagtacgcccaagacgcgcgcaactcccgcaacaccgtcgagctgcgccagatcaaccgcggccagatctacgccggcgggcaagtgctcgccgaatctcagcgcaccgaggacggtttctaccagcgcttctaccccaacatgccgttttccttcgcgccggttctgggctacgtctccgaccagtacggcaccgctcaactggaatccggctacaacgcagcgctaaccggcgacaccgccggcggctcctcccggttcttgcgcaccgggttggaagacgaccaggtgggcaacggcgtcgagctcaccatcgatccgggcctgcaggcgctggcgtacgacttgctctccgggcctgggtacgagggggcgattgcggcgctgcggccgtcatccggcgaaatcctggcgctggcgtccaccccgtcctacgacccgaacttgatctccaacccagccagcgccgagggcgcgtgggccgaggtgaacgacaacccgggcaggccgcttctaaaccacgccacgcaggaccagctgccgccggggtcgatcttcaagatcatcacaaccgccgccgggctgcgcgccggctacacgccggactctatgctcaccggcgaggccgtgactatcctcccgggtaccgagatcccgctgaccaactacggcggccaagtgtgcggtggcggtgggcaggtcaccctcgccaccgcgttcgcgctgtcctgcaacaccgcgttcgtgcagatgggtctggacgtcggcgcggacgcgatgcgcgaggcggccaccgccttcggcgtcggcgagcgctacgaccttggacttcccaccgccgccggctcgctcggcgacctgccgagcgcgccggaggtcgcccagtccgcgatcggccagcgcgacgtcaccatgacggcgctgcaagccgccgtcatgacaggcgtggtcgccaacggcggcgtacgcatgaacccgtacctggtgcggcgcgtgctgcgtccggacttgaccgaggcctccgcgaccgaaccgcgcgtgctcaacgaggcgatctcgccggaggaagccggcacgatcgcgcaactgatgttcggttccgagcgctggacctacggttacgacggcaacgggttcgcgtccaagaccggcaccgccgagcacgccgagggcgccgcgccgcacgtttggtacgtggcctttgacccggcgaaggacgtggccgtggcggttgtggtgaaaaacggcggcaacctgggcgccggtgccaccggcggccaggtgtcctccccgctcggccgtgcaatcctgcgggccgcgcccgcgcccgcaccgagcgaagaaccgaccggcgagcaggcaaactaggcaggcgaggtgaaccctatgaacactgagaaccgagacgacttgcagcaactgatcggacccgattaccagttgcagtgggtgatcggccacggcggtatgtccaccgtctggctcgcagacgatgcggtcaacgagcgcgaagtcgcgctgaagattctgcgcccggagtactccggcaacgaggagttcctcgcgcgcttccgcaacgaggcgcttgccgccgagggcattaactccccaaacgtggtggccacctacgactaccgcgaggtgcagacgcccgccgggttcaccatgtgcttcatcgccatggagtacatccgcggcgagagcctggccgacatgatcgcgcgcgagggccagctggaggaggacctggcgctcgacgtgctggagcaagccgcccacggtctcgccgtcatccaccgcatgggcctggtgcaccgcgacatcaagcccggcaacctcatgctgactcagaacgggcagatcaagatcaccgacttcggtatcgccaaggccgccgctgccgtgccgctgacgcgcacaggcatggtggtcggcaccgcccagtacgtctcgccggagcaggctcagggcctgagcgtgaccactgcctcagacgtgtactcgctgtccgtcgtcggctacgagatgctctccggcaaccggcctttcaccggcgactcctcggtgtccgtggcgctcgcgcacgtgaacaacgagccgccgccgctgccgatttccgtctccgcgccggcgcgcgagctgatcgagatcggactgcgcaagaaccccgaccagcgcttccgcgacggcaacgagatacagctggcgatccgccaggtgcgcgacggcgtgcgcccgacccagcccggcggccgaacccaggtgatcgcgacggaaccctcgccgagcgcttcaacgcagctgcttgccgacgtcgccgataaccgcaccacccgacccgcagggcagtacccgccctctgccacccgcgctgtccaagccagccgccagcagcaggccccggcgcgcccgcggccagcgcaacccgcacccgccccgatgcctgcccgcgccgcctccccgcgccccgcgcagccgaaaccggcagcggaaacgaagggctcggtagccggcccgatcatcgccaccctgctgctgcttgccttgatcggcggcggattggcgtgggcgtggacctccggcgccttcgacggcgttcgcaccccggcgccgaccacgccgccgaccacggtgacggagaccgagacggtggaggaggaaccggcgccgccgcccgagaccaccgttgtggagacggtgcgcgagacgccgacgcaggaagcgccgggcacgatcacgttcgaaccggagcccgaaacgcaggccccggcgcccgagccggagacaaccgtcccggagccgagcacgcccgcgacccagacccgcgccacgccgcaggacgcgccggtaacggcccaggacaacggtgggataaactctcccagtacgactgcagtcacgggaggtgactcttaaccacatgatgatcgctgaccgttacgagctcggggaggtcatcggcaccggcggcatgtccgacgtgtacgccgcgacagacaccacgctcggccgccaggtcgccgtgaagatgctgaaggccgacatggcccgcgacgagaacttccgcgagcgcttccgccaggaggcgaagaactcggcgcgcttgaaccaccccaacatcgtggcggtctacgacaccggctcgcagaacgtcgacgggctggaaatcccgttcatcgtgatggagcgggtagtcggccgcaatctgcgcgacatcgtccgcgcggacggtccgctcagcccaaccgaggccgcgagcttcctgcaacccgtcacgcgcgcgctgcagtccagccacgacgcaggcatcatccaccgggacatcaagccagcgaacatcatggtcaccaacaccggcgaggtgaaggtgatggacttcggcatcgcccgcgcgttggacgacgcgacgtctgcgatgacccaaacttccgcggtgatcggcactgcgcagtacctctcccccgagcaggcgcgcggcaaagccgccgatgcccgcagcgacgtctacgcgctgggctgcgtgatgtacgaggcggtgaccggccagccgccgttcgagggcgagtcgccgtttgccgtggcttaccagcacgtgcaggaggacccggttcccccgagcgagcgcatcgaggcgcaactcaacccgaacgaggccgtgaacatcgactcggtcatcctcaccgcgatggcgaagcacccggccgaccgctaccagagcgccgatgaaatgcgggctgacctggagcgccttgagcgcgggtcggtcaccgaggccgcgcgcaaccaccttgcggccgcggagagcgacatggacccggatgaaagcgcggaccgcaccgtggtcggcggcgagccggtgcccgccggcgagtccgtgcgcgtgcaacccgcccgcagcgattcgcgccacgacgcggtgcgctacaacaacgcccgcggcgccgaggcggaggcccagccgtcgcgctacgccgaccaccgccgcgcgaacgagaagacgaagtcgccgtcctggctcaagtggctcgccggcatcttgggcttggcgctgctcgccgcaaccggctggctcgcctacacctacttctcgcaggaagaggagactgtggcgcagcagcagatgatcgtcgtgcccgaggtggttaaccgcccgcggcaggaggtcatcggtgagcttgaggggctcggtttacgcacggttgtgtcggaagaacccaaccccgacatcccgcgcggcagcgtcatcggcaccaacccggcggtcggctccgagctgcccgcagggtcgttggtaaccgtgatcgtgtcctccggccgcgagctgacagacgtgccggatctgaccaacctcaacccgcaggaggcggtcgaggccctcgaacaggccggcctcgagctcaacgaggaaatccgccgcgagccctccgacacgatcgccgatgggatcatcatctcccagcaaccggcgcccggctcgcagctgtcgaagggttcgaaggtgatcgtcacggtctcctccggccgcgagaaggtcgaggtcccgtccttagttggcctgaacgtgaaccaggcaacggcaacgttgtcccagctcaacctgcgagccaccgtgacccgcgtcgactcggagcgccccgacggcgaggtcttggctgtcgccggcgcgaacaccgaggtggacaagggcaccaccgtggaactgcgcgtgagcaacaacatgctgatgaccatgccgcagatcacccgcatgaccccgaccgaggcggaccaggccctgcgcgagctggggtggaccggtcgccttgtggcgggtcccactgtgcccacgggcgcggccattgacgcgggcctgatcggccaccaggaaattgccgcgggcgacaccctgcgcaaggaccaggccgtgaactacaacgtgtggcagttcgacccggccgtgctcaatccactcaacaaccagtccaacgccgccggtgataggatgcagccgaacatctcgctgccggatcttcggctgaacttctagctggaaggaccctttcctcatgcctaaagcgaaagtaactaaggacgccgcccgcccggtctccaccacttcgtccggtgcgtcgcgcaccccggtcaagatcaacaccggcggcaccccgacctggtacaaggtcatcatgttcgggctgatgattctgggccttgcctggatcgtcgcgttctacatcttcggcgaccaagttgagttcctgcgcgagctcggcccgtggaactacggcatcggcttcgcgggcatgatcctcggcctgctgatgaccatgggctggcgctagcaccgcctgccacctgcccccggacactgggttcgggggctttttcatgtcaaactttctttccacagcctgtggataaacctgtgcacaaactccacaactcgataacatgttcaatcgaacacgtcgtgtactgcatgtttaggcgtgctcatcagatcaggttcgaaaaatcacgtccatgtgatttatccacttgtggacaactcctgtggaattagaagaccatcgtggacatcgggatcgtgggaacccacgccgcgactatcgctacagcaagacccgcccacgcggcgatccaccgggagcggttgcttgtcgacgtcaacggccacgccagcaacgcgccccacacaagcccgcccgcatgcccccaaaagctcacgttcgaggcgaggaaggtgtaggcaacgttgacgaggatgaggatgatgggggcgcggaggtcggcggagcgtcgataagcaattgctactaacaccgccatgagtgcgtacagcgcgcctgaggcacccgcggtgggcaccgcgaagttgaacgcgagcaccgacgccgaggaggcgaccacgaacgcgaggtacgccacggcgtaggggccggtgccgacgaagcgctcaatctcggagcccaccagcaccagcagcatcatgttgagaaacaggtgcgtgatgtcgaggtgcaagaacccggcggtgagaatacgcaggtaaccggggccgtcgacgtaggggccccaaaggatcatgttctccgcgatcggggaattccacaccacgtcggtgatcgaacgggcttggatcgcggtgacgatgaagacgaaggtgcacagcgcggtgaagagggctgttgccggggcgcccttgaactgttgtttcagcatgatctcctcagcatggcagaaaaaacgcccccgctgttggagcgggggcggcagtgccttggcggcgcgaggttagttgacctcaacggactcgatcacgacgtcctcgaccgggcggtccatgcggccggtctgcacgcctgcgatctcgtcaacaaccttgcgggatgcctcgtcggtgacctcaccgaagatggtgtggcggttgttcagccacggggtggcgtccacggtgatgaagaactgggagccgttcgtgcccgggccagcgttggccatagccagcaggtacgggcggtcgaaagagagctccgggtggaactcgtcggcgaactggaagcccgggccgccggtgccggtaccagtcgggtcaccaccctggatcatgaagcccgggatgatgcggtggaagatcgcaccgttgtagaacgggccctcgttgctgccggacgcgttctgcgtggagtactcgcgctcgccggtggccaggccggtaatggtctcgaccgtcttcggcgcgtggttgccgaacaggtcgaccacaatgtcgccgtggttcgtgtggaacgtcatcgtctgtgtcttctgagtcatgggttcaagcgtacgcgggttcactcgctcgggttgccggtggtggtcaaccacggggcaagtgagcggagagtgtgggtggattatgcgcggcataatttcgtcccacccgtctcagacgtcacaggtcccgaagagatccaccggggccattatgcgcggcataattgcgtcccacccgtcacgctcccaccagccacggccatgagagcactagggtcgtaaaaccccaggcgattatgcttcgcataattttgcaccacgagcaccacgtgtcacacgcccaggtcagcggccgtacgtggattatgcgcggcataatttcgtcccacccgtcacgctcgcaccagccacggccatgagagcactggatgtaaaaccccaggcgattatgcctcgcataatttcgcaccacgagcaccacgcgtcacacgcccaggtcaggggtcgaaagcagattatgcgcggcataatttcgtcccacctaccacaaccgttaaagggtcaggacggaatgagataaccccttcgttgcgaccgactctccacgagtcggctggctccgaaggggttcaactgcagcctggctcccgccttgttacagcccgccgacgacctcgtcgcgggcggcgaccaggttgcgcagcgacgggtcgacctcggcgtagccgcgggtcttcaagccgcagtccgggttcacccagaggcgctcggtcggcacgtgcttgagcgctgcgcgcagcaggccggcgatctcctcctggctcggcacgcgcggcgagtggatgtcccacacgccggggccgatctcggagtggaaggactcgtcgatgtcctcaagcagctccatcttggagcgggcggcctcgatggaggtcacgtccgcgtccagcgccgcgacggcgtcgatgatctggccgaactcggagtagcagaggtgggtgtggatctgggtctccgggttcgcctgcaaggagaccaggcggaaggcgcgcacggcccagtcgaggtaggcctggcggtcgtcggcacgcagcggcagcaactcgcgcagcgcgggctcgtcgatctggatgaccttgatgccggcctcctccaggtcgcggacctcgtcggcgagcgcgacaccgatctggtcggcggagacggacaacggaacgtcgtcacgcttgaagctccaggccaggatggtgaccgggccggtgagcatgcccttgactggcttgtcggacagggactgggcgtacttcgcccactccaccgtcatcggggccgggcgggagacatcgccaaccacgattggcgggcgggtgcagcgggaaccgtaggactggacccagccgttctcggtgaccacgaagccgtcgagcagctccgcgaagtactgcaccatgtcgttgcgctccgcctcgccgtggacgaggacgtcgaggccgatctcctcctgcagctcaatgacctgcttgatctcctgcttgagcgcctcggtgtactgctcgtcggtcaactcgccggccttgtggtcggcgcgcgccttacggatctccggggtctgcgggaaggagccgatcgtggtgatcggcagagccggcaggccgagcgcgtcgcgctggacctggttgcgctcggcgaactccggcgcacgctgcacgctgccctccggcagctcggcgacgcggttctgcacagcctcgttgtgggtgcgctcggactcggagcgggtgcgcacagcgcggtcggagcggctgaacgcctcggcagcctgctcctcgccggcgaccagcgcgaggatctcggcggtcttctcgtctgcgaacgagaaccagttcgcgacgtccaccgggatgttcttctcggcgcctagggtgtgcggcacgtgctgcagggaagtcgaggtggtcacggaaacgccctcgcccagcgaagccaggatctcggcctttgtgcgaaggtcggcggcccagacattgcggccgtcgataagacctgccaccagtgtggtcccggcagccttctcggcaacctgggtgcgcaccttctccacgtaatccgggtcggcgtcgagcgtccacggggagaggtcgacctggagcgcctccggggcgagctcgccgagcaccggcagggcctcgcgggcggcgccgtacggcgtggtcaggtacacgttcgggcggtccttctcgcccaagagctgggaccaggcctggcgcaggtaggacgcgatctcggcgtccggggtggacaggtctgcgaccacagccggctcggcgatctgcacccactccacgccggctgccttcagcgcgcggaagacctcggcgtaggcctccaccaggctcggcaaaagcgaccactcggccggcttggacagcgcaagcagcgtcaccgggccgacgaggtaggggcgcacagtgtggccagcttcgcgggcctcctccaccaggcgcacaatgcgctccggtgcaggcgcgatctcctggccctcagcgatctcgggcacgaggtagtggtagttggtgtcgaaccacttggtcatctccagcggcacgcgctcggcgttgccccgggccagcgcgaactcctcgtctaagtcggtgccgcccgcaaccagaccgacggtcagcgcggtctcgagcacctggtcgtagtaggccacgtcggcggggatggcgtaatcctcggtcaggccgaggtcgcgcaggtggttgtaggtgtcgatgcgcagtgcgcgggtggtggagcggaacgtctccgcgtcgatgcggcccgcccagtaggactcgagcgcgcgcttcagctcgcggtttgcgccgatgcgcgggtaaccctcgattgttgccttaggaaagttcatggttgtccttttcgtggatgccgatacgctggagcaggtcgcgcgtcacggcgaggttgttgtgtgtgtaaatgtgcaagcccccagtgcccgcatccagaatggtgcgcgcgagctcggcggacagttgcatgcccagctcgtactcttcttcgggggtttgagcggagctcagctgcttttcgacgcccaccggcacctccagccccgacaactgccccatccgccgcgccctttgaaggctggtgatcggcatgatgccgggaatgagcgggatgcggacacccgccatgcgggccacgtccacgaactcgaggaagtcgttggcgtcgaaaaacagctgcgtgatggcgaaatccgccccgagacgctgcttggccagcaggacgtctaagtcgtgatcgaagttcttgctctccgcgtgcccgctcgggtagcaggccaccgacagcgcgagtttgcccgcggcgaggtggaaggcctcctcctcctggatctcgttgatcaggttcagaagatccgtggcgtacggcaagtacccgtcgggcaggcgggattgccccggctggaggtctccccggagcgcgaggaaaccccgcacgccggcgtcgataagctgcctgatccaacgctccaactcggcgcgcgtgcctgcggtgcaggccaggtgcgcgatcggacgcaggtcggtggtgttggcgaggcgctggatcagcgcggaagtgccttccaaccagtcgctacgcatcgagctggtcaccgacacgtagtcggggtggtaggcggcgaggccgtcaatcagctcggtgagtttcgcctcgtccgcatcgtggcgcggcgggatcagctcaaagctgagcgccgtgcgggtgcggccgcggtgtcgcgccggtgcgccgttatgcgcttcgtcgtggctgtctaaaggtgccgaggcagacagccgcgtcgaagcagagttcccacgcatggaaatgcactgcctttcgatcttgatagggcggctggccgggctcggcacttacgcatcaaccgttttgcaacggtgcttgtgaaacttattgcggtggtttttcacccacaatgtacctctcggtctgtttgatgtttgtgcaggtagtgtcagttttgatcgtgaatataaaagggcgcggtggacagcttggtacggtcttgcacccgggactcggccgcgcggatttcggtacggttgggaagcgaatgtcaacgtggcacacaacacgaggagtgagacccatgaacccgatgatcaagctggcgctcaagggcgcgaccggcgcatacgcttactaccgcaactcgaaccgcaagcgcgagagcgacatctacgattcgctgctggacaacctacgcaagggcaacctgaacaacctgcacaaggacgccaacctggatgacctcgaggacgtgatcgacgctgcccgcctcgaggccggcgagattacccgcgacctgcacgacagcctcgaccgccggcgcgcggccttcgccgcggcagctccggaccgggaggcccggcgcaaggcgctgaagcaggacgcgaaggcccgcaagaaggagaactcctccggcggcgctgggaaggctatcggcgccgtgctgggcctcgccggtgctgcggccgctggctgggcagtgtgggagtactggctctcggacaagctggccgagaacgacaagaagacggtgaaaaccgtgaagactcagaccacgccggcggcgaagccggccggaagcaccaagctggtgtactccaccaccaccgaggacgcgggcaacgagatgcgcccgaaggccgacctcagcggctccgccggcccgctgggcgaggagccggccgtgcgcgacgaggagcttttgtcctccatcgacgagcagctgaccaccctcgacgcgctggacgacgatcagcgtgaggccaccacgccgcaccactcctccagctccagcgacgtgctgcacgacaccggctccggcaaccgcagcgacaaggtctccgacgccgacaccaccatcggcgcctccggccgccacgaactgcgcaaggacgccgaggacaagaactagaggttcgctgccgctgcctgccgccacgcggcgagcaggtggcggacgaggcgctggcgcacgtccgggaagagctcggtgaacttcgggtccatcgggcgggtcaccacgatcagctcggtcgctaactcgacggcggacagggacgggtccaccagcccgcagccggcggccttgtccagcaggacctcaatgtcggcgaaaaagcgcgtgcgcgtgtcgtcggcttcggccacggtaggcagctcgttcaccatctcggacacgagcatgcccaccccgtagtccaccagcgtccagacaaattcctcccacttagcggcggggtcttcgtcgaagccgtcgacggttgcggccagaaactcgctgaacaggtccatgaacccgagcgcgcacgcctgctgcaggtcggcgcgcgaggggaaatggcggtagagcgtcgcgatgccgacgccggcgtcggcggcaacgctctcaagcgtcaccagcgaggccggcctagtgcgaaactgcgccatcgcggcgtggacgatctgggatcgtttgaggcgggcgtcggcacgcaaaggatcctccttttgacaccgatcgaacgggcgacgatgatatcacctgttctaagtgatagctaaccctccatttggagtcaatatgaccgtgatacttactgcagacgagctggtggtgcgcgaaggcgcgaccccggtctcgctcgttgccgaggaggggctgaccatcctgcagacgaagcgcgagacgggcggctcactcatcgccatgtcgctcgccggcaggtacaaaccctattccggcactgttgacggccccggattcaagcgcaccgcgcttgccggggtcgagttcatcgacaaacttgagcgccaggtttccgcgcgcgaatcgatccgcgaacaggtggcctgggcgcagccgtttttggcccgcactccgaaagacatcatgagtcacaagcttgtccagccctggctcgagccgctgcggcttgaagatctggatgtggacaagccggttggcaagatcggcgtgatggaccgcttccgcctgcgcattatgctcggcctcgtcgcccggccaaacgccgagcttctagtggtcgacgacattgaccagctgaagaagatgagcctgcgccacgaaatcctgctcgacctgcaggaagtggcgaggcgtgtgcccgtgatcgcaacgaccgtgaatgaggaactatgagcggactgcatattggtacaaacttccggaagttcttccacggcaccctgccgcctttggcgctcatcgccatctcgcttctgccgctgctcttcggcggcctgttcgtgtggagctacttcgacccgctgggcaactttgacaagatcccggtcgccttggtcaactccgacgacggcgaggctggcgaccaggtggtcgatgagctcctagaacagtcgccgatggacttccacctggtcagcgccgatgaggctcgccagggtgtcgaagacggcacctactacctggccatggaaatcccctcggacttcaccgacgcggccacgagcgtgaactcggacgacccacgccaggcaaaaatcaacgtcacgctgaacgagacgaacggcttcatcccgaccatgctgggcaacatcgcctcctcccaggtggcggaggcggtttccagcaccgtcggcgcggaggtggtcgaccagctcttcgtcggcttcaacaccatcggcgagggcatggaccaagcggccgaaggagcagggaagcttcatgacggcgcctccaaggccaaagacggcggcgagcagctcgacgagggcgcaaccaagctcgacgacggcctgcaggagttcaactcccagctgcagaagatgccggacgcggcggcgaagctggacgacggcgtcggccgcctgcaggacggcgccaccaagctcagcgatggaatcaacaccgccgccgacggctcccaacagctcgcgtccggtctcggtgaactgcagtccggcaccgataccctcggcgagggcgcggcgaaggttgccggcggcgtggacaagatcaccggcgtggctggctctctaggcgaggcgcagcaggcgctcaacgacatcgacgccaacctggcgcaggtcatcgccgacctggacgcctcccccatcccgggcaccgaaatcatcgccgaccaggcccgcgccatccgcgtgcagatcaactccggcgcgctttccgccgtgaccggcaacgacctggtcagccagatgattcagctgcagcagggcgcacacgagatcgcgaaccagctgcagaaccccgaggcgaagtaccgctccggcgtggacaaggccgcggctgcgtcccagcagctcgccgccggtttggcgcagctccagggcggcaccggcaccctgatggccggcgtgacccagctcaaggacggcaccagccagctggtgattgcggcgaacacggcttccgacgcgtcgtccaagctggcctccggctccaaccagctggtggtggggctcggctcgcttaacgacggcctcgtccaactctccgacggcaccggtgagctttccatgaaactttccgacggcgccgagcaggcaccccgttgggagagcgaccgcctcgacaacgccgtcgaagcagcctcccgcccagtcgtggtcaaccaggtcggcgactccgtgaccttcttcggccgcggtctctccccgttcttcctggccctgtccctgtggttcggcggcctgatcatgttcatggtgctgccgccgctgtcgcgccgcgcgatcgactccggcacgccggccttccgcgccgcgttcaacacgctgatccccgcctacctcatcggtctggcccaggttgttgccctgtggattgtccaggtgttcgtcctcgacgtggagccggtgcacccaggctggttgttcctagtgctgatgatttcctcgtgggcgttcctcaccacaatcttcgccatcaacacgatctttggcgtctcggtaggccgcctcgtcaccatggcgatgatgtcgctgcagctcgtcgcgtccaacggtttgtacccgccggaggtgcagccggagttcatccagtggctgcaccgcctcgacccgatgacctacgtggtggatctgacccgtatcgcgctcttcggcacgacccccaccgatccgcgcatggcccgcgcgatcattgtgctggtctgcctcgcggtgggctcgtggctggtggccagcttcggcctcatccgcctgcgccagatccgcgagaaggacatccacccggagatctccgtgtaagttcttcaacctccctggctctggcctcgtgggcagctgctggtcaggcgcgatcccccgattgcgcttcccccggtgcagctgcccgcttttcttttcccccgggttcccccggtc

SEQ ID NO: 14 - DNA, 61905 bp, Corynebacterium cassirii
  source 1..61905: mol_type = genomic DNA
gtgggtgagcgctcaaccggtctcgggggggtggaccgtgggcgagaggacctacgtgaagcagtataagaccaaggcgcgtgggctgtctaccccaaacggcaacagagttttcccagttagttttgtcgacactacttaaatcgaagtgaactgatgaacgcgaaaagaacgccgagagctgccggttatcttttggtgaattgttcaattctcatggtgtcaacgtgctaacccaggcgcataatttcgccctgtgagtatcacagtcctcctcgtcctcatcatcgtcgttgcgctgttcttcgacttcactaacggtttccatgacactgccaacgcgatggccacctccattgccaccggcgccctcaagcccaaggttgcggttgccctggccggcatcctgaacttggtcggcgccttcctctccgtcgcggttgcgaagaccgtggcagaaggcatcgtcaagctcgacgtgttcgacctcaacgaccagctcgactccgagcgcctcctcctcgtggtcttcgccggcttggccggtggcatcatgtggaacctcttcacctggctcttcggcatcccgtcctcgtcctcccacgcgctgttcggtggcctcatcggcgccgcgatcgcttccatcggttggaacggcgtggtgtggaacggcgtgctggataagatcgtcctgccggctgtgttcgccccgttcgtagcgggcctcatcgcggccgtcggcacttggctcgtgtaccggattaccgccaatgcggagaagacccaccgcgacaactacttccgctggggccagatcggcaccgcctccctggtggcgctcgcgcacggtacgtccgacgcgcagaagaccatgggcgtgatcttccttgccatggtcgctgccggccagttcgatgccagccacccgatgccgttctggattcagctcgcctgcgcgctggccatcgccatcggcacctactccggcggcttccgcgtgatccgcacgctgggcaagggcctggttgagattcaccctccgcagggcatggctgcggagacctcctccgccgcgatcatcctcacgtcctcgcacctcgggatggcgctgtccaccacccacgtggctaccggctccatcctcggttccggcctgaccggccccgcgggtgaggtgcgctggaaggtcgccggccgcatggcgctggcctggatcaccaccttgccaattgctgccttcgtatccttcgtcacctggtggattgcgcacggcgtgtctgagctcggtggtgatccgctctggggcggtatcgcgcttgccgccatcatcgccatcggcggtggctacatgttccacaaggcgcgccagaagccggtgcacaaagacaacgtcaacgacgactgggaccacgagtccaactccgccgctaccaccggcaagacggccgactctcaggatgatgaggacgacaaccgcaccgacaccacgcggcgtggcggccgcaagagcaaccgcgtctacggcgagccggcagacttcgtcgacaccagcgcgggtctgacgcaccagcaccacaccggcggctccaccgcggtcaccgaaaacccgagccgctaacccagatcagattcgcgaaaaggaaatatcatggctgatctcattcaatcactactgctggtcaccggcgtgggcctgctgctcggcgccgggctgccaacgctgttctccctaagcattcacttcctttcccccggcgaggacggatccgtctccggcggccgcaaggccatcggctggattttcctggccatcgtgctcgttgccgttgtcgcagcactgctgctaatcgcacgcgagcgcatcgagtacttcaccggatgggacccgtaccccttcctctaaccaccagctcaccccatacgctgcgcaaagcagcaccaccgccgggccttcgggcccggctttcgctattcctggagaagggataatcgttggtgttgacaaacgattggcgtaaacctacagtgtccacaaagtgaacgggaggtaaacaaattcccgtttccgagaaaggaggtagctcatgaaggacattatgaacgccatccgtgagtggttccgcgttgacggtgagggtaccccctcgcccatcgacgtctccccgctcgcagtgctcccacgcacgaacggctaacgtttcacccgaacttcacccgcaggtcaccttctgggcaacctgcgggtttagcgtgctgtgatgaacccctcacttctctcacaggagccctgaaagccatgcccatgcgccgccggattgccactggcgtggtgctggcgctgacggctactaccgtcacgccgctgaccgcccacgccgctggtaacggggacctcgcgtcccgcttcaccctcgccgttctgcccgacactcagtactacgcccgctacggcaccgaagccgccggcaacatcttcgtcgatcgctacgggtccaacccatttcctagccagacgaacttcctcgctcagcacaaggacgagctgggcctagagtttgtcacccacctcggcgacgtggtggaccagccgaacgaccgcgccagctgggagatcagctcggcggccatgaaggtcctcgagcaggcgcggatcaactactccgtgctgccgggcaaccacgattacgccatgttcggcgaccgctccgccttcgacacctacttccccgaagaccgagctcgcgcgaacaccacgacgttccgcggccgcacccagtccactggcgtgcaccgcgctgcggactactccttccccggccagacggtggatagtgagtaccacatcttcgaggccgaaggtcaggagtacttggtgctcgcgctgggcttccgcgcgaaccaagacaccttgaagtgggcccagggcgtgatcaacgcgcaccccacgctgccggtcatcctcaccgcgcacgagatcacgggcatcgccggcgacggatccacgtactacaccaaggagtacggcgagtacctgtggaaagagctgatcaagaaaaacgaccagatcttcctcaccctcgccggccaccaccacggcgccggctaccacctgaccaccaatgacgccggccaccaggtcatcaacatcctgcacgattaccaaatgtcctacctcggcggcaacggcctgatgggccaactcgagttcgatctgagcaataacacgctcgagatgaccgcgtattcgccgtgggtgaaggagaaggaaaccgccaagctcacgcacttcgacaacctgctgctgaccggcaagaacgacgcgttttccatcccgctgaactacgcggagcgcttccgcggcttcaacccggagtggaccatcggcgacgaggacgacccgagctacaccgaagccctgctcaacacgctgaccaccggattcaccccgtaccaggttgaagaggcgcagcgcccgaccagcgccgaggactaccccaaggttgcaggcacggttgcgcattggcgcccgggggcacttttgcttgacgacgccgctccagtcccctccggctccaccatcccagacgtggcgggtgggtcggacatgacgcgcacccgccaccgcgcattcgcaggggccgacgccatcacctttgagaccgacacccacccgctgtcctccgataccggcgcgttgcgctgggccaagccgaggaccaacttcgctgtcgccttctttgaaaccgcggctggcgcaccggccaacaaggctaacttcgacaacggctacacgcttgaggccttcctcaagctggatcccgagttcaacggcgacgaaaacggctgggcgaacgcattgatccgtgatgcctctggcactgagcacggccagggccttgatcctgagccgattcaaatgctgggtgtttcctcgcttggtgagctgcgctggtactccctcggggacaacggccggggcttctccaactggtcccacgaagtgccgaagggcgagtgggtgcacgtcgcagtggtgaacgacccggctgaccagtccgtgcgcatgtacctcgacggcgcgccgattcttcgtgatggctacggccccgtcggcatggccggcaacggtgccaaatggatcctcggcacctccgccgccgccaagatcgaacaggaagggtggtttggctccatcggtgagatccgcatggtggaccaccccatcggccccgaccagtggctgactgcgcgtgccccgaaggaagacccggcggaaacgaccaccgcgaccgagaccacgacggttactgaaaccaccaccgcgactgaaactaccactgcgaccgagacggtgcgcgtaactgagccggtgaccgcaacggttgaggttaccgcgacgaagcacaccaccgtgccggtgacctcgacctccactgagacgagcaccgcgactgagaccgcaaccgttactgagaccgcgacggagacggcgcgcgtcaccgcgactgagaccgcaaccgttactgagaccgcgacggagacgagcaccgcgactgagaccgcaaccgttactgagaccgcgacggccacggagcgggtcaccgaaccggtcttggtgaccgccacggagaccgcgacggagacggcaacggagacagtgacggagaccgcgaccgtgaccacgacggtcaccacgactgaaccggtgccggcggtgaccgtgaccgaaacggccagggtcactgagacggcgaaggtgacagaaacggcgaaggtgacagaaacggcgcagccggttgagaagggcggatcgtcccagtccagcaccggctcgaccattctcggtgtgatccttggcgcgctcggagcattggtcgctgccatcgctgcgcttgaggcgatgtacccggaccttacagcgcagatgcgggagcgcgccgggctgtagaaaaagttgccggcataaatcgctctgggcttcctcgggttcctgatgcgtcgctacgaggtgccgatcgcgccgctgctgatcggtgtcatcctcggcccgcttgcagagaccgagttgcgccgcaccctcgccgtgtccgaagacgacgtcagcgcgctgttcgtcttcccgatcaccatcggcgtctacctaatgctgttcgctgcgatcgtcatcgcggtggtgcagcacttgcgcggcatgcgccgcgagcgggcgtcgtcaagcgaagctgaagctctagcttgacgacgcccacccgcccctttcaaacacgatgaagggggcggctacccaatattccaagcgtcgggcgcggatacgccgtagtcgacgccgagcacggcgaagtgtttgcgcgcggcgcggatcttcgctttttcggtctctctgagcttgtgctccaaattggtgctcttcgtttcacggatcaggtacagtctgtcctcgccttggactcgtttgatgatcgcccagtcagggttataaggaccgacaggcgtcggcaccttgaacttggggggaagcttcgtgaacaaccgaacgtctttgtcattgtccagtagttttgcgaagtccttctccacttgcgagtcagtgacaacgtagttgaagtccgacttctgcttgttctgcagttcgtagagcgtgtccaagaagaactgcttctcctccacgccgtccgcctgcagctcgcggagcgagtacacggagccaccaatcttctcgtactgcagcccgtcttcgaccaccctggcgagcacggattgaatcgcttcgtttgccatagcgataaatccgttcggattcttcgtgaactcggctaacctgcccgaaccgatcaagatgtcggcaatggtgcgccgcgtcagcgatgtcgactcctggagctgagcaatgatgtccggaagttcgaatgaatcctcaatgttcgttgagcgttgatccgtccgagtcccttctgttccgccccggttcacggtgacggttgccttcgtaacgttaacgcgcagaggagggatcgtaggtgcttgtttgatggcgtcgattgcttcggacaccagctggtttctatcgaaagcaacgctgtatgtggttcgttgagagattgtgtcccacatttccgcgaactggggatccaagtagacctctttattcagtttgcgcttgcgtcgcttccgcagaggcttgacctgggcggcaacagataccgcgcgcatggcatctataaccatgggttcaagacgctccaagtcaccgaggtgcagagagaagaagtcctcgtcgggagtaaatcgagatgtaatgaacccttcggcgtcaataaaaccactcgattgaagcatctgcctgatcccctgtgactccgcggctccgatggcgctacctgtggccgggtcgatgatcttggcgaattcctggggtcgaacaaatccgatttctacgcctgcacggatgtactcgtcctgtaaacccttggcaaagcgggtatagctctcgttcgcaaccaccgtcaactgagcgatcgaccggtcggagtaacggttaccttgttggtcaaccggcagacgcaatcctcgcccgagcgtctgacgccgttcagtttctccacccatctcacgcagggtgcaaatctggaaaacgttggggttatcccacccttctcggagtgctgagtgggagaagatgaagcgcaccggctcgtccagagaaagcaggcgctctttatctttcatgattaggtcgtatgcgcgtgaatcgtcgtcgctgttgccgtccttggaatctttggtgacgcccttttttgtcgaggcgaagtaagcgctgcgtgtctcgtctgggtctattgccacagacacaccgaaatcagggtttagcatcatttgacgctcaacttcagattggtagatctcgtcgaaccactgagcaaatggaccgttcgcggaggcgagtgaatcgccatcgcccatgtaactagcaaccttgtccacaaagaacaggctcaggaccttgatgcccgattcgcgaagactctcttctttctcaaggtgctcccgaatcgtttcgcggatcatgtcccggtagatggcttcggtgttgccaccgatctcctctccgacgagaaggcgaggatgatggctgagctcaactgcggctggttcgatgctcatcccggtaacgaaccaattgttcgagtaagcagggttatcggtgacctgctccaagttgcggtcctttttaacattgaccgccttcttaacaatgttcccgttcttgtcgcggacagctagttcaagtttcgccgtccaattcttaggattcacgtccaagagtttgatgtacggtgtggcttccaccccttcctgcacgacctcggcaacgacgatttgcttcaccagttccaggttgtgtgcatctaccgggtcgagttggtaaacaaggttgcggcgtttccggtgagtagcggaataccgaagaattgcggagtagttgagctttccaatcgacgcctcggagagatctgattccatgttctgcggctcatccaaaatgacgaacggtcgtacggctcggagatagtcgactggtgccaggccaccgagttcctctcggctttggtggaaaatgcggttgtttttcgttcccttaatcgccgccaccgtcatgatcatgatttgaatagaggtgccggtggcaaaaccgtgcacttgcccggggttgtcgccggagtatacaaagtgactgaacggctgtgtcgggtacagctctcggaaatgagcgcgcataagctcgatgctcttgttcacaccctcgcggatggcgacgctgggcaccaggatcacgaactttttgaagtcgtacttctccgccaactcgaaaatggtgcgtaagtacacgtaagtcttaccggtgccagtctccatttcaacgtcaaactgcagaccgtccaccagttgatcgctcaccatcagttggttctgctcttggacacgctggagattgtccaaaatcgtgtcctcaccaaggaacagatggtttccgacggcaccaatttccaaactcagctcctgctggcctacaccgatgtccagactttgttgatctgtctcgaaactgagaaacccacggaggatttctcgaaattgacctacgtctttcggctggccttcgaaaagatcgacaacggaactaattgcgtccagctgatattgctgacggctgtcaaacttgaacttcatcagctacatccccttatgcggtcttcagctcgatgtcgtgggtggcgcacatctgcttcaaattggttttgagctggtcgtcaccggcaaaagcgtcttcgagaaccaccagacgtccgggccgcagttcggttaatgcgcgcagctgttccagagatggctttacgtgctcgttgacgtacgcaatcagcacgtatttgttttccagttcggcatccggagcgtcattgataactgcatggcagcccagaccggctgcttcaatttcggagagtgtctcggtaagagacatgccctgcttcagaagtagctcggtgagtattgcgtcttgcctagcggtgtccttggtagattcccgaacattgagaatctgttgctcggcactcttaatagatgtatctgctctcagatcccacttcacgaaattcgtgtcggccagtttatatgctcgaaagccaatgtctagaggagtggttctattggctgggttcgccgcacaaaattccgcaattctctctccagaaactgcgattctgttcctagcaagatcggaaatcgtacgaaaacccgcctgacgggctgagctattctctggcgtcggttcgggtagctgaacttgaatgtgctggcgactgccgccatctctggcgttgagatccattacagcctgagccgttgagccagaaccagaaaagaagtcgaggactattgagtcaggtgcagttaggagccggcacagctcgataagaaattccggattcttcggcgattcgaacggtagctccatgccggagggctttttcataaccagtagatctgtccagttggaagacctcaacttatccgcagcaggagagatccaatgttctacaccggaatttttgcctttacggctgtcgccgcggcggatgaattccaaagtcttgccagttgtggcccagtattcctccaatgtcattttgtctgcgtaggaagtctcgtacgtctgataattatcaaccgctcgctgggcgcgagcggactcccacttccactgcccagtctccggtgtgaatccaagaaggtcatagcgcatgctcgggcggtccggtgaattccagaaccccttccagtagcccttttcagctctatcgcggtctttgagttctgttcgaattgggtttagcgatgcatgcagttgcttcgcgtagattaggcagtactcgacgcctacgttcaacgatcgcaatccgcgttccacgaactgattgttcaggtttttgtcttgccgacgcacagtcaaaatattaactaggttagcttcgccaaaaacgctgtcgcagagtagccggagattggctagctcttcgtcgctgattgagatagcaataaacccatcgtcggagaggaggttgcgtgctagcttcaggcgaggaaacatcatgttaagccagtttgtgtggagccgaccaccggtctcggtgttgcttgaaagcttctgaccttcctcattaacctgctttgaccacgagaggtagttctcaaggccctctcggtagttgtccgggtaaacgaagtctttgcctgtgttgtaaggcggatcgatgtagatcatcttgatcttgccgtggtagtgcttctgcaagatcttcaaaacttcgaggttgtcgccctcgatgaacacattctgggttgtgtcccagtctttggagttttcgaaatcgggtgcgagagtggcgctagtcggggtctgagcggctcgcattgcgcgctttttccctggccagaacaagccgaatcgctcagaagtgtcggaagcgtccccgtccagcagttccttcagggtctcgatatcgatcttgccgtcagcaactgcctcgggggcgagctttgccagctcggtagctaatgcagtgcgaaagtcaggggaccacggttcgattcgggtttcatcaaagtcgaaatcactcatgcaaatgaggttgccacatgcatgcgacaagcgtggtttatctttcgcacattgaggcgagcgacatctacggttccactcgccaacgcactgagaacaaatcctccacgtgttctgtgccaccgagagcctgctctacggcttccaagtaatcgacagatcgggcatgaagggtgcggcgttcgcgcgcgaagtcgtcctcagcgtcgtaaatcttctgctgaatttggttcgacttcttcttaaaccgcaaggattctgtcggatcatcggtgtttcgagctcgctttctcagatctttcagttcagcttcaagcttggcgacctgctggttgaactcagcttgacggtcttctcggttgcgttggaccgcatcctcctgctcgttgtagaacttcgcattccgagcttgaacgtccttgtggtgggattccgactgtttgtccagatcggcttccaggatgcctaggtccaccggctcacagtcttcaatcgacaccacagtgagatccattaagttgccaatgtcctcggcgttgagcttcctacggcgactggtgagcccagcgcagagcaaataagactctgtgacgtcttgagaccctgcccgcatctcgaacgtcactttccgcactgctagttggccatgttggcctacgagctccgcagctactccaccgactcgatgagaagcaccaaggctgaaaacgagttccttggtgggggtgtactcgcttagcgcctgcccaacaacgtattggcccagtggtccggcataacgatattgatgggcgccaggcacctgctccttgaaggcgtaacggccagatggagcatcgggcaccggtgagtgttccaacgtgaaggtgttcgaagaatcgtcaaacactgcgtccgaacgcagttcgtattgagtgagggccaggaacaggcgctcgaactggttaagcgttaccgttgactgttcgtcgtggctacgaaggcggtcttgcacctgcgggtcaagattgtcgaagactttcgaacgaaccttcttcatttccgacgaaatctcggcggaaaactttttctccagctcgtcgaacgcggcgttgatctcgtcttcagttctgcactgcttcaggatgtgtgcgatctcttgctcaagatcaacgccgtcttcaatggaaccgagcacttcgtcgctggcaccgaacaccgaggtaaacagctgaaacttttcggtgagtaattcaaggattcgccgctctgcggtgtttcccttgttcgaaaagttggccacaaccacgttgaatttttggccgaagcggtggacgcggccgatgcgctgctctactcgttgcgggttccaaggcaggtcgtagttgatcaacatcgagcagaactgaaggttcacgccttctgctgcggcttcggtggcaatcatgatggttccttcatcgcggaagtaatccactagggccttgcgtcggtcggcggctgcgatgccggttacagcatcaccgccttcgttcttctctagccaggctttgtagatagcggaggcttctggggatgtattcgtcccgttgaacaagacgaggccgtctccccaccccgtgtctcggaggtgctgggcgaggtactcctgcgtgactgtggagtccgtgaaaatgatggctttctccggtgctccaatttcccgaagggttgcgaaaccgcgttcaagagcctcgttgagatggacggccttctggttcactttgatagagcgggcgagagctgcgaagttgcggagatctcggatctccgcctcgatcttgctactaacgacgggatcggcgtagttaagccggtcatcatcaaatgtgtcgctttccatgcgttccagctcgtcgctggtgaaatccgcatcggcttccggcgcgagcacaaaaccgcctctgcctcggcgcattcctgtggtgagttcatcttgcaggcgatctgccaccgactcgagcgtgctcgcgattgcgtatgtcgaagaaccgaggcgcttgcgaagaatcatcgccgataggtgcatttgggacttattgaaggcgtagatcttatcgcgttgcaggtaggcgtcgataagcgaatgaagctccaactcctccggtgacgggtcgaactccacggtgatcggcatgcgttgcgtgaaacgaacgtacttttctgcattgcggcgcagcgtgcgcttcgcgattggggctactcgatccgggagatcctcggtgctccctttcacgtagcgttctttgaaggcgtcgagcgagtggaagtactcgtcatcgaagattgaaactagcccgtagagttcttcgaggcggttttgcaagggggtcgcggtcagcatcagcattttagaggacctatttgcaatcttcgagatggcagttgggactttgccccctttccagtagttacgcagccggtgagcttcatcagctaccagcaggtcccagctgcgctcaaggcgagcttcgttccgggccgcgaactcgtacgagcagatcagcacagtctgcttttggtttggggcgccgatgaacgcatctgctgtcttggaatcaagcagttctgcggggatcatgaacttttcccacagctcttgcttccattgctggcgaaggctggcaggggcaatgatcaatatgctgcggcgtcgctgcgaccagtactgggatatgacgatgcccgcttcgatggtcttgccgagcccgacctcatctgccaagatgacgcccttctgaaaaggtgagttcaacgcgaaaagtgctgcgtcaatttggtgtggcttgggctcaacctgtgcgtcgaacagtaagcccgccagcttccccacatggtcattggcgtgggagcgttcgagttcgttggcgaagaacttcgcttggtgcggggtgaggtgagcgccgtagttgttcaccccgtttaccttgccatagctgtccgagaagcagggctccggtcgaaccccctgcttcccttacgcagcaagtaactggttattacgacacttcactcgagttctgggtgtcgggggaaggcgcatctggcaacaatagagatagctccatgcgctctcggatagaatggtcaaaatttgattggtgaagatagccattcggaaacgtatcgagattacgaatttggtgcttggttgtgaatgaatcgggcagctccctaataagtcctgcgtacgaagcgcggtcaaactgcgccacttcgcgatgttggggtacctctggagcaaaatcgtaatacaggaataatgctgggaggcgacttgccaaatcagttggatagaaatccctctcgcagaggtgttcaaccagctcagcggttaaattgtagcgcattacaaatatgatgtcgggataagcttgtattgtttcactctcatcctttgaggtaagaaactcgctgatagatcgaaacgtgcggcgtccgaagaacttagcccaactgtcaccgcctgctcctcggtccacggccatcgagatgaaggatcgtaattcgcggactgagggctcgggtacggcgtccaaagcgtcagcgatacggtcttcaaagtgggcttctgctgggacatgcaggaggaggtctgcaatccaatccaacagtttgaagtacggatcgaatatcccatcacccgacgcctgaagctgcggcaaagctgctatcagggtcttcgccacattgaaacattctaccggggtgaggtcgggggtttccctgcccttcgtaatcgctaagctagccaccctctgattctcgaatagtagctgcatcaggccttgtgattcaccgcccgctgattgccgcagggccgcccgcaccttctcatccggaacatctccctgcggtacatgaccgacgaagtagcggtcaaagtagtcgacgtgggcgatagagcgacgtggagcgctcgatccgtgaaatcccctgcggtctgaaaaggagattgaagggaacaatgctacgaggatcttttggacttccaccttgtcttgctcatcaactccttctgccacgctggcagcggataacgtatccctcgaataacttgaggttaacctcgtccgatagttcgaatcgccagagatcagttgcatcttgagaccccacaggcggtcgtagagatctggggataccgtttggatgacggtgagcagaaaaaggtcaccggccaaaacttcgtccaaaggaatcagatcggaatgaattgataaccgactcttaaatcgtttcaggcgccttggtgtgcgaagcaggtgaactacagctccctgtgttagttgtaggttcgttcgaaggtcatccgtatcgaaggcctggtgatgagagagccactctgctagagaacgttcgacctggtactcgtttagcggcggaatcggaaacgaaacctgaacgaatttttccaaatacgcttcggcttggctcgttcgctggctgtctaaagttgcattcaatgtgtttctgataacccctggatcgaataccaaaaggtagtgaacatcacggatccttccaagcagccgggccaccttcaggacgtttacgagatctgggcccggtaagcgatccaagtcatcgatgattacgagtatctgcgtgtggtgcttttgaatttctgtctgtatgtcggacagtaaattttcccagttgcggctctctactcgcttactcatgaggtcggagacaccggacgagagatcccccaccgcgccgggtattaacgaagtgtagctagtggtctttaccagccactcacttagtaattgctttatgtgtccgtcttgtgtccgaggtattgcaccgataattgtttgggagaactcaactaacatagcgtcggagctgctggtcgcccaaggtgtaaaagtaactacggaccacggataactgtctttgctgtgcaattctcgaacaagcagctgggccactgacgtcttgccaacaccccaagcgccagtgatcgcaaaaaccgtactttccgcgtctttcggtattttttttattgcatggcctatgcgccgtgcataagccgcgtaaccgtacttatcctcttcgcttgacttaattgctgtgtcatcccaggattcgctcatccgacaacctaccttaatcgcttcaagtggcctacttccgcccctgcttcagcttcgggttgacgcatgccaacaaccctacatttcaagtaccttattcggccattggctcaatcgcgcatgacttccccacccacgagactcaagtgcggagccgtgctagcgggagcgctcgctgctctgcgtcgccgcagcgcgcgcccgcgacgcgttggtgatcaccacggttggtgagcgctcagagctcctgccggaggggtaacagagctgggcggatcgtacgcaccgattcgctagattttcgctgctcccatcgccgcgtttttgctaaaacggattgaacgcaccgaattgggcggtaatgcggtaaggtcctctctacttaccggatattcggtgcgatcgctccggtgcctagggcgccagctgtagagaggagtggctcatgaaagtcgaggagatcggggctttcgtgcgcgccaagcgcaaagagcgcagactgacccagcttgaagtcgcggagcttgcagatgtgtcggaccggttcctgagggaattggagcacggaaagccatcggcggagattggcaaggtgatcgatgtactggctgttcttggctttgacctcgaacctgtcgtgcataggagtgacccgctatgacctcgcagggtattgccgctgacgtatacgtaggagacgagctcgtcggtcacttctacaaacgtgtggatgggctcaccgagttcgattaccttgacggtgtcaccaccccagtggccacgacgttgccgcttagcggagctccttacaccactgcggccggtgcactcccaccgttctttaccaacctcctgccggagggtaggcgtctttccacattgaagcgcactgtaaaggcctcccttgatgacgagcttgcacttttgctcgccgtaggctccagcacggttggcgatgtcagcgtcgtaccgcacggtcagaggccgaagcaccccatggcctcaattgatttgtccggcgcattggatttctcggcagctcttaacgccgcaggtatcgcagacccgatcgctgttcccggcgtccaagacaaggcttctgcccgcacgatcgcggctccggttcgcaaccgtaacgcggagtacatcctcaaagtttccccacccgagtaccctaagctcgtcgaaaatgaagccgaatgcttcagcattgccggtgccgcaaagttcccgctcacagaaacgcagttgctaaccgacgcctttgggcgccccggactcctcatcacacgcttcgatcgagtgggcggcaaacgcctccacgttgaagatgcggcgcaggttatgggcttgtaccccagtgcaaagtacgacccggcgatggaggatgtggccggagcgttgatgggcgtgagctcgtcacaaagcttgaccgcacgatcaatcgcgttccaagtcgctctcgcctggctgactgggaacggtgacctgcacgctaaaaacatgtcgttgatctggcgcaatggcggcgtggagatggcgccgatatacgacataccctcgacggtgccttacggcgactccacgatggcgctatcggtgcaaggatggaaagacaatattagcggcaaggcgtttcgggctttttgtggcgaaatcggattgggcgagcgcgtggccgagcgtgtgatggggcaagttctgcaattgacggagggagcagctgaacgaatcatcgcagcggcagacttcgacccgcgccgtgcacgcgatctcaggagggttctggcgagtcggagaagggcgtggggttaaggcagaaggtggcgctccgtcacagcggctcgaaggattcctcgcggctcaggagtaagcgatcttttgctttccgaacagacagacaaagttagaagcataagtttggtagtctcaggaatatgacgtggccgaaagctggcgtggagaccctcccttggtcccctgctcccgagatggtctcccggcgggctgcgcgcaatgccccgcgggagtaccaggcctcagttgtgcccttcatcgccgatgagtcgctggagctcgcggatgaaactcgtgcactcgtcgagcaagcgacagtggagatagtgcgtttcgatgccaccgacgcccatcgtctcatcccgtttacgccgctactgctgcgcagcgaatccgccgcgtcgagccggattgagcagctcacatcgtccgcgcggaaagtgctcgaggcagaggtaaccggaaagggtaaaggtaacgctgcgctgatcgctgccaacactcgccaaatggagcaagccgtcgaacgggcccgcgcaagtgtggacggcattgtcgacatgcatcgcattcttctcgcggaatcggcgccggacatcgcgggcaagctgcggaaacagcaggtctggatcggcggcagcgacttttctcccgcgggggcggtgttcgtaccgccaggggctgcgagcgtggagaagcttatggcggatctggggcgattcatgcagcgcacggacattcccgcgctcgcgcacgcggccgtggcgcacgcgcagttcgaaacgatccacccgttcgcggacggcaatggccgaactgggcgtgcactagtccatgtgatgttgaaggaacgctgcttaacaaggagctccgccctccccatctcagccggtctcctcaccgattccgccgggtattttgcggcacttgacgcgtatcgcgacggcgacgtggagcaaatcgtgcagctgttcgcccgtgccgctattgaggcgtccgagagaggcgcgcggttggcgaaggagctggaggcgctgcgcattgaatgggacggcatcctcaccgcccgtgcagacgcgctcgcttggcgcgtcctcgacctcctacagcaacggccggtattgaccacaaacgctgtctctaccgagtttggcgtttcggcggagacagcccgcaatgcgcttgaacgattggagcaggacgggatcgtagtgtctgcgcagctggacaaacgccagcgcgcgtggcgctcccccgacgttctcgaagtgctggacgaattcgctgaaatgagcggacgtcgggtgtgacgctcgcgctgttccttgcatgccacaggagactcaaatgcaggttgaaagcacagttgacgccaccgaaacccacatccctgcctctctatgatccagtagagcgcgatgttcagttagacgaaattgacgctgctgggcatcgtaggatctcggtggtaatccctcataggatgtgaaatgtgcatcggaaagcaacgggaagaaggggtcatcagtggcgctgcagggcaatcagatcgacgcaaaagaaatcaacgtaggaaggttgctcgccagcggcgactacgagttcgtcatccctgagtaccagaggccatacgcctggggagttgaggaaactttacagctgctgtctgatcttgtcggtgcgctagaccgggacacagatgagccctacttccttggatcgattgtcctagttaaagagcccggatctccgcgctccgaggtcattgacgggcagcaacgcctcaccacactgaccatccttctcgcggtaatgagagatttggtgaaggatgaggagcttcaggcatccatccatcagctcattgagaagcctgcggttgtgtgggcgagcgaagcggcgagcccaaggttgcgcatccggccgcgggaccagaagtttttcgcaacgcacatccaaactgctggcggaaccgagaagctggtaagtctcagcgagaactcactcgatactgatcctcagcgaggtattcgcgataacgcgatcgcgcttcggaaagagttggaaacgtgggacgagggccagcttcaagcgctcttcgttctcgtggcgcaacgggcgtttttggttacggtggcaacccccgatctcaacagcgcttatcggatcttttctgtcatgaacgcccgcggcctgcctctgtccccccaggacatctttaaatcgcaggtaatcggcgccactcccgaaggacaaaaggacgcctacgcaaacgtctgggaatcgcttgaggagaatcttggccgcgatgagtttggggacctgttcctctacattcgcgcgatcaagtctcgtacgcgcgcagtcaagggtctgctccaagagtttccggatcaggtattaaatgcttaccttccggataacggcatccgcttcattgaagaagtgctggagccctatgcacgtgccgacatccgccttttagcccaagatttccacggtgaggacccccgctggcaggaactgaatggctggttgaagcggttgagccagctcgacaacgacgattggcgtcctcccgctctgtgggcactcaaggagcacggtgacgatgtagcgttcctgatcgcttttttcgagaaactggagcgcctcgccgcgagcatgttattgcgaagggtgtacgccacaccgcgccagcagcggtacatggagttgttaaaacagctgactgacggcgacgggttggattccccagcgttccaactttcggattgggaacggtccgaaacactgaagcagatcgacggcgatctctacctgcttaccagggttcggaagtacgtcttgctccgattggattcggttctagctaatgacccaggagcgtcctacgaccaccgaatcatcacagtggagcatgttcttccacagcagccgccggctgacagcgagtgggcgcgcacattttctccggagcagatggaacgttggacccatcgcttgggcaatcttcttctgctgaataggcgctccaactcccgagctcagaactacgacttcggcgttaaaaaagataagtacttcgcgtcaggcgacggcgttgcggttttcgcactcactacccaggtgttaggtgagcgggagtggacaccggagaccatcgctaggaggcagaacactctagtagagctactggctaaagagtgggatctgaagtagcgagggggggagaagttcctaacagggaactctcctaccaacgcgatgaggttgcgcgggtggcgtccgctaaggcagcctacttcgccgcgttcgcccaagcgccgttcgggttgtacgggctgaaccagccgtagatgcccatgaatgccaccaggagcactaggacggcgatgacctcgccggcttcgctgctggagttcgaggtatccgtgttcgtagcgagcgtggtgacgtgctgggtggtcggtgccggcgcggcgctagcttcgggagcaacggcgacggtggtcagggccaaggcgcctgcggtaatggtgcttgcgagtttctgcttcatgggtctgattttgcactatcgccctgtggcgcgcgcgacgcaaaccctagacgctagaccgcggtgtagccgccgtcgacgaggtggtgggagccggtgatgaagctggcgtcgtcggaaagcaaaaatgcaaccaagttggcaacatcctccggccggccgaggcgaccaatcgggtgcaggtctgcaagtttctgctgctgctcggcggagtagcgctcgaacatgtgggttttgatgtagccggggccgaccgagttgacccgaatgttgtgttcggcgtagtcggcaccgagtgccttggtcagcccgatgacgccgtgcttggcggcggtatacgcatccaggccgcccttgcgcgccacggtgccgtggatggaggacatgttcacgatcgcccgcggggtgtcgtcgccttgggcgaggaattgcttgagttggtagtggcacccgtacgccacgccgtggaggttcaagttgaccagggaatcccagtcatccagatccttctccgcgaggggagcgcggttgtcgccccggcccgcgttgttgaacgcgaggtggagtgcgccgaaggtgtcgaccgcgaacttcaccgcgttctcgttgccctcgcggctcgaggcgtcgagctcgaacgcggcggcctgtgcgccgctcgcggtgagctcgtcgcccgctgccttggcggcgtcgaggtcgaggtcagcgatgacgacgctggcgccctcagcagcaagcttggttgcggttgctttgccaatgccggaggcgccgccggtgacgagggcgacgcgtccttcgaaacggttgctcatggccccaggctaactcctacactggccgcatgcgtgtcgtggatttcaacgaggcaatcgcaacgcttaagcccgcggaggcggtcgaggcgatccgccgacccctgctcgcaggtttcgacccggcaaccgatccgcaccggcagaaagtggccctcccccacggtgagatgcatctgctcccctcggcactcgacggcgcggtgggcgtcaaagtgctcggcatccagccgccgggctccaccgagcaggtgccgcttgtccaaggctcgtatgtgcttatggatggtcgcacgctcacgccagagatgcttatcgacgccgccgccctcaccaccctccgcacgcccgccgtctccgtcgcaggggtcctagagcggctccgcgcctccacggacgtcctcgaggtggccattttcggcacaggtgcccaggcccgcgcccacgccgagaccctcaccgacacccttcgcggtatccgcgaggtgcgctgcactttcatctcccggcacgaccccgtggctcccgcagtttcaaaggcagagctcgtggtcaccgctacctcttcgctcgagccgatcctcgacgcggagcatttgctaaccgacgccaccgtcatttccgtcggcgcccacaccaccactacccgcgaactgcacgaggacgtgctcgtcggtgcccaagtcgtagtggaagacctcggggccgccaagcgcgaggcgggggacgtcgtgatcgctgtcgaaaagggggcgctgtcctgggacgacgtgcttccgatgcgtgatgtggtgcgcggtgacgtcaccctcgacccggaccgtcgcgtcgtgttcaaaactgtcggcatgccgtgggaggacctggctgtggcgggggcgttggcgcatgcaagcaaaagcaggccctaaaccacggcacaatggagtcatggcctgcacagttttgtactcctccttttacggctcaacccagcagtacgcggaagccttagcggcgcgcctgggcaccacagcgaagcagctcgagcaaggcgttccgctaagcggcccgaccgtcatcctcgcgccagcgcacggcccgatgcatgacggggtgaagtacctgaagggcctcgacgccgctactgtccaacacacgcccgtcgcgctggtcacggtgggaatgacgcttgatagtgaagtggccaaggcagacgccgccggtcagctcctcggcccgcttgcggcacacgttgagcgtttctacctgcccggccgcatgaactattccgagctttccactcagcacaagacggtcatgaagggcctgatcaccgcgttgcggatgaagccgggcaagagcgccaacgagcgcaacatgatcgacacgtacggcaaagacgtcgaccgggtggatgtgtcccggctggacccgattgtggagtgggttggggcgcaataggcgcgcagaaagatatcgaaagatatcggaacaattagctgacctgcataaacaggtcaaaaacttcggtttgggggcgctatatcttcgctatatctttccggtatctttcgcgatccgcctacgcctgccgtgtagtgggcacctattacactggctaaccatgactaacgcgagcgaccacggccccgcccaccgctacaccgcggagttggccggcgacatcgagcagaagtggcaggccttttggcgcgacaacggcacgttcaacgcgccgaaccccaccggcgacctcgccaccggtgacccgctgccgacagaaaagctgaacatccaggacatgttcccgtacccatccggtgctggcctgcacgtcggccacccgctgggttacatcgcaacggacgtatttgcgcgctacaaccgcatgctgggcaagaacgtcctgcacaccctcggctacgacgcgttcggtctgccggctgagcagtacgccatccaaaccggcacccacccgcgcaccactaccgaggcgaacattgagaacatgacccgccagctcaaccagctgggcctgggccacgacaagcgtcgcgcagtcgccaccacggatccggagttctaccgctggacgcagtggatcttcctgcagatctacaactcctggttcgacgaggagttgcaaaaggcccgcccgatcgaggacctggtgcgcgacctgatgacaggtgtgcgccagaccaaggacggccgcgacttcaaggacttgaacacagaggagaagtacgcggcgctggatgagttccgcttggtctacctctccgactccatggtcaactggtgcccgggtcttggcacggtgctggctaatgaggaggtcaccgcggacggcaagtccgagcgcggcaacttccccgtgtaccgcaagcggctgcgccagtggatgatgcgcatcaccgcatactcggaccgcctgctggatgacctggatcttctggattggccggagaaggtcaagtccatgcagcgcaactggatcggccgctcccgcggcgcgcaggttgcgttcgagtcccccgcaggcgcgatcgaggtgttcaccacccgcccggacacgctcttcggcgcgagctacgttgtgttggccccagagcacgagctggtggaggagctcactgccgaggcctacccggagggcaccgacgagcgctggaccaacggcgaggccaccccggccgaggccgtggagagctacctgaacaccatcgccgcgaagtcggacgtggagcgccaggagaacaaggagaagaccggtgtcttcctcggttcctacgcggttaacccggtcagcggcgacaaggtcccgatcttcatcgcggactacgtgctcaccggctacggcaccggcgcgatcatggcggtgccggcgcacgacgagcgagactacgagttcgccaacgtcttcaacctgccgatcacggcggtgctcgacggcgacgtctctgaggaggcgttcaccggcgacgccactcacatcaactccgcaaacgacaacggcctcgacctcaacggcctgggcaaggacgaggcgatcaaccgcgccatcgactggctcaccgagcgcgaagccggcgaggaaaagatccagtacaagctgcgcgactggctgtttgcccgccagcgctactggggcgagccgttcccgatcgtctacgacgagaacggccaagcccacggcatcccggaggaccagctgccggtggagctgcccgaggtcgaagactacaagccggtgtccttcgacccggacgaccgcgactcggagccctctcccccgctggcgaaggccacggactgggtcaacgtcacgatggatctgggcgacggcccgaagcagtacaagcgcgacacgaacgtcatgccgcagtgggcgggctcgagctggtaccaactgcgctacatcgacccgacgaacgatgagcagttcgtgaacctcgaaaacgagcagtactggaccggcccgcagccggacgttcacggcgagaacgacccgggcggcgtggacctctacgtcggcggtgtggagcacgccgtgctgcacctgctctacgcccgcttctggcacaaggtcctctacgacttgggctttgttacctcgaaggagccgtaccgccgcctgttcaaccagggctacatccaggcgtacgcctacacggacgcccgcggcgtgtacgtccctgctgtcgaggttgaggagaaggacggcaagtactacttcaacggcgaagaggtcaaccgcgagtacggcaagatgggcaagagcctgaagaacgccgttgccccggacgacatcgcccgcgatttcggcgcggacaccctgcgcgtctacgagatgtccatgggtcccttggacacctcccgcccgtgggcgacgaaggatgtcgtcggcgcgcaccgcttcctacagcgcctgtggcgcctggtggtcaacgaggacactggtgagctcgcggtcagcggcgccgagctgaccgccgaggacgaaaagcagctccaccgcaccatcgccggcgtgcgcgacgattacgagcacctgcgcgacaacaccgtggtggccaagctcatcgagtacgtcaactacctgaccaagacctacccggacagtgccccgcgcgccgccgtcgagccgctggtgcagatggtctccccgctcgctccgcacatcgccgaagagctgtggtcgcggctcggttacgacggcaccatcaccttcgtgccgttcccggcgttcgaggagcacttgcttgtcgacgccaccgtcgaactccccatccaaatcaacggcaaagtcaaggcgcgcatcgacgtgccgacggacgcctccaaggacgagatcgaaaagctcgccctgggcgacccgaaggtcggcgaactcacggctggcaagaacgttgtgaagaccatcgtggttcctggccgcatggtcaacctcgtggtgaagtaggcgccggacggtacactcgcactggcgtaagacttcacaagtttttaggtaaggagagcgccggtgacgaaccagggctacggcaactacccgtcctacggaggggacccgcagggcggggacaaccccggttacaacgggtacaacgactacagcggtaacaatggctacagcgagtactcccagttcgaggtgaactccgccgaggcgctctcgggcgcggacgcgcagcgcttccacggcacccagttcgtggacggctactacggcgacggcgccaccccgcacccgattaatgacccgaccgccaacggctggacccacaccaagggcaccggcaagctcaaggtcggccaagctgtgggctggggcttcaacgcgtaccaggcgaacccgggcatctggctcatcgtgggcctcgttctggcggcgattggcctggtcagcgacctccccgccctcgcagcggtcggccccttggttagcctcgtcgggattttcctcgagccgctgtttgtcagcgctggcctgcaacagaccctgaccaagaacttcaaggggatcaagaccccggcctacggcaagacgctgggcatgctgatcgtggtctcgctcctctttggcttcatctccggcatcgtcttcctcatcggtttcctcatcgcgatcccgttcatgaacttggacccggctctttttgaggacccgaccgcggtgcaggacccggccgctgtcgccgaggtcctcggccagatcgcgccgggcttcatcatcggcggcctgctggtgctgctggtcctgccgttcgcggtctacccgatcttctacgccgcggataacgccggcaccttcggcaacgcgctcggccagggcatcaaggcgggcggccgcaactacggccagaccctgctgctggtggtgatcctcggcgcgctgaccatgctcaccgcggtgccgtcgctgctcaccgtcacgatgggcatgaacgcgtggttctccatcctgctggcgttcctgctcaccgtcgtgatctcgccgcttcgcttcatcatcggcgcccatgcctaccgccaggtttccggcgggccggttccccatgagacaaccgcgtaagcgtctcctcatcacgagcaccctgctgattgcggcagtggtgctcgttcttactgtgggcaaggcgtacttctctgtgccgggcctgtggtccgccgaggcgcaccaagtgcgccaaatccgcctcgtccccttcgaaacattcgtccactaccgcgtgtggtggggcccgtggctgaacttcttcggcaacatcgcgctatttttccccgtggggtggctagcccacgcctggaccggttcagtgcgcaaggcgctactcgccggggtcgcgttcagctgcggcatcgaggttctccaattcgtgctggccgcaggctacagcgatcttgacgacgtcctcttcaactccctcggcgccttcctcggcgcgaaggcccgagagaaggcccgtgagaagacccgcgctagtgcccgtgcacgtacagcgagagaatccgctgcagcatccggtacgccgaccccgtcagcgtagagccttggggcgcgacctcgatcgcgccgaggtcgacgaggaagcgaaacaccaggtcggtcttctccggcactgattcaaatggcggcggggtgatcccgtagtcgccgccgatgctgtaccagtccgcgagcgcccacagcaccgccttccactcctcctcgccgaaggcgtgctcgaagccggccgcccactcggcgatgttgagcccggtgtcgaagaactcgtacgccatgcggccgagctcgctggccaccagtgcgccctcgcgctcctccacaaacccgccgcccaccagcagcagccgcacgtcgtacacggaggggaaagtgttctcgcgcggctgccgaagccgtgagttgatgtgcaggagctccatcatctcccggatcgtggccaccggcatcttgccggtcttggtcagctgcaccggctcgaggaagagcccgatgagtgcgcgcagcgtgatcgggaaccgatccacgaagtcgggctcattatcctccaccgcgccggggaacaaaatgacgttgtcgtcaaggtctccgtcgtcgcggtggtcgcggccgcccgggggcacgagaccggaggggtgcgggcccgggcgctggtcgaagaagtccgaaaccgccgcaagcaaggtcgggttctggtcggggtacgggtcgtcttcaagaatcgcctggaggtcggggcgggaatccaaaaactggccgaactcgtccgcaagcgtcggcgcgtgcgggcgcggcggctggtcgaccgggtcgtaaaagagttcctcggcgatgtagctcacccgcgtggccacggtcaccgggtccgcgatggtgaggcggtctaacatccgctccgggctcatgaccggcaggaagctgagcaggagcggggtgacctccatgttcggcggcaggcctgcggcgatgcggcgcgcctcgtggcggaacttcgtcatcaactcgggtccgttggcggattcgatgatgtcgggaccggctgcgtcgacaagcagcggcgtcgggccacccagctcactggggccgagtgcctcaacccggatgttccaattcgccgtggggtcgtagatgtaggtgatgtcggtgaacttcgagacgaacacttcgctctcgtcggcctcgcccgcgcccggcgactccgagaacacctgccggaatttccccgagccggtgatgaagaggtggctcgcggcgccggagaagccgaaggcggcgtcgatcacctcggcgagctgggtcaggtcaaggctgtcgtcgacgttgacgcagcgggagacctcggggttggacccctccagcgtcatcagcagggtgacaatcattgcggcgcgccaccgaagatgacggcgtacgcccacgcctcggaggcgttcttcacaccccacgtggtcgtgcccgcctcggtggaggcgacctcgccgcgcggtacctcgacgttttgcaggctgaggccctcgctcagcgccagaaagccgtgctcgaagtcggggttcagcgtgaacgcgatctcagcacccggcgcgacgcggatctccgcggccacaatgtcgctgccggtcgctaccggcgaggtttggccgaacatctcgccggcgaagacgcgcgcctcgccggagacccgggtggtcacactccgcagggcaaagggctccggggcgaagatttccagggtggtggcgtctgcggtggcgctggcaagcagcctggcatctaagcgcacgcaccgtgcgccgctggctgcctcgacctgcaccgacgtgctccccggcgcgataacggcctcgccgacctcaaccgtgtcggcgacctcgccgccgcgcagctgcgcccggccgccggcgacccagatgaagctctggtggccgggcgcggcgtgcgtaacgccactgaactcgccggcgaaatcgaaggggccgatcagacccccggcggccccgttttttgcgctgccctgctggtaacccatgtgcgttatggtacctgggtgcagaaactttcggctggcttgatactggcgcttgcgtttttcgccgcggccgcgccgctgtccatcgacatgtacctggccggcattcccgcactgcaagacgagtttgccacctccgcctccgccgcacaggccaccatctccggcttcatgctgggcatggccaccggcaacctcgtcttcggcccgatctcggacgccaccggccgcaagcgaccgatcgtcatcggctcggtgatcctgtttctcaccgccgtcgcctgcgccatggcgcccaccatcggcgcgctgattgccgctcgcttcgtccagggtgtcgccggcggctgcgtggtggtggtctcccgcgcggtgatccccgacctggtcaccggagccgcggccgcgcgcgggttctcggcgctcatggcgctcacgggcttcatgcccgcaatcgcgccagcgctcggcgggttgctcctgccgctgatcggttggcgcggcgtgttctggttcatcgccgcggtcaacctcatccaggtcggccttgcgctctggctgccggagtcgctgccgcccgccgcgcgcaaaccgaacgcgctggcagggctgttcctccgcatcggccaatgcctgcgccgccccgcgttcgtcggctacatgctcgccggcgcgctcggcttcggcgcgctgttcgcctacatcgccgcctccccgctcgtgctccagcgccagctcggcttcagccccaccgccttcgcgttcacgttcggcggtatctccctgctcatcccgctcgccaacgccgtgaacatgcggctggtcaagcgcgtgcccccgcagcggttgctcaccggggcattgcttatcgacgccctcctagccctcaccatcctcctcatctcactgggcgagccctccatcttcatcgtcccgctggtcgcggggctgccggtaatgggcgggttcatcggcgccaacgccacggcgctggctgtcgaggagatccgcgacatcggcgcgggcgcgggcaccggcgccatgggttttctgcagttcgcggttgccgcgcttgtctcccccgccgcgggtctgggtaccaaccacgccctggtgatgggcgcggtctccctcgcctgcgcgtgcgccgcactcgtcgcgctgcgcacgcttaaataatcttgcgctcctgcgcgcgctgcaccgccgccgtgcggttgtccacgccgagcttgccgtagatgtggatcaggtgcgtcttcaccgtcgcctgcgagatgaagagctggttcgcgatctccctgttcgacgcgcccgtcttcagcgcctgcaggatctcgatctcgcgggcggagagcgcctcgtcgggtcggctgacccgctccgcgagcgcccctgccgcctggggcgagagcacgcgctgccggttcgcggctttcagcaccgcggcgtggagctcgtcctccggggcgtctttgagcaggtagcccatcgcgccggcctccatcgcggcgatcacgtcggactgcgtgtcgtacgtggtgaggatgagtaccggcgggccgccggccgcggtgaggagccgagtgagctcgatcccgctcacctgcggcatctggatgtccgtgaccaccacgtcgacaccctcgggcacctccgcgccgccgtccgcggcctcagcgaccacctcgacgtccccgaacgagttcaggacggcgtggaggccggcgcggacgaccgggtgatcgtcaataagcatgatgcgtatcatttcccctccactggaacgctggccgcgagcacgctgccgtcgatggtcagttcgccgccggcttcctcgacgcgggcgcgcaaacctttgagcccgtagccctcgttctcgccgatgcccgggccgttgtcgtagacatccaccgtggcggtgccccccagcatatccgccgtgaccacggcccggttagcgctcgagtggcgctcgatgttgctgataccctcgcgcgcgacgcgctcgatcaccgccgcggcggcggccggcaccgcgtacgccccgtcggcgttcacggtcacctgaagctcgcggccgagggcgcgctggcgctgctcagcggcctgggccagctctttgagacgctgcggcagcggtgcttctgtgcggttcgcgtcgctggcgttgtcggagacgaaacggcgcgcttccgccaggttgtcggcggcggtggcgcggatcgtgttcagcgtcgcccgcgctgcctcgttgtcgccgagctgcttgtccagcgcccggcccagcagcacgatggagcttaagccctgcgccatggtgtcgtgcacctcgcgagagagccgcgcgcgctcctccgccacgcccgcggcgtgctcgaggaccttgtagtgctcggtttcgtcccgcagcgccttgtatgcgtagacgatgaacaccgcgagcgcggtgccgatcgtcggcccgatgaacccgccccagcccgattccgggactgtggtgaacagcgtgccggcgagcagcaacgcggagatgagcaggccgaacggcgtggcgagcaggaagcacgccagcatgaccagggggaactccagccacacgaacgcagacgagcgcaccgcgagctgggcccagacaacgatgacgatccccagccaggcctgctccccgttggcgggaatcggcttgccgcggttgaaccagaccgtgcccgccagatacaccgcggcgaacgctacggcgaggccgagggtgattccatccagctcgcccgcctggttcgcccccacgagacccacggcaagtagcaccgcgaccagcacgtgaaggctcactcccaaaagggtcaggatccggttggtgtgtttcacatcgaccaaggctagtacgggcaatcaaccgatcggttgattccggtttcaaccgccctcccgatgtgtaaacccccagctcacggccaatattaagggcatgttcttagcactccgtgaaatcacatcggcgcgcggccgtttcggcctgatcgccggcaccgtcgcgctgatcaccttgctcgtggtcatgctcaccgggctcaccaacggcctgggcaagcaaaacacgtccgcgctcgaggcgctcgacccgcagtcggtcatcttccaagacaacgacgatccgtcgttcaccacctcccgcgtcgacgcgcgcgagggcacgaccccgctcggcaccggccagagcctgctctcgcgtgacgacggcaccgaggaagccgtcgccatcatggcgcttccggagggcaccgagctgcccggcggcgaggtgctgggcgccggcgcagtcgcgtccgaatcactcggcctgcgcgagggtgagacggtgacggttgggggcgttgaggtgggcgtcgacaagcaaagctccaacctcgagttttcccacacccctgtgctgtgggtgccgaccgcaacctggcagcagaccatgcacaccgacgccgacggcaccgtcctgctggcgagcgacgactccgggctgagcctgaaggattccttccagggcctgccggcgtacagctccgagcagggctcgctgaagatgatccagggcttcctgtacgccatcgcggcgctggtcatcgttgcgttcctgacagtgtggaccatgcagcgcacccgcgacctggccatcttgaaggcgatcggcgcgccgaacagctatttacgacgcgacgcgctcggccagtccgccgtcatcctcgccatcggcgtcatcctgggcacggctgtcgccctcggcctcggcgccttggcagcaggcaccgtgccgttcacgctgaccgtgctcaccggcatcgtcccaccccttctgatcttcgcgctcggcatgatcggcgcgctgatcgctacccgctccatcaccaaagttgaaccgcagctcgcactcggaggtatcgcgtaaatgctcaccatggaaaacgtcaccgtcacgttccaagacggccaagaccgcatcaccgccctcgactccgcgaatttcgaagcgcgtccgggccagctcaccttcatcatcggcgagtccggctccggcaagtccacgctgctctccgcggccgcggggctgatcacccccgattcgggctcggtgcagcttgacgacgtcgcggtttcagacgacgtgcggttgaacaagatcggcatgatcttccagcaggccaacctgatcggcgcgctgaacgtgcgcgaccagctcttgatcaccgaccacatgcgaggcgtgaagccgcgcgccgaccgcgccgactcgttgttggccaaggttggcctggaggggctcggttcgcgcaggatgcagcagctctccggcggtcagcgtcagcgtgtgggcatcgcccgtgcgctgatgggcgagccgtcgctcgttcttgccgacgaacccaccgccgcgcttgactccgagcgctcggtagagattgccacgctgctccgcgagcttgtggaggaaaacaacgtggcgtgcggctttgtcacccacgaccgctcactgatcgagcagggcgacgcagtgtacgaggtgcacgacggtcaggttgagcgcgcccgcgctgcggttggggctgcgtagcggggctgtgttttagcgcaggcgggggcgggagaaccccgccagcgccacgagtgctgccgcgccgagcacgagcgtgatcaaaagggtgccggaaaggaaccctgcgtcgacgcttgccgcgccgagcgcggagccggacgcgatgccgacctggaacgtcaccacgtagatcgagctcgccaggtcctggttgcgcttgccggcgtgcaggaagatcgtggtgccggcggtgggcagcgcacccgccgcgaggccgagcacagcgaccatgatgaacataatcacgccggaatccagctgcagcgcgatgaggccggtcatcgccgcggccatcagcagcagcgtgtcgagaccgttgatgcggatcatgcggcggtccacccggcgaccggtggccaccacgcccaccaaaccgaagatgccgtacatggacaggcccaccggcacccacgcggggctggtggtggtctcaataaacagagcgaggtacgtgaacgcggcgaatagggacgtcaccgcgaaggcgaggtagaacaccagcggcgggatcgcagacttcgtgcgcgccgcgtccgccagctgctcagccggacgcgccggcatgctgggcaaggtgcggatgatcaggagaaaggcgacgatgaccgcgatgcctaagatccatgtcgcgccccgccacccgatcgcgtggccgatcgccgtggacagcggcgcgccgatcacggtggacatggtggagccgagccccaccgccgcaaccgccttgccggtctggcccgggggcgcgagtcgccccgccatcgggttgaccaacgaccagaacaggccgtgggtcagcgccgcggtgacgcgcccggccaccaagacccagtagttcgtggccagtgcctgtaggacgatgccggtgaggaggaacgcgagcgtcgctaagaacactggcctgcgatcgagatgccgggtggcgtgcacgagcgggatcgtcaccacggcgacaaggccggcgtagatagtcatgagcaggccgatgcggccctcgctcacccccaggtccgcagccatcggtgtgatgaggccgaccgaaaacatctcaaacgtgacgtacacgaacgccgcaaaacccatcgccgcgattggtacgcgctgaagcgttgtgtactgaggctcttgatgggcgctggtgttggtcaccggtgcagggtatgccctgtggggcggtttcgccagacgggttgctgcgcgctgtagctcccaaggattttggcttgatccggctccggaaaggcactggtcagagcgctaattattctctcagattccttgggagctacagcctgtagctcccagcgctaagagggtggtttctgccacctgtttccgcaggtggggtgtgtagacaaatccttgggagctacaggaggggagcctacgtcaggtcggcggtggcggggcggatgaactccgcgatccggctggcgggggccgcggccgacccgaagggggtcatcgaggcgagcttggcggccaccgcgtggatggtgactgactgggcgaggatgtccgcgatctcctcaggggactcgtccgggtcggcggcgcgggcgaggcgggcgccgatgaggccggaaagcacgtcgccggagccaggcgtcgctgcccaggaatggccggcgtcgacggcgaagcagtaatcgtcggcgtcgggcgtgcagatgagggtgacgcgccccttgcgcacgatgaagcagcgcagctcagaggcgaggcgaagtgtttggtccaggcgggcggtgtccgccgtgcccgcagacgcgagaccggcggcgtcgtagaggcgggcgaactcgccgtcgtgcggggtgagcacggtcgggtgggggcgctgctggataacctcgcgcaggtcggggtgggaggcgaggagggagatgccgtcggcgtcgataagcagcggctccttctgttccagcaaccaccgcaactccgccgcggccttgtcgcccgtgcctgcgccggggccgaacacccaggcctggacgcggccggcatcttgaagcgtgtccgtcgccaccacttcggggttggcgcgcaccacctcgagcgcctgcgggccggcgtagcgcaccatggcgggcgtggcgttgaccgcggcggtggtgcacaaaatcggcgccccgggatacgcgtcgctgcctgcgcggatgccgaccactccgccgctgtacttgtcgtctcccgggcccggctcgatcggatccgccatcatcgtgggcagcgggtgggcgtaggcggtggaggcgaagtcgccgttcaccgcgcggctggccagcaccatgagggtgtcgccgagctcgccctcgtcggacatgtccgcgagcacctgctccagcgtggtgccgcctgcggagatgtccacgcgcagctggtcgccgcaggccgggttgagcacgtgcgcgcggcgccacccaccgaaagtgacggtcgcgtccgcggtgacgtggaggtcgccgccctcgccggtgtcggcgtcgattccggacggcacgtccaccgagagcacgcgcagatcggggaaggttaagtcctctaccagctccgcgtactcctcgcgcaggccggcggtgccgccgatgccggtgatcgcgtcgatggccaggtcgtactcccagatcatatccggggcgctgtcgagcactttgccgccggctttgcggaaggcctgcagcgcgcgggtgtgggcgctgcccgcggtgaggtgcaccgcgacgtcgtggccgtccatcgccaagcgcgcgccggcgtacagcccgtcgccgccgttaccgcccgggccggcgaggatgacgatgcgcgagcgcgcgccctcgctgcccgccggcagctccgtcatcatggcgtgcgccacgttcgcaacggcttcggcagcggactgcatcaactcgtccgggaaggcctcgcgctcaagcagcacggcctcggcgcggcggatctggtcgacggtccaggtcatgtcgttcatgccgacccagcgtaaccgcggcggtactattgcgcccatgccgtacaacgtcggttttgaccgcgagcaatacatccaaatgcagtcggagcacatctcggcccggcgcgccgaggtaggcggcaaactctacctggagatgggcggcaagcttttcgacgaccaccacgcctcccgcgtcctgcccgggttcacgccggacaacaagatcgcgatgctggaccgcatcaaggacgaagtggagatcgtggtctgcttcaacgcgggcgacgtggtgcggcaaaaggtccgcgccgacctcggcatcacctacgaagacgaggtgcttcggcttatcgacgtgttccgcgaccgcgggttcctcgccgagaatgtggtggtgacccagttggagggccacaacgccaccgttgaggcgttcttggagcggctgcgccgcttaggcctgaaggtgtcgcgccactacctcatccccggctacccgcagaacaccgacgtggtggtctctgacgacggcttcgggcgcaacgagtacgtggaaacctcccgcgacctgatcgtgatgacggcgccgggcccgggctcaggcaagctggccacctgcctctcgcaggtcttccacgagcacaagcggggtatccccgccggttacgccaagttcgagaccttccccatctggaacctgccgctgtcgcacccggtgaacttggcatacgaggcggcgacggctgatctggacgacatcaacgtcatcgaccagtaccacctcgacgcgtacggcgagcaggccaccagctacaaccgcgacatcgaggtgtttcccctgctgcgcaccctgctgaaggaggcgacgggcacccagccgtacaagtcgcccacggacatgggcgtgaacatggcggggtactgcatcagcgacgacgccgcgtgccgccacgccgccgagcaggagatcatccgccgctactaccacgcgctagtggaagagcgccggctggatctggcgtcggtgacctcggaccgggtgatgaacgtgatgcgcaaggcgaacgtcaccaccgccgaccgcgcggtggtggcgccggcgcttgaggtggcaaaacttacgggcagccccggcgtcgcgctcgagctgccgagcgggcagattgtcaccggcaagacgtcggacttgctcgggccgtcggcagccgtgctgctcaacgcgctgaaagcgctggccggaatcccggacgaggtgcacctgctctcccccgactcgatcgagccgattcagtcgctcaagacgcgccacctggggtcggtgaacccgcgcctgcacaccgacgaggtgctgattgccctgtcggtgtcggcttcgaccaacccgcaggcggcggccgcgctggagcagctgaagaaactgcgcggctgcgacgcgcacaccaccacgatcctgggctccgtggacgagggcatcttccgctccctcggcgttttggtcacctccgagccgcagtactggaagaaggcgctgtaccacaagcgttagggctgcttggctagggtgggccgcatggaacgcttagcgttgaccagcgaagatcgggtgctggcggttgtcgcccacccggatgacatggagtacggcgcgtcctgcgccgtggcgaagtgggcggaggcgggcatcgacgtcgcctacctcctccttacccgcggcgagcgcgggatcgctggcatggaccccgcgaccacgcgcggcgtgcgagagaaagagcagcgcgccgcctgcgacatcgtcggcgcgggcgagcttgacctgctcgacttccccgacggcacgctgacctacggcctggagctgcgcaaggcgatcacgaaacgcatccgggagttccgtccaactgtggtgctcacccaaaactgggcggatgtcgcgccgtgggggctgaaccaggctgaccaccgcgtggccggcctagccgcggcagacgccgcgcgcgacgcgggaaacgagttcgtcttcccggaggcaggcgggaagcaccaggtaagccagctgctggtgaccgggcacaatgacccggactgcggcgtggaggtgtccaagcgccacgtcgacgccggcgcggcgtccctggacgcgcacgaggcgtacttcaaggcgctgccggatcacccctccggcgcggagctggtcggcggcgcagccaagcagggcggcgaggcgctcggctgcgacttggcaattttgttcaagcgctaccagctctaaactggccggttatgaccggaaagatcctcctgtactacaagttccagcccatcgcggacccggacgccgtgcgcctgtggcagcgcgacctgtgcgaggggctggggcttaccggccggatcttgatttccaagcacggcatcaacggcaccgtcggcggcgacatcgacgcgtgcaaggcgtacgcacgtaagaccaaggagtatttccgcggcattgagtacaagtggtccgaaggtggtgcggaggacttccccaagctgagcgtgaaggtgcgcgacgagatcgtggcgttcggtgcgccgggcgagctggaggtggacgagtgcggcgtggtcggcggcggtacccacttgtccccggagcaggtcaacgagctggtggccaacaaccccgacgtggtgttcttcgacggcaggaacgcccgcgaggccgagatcggcaagttcaaaaacgccgtcgtgccggacgtggagaccacgcacgacttcatcgccgagctggaaagcggcaagtacgactggatgaaggacaagccggtgatcgcgtactgcaccggcggcatccgctgcgaagtgctcaccccgctgatgaaaaaccgcgggttcgaggaggtctaccagatcgacggcggcatcgtccgctacggcgagaagttcggcaaccaggggctgtgggagggctcgctgtacgtcttcgacaagcgcatgcacaccgagttcggcgcgccggacgacccggcgtatgtccaactcggccactgcgtgcactgcggcgaggcgacgaatgatttctacaactgcgccaacgagccggagtgccggcaccagtacctgtcgtgcgaagcgtgccgcgagaagctgccctactgcgccgactgcgcggccagcatgccgacggtgatgatcaaccagaccatggtgaacggcactagcggcagccagaacacgcccatccagggcgcccagcgctcgtagcggttgagcttgcgcaccatgatcaccgcgcagccgatgagcatggcgaacggcgggatcgaggtgagcaccgcccaccaggtgcgccacgtgtccgtgcacaaccacgtcgcctcgccggcgtcgcacagctcgccgccctgcacacgcgagatggtggccaagatgagggcgaagaggagggtggaggcgatcgtcgctaagccgtagcccactgcctgacgcgtggagtgctggttgcgctcggcgaccgccagcggatccggctcgtcggccagatcgtcgaaagtcttcggctcggggcgcggccgggagaagcggtcctgcgcgcccgtgaggtcgttttcggggtgctcgctcggggtgtgcgccatgtgccctacgctactcccccggttattcagcgccgcgcgggtagatgatcaccggcaccggcgcgaagcggatgaactcgctctccctcgagccgacgaacacgcgcatgagctggccagacggctgggagccgaggcacatcacgtcgcccttcttccacttcaccgcatcggttgcgcgcttccaccctttgcccgtggccaccgtggtgtgcacgtcgaaggtgtcggcgaacgccgggtcgagctccgtggccaccgcgaacgcctggtcgcgggcgcggtccagctggccgagcaccgcctcgttccactcggctgcggcctcggagaggctgatggactgcggcttgggcgaaaacgcgacgatgcgcagcggcacgcccaaaacgcaggccatcgtggccgcgtacggcaggccggagaacgtggtggtgtcctcgatatcgtcggcttttgacggctcgatcagcgcgtaggtgacgcgggtgacgcccttgcgcgataagttcacgcctttcggggcgagcccgagcggcaccggcgaggagtgcatcagctcgtccgccaccgaggagggccgaaaccggctttttgccgtcttcgcgcgcgagcccagaaggatcatgtcggcgtgggtgtccttgaccgtctcgcagaggcaaccggtgatgtcggagcgttccgcgagctgggctgcggtcttcgcccactgcgagcgcggcaggtgcgccttcagcacgcgccgggcctggagctcgaactcctgcgagcggtcgcggaaccagcgcttgtacttcttgccggtgagcggcttcttccacgcgccgtcgacagcggagatcgcggaaaccacctgcaccttcaccggcagggagcgcccgagccacgcggcgaactcgatggcctcggtgttttgcgcatcccagccgacgacaatctgcagagggcgctggttagcgtgcgactctgctaaatcggtggtaaatgcgcgggaaaccattgccgagcacattacttggcgctggtccccagctgcgaattaccgcctagatgtgaccaatctgaccgcgcttggccgcaagctcggccgcgttgtagctgcgcgccagcgcgttgatcgcgtctaccgaggtggcgaggctggcgagctcctgcgggtccagggtggcaagcatcgcggcgagcgactgcgtgcgctcctctcccacccgctcgagcacttgccggccgagttcggtgagctcgacggtgacaccgcgccggtcctcggcgaagcgagtgcgctgcaccagcccgcggctctccagaaggttcacggagttggacgcggtgggcattcgcacgccttccgcctcggcgagctgtcggatgcggcacggtcccgtctcctgcagtcggtgcataatggaaagctgcggcccggtcagctcggagtgctccgcggtgcggaagtagctgacgtaaagcctggtcaacgccgggcggatccggcgggcgagctctacgggatcgggtccatcactcacggccatcaatgctcttttctttattgaacatttggatgttgacagataaaaacaatagcaaccacgtcccgcgcgtcacttacgcgcacgaagtttcgcacgagtggcgccgcaggacggtgctcaaggggcttccgcttgccgacgcccaccggttccacgccgaccacctcttgttggcagccgccgaacaccacgggcgcgacaccgaccgggcctgccccgtgtgcgcctcgccggatctccgcgaggtcgcctgggtctacagcgagaaactcggccgccgaagcggcaccgcgcgccgggacgacgaaattgcgcgccttgttgctgaggttggccccatcaccgtgcactttgtagaggtgtgcccgcactgccactggaatttcttgctgaaagaagttactgctcatgagccaaggtagtgtgtccccttgtggtagagaacgagcaaaagccttccgctaagaagggcgggtccactgctgttaagaagaaacgcaaggtgcgctggggccagtggctcctcgccctgcttctcctgttgcttttgcttgctgcgattccgttgacgtggttctggctcaactaccgcgaagcgcacatcccgcagcccaacgagatcgagaccgcccaggtctcgaacatctacttcaacgacgcggagacggagctcgcgcgcgtcgtcccgccggacggcaaccgccagcagatcccgctggacgcggtgcccgagcacgtgcagaacgccgtgctcgccgccgaggaccgcgacttctgggacaactccggcttctccttcaccggcttcgcccgcgccgcaattggccagatcactggcaacccgggcgccggcggcggctccaccatcacccagcagtacgtcaaaaacgcgctggtgggcaacgagcactcctacgagcgcaaggcgcgtgagctggtctactccgtgaagatgaccaacgagtggagcaagcaggacatcctcaccgcctacctcaacaccgtctacttcggccgcaacgcatacggcatcgaggccgccgcgcacgccttcttcggcaagccggcgagcgagctgacgctggaagaaggcggtgtgctcgccgcctcgatccagctgccgtcgcagctggatccttggaccaacccggagggcgccaccagccgctggaactacgtcatggacggcatggtggagatgggcgcgctttcccccgatcagcgcgctggcctggagtaccccgagacgcgcgacccggcctcctactccgcctacaccgaggccacgggtccgaacggcctgatcaagaaccaggtcatcaccgagctggaggcgctcggcatcacggaggacgacctgaccaagcgcggtctgcagatcaccacgacgatcaaccgccagacccaggagacggtcgagcgcatcgcccgcgaccagctggccaacctgcaggacgacgcccgctccggcgtcgtcgcggtcgacccgaactcgggtgccgtgctcgcctactacggcggcgacgacccctcgggctgggactacgccaacgcgggtctgcagaccggctccacgttcaagatcttcgccctcgccgccgcgctgcagcagggcatcccgctgaccgcgacgttcgactcttccccggtgaagctgccgggcgataacgtggtgacgaactgggacggtggcggcggcggcatgctcaccgtgaaagacgcggtgcgcacctcctccaacacggcgttcctgcgcatccaggacgatctggacgacggcacccaggacaccgccgacatggcccacgcgctcggcgtggcgcgctcgatcccgggcatcccggtgacgctgcgcgaaaacggcggccagccgtacgagggcatcgtgctcggccagtaccagtcccgcgtgctcgacatggcggccgcagtttccaccatcctggaccgcggtgtctaccacccggcgcacttcgtcgagcggatcaccgacgcctcgggcgaggtgctctacgaggtggaccaggactacgcggagcgccgcttggcggagcaggtcgcggacaacgtggtcgaagcaatgcagaccgtggtcggctactccaacgccaccctggccggcggccgcccagcggcagcgaagaccggtaccgcccagctgggcgacacgggcaacaacaaggacgcctggatggtcggcggcacgccgcagctgtccgtcgccgtgtgggtgggcaccgccgacaacacctccccgatcttcaacgagtggggcggcaacatgttcggctccggcaccccggcgaagatttggaagcaggtcctcgatgaagcgctcgacggccaggagatgctgcagttcccgaccgcgagcccggtctactggggcgtggatccctactcgggcggcaccaacctgggcggctactcctcgggctactacaacacgccgacctatggctacggcaccggcacgggcaccggcgctggcactggcgcagatcaagcgccgtcctcggcggctgaccccgcaccggaacctggccccgagcctgcgcctgccccggcgccagccccggcaccggctccggcacccgcgcccgcacccgtcccgccggctccggcgccaatccaagacgcgattagcgacgccctggatagcctgggcaccatcctccagtagcagcacgaggtagaacatgacgacgacgtgggcagatcccgcctaccgcgtacagccgggaaaaaccgaaccgactgctaaggggtgggtgaactttctcggcgggccgatgggccgcttcgccccgatcgggcgcgcgaggttctggactcccctgcgcgccattttggcgctggcctacaccatgctcacgctcggcgggttgtcgaaggcgaactgttcgctcggccgcgccgacgaatctggagtgttgcgcctgaactgggacggcaaccgccagtacacctcgttttgctacaacgacatcgtcccgctctacggcgcgcgcgggctggaccagccgggcttcgtctacgactactcgtgggtcgaggacgggctgacccgctacatggagtacccggtgctcgccggcctgttccagcagttcactgcgttcatcgcccgcaacacgtacttcctcgtcgacaacatgctccccgacgtgggctggtacttctggctcaccgcgctgttcctctccatcatctgggtgtgcaccgcgcggatggtggcggagctggccggcaaccggatctgggacacgctgctggtggtcggctctcccctgctgatcatgcacgcgttcaccaactgggacatcccgtcgatcttcttcctcgtcgccgcgatgctggcggctcgcaacgagcgctggtggctcgcgggcatcctcgtcggcgcgggcacgtcgttcaagctgtggccgctgttcgtgctcggcgcgtacctgaccatcgcaatccgcaagcgcaccttcgccccgtttttcaagatgctcgcggccaccgtcatcacctggctggcgatcaacgtgccggtgtacctgcgcaacccggacgcgtggggcgagttcaaccgcctcaacaccgaccgcggctgggagtggaccaccatctacgcggttgcttcccgcgcgttcggctggaccggcttcgaccacggcgagggcgcgccggtcatcctgaacacggtgacgttcctgctgttcgccggcggctgcttggccgtgctgatcatgggcctgaagtgcccgaaggagccgcgcttggcggagttgctcaccctgatcgtctgcttcttcctcctgttcaacaaagtgtggagtccccagtactccctgtggctgatcgtcccggcggtgctcgctgccccgtactggcgcttgctgttgagctggatgaccgtcgacatgatggtgtggccgatcctcatgtggcacatgatgggcgccgacaacttaggcctgccgggtgcggcgctcgacatcgtgatcatctgccgtgacgcgttcatcgtcgcgctcatggtggtggtggttcaacaaatgtttgccaagcgcgccgacaaggtcgccgacgcgcacaacgggcacgaccccctgctcacccgccccgccgactgggatgagcccgcacatgcttaacgccaccaccatcgccgggattgtttcgatcctggtggcgttcgcgctgttcatggcagcgttttacttcaccacgaagaaacgcaccaagctcgcggtcgccttcggcatcgcggcgtttctcttcatgacgctgatcccggtcactctcgccgtcttcggcgcggcggcgaaccccggcggataaaagctcgcatgaaagctacggtgggcggcatgcgacaccgacttcgagtttctgtccttgtagccgcggccctcgctgtgccggcactcaccgcctgcggaacctccgacgaggctgtacccgagaccgcagcgcctgtgcaggcggcgtcgccggcagccgaccgcgacctgcccaccgccgtcaccggctacaccgacgaggcccgcgaagagatggcggacgacgggctcgcagaagccgacgttgaaggcgtgctgcaagccgcgctcgacggcaacgccgatgtcgagtgggacgacgacggctacttcgaaattgagttccgcgatatcgagattgacgttgaccctcaggggttggtgagggatgcggataggtaggcgtcgataagcaaaaagctccttttggtgcggtgacgggcgtgcggtacgctaccaaggttgcttgacgccaagcgaccctcctgccaccgccacaagggcggcggccgataaaccaaagaccataggaggtgatgaggtccgtgcgtcactacgaagtaatgatcattctcgatccgcaacaggatgagcgcaccatcgccccgtccctggataagttcctcgagaacgtccgcaaggatggcggcacggtggaaaaggttgatgtgtggggcaagcagcgccttgcttacccgatcaacaagaaggacgagggctactacgccgttgtcaacctcgtttgcgagtctgacaccgtcgccgagctcgaccgcgtcctgaacctgaacgaatcggtcctgcgcaccaaggtgctgcgtaccgacaagtaagaacagctaggctcgtccacagatcaaccgcaaataaaaggtagggacagatcatggcacaaggcgacacacaaatcaccgtggtaggcaacctcgttgctgaccccgaactgcgtttcatccccagcggcgcggccgttgcgaacttccgcatcgcgtccaccccgcgcacgttcaaccgggagacgaaccagtgggaagacggcgaagccttgttcctgacctgcaactgctggcgccagatggcggagaacgtcgctgaaaccctgacgaagggcatgcgcgtgatcgtcaccggccgcctcaagcagcgctcctaccagacccgcgagggcgaaaaccgcaccgtgttcgagatcgaggtcgacgaagtcggcccgtcgctcaagtacgccaccgccaacatttctcggaccacgcgtgagggcgggtccggcaactacggcggcgggcggcagggcggctccgagcagggcggccagggcggatttggcggcggcgctgctgccgggtcgttcggcggggcgccgcagggtggcttcggccaaggcggccaggggcagggcaaccagtcccagggcaaccagaacgccaaccagccggccaacgatccgtggaattccgctccgtcctccgattccttcggtgggatggacgacgagcctccgttctaaacagacaattccccacacacttttcaaccagaaggaaggttaggatttatgaaactgatcctcaccgctgccgttgagaaccttggagagcccggcgacgtcgtcgaggtcaaggacggatacggccgcaacctcctgctgccgcgcggactggctattccggctacccgcggcgcggagaagcagattgcagacatcaagcgcgctcaggcagaccgccaggtgcgcgacttggaccacgcgaaggagctgcgcgaccagctcgaccagctgagcgatgtgaaggtgcccgtacgcacctccgagagcggcaagctcttcggctccgtcaccgccgctgagatcgcggatgccgtgaaggctgccggcggcccctcgctggacaagcgccgcatcaccgtgccgaagggtcttgtgaagaagaccggcggctaccaggtgaaggtcaacctccacgatgacgtggaaggcaagattaacttcgaggtcgtcagcgcttaagagcattttgcttgacgacgattgcgtggcaccctaaccccgcaatccaacgacaacagcatttttgataaggcgcgggttccacttgtgaggagtggggcccgcgccttatcgtgtggtgtggccattacgcaggtgcgcatcgacgccccggttgccgggtacgcggccgggctcgccgtcgtgcgcgcgctttcggagcgccctctagacattgccccggtcactatcttcaccggcgacaacggggcggggaagtcgacgctcgtggaggcaatcgctgcggccgcgggggcgaacgccgggggagggtcgcgcaacgcccgcttcaccgccgccgaccactccgcactccacgagtcgctgacgctgcgccgcaccgcgaacttcccggacgtctactttctgcgcggggaaacctacatcgcgctcagcgagtaccacgccggcctcaccgaagacccgctgtcgcacttgactcgacgcagccacggccagggcatcatggagctcgcgcgtacccgcttcggcgcaaactcgctgatcgtgctcgacgagccggaggacggcctctcggtcttctcccagctcgagctgctcggcctgctcacggtgctgtcgtgccgcggcgcgcaggtcatcatggctacgcattcgccggtcctggtcgctgtgccgggcgcgcgcattgtcgaagttccctcactggagcaggtgcactatagtgccgccgaacccgtcaccgcgacccgcgaatttatccgcgaccccgcaggaaccgccgcgtacctggtggagcctctaggggggccgtgatgtttatcaaccgcgtcactgttgatgctgcggctgcgccgcagtgggcgctcgaggcgagcgtcatcgactacgtcgcccagttcgatctcgccttcacgcacccgatcacgctaatcaccggcggcaacggggtggggaagtcaacgctgctcgaggggatagcgcgcgggtgggggtttaacgcggagggaggaacgtggggcgtcggcaaggctggtgcccgcgatgcgctctacggtgccgttggcttgcacaccgggccgcgcgctaaggcgggctacttcctgcgcggcgagacgcacacgcgcgtcaccgagttcggcggccgctcccacggcgaatccgtgatggagctggtgtcccggctcattccggacgcgctgtacctcttggacgagccggagtcgggtctgtccgccgtctcccagatggcgctggtggcgcagctgcacgaactgggtcagcggcgcgcgcagatcatcgcggtgacccactcaccaatcgtgctgtcgattccgggggcggagattatcgagttcgacgagcacggggcacggcgcggtattggggtagaggagacgctcgcgttccgggccatgcgcgacttcctcgccgagccggaggaaatcgccgaatacatggccgagtgggcggagtcggagatctaacgcacccaatcggtggtgtgaatagctgtggagaaataaccgcagcacaccggcgtttttggcgaaaacgagcctgaagtggcgtgattttcggtgttgtcaaacaccgtggtggcggggttatcccccgttccgggctttgagaggccagttgcataaaatgccgctgaagtgcggtatctgggatttccgctggcattttgccggcctcatccacacgatttccacaggccgaccgggcgcgctgtggataactctggcgtgcgatggggagtttcccacaaggcctgtggataacgtattgtgcagtttgcgttgcggggtaatctcatacccacattgaaaggggagcatatgggtttacacgacagtttcgacgacgattatgtgccgccgccggagcccagcgacgacgcaccgccggagttctccgaatcggcgttcgctccctcttctggttcgacgccgccgcgccgcggatccgaccgtcgcggggggaggggcggctccacgcgctacgaccgcgagcgcggcaccgacgcggagtaccgcaccccgccgcacgacgagcgcgcggaacgttccgtcctcggcgcgatgcttttgaaccaggacgtgatcgcggacatcgttgaccgcctgcgagcggaggatttctatttcccggcgaaccagctgatttacagctcgatcattgacctttactcggaggccagcgagatcgacgtgctcatcgtcgccggccggctcgaccgcttcaaccagctggagcgcgtgggcggcgcgccgtacctgcacacgctgatctccgaggtgccgacagcggcgaacgcgcagtactacgcgaacatcgtggaggagaagtcgctgctccgccagctggtcaacgccggcactcacgttgctcagctcggctacgagggcgaggagggcatggaggtcgaagcgctcgtcgaccgcgcccagcaggaagtcttcgccatcgccaggaacgaccgcggccaggactaccgctcgctctcggagcttttgaagccgacgattgacgagctgacgcagatcgccgccggcggcgcgctcgaggccggcgtgccgaccgggttcattgacctggacaacctgaccaacggcctgcacgcgggccagatgatcatcgtcgcggcccgccccggcgtgggtaagtccacgctcgcgctggacttcatgcgctcgtgctcgatccacaacaacaagacctcggtgattttctcgctggagatgagcgcctccgagatcatcatgcgcctgctgtctgcggagacggagatcaagctgtcctcgatgcgctccggccagatggaggagcgcgactgggagaagctgaccaagcgcctcacagagatccaggaggcgccgctgtttatcgacgattcaccgaacctcaccatgatggagatccgctccaaggcgcgcgcgttgcagcgccagcacggcctcgatctcatcgtcctcgactacctgcagctgatgagctccggcaaaaaggtcgagtcgcgccagcaggaggtctcggagttctcccgccacctaaagctattggccaaggagctcaaagttcccgtaatcgctatctcgcagctcaaccgcggtcccgaagcccgcaccgacaagcgcccgcagctggctgacctacgtgagtccggttccctggagcaggacgccgacatggtgttcttgctgtaccgccccgactcccaggaccgcgacgacgaacgcgccggcgaggccgacatcattgtggccaagcaccgcggcggcccgatcgacacgatcccggtcgcgcaccaactgcactactcgcgctttgtgaacatggcgcacgggtaagtttcaagcaaaggttggcaagactaactgaagttaggagtggctttccaacggtgacaagcaggtcaacggtgtttattatcgctcggtagataccgaccacaccacaggccacaccagaggagaaagccatgaccgtgcgttccattcacgcgccggccgcttgcgcgagcacggtggcgcagctcgagccgggcatcacgatcgcccacaccgagaagtccacgatgctgctcaacctgccgcgcagcatcgacgagctggacaaggcgacgggccgcgccgacgccggcaagcagcgcggctttatcgcccgcctctggaagtaactccagccagcgcgactagttcagcgcgacgcctttctgctccgggagggtgaacgcggcgatgcacgcgatagcgaacgccgccgcgaagataccgaacacagcgatgttgccgccgaacgcgagcaccggcgggacgatcagcggcgcaaggattgagccgacacggccgaaggacgcgcccgcgcctgtgccggtggcgcggatggcggtggggtagagctcggggccgatcgcgtacagcgcgccccacgcaccaaggttgaaaaacgacagcaagcagcctgcggcgatgatctgccactccgcaccggcgagcccgtagagcagcgccgagaccgcggagccgccgaggaaggcggcaagggtggtgcggcggccccagacctcaatcagccacgcggctgccgcgtaaccgggaagctgcgccagcgtgatgatgagcgtgaaggaaaacgacttcaccagcgtgaagccttgggcgacgagcagcgacgggatccagataaacgcgccgtagtaggcgagcgacacgcagaaccacacgatccagaacgcggcggtgcgcgccctcaggtccggtccccagatgccgccgcgcaccgggtgctcttcagcgcggactgcctcgtcgtagtcggctggatccgcctcggcctcgaaggagcgcacgatttcctcggcctcctcgtggcggccctgcgactccaaaaaccgcacggactccggcagacccatgcgcacgtagagcgcgtagagggccggcacggcgccgagcgccaagccccagcgccagccggtctcgctctgcgcgacgacgaaggtgccgatgaccgcagcaaggatccagcccacggcccagaacgcttcgaggatgaccaccatgcgcccgcggacccgccgcggcgaaaactcgctgacaagcgtggaggcgacgggaagctcgccgccgagacccaggcccacgatgaagcggaacaccatgagtgcgccgacggaggtagcaagcgcggaggcgccggtggcaaggccgtagatcagcagggtgacggcgaaaacttggcggcggccgatcttgtccgctagaaggccggcgacggaggcgccgatggccatgccgatgaacccgacggacgcgatccacgaggtggtcgatttgtccaagtcccagtggaccgcgagcgcggcgatgatgaaggagacgagtccgatgtccatcgcgtcgagggcccagccgatgccggagccgatgaggaggcgtttgtgctttccagtgaccggcagtcggtctaggcgctcggtgcgggtgagctgggtgcgggtgagttcagcagggtttgtcacccatcgaattttgcctcaaaaccgcgcagccgcagcgaattagatacaacgaacaccgacgagaacgccatcgcgatgccggcgagcatcgggttgagccagccgaacgcggcgaccgggatgaggatgacgttgtaggcgaaggcccagaacaggttgcccttgatcgtcttcagggtacgccgcgacaggcggatgccgtccaccgcggacccgagcgaatcgtgcatgagcgtgatgtcggaggcctcgatcgccacgtccgagcccgcgcccatcgccatgccgaggtctgcggcggccagcgctgcggcgtcgttcacgccgtcgccgaccatcgccacgttgcggccctcagactgcagctggcggaccacctcgaccttctgctcgggcaggacgccggccgtgacgttggcggggtcgatgcccacctcgcgagctgctgcctgggcggcaccagcgttgtcgccggtgagtaagtgcggggtcagacccatcgccttcagctccgcgatggcgcgcgcggagtcctccttcacggtgtcgcgcaccgcgatgacgccgatcggctcgccgtcgcgctcgaccgcgatggcggtcgcaccgtcggtctcggcatcgtcgaacgcctgctgcaaggcccccaggttgctggtggggcggccggtgtagatgcggtgggcgtcgataagcgaagaagctccgctacctggctcgttgacaaactccgtcccctcgggcgcgtcaatgcctgcggcgatggcgcgggcgatcgggtgctcgctctgcgcctccacacccgcggcgaggcggtggacctcctcggcggtccagccgctagccggggtcacggaggtgacctgcatctggccggaggtgacggtaccggtcttgtccagcacgatcgtgtccacctcgcgagtggattcgaggacctccgggcccttgatcagtagcccgagctgggcgccgcggcccgtgccgacgaggatcgcggtcggcgtagccaggccgagggcgcacgggcacgcgatgatgaggacggcgaccgcggcggtgaacgcgtgggcggtgccgtggcccatagcgaggtgcaccacgagcgcgaggatagagatgccgatgaccacggggacgaaaatctgcgagatcttgtccactaatcgctgcactggggcctggccggactgcgcgtcgcgcaccagcttgcccatctgggccagtgtggtttcggcgccgacgcgggttgcctccacgatgaggcggccggaggtgttcagggtggcgccggtgacgaggtcgccctcgctgacctcgacgggaacggattcgccggtgagcatggaggcgtcgacggcggagtggccggagacgacttttccgtccgtggcaatcttttcgcccgggcgcacgacgaactggtcgccgactgctacctgggcgatggggacgcgggtctcgcggccgtcgcgaatcaccgcagcgtctttcgcacccatgtcgagaaggttgcgcagggcctcggaggattggcccttggccttgacctcgaaccagcgaccgagcagcaggaaggtgatgaccacgcagacggattcgaggtagatctcatccatcgacgcgtgcgccgggttgatgctcatttccatggtcatgcccggctcgcccgcgttgccaaagaagagcgcgtagatcgaccagccgtaggcggcagtcgtgcccaaggtaatgagcgtgtccatggtgaagctgccgtggcgcaggttgagcagggtggcgcggtggaacacgcggcctgctgcgaagtacaccagcgtggtggccgcgagtgccgcccactgccagtgcatgaactgcagcgccgggatcatggagaccagcgtgacgggcagcgagacgatcgccgcccagatcgtggtgcgcttcagctgctcggcctcttcgaggcgcgctgtgtcgcgggcgtccataccgccgcctgcgggagcttgttggctggcgtcgtccgcgttcgagtccgcgctggaggcgcccggctcttccacggcgaacgcgtcgtacccagccgcgcgcaccgtggcgatgagttggtcggtgtcgaccacctgcgggtcgtagtcgacggtggcggtctcggtggagtagttcaccgaggcgtccaccccgtcgagcttgttcagcttgcgctggatgcgcgaggagcatgaggcgcacgtcatgcccgtgacgccgagctcgatgtgttgcagggctgtttccataagccccactgtatgcctgcggggctaagaacagaaccgagggagggtgcgggcttacgccagcgtgtagcctgcttccttcacggccgctgcgacagcgtcgtcggagaagccctcgccggtgacctcaacgtcgccggtggtgtggtttgcgttgaccgcggtcacgcccgcgatctcggagatctcctcctgcacgctcagctcgcagtggccgcaggtcatgccttcaactttgtagttcttcgtagccatggcttccaacctacgccgaaagtacgaactacgccgaaagctcgaaccctgcgttcgccgcggcctggttcacgtcctccgcggagaagtcctcaccggagaccatcatggtcgcctcatcgacgttcacatcgacggtgtggatgccctcgaccagctgcacctcatcaatcagcgagtcgacggcggcctcggtggacgggcccgagatgcggtaattcttcgtcatcggatgtgcttcctcctcaatgcattccccgcttggcgctcttcgcaggtcggcgggggaatactcgcgcgctggtacggttgaagtatctggcacgataacaaatagttgaaacggagtacgtaatgagcactatcgatgtaaccgaggacacattcgagcagactgttaccgccgacggcattgttttcgtcgacgcgtgggcgtcgtggtgcggcccctgccgccagttcgcgccggtctacgaaaaggtttcggagcagcacccagacgcgacgtttgccaagctcgacaccgaggcgcaccagggcctcgcgtccgcgctcgagatccaggcaattccgacgctcatggctttccgcgacggcatcatggtcttccgcaacgccggcgccctgccggaggctgcgtttagtgatctggtcgaccaggtgaaggcccttgacatggatgaggtccgccgccaagttgaacagcagcaggcgcaggcccccgaggacgccgaggacatcgacaacgaggactaagccgctggttccagccccgcttcggcggggcttttttcgtacactgaggggcaattgcttatcgacgaaaggtggcacccatggcgaacccattctccaagggctggaagtacatgatgcagtccttcgactccaagattgatcagaacgcggatccgcgcgtgcagattcagcaggcagtcgcccaggcaaagaagaatcaccaggaaatctcgcagcaggcggcctcgatcatcggcaaccgcaaccagcttcagatgaagctcgaccgcctgatcaagtcccaggaggacctgcaggcgaagacccgcaccgcgctgcaggctgccgacaaggcggcaggcgccggcgacaccgagaaggcgcagcagttcaactccaccgccgaggtgctcgcctcccagctcgtctctgtggagcaggagctggcccagaccaagcaggcttacgagtctgccgagcaggcggcgcgcgaggcgcaggcgcagcagcagcagtctgaggcgcgcctacaggagcagctggcgcaagtgtcccagctggagtcgcagctgaaccaggcgaagatgcaggagcagaccgccaagacgatggactccatgcagcagttcaacaccgacgacagtgtccccaccttagacggcgtgcgcgacaagatcgagcgccgctacgcggacgcgctgggccagcaggagatctctaaaagctccatgaccgaccgcatggcggaaattcaagccaccggcaccgacatcgccgcgtcgaaccgcttggatgagatccgcgcgtcgatggcgggcgaactggagtcggcacccgtgccgcaggccgagcgcgagctggaggccggcggcgtcgaggacgcggaggcgtacctctccgagagcccagtcgcggacgaggacaacgagaaccgctagcgaaaaccgctagcggttacccgcggtggatgttgatcagcacaccgcggatgccggagtggaacccgtcgcgcaggttcacgcgctgcgtctcgctgagcgtgtactcgtgcagcgtctcgcaggcgaactgcagcagcgggcggtcaatctccggcggcaggccgccacccgagagcatgtgcgctttgtcgcgctgttccaaggttgcggcgttttcgtaccaccaagccgcgtactgctggccgacgtcgtacggcgtctggaagcctgcagacgaccacacttcctccggcagcggcacgtagcgcgagcgcagcttgcggcgcggcgccatcatcgacggcttcggtgccggcttcgggcggtccgctgtctccgggttcgtcagcgcgtggttgcctggcaggttggactcggtgttcgcctcgacctgggcctcgctcggctcgtcgtgctctgggtctgccggcgggtgggtgcgctggaactccggcgcggtgccggtcgttggcgtcgtttctgcggccgtgtcagcgtctgctccagcgctttcgatatcgtgccgctgcgcggcctcggcgaccatcgccggggtcggctgcggcgctgccggctccgccggggcttccagctcgggagactctggctgttctgcctgctcaggcaccccgggtgcctccgtctcctccggcgcgcgcagcgggtcggggccgagcccgggcaccgcagacggaccttcgtcttggcccaccggttccgcgtcgttcagcgggcgctcgcggatggtcggaggcaggggaccctcgagcacctgcagctgcatggcgtcggcgaagtcctcgcgcggatcgatgatcgtggtggagtcgcaggcgtggcgcagggcagacgacatggagtcccacccgaagccgtacaggtgcacgcgcacgcccatgtcggcggcttcctgcacgccggggatcatgtccgcgtcgccggagaccaacacgaagtcgctgaactgctggcgcgtggcgttgacgacaaggtccgccacgaggcgggtgtccacgcccttctgcgtgcggcgctcaccccactcgatgagctggcccgtgcgcagctgcacgcccgcacaggagcggaggctgcgctggtagcggtgcgggcccgaatccgggatgccgtcgtaccagtactggcggtggacaggttggttgagctggtgggtgatcatggtcccgagttccgccaccacctcgggaaggtcgatttctaactgtgcgcgggcgccgatctcccacgagttgtaaaagctcgcgagcaggtacgacgtgtcgacgaacacaagggtgcgttcaatcatggctcctaaattccgattctttttcgttactaaattgggtttctcgaaccagtctgcccgaaaccttccgcacttaccattgcgttttgctcacaacgttgttaaacagttagttactgcagtaactaaccaaacaacaacactttggaaggggggagcgcgtgaatccggacgcagagccgctctttgtgcaggttgcgcgcttcgtggaggacctgattgtcgacggcgcactcgccccgggcgaccaggcgccgtcgatgaaccagcttgcggagttccacgaaatcaacccggccaccgcacgtaaggggctttcattgcttgccgacgcccacgtaatcgaaaaacgccgcggcctcggcatgttcgtcaccccgggggcccgcgagcgcatcgtggagaaccgccgcgacgccttcgccggcgagttcatcgcaccgcttatcgacgaagcggtgcgcctcggccacacacgcgccgacctccacaatctcatcgaccgagtcgccgaaagtagaggaatgtaccaatgacacacgtcaccgcgcgcgcgctcacccgtgcatttggcaagaagcaggtgctggacggggttgactttgacctcgggccaggaatccacggccttctcggcaggaacggcgtgggcaagtccaccctgttgtcggtggttgcggggcagttgagggagagtgggggtgaggtgggcgtcgataagcaaaagccctttgacaacccggaaacaatgaaccgcacggcgctgaccggcgtcgatgtcacctacccttcgccttggagccttcgcgacatcctcggcgcggccgcgctgcgctacccgcgttgggacagcgcgctcgccgaccagctggttgccgactttggcctcgatgcggctttggctgagatctacggcaatctctcgcgcggtcagcgcgcgatgaccggcattgtggtcgggctcgcgtctggggcggagctgctgcttcttgatgagccgtacgtcggcctcgacacgcacaacacgcaggtgttttaccgccacctgcttgatcaggctggctcggggcggaccatcgtgatggccacgcaccacatcgaggacgcggcgcggatcctggagtccgccctgattctcgggcgcgacggccgcatcgccgcgcaccttcggcccggggacgcggacggctaccaggtggtcctgggcggcgagtcgaagcgcctggtgccgctaggggagcaagtgcccgcaggctcccgcgcccgcaccgccggcttcgacgatctcatcgagtcctacctggaggtgtcgtaaatgacgtggccaatcttctggcaccagttcaaagcggggccctggtggcgatttgtcgccgtcggcttgttcgccgcgtttatgtcgcttgcgccgattttcgcgagcccccttctggcgatgctcacgcccgcgatcgccgctaccttgtggttcttggtcttccttcccgataccgccttcgcgcagagctacggcctgacccgcgcgcaggcgcgccgcgtcttcgcctttggtgcggtaccagccgggctcctcgcctcggtgccggcgctgaccaggctcgacgcgggaggcgttctcggcgcggcgctcgcgtggctggtcaccgcggcgatggtgggcacttcgctgcccaacggtgagccgaagcgtcggattggaggcgagggagcgcggttcaaaggctcgtcgctggaattcccgctgttctggcgcctcccgctcgcgtggggcctgggttccgggctggccgtgggccttgccgcgtggatcggtcgcggcattggccacgagacgatccgccaggtgctcatcgccttccccgtcatcgtcatgtggttcgcgttgcttggcgcgccgggcctgcaacccgccaccgtccgcagcctcggcatgacgcgaaaggcgtgggcatcgcgctgcttcgccgtggccatcggggtcaaccttgtgttcctcgccgccgccgggagcatttggatgcttatcgacgcccccttaacccccctcgccaccaccaccgcaataagcgccgccgtggttttcgcgtcccacgcgctgatgccgacgacggagtttgttgccttcgccctgccagtcctgttcttcttcccgacgcgcatgatgctcgacccgctcgtccccgccgaccgcgacgcactgatcgcgaccgcggtactcggcgcgatcgctgtggttgcgggtctggtcgtgatggcgctctacgtggcggggcgcgtgaacgtttcgcgccgcagcgaaagcttctccggtgtgaatcagcgcgcgtaacgacgattgttgtgcatcagaaaaccgcttctgtgctgggggtttgtgttgtgttggtgtggtgtgtaacttagttcgagtcagcgagaccgacagcgccccgcgagagagtgtgaaacttcttgtggtgtggcgataagaaaacgatcgtttggcgaaaattttttactgctgcttacgcaactggctgtgtttggttggttgtggggtgtgcgtgtgttgtttgagaactcgatagtgtgccaatacttttttgtttggtgtgattgttgtgcgtgtgcgccatgatttttttgttgtggtgtgtgccggtggcagtgctgctttttctttgggtggtgctgttggacggtgggacgtgtgatggtttcactattttttgttggttgtggtttttcctcgtcggatacatgacca

SEQ ID NO: 15 - DNA, 47862 bp, Corynebacterium cassirii
  source 1..47862: mol_type = genomic DNA
gggtgtggggtttgtgggggcgtcgataagcgaaagccctggaacctgggccgcaggacgcgcagcgatggagcggcgcgggaccaccggccggccctggcgcgcgaggttgggcagcgtgccgttgcggcgtgcggcgtcgcgccaacgcacgaaggtgtcatggatcagatcgctcaatcgtgctcaccccctcctccatcgtcacagcgtagcgggcggtcacggcgtcgtcgaggttcgaaggcaggtcgtcgccgaccgctgcggtgatgagcacctgctccgccgactcggcgacggcgacgaggcgctcgcggcgtttcgcgtcgagctccgcgaaaacgtcgtccaggatcagcaccgggtccgtcccctcgctggcaagcagctggtactcggcgaggtggagcgcgagcgcatacgaccaggtctcgccgtgggacgcgtagcccttggcggggttgtcgccgagcatcaggacgaggtcgtcgcggtgcgggccggtcacggtggtgccgcggtcgatttcctcgcggcggcggcggcccagctcggcgagcatggcggcttcgaacaacgcggagtcgcggggtgcgtcggttgttgagtcagtgccgatgtcaccgatcgtggtcttgtagtgcacagacgccgggcgggattcgggcgcgacggaggcgtacgcggaggtgatgagtggggccagggcgtcgacaagctgcaaccgccccgcgatcagctgcgcaccgtgcgccgcgagctgggcatcccacacgtcgagcgtggcaagggccgccgcgcccgattcatcctggtagccgcggcgaagcgccatgttcgacgacctgagcagggcgttgcgctgccgcagcacgcgttcgtaatccatgcgcacgccgttcaagcgcggggtgcgaagcgacatcaaatcgtccaagaaacggcggcgctcagccggctcgccgacgacaagcctcaagtcctccggcgaaaacatcacgcagcgcagcacgccgagcaactcgcggggcgacttcaaacgcgtgcggtttatctgcgcctggttcgcgccggaggccttcagcagcaggtgcgtggtcagcgcacggccctcgttgaccgtggtggcggagacgcgggcgttatctgcgccgctcaaaatcagcgggccgtcgctgctcactctgtgactgcgcaggtgggcggtgtaatacaccgcctccacgatgttggttttaccgtgcccgttgcggccggcgaacactgtcgcaccgggcgcgagctccaagcgcagctccggccaagagcggaaatcgcgcaggtcgagctcggagacgtacaccgtttaacccggcagacgcaccggcatcaacaggtacgtgaagtgggtctccggcgttgggaacgtgccgtccgcgtccgcctccggcaaatcctcgggctccgggatcatgatcgcgggacgcgacgcttcggtgaagccgaacatgacgcggtcggtgccaatcacggacagaccgtcgcgcaggtagcccgcgttgaacgcgatgagcaggtcttccgcgccggtgaacgcagccgggatggtctccgacgcctcgccggaatccgcgccggacgcgtagagcgacagctcgccatcgcggaagtgcaggcggatctgcgcgtttcggtcggcgaccagcgagacgcggcggatcgattccaacagcggcgcgatctccaccgtcgcgatcgagctgtgcgctttcggcaacagcggcgcgacgttcgggaaatccgcgtccagcatgcgcgtggtggtctcccggttgccggtgtgcagaccgaacagaccctccgcgccgacgttgcccggaccgccgacggcgatctttactggctcgtcgatgtgcgtgtccagggtgcgcgcgttatccagcagcgtcttcgctgggatcagcagcttcgcctccacgtccggctgcgccggctcccactcgagggagcgcagcgccaaacggaagcggtcagtcgcggtaagtttcacgtggctgccgttgatctccatgtggataccggtaagcatgggcagcgtgtcgtcacggcccgcggcggcggcaacctgggttacggcagcgctcagcgccgccggcgcaatctggccggtgacctccggcagcgtgggcagctgcgggtagtcatcgaggctcatcagcggcagctcgaaccgcgcggatcccccgcgaagctccagcttgccgtctttcgttgtcacctcgaccggcttcggcggcatggtggccacgatgtcggagagcaacttgccggcgacagcaacgcgacccggctcatccacctctgcggcgatgcgcacgcgcgtggacacttcgtagtcgaagccggcgaattccaacccgttgtcgtcagcggtgatgacaacggcgcgcagcacgggctgggtgtttttggtcgggaggttgcgggcgacccacgcggccgccaccgacaggtcgtccttgtgaacccggaatgccaccgtgttcgtgcccgcggagcttccttccatggcgcgccggcccccttcgtcgtcgttgcaaaaacgtgtaattaccggttttcaatctagccaagcgccggaggaatttcataagcgggacgttgcttgtcgacggggcgctcacatcccctgtttctctctgaagaattacaagttaaagagttggtaactgcagtaagtcctgtggaggctgtggatgcgcccacttttttcgaggtggcggcggcgtgtcgcggtgtggtttgccctgtggataacttgtggataactccgtgtggttgtggataaacttttccctctttgaaaatcccacaaggaacccgatttcttccaccgatcatccacaacgtggggcgttgttgtccactgggggtatttgggggaatttacggaagttacaccggtgtaattacacagctgtggacaacactgtggatagtgttgccggcgccggctagcgggtgcgggcgcggttcttgattacctgcgtgagctcttgaatctcgtcgtaggtgtcgcggttttctgagatctccttgcggatcttgcggtccgcgtacatgacggtggtgtggtccttgccgccgaactcgtcgccgatcttcggcagcgagagatccgtcagttctcggcacaggtacatcgcgatttggcgtgcgtgggcgacctgcctcgtctttccggcgccggtgagttggtcgacgccgacctggaagtactcggccgcggcgtccttgatcgcgctcgcggtgattgtcacgtcgttttcgtccgggaggatgtcgcgcagcgcgacctgcgcaacttccatcgtgatcggttcgttgatcagcgacgaatacgcggaaacgcggatcagcgcaccctcgagctcacggatcgaggactcgaactgcgaagcaatcagttccagcacgtcgtggctgacgtgcgtgccgtcggcggccgccttcttcatcaagatggcgatgcgcgtttccaaatccggcggctgaatatcggtgatcaacccgccctcgaagcgggtgcgcagccggtcttccagcgtggtcagctgcctgggcgggcggtcggaagacaggatgatctgcttgttctgctggtgcagcgcgttgaaggtgtggaagaactcctcctgggttccttctttgccctcgaggaactgaatgtcatccaccatcaaaatgtccaagttgcggtagcgccgcttgaacgattcctggcggtcgtctcgcacggagttgatgtagtcgtttgtgaactcttcagaagagacgtacttaatgcgcaggcccggctgcagcacgcgggcgtaattgcccgccgcgtgcaggaggtgggtcttgccaagaccggagccgccccaaataaacagcgggttgtaggcgcgggccgggttttccgcgaccgccaccgccgcgccgttagcgaagcggttggacgagccgatgacgaagttttcgaaggtgtacttcgggttcaggctcgcctcgcggtctgggtcgtgcgccggtttctcgcgggggatgcgctgcggcggctgcaccgtggggtgcgcggtggaatttcgctgctccgcctcggtgacctgcagcgcgtgcatctgcgcaagctcgtcgagacccatgggaatttgctcgccggcgccgacgaagtgcgcgtagttgtcgttgacctggttcgcggtttgcgacgacgcccagtttgcttccgccccgcccaccgagccagccgagctttcccgggccgccggggccggagccggcgcggcaggagcttgaggcgccgcaatggagacagcgagtgtgcacggcgtgccggtgcgggattgcaaaagggcggtgatgtggggggcaagggagtcctccaccaccgttttcgcggcggcgtgcggtgcggacaaaatcgcgtaaccgttcaccagcacttccggacgcaccaactgcaggtaagcgcgttgctggtgcgtcagcgtggggacggaagagttcggacgctcagatagctgcagcaattccgacacaacttcgcgccacagcgcctcgagctgttggtccgccacacgcgctcctttcaacctcggacaatttcttcaccgtcaatcccctgtgatttccacacggggaggctgggacgtaaccgccctcacctcatgttccacaatgttgtccacacctgtggataactcggtggcgccttgttatccacagggggtggatgacttgtggataacttctgttgaatatccccaccccttctacctgcagttacgcggcatttcggggcaaagtctcaacctttagttcacattattccacaggctgtccccaccccagggtgtgacattgtgttaatgaaatcattgttaccgcgttcaacggcgcgatgtctaacacttcgctgtgcgtacccctgtggataactttccgcccgccgtcgccgccccggcgccggatgccgcgccacagcgacttcgcaggatttgccggcgtgtcggtgccgccgccgaaaaggacactcgtgtaattccgggggtgcttctgagctgggcggggaggcgtgaaagccgatttggaaccgcgggcgaaagtgacgtaatctgacagcgtctgtcacatcagtgtcgtctggtgtgcttgagagcaccgcctggagatcgggcgatgcgtgcgcatccgcaatctcaaagtaaaacttcgccgtaacggccggcctccgggccagccgttcgtacaaacgttaggagcatttccgtgtctaagcggactttccagccgaacaaccgccgccgttcccgtaagcacggcttccgcgcccgcatgcgcacccgttccggccgcgcaatcgtgtccgcgcgccgcaagaagggccgcgccaagctgagcgcgtaagcctcacgcacgtgttaccccgcccgcacaaactttccgcctcctcggatttcaaggagacgattcgaaagggtgcgcgagcggggtcttctgcgttagtggtccatgtgcgcgagcgcgacgacctcatcacccgaggaggtccgcgcttcgggctggtggtgtccaagcaggtgggcaacgccgtgaccaggcacgcggtgtcgcgcaaactgcgcgccgtcgtgatggatagcgctgtcggcgagctcgacgcgcagtgggacgtggtcatccgcgccctgccgcctgccgccgaggcgtccagcgctgagctggcggcggagtttgcttcatcgctgcagcgcgccgtccgcaaagcgaacaagcgctgatgcagtactacaacttcatgggcgatgaaattccccagccgacatcgccggcggcgaaggccgcggtggggatggtccgtggttaccaaaaatacctttctccccttaagatggggggcacctgtcgttttatgccggtatgcagcgcatatgcgctggaagccgtgtcgcggcacggtgctgtgcgcgggggcgcgatggccgttgctcgggtgtgcaagtgcggtccttggcatcccggcggattcgaccccgtgccaggcagtgtggcgaacgttgatgaggagtaaaaccgaaccgtgctgaatttcatttattggccgatctcgtgggtgctgaagttctggcacgaagtggtcggctttgtcttgccggaggattccggtgtgtcgtggctgctggcaattgtgctgctcacgttcaccgtccgtatcttcctggtccgcccgatggtcaagcagatgcgcacgacgcgcaagatgcaggaaatgcagccgcagatgcaggccatccgcgagaagtacaagaacgaccaggccaagatggccgaagagacccagaagctgtacaaggagatgggcaccaacccgctcgcctcctgcatcgtgccgttggtgcagatgccgatctttttgggcctgttccacgtgctgcgctccttcaaccgcaccgccgggccgaaccagccgggcttgagcgttgaagaaaaccgcgagattgccaactacgccttcccgccctcggatgtgcagtccttcctggacgccgactttttcggcgtgccgctatcggcttacatgtcgatgccggaggaggcgttcgccgccttcaccggtgtggagctgacccgcgcccacatcatcgcggtgtgcctgccgatggtcctggtctgtgcgctgttcacccacctcaacgcgcgcatgtcggtcaaccgccaggcggagcgccgcgcgtccggcaaggttgccgccccgcaaggcgaggccgccgcgatgatggaagcgcagatgggcatgatgaacaagatgatgctgtggttcttccccatcatgatcatcgcttcgggtgtgatctggcacgtcggccttttgacctacatgctggcgaacaacatttggaccttcttccagacgcggatcgtcttcgacaagatggacaaggaagaggcggtcgaggaggagcagaagcgcgaagccaagcgcgcatccgcaccgcaggtcggcgcccgtaccgtggacaagcgcaccaagaagcagcgcaagaaggggcagtagcttatcgacgccccgtgcaaccgcaacccccgcaaccgcgggggttgctcgcatgttggggccgtttactagagttgggtgctatgtcggattcgggagaaattgcgggcgaggtgtttggggatcgcctcgatttggccaaggcgtaccacgactcactggccaccaccgccgccgaacgcggcttcatcggccctaaggaagtcgaccgtttgtgggagcggcacatcctcaactgcgcggttatcggggaggcgttcggcgagggcatcagcgttgcggacatcggctcaggcgcgggcctgccgggcattccgctcgcgatcgcgcgcccggatttgtccgtcacgctgattgagccgctactgaagcgctcggtgtacctccgcgaggtgacccaggagctgggcctggataacgtgaccgtgatccgcggccgcgcggaggagcagcagcgcggtaacttcgacgcggtgacctcgcgcgcggtggcgccgctgggcaagcttgcggggtggtcgttgccgctggtgaagcacgggggcgtgatggtggcgatgaagggggcgtcggtaagcgacgagctccagcgcgatgagaaggagatcgcggctgccggcggcgaggacgctgaaattttcacggtcggcgcggtgcttccgcagccgacgacgctgatccggattgtgaggaggtagcccgtgactcgcgtgatcaccgttgccaaccagaagggtggcgtgggcaagacgaccacgagcgtcaacatggccgcggccctggcgaagcagggcaagaaggtcctcgtgatcgacctcgacccgcagggtaacgcgtcgacggcgctcggcgccgagcacacctcgggcacgacgtcgagctacgagatcctcatcggcgaggctggtcccaccgaggcgatgcagcccaacccggagaacgacaacctgttttgcatcccggcgacgattgacttggccggagctgagatcgagttggtgagcatggtgcgtcgcgagtatcggctgcacgacgcgatccggcgcggtttcttgaatgagaacggcttcgactacgtgttcattgactgcccgccgtcgctcggactgctcaccatcaacgccatgaccgcggtggacgaggtgatgatcccgatccagtgcgagtactacgcactcgagggcgtggggcagctgctgggcaacatcacgatgatcagggagcacctcaacgaaaacctgcacatctccgctgtgctgctgaccatgtacgacgggcgcacgaagctcgcctccgatgtggcggacgaggtgcgcggccagttcggcgaggtggtgctccgcaacgttatcccgcgctccgtgaaggtttccgaggcgccgggttacgggctgaccgtggtggactacgacgcgtcttcgcgcggtgcgctcgcctacctcgacgccgccaaggaactccaccgccgcggagactacgcgccgcacccggccactggaccgatcggcgtcagccccgaggtgtacgcccagctggatgaggcgggcgcggatatgaccgattacagcgacgagacaagcgaggagtaaaccatggcacaggaacgcaagggtggactcggccggggccttgcggcgctgatcccgtcgacgccgctgcagatggacacctccggcaagaccggcgggattggaggcggcgcttccgacatcatctttggcaagcccgacggcgggctcggtcagaagaacccgcccgcgaagaagccgaagccgtccaagggcggcgatgccccgaagggcgcgaagcagacgaagggggccccgcaacttagcggcgcgccccgcccggtcgccggcgcgcccacggttaccgccagcacggacgcggtaatgcagccggtgccggtcggcggcgcgcgttaccaagagatcccgctcggttcgatcatcccgaacccgaagcagccccgtcaggtcttcgacgaggacgaactcgctgagctggtccactccatccgggagttcgggctgctacagccgattgtggtccgcgacacccccgacgggtttgagctcatcatgggcgagcgccgctggcgcgccgcgtccaaggctggcctcaagcacatcccggcgatcgtgcgcgagacctccgatgaggacatgctccgcgacgcgttgttggagaacatccaccgcgtccagttgaaccccctcgaggaggcggccgcgtaccagcagctgctggaggagttcggggtcacccaggagcagctggctgacaagctcggccgctcgcgcccggccatcaccaacgctatccgtctgttgaacctgccggtggcggtgcagcgccgcgtggctgccggtgtgctctcggcgggccacgccagggcactgctgggcatcaagctcggcgacgacgagaaaaatgcggaggcacagggtcagctcgccgaccggatcgtggccgagggtatgtccgtccgtgccaccgaagaagccgtcacgttactaaataagaacggcactgtccccgacaagccgaagcgcgagccaatcccccagccggagtacttgaccgccgcggcagagcgtctcgcggacgagtgggacaccaaggtgtctgtcaccatgggcaagcgcaaaggcaagatcgtcgtcgagttcggcgaccgggacgactttgagcgcatcatggatctcatcggctcaggcaagtagggtgcaccccctgcggtatcgcaccgcaggggttatctatcgccgaaatacgattacatcgatgtaattaattgatggaaattgatgtaatatcgccactatgcttgaagcagacattcggcagctcatagcgcaaggcgaatcactttccgtcgctttcgctcgtcgcgcttccgcggcatacatcaacgagcgccgagtgattgaaacgatggcctgcatggccaacgccggtggcggcacgctgctgatcggggtagaccgcgatgggacggtcagcgggtgccacccgttccacggcgacgtgaccgacccggcgctgctctcctcggcggtgttccgccacacgaccccggggctgcccgtcgaagtgcgcgaggtgcgggttggcggtctgcccgttgtagcggtcacagtcgcggcgcagccgtccccggttgccacttcgtggggtgtgtaccgcacgcgccgcgtcaacgcccagggcaccccggagtgcgtgggcatggatccggcgacggtggtcacccggtaccgagacgcgaacgggatggactgggcgcaaactcccgccctcggagcggcaatcgcggacgtgagcccccgcgccgtggatgcgtaccgcggcctgctcactgatactcgactggcccagcttgataacgaggggttgatccgcgccctcggtttcctcgacgactcggatgacccagtcgcgctaggtgccatcgccctgttcggcacacccgacgcagtgcggcgctacctgccgtaccacgtgctcacggtggctgaccgcaggaagacggaaggccgcctctcccccgccacaatccgcagctccgcgccgcttgcgccaatgctggcggacctcaagcgcaacgcagataccttcgggcccgcgttcccgctggtcatcaacgcgctgacacaccgcgactacttcctgcccggcccggtgtacgtggcgttggacgacaagggggctaaagtctccagcccaggcggtgccccgcgcggcgtggacctcgccgaggcggcctccggcaacgcgagctacgccccgcgctcgctgtatctttctacggcgctggcgcgcacatcggtctccgaaggcgcaggcactgggctcgctggaatggcggggacaggtgtgtccttcgatggcagccacgaccagggcgtcaccgccagcgtcagctgggcctcggccgaggccagcgagctcgggggtaacgaggcaaaggtgctgctggcggtgcgggaagtagacggcgacggcgcgtcgagcagcgacatcgcccgggccgcgggtctgagctcgcagcaggcgtaccgcgcgctgcgcaagctggttaaccggggtctaatccggcgcaccggagagaccaggacgacccgctacctgccttaacccgacagttaggcgtgctcggcgcgcagcaggtcggagaaggtgtaggtgcctgtgggctggtcgtccatctccataaggtaaagacgcttcacggccacgacgattgcctccgcaatcgcgtcgcgctgtttggggttagtcagcacggcaacgtcgcccgggttggaaaggtagcctggcaccacttccaccgtgggcatctgcgtcatgcgcagcatgtcccaggtgcggccgtggttgcggcagttgcgcagatcagtgcgggcggcgatctcgcgctggatgaaatcggacaaggtctcccccgtcatggacgagctgccgtgctccgatccaaagtagaacgcggcggacccgttcgccttctcgtttgggtaccggtcgagtttcagcgaaatgaccacgtcggcgccgaagccgttggccaagtcggcgcgcgccttggtcgacgggttgtcaccgcgggtgcgcgagaggatggtctccatgcccgcagccaccatgcggccctcgatgcgctgggccaaatcccacaggatcgcttcctctgcgatctcgccgtacaggccctggaccgtcgtgccctggtcggcgccgccgagtgcggggtcgatcacaacgcgcttgcccgagaggtgcgggcccgcttggcgcacgtgctcgcgctcgcggatggcgtgagcggagccaccggtgatgcgccggcccaggaggctcagcgcgcgcagggtgtcagggccgcacacaccgtcgtcgtcgagaccggtgtcgagctggaagttcgccacggcttcgtgcgtgagctggccgaaccggccgtcgacgcggtgttggtagaacccgagctcgtgcagctggttctgtagctggcccacgtcgtcgcccacgaggatctggttcggctggtagctcagcacccgcgctccgagggtgtacgaggcttcacgcagctcgcgcagggtgacatcgtcgattgttccgctcggaacgatgccgcgcgactgttggaatgcgcgaagcgtttcggccaacgcttcgtcgaaaagcatctcctgcttcgagaactgccgggtgttccagtcacccaactcaccctcgtagcccttaatcaagccgatgcgggcgagtgcggagcgcacttcagccacgcgcgcgcttgaatcgcccacacgcagtgtgccgggcatgcgctccaccttccttacatcttaaaacagttggctaaacctgggcctggactcgtttgacgatctcgctcttcgggcgaagacccacgaattcgtcgaccttcttgccgtccttgaacagcagcaccgtcgggatcgacatgacctgaaacatggcgccgagcgtgcgctcgttgtccacgttgaccttggccactttcacctggttgcccatctcagccgcgatctcgtcgaggacgggtccgagcttcttgcacgggccgcaccactccgcccaaaagtccaccagcaccggcgtgccggcttcgatgacttcggacttaaacgttgcctgcgtgacatcgatcggagagttcatagtggcctatcttagttccgccagcaggctgagcgcatctaccccaccgcgaggagcggtgtgatgtgtgcgccggtgcccgttctacagcgccgcgaggtagtgctgggcgtcgagcgcggcccggcagcccgaacccgcggcggtgatcgcctgacggtaggtcttgtccactagatcgccggcggcaaacacgcccgggacgctggtgagcgtggacgggtctgccacctcgacgtagccgccctcgtccacagcgacctggccctccaagaaccccgagcgcgggtcgtggccgatggcgacgaacatggcggtggcgtcgagcacgcttcgctcgcccgtctccacgttcagcacgttcaggcccccgaccttgccgccctcatcctcgaccgactccaccaccgtgttggtgaggaactcgatcttgtcgttctcgcgggcgcgctccagcatgatcttggacgcgcggaagttctcggagcggtggatcaaggtcaccttcgagccgaacttggtgaggaaggtcgcctcctccatcgccgagtcgccgccgccgacgaccgcgatgtggtggtccttgaagaagaagccgtcgcaggtcgcgcaggtggatacgccgcggccggtgagttcagcctcgccgggcacgcccaagtggcggggtgccgcgccggtggccaggatgattgccttcgccttgtactccgtgtcgtcgacgtagaccttcttcacgtctccggagaaatctacgcggtcaaccagctccggacgtaggtcagcgccgaacttctcagcctggtcgcgcatgttggacatgaggtcggggcccatgacgccgtcctcgaagccggggaagttctccacctcagtggtgttcatcagctcgccgccgtactcgaaaccctcgaagacaagcggcgaaagttcagcgcgggcggcatagattgccgcggtgtacccggccgggccggaacccacgatgatcaagtcgtgcacgtggtcgtcggacgtcgcggtctgggcggcgccttgcgcggcggcctcgttgttgcccaggctgccgaggttgatgaatccggggttggtcatacgcatcagtgtagcgccagagccaccgcctccctggcgcggtggcggcgcgacttcaccgtgcccgggcgcacgccgagctcttcggcggcgtgctcgacgctcatcccgtagacgtccacaagcacgagggcccgctgctgcgcggccggtagctgagcgaccgcttggcgcagcgcgaggaactgctcgagtgtcgccgtcggatcgtgcgcgagtaggcggttggagtcctggtcaatcatggtgtggtcgtcgtagctcacggttcgctcgcgcttgctggccttgcgctggtggtcgagcgcggcgtttgtcacggtgcggtgcagccacgtgctcagctgcgcctccccgcggtacgtgtggagactgcggctcgcgcgcagcagcgcctcctgcacgatgtcttgcgcgtcctgctcgttgcgcgcgtagttgcgtgccacgtagtacatgcgctggcggtggcgcttcacaattaccttgaacgcgcgcgtgtcccccgcggcgtagtctgccgccagctggcggtccgtccggtgcggcatggcttccgtttccccctggttatctggtgtgcccctggtgtacccgtagaaagcatgcacgcccgccccctgctttcacagggtgcgggcgcacatctcagtggacaggcgtgccggcggagttacggcacttcgcggaagccgatcaaggacacctcgcggatcgtcgcggtgccggggccttccgcggtgccggcctcaccgccggcgtcaccgtgggcgtcgcccccggcgtcgcccacggcgacgcgcggcggcagccccagaatcaccgcatcgagccgcaggttcgccaacgtcaccgaggtgacgtcgatgttgttctgcccggcgtggaacgtgccggcggcgaacaacggcagctcctcccagttcgggccgtcggcctccacttctcccagcctgccggccggcacgccgtaaatctcgtacggcccgccttcggtcgtggcgtggatcagcaggtgttcaagggtgaacggggtggtcacaccggtcgggcgcagcagcaccgcggcgttgcgctcggtggtccacgaggtcgccttgtcaccgtcgacgatcgcctgggcatctgtgccgctttcggcgctctcaagcagctgcgccttcagcggctcgatgaccaccggcagtttcgtcgtgggcgcggcctcggtcgtctgcccgctctggatggattcggagctgacgggcgcatcgctgtcgccggagaacacgccgatgaggtaggtggtcagcgcggcgatgagaatcaccgtcatcacggctgcggcggtcagcagcgccaccgtcagcgggcggtagcgcgccgcgccgaagccgccgcgtagcgcgtccgggtccttgtccggggcgtcgcgctgcacggtgcgcaccagctggccgtcgcgggactccccctccgcgttcttctccgcagcctgagcccgcgcggcaaccgccgcctcagcgtccgtcaccgtgcccggcaggttcgcggcgcggcgcagagcgacctgaatgtcgcggaagtcctgcgcctcaatcgcctcggcgtcgaccaacgcgcgggtgttgcgggtgagctcgtccagcgccccggagttcacgttcgcggtcagcagttccagaccggaggcgaaggacgtggcgtcctttgccgcggacgagcccggaagcaccgccgggaaggcgaggcggatcttgccttcggtgtcgatgcgcaggcgctgccggttgtccaagcccagcgggatgtccgcagtgtgggccgccgcaatcgcgcccgcaagcggtgcgagtgcgttggccacggcttcggtgtgcagggtttggccgctgtcggtcacggccttcagcgagctgccgtcgatccagtcggccacgatcaacgcgccggtgcggtacgacaggatctcgatgttgtccgcgattgcggggtggcgcagctgcgccaggcggcgcgtacggcgcgccacgccggcggcgctgatcgccgcttcgcgcgggctcgccggcgccatcggggcggcaccggtggtgtcgacgaacgtcagcgctacagggcggccagtggccacctcgcgggcctgccagaagcgagcgcccgtggtcgcgccgtggtcgcggatcaggcggaaacggccgtcggacaccagcgcgcccggcacgaggcggggcccgcgcaccacgccggcggacatcggcggtggcaccggcgtggcgttgaaggtgtcggaggcgaggaactgggtggacacgtcgcgcgggtcgacctcgccagtgtcgatggcgcgctcctcgtctgggcggataaagcggcccaagcccgggatgcgggtcagcgcgcggcccaggttctgcacctcgggcaggcccgaacgagccagcaccacgccggtggcgacgacgaagaagacgccgagcagcgccacctcaagcagcatgcctaccgacggcatgcccaaccagtcccccagcatcccgggcaagtcgatgccgatcacgtcgcgcgccatccaccgggtgaagtacatgacggcgatgccggcgagggaggacgccgcggcccaagccgaggtcttcagcacggagccagcttggagcgtgcccaacttgcgccgcagcagtagcgcgccgatgacggcgccggcgatgaagccgaagccgttggcggcacccagcagcaccacgacgtgctcggcgcggttcgccacgagcggcgccagcgcgctgagcagcaccttggtggcggtgatgccggcgatgatgaaggtcggcgtccacgcctcttcgcgggcgtagaacacgcgcaggtgcagcatcaccagcgcgtaaggaatcaaagtgaacgcggcgaagctgatggtcaggccgagcgtgcgcgaagcctccggcgggaagtcgccgtaggcgaacagggcgtggccgatgtcggggcccagcgccgtcatgaacacgatgatggggatcaacgcgatgaacgtcagcttggtgcccagcgtgaggtcgcgcaccaccgcttcgtcgtcgccgtccgcggcgttgcggcttagccgcggcatgatcgcggtcagcagggtcacgccgatgatgccgtacggcacctgcagcagcatccagtgctgctggtagataaatggcgcactctcgtgcgcgttggacgcgatgcgggtggtcacgatgtagccggcctggctgatcgccacgtaggtgatgatcgccatggccatcccgccgaactgtctcagccggtcgtccaggccccacaggggtttcaagttgatgcccagcttgcgcagcgcgggcagcatgatcaggcattggaccaccacacccaacgtggtgccgaggcccagcaggagcacatgggggttgcttatcgacgccggcgccgccgcattcaaccgccccggcagagccatgtacgcgatcagcaccgcgatggacactatgttgttcgcaacaggggcccacgcgccaggccggaagtgttccttggtgttcaaaatcgccatgaagagcgagaacatgccgtagaagaagatctgcggcagcacgaggtaggcgaagctggtggcttgcaccacgttgaccttgccggcgtcgttaagaaacagccgggtcaaaagcggcgcggcggccacggcgagcaccgtcaccgcgatcatcagcgtgagcgtgagcgtgaacagctggcgcacgaaccgctcgccgcggtcagggtcctctttctccgcgcgcacgagcaccggcaccacgagtgccgtgagcaccgagccgagcacgatctcggtgatgatgttcggcagcgtgttcgctgtgttgaacgcagacgccaccgccgggcccagcgcggcgccgatcagcactgtgcggatgaagcccgtgatgcgcgagatcagcgtcgcaaccgccatcgagccggtcgcgcgcacgaccgattcgttgggcgtgccgccgtcggccgcggcgccctcgccgtcgcggccattggcggtggcgaccgccgagcgcgccacctctacggcaccctcgtcgcccatcgcggtgaccgctgcggtctcagccggcactggcggggcgatggtctcgcccttggggctggtggtcagcagcgagcggtccggctcccccggcttcgtggccgcctgggtcggcttcggcgtgcgcggcgcgggcactggtgcgggcggcgccggtgtgacgatgcggcgtcgtaaaccagcgcttggctgggactcgcccttccgggactcgtcctgtgtcacgtcctagtctccattcttggtcggtgcaggtgctcttgcgtgcgcggtgctcgcgccgtccttgccgtttggcggcgggcggacgtcgcggcgtctgcgcctgctgatgctgaacagcagcatcagcgccacgagcgccgaggcgagcgcggccaacaacccactgtgcagcgcgtgcgacgctgtgcgcacggcgatgtcgacgggccgcgagattgccggcccctggttgcccgccaggtaaagctggaggtgggtgtcgcgcgcgtcctgcggcaggtcggcggtcatctgaaccgtgaccgacccgcgggccgggatgcgcagctcgtccggcacgttgaggcgcacgccctccggcgccacgtagcggatggaggtgtcgaccggcagcggcatgccgttttgcgccacgatcagaagcgggctcgacggcgatgttctggtgtacacgttgcccggcgggatcagggtgacggcggagcgcaactcgccaagcgtcgcgcgcgaacggctcagccacgctgcggtgtgctccactgcgtcctcgtaaccctcgcgcgagcgccgcgcgggcggggagaacgccgccaggatgtcgcgccgcagcgggagggtgaagccgtagcgggtcagcgcgatcgaggggtctggcgcgaggatggtcgacaggtcggtgatgaagctggcctgctgggtggcggagaggacttcggcgtcggagtatgcggcggggtcagaaaacgccggttgcacctgcgttgcgttggctaccgcggcacccgcgggcacggtgaggtagtcggcgaatgcgactgggcttgcggcgccggcggaaatcagctcggcgagcgccccgagcagcgccgcgccgtcgtcggcggaccaggaggccggcgggttcaccagcactggttcgcgcggtggctgtccctcccaggtccacgcggactgcgcggcaacctgcacacccgaggcggcgttgacccgccgcgccaactcggaatcgtccgtgtagtcgtagcgcagccagtcggtcgagtatcccggagtctgcgggttcggccccaccgccgcccacgtcgaggcgagcgagtcctggtagctgacggacaggatgccgggcgccgcccacgcgaagcggtcggccggaaggggcgcgggttgcccggggtcggtggcggttgttgccaccgggacagaagggtccgcaacgactgaagacgacggcacgagcacgcgcacgggtgcggccggctgcggggcggcggccaaggcgggggccgccatgtcgcggcgctcaagcgcgctgccggagctgggttgcccttgcgcttccggcgcggccgcgtttgctgcggtcacggcccgttcccacgcgccgcttaagccttcggtcgggattgtggacctcgtgtggtctgcccagccgagcgcggcgaccgcgtcgtcggtgacgtaaccggcagacgggatcaccacgttgagctcgcccggtgagccgaggacgcggccgagggtaaacggcccgcgctcgatggcttcccgcaccagccaggggtcgccggtgcgcaccagcgcgttgatgtcggtgttcgcccacgggagtgcgacggtgcagccggtggcggagatgtcgcgcagcttcgccagccaggccgcggcgtcttctgccccagtgccggcctcccctgcttcggcgccgccgctgccccacgagtcgcgcaggcgcttcggctcctccaccacggccgggcgctcgtcggcgacgaggtagccccggctcatgcggtcgacggtgtcgatcagcgccgggtcgattgctgcgcagatcgcggtgcccacgcggggatccgcactggccgcgatgtagttgtctaccaactcgtccagcctgccgccgggtgcaagctcgccagcgagctcctccgaggcgaggatgagcggcggatcctctggcgcgtcccctgtctcgccggggagaatgtccacctccgcggagatcgggtacagcgcggtcatccccgcgggccgggcaccctccggcatcgggccggcgccgctgaggtggaagcgttcggtgtccagggtggcgccgtactcgtcgacaagctgcagcatcaccgggtacgtgccgcggtgcgccggcatctcgatgtcgagctcgacctcccgctcggcgccggccttcagcgcgggacccagctcgatgcgctggccgaccggggtgtactcgccgatttgggcgacggtggctgcgcgctgatcccacggggagccagtcatggggccccgcctgagcacgaccgcgagctcctccatcgtctcgtccgaggagttcgaaacacgaagtttcacgtgaaacatcgtgtttggggtggaggggttcggggtggcgtcgacaagcctgagctccgccttgtccccctctcccgggcgaatcgccgggttgacccactcgtcggcaacctgcgggttctccggatcgacggggaccggcgcggcggctgcgggcaggccggcgctggtggcggcggtgacgcttgcgccgcaaattagcgcgaccagccgcgcggcgcgtttcatcgcggggtggcccttccggcgcggcgttcctttcttgccagttcgggcatgcggtcgacggcgatgcgcgcaagtttgcgttcgtcggcgtaggcgaggcgctcaatcagttcgctcatgggcacccaggcaacttcggtgacttccgggtcctcgtcgttgagctcgccgtcgacgtagcggagcaggttgtggtgcaccgtcttgtgaatgcggacgccgtcggagacgaaccagtaatcaatggtgccgagctcgtcgaacgcctcgccgtagatgccagtctcctcccacacttcgcgctcggccgtcttccactggtgctcgccgtcctcgacgtggcccttcggcatcgaccacaacaggcgcccgcggcggtcgaggcggccaatcagcgcggcgtagatctgcgacatgtccacgtccccgccggcgttgaccgcctccgccatcccggaaaccaccagtcctccggccgaggtctcgtcgcgggtcgcgatcgaggagtcgtagcggtcggcgtactgcggacggcggcgctgctgcggcttggctcccggccggttcgactggttcttgccgccgcggcggcgccggcgctggttgcttgactggggcttgctaccctgcttcgccggcggcttggagggttgctgcttctcgccctgcggcttgccgccctgcgcgggccggcccttgccccggctgcggcggcgccgacgcttctgcggcccctgggaggtgtcccggggtgcagcgtcgcccgaggagggctgcgaggtgcggttttggtcagtcattcacctcatcgtatcgggtctcgagagaagcgcgggtatcgtgtcacgggtgagtgtttatgagctgccggaaccggatgatccgaacgcggtggcggtggtcatggggagactgcagcggggcgtcgacaagcaaaaagccctgctagaaccgttggctgccgccttcgccgagcgcggggagtccttatatcttgtgggcggcccggtgcgcgacgcgatgctgggcaaagtcggccacgacctggacttcactacctcggcgcggcctgaggtgatccgcgagattctcgacgcgtggggcgagaaaacctgggacaccggcatcgatttcggcacggtgagcgcggtgaagcacggcaaccaggtggaaatcacgacgttccgcgccgacctctacgacggtgtgtcgcgcaaccccgaggtcaccttcggcgacacgatcgagggtgacctggtgcgccgcgatttcgcgtgcaacgcgatggcgctggagcttttgcttgtcgacggccacctcaaccccaccttccacgacccctgcggcggcctcgaggacgtccttgcgcgccggctggacacgccgcaggcgccggagctgagcttctgggacgatcccctgcggatgctccgcgccgcccgcttcgtttcccagctggggttttccgtggcggaccgcgtcttcgacgcgatgcgcgacatggcggatgagatcaaccgcatcacgaaggagcgcgtgcaggccgagctggacaagctgatggccggcgcgcagccgtgggagggcattgagctgctcgtggagacgggtctggccgatcacatcctgccggagatccccgcgctgaagcttgagcgcgacgagcacatgcagcacaaagacgtctaccgccactcgctgaccgtgctgcggcaggcgacggagctcgaagactcggaggagggtcccgacctgaagctgcggtgggccgcgcttctgcacgacattggcaagcctgacacccgcgcggtgaaggagggcggcggcgtgagcttccaccaccacgaggtggtgggcgcgaaaatggcgcgcaagcgtctgaaggcgctgaagtacccgaagcacgtcatcgaggacgtggggcagctggtgtttctccacatgcgcttccacggtttcagcgagggccagtggaccgactcggccgtgcgccgctacgtcacggacgcgggcgagcttctcccccgcctgcacaagctggtgcgcgctgactccaccacgcgcaacccgaggaaggccgcgcggctgcagcgcacctacgaccacctcgaggaccgcatcgctgagctggcggaaaaggaagacttggctcgcgtccgcccggacctggacggcaacgagatcatgcagatcctggaccttaagcctggccccgaggtgggcaaggcgtggaagtacatgaaagagctgcgccttgagcgcggcgagctggaccacgacgaggccgttgcggaactgaaagcctggtgggctgcgcagcaggacggaaacgccgatgcctgagtttttctacgccgaccggttgttcaacgcgctggagcgcgaggagccggcgccgggcatgctgctggtctcctcgcccgggatgctctcccccgagttcgcccgcaccgtggtgctcatcttggaacgcgacatcgacggcaccgtcggcgtcgtgctgaaccggcgcagcgagctggcgatccacactgttatccccgagtggcacgacctcgtgtcctcaccgcgcgccctgtacattggcgggcccgtgatgccgcaggccgcggtggcggtcggggtgacaaagaacggtgtggacatcgaccaccagccccactacaccaggcttgccaacaagctggtgcacatcgatctaggcgtctcgccagaggtgatcgcggacgacattgagggcttgcgcatcttcgccggctattccggctgggacaccggccaactggaggaggagattgcgcgcggcgactggtacgtcaccccggcgctgccgtcggacgtgatcgcggccggcgcggcagatctgtggggcggcgtgatgcgccgccagcccatgccgctccccctctttgccacgtttcctgcaaaccaagaggagctctaggcggggctagggatggctgtttcacgtgaaacatcgcgcgagttacggcgcgggctgaaggacatctggctcgtcggcctcgggctgatcccgctggggttggccttcggggtgctgatgacgcagtccgggttcgcttggtggtggaccccgatcttttccgtggtgatctacgcgggctcgatggagttcgtggcgctcaacatggtgctggcgggcgctggccctgctgccgctgcggtgaccggcttcatggtgaacttccggcacattttctacgggctgacctaccccctggaaaaggtccgttctccgcttggccgcgcctatggcgcctacgcgctcacagacgaaagctacgccgtcgtctccgccttgccgaagaccgagcgcctgactggcgtgcgcatcctgacgatccaggtcgtcgttcagctgttctgggtgctgtccggcatcgtcggcgcgcttgctggagcggtgatccctccggacgtgaagggcctcgagttcgctctcaccgccctgttcatcgtcctggcgtacgaagcgtttcagtccacgcgcgatgtctccctagtggtgactgcactgctggtgggtgtgatcgcgttcctcggcttccccgcccagatgctcatcgtcgcgctcgtgacctactttgtgctgctgctggtccggttctggtcgccgcttgtcgacagcgctgtgctgtggaaggtgtaagcggtgggacttcctgccagcatcaccgcggcggcggtgtggagcgtgctcattcccgtggcgaccgtgacactcgtgctccgcgcgcttcccttcgtcttccgccgtgtgctccgcggcagcccgctgctggacttcctcgggatcaccatgcccgtgggtgtgatgacagtgttagttgtctactccatcgggggcgccgagagcgagaacgggggtatcgccgccgcgcttttggctgcggctgccacccttggtctccatgcttggcgacgctccatggccctttccatcctcgccggaacagccatctacatggtgtttgtcaactgggtgttctaggtagacggggctttgtggaagcccgtatcggcgcgggtactgaccgcgttacaccttaaattcccaggataaattgtttgctcttctacggaagcccgggttatgttggcttcgtcagaactactggcgctccattcaacttgacaaggagacaccccatgaagcgtttcaccgctgcaaccctggctgctgccacctccctcgccctggtcggcatcccggcacaggctgctgagaccgaccgctcgtccgagaccaaccgctcttcggagaccacgcgttcctcggaactggacgacagctacgtgaccggctacatctacggtggcaaggtcaaggagctcatcaccgagggctctgggttctccgcgccctacaagaagtcgtctgaaggcaagagtgtcctcgagcaggtcaattcttccactaggaacgacgccgcccgcggctacaaggtcggcaccacccacgacatcctggtcggcaccggcatcgccgctgcgatcctcgccgtcctcggcggtggcgcatgggcgttccagcagggcctgatcaagttctaaggttgccttagcaggcgcaagccaaacccccaccagattcaccgggccggtgattgtggtgggggtttcgtcgttaagcagcaatgccctagtgggggaacttcgcgctcgcttcctcccaaagcccctcgaactcttctgcggtgaggtgggtggcctcaatgccttcgatggcgccgtacgtctttgggtggggcacggtgtccatgggcacgttggcctggccgtgcacgcggccgtcgatgtagatgcctgtaatcgtttcggccgggtcgagctcgatcatgcggagcatggtgcacgcggcgtcgttgatctcctccaactcggcgatattgagcagctcgccgccgagctcggggacggagtagtggagccgaacgtaatgtttcacgtgaaacgcctttcgtgggttatgcgattgcggtgtcgctctcggcgatgcgggagacgtacgcggagcacatcaccagctgcaccatgtggtagatcatcagcgggatgatgagcacgcctagggcctcgccgccgaagatcaccgttgccatcggcaggcccgtggcaagcgatttctgggtgccgcacatctgcacagtaacgatatccgcgcggtcgaacccgattgccctcgggactgccttggtcagccagagcatcgccgccaccaagatagccgtcagcacgatgagcgacgcgatctctaggaacgtcacgttcgaccacacaccagagacgacgcccttggaaaacgcggcgtagaccaccatccagattgagccccggtccacaatcttcgttgccttggacttcgctacgtcagcgatcttcgggacgaaattgtgcgccagctggcccagcacgaacggcagcagcagctggagggcgatatcggtgaacaccgacgcgtccacctgcacgccgttgcccgcgcccatgagcaacatgacgagcagcggggtgacaatgacaccgacgagggacgacactgaggcggccacgaccgcgcccgagacgttgccgcgcgcgatgcctgtgagcgcaaccgacgattgcaccgtcgacggcaccagcgtcatgaacagcacgccctggtaaagctccgtcgacatgaacgcggtcatcggccgcagcgctagtccgatcagtgggtacacagcgaaggtgaacgcgaggatcaccagatgaaggcgccagtgcgtgaggcccttcagcgcctcctgcgtggacaggcgcgcgccgtagaggaagaagagcagcgcgatggcgactttcacggcgacgtcgaaaccgtccgcgaatcccccgcgggcgggaaaaatgaacgcgataatcgccgcgacgaagatgccgatgagcagcggatcgatttttcttaagaaaccgggcatgcaggtaattctacgaacggcccgcgtctctcgggcgtaccctcgcgagtatgagcttgaatgaacctttgactatccgatccgccaccgcgcgaaaccgcatctggctcccgccgatgtgccagtaccgctgccgcgaggaagacggcatgccgaacgactggcacatgatgcactacggggcccgcgccgccggcggcttcggtctcatcgttgctgaggcgaccgcggtggtcccggagggacgcatctccaactactgcgccggcctgtggagcgacgagcacgctgcggcgtgggcgccgatcgtggccttcgccaagtcgcagggcgccacatttggcatccagctcaaccacgccggccgcaaaggttcttcgttcgcgatgctgccgcagctggcaggccgccgcaccatcccggttgaggagggcggttggcagacggtgggcccctcccctgttcctgccggcggccacaacccgccccgcgagctcacgaccgaagaagtgcgcgctctgcccggccacttcgctgaggccgcgaagcgcgcggtgaacatcggcgtcgatttcgtggagatccactctgcccacggctacttgctgcaccagttcctctccccgttctccaacgagcgcaccgatgagtacggcggcagctgcgagaaccgcgcccgcctcctgctcgaggtcgtcgatgcggttcgcagcgcgatccccgacacgatgccactcttcgtgcgcctctccgtcagcgagtggctggaccccgagggttggacgctggaggattcgcagtggcttgccccgcagctgaaggaccacggtgtcgacctgatcgacgtgtccaccggagggaacaccaaggcaaaggtgccggttgctcccgggtaccaggtggaccacgcaaaggcggtgaaggaagccgcaggcttgccgacggccgccgtcggcctcatcaccacaccagaacaagcagacgaggtcgtggcatccggtgccgccgatgccgtcatgatcggccgcgctgcgctgcgcgactcggagtgggcgctgaacgcattgagtgaggggggcgtgcccgcagaggagctgccctacccggactcctacttccgcggttgggcctagcgaggtcggagctactcgacggtgagcgtaccgccgttgtttatcaccgacgccggctgcagcggcttctctgccgggccggtaataacggctccgtcttcgattgcgaaggtggagccgtgcttcatgcagcggacctcgtcgccctgcactttggtgatgcgagcgccctcgtgcgggcacagcgtcgagtacgcgacgtagttgcccgcagtcggctgggcaatgatgaagttgtccacgatcaccgcgctgccgacgggaacatcggtctccgcaatctctgccggggcgggcgagccgcaggcagcgaggaacgcgccggcaaaggtggtcgccgagccgagcaggaacaggcggcgggagcaggacggttgagcggtctcaggtgcgtgtgtcatggcttcaccgtagcctgtttcatggcctgaacgtatgccgtcagctccgatttcagcgcctccatgtctgttactcggcctgggttcgggtgctcgtgttccacgtgcttcgccacgatgttcgcgattgcggatccggtgatggcgccggccgcgccagcggcgatcgcatcgcggacgtgctccggcttcgaaatgccgaagccgaggagtaccggagcgccgccgaaggcgcgcacgttgtcgacgacttcgcgaagcccgtcaaccgttgcctccttgtctgcgccggtgacaccgtcgcgggagatggcgtaaatgtagccgcgcgagttcgctgcgacaccctccagagtctccttagacgccttcgccggagcgatgtaaatcgggtcgatgcccgcggcttcggcagccgcggtgaacggctgtgactcgcgcacggggacgtcgggaagcaagatgctgtcagctccggcttcgctgaacgcggtgtagaactgttctaccccgcgcacgtatgccacgttggcgtagatcaacatgccgatcgggatctccggatagcgctctcgcagtgcggagatctgctccagcgcctgatccacggtcgcgccgccgtcgagcgcgcggacgtgcgccccctggatcgcgggaccgtcggcgacaggatcagagaacggcacgccgagttcaacagcatcggcgccggcttcgatcacggtcgagatgatttccaccgcgtcctccggcgtgggatccgacagcatgatgaaggggacgaatgcgccctcaccgctgtctgcgaggcgagtgaatgtgttttcgtagcgggtcatctacttcgcctcctcggcgtgttcgggggaaccggtggtctcggtgtcggtctcggtgtcggcggcgcggagcttgcccgggatcacccagtcggtgtgctgctccagcgtctcgcgcacgtgggcgacatccttgtcgccgcggccggagagggagaccaggatgttcagcggctccgcgtctttcgggtgatcggcagcgcgctgtagcgcgtatgccagcgcgtgggaggactcgagcgccgggatgatgccctcctccttggacagcagctggaaggcgcggagcgcctcctcgtcggtgacgggtacgtaggtcgcgcggccggtgttggccaagtgcgcgtgctccgggccaacggccgggtagtccagaccggcggagatggagtaggactcctctacctgcccgtcggcgtcgcgcatcaagtaggagcgggtgccgtggaggatgcccacagtgccggcggcgatggccgccccgtgcttgccaacgccgaagccctcgccgcccggctcggcgccgacgagttccacgccctcgtcatcaataaagtcggcgaacatgccaatggcgttggatccgccgccaacgcaggcgaccacaacgtccgggagctggccgatgcgctccagcatttgggcgcgcgcctcggtggagatgacgcggtggaattctttcacaatcttcgggaacgggtgcgggcccgcagccgtgccgaggaggtagtgggactcgtggaacgttgcggtccagtcgcgcagcgcttcgttcaccgcgtccttcagcgtgccggcgccggactcgacgccgaccacctcagcgcccatgagacgcatccggtagacgttcggctcttggcgggccatgtccaccttgcccatgtagatgatgcactcgaggtcgagcagggcgcaggcgagcgcggttgcggtgccgtgctggccggcgccggtctcagcgatgatgcgcgtcttgcctatcttcttcgccaacagcgcctgaccgatcacctggttcgtcttgtgggcgccgccgtggacaagatcctcgcgcttgagaaagatgcgcgcgttcgcgccgtcgagcggcaggttgcggcactcggtgagcggggtcgggcggccgaggtagtcgcgcagcagagcgcggtactcgctcatgaactcctcgtcctccatcgcgtcgacgaaggctcgttcgagctggtcgagcgcgggcaaaagggattccggcacgaactggccgccgaactcaccgtagtaggcgggcaggatggtgctgccgccgtgagcgtaatcagacatagagtgctctttcagataatgcgggtttagtagtggaagttgccgatcgtgcggaagacgttgcggagtgcaccagcgtccttcttgcctgcccattcccctgcggtggcggggtactccacgccggagttgaggtcgacgccgaggcagccaacgcgaagggcggcttcgatgttctccgggccgatgccgccggccagcagcgagtggtgcttgacggtgtcggagacggtcgcccagtcaaaagcttcgccggtaccgccctggccggagtcgaggaccagccggtcggcgagacctgcctccgccaagaagttggcggtctcggggccctcgggcgcggtcatggagacggcgcgccagacttcagcccgtccgtcgacctcgtcgcggacccgctcgagcagggcccgttcggcctccgcgcttccctggtagggggcgtggacttggacggcgacgatgccgtcgataagcaaagccccgtagccctcgctgcggcgggataccgcgacgtagcgcagacccagttcgtggtcgatgatgtcgcgcgccgtttcacgtgaaacattgcgcgggctcccatcctcgaagatgaggccgccgtacactgcgcccgcagctttggccgcctgggccgcggtccgcgaggtgagtccgcacaccttgttcgggccgtacacgagttcgcgcacggcgaggtcgacgtctggttggctcgtgagttgtgatccgacgaggaagccgtcggagtgagcgccgagttggcgcactgtctcaacggtgcggatgccggactcggagacgacggcggcgtcggccggggcgtgggctgcgaggcgggcggagcggctgaggtcgatgcttaagtcgtggaggttgcggtggttgacgccgaagatcttggcgcccaggcgggcggcgcgctcggcttcttcttcgtcgatgatctcggtcagcacgtccatgccgagggagccggcaagggcggaaagtcgggtataggtggcatcatcaagcaccgaaagcatgagcaggattgcgtcggcgccgtagtagcgcgcggcgtagacctggacctcgtcgatgatgaagtccttgcacagtaccggcaagtgggtggtggcggcgacggtggcgaggtgatcgtagtccccgccgaagcggtcgggctcacacagcacggagatgcccgccgccaggttccgcgaccgcgagtataccgcggcgatctcccccggttcgtagtgctcgcggatcgtgccgagcgacggcgaggaggacttgcactcgaggatgaagctcgttccggggcgcttcaagttgtcgtacagcgagcgctccgatttgggtaacgtgtcgaaatcaacgtgtgctacgcgttgccggatttcgtcaaggtgacgtttccgtccctcgacgatttcttcgaggacggtggcgaggctactcactgtagtccgcctcctcgtgcgtcttcagccactgggcaaccgttccgttatcgatcagcttgcccgcgtgcgcgacgccgtccgcaatggtgttggtaatgccgtagaggtagaacatcgcgccggcggacacggcgatcgcgtcccggtgtgcgcgggggccgacgcctgcgaaggtgtctcgcatcatggcggcgttctcggcgccgtcgccgcccgcgaggtctgctagcgagtgccgggtgacgccgagctcctcgggggtcacggtgtagtgggtgatattgccctcgcggtcgagctcccacacgagcgtctcgccgtggacagcgatctcgtctgtgcccgccccgtgcacgacgagtgcgcggccgcggcccaactcacgcagggtttccgcgatcatctgcccctgcttggggttcgcgatacccatgatctggtattcgggatgcgccggcgagagcagcgggcccatggtgttgaacagcgtgggcacaccgagggccttgcgcaccggctgcacgtgcgcgaccgctgggttgtaggcgggcgcgaagaggaacgtgaagttcgaggactcgaactggcgcacggcgcgctccggatccaggtcgagcgggatgttgagcgcctcgagcacgtcagcggagccggacttcgaagacacggagcggttgccgtgcttgaccattttcacgcctccagcggccgcggtgagcgaggcggccgtggtgatgttgatcgtgttggctccatcaccgcctgtgcctgcggtgtccatgatcccctcccccgtcacggggaacggccggcccgcggcgaggaatgcgcgcgcagcaccggcggtgtcggcgaaggtttcaccccgggtgcggatcgtggccagaagggctgagatgtggacgtcgtcgtagtcgcccacggtgagcggagtgaaagcctcgatggcctcctcgagggacggctcgcggttgtccaaaaagcggcggagaatttcgagcgatgtgtcacttgccattgttcggagtcctttcttcaagcaacgtggttacgcaccgctcgagcagaatcggcccagacggcgagaggatggattcggggtggaattgcagcccgatagacatgctatcggtcgtctcggcggccatgatgacgctgccgatctcggtctcggtccacgcgagagcgcgcacgccgcccggctcgcgggtcgcgccgagagagtggtagcgcgccaccggcacgtcgatgcccggctcgcctggggtgccgccgagggtcaagccggtaaagagcgggctgtcctgcccggccggggtgagctgcatgcttatcgacgccccgtgcaccggcccacacggctcaaccgcgccaccgaagtgctcgatcagcgcctggtacccgaggcagatgccgagcagcgggattcgcccctgcgctttggcgataacctccatcatgcagccggcgtcggccgggtagccgggcccgggcgagagcacgatgaggtctggctccttctcccccgccccgccaccgaggacggtgtcggcgggcacggtgttgcggtacaccgccatctcgtggttaccgatgccgtgcagcgcgtccacgaggttatagacgaaggagtcctggttatccagcagcacgattctcatttggtcacctccagttcggcgctggcggcctgcgccagcgcgttgagcacggcgtacgccttgtgcagggtttcgtccgcctcggcctgcgggaccgagtcccggaccacgccggcgcccgcctgaacgaccgctgtttcacgtgaaacataggcggaacggataacaatgcaggtatcgaagtcgcccgtgccgtgcaggtacccgacggcgccgccgtacgagccgcggcgggttccctccgcctcgcggagcagctccgtggcccgcagcttgggcgcgccggtaagcgtgcccatgttcatgcaggcgcggtaggcatcgagggagtcaaggtcgtctgcaagcgtcgccgtgacccggctgacgaggtgcatgacgcgcgagtagcggtccacctgaagcagctccgccaccttgcgggtacccggcttggccacgcgggcgaggtcgttgcgggcgagatccaccagcatggtgtgctctgcaacctcctttgcgtccgtgcgcagttgcagttccatccgggtgtccagctcgtggttgacggtcccgtcggcgttcaacccgcgcggccgggtgcccgcgatcgggtacagctgcacttcgcgtgtcgccgcgtcgaacttcaggttggattccggcgacgcgccaaagagctggtacggctcgcccgccctgtcaacgccgcggacgtagaacatgtacggcgaggggttggtcgcgcgcaggcgccggtacgcggcaaacgcgtccgcgcactcggcctcgaaggcccgcgcaggcaccacttggtagatgtcgccgttgtagatggaagctttcagcttgtcgacgctcccacaaaactccctgtcccccacatcagcccgagttacaagcgtcccggcgccgcccccggcagacgagtaggcgtgggtgttgtcggggtcggctgcgtcaatcgccgcagcgagttcgtcgagatcgatcccgtcgcccgcggcgtccacgccggcgaggtacgccgtctgggcttggtggtcgacgcgcagcagcacttctgcgaggacgaattggtagtcggggtacgtgttcgggccgtcctcaaccgcgggcagcgtctcgaaggtttcgaggtagtcgaacgcgaagccgccggccagcatcgggaaatcctcgttgctgtagtccgcacttgtggtcagcgcccgcagcacctccaccgacgatgtggcggtgagccgctcgcgctcgtcctcggcgcgagaggcgggaaactcgtaagcgtgctcccccgctgcgtactcagtgagttgctgggcggcgcgggcagcgagtacctcgcccgaggcggtgaacggctccaccgttacccgcgtgccgttgcatgtcacgcgcagcgacgccttgagcaccgcaagcgaatgcagccccgacttggtggtgatatcggcggactctaaaagcaccgaatcggtctcgtctaatccgccgaggtgcgcgaagaggctggagacgtcctcgtggtagcgcacctcgcggcgcgtgaaccgtggtggtggtgggttgctcatctgttgtccttggttttgttctgtgcaccgagggtatgtagagcaaaggcccgcggtgcttggtttgaatcaagctggcgggccggagaatgtatgagagattgttgcagactcatggcacgccgtctacgcgcgccaccaccagatgctgagttgggtgttgaaacgagtcacggatcacagcgtagcagtaactacgcctcgccgtctgctttacttgcagcgttgcgcagcgcgtccagatccacggcggggctgggtgcgggttcggcggtggtggagttctgggctgcgtcgacaagcagcgctgccctggcgccgaagttccctcccaccgacagcgcaataactgccgcaaccagcgcgataaccggcgcaatccacacccagccgtgcgcgatgaacgcgaacgctgcgccgatggccatggcgaggccggtgaggacccagaacgggccgacgacacggtgcgcctggacccacgtggattcgttcttccgcacctcgggcacgcgcaggccgatcacagtgttgccggggagtttgccggcggttgccatgccgccagtgacgaggaagaagatcgccgcgagcaaaaagatgataccgaggaccacgttgagggtggtcgtagtggcaaatgggctcatagcaaccagcataaaccgggcggggtgaccaataaaattctccaataattcctcgattggcccatccgtgggggaaaatggtcttgcaattcccgttccactagtgaaggtcttccggtatgaaatcgaaactcctgaactcgctgctgttctggatcgtggtcgccatcatcggcggctggttgtgcagcttgtttttccccgcctggctggcgcgcgtcttcgtcacgttcaacggcctgttctccaacttcctcggcttcttcgtgccggtgctcatcttcggtctcatcgcgcctgcgatcgcgggtcttggccaaggcgcgggtaagtggctgggggctacggccggcattgcctatggctccacggttatctccggcctgattgcgtggggtacggcttcggcgctgtacccgaggcttcttgacggccgaaccctcatcaccaacgtggacgacccggaagctggcggcctcgccccctacttcaccgttgagatgcccgcgccgttcgcggttatgtctgcgctgctgctcgcctttgtggtgggcttggccatgacggcggtgaaatccgacaacatgtacgcgctgctgcaggagctcaacgaggtgatcctgaaagtggtcaccagcttcgtcattccgctgctgccgatctacatcttcggcaccttcctgaacctgggcatgaacgaaaacttcggctccacgatggcggccttcggcacggtgctggtgctctccatcgtcatgacgctcgtcatcatcctgctgcagtacctcgtggcaggtgccgtggctggcgtgaacccgttcaccgcgctgaagaacatggcgccggcgtacttcaccgcgctgggtacctcctcctccgccgcgaccatcccggtcacctacgcctccactttgaagaacaaggtggacgaggatgtcgccggtttcgtggttccgctctgcgcaaccatccacctctccgggtcgatgatgaagatcaccctgtacgcgctcgcgatcgtgttcatgggcaacttggacgttggccctggagagattatcggcttcgtgctgctgctgggcatcatgatgatcgccgcgccgggcgtcccaggtggcgcgatcatggcagctgttggcttgctgcaggcgaacctgggcttcgacgagtccatggtctccctcatgatcgccgcctacatcgtggtcgactccttcggtaccgctgcgaacgtcaccggcgacggtgccatcgcgctgatcgtgaacaagttcgcgtccggcaagatctccggtaatgtttcacgtgaaacggagggtgctgcctctgagggttccaccgtcgtgcgctaaccaagcgttggatctttagatcaccactccccgatcgcgggctgagcaatcagccgcggcggggagcttttctttggcctcagtgcacgtcacttagccgtcactgtgtcctcactgtaaaaatcgggtcgtcactatggaaagtgatgctctcagtgaacgaagtgacgccaaatcaggtctgtcactgtaaaagtgacgtcttcactgaagaatctcactatagtgacggtgtgagtgaacgcatggagcgcatcatggaacgcctcaaccgtcagggagacgacgaccattgcgttgaggccaagagtggcacgggcaaactggacaagggattttggagtacggtgagcgccttcgcgaacactcgcggcggcatcatcgtcctaggtgtctctgaagatcagcagcgtggaacgttccatatcagccggattttgattatcgtcgcgcggcggatcgggtcgaggacgcgttccgcccatctagagaagatcccggcgtcactccgatgccgcggacggagattgaggccgacgagtttgaagaccagccggtcattgtgatcacggtgcatccgatgcgggatgacccgaagctcggtaagcagatgccgtgcttcgtaacgtcgcaaggcccgcgcaacggttcgtacaagcgggtgctggacggcgatcagaggttgtcctcatacgaaatcttccaactgtcgtcgttgtttgagacagacgtagcggagctggccacgccgccactggctgcagtcgacgatctcgaaaggtctgcctgggttgctttattggattcgtttgtgaagtccggatcccgtctgatgtacggcactcggaatgacactgaagcgctggagcgtctccatgttgtcgatgctgagggcaagccgacgttggctgggctcctagcgcttggaacatatccgcagcagttctacccgcagctcttcatcgacgttgcggtgcacccgatgactgagaaatcggccagcgaagtgcggttcctggaccgtaagcagtgcgacggcccgctgccgattgccgttgaaactgcaatccagacggtgatggcgaacttgcggactcgggcggtggaacgagattcggtgatggtcgatgaaccggagattccggagatcgcgatccgcgaagctgtggtcaacgcagtaatgcaccgcgactacaaccctcaggtgcagggcaggcaagtgcagatcgacatctaccccgacagggtggagatcaacaacccgggcggtctctggggcgatcgcactgtggagaatttggacgaaaaccgctcgacgacgcgcaaccctgcgctcgctaacctcttgagccacctcccgtcgccaggggggtcatcccgtgttgcggaaaaccagggcagcggcatccagcgaatgaagctcggtatgcagcaccagggacttccccaaccgttgtttaccgccactatcagtgatttcaccgtcacactgtttcgtttcggcctcctgactcccgagatcgccgcgtggttagaatctgtcgctcctgacgccacacgcgaggagcacattgttctggcgattgcgcacggtttaggggccgtatccgttcgagagctgaagaacaacattggtctggatagcaatgacgcgagagaggtgctcaacggtctcgtcgataagcacattctggctccggcgggagaaacggactccttcacctttcaatcgacgcgaacggcgggggctgatgaggaaatctcgaggctgctggctgatggggttgagttgtccgcccgagagattgcggaggcacttggtatcaccctcggaagtcttcgaccccgtttacgcaaactcatcgatgcaggcgagatttctccaactgccccgcccacgagccggaatcgcaggtatcggctagcaaagtaactaacccgctacgctagcctccatggcttttgagatcgtttccaaccacttcgtcgcacacgaggaggacctcgacgacgcgtacgagctcttccgcgctcgcgtaagcgcgagccgcgccgaggtggttgcgatctcgccccggccccacccgatcgagagcgacttcttcctgtgggacctgcggtgcgaagcggcgtacgcgaacatgcccgccccggagacgatgaacctctacgagctgaacgcgctggttgatttcgtggtagcggaccgggacgaagccatggaggacttcttcttcgaaggccctgctgatcccacccgctacccgtcgaccctcggcggcatctcggagctcgaggtccgcgacggcatcgagggcgagctctccctcatcaccgttgtgtacctcggcacggaaaccaacgaggcggtggcacagcagcttttcagcgcactgcttgccgacgtcaacgccgtcgccttccaccccaccatctccgagatggagagcacggagcaggcgaagtggatcgggccgctgtgggttcgcgacgcgacgctgaacatcatcggcaagggcgacggcatattctcccccggcaagactgcctgggcggggtggttcctcacctctgaggcgctggagagcgtcgaggcgaagctgaccgagcgcattgacgagcaagccgtggtgctcgcccgggcggtcgcggagccgttctaggcggctccgtctagtccaccccggcctagtccaccccgagctgctctccaagcggccccgcgatcacgagccgaatgaggtagatcgcgaaggccggcacaaagaagaacgtcagcggcaccgcccacgcgatgggcaacgccacgatgacggcggcagcggcgacgaggatcgcgactgctagaacggtgcggccgaggaagcggaacgccatcagcgtggccgcggtgaagtagtccgcaaacccacggtcctcaccgcggtcctcaccgcgggtggaggcgagcccgaagaaccagacgctgatgccggcgatgatgaacgcacccgagagcgcaagcgcctgaatgaccgtgagcgcggcgccgcccacgccggcttggaaaacgacgaactgttggtagaccaacagcgcgctgaggactgcgaagagaccccagaaaagggacaccggcttccaccgcaacgtgagctcccggaagaactgcaagtggtagcgcgacccaatgccggcggccatatcgcgtgcgacggcgctggcggcacgcacagcggcgcccaccgtcacaattggcaagcagctgaccaccaaaagcatgttgagaatgacaatgtccgccatcaaggtgatggcggacatgaaccgagagtcagggtgcagcacccgatagagcctagcccttcacggcaccagcggcgacaccttccacgatgtgcttctgggcggacatgtagaagataacgatcgggatgatcgccagcaccagcatggccatcatggcgcccatgtcgcggttgccctgggagccgacgaactgctggatcacgaccgggatcgtgcggtacggggtggacaggccgatgaccaggtacggcagcaggtagtcgttccacacccacatggcgttcaggatcgccaccgtaatcgcggtgggtttcagcatcggcagcaccacgcggaagaaggtggtcagcggcgagcagccgtcgataaccgcggcttcctcgatctcaagcgggatcgacttcacaaaaccagcgaacatgaacacgctcaagccggcgccgaagcccatgtagagcacgaccatgccgagcgggttgtccaggctcaggcggtcggcgatggccacggtcggaaacatcaccatctggaacgggataaccatggagaagacgaacaggtagtacagcagcgccgtccaccacgtcttcacgcgggtgatgtagtacgccgtcatggagctgaagaacacaatcgcggcgaccgagaggatcgtgatcacgaacgaccagacgatcgccatgccgaaaccttcgccctggatgccggtgatgtagttctcgaacccggcccacatgtctcccagcgggagtgcgaacggattgttcgagatggagaacttctgcttgaaggagttcagcaggataaagaagatcgggcccaagaacacgacggtgaggaagaccagcaccgcgtaaatgagcaccttcgcgccgccggagacgcgcgcctgggaggcagctgcggcggactcgcgcttacggtcgcgcttcgaggtgccgaaaacttccgcctcggtgtcggtatccgcgtcgagcgcgagatccgaagtcccgctgcgcgacgcctcggtgtccacgcccaccttgccctcgttggggcctggtgtggagttcatcgatgggttgatacggctagtcatggtttctacgcctccacttccctgctgcgggtagcgcgcagctggaacattgcgatgacaacgacgaccacgacgaagatcacggccttcgcttgacccacgccttccacgccgacgcggttaaacatggtgttgacgatgttgagcgccaccatctcggtctgcccgcctggggcaccgttggtcagcgccaggttctggtcgaacagcttgaacgtgttcgacagggtgaggaacaagcagatggtgatcgacggcatgatcatcgggatggtcacgtggcgcagcatctcccagcgggagacgccgtcgagctcggcggcctcgatcagctccggcgggacgttctgcaggcccgcgatgtagatgatcatcatgtagcccaccagctgccagttcagaaggatgatcaggccggcgaagccgtacttccagtcggacacgatggtggtgccgtagcgggccagcaccgcgttgatcatggactgccaggtgtagcccaacacgatgccgccgatgaggttcggcatgaagaagatcgtgcggaagaagttggtgcccttcagcttgcgggtgagcacccaggcgatggcgaacgcgaagacgttcaccgtgatgatggagacgatggacaccagcgcggtgaacccgaacgagcggacgaatccctcgcgggcgctaaacgcttgtgcgtagttgtctaggcccacccaggtggcgttggtgatcgtcgtgaacttggtgaacgagagcaagaagcccatgacgaacgggaccaagaacgcgatcagaaacgcgatcagggtgggcagcacaaagattgggaagtacttcttcaaagattgctgcatcgggtgcctctttcggaaaaacgcgaagcacacggtcgcctactcggcgatcgtgcgctccgcgttcgtattcatttcggtgcgtataagcgacttagttggtgcgcttctcagccttccagtcctcgacgaacttggccactacatcatcccactccatgttcccgcttgcatactgcgcaaggttgccgccgaagaggtccttgaactgctgggaggggaagtactggaagtcccacgggatggtggtgacggaatcgtcagagatcgctgcctggacctgcttcgccagcgggtcagccgggacgtcggtctcggagtagttcttaaacggggcgatgaagccgaggtcgttgatcacgtgctccttgcccttctccgaggtgaacagccaatccaggaagtccttggacgcctgctggtcctcctcggaggcttccgagttcacggcgaagtagttctcggtgcccacgttgatgccggtgttttcctcgtccggcaggcccatgtacatcgggaggaacttgatcttgtcctcctcgaccacgttgccgttgacgtcggcgatctggctccacgcccagttaccgttctgcaccatggctgcctggccaagcgcaaactcagccatggaatcggacacagccttggacggtgccaaagacggctccacggtggagttctgcaggtagagatcgaagaggttcttgaactcctcgttgtactcgaaggtcacgtcggcggtgttcgggtcgccgatgttctcgaactcgtagtgcatcgggccgttggccaggtgggtctgccagcgccagtcctcaccggaggtgagggaggtggaggcaaacgcgccgtcgatacccagctcgtccttcttcgcctgcatgccctcggccagcttcttcagcgactcaaagttcttcacctggtcgatggaggtgatctcggcgcccggcagcgcgaagtacttgtccaggatctcctcgttgtagaggatgccgaagccttcaacggcgaacggaacgccgcgaacggagccgtcctcgccggtgagcggggtgacgtcctcgttgagctgcttggccacctcggtgtcggagaggtcggtggtgtagtccttccaggtgtcgaagccggtcgggccgttcatctggaacagggtcggggcgtccgacttggacacctcagtacgaagcgtctgctcgtacttgccggatgccgcggtgaccaccttgaccggcacgccggtctcctcggtgtactcctgggcaatctgctggtaggcagcgtcctgctccggcttgaagttgaggaagtagacgctgggaccgtcttcgccaccgctgccgccgcaggcggtgaggctggtcgcggtcagtgctgccacggcggtggtggccagcacgcgggaaaacttgcgcatgagcaatccttctactcggaaaagtaacaactttcattctagtgacgtgtgcacaactgacaaaacggtgtgagcgtgatcactcccccgcctcgttgggcaggcggtacaccatcgcctcgtcccggcggctgggcagcacccagtcgaagtaggactccgcggcttccgccagcggcacaaagcgccggtcgttctggctcataaaccagcggtggtccaggatctcgtggaagatctgcgccggctccagcttttcgcgcagctcctccggcaccaggctgaccaccggctcgtactctttcaccatccagcggtgcgcgacggcttccaaaggcagcttgccgccgtagcgcacggagcggtagacctccatctcgcccagcaaccgctgcgcctggcggtcctgcacgtccaaaccggtcagggccatcagcttgcggcggttgaagccggtggagaacaccgccggctcgatgcgaacgtggtggacgccgtcgcgggtggtgatctcggtttctccgacgtcgaagccgagctcgttgatgcggcgcacccgctccgcgatcgcgtcgaaggcgtggctgtcctcggccaccagctcgccggtcatgagttcccacaggtcgaggtagttgcgctcgatgtcgttgccgagcgcgatgacgtcctcgtccgcgccgatcagccctccggactggaggtccatcaactccccgatgatattgacgcgggctacgtcgacgtcgtaaagcctgcgcccctcggacagcggctcgtggaactcgcctgtttccgcgtccaccaggtaggcggagaactcgtcggcgtcgcggcgaaacagcgtgttggacagcgacacgtcgccccagtagaagttcagcaggtgcaggcgaaccaggagcacggccagtgcgcgcaccagcttggtcacggtgtccggggagagcacgcgggagaacacgtcgcggtacggcagcgagaaacgcaggtgctcggtgaccaggcaggcggtgagcggctcgcccgcggcatcggtgcggtgcgtgatcaccgccaccggctcaacgcagggcgcgtcgagctccttcagccgccgcagcatgcggtactcgtggtacgcgacctcctcgccgatctctttgacggcaaacaccagcccgtccgccgagattaggcgcacagtgtggcgcgagatgccgcgcggcagggccgcaagcaggtcgccgctccactgctcaaggggtagcgaccacggcatcttcagcagcgtgggtgcgtactgcggggaaacaacgttgagtttttccacctaggccgccgcctagatgcggttgccggtcgccttggagaaggcgtgcaggccgccgtccttgatgcggacgtggataacgtcgccctcgcgcgcgccggacaaaggtggggtgcgcacgacgatctggcccgcatccgactcgtcgcggcccgccgcgcgccagctgccgccggccaggtggccgtagacgtaggagtcggagccgagctcctcaacgaagtcgacttccaccgggatggtgtgctcctgggaggccaccgcgccgtccacaagctcaagtgcctcgggcctaaaaccaagaatgacctgcccgttgtcttcgggggtgatggcggccaaggtgtcttggctaagcggaatgctggcctcaccgatgcgcgcggccttcgatgcggcgtcgacgtcgaaggtggacaggttcatcgccggggagccgatgaagccggcgacgaagacgttgtccgggtggtcgtacagctcgcgcggggtgcccacctgctgcagcacgccgaagttcaacacggcgatgcggtcgcccatggtcagcgcctcggtctggtcgtgcgtgacgtagatcgtggtcacgcccatgcggcgctgcaggttggcgatctgggtgcgggtctgcacgcgcagctttgcatccaggttggacagcggctcatccattagaaacacctgcggttcgcgaacaatggcgcggcccatggccacacgctggcgctggccgccggacagggccttcggcttgcggtccaggtactgggtcaggtcgagcgtctgcgccgcttcctccacgcggcggttgatctccgccttgtccatgccggcgatcttcagcgcgaagccgatgttctcgcgcacggtcatgtgcgggtacagggcgtagttctggaacaccatggcgatgtcgcggtccttcgggctcgcgttggtcacgtcgcggtccccgatcaggatgcggccttcgttggtctcctccaggcccgcgagcatgcgcagcgcagtcgacttgccggagcccgacgggccgaccagcacgaggaactcgccgtcggcgatgtcgaggttgagccggtccacgctcggcttgtccgcgccggggtagatgcgggtggcctgctcataggtcacagatgccatgatgttctcctccatcggcaggtacgtgccgaacgatccgtagtggggttgtacagcttgaacgtagcacgggtggcaacaggacaagttgcttatcgacgctcccttcaatccctcccccgccgccgtactatgaacccatgtctgaagcttccaacggaaatgtagacaagggctaccgcggatcccggagcacgccgctgaaggactgggccgcggtgatcgggatgacggcgcttgcgaccgtgggcgccggcgcgctcgggcacacgcttcctgacgtgccggagcctgcggcaatcgccacgcaggcccaggccccgcacgtggagatctccgacccgagcgacgtagtcagcccggaagacgaggagcgcatggtgcgcgacgccgagcgcctgccgcacccggaagtggtcacgaagctgcactacatcacgcttgccgaggggcgcgacaacgtcaacgactcggtagaaaacttcctgcgcgaccactacccagacgagatcggcgacgacacgttcgcggacggagtgctaatcatcggcaccgatgttgagggacgaaacaacttcatcttcgccggcgaggacgtggcgagcgagctctacctgcgctccggtcagcgcttggagtccgcgctcgaggcgatgaaaccggggttgcgcgacaacaacctgccgggcggctacttcgccggcgccgacatggcgttggatactgagagcgcccagaactacccggtggaggacggggagaccgatcaggccttagcggcgatcatcggcggcatcgtcggcggcggcgcaaccttaatcggcggctccgttgccgcgtcgcgccgcggtaagcgccgcaaggccattgcgcaggcgcgcaccgaccacgagctgatcggcgccgactacacgggtctgtcgcagcggttggacgagctggacatccgcgcgaactccgtctccagcgcgttcgccaacgccgagctgcgcaagcagtgggaggaggtgcgcgaccgcttcctgagcatgcacgacgcgatgcagctggaggtgggcaccgaccgccaagcgtgggagaaccacaagcagctcgcccagtacgccgagaccgtgcaagacgccggcaacgcggaggagaacatcaaccgcctcttcgccgtggagcagggcgacgcagcggagcgccgcgtgatcatcaccgaggtccgcgccgacgtgattcaggcgcgccgcaaagtgaaggacaaggagctcaagcgggacctggcagagctggaacgcagcctggactacctggaccagaatccggactacccgcagttcgtcgaccagttcacccgcatcttgggcgactacacgctggtgctcgaggagatcaagcgccgcgagttctccgacgtgaaggagtacaacgcactgcaacagccgcgcctgacggacccagacttcatctacgtcaactacgtgccgtacgcgacgatgaactcgtggcacgcgtccaacgtggcggcgcaccaggccgcgcaggcgcagagctcctcgtccagcgcgaacacgggcttcagctccgggttctccggcgcgggcgggtcgagctcgtactagttcgagcgagctcctacgagctgagaagggggcccgaaaagggggcgaggccctcccgcctacttgcgctctaaatggggg

SEQ ID NO: 16 - DNA, 45353 bp, Corynebacterium cassirii
  source 1..45353: mol_type = genomic DNA
cccccaccacctccgcccccacctcctcggtggtgaccacgtccacatcgagcacggcacttcgcgcgctcaccgcctccgacgtcgtccacttctgccgcaaagacttcatcgctgaactcgacgcaaaccggatcggccacaacgacgtggtcatctccgagggcgatatcgacaacgcggacctcacctcagacagctacttcggtctcatccccgccaccgtgaagacggacgccggtccgtacgaggtgcagatgagctgcgacatcgacgtggcgaaagattcggtcgttgcagagctcgtcggcatcgtctcgatgcccgagcaggcggtcacgtcagccccgcccacaaccgcaccgccggcggcgcaggctcggccgacaaaccaggcccccgccgagaaaagccgccgcgacaacctcggcatctactaccacaacttccccgactaccgctggctaagcaacccaggcaagatcgtgccgggcgggctcatgtacaaaattcagccgaacggtgaggcgtattcgtgttcgatgggctggatggcgtatcggggcgagaccccgtatatcgtcaccgccggacactgtggcgaacccggcgaggtgatgtatatccccggcccgaacggcggcatcgagatcgggcgtatcgtggcgtcgcaatacgagagattcaacaacggcgaattctcacgcgattacggcctaattgaaatcaccgatccatccctcgtcgacccctacctgcccacgggcgaagagatcaagggctggcgcacacccgagtgggccgaggcgaacgggtacgcgatctgcaaactcggcgccacctttgggtactcgtgcggcgagtttatctcgatggagcgagacggccagttctccttccgaggttacggcgagcgcggcgactccggcggaccggtgtgggcacgcaccccggagggagatgcctacgcgatcggggtcttctccaacctgaacgactactccaagattggcctcggcgcgatgagcatcgaggaagtcatggacggtgtcggactcaccctctgggcctacaacaactagaaacaactaggccttgcgcatgcgcaccaagttggcgcgcgcggtgacctccatcgtctcaggaagggaggcgaggcgctcggcgagcgtctccgggtccacgtggcgcgcggacgggctcatgcccacctgcgcggcgatcgcctggcgctcgagctgcatcgggaattcgatgagctgcggctcaccaacgatttccaagtggcctgacgcctgctccagcatccgttcgagcttgccgtcttccacgcccaggatgccaaggggctctcgcaactcgtcgaggtggcctttgtcggcggtgagaatgacggcctcgccgccgtccgcaagcacgcgcgcgaactcggcggggttgcggggggcgaagatgacggtgagggcgttcacggtggcgtcgataagcggaatgccctcccacacatccgcaaccaccgccccaaccatcgggtgcgccttggccaggtgcttggccgccggcacggagatgtccaggccgacaccgcgcgcgccctcgatcgaatccagcgtgtgcgcgaggtagtaaccggtgccggcgccgacctcgaggaccaccggggattccacagccgcagcgtcgacgacgtcctccaccgcagcggaaaccgcctcgacgaacggcgcgaagtaaccctgcgacagaaacgcctcgcgcgactgcaccatctcgagcgaatcaccgtcgtggttcagccccttgccgcccgcgagggtgacgtagccctggcgcgcgacgtcgtacgagtgacccgtcgcggagaccaggcgggtgaaatcgtcggcgccggtcagcggcgagcggtcaaccgggtcggcgagaacgtccacgatatctttcagcatgcgctgatcgtaccccaccaaagaaaaaaccccgctgggcggggcgatggggcgaaaacgggttacttgctggcgtccaaaagcagctggcccagctcgccggcctcttccttgctcatttccactacaagacgcccgccgccgtcggacgggatgcgcattacaatctttcggctttcctcgacggcctccatcgggccgttaccggtgcgcggtttcattgctgccatgcgtcgcttctccttcaagcagaacagtttcttccggcaattctacgctctcgtcgcgctcagcgtcaccggtcaattgcgcgatcagcgcgtcgacctgatccatgcggtagccgcggtggacgacctcgagctggatgtcgtcgaagcggccctcctcaacggcctcccggttcgcggctttcacgttcgcggtgtcctccatagcgggcagcgcctcgccgcggccgaagatggcggagaacaaaagcatcccgagcatgctgaacaggatgagcgcgaggatgagcacgagccaagaaaacatggcgctattttacccacggctcgcgctgcgccaccggctcgaccccgggcggcagcgcaccggcgcgggtgagcacggtacgcgcgacgatgtcggccatcggcccgagctgcgcaagcgggcggttgcggtgggtgcggcggccgaggtcgacttgggtgatggcgttggggtggagggaggcgacgtcgataagcaagcccacctcaaccccgtaccctgcgacgaacggcaccttcagcgcggtgctgcggcgaatcgcgtactcccccgccagcggctggtccagcgcggcgagctgcgggaagtacgtgcgcagaagcggtttcgcggtcagctcggtcacgcgcccgccggcgccgtcgcgggtgtagctggctttgaccaggtggatggccgggtctgcgaacggctcggcgagcttgtccacccaccacggctcggcgttggtgacatccgcgtccacgaagaccactacctcgcccgacgccgctttgacaccgcgccacagcgcctcccccttgcccggcaggggcaattgcttatcgacgtcccgccatcccaccacccgcgcccccgccgcgcgcgcgtttccggcagtcgcatcggtggagtcggaatcgatgacgatcacctcgtcggtgttcgatgcgaggcaggcgcgcgccacgtctgccacggttttctcctcgttcagcgcgggaatcaccacgctgactgtgtggccggcgatcacgcaagcccccggactgtgttaattggggcggctgagccgtcgatggcggcgaccatgcggatcacgtcgacggtttcccgcacctggtgaacgcggaaggccgccacgccgtgggctgcggcccaggcagtagcggcgagcgttccggcgacgcgttcgtccacgccgcggccgaccgtttcgcccacgaagtccttgttcgacaaagccatcagcaccggccagccggtggcgacgagctcgtcgacgcggcgcagaatctcaaggccgtggaaggtgttcttgccgaagtcgtgcgcagggtcaatgaaaatcttcgcctcgtcggcgccgaggtcggcggctcgttcggcgagcgcggtggtctgcgcgatgacgtcttccaccacgtcgtcgtagcgcacgcggtgcggccgggtgcggggaaccgcgccaccggtgtgcgagcagacgtagccgacgcggttggcgccggcgacctcgatgagctcggggtcgtagcccgcccacgtgtcgttgatcaggtccgcgccggcgtcaacggcggcctgcgccacgggcgcgcgccacgtgtccgcgctgatgacgatgtccgggtgcgcatcgcgcacggcggcgatgacggggacgatgcgctcgatctcctcttgctcgtcgacgttgtcgccgggtccggctttgaccccgccgacgtcgataatcgaagccccgtcggcaaccgcctgccgcgcccgctcgactgccttgtccaccgcgaacgtcgcgccgcggtcgtagaaggaatcgggcgtgcggttgacaatcgccattacgctcgcgagcgggctacccatcgtcgcgcaggctggccaggcgctggtccgtcatcaccttgtgcgcctcgacgatgtggctcacggcctcgtcgacggagtcggtgacgatgaacaactcgtcgtcgccctccgaaatcaggcggcgcgcgagctgctgagagcggatccagtcgaccagcccggaccagaagtcggtgcccatgagcacgatcggaaagttggtgaccttgcccgtctgcaccatgcacagcacctcgaagacttcgtccatggtgccgaaaccgccgggcagcgaaatgaacgcctgcgagtacttcagaaacatcgtcttgcgggcgaagaagtagcggaaatttagaccgaggtcgacccagtcgttgaggccctgctcgaacggcagctcgatgcccaagcccacagagacgccgccggcctcgtgcgcgccgcggttcgggccctccatcagccccgggccgccgccggtgatcacggcgtagccggcctcggtgagcgcctggccgacgttgcgcgccatctcgtactcggcagtgccctcgccgaggcgcgccgagccgaacacggtgactgccttcggcagctgcgacagcgcgtcgaagcctgcgacgaactcggactggatgcgcatcacgcgccacgggtcctcgtgcttccacgcgtcgtcggtttggcccagcgactccagcaggcgctggtcgtgcgtgctcggctgatgctggtcctcgctgcggaccatcagcgggccgcgcagcttgcggtcgcgctcggggcgaggggtgatgtggggggccaatgtgttctcgcttcctatttcgccgtgaggtagtccatgagctgcgcgtagacgtgctcgatctggtccaccgggcactgctcgtcgcgcttgtgggcgaaaccgggatcgcccgggccgaagttgacggcgggaactcccagactagagaagcgcgccacatccgtccatccgtatttcgcgcggaacttcccgcccacggcggccacaagccccccggccaccgggtcgtcgaggccgggcagggcggcgggggcgatgtcgtcgtaaagcaagctcaaaccgccttcaagcgcaagcacctcctccaagtgcgccttggcgtcctcgacgctgcggtccggcgcgtagcggaagttcaccgtcaggcgcgcgtggtccgggatcgtgttcgtcgccacgaagccctccatgccgaccacgttgagcccctcgcggtactcgcagcccgcgatctcgaccgagcgcggcgtgtaatcggcgatgcgttgcagcacaccggcgagccggtgcgccgcgttatcacccaaccagctgcgggcggagtgggcgcgggtgccgtgcgcgtccacgaacacgcggatcgagccctggcagccggcctcgatgatgccgccggagggctcgcccagcagcgcaaggtcgccggcgagcagttccggatggtcgcgctcgaggtggtagaggccgttgaactcggtggcgacctcctcgccttcgtaggcgatcagcgtgaggtcgaacgcggcccgctccgggtcgcgcgcgagcgccgcgaaggcggaaaggtagcacgccagccccgatttcatgtcgacggcgccgcagccgtagaggatctcggcgccggaggcgtcgcgctcgatgcggtgcggcgtgttgtccgccagcgggactgtgtccacgtggccggcgagcaccacgcgctgcccgcggccgaagtgcgtgcgcgcaacaacggtgttgccgaagcgctgcacctccacgccgtcagcgtcgagcgcggcaagcgccgtctccacggcgtcggcgatcgcggcctcgtggtgcgagggcgattcgatgtcgatgagttgggtggtgagggtgacgggggcgtcgataagctgaagctccattgcgccaagcgtagtacgatgcagcaatgccgcagggagctgaaggaaccggaatcgccaacatcgccatggacggcaccgtgctcgacacgtggtttcccaacccgcgcctggtcggcgacgcagcggagctgaccaccggctcccgccgcgtctccgcgcgcgagctgtccgaccgcttcttaaaccttgtcggcatggaccgcgaccggctggtcgagctcgtgcccgtgcacacaaccatcgccgacctaagtgctccgcccgtcgacgcgcacgacgtgtacctgcgcctccacctgctctcccaccgcctggtcaagccgatggagatcaacatgctcgactgcctcgagcacctcgtgcccgtcgtgtggaccaacaaaggtccgtgcctgagcgacaacttcgaatacatccgcaccaacctccgctcgcgcggcacgatccaagtcatcagcatcgaaccgctgccgcgcatggtggactacgtcgtgccgtccggcgtcaccatcgccgaagctgagcgcgtgcgcctcggcgcccacctggcgccgggcacggcggtgatccgcgaagggtacgtgtcgtacaacgcgggcacgctggggccggcgcgcatcgaaggccgtctgtcgtccaccgtcaccatcggcgagggcacgcgcatcgcacagtccgcggtcgtggtcgccgacgagggggtccggcgcaaccgcgtgccgctgacaatcgggcgcgactgtcgcctcaaccacggctccggcaccatcggggtcgacctcggcgacaactgcgagctggggctcggagtactgctggataagggcacgttgctttacgacgcccgcgccggccaccaaatccacgcccacgacatcgccggccaatccaacctcgtgatctgcaacgaaccgttctcgaactcgccggtgttgcgcgaaaaggcctaacgtaaagtattcctcatgtcttctgatacctcgctggggcggggcttaaaaacgcgtcatttgaccatgatggggctcggttccgcgatcggtgccgggctgttcctcggcacgggcgtcggcatcgccgccgccggtcccgctgtgctgctggcctacgtcatcgccggcgccatcaccgtgtgcatcatgcagatgctggccgaaatggtcgccgcgcgcccctcctccggcacattctccacgtacgccgagcaggccttcgggcggtgggccgggttcaccatcgggtggctgtactggttcatgatgatcatgattatggcggtggagatcaccggcgcgtctgcgatcatcgcgggctggttcggcatcggcgcgtggatcccggcgctgatcgcgatcgtggtgttcacgctgatcaacttcgccgcggtgaagaactacggcgagttcgagttctggttcgcactgatcaaggtcgtcgtgattgtggcgttcttggtgctcggcgtgctgctgtggctcggcgtgctgccggcgagcggctttgtggggctggacaacgtgcgcgaagtcggcttcatgcccaacggctggggcggtgtagcgacggcgcttctggccgtcgcgttcgcgttcggcggcattgagctggtcaccattgcggccgccgagtcagaggacccggaggttgccgtgcactccgcgatcaagtccatcatctggcgcatcagcgtcttctacatcggctcggtgttgttgatcgtgctgctgctgccgttcgagcagatcggcggcgcgtccgaagcgtccgagtcgccgttcaccgccgtgctgcggcttgccgagatccccggcgccgtcggcatcatggaagccgtcatcgccgtcgcgctgctgtcggcctgcaacacgcaggtctacggctcttcgcgcttcctgcactcgcttgccgtccgcggcgacgcgccgcgctccttcgcagtcaccgattcccgcggcgtgcccgtgcgcgccgtgttggtcagcgtgttcttcggcctggtcgccgtcggcctgcagtactggaacccgccggggctgctggccttcctgctcaacgccgtcggcggctgccttgtcgtggtgtggtttgcgatcgcgttttcctatctgcgcatccacccgcagcttgtccagcgcggcgagatcacccacgtccgcatgtgggcgccttcttggctgccgtgggcgacgatcgcgctcatcggcgggctggtgttgctcatgctcacgaaccctgatgggcgcttccaagtgttcgccgtcgctgttgtcgtcggcgtgatcgcgctggcaggtgttattactacgaggactcgccgatgacttccacccacacccccaccaccccaaccgccgagagcaacctcggcaacggcctcaaatcccgccacctgacgctcatgggtctcggcaccgccatcggcgccggcctctttctcggcgtcggcgtgggtatccgcgcggctggccccgcgatcctgatcgcctacgtcatcgccggcgccatcgtcatctccgtgatgcggatgcttggtgagatggcggcggcgcggccgtcctcaggatccttctccacctacggccgccaagccttcggccactgggcgggcttcctcctcggctggatttactggttcctcctcatcatggcttgcggcgctgagatgacaggcgcgtccgcgatcatggccggctggttcggtgtcccgcagtggatccccgcgctggttgtggtctcgatcctgaccgcggtgaacctggcgcaggtgaagggcttcggcgagttcgagtactggttcgccatgatcaaaatcgcggtgattgttggcttcatcgccatcggcgccgcactgtggttgggtcttttgcccgcctctggcttcgtcggcttcgacaacgtgcgcgagtcaggcttcgcccccaacggtttcaccgggatcgcggcggggctcctcgccgtagccttcgcgttcggcggcatcgaggtcgtcaccatcgcagcggccgagtcggagaatccggcccagtccgtgaagaccgcggtgaacacgatcatctggcgcattgccgtgttttacgtcggctcagtgatcatcatcacgctgttgttgccctactcccagattgacggtgccgattccgctgccgactccccgttcaccgccgtgttggagatggcgaacattccgggcgccgccggcttcatggaagctgtcatcgtgctggccctgctgtcggcgttcaacgcgcagatttacggcacgtcccgactcgcgtaccaacaggcgctcgagggcgacgccccgcgctggatggcgaaaaccacaaacgccggcgtgccgcgcaactcggtgctggtctccgtgttcttcgcgttcgtcgcagttttcctccagtggtggaacccgccaggcatgatcgacttcatcatggcggcaaccggcggttgcctcatcgtcacctggatcatgatcacgctgagctacatcaaactgcacccgcagatcaaaaactcggcggtgaaggtccgcggtgcggcgtgggtgccgtgggtcaccctggctgcgctgttggtgctcgtggtgctgatgcttttcgacgacgcgtcccgcacccaaatcatctccgtctccgtcctgtccgccgtgttaatcggtctgtcgctgctgaccaaagacaggtcgcgctaaggtgcttcctatgacttctgcatccgcccgcggtttggccaccgtcacgcatgacggcactgttctcgatgtctggtacccagcgcccaagctggacgctgaatccggcaaggagtccggaacgcagcgggtggatgaggaggacccgcgcttcgcggagctcgccggccctgatgaggcgcgcggggtggctcgcgtgaccgtcgatacgcacattgcggacctcgaccagcccgcggtcgacgcctacgacgtctacctccgcctgcacctgctatcccaccgcctgatcaagccgcacggcgcgaacatggacggtgtgttcgggctgctcgcaaacgtggtgtggaccaactacggcccgtgcgccgtcagcgatttccagatgacccgcggccgtctcgctgcgaacggcccggtcatcgtctactcggtggacaagtttccgcgcatggtggattacgtcgtgccgtcgggcgttcgcatcggcgacgcggaccgcatccgcctcggcgcgcacttggcggagggcaccaccgtcatgcacgagggtttcgtgaacttcaacgccggcacgctcggcgcatccatggttgagggccgcatttccgccggtgttgtcgtcggcgacggcaccgacattggcggaggcgcgtccatcatgggcaccttgtccggcggcggtaaggaagtcatttcgctcggcgagcgctgcctgctcggcgccaacgccggtgtgggcatttcgcttggcgacgattgcgttgtcgaagccggcctctacatcaccgccggcaccaaagtggtgctgaccgctcccgttgccgaagccctgggcaaggaggcaggcgcgtccgttaaagcgcttgagctctccggtgcgagcggcctgcagttccgccgcaactcgctgaccggagcggtcgaggccgtgcccgccaagggcattgagctcaacgaagcgcttcacgcgaactaacccctcgctccgaacagcaccgccatcgcgccgtaggggtggtaggtgttgtccgccggaaacccgttcggcgacacccacttcggcaccccaccgatccgcttcacactgcctcgcctgttggcgtgcgacgcgttgtcgtgattgatctggttgtgatagcggcacacgggaacgaggttgtccatgttcgtctcgcctccctgcgaccacgcctccatgtggtggatctcgcagtggtcggagccgtggcggcaaccgggccacgggcaggcggtaagtgtcattcgtgcgaggtcgcgctgcttgtcgctggcatgtcgctgtgtgcggtacaggttcaccgcgccgaccgcggggtggaacatggcgacctcgtccagacccggttgcatcgcgaggtactcggcgccggtgatggtggtgccgtcggtaagcccgaggaccacgtcgtcggcctcgccgcgcaggatctgcacgtgctgatcaagcccgaccactacgattggccgacgcacgctggtcggaatacccccggcgccctctagcagttcgagcagccgtctcagcatctgcggccccggcggcttcgtggggtcaaggccgtcgcgaaggtagtgctcgatgtcggccgctttgtgctcatcaagcgtcgcgtgaatgcgccgggtgcccatcaccgacctaccgatggtcacgcccagtttggggcgggttcggacaggtttgggaatgagccggtccgctttgtccttgagcgcgttgtgggtagaccgccgttcaagcagctttcgccggacgcgccaccgctcggcgtcgttgggtatctttttcagccgttcctcgatgtacaccagctggctcagcgtaaagccctgggcagctttgaggctgaggcgctgctgtttcgcccacctagttgccccgtaatacaccgagtggatcttggcccatttgttggccaggctgggcataacaccggcggcaacggcggcgcgtttatcgaaaccaatcagcgaggctattgagggttgcgtacttaagaattcttcaaacggagtcatgcacgtcacgctaaggcggcgcgcaaggatggtaaaacgaaattccacaggcggctgcgaaatcagggcggcccgggccgggttatccacaattcggcattgccggtagattcgcgggacgcgatactgctacgttggaagtttcggcctagcgaaagcccagaatctgttgatgatgaaattcaccggcatcgccacgaaggtggagattgcctgcgcccagtaggacttggtgcgcaagcccgtggagccgtcaaagatgtggtcgggcaacccaactggcgtggtggggttcatcagcagcgtcatacaggtcagcgatacggcaagcgagagcaagccggtagcgaggaacgcgaagtagcctctcagccacgatcgtttcgactctccgcggaacgtccaagaacggttgagctggtagttccacgtgtttgccacgaggaaggcaagggtggacagcacgtggtaccagcggacgttccacctggtgctgaggatctgcgcaacgacgtcgtcggcgtggagaccgaatccgccctcgagcaacttgttggcaaggtagaacaccgcgaagttcacgatcacgccggagccgccgacgatgccgaacttcaaaaactcgcgcaagctcgcagctacaccacgcggcgggaaagcgctttccggcgcaccggcgggcacgccagcatcgagaggttggacgggattaagcacgtgacgagccttgactacgcagtgatgcgcgcggccgcttcagccacgcgctcgtccgtggctgtcagcgccacacggacgtggttcgcgccggcagggccgtaaaagtcgcctggcgcggccaaaatgccgcggtcagcgagccaggccagcgcgtcgcgcgacgacatgccgtcgcggcgggcccagaggtagaggccggcttcggagttgtcgacagtgaacccggcatcggtcagcgccttgagcagcacgacgcggcgcgaggcgtaggtggtgcgctggaggagttcgtgggtgtcgtcgtcaagcgctgcctccatcgcgtgctggatggggcccggaacgatcaagccggtgtgcttgcgcacctccagaagctcctggaccagcgtctcgtcgccggaaacagtgccggcgcggtaggacgccaggttggaggacttcgacagcgagtggagggcgagaagccccgtcatgtcgccgtcgcagatgctcgggtgcaggattgagacggggtccgcggaccagcccagcgacaggtaacactcgtcggaggcgattatcgcgcccgtgtcgcgagaaaactcgacccagcggcgcagatcctcggcggtggcgacgcggccagtcgggttcgaaggcgagttaatccacgcgaacgcggcgccgtcgacaggctcgttggaacgcacaatgtcgcacccggcgatcaaggcaccgacctcgtaggtggggtaggcaacctcgggaatgacgacagtctcgccgcgcaggccgagtagcgtgggcagccaggcgacggcctccttcaggccaatcaccggcagcacggagcgcgtggtcaacccggcgataccgaagcggcggtctagggcgcgcacgatagtgtcgcggagctgcggagtgccggaggtctgcgggtagcctggggtcgcggcgtgctcggcgagtgcgagctggatcgacggagcaacctggtcgacggggccgcccacggagaggtcgatcaacccgcccgggtgctcggcggcgtgcgccttcacgtccgcaatcgtgtcccaggggaaatccggcagaagagagcccagaggcgtgcgggacacggccctaatcctggttctgcgggggaagcgccgcgacgaacggatggtcgaagtccagcgggccagtcttggcggcaccgcccggggagcccagctcgtcgaagaaaccgacgttgacgtcgtagtactcgctccactcgtccggggtgtcgtcctcgtagaagatcgcctcgaccgggcaggccggctcgcaggcgccgcagtcgacgcactcgtccgggtggatgtagagcatgcgcttgccctcgtaaatgcagtccaccgggcactcttcgacgcagctgcggtccttgacgtctacacagggttgagcgattacgtaagtcatgcgctctagtatgtcacttccggttcagcaagggccaaacgccgcccgctatccccgccggcacgatccaagaggcgccgaggagcgcccacaccgcgcaccacacaccaagcgggatcagcggaacgagggagttggaagtccacaagcacgcggttttcgtcagcacagcgttgaagagcaacgcaaaagccgcggcgagcgcgaccgcggccggacgggcagctgcgaactgcatggttgccgacgccgcggcaaagatcgcaagccatacatacgcctgaacgatctcgcgccgggagtattggcgggtcacagctcggcgggaagctcccccgccccgagctggaagtgctcaacgcgttgaatcggctgcacgatcaagttcgagagcgcgtagtaaacaacaggtcccctcccgaacgcggcgtgcggattcgtgcgcgacacctgcccgtccgcgatccacaactgggtggcgtgggcccgcatggaggagattttggaggaataggcggcgtcgtcaagttgcatgctccaatccgccgtgtcgacgccgtcgagctctccctcctccggcaacctccagccctgcggggcctcggcgggcatgagcgcggcggtttctcgcgcgaggcggacagcgtggagaatgcacggcacagcgacgcgctcggcggccgcatgcgtgatctcgtgtgcgcggacgtggtccgggtggccgtacccgccgtcggcgccgtaggtgatcaccacgtgcgggcgctcggcggcgaagatttgtgcaagcagctcgacgggcgcgtcgccggagttcacaaacgcgcgcgggttgcggctcgccttagaaccggccataccggagtcgcggaaacggcccgcgccgccgaggtacgcgccgcgcgcaccgagtgccgccagcgacgcgtcgagctcccgcgtacggaacccacccagctgatcggcctcgtcggcgacgaggtgctggtacgtctccccgatcacctcgccctcctccccgagcgtgcaggtgaccacgaggatgtcggcgccgcggcgcgaaagcgcggcaatggtgccgccggtggtgatcgcctcgtcgtccgggtgggcgtggactaaaacaacgcggaagccggtgagatcgcgcatgctacttgttcagctgcttcgcgcgggaacgggcgcggccgcgctcggtggcgtccaggatgatcttgcgcacgcgcatcgcctcgggcgcgacctcgacgcactcgtcgtcgtcgcagaactcaattgcctcgtccagcgacagggtgcgcgccttctgcagcgtaaccgtcgcgtccgcggtggcggagcgcatgttggttagcttcttttccttagtgatgttgacgtccatgtcctcgtcgcgcgagttggcgccaacaaccatgccctcgtaggtctccgcgcccggctctacgaagaagtcgccgcggtcagccagctgctgcagcgcgtacgcggtgacctggccggagcggtcggcgaccagggagccggtcgggcggcccttgatctcgccggcccacggacggtgctcgatcgagtaagagttggcgatgccggcgccgcgggtctcggtgaggaaggtcgtgcggaagccgatcaggcctcgcgacggcacgtcgaactccatacgcacccaatcgccggaaccggcgttggacatcgaggtcatctggcccttgcggttggccatcagctgggtcaccgcgccctggtgctcggccgggacgtcgatgaccatgtggtcgtacggctcgtaggtcttgccgtcgatctccttggtcaccacctgcggcttaccaacggtgagctcgaaaccttcgcggcgcatcgtctcaatgagcacagtgagcgccatctcgccgcggccctggacttcccacgcgtcggggcggtcggtcggcagcaccttgatggagacattaccgatcagctcctgctcgaggcgggccttgaccacgcgggcggtgagcttgtcgccgccgttgcggcccgccatcggggaggtgttcacgccgatggtcatggaaattgccgggtcgtcaaccttgatgcgcggcagcggctcaacatgctcggggtcgcacagcgtgtcgccgatcatgatgtcctcgacgccggagatggcggcgatgtcgccggcgatgacctcgccctgcgccggaacgcggtcaaggccctcggtgaccaaaagctcggcgatcttgacgttcttgacctgctcgttgccgtcggcgtcgtagtgcacccacgccacggtctgccccttcttcaccgagcccttgcgcacgcggatgagcgcaatgcggccgaggaaggacgaggagtcgaggttggtcacctgcgcctggaacggcgcctcaatgtcggcggacggctccggcagcacgtcgtagataacgtcgaacagcggctgcaggtcctcgttggccggcagctcgccgttgcccgggttctccaaagcggcgcggcctgcgcggccggaggtgtagagcaccggcagctccaacaggttctctgcggcctcggcagcctccggatcctcgagcgacgcgccgagctccagcagcaggtcttgggcctcctcgacaacctcgtcgatgcgcgcgtccgggcgatcggtcttgttcacgcagatgatgaccggcttcttcgcctcgagcgccttgccaagcacgaagcgggtctgcggcagcgggccctcggatgcgtcgataagcaggacaacaccgtccaccatggacaggccgcgctcgacctcgccgccgaagtcggcgtggcccggggtatcgatgacgttgatgatgaggtcggagccgtctttgcctgccccggcgcgtcgaatagcagtgtttttagcgagaatggtgatgccgcgctcagactcaagctcgccggagtccatcacgcggtcgccgtgctcaccgtggtcgccgaagacgccggactgctcaagcatggcgttaacgagagtggttttgccatggtcaacgtgggcgacgatggcgacgttacgaaattcggggtgcgacacgagtaaccgctgctccttatatatatgcggtacagaacggttaaacactacccccaacggggccgcttcgctcaaagcgaccggcggcggggtgcacatttccgcttgacgatgttacggatgtgactaatgttgcttaggtgcgtaccctgacccgtgccctggcagcagcatgcctcgccactaccctcgccgttgcgcaggtgacccctgccgaagcgcgaagctccgcgtccagctttaatccgcttctcgacgagctggggcgccccacccccgaagtcgtcaggcaagtcaactccttcgctgacaagccgtacgtgccggagcgcgtaggcaacgcgctgcgcaccgccgtgaatttctacggcggcacgggcgagctcggcggtcccccgctgcccgcagacgccccgccgttcacgcagttttactggccgacggtctccagcaactgcatcgggcccggactgcactccaccgcgtccgcgatcgcggtgccgggaccgaccaccacccccgcacccggcgcaggcccgggccaggcaacgttcgtcttcaccgcgctgggtaccccggccgccgcgccgcagcagaacctgatgcgcgtgtactggctcaacacgtcgaatttccgcaccggcgtaacaccgctcggcaacaacgggattaacccaacaggaccggcaacgctgtccgccaccgcaaacacgggccccggcaacgtgatcgcggtggtcgacggcggtgtccgcacccttgatagggtgtgcaacttcgccccgaccgcagcttcgttccatgtgaggtgatgatgagcaccgttgacttgcacccggtaaagcaggagaccttcgacactgcgtcgaagaccaacacggacccgaaaggtttcctgcgcaacgtggacacgttccgagtcacggacttcggcctctacatggcccgcggtgcgaaccacccgcgcttcggctacctggagagctggttgctgccgaagttggggttgcgtgccaacatcttccacttccgcgacggcgtcgacgttgagcaggagttctacttcgacgtggcggacatcgacgtcgacggcgacgtgtgggtgacgcgcgacctctacgtcgacctcgtttccaacaccggcatgccgatcgacgtgctggatatcgacgagctcgccgccgccacctccgctggtttcatcacggccgaggaggccgagaaggcgattgacgtcaccctcaacgcggtggagggcattacccgccacaaggacgacgcgatggagtggttgcgcgcccagggcatagacctgacctgggcggatgaggtggagctggcgcccgtcggttagcaaaaagcccctgcttaacgacgaaacccacccgcagcccgggtgggtaattttcgtgcgcgcgtaacttagatcagctggcggcggccaaacacgaacgccgcggcgcccagcacggaggcgagcagcaggctcaaaagaccagccgggacctcgtttacgccggtggaggcgccgataccgcgctcgccgttagcggcgttgccgtcggcggcatcgccacccttcgcatccgcgatctgcgcggcgatctcctcgccgtgctccgccatcagctggtcggacttggccttctcctcggccgtggccttctcgttgacgcggttcgggtcctcaaccaagacaccgtccttgttcatgaagtacttcacgccttggatcagtagcacgaggccggcgatgccggctgcgataccgaggagcgcgccggtgttcttctccgcgtccttgacctccggcagcgaggtcgccggcacaacgccgtcgatccactcgtgctggtcgttgatcgcgcggccgcggttgtcgatgaggtgccacacgtagacgccgttctcgtcgatgaagagacccttgtccttaccgtcctcgaccttggtgatggtggtcttggggccgaagttgttcatctccgccggctcggtgccggtggtggagccgtccatgacaggcacgccgttgccctcgaccgggtccttgggcgcgataccgtctacccaggtttcaccctcctcgccagccaattcttccatcgtgaggtcctcgcggccggcgaccgggttctcggactcgacgaactcggcgccctccttgccgaatacgtcggtggcatcgaggtcctcgcggttagccgggttctcgtcctcgttgaactcggcgctctcctcgccgaagagctcagggccggttagctcgacgggatcagccgggtacgggttttcctggacagcgtcgacattacccggcaccggcaccacctgcgcccctgccgcggggatgacaccgaagcccagtgctccggcagtaacgagggcaatggtggtcttgctcatgcgcttcatgagttactccttcacgtgcgtggttcacccaacctcgtgcgggaccgatttggccccaggctcacaaggcaggcatcacactcggtctatcgctacgccatcccgaagcgttaacatctgattcttaggtttcgcgcaatggctacatacatgcagctcagaaacaccgatcgaccggcatttctaagaagatgctgacaatccactgtccgtgaccacgctgtcgaactgccagcccacaacagcatttcttatcgacggggcgtacatcggcggctgaatacagctaatcgtgagcaaccgccccggtgtcgcgccggtcccccacaccgctgcgtcgccggaaagcagctccttctgcggctcgtggaggtcggtcgcgacgtatttcagccacgccgctccggatgcctcggtgcgcacgtacaaggcgtctccggtgtggacgcggtggtggttggcgtggccgtcgtaaagctggttgaacactgcttccaccccggctcctgtgtgcccggcgatgaccacgatgtccgggctatcggtgcccggcagcgagtaagggcggtcgggcgcggtgtacgcgcacgccaggtcgagcgtggccgggtcgatgttgccgtcgaccacccggcagtccgtgtcttcgaaaccggcgcgcagcccgatggcggggatggcgatctcgacggggcgcgacggttcgatgtagatgtcgggaaccggtgcctccgcggtaggcggcggaggcggagcgccaactggggcctggcccccgccgccggggaagccgcgcatcgcccacagcgccgcgacggccaccgcgagcgcgatgagaagcgcgaggaacgtcgcccacaccgggtggcgccccggcgtgcgccgatgccgtcccccgtactgttttccctgtgccgcgcggaccacggccaactaagcgcccgtacccaactcgatgccgagaccgggcaccgagttgatcaggttctgggtatacgggtcctgcgggttgccgaagatgtcgtccgcggttccctgctccacggctaccccctggcgcatgaccaccacatcgtcggcggtctggcgcacgacggcgaggtcgtgggtgatgaagaggtaggacaggtccaactcatcctgcagctgcgcgagcaaggtgatgatctggttctgcacgagcacgtcgagggcggagaccgcctcgtcgagcacgacaacctcggggtcgagcgccagcgcacgcgcaatcgcgatgcgctggcgctggccgccggagagctcgttcgggtagcggcgcatcgccgagcgcggcatctgcaccatgtcgagcagctcggcgacccgcgcctggcgctccttgcgcccgccgatgttgtgcagcgccagcggttcctcgatgcacttgtacaccgagtacatcgggtccagggatccatatgggttttggaacacgacctgcattttgcgccgcatagcaaacaactctttgccggtgagctgggcggtgtccttgccctcgaacagcacgcggccgctggtgggctcaagcaggcgcaacaccatgttcgcaacggtggacttgcccgagccggactcccccaccagcgccaacgtggtgccacggcgcagagaaaagctgacgttgtcgacggcgcgcagcaccttcttgtcgcccttctgcccgcgcacgtcgaactccttgaccaagttctccacgcgcacaacctcgccgccgccgcggcgcccggcggtaagttcggagctttccagccccttctccttcgcggactgaatgcgcgcggacgcgagcgacggcgccgcggcgacaagccgattggtgtaggggtgctgcgggttgcgcaggatctgcaggctgggtccgcgctccacaatgcggccgcggtgcatcaccaccaggaaatcggcgcgttccgccgccaaacccaaatcgtgggtgatgaacagcagcgacgtcccgagctccgaggtgagcttttccaggtggtcgaggatcttcttctgcaccgtcacgtcaagcgcagaggtgggctcgtccgcgatcagaagcttcgggcgcgcggcgagaccgatggcgatcaacgcgcgctggcgcatgccgccggagaactcgtgagggtactgcttcgcgcggcgctgcgcgtcgggcagacccgcttcctcgagcagctccaccacgcgcgcttcgcgctcgcttcccggcacgacgttgttggcctttagcgattcctcgatctgcgtgccaatgcgccacaccgggtttaagttgctcatcgggtcctgcggcaccagcccgatctcagagccgcggatctcctgccactggcggtcgtccaggttggtcaggtctttgccgttgaaggtgatggtgccgccggtaatcttgccgctgccgggcaaaagccccagcatcgacattgcggcggtggatttaccggagccggattcgccgacgatggcgaccgactggcccgggtagatagtcaggtcgaagtcgcgcaccgcgtcgacgaccccggtggtcgaatcgaacgtgatctttaggtcgttgacttctaacagcggctgggtcatcgcttcctcgccttcggatcgagggcatcgcgcaccacgtcgcccatcatgatgaaactcaaaacggtcagtgccagcgcgatcgccgggtagaacagcaccatcggctgggtgcgcagcgacgcttgcgcgctcgagatgtcgcctccccaggacacgacggacgtcggcaagccaatgcccaagaaggacagggtggcctccgcgacgatgaacgtgccgagcgcaaccgtcgcgtagacgatgatcggtgcggcagcgttcggcaggatgtgggagaagaggatcttgctattcgacgccccgagcgcccgagcagccgccacatactcctcattcttcactccgaggaccgcgccgcgcgtgatgcgggcgatctgtgtccagccgaacatcgaaagcgcgatcaccaccatccagatggagcggcggttctggaacatggacatcaccacgatggcggccagcacaagcggcaccgcgaagaagatgtcggtcaggcgcgacagtagggtgtcccagataccgccgtaaaagccggcgatcgcgccgataagggtgccgagcagcgtgaccacgatcgtggtcagcacaccgacggtgacggaggcgcgggcgccgtagattgtgcgcgcgtagatgtcgcacccctgccggtcgaagccgaacgggtggcccggcgccggcccgtcgagcgaacgcgacaggatgcactcgcgcgggtcggtcgaggtaaacagctgcgggaacacagccatggcgacggcgagcaggatcagggcggaggagatccagaaaagggggcggcgccgcaagtagcgccacgcctcgccccactggctggacggcgcccggtcgtccggcaccgcgtcgacggcacctaacccggtctcatcggtcgcggcgacgaagtagtcctggccgggcagcacgcgatcggccgccgcggcggtgttgaaatcgttgttacgcatagcggatcctcgggtctagtacggcgtagagcaggtcaacgagcaggttggccacgatgtagacgatgacgagcacggtagtgaacgacacgaccgtggcgggctcgcccttgataatcgcctggtagatcgtgccgccgacaccgttgatgccgaagatgccctcggtgacaatcgcgccgcccatcagcgcgccgaggtcggcgccgaggaacgtcacgacggggatcatcgagttgcgcagcacgtggcggcgcatgacctggccgttgctcaagcccttggcgcgcgcggtgcgcacgtagtcggcgcgcaggttctcgctcacggactggcgcgtcagccgcacgacgtaggcaaacgacaacgcgcccaacacaaccgccggcatcaaaagcgcctcgaacgtttcgttgcggcccacggtgacggggagcaagccccacttcacgccgacgacgtactgcaggacgaaaccgatgacgaagctgggcacggcgatgacgaacagggaaacaaccagcacggtggagtcgaagatgccgccgcggcgcacgccggcgatcacaccgaagatgacgccgaagaccgcctcgaacactagcgccatcaaagcgagtttgatcgtgaccgggaacgcctgcgccatcacggaacgaaccggctggccggagaaggtggtgccgaagtccagcgtaaaaatgcccttgatgtagagcaggtactgaacgataaacggcttgtccaggttgtactccgcggtgatgcgctcgcgggcggcgtcgcttaagccgcggtcgccgccgagtgcctctaccgggtcaccgggcatgaggaagacgagcgcgtagagcaaaaacgtggccccgaagaagacggggatcatctgcagtaagcgtcgtccgatgtagcgccacatatcttgctagctacctttcaatcggtgtgaacgtgagaaaccaagggtaaaacccacacccgggcaagcaagttaccgggatgtgggttctcattggttagaaacgccgcgtatctacttcttggtgatgttgtggtagaccggcacctgcttccacgagaacgccacgttatccacgttctccgagtagccgccggtgacgttggcgtaccacagcgggatggcgggcaggtcctgcagcaggatctcttgcacgtcgttgtacttggcgttcgcagcgtcgacgtcagcagcgttcgcggcttccttcagcaggcggtcgacctccgggttggagtagtcgccgtcgttggaaccagcgccggtgccgtacagcgggccgaggaagttacccaacgacgggtagtcagcctgccaaccggtgcggaacgcgccctcgatgttgcggttggtcacgtcgtcgcgcagggacttgaagtccgggtacgcgttgccctcggcgtcgatgccgagcgtgttcttgatcgagttggccaccgcgtcgacccacgcctggtggccagcgtcagcgttgtaggagatggtaaaggtgccagaccacgggctgatcttgtcggcctcagcccacaggcgcttcgcctcgtcggcgtcgtagttgagcacctcggcacctgggaggttgtccgagtggcccgggatcaccggcgaagtgaagtcggtcgccggggtgcgcgtgctgtcgaagatcgtcgcggtgatctcgtcgcggttgatcgcgcgcgagatcgcggcgcggcgcagcttgccctcctcgccgccgaagtgctccacgctctccgggatggtgaaagactggaagacggctgccggctggttcacagcgcgctcgcccagctcagattcgaaggtggtgaacgcggagtccggaatggcgtcggtgacgtccaggttgcctgcaagcaggtcggcgtacgccgcgtcgtcttgggcgtagaagacgaagttcacgccgtcgttctggggggtgcgctcgccgtcgtactcctcgttcggcaccacgatggcgtcctggttgtggttccactcggccagcttgtacgggccgttgccaagcggggactcgccgtaggcggcgagatcgtcgaacgcggactcgtgcatcgggtagaaggcggcgtagcccaggcgcgtcgggaagtcggcctccggctgcgcaagttcgatggtgaaggtctggtcgtcgatgacctcgaggccctcgagcggcttgccctcctcgtagcccttgatcggctcgaagaagtaggcgcccagcatcgcgtcctcgacgacgcggttccaggtgttgacgaagtcgttggcggtgaccggggtgccgtcggaccaggtgatgtcgtcgcgcagcgtgaccttgtacgtggtgtcgccctcggcctcgatggacttcgccatctcgttgtggatctcgccgtcctcgtcgtagtagacgaggccggagtagagcaggtcgacgatgttgccgccgccgacttcgttggtgttgcccgggatcagcgggttttgcggttcactgcccttagcggtgatgtagttgccgccgccggcgctgtcgccgccgcctgcggaactgtcagagctgcagctcgccgcagcaaatgtcattgcgctggcggcgaggacggccaccactttcttgacgctcattgtgcttctccttcgtccgacgacaggtttggaacgcctgtcacactgctgggggatttctagattcaatcacaaaagcaactgggtttgtaccaaaggggtcgtttttcgttccaatttcgtttacctccagttcatcggcgcgttctcaaagggtgcaccaacagctgctaagttcgaatcacaatttcgcttttcggaaaggtttctcatgcccggtggcttgctagcactgcttgacgacgtggccttgatcgcccgcaccgccgccgcctcggtggacgacgtcgcagctatgaccgcgaagacctcgatgaaggccgcgggcgtggtgatcgacgacgcggcggtgaccccgcagtacgtctccaacgtcaccccggcgcgcgagctgccgatgatctggaagatcaccaagggaagcctgcgtaacaagttgctcatcatcttgcccattgcgctgctgctcaacgccgttgcgccctgggcgctggtgccgatcctgatgatcggcggcagctacctgtgtttcgagggcgcagagaagatctggcacaaattcaccaccgattccgaaacccagcaggaacaggcggtgaacaagacaccgcaggatgaggactcgctggtcaaaagcgcgatcatgacagatctcatcttgagcgcggagatcatgatcatctcgctcgacgaggtctcggaccagcccatctggatggaggccgccgtgctgatcgccgtcggcatcttcatcacgatcgcggtgtacggcgccgtggcgctgttagtgaagatcgacgacatcggccgcggcatgatcgagcgcggcaacgcgccgaagacgggccgcgctctggtcaagggcatgccgcacgtgttgaacttgatcggcattatcggcacggtggcaatgctgtgggtcggcggccacctcattatccgcggcctgaacgaagttttcggctggcactggccgcacgacatcctcgagcgcggcgctgaagccgtgggcggcggcgcggccggctggttcgtcgacaccgcaggttcgctcgtcgccgggctgatcaccggcttcatcatcctcggcatcgtctcgcttctccgcggcgcccgttccggggagaaggcagcccagtcgtaatggctgcgcgcctctacccgctggcgccgtcggtatggggcgccgccctacagctgccggtgcgcgacgtggtgcaggcagcgctgttttctgagttcgccgcccaccccggcaccgcgttcgtccccgtccacctgcaagcggagccgctgagcggcgggtggaaagtcaggcacgcgaatggcgcggcgcttggcacgctgccggcgagggagcgcgagcgcttcgaggacctgcgccgcgttgaggcgtcgctgctcatgccggtaacgcttgccgaggtgtacctgagcccggagaccggccgcttcgaggtcaacgtgctgctgccgccgccggagctgatcgtgccgcgaaacgacgccccacccaccgccgtcgtcctgcagcccggcgacatgctggtcgtcgacacctcgaggggcgagttcagcgccgaagaactcgccgtgcgctcccccggccagtggctcgtcgcgctgcacccgatcggcggcgcggtggccgccaccttgggcggcaaggtgctcggcggcgtcgagtgggagggcgatccaacagagctcgttggcgacggccaaagcgaggtgtacgcccgcgcggtggtgctcgacgggatggcggcgctcgacgtcgcaccagaactcccggcggcccacgtgcccgcgctgaaggtgccggatccgcgccccgtcacgccgtgggagctcaccgacttccccgacgggacgtgggcggtgaccgtgctccgccaatactcggtcgacgaggccgacacgctgcgccccgcgcacacgtcgcgctacgtctcgctttccggtgaggaccggccagacgacgtggcggcgccgacggagatgttccacaccgtggacctgccggaacctgagcggaaacgcgctacccccatcgcgtccgtgcagaccgcggcggaagtaaaggacgtggaggcggcgggtgagtttttgacggaggttgagaaggtgaggttgcgtcgtcaagcaaggctctcgcgccgcggcgggcggcaccgcaagtagaacttccgtaccctggggcctatgagcaacgatcatggacccaacccgtacatcgtcaacatcgaagaggccacgctttccaacgaggcgttccgcgacaccctgtggaccgggaagaacctccagctgaccgtcatgaccatcccggccggcggcgaaatcggcgccgagatccacgacggccacgaccagttcctccgcctcgaggagggcgagctgcgcgcgaagatcggcccgagcgaagacgatctcgagatcgaccaggtcatcggcgctgactgggcggcgttcgtgcccagcggcaagttccacaacttcgtcaacgagtccgacgccccggcgaagctgtactccatctacgcccctgccgagcacgagccgggcacgcgccacgagacgaaggctgacgccgacaacgacccgcacgaggacgctggcctgtaaccgctagcgcaacacccttgagttgccgtcaacgcgccgggtcacaccgcgcgcgtcgagcagctcaagcagggggatggccactcgcctggtcgtcccccattttttgcgcgcgtcagaggcggaaaacggctgatcgagatcggtgagcatggcagcggctttcgacggggcgtcgccaagcagcacgacaccgtctgcgatccgcacgatggcaccggcgcgctccgccgcggccagctctcctggccccacgccccacgcctccaagtcgcgggcttccggcgccgcgaacgggtcgcgctctaggtgcgctttcagcttttgcatccccgggccgagatccaccgcgcgtccgctggaaatcacgtcggtgacggtcagcttcgccgccgcggcggcgagcggcagcagcttggcgtcagggagcttcagcttgtcgacgccctccttcaaccccaaccccgccgacagcggattcgcctcctcgtgctccgcgacagctcgcagcagctcgtccttccactgcatgacctggcccgcgcggatccagtaaccggcgaacgcgaccgaaccggccggtggcgcctcccccaccgcgaaaccgaggcgggcgaggtccgcgggtgcgacggcgacgcggcgggcgatctcgcggtcgatatcgggcagccccgcgagctcctcggcgcgccgggcggcgtcgccgcggcgggtaaacgcgggcgggtcgacgtcgacgacttcggcgctggcgaggatgtgctgctcgccggagccgcgcagcaccacgcggtcgccgatggtcagcggcagcgggcgctcgaatgtgaggcggacaaagtcgtcgccgagggtgcggaccgcgcacgggactgacgcggtgcccacgtgggctacggcttcgcgggagatggtggaggtggtggtggggttgaaggtggcgtcgataagcgtggtgctccaccacgcacctggggtgagaagcgcgtcgccgcggccgatgcgggcggcgtcgatgccgcgcaagttgagcgcgacccggcgggcgggtgcggcggcgtcgatgggggtgtcttcggactggatgctgcggacggtgacctcgcggtctccgagcgcgagcgtgtcgccggggcggatcgtgccggcggtgagcgtaccggtgaccacggtgccggcgcctttgacggtgaacgagcggtcgacccagaagcgcacgcgggcgcccgggtcgggctcggacgcggcggtgagcacgtcggcgagggtggattggagctcggcgatcccctcccccgtcttcgccgagacctcgacaaccggccagtctgcgcaggtggtggcggaagtcttggcggcgatctgcgcgcggacctcggcgcggcgggcggcgtcggcgttgtcggcgcggctcatcgcgatcacgccggtggtgatgccgaacgcgtcgatcgccgcgaggtggtccgctgactgctccttgaatccctcgtcggcggcgacgacgaaaagcaccgcgggtgccgggcccacgcctgcgagcatgtttgcgataaagcgctcgtggccggggacgtcgacaaacgccacatcaatggggccggaggaggcgtcgaacgaagcccacacgaaaccgaggtcgatggtcagcccccgcttgacctcctcctcccagcggtccggctccatgccggtgagccgcttgaccagtgtggacttgccatggtccacatgccccgcggtggcgacgacgaaggttttctggctcatcggcgcacccgctcgattgcgtcggcgagctcctggtcgcgctctggcggcacgcaacgcatgtcgatcaggaggtggccgtcgtgcacgcgtccgagcaccgcgggtgtgccgcggcgcagcggggcggcgagcgcctcgtccaaacgcaccgcgaagccgggcagcgggtggccgggggctcccccgccgccgacacgcccgtcgtgggcaaccacgtcgccgccgacacgcgcggccagcgcctccgccctgcgtttcagctccgcggggtcggcgtgcaggtaggcgtacgtggggttgtcggctgcgcgcagcgttgcctcgagcgccgcgaggcgcaccttatctatccgcacggctcgcgcgagcgggtgcgtgcgcatagccgcgatcgcgtctgcacgccccagcaccacgcccgcctgcggcccgccaagcagcttgtcgccggagaacagcacgacgtcggcgccggcttcgagcgcggtggtggcgtccggctcgtccggaagcagcgggtcggggcgcaagaggccggagccggtgtcgacgatgagggtctggccgtgagcgtccgcgatcgcgcgcagctgcggcaccggcacgctcgcggtgaagccctccacgcggtagttcgaggggtggactttcaatatcgcggcggcgtcggcggcgcgctcgtaatcgacagcgtgggtgcggttggtcgcgcccacttccacaagctcgacgcgcgccgactcgatgagctcgggcaaccggaacccggcgccgatctcgatcagctcgccgcgggagatgaccaccttgccgccctcggcaaacgcggcagcggcgagcaagagcgcggccgcgccgttgttcaccacgagcgcgtcctcagctgccgggcacgcctcgagcagcgcggcggtagcctctttaccccgctcgcgcgagcgcacgccagcgtgcaagtccatttccacgtcgacgtacccggcggcggcgcgcatggcctcgacggcgccggaagacagcggtgcgcgaccaatgttggtgtgcaccaccacccccgtggcgttgagcacaggggtcaacgccgtggcgcccgcggcaagggaggcgaggaacacgtctttgacgtcgtccggggcgatctcgccgcggcgggctgcgtcctgcgccgcgcgcgctttggctttgagtgtgggctgggagaggttcaacggggcgtcggcaagcagcaacagctcatcggtccgagggatgctgcggcgcgggtccatgaaagcctccttcaagcacaagtggcggagacggacaggaatcgaacctgccaagccgagatgctcgacttcaccagttttgaagactggggcgcccaccaggacacgtacgcctccgccgcgaaacgctaccatgacggcctatggataccattcgtttgacccagtttgccgcaggcggcggttgcgcctgcaagattcccccaggtgagctcgaggatgctgtgcaaggcttggttggcttcaccgacccaaacgtgattgtgggcttggacgacggcgacgacgctgccgcgatccgcgtgcgcgacgacctcgccgtgatctccaccgcggacttcttcacccccgtcgtcgacgacgcgtacacgtggggcaagatcgccgcggtcaacgcgctcagcgacgtctacgccatgggcggcaccccgatcaccgcgatcaacctgctcgggtggccgcgcgacgtgctgccgcaggagctcatccgcgaggttttgcgcggcgggctcgacgccgcgaccgaggccggcatctccgtgacaggcgggcactctatctcggcgccggagccgatctacggcatggccgcaacgggcaccgcggatcccgctcgcctgatgcgcaacgacgccgccgaagcgggcctgccgatcaccctgaccaagcccatcggttccggccttctgaacaaccgccacaaggccaccggcgactggttcgacggggcggtcgaggtgatgaccacactcaaccgcgacgcgtccgagaaggccgtcgccgctggcgcgaaggctgccaccgacgtcaccggcttcgggctgctcggccacctgtacaagatgtgccgcgcgtccggcgtcgacgcggtggtggatttcaagagcattccgcttatcgacggcgccctagacaccatcaaggccggcttcatcccgggcggctcgcgccgcaacctggactgggtccgtcccaacgtcgactccgacctcagcgaggaggagctgctcatcgccgccgacgcgcagacctccggcggccttttggtaatcggcgaggtgccgggctaccccgtgatcggcgaaaccgtcgccggcacggggcgcgttagcctgcggtagtgatcgaatccgccacgtcgcccgctgcgcggcgggcggccaagcggttgcgctgcggctcgactacgtacttcgggtcttgcgtcgagcgcttacccgcagccatgatgccgaaacgggtcaggcaggagcccgccatcagcgcggcacccgaaagcgccgcgatcacgcggtttcgcccgccgaccagcgcgcccacaccgccggcaacgacaagcgcttccgcggcggaaagcatggtgcccgccttgccctccttcatggtctccggcagcggttccggcaggttgcgctccacgcgcttcgacgccgcgatgtcgcttaccgcgccgatcaccgccagcgctcgagccggcccgttgttcttggtcgacgtggtaatcagcgccgcaccagaggcagcggatgccgccgaggaggcgaacagcgcgggcaggtcgttgcgcgccgcctgccacgtgggcacggaggtgtcgcctaaaagcaccgcggtgtagaccgcaagtggggcgcccatcacgccggagaacacgcccatcggggtcgccaccgcgtgcagggtgtcgcgcacgaaccccggtagcgggaggacctcgccggtgagctcgtccacttccgctgccgcggcgactgctgcggaagaggagaacgaacctaaaatccacgaccccaccgacatcggcgaggacagcttgaacacgcggaacatgttcagcagccgctctgggcggccgagatcggcgactaggaagagcgaacctacggcggaagcgcctgccgcggtgatgcgggtgttgcgctgcaactcccggtcaccggtcgcacctgcgccaagaccgaggatcgccgagccgccggcgacgccgccgaggaagaaatagcccgcgatcggccactcccacggcgggaacttcacaatcgggcggccgtagtacgagtcgtccttggagaagtcctcgaactcggcgcgcggcaccataagctcctcgccgcggcgcaccttgcgagacgtgcccttggggcgctggcccttgggccggcgtggctcctcgggcgggcggaattgatcaaactctgccactttctagctccttcctccgatcgcgaacgccgctgccgcggcacccaccaggcccgctgccgcgtacgcggcgcgcttggccatctgcggcaggttcgcggtcggcacttctgggtccggcggcaggccgtagacctcgggggcgtcgagaagcaagaaaatgctcccggtgccgccgacgccgtcttcgctgttggcgccgtagaggcgcgcttccgtctggccctgggcatgcagctccgcgactcgcgccttggccgtggccagcatctcgtcgtaggagccgtacttaatcgaggtggtcgggcacgtcttcgcgcacgccggcccctcgccgatctccatgcggtcgaagcacatcgtgcacttttgcgccacgccgacgttcttgatcggcgcgacctcgcccgcggtgaagtcctcgcccacgcgcggggagcggtcgttgcgtttctgcacgccgccgtcgctgcggcgctcaatcaccccgaacgggcagcccgccacgcacgtgccacagccgttgcacacgtcgtcttgcaccacgacggtgccgtgttcggtgcgaaacagcgcaccggtcgggcacacgtccaggcagccggcgttggtgcagtgtttgcacacgtccgacgacatcagccagcggaagtccggcgtgtcagccggcatgaccttctccggctccggggtcgcgtcgcgcacgtcctgcggacccacgcccggcatgccgagcgaaatcagctgcgcaccctcctcgcgggcgcgctcgatgcgctcctgcgactgctccacgaacgcgacgtggcgccacgtgttcgcacccagcgagcccgtgttgtcgtaggacatgcccgagaactcgtacccgccgtcctgggggttgcggttccactccttgcacgccacctcgcaggctttgcagccgatacagatcgaggtgtcggtgaagaatgctttgcgctccgcccggtcgtaaccgacgtggtagggcgcttcggtgatgctgttggttttagccattggcctgtgttcctagccttccctctccgccatgttttccttggtgctgtccttctccgcggtgttttcgtcgtcgagcccagccgcggcggtggcgtcgtggttgcccagcgtcgcaccggtgtcctcggtcagcccggcgcgcttctggtactcagccacaagcgcgtcgcgctcggccccgcgcgggcggcggcccgggcggatatcgatcgcggaaaccttcgacgcctggatgttcacgttcgggtccagcatgatgcccagcaggtcgttcggcccgtcgccctctacctcggcgtagttgccttggccgtagtggaacggcatgcccacctgctcgtagtcgtggccgccaacggtcaacgactggatgcggtccgtcaccagcacgcgagactcgatggcgccgcgcggcgagatgattgtcgcccagccgccgtgttccaacccgaccttctcggccagctccggcgagacctcgcagaacagctccggctgcagctccgcgaggaacggcagcgtacgcgtcatagcgccggaggtgtacatctccgtcaaccggtacgtgttcagcatgtacgggtagacaacacccgcacccttctcgccgtagttaggcgccgagaggttgttcgggccgcgcatgacaatgcgcgacggcgactgctgctgcttgtacaggaagttcgggaacggcgactcctgcggctcgtagtgcgtcggcatcgggccgtcgaccatgccgcgcggcgcgaagagccaacctttgccgtccggctgcatgatgaacgggtcgtcgccggcgagcgccgcaggccccaccgcgtcgcggtcgggcttgaagcccggcgccttgtccaccgggaagtccaccacgtcgttggactcccacttctcggtgtcctcgttccaccacacgagcttcttgcgctccgaccagggcttgccgtccgggtccgcggacgcgcggttgtagagcacgcggcggttcatcggccacgcccaaccccagtcgagcgccatctcgtcttgttcctgaccagggcgcttgttggcggcgcggttgacgtcgcccgcgaacacgccggagtaaatccagcagccacaggcggtcgagccgtcggccttcaggtcggcgaacttgtccaccagctcgcccttgcgcgggccgtcgaggtagtagccgttgatctcgcgcaacacggactccgggtcgatctcgccgtgctcgtccacctcgtagtcccaggtgatcttctgcagcggcaggtcgcgcgggtcggtcgagtccttgactcggtccttaatccgcaggccgagctcgtagaagaactgcagatcgctgtccgcatcgcccggggcttccttcgccttaaagcgccactgcagcatgcgctgggtctgggtgaaggtgcctgccttctccacgtggttcgcggccgggagcaggaagacctcggtgtcgatctcctcggtgaccaagtcaccggaggcaatctcgggcgagtccttccagaaggtcgcggtctcgatctcctggaaatcgcggacaacgagccacttcagcttcgccagcgccatgcgctgcatgcggccgttggactgcgccacagccgggttctgcccgaagacgaagtagccgtcgaccaagccctggttcatcagctgcagcgtgtggtacgtcgagtgcgctcccgtcagccgcggcataagatccatgccccagttgttgtcctcggtggccgcgtcgccccagtagctcttcatcaggctgacggcgtaggtgtcgcccttctgccagaaacccttctggtcgcgcttggacaccgtgtccaagtactggtcccacgtctgcacctccgcctgcggcatgggcaggtagccaggcagcaagtggaacagggtcggcacgtcggtcgaaccctggatggatgcgtggccacgcagcgccatgatgccggagccgggtcggccgacgttgcccatgagcagctgcagaatcgcgcaggtgcggatgaactgcgcacccatggtgtgctgcgtccaacccagcgcgtacgcgaagcaggtggtcttctcgcggccggagttctccgcaatggagttcgccaagtagtagaagtcgtcctgcgaaatgccgcagaccttctccaccatctccggcgtgtagcgcgagtagtggcgcttcaaaatctggaacacgcagcgcgggtcctgaagcgtctcatccttctccacgtcccaagacacttccgcgtcccagaccttctccggctgccacgaggcgttgtcgtacttgccggtctccgggtcatagcccgaaaacaggccctccaagtcctccgtgtcgcggaagtcttcgctgatgatcgtcgacgcgttagtgaacgccttgacgtactcctcgaagtacagctcgttttgcagcacgtagttgatcacagcaccgagcagcgcgatgtcggaaccgccgcggatcgggatgtgcttgtgcgcgattgccgacgtcctcgtgaacctcgggtccacgtgaataatccgggcaccgcggttcttggcttcaactacccactggaacccaacggggtgcgcttccgccatgtttgacccttggatgacgatgcagtccgcattcgccatgtcctgcagcggctgggtcgcgccgccgcgtccaaacgaggatcccaaactgggaaccgtggaggagtgtcatatacgcgcctgattttcgatctgtaccgcgcccgaggcggtccagagcttcttaatcaggtagttctcctcgttatccatggcggcgccgccgaggccggcgatacccatggtgcgacggatggggttgcccttctcgtcgtagtcctgccacccgttcttgcgcgcttccatgaagcggtcggtaatcatctcgagcgcggtgtcgcggtcgagcttcacccactccgtggcgcgcggcgcgcggtagaggatttcggtgagacggttcggcgcgttcacaagctgctcggaggctgcgcccttcgggcacaggcgcccgcgcgagtgtggcgagtccgggtcaccctcaatctggatgaccttctcgtccttgacgtacaccttctggccgcagcccacagcgcagtacgggcagacgctcttgaccacgcggtccgcgtcagcagtgcgcccctccatcgcctgtgtctgagcagattcggtgttctcgccacgcgcgaacacgtctcccccgcgcagctggcgcacgactggccagttcaacggactaattcgagacatagaccacacactaccccgccggtgaccaaaacacggcaccaagcacgtgcccccgcacgccccgcgtaaagaatacgggcgtgcgccccggctgtttgctaaggtgaaaacgcttaaaaggaccctcattatttcctgcgaggaagttacatctcatggctcgccgccccttttcccgcgccctcatcggcgctgcaaccgtgtctgcgttaacccttgcgagtgtggctgcaccgcccgtgggtgcccaggaaaccgaaaagccggaggtaaccttcgacaccgccgacccgcaggatgaggcggaagcgatcgcggaggccgctaccgaggagggtgctccgctcagctacttcgacaagcgcactgaacgtatcgcccccgcgatgggtgcccgcgccccgcgcaacgtcagccgggatgtttcggtgcaggtgatgggcgacatcctcggccgctactcgcagcacgtcggcttccgctccggcgatctgggcatgatggccccgatcaacgccgacggtgagttcgccatgatcttcggcgactcgttccgcggcgacggcgtgggcaagggtgagtggatgagcccggtcggtgtcgtggcgaagcgcgacgcgaacggctacgtggacatccagcgcccgctcaaccgcggcgagcgcgttgagcagaccatcccgtacttgcgcgacggcaacctcacactcatcccgtcggacatcatcaacatcgacggcacgctctacctgcaggcgatgtggacgcgcggcctgcacaacgtccagtactcgcagttctggaagtcgaccgaccagggaaagacgtggcagcgcgccggtcactactacacgggcatgaagcacaaaaccagccgcaagggcctcgacgagatgctgtcgtgggaaatgggcccagacggctacgtctacatcgtcaccacgacgttcgaacgagaccacgcggcaccgctctacctcttccgcgccgccccggaaaacatcaccaaccgcaacgcgtgggaaatggtaaacctcaacgacggcacctgggttgccagcgacgagcccggcacctcgatcttggagaaggaccgctcgggccggccggtacagatcggcgaaatgaacctccgctacgtcgacggctactgggtgctcgtcgcctttaacgaggcaaccttaagcgtcgaggtgcgcatttcggaagagatcgcgaccgactggaaccaaatcccggcggtgacgattgcgaagaacggcccgtggggcaacgagcagaccccgaacaactggtcgcagccgtacggtggttacatcgtcccaggttcgagcatcaacgacatggacattgtggtttcgcagtggaacacgtccaccaacaaccgttacatgtcgacccagttcagcgtccgcggcctggagacagccttcgggctcgagggttttgatcgcgtcgcaccgcgccagtccttcggcgagaagacggtccgccccgcactgccggagcccgcgatcacggctccggcatcctccgcggccgcgcgcaccgctgtgatcgtcctcggcgtgatcgccacgctcggcaccctcgcggctatttcgtggccagtactgcgtccgctgttgccgccgcaggtacagcaccttctgccgttctagtaccggctgtaatcgcgtagcatcactgcggtgacccgcaccgaaacgccgcagaagcagcagtcgccctggcccgcgttgtggtcgatgatgctgggatttttcatgatcctggtcgactcgaccatcgtctccgtggccatccccgccatcaccgcgggccttggcgcctcctacagcgaggtcatctgggtcaatagcgcctacctcttggcgtacgccgtgccgctgctcatcaccggccgcctcggcgaccggttcggacccaaaaccgtctacctcatcgggttgaccctcttcacgctcgcctcgttggcgtgcgggttggcgtcctccgcctcagcgctgatcgcggcgcgcgctgtgcagggcctcggcggcgcactggtcaccccgcaaacgatgtcggtcatgctgcgtaccttctcccctcagcaacgcggcagcgccatgggagtgtggggtgccaccgccggccttgccacggtgacaggtccgctgctgggcggtgtgcttgtcgacgccctcgggtggccctggatcttcttcctcaacgtccccgtcggcgtcgtcggtttcctgctcgcttaccgcaacgtgccgcggctcgaacaaaccaaccgccgcttcgactggcccggggtgctgctgagcgcggtcggcatgttctgcctggtttacggcatccaggaggcgcagcgcttcgactgggactggcgcgtctgggcgttgctttcagcaggcttgacgacgatgctcctcttcatcgcctggcaatcacgccgcggcgacaacgcgctcgtgccgctcgagctgttccgcagcaagaacttcgcgctcgcggggctgaccatcgccaccgtcggtttcgcggtctccacctttgcgattccctggatgatctacgtccagtcggtgcaggcgtattcccccacccgcgcagcactgctcgtactgccctccgggttggtttccctcttcctctcgccctacgtgggcaaactcaccaacacccacgacccgaaacccttcgcgatcgcgggactcacccttgccgccgcctcgatcggatggacggccctgctcgcggacccggccgtcgacccccgctggatgtacctctcgtccgtgctctacggcgtcgccaactccctgatctgggggccgctatctatggtcgccacccgaaatctggagcgccgactcgccggctccgggtcgtcggtctacaacaccatgcgccagatgggcgcggtcctcggttccgcggcgatcgccgccgccatgtcgtcgcagttgcagaagcagctcggcgctcaggctggcgacaaccccgcggcggccggcgccgggttcaacggcccgctgcccgaggcgctccacgagcccttcgcccaagccatgagcaacgccatctgggtgccgtgcgcggtgattctcgcaggcgcagccctggcgtgcttcttcaaccgcaccgaatcctggaactcgtgagaaaaccgcgcgcgcccaaacgcgttatcgccggcacgtacccgatcaacaccgggaccgcggccatcctgccggatccgcttcgcgacggtgcgttcaccctcgaagtcaaccgtgtcccctcttcctacgtcgtgctggatgcgcccgaggtgctccacttcgactacatgaggtgggtagcggggttcgtcgctaagcaagcgcaacctttcaccgccgtccaccttggggcagctgggtgcgcactgccgtcctacttcgctcaccggtgggacagctcgaacaccgccgtcgagatcgacgcaggcctagccaagctcgtgcgctgggcgtttgacccgcctgtcgcgatccgcgtcgccgaggcgcgcgctttcacccacgcgatccccgcaggctccgtcgacgtcattgtgcgcgacgtgttcgccgggcccgccgtcccgcgacctttgaccacggtcgagttcttccgcgccgtccgcgcagcacttgccccgggcggggtgtacgcggcgaacgtcggcgaccgcgccgggctggcgcaaacgaggcaggagctcgccggcctgagcgaggtgttttcccacctcgcagtcgccggcccctcggcgatgctggacgggcgcgagtacggcaacctggtgatcgcggcgtctgatcgcccgctgtcgttcgacggcgaggtgccgtgccgcgacgcgtcttaccttctcgacggcagcgcgcggccccgccgggaccacgaccacggctagaactcgaattcggtgctaaggctcggctggtaaaacgcagcgcgctccacgttgaggtcgttgaagtggggggaggtggcgccagcaagcgcagcaatatagtccgggaccatggctttcgggatgcgcaaccccatcgtcaggtgaggcacccagcggtctccgcggccgtccgggttcatcgagctcaacctccgcgcagcttgctccagctcctccggtccctccatcagccaggcaatggactgcttcgacttcgtgccgaagacgacgacgccgacgcgtcggaacacggcgggcagcagcggaggcaggaccacagccgcctcccccaccacgcgcgaaggcattttcggcgcgaacgtaacggaaatgtgcgggcgctgcttctgcggcgggaacccttgttcctctagaacccggtaaatcccccgaacctcctcctcgtggctcgccgagagccggaggaggatgttttcgggggatcgctgcgacacctagaaacgaataccaaactgtgcggcgagctgcacgatggtgtcgatgttgaacgccagaacgccgagcagcgcgaacagcgccgccagcaccagagcgacgatcgagccgaccgagctacccgcggaaccctgcgccggtgcgggctcgttggtgttcgagcggacggtggaggtcacggtcgcggtcgcggtctcggtctgcgtctgggtcacggtctgagccggagcggcaccctcggtcacggtctgggtgacggtgaccggaacttcgcccttggtctccgtgaccgtctcagtgacctgggtggtctcagtctcggtcacggtcaccggagcggcctgctgggtcacggtcgaggaggcggtaatggtggcctgtgcggtttcagtgacctgctgcgtctcggtcaccttggcggtctcggtgacggtcgacggctgcgcggtttcggtctgcgtcaccgtcgtcggttcgagagtggtggtagtcgtctcggtcactgtcgtgggctcgagcgtcgtcgtggcggtggtggtcgcgaccaccgtctccgtggtggtcaccgtcggcgttggctcttcggaaggctgcggggtttccgtcggcgtgtttgtgcggtggttcagggtcacctcgtcaacgatcgagttgtcgtagacgttgtgggtgcgcaccgtgagtgcgtgcggggcgacctcgataacggagtagtccggagtgcggtcctggttccaccacgcgatcgtcggctggccgaggtcgcgctcgcgggcttcctcgatggtcatgtcgcggtgcttcttgccgttgcggtcggtgaagtcgtagaacttgccgccgccggcggtggacaacgtcatgtacaacacgtcgccctcggccgggttcagcacgtcgccaggtgccgcaagctcgtccgggattgtcgcctcggtgccgttaaccaagtgcgagcggttgtgcatgtggtcgtggccggagagcacgagatccacgcccacctcggagaagaccgggccgagggtgttgcgcatcgccacgatctcgctgttgtcgtagcggccgccgtgggagtacggcgcgaagtgggttgcggcgatgatccagtccttgccctcgccgtgctcctcgactgccttgcgcacgaacgcggcctgggtgtcaagccccttctggtctttgaggttggagttcaaaccgatgacgaggacgttgttgaactcgaaatagtagttgtggtcgccgtcgtcgttcggcaggttgaagtgctcggcgaagtgggactcaccagccgagctcgggtaggtctcatggttgcccttgaccacgccggtgcggtacgcgcggatctgctccggcgagaagaactcgtcgtactggtcctcggtgttcagccagccgttgacctggtcgcccatcagcatcaggaacgaggcgtcgctgtagtggatggtggacgcgtttgctgcgtcccgccactgtatgccctgctgcgcgatctcgttggcgacaccaatctgcgcgtcagcgaacgcgaggaagcgccaatcgccctcggcggcgtcggtgacgaaacggtgcacgccggaccagccgccctcgtcagagcccacctggtacaggtacgaggtggacggctcgagaccggtcacgaccgcggtcagcgaacggtagccaatggcgcccttgtccctgtcgttggccttcaccacggttacctgatcaggctcgatctccttggcgatgcggacatactcggcgcccctgaagttcgaacgccacgtcatgttcgcctgggaggcgtcggcgccgatgcctgtaatggcgcggaaggtcgggttgaaggtgtccgcggacgcgggagccgggacggcggcaaacgtcagggctgcgacgacggcaaccgacgtcgcgcgggtggaaaagcggcgagggacgatagcgatggacacggggaatcctccgggaatcgagccaggtaagactttggcagcagtaatgaccacgtcatcccaccacaacaaggtaacgccaaggttgctaacagttgccgggaaggttacgtttccccgcccgcgctaggatggtgcacatgaaaaacgatcccgcaaagcccggctacaccactgacggttcggccaacaagcccgtcgaccacgacgacgaccagttcgcgcaggactccggctccgcgctcggttacggcgaggaagccagcgacgatgttgaagaagcgcagatcgtctacgacgagtccgtcgaggacgagggcgaccacccgacgcttaaggactaaacctcccagcgcgttagatttcccagcgcacctcggcgggcgacttgtcgtcgcgccacccccgccagcttgcttggcggacttttccgccagcagttttactggctaaccgcacctcggcgacgcgcttcggcgtcacccagaacaccccgtcgcggtcctctttcgggacctccaccggcggggttttgcgttgcatgcgccgaagttcgcgctctatcgccgagaactccttgccgctgaagccggtgccgacgcgcccggcgtagcgcagctcgccttcctcatccggcacggccacgagcaagcttttaccttcgcgcacaccaatgaccacgacttcttggtgcaggtcgcgcttcactttgagccacgcgcttgaacggccaggctcgtagtacgagctggtgcgcttggccaccacgccttccagacccatctcgcctgcaaccttccaggcggaggcgaagctgccgcgaaacactggtggcacggcgacggtggtgttgttgccggtggcgtcggcaagcttctccagctcagcgcggcgcactttccacggcacggcggtgaggtcgcgctcgccgatgcgcagcaggtcaaacgccatgtagcggaggttcgcctccgtctccccgttgcggtcggcgttgtgcagcagcgagaaatcgggcacgccgtctgaattgagggcgatgagttcgccgtcgaaggtggcgtcgtcaagcatgagctctatctggggaaacaagtgcgtgtattccttgccgcctcggctgattaaccggacgccgctgggggtggcgtcggcgaggatgcggtagccgtcccatttcatctcgaaggcgtactcgaccccgtctttcatcgcgagtttgatgtcggcttcggtggcggcggtggcgagcatcggggtgggcaggtcggcgggttcggcgg

SEQ ID NO: 17 - DNA, 44965 bp, Corynebacterium cassirii
  source 1..44965: mol_type = genomic DNA
gggctctcagccttaccgccgccgccaaccccgacccccccccccccccccccgcaccccccaccgccagcaccttgccccctgcggcggccgggaccgttgcgcgctgtgtcaacatgccaagcgcgcgcaacagatccggcgcctgcgcgggcagggcgaacgcgcgcgggttagcgggatcgggctggtcggtgacgacaaagacgttgtcgctcgggtgggaggggtcggtgtgggggttgaagggggcgtcgacaagcagcgcaaacgctttgtgcctgctgcgctcgagcgctgcggcgtcgcggacctcgacgactgggcggccggtggcggcagcgatgtggagggcctctgggtgcacgagcgggtgctcgacggcgacgactacgggacggattgcggcggtggattgcatggcgctagcgtgcccagcaaaaactagccggtcaacggccggtagcccgattgtggataactattttctgctggccccgaaatgccacctgcctgtggataaccgcttgcgcgtgcaggtcgtttttactaacgccgcccccttctagggcgcggtacaaaaggtcaccagcaaagtgttgcttgcagatggtcatcaaccgggtaaacgcaacgagacgattttcctcgacggcggttagtgaccatttggtggttaccatttggaggtcacccgcgtcgcccggacggctacaatgacagggtatggttgctcacgctcaagcacacgccgcggcgttttttgaccttgacaagacgattatcgccacgtcgtcggcgttcgcctttggcaaggagttcctccacaacggcatgattagccgcagcgaggcgtgggacatgtactggtcgaaggtctcctacatgctggtcggccagtcaagcgacaagatggacagcacccgcgactcgctcgcggagatggtcgcgggctgggacgtcgacgacgtcgcccgcatcaccgaggcgacgatgcgcaccgtggtcaccccggctatttacgcggaggcccgcgagctgatcgacgaacataaacgcgcaggccacgacgtgatcatcatctccgcttcggcaaagattttggtcgagccgatcgcgcgcgaactcggcgtggacaccgtcgttgccaccgagatgagcatcgaagacggcaagctcaccggcgaaatcaccagctacctcaagggcgaggcgaaggcggatgccgtgcgcgccttcgctgcggacaacagctacgttctccaggagagcttcgcctactccgactcggcgacggacatccccatgctttcgctggtgggccaccccaccgcggtaaaccccgaccgggctttgaagaagcacgcgctgtctcacggatggccgatcctgtcgtttaagaaccccgagccgctgatgcaaatgccgaacgcgaaggaggtcaccatcggcgcgggcgtggtggccggtgtcgcggcgctcatcttgggcgcaacgctgatcacccgctcactgcacaaggaggtcaaaggcccggatgccactgcgcaagacgcgcagtgagcaggcgctgcgaatcggtgtcagcggcgtggttgccttccaccgtgccacccaacatcaactgccaaccgttgcccaccgcctctgcgtccgggaagaagacgtggcccgcgccgggatagacgtgcgcctcaacccgtgggttctgctccgccagcgcacgcgccgcaacgtcagagggccacatttggtcgtcctcgccagcgaacgctaggacgttgccgccgaagcttgagacgtcgatgcgcgcgtcgtcgcccgcggcggccgccaactgttcgtagacgctccggtagctagttggataagcggtcatgccttcccacatcatcttcagccccgtgcgcgcaggcagcgtgcgaaatgacgcgtacggcagctcctcgccacggtcggtgaaagatcccccgttcatcccgcccgatggatccagcccgttgtaggtgtagtgcgccggcgcgaaggccaccacgttgtccaccgggtagccgtgctcggcgagcagcagcgcgaactccgcgcccttcgacgacccgatgacggtcaccggccgcgggtcggcgatatgtgcgtcaatgtagctttccacctcatcaaactgctcgaggggcacgcccgccagcgccggccgctggttgtcttggccgaagaaatacaggctcaacacctcataaccggcatccgcgagctcaaccgccctgcccagcgccgccgacccctccgacccgccgtaggtcaccaccacacctgcgtatttgcggtggtcaggcactacatggaacccgttgaggtagtcccccgcaatggggctcacgcttgacgacgcccccttgatctccccctccgcccccaccaagtcagtcgactccatcaccgggaatcggttcgtattcacggcgcgaacgactcccaccaccacagcgaacgccaaggccaccatcagaagccccaacactgccttacctagcccgcgcagaaggttcatacgcgtcattaaaccaaaaaaatctcacgtcaccggggcatgtattgggcacggcagcgaaatagtgattagtcttagcttggataacgcttgaaaacggcactgtcgcttaaggaaggttagaacagtgagcaaagaaggtctctacactagcggctccacggccgtgtccgcgaaggtggattcgatcccgctgaccgacaccggggtgacccagccgggcaaggactccatcggcaccctcatctccaacgcgtctgagcaggtctccaccctggtccgcggcgagatcgagctggccaaggctgagatcgtcggcgaggtgaagaagggtgccctcggcggcggcctgttcgccgctgccggtgtcatcgcgctttactccacgttcttcctcttcttcgcgctcgctgagatgcttgcttcttggatgcaccgcggctgggctttcctgatcgtcttcctgatcatgctgctgctctccggtctgctggcgttcctgggcttccgcaagctgcgtcgcatcaaggctccggagcgcaccatggagagcgtctccgagctacgcaacctggtcccgggccaggcgcaggagaacctgcgcaaggacgagtccggcctttacaccaccgccccggtggcagcgccgaacccggctccgacccgcaccaccgcgcacgctcacaccgagccgcgccgcaccgcgccggtgaagaccgtcaagacggtcaccaccgaaaccaccacccgcgacggttcgaccggcggctccaccgcagtgacccggaagtaggtcacctcccccgcagcattactcgcccgcagtcctcactaaggaccgcgggcgttgctcattcccaacacccgcacaggaggtgaccaaagaccgtggcagccgcgcactccccaagtgtggtggagctttccggagacttcacccaccgcatgctccacacccgcggtgtccgcctgcacgcggccacggccgggaaccacaacgacccgcttgttgtgctgatccacggcgccttcggcggctggttcgacttcaaggacgtcgttgccccgctcgcccggcgcggcttccacgtcgcggcgttggatgttcgcggctacggcatgtcggacaagccggctgcccgcgctggggatctcctccacctgctcgccggtgacaccgccggggcgattcgaacgctggggcacgcgggtgcgacgctggtcggctcggatacgggcgcagtgattgcccgcgcaacggctagccgctaccccacgctggcgaccgacgtgatcgttcttccgcagtcgtcggggcgcgcggctcgcgcgtcgcggctgcccgcgcggctgccggccaaaatcgccggcgcaagtaaccacgcactcgacgcgatgtggcgggccaacctgatggcggacaccaccgacgcctttcaccgcaccggccgcttcaacgagttcctccagttacgcattgcggcgcgagacatcgacaacgcgctcccccacatcgcggcgacgtcgcgcctgcgcccgcgcaagttgccggcgacgccggggttcggccccggcaacttgccccacatcgaggcgccggacgtgttcgtggacgctgtggcgcgcgccctggctgccggcgcccgctagagcgccccgacgcacacctgcgtatccactgccgcggtgagccgctccacgtccccgatgcgggagcggacttggtcggcggtgagcgcgtagcccgtgtcggatgaatccagggacgcgccgaagatcatgcccaccacgtcacctgcggggttcagcagcgggccgccggagttgccctggcggatctcgccgcggatgacgtaggcctcgcggtcgacacgcccgcgggcgtaaatgtccgggcccgagatacttaggcgaccgcggatgcgggcgggggccgcttcgaacggcccggagagggggtagcccatgacgagggtgtcgtcgttgagcatcaagggctcctgcgcccagcgcagcgggtcgatgcccagcttgtcggcgcgcagcacggcgatgtcgacgtccgggtcgtagtagacgacctccgccttcttcatcccgagcaccgtgtcgagggtgaccgcgtcggtgccggcgacgacgtgcgcgttggtcagcacgtagttgtccgcgaccacgaacccggaaccggtgagcttgcgctggcaggtgccggcatcacccatgacctgcacgacggcagcgcgcaccgcctcgaccacgtcggggtcgaggacgtctgggtcgggagccgcgacctgcgcgccgcgcggcggatcgaacggggaaaccaaaggcggcaggccggactcgtcgagcatggccgcgagctttgccgggaccttgcccacgccggcaggtgcggccgcgtcgattgcggtgaagaccttggagccgcgcacagcgtcgccgacctgtcccggcaaggccgcggccagagggatggagatgaaccacagcaccagcgccatcgccagcgcctggaacccggcgccgaagagcgaatcgacccggcgcgtggtgcggctgcggacgctgccgcgcacctgcgcaccggctgcggcgcccgcggcgttgccgacgctgacgaacacaaccacgagcgcgatgagcagcgcgacccgtagcgtggtggagtcggtcgccgacaacgcgaacggggcgatcgccagccccacaatcaacccggagaccacaccgacggccgttatcaccgcggcgagcgctccgcggcgccaacccccaacaagcgacaggccgatcacgattaccaggccgatatccaacagcatcgcggttaactttcgtcgttgcacgaacgcgcgagcgctttgcgaaggtcttggggctcccggtcccactcgccggcccagccaccggcgtcgagcaccaccgacagcagcgcgccggtgaatccccagatcaggtagcacctcgcccagaacgccggacccgaccacagtttccagccggcttggatgcggtttaccgggtccaccagctcgcgcaccgggacgaagaagacgtcgtcggtttcgatctcgctggcggggtgcactgtgcccgggctcgccgagtacgccaccacaggccgcacgcggcggcgtgaaccgccggttgtgacgggggccatcaccgcaagcggcaccacgcggtcgcgctcgagggcggtttcctcgtaggcctcacgaagcgcggcgtcgacggggccgcggtcgcctgggtcgatgcggccgcctggaaacgccatctggccggagtggctgcgcatcttcgggtggcggtgggtgatgagcaccgcggcgtcgtcaggcaactgctccgcagacggatcccccgtgaacaggatgagtaccgcggcctcgtcggcgccgttgcgctggggcacccggctggccagcatggtgcgcacacgcgtcgcgtgctccggctcggccagcgccgtcagtaacggtgcaagccaccgcggggcgcgctcgggctgcagggcgacgtcggccatttagagcacctccgccacggcagccgccagcgcgtcggcggagtcgaaggtgcgcgggaacatcccgacctgctcctcacccacgaagacgagcgtaatcggcacaacacccggcaagccgagctcgccggcgaagcggccggtgtcgtcctggtagctggctaacgcaacacccaactcgttgagcaaagcagccccgcgggcggcgtcgggatccgcgtgcacgccgaccacctcgtactgcgggttggcggcggcgaactgatccagcaccggcagctcgcgccggcacggatcgcaccaccacgcccagacgttgaccacgcggaccgcgtctgccgcggggcgctcgccggcctcggagccgccgaggcacggcaggtcgacgccgccggcgccgcctggcaggcaatcgggccgccgcggcacgggctgcaccgcgggcgcggcggcagagttttctggcgcagcattctccccgcccccgcccgcgccgccgcgcagcatcgccgcagcccctgcaaccaccaagacggtggccaccacggcaccggccacgctcagcagaacctggcggttcacttgtccccctcgtagtccgccatcgcgaggatgtggtcgcgctcagcgcctgtgaccagcgcggcggcctcggcgggctcagtaggtcccacctggccgaaactcgggcagtcgaacgcaaccgggcacaccccgcacgccgctttgcgcgcgtggcagacgcgcctgccgtggaagatgatgcggtgggagaacatggtccactcgctgcgttcgatcaggtcgcctacggcgtgttcgattttggtgggatcggtggcgtcggcaagcatgagccttttgaccaaccgctggaaatgcgtgtccaccgtcagccccggcagcccgaaagcgttgccgcggactacgtgcgccgtcttgcggccgacgccgggcaaggtggtcaggtcctcgaccgccaccggcacctcgccgccgaaatccgttaccagcttctgccccagcccgatcacgttcgcggccttcgcgcggaagaacccggtcgggcggatgatctcctccacctcagcttggttggcctgcgcgtacgcctccgcagtggggtatttcgcaaacaaagcgggcgtgacctggttgacccgcacgtcggtcgtctgcgccgagagcaccgtggcaacgagcagctcaagcgggttggtgaaatccagctccgcgtgcgcgtcaggaaacgcctccgccagcgtgcggttgatgcgccgcgcgcgccgcacccgcccaaggtcggtctccttgcccttcgccgcagggtgcgtccccgggcgccgatgggcttttttgcttatcgacgtcaccttcaacaccctacaatgacgaccatgatgatcctcgctgccgtttccgtcccgctcgccttgggcctgttcaccgtcgcgatggagcacatcgagcgccgagtatgaccgtttccgccccagcgctgcaaacgtgttggtaatctcagtgaggtctatctacaaggaggttcaatggaaggcgtgcaggagacccttgcccgtgcgggcatcttccagggggtggaccccgatgcggtggccgagctgatcgaagatatggagacggtgacgttcgcccgcggcaccaccatcttcgacgagggcgagccgggcgaccggctctacatcatcgttgagggcaaggtgaagcttgcccgccacgcaccggacggccgcgagaacctcttgtcggtgatgggcccgtccgacatgttcggcgagctgtccatcttcgacccgggcccgcgcacgtcctccgccgtgtgcgtcaccgaggtgaccgcggcgacgatggactcggtaatgctgaagaagtggatcgacgagcaccctgagatctcgcagcagctgctgcgcgtgctggctcgccgcctgcgccgcaccaacgcctcactggccgacctgatcttcaccgacgttcccggccgcgtggcgaagacgctgctgcagctggcgaaccgcttcggcacccaggaaggcggcgcactgcgcgtcaaccacgacctgacgcaggaagagatcgcccagctcgtcggcgcctcccgcgagacggtgaacaaggcccttgccaccttcgcgcaccgcgggtggatccgcctcgagggcaagagcgtgctcatcgtggacaccgagcacctcgcccgccgcgcgcggtaggcgctttcgaagcgcctacgccctaccgctcgctgctcaagtaccgcagcgccacgcgggtcgactgctccgcggcgccgcggagcaccgggtcaacgtcgtcgtagattgcgtccacgatggtgttgatgtctgcgtcctcgccgtgggtcttcagggcctcgcggatctgctcgaggcgctggttgcggcggtcgatgtacttgcgggcgaaagcggagaggtcctcgccgtctgggccgtggcccggcaacagcggcacgcctgctccggcctcttcgagcttggccagcgattcgaggtaggcgcccaagtcaccgtcggtctcggagatcatggtggtgtggcggccggcaatggtgtcaccggtgatgatgccttccagctcgctgtcttccgggtcgccgccgtagacgaagaagcagacggaatcggaagtgtggcccggggtgtggaccaccttcagcttcggcgtgacgccctcgacggagacaacctcgccgtccgtcagcgcctcagcgcccgagcagtactgcgcgtcgaacgcgcggatcggcgccccggtgagctggcggaagcgctcagcgccgtcggcgtggtcgtggtggcggtgcgtgagcaagatcaaggcaactttgtccgccttcgcctgcagcacgttgagatgaccctcatcggccgggcccggatcgacgacgatgctgtacccgtcctccgggtcgcggaccacccacgagttggtgccctcaagggccgcgtagctggggttcggcgcaagcacaacggcggccgaagccgtcactgggcgcagctggctgtaagcggggtgtttcatagcacctagcctacagggcctgccgcgccacgtgccgttttacgccagctccaccacgagctcgagctcgaccggggcgtccagcgggagcaccgccacgcccacggcggaacgggcgtggctgccggcctcgccgaaaatctcgccgatgagatcggaagcgccgttgatcaccttcggctggccggtgaacgacgggtcggaagcaacgaagccgacgaccttgaccacgcgggcaacgttatccaagcccacgagcgcatccaccgcggccagcgcgttcagcaccgcctggcgcgcgtagcccgcggcctcgtcctcgctcacctcggcgccgaccttgccggtggcgggcagcacaccgtccacgaacggcaactgtcccgaagtccacacttggttgccggcgcgcacggccggcacgtaggaggcgaccggcctagctacgcccggaagctcaatgcccagctcttgcaggcggcttaaccacgcagccatctactcggcctcgcgcttcatgtacgcgaccatattgtcgggggttggccctggggtgacggtgaccagttcccagccgtcttccccccaggtatccagaatctgcttggttgcgtgcgtgagcagcggcacggtggcgtattcccatttcgtcatggcgtccaccctaccgcggcgcgggcccgcacccggcggattatttacagaccctcaacctccgcgccggaggcgaggtgggcagcccaatcggtgacgtgcgggttcttgcgcagcaccgcgcggcgctggcgctcggtcagcccgccccagacgccgaactccaccttgttgtccagcgcgtccgcgcggcactccgtcagaaccgggcagtggcggcacacggcggccgccttgcgctgctcagcgccccggacaaacaaggcgtccgggtcgccgccgcggcactgggcgcgggtcacccaatcccctcgatcgaattccaggtggccagaggcgttgctcttgcgggcggtggtcagcgtcgtggtcattaccaacctctttcaaacgaggatccgcgctcgcgctagtgaggctgcggatgcttgtagaagcgaatttcttcgattcccaacagaatgcggtacgcctgtaagtgtattcacaggtctcaatttctgtcgaatggatcacaataatggggggagtggttcattcccccaccgcaccggcatcatttactgtaaagagcgtgtctgccttacggtccctaggaaacctgctggccgccatggtgacggcggggcttgcgatggcgatctgcatcgccccgatcgccggcctcggcggcatggcggtcgcgcgcacggatgagacgatgcagtccaacctctcggacatgtccggcggcgaggtgcccggcgtgaccaccattacggacgtcaacggcgacaccatcgcctggctgtacaaccagcgccgctacgaggtggccagcaacgagatctctgaccacgtcaagaacgcgcttgtgagcacggaggaccgccgcttttacgagcacgaaggcgtggacatgcaaggctttgcccgcgcgctggtgacaaacgtcttggccggcagcgtggagcagggcgcgtccaccatcaaccagcagtacgtgaagaactacctgtggctgatcgacgcggaaagcgacgaggacgccaaggccgccaccgagcagtccatcccgcgcaagctgcgcgagatgcgcatggcctccgacttggacaagacgctggacaaggaccaaatcctcacccgatacctcaacctggtcagcttcggcaaccacgcttacggcatcgaggccgccgcccgcacctacttcgacacctccgcccagcgcctgaacccgggccaggccgcacttttggtcggcctgctgcagtcggtggagtacttgaacccctacaccaacccggagggcgcgaaacagcgccgcaacacggtgttgatgaacatggcggcccagggctacctcccgcaggaagaagcagacaggtacgccgccacaggcttaggagtgctcgagaggccttcgctgcttaccgacggttgcatcaccgccggagacaacggcttcttctgcgactacgcgctgcgctatctggccgacaagggcttaagccaagaggagatcgagcgcggctcctacaccatccagaccacgctcgacccggccattcaagccgcggcagtcggcgcggtgcgcaacaacgtcgcgccggaaacccccggcgttgccaacgtgatcaacgtggtgatgccgggcaccgattcgcgcgacatcgccgccatggcgtcgtcgcgctactacggcctcgacctggatcagagccagacgatcatgccgcaggcgtcgtcactcgtgggcaacggtgcgggatccgtgttcaagatcttcaccgcggctgccgcgatcgagcagggctacggcctcgacaccgtgctggaggtgcctgcgcgctcggtggtctacggcatgggcaagggcggcgccgagggctgcccgccggacgcgtactgcgtggaaaacgccggcatctacccgccgcgcatgacgctgtcggacgcgctggcgcagtcgcccaacaccacgttcattgagctgatccagcgcgtcggcgtggcaccggtggtggatatcgcggtgcgcttggggctccgctcctacctcgacgagggcacgttcggcgacggccgctccatcgccgaagccgccaaggaagagaacatgggctcgttcaccctcggccccaccccggtcaacgcactggaactgtccaacgtgggcgctaccttggcgtcgcgcggcatgtggtgcgagccgaacccaatcaaatccgtcaccgacgagcacggccaccaggtcttcatcgaccgccccgcttgcgagcaggccctcgaccccgaggtcgcgggcgcgctcgcccagggcatggcgcaagattccaccaacggcaccgccgcccgcgccgcgggcttcaacggctggactgccccggttgcagcgaagacgggcaccaccgagtcgcaccagtcctcggcgttcctcggcttcacccgtggcgtggccgccgcgccgtacatcttcaacgacggcacgcagacaaccccgctgtgcactgggcctgtgcgccagtgcccggtcggcaacctcttcggcggcaacgaggccgcggacacgtggttccaagcggctgcttgggtgccgggcgcggcctacgcgggtctgccggaatcctcgtggacgtaccgcaagggcacccggcgcgcagcgctggatgagacgatcggcatgcagtccgccgctgcccgcgccaagctggaggctcagggcttcacggtcacggtggtgacggtcagcggcggcggcgcgccggtgggcgaagttgtttccgcggaagcgagcgaccccaacctctcgcgcggctcggtgatcacgctgaacatctccgacggcacgggcacccccacctcgtcacccaccaccacaacgggcacgccgacgacaaccccgggcacggcaaccagcacgcccgcctcccccacgggcacggccgcggttcccacccccacagaaccggcgctcgacctcgatgacttgcagcgccaattcagcgacgtcaccgagggcatcgccggcatctttaactagctcaggcgagccttgaccgcctcggagatgcgcttgccgtctgcacgcccggcggcctgagcagtcgcctccttcatcacctggcccatctgtgccatggaggtggcgccggtggaggtgacggctgcgtcgacaagcgaagctagctcctcgtcatccaactgcttcggctggtactcctccaggatcgctgcctcggcgagctcctgggtggcgagatcctcccggccgttggtctggtaaatctcggcggattcgcggcgcttcttaatttcgcgcgcgatgatcttctggatctcctcgtcatcaacctcgtgcttggagccctcggtctcggcggtctggatcgcggcgagcagcatgcggatggtgcccgtgcgctccttctccttcgccttcatcgcttctttcaggtcggcgcggatctggtctttcaattcactcatgggctcgagcgtagttgagcggtacagtcgacgggatgaagcgcacccgcccgatcgccgccgtaggagcattaggcttatcgacgctcacctactcccacctccaaacccgatcgtttgtcctccagcagtacgacctcgagctcctcgcaccgggcgcgctcccgcgcggcaaggactcgttcgacatcctgcacgtctccgacctgcacatgatccccggccagcgggagaaggtcgacttcgtctccggcctggccaagctcgagccggacttggtgatcaacaccggcgacaacctttctgacgctgcggccgtgccgtgggtccttgacgcgctggacccgctgctgtcgcgccccggcgctttcgtcttcggcaccaacgactactgggcgccgcggccggtcaacccgctgaagtacctcaccggggcaaagcgcacgccgtcgtacgtcgacctgccgtggcagggcatgcgcgcggcgttcatcgagcgcggctggcgcgacgcaacgcacgcccgcctcgagttcaaggcgtcggacgtgcgcctggcgatcaccggcgtggacgacccccaccacgacctcgacgactacgcacaggtcgccggcgcccccaacgcggatgccgacctcaccatcggcctcctgcacgcgccgtaccgccgcgtcctcgaccagtttgaggccgacggttaccagctcgcgctcgccgggcacacgcacggcgggcagatccgcctgccgggcggccgcgccatagtgacgaacgcggacatcgaccgcgagcgcgcctccggcctgcacgtctacgggtcgatgtggatggaagtctcccaggggcttggccaatctaagtacgcaccggtgcgcttgttctgcccgcccgcggcgtctctcatccgcgtcaccgagcgttcgaagtagccttgaactggcgttttggttcgtgagagcgccgcgagtacgctgtatcgagtaccgcggagcttctccgaaagtacaaccgggatatggcgcagcttggtagcgcgcttcgttcgggacgaagaggtcgcaggttcaaatcctgttatcccgaccaacaacctccagggtttatgccttggaggttttcttttgcctacgccggtgtaaccctcggccggcgcttagcgttctaacaagtgaccccttactgaccaaagaaggagccacccatgtccacgccccgtcttgccctcgcgaccgcggtcgcgctaggcctaaccacgatcgcctctcctgcccacgccgccaccctcggcgatcgcacgcccacaaacgagtgccgcgtcaccctcaccgccgacgagcagaggttcgcacgacagcttttcgacgaccgcgccaagttcggcgaacacgaacgcgcccgcgacgagatcgccgcgattgagcaggtcttccccgccgcgaagccggtcggcgaccacctcttcgccgcaggcaagcccaaggccggcaccgtatggacgatcgcagcagcggaccgcgcggggttggaaaaggcggggttaggggcttcgcttatcgacgcctacgccaacgcccacctcgaccaactctggcaccagcccatcaagaacccctccgacgtgaccaaggaagacatcgacctggctaactggaaggtgaaggccgactcgagcggggccaaccagtccgctcggatcgcgacggtattcccagtgaaggacccgtcgacggtggacaaggagaccctggccaagctgacggacgcgtgggtcgctacccccaccggcgagtactccaagcgcgagaacgcgtttaactcggcgcagaagcaggccgcgcaggcctgcgcgctgggcaccagcaaggtggtcgccttccctgagcagcagggcgatctcaccggaccgggtcttggagtcgggtcagtgagctccgagggcagccgcttcgacatcatcgcgggcgtagtgatcacgatcgtcgtggcgatcgcgggcctgatcgccgccgtgccgcagatccgtgaggcgttcgcctcgctgctgccgaagagctaggaagcgttaggagcggggctcgatctcgctctcaacgacccacttgtgccgcttcatcgtcatgtcggggctgtcgatgtcgaccatgtacaccgtctcgtcggtggaggacacgatggtcgcctccgcaccctccatgccttgcatgtggttggcgaggatggttttggtggtgccgtcggcaagcaactgctcccccgcatcctccagctcctcctgcacaacccacttgtggtcgcgcacgggctcgccgccgtccgtcggggtgtaatcgatggcgtaggtgtaggtgtcgaacgcgccggagatcgtcgcgttggcgccgtccatgcctggcatgtggtcagcggtgagcgtgacctcggtgccgaccgggtacttcgggttcgccgcctccttgatgccggcaggtgccgggccgccgtcctccgggtggtcgtgggctgcgtggtcggtgttgtcctgcgtcatcgtggcctccgtttcagtggtggtgtccgtcgtcgagcaagcggccgcgccggtgaatgcgagcgcggccactgccgcggttgcgagagtgcgtgctgttgtttttaccatgtgccccactgtacgcgtgcgtgaaaacgcgaaacaccctgcggaaaccggttggtcaccgcagggtgttggcgtgaagctagcgcttggggttagcggctgctcgagcccgcgatcgggccgaggagcgcgtcaacctggaacgggaagatcagcgcgatgatgctgaacagcgccgtcaggccggtcaggccagcgaggatccagaggatgatgctggaggcggaggagccggtggccggctgctcgaccggcttctcagtctcccacttggtgccgagattgaccgcgccgttggtgttcaacgcgtcgatgccgagcgccttgttcacggcgaagaagatgtcggtctggtcgatctggccggtgatgttcgcagcacccgggccggaggccgcgatgcgcagctgagcgccggtgtgctcctggccgccgagggcatccttgtcctcgttggtcttggaggtagcgaagttcaccgtcatgtcggaaccgtcggcggtgcgcagcttcgtggtgcggccggcggtcacggcgtcgttgtaagtgatctgcgcggtgtgagcgtgatcagcggtagcgatgatcagcgtcggctccccagtcttctcaacccactgctgcactgtctggacagcctcgtcgagctggccaacctcaccgatcaggccgcaggcgtcagcctggtggtcggccttgtccggggaagcagactcgacctggagcaggaagcccttgtcgttctgcagcagctcaagcgccttggtggtcatcgcgcccaggcgcggggtctccgcagtgaactccgggttcgcctcacagacggcggcatccgccttggcgccctccagggtcgggatggtctgctgcagcgtgcgcggcatgttgccctccgagaagaggcccagaaccggcttgtcagcgttcgcctcagagatggcctcgagctcagctgcgttggtcacaacctggtagttgttgtccttcgcgttctcgagcacggacttgccggcggtccaggtggtctggtcccacttgccacccttgaccacctcggtgtcgaagtacttgcggccgccgccgagcgtgacgtctgcacgcaggtccaccagctgctcggagatggagccgaggccgccgttctcgcgtgcgtcctcagcgccgacgaccttcttgtcgcccgacggcgcgtagtaggagcgcttccgcgagtgcacagcgaacgcggccggggtagcgtcctggatctcagaggtggtgacgttaccgatcttcaggccgttggccttcgccagctcacccagggtcggaaccggcttgccggcgttgtccacgccaagcgcaccgttgtaggtcttcacaccggagttccagccggtgccggaggcagcggagtcggtgacgtagttcggcagaccgctctccttgtccagcgcccaggtggtctggtagccggtgtagtcgagggtgtcgaggccgtcgaagcggcctgcggagcccttgaggtagttgcgagcagcagtgatttcggagtcgccggtgccgtcgccgatcagcagcacgacgttcttcgccttgtcgttgtcgataccctgaccctcggtgccgaactgcgcacaatcgccaaccttcggggcctggccagcggagaccatgtagcagagctggtcgcccggctttgcagagcgacggttagcaaggttcatcaccttgttgcccttgttgatctcccacggttcctggccaccctcggtaccaccgttgaggccaagcgcgttggccataacgtagaacgcgtcggtctggtccagctggccgttgacgttctcggagcccggaccgaagcccgcgatgcgcacctgggcgccggtgtgctgcatggaaccagtcttgaacttgccgtcctccacggtccacggctgggtgccgaagccgacggacatgatcgcaccgccgtccttgggcgactgcagacgggtaatggcggagacagactcttcaccatccggcacaatctcagcggtgtgggcgtggtcggcggtgaccacaacgagggtgttgccgtcttccttggcaaagtcaagggcttccttgattacctcgtcgatctgctcggtctcgccgatcatgccgcaggcgtcagaggcgtggtcagccttgtcgatggaagcggactcaacctgaaggaagaagcccttctctgcgttcttgtcatccagcagctcgattgccttcttggtcatctctgctgcggtcggctcgttgccggtgtcctgcagcttgcactcctgcggctgctggtccttagcgtggcccggcacggtgggctcgtagcgacgggtcatgttgccgtcattgaacaggcccagaaccgggttgtcctggttagcgaactggatcttctccaggccttccttgtcgtcgacaacggtgaagcccttcgcaatagcgttctcgcgaacggacttgcccgcttcccagtcagcaccgccgtcgttcttctcggtcaagaacgggttacggttctcgccgccttcctgaacctcggtgtcgaagtacttgcggccgccacccagagtgacgtcggcgcgggtgtcgatcaactgctcggagatggagccgaggccgccgttctcgcgggcctcttcgcccttgacaaccttcctgtcaccagacggagcgtagaacccgcgctgcgagatgtgcgagcccaacgcgcccggggtcgcgtcctggatctcggaggtggtcacgttaccggtgcgcatgccggcgttcttcgccatctcgaggaggttctcgtgcggcttgccctcgatgtccacggacagcgcgccgttgtaggtcttcacaccagcggaccagccggttgcggacgcagccgagtcagtcacgtactggcgctggccgtccttgcccacagcgaaggtggtgtacgcgccggatgcggtcaactcgtcgagaccctcgaagcggccgttggcgcccttcaggtagttgcgggctgcggtgatctcctggtggcccatgccgtcgcccaggatgaagatgacgttgcgggcctgagcgtcggtgttgccctggccgcccttgccgaactgggtgcaatcgcccggctgcggagcgcggatgttgccgttggaatcgatggtgatgcaggactctttgccgttgaatgcctgctccgccggtgcggcgagagcggcgggcaggttcgacatcgcgagcgcggaagcgctgacaatggcggctgctgccttgctggagaagcgcatgagaactctttcttcgaaaaagctggtgaggatgaaagcaatcggtttttaaaccgataggtaacctatccccagataattgccagcaaacggcatctaagtgaactttacgttacagcgccgtttggccagctcagaggttctttttaattcttctctaatgaaaacagttcccagttagcggtagattccaactaacccatcaccatcggcatcgcaacaaccgcagcaccgacaactgcgaccaacgccagcagcacaccgatgacaatcccagcggagctcgacccgccaccgcttggcgcaggcgcgttcgacgccgtggacgttgtcggcgacgtctttgtcggcgtcttcgtcggcgtcgtctgggtggatttagtggtggtggaggacggcgcgggggctttctccgtcgtcggcaccgcagtcaccggtgttccggtcaccgcgggatctagggcgcgcggcgcattcttcgacttatcaagagtgaaggtgcgggttcccgatggttcccgcactgtgaattcggggataacctgggccttttgcccgtccgtcagctccacggtgtaggtgacgttgtagcccttggtgtcggtcgggttggacaccgtgcgaactccaagacgcgcccgagcaccatcagggaggtagaacggcaccccgctcgactcggcgagtctagttattgcatcggggataaggaacgcattgcctcgactgtctacgcgtactggcagctcgccggtaaagaacatcgttgtggcccacacctcgccgtctgatgttcgaacgagaccaaggcccatcccctgaaagccggcactcagcatgtttgcgttgtggtctggtgagttccgccagagttcgaagagatcttcggccgcctgtcgccagccatcaggcgagtcattgtacgggccgccgaggcaatattttctcccgaataccccatcgtctcagggttcgagtgacggaacgcgccgtcgtaaaccatgacctcaccctcgaactgcgggtgccccagtgaaggatcatccaggtctgcgatcatctgctgagtccaggcgagcgcctggttgtcgtacagctcatgggtgaccaatgcgtggagtccattagccacgcgatactcgttgatcagctcctctatcgcctgggcagcgaggcgcgcgtcccgcgaagcttggtcgacggcagcagtaccggccggctgcgcagctccaaccggtgcttcgactacctgggcaactgtgaaagggagcgctacagccagggcgagcgcggcaatgcgggtgcgtttcgtgcacgcacatgctacgcgcggaaacggcaaagcgcccactttcaagtaaaagaaagggcggcccgttaccggaccgcctttaggctcattccactacgtcagaaggtctgcctagcttttcgacgaaccgagcacagtcatcccgttgtcgaaaccctcctcggtacatgcctgcgcgatgagtacgccggtcaacgagatagccgcgatggcgccgagggcgatgcccagcggctcaagctgcttagcaaccggtgcgaactggcggttaatcgcgtcgacctgtgcgttgatctggcgcatccactccggctgctcgaagccgtggccgataccgaagtcagggatgttgcggcggacctgctcattgatctgcgcgctcacctgctggatttgcggaccgaaggcctcgttcactccgtagcccacagcgccgagcagcgcgataggcagcagccacaggaacgggctgttcgctgcaaacgcgttctcgaggcatcgcttcgccttgtcagacgagccctgcttgttcggggtcggtactacgtccttgtccatgaccttcaccttggcgtggactgtggacttaacaccgtttacatcggtcacctcgaccggtagctcgacttcggtacccggcttcgcatccgccggagtgatcacgcggacttcgccggtctccggatcaacagtgccctcccagcccttcggccagtcgagcttgcggtactggttgcccttcacagcgttcgccggctgaatgttggcggtctgtcctggctgcagcgtcacaaggctgtactcaggctttgcgacggtcgccttcgtgcccacctcgagaatgtaatccaccggctcgcgaacgatctgctcttcgccgttgacaacttgcttcagacccggcaccccctcctgggcgatacgggactggtcgcgggtgagctccgggttctcgcgaacgacaacctcaaacggaatctcctcggtccactcaacgtcaccggcaggcttggtgcccacccggacaacgcgctggacgggctccttcacggtctccaccgttgcacggccgttgacgacggtgactttgacctggccgttttcaccggccacgtcctcgatctcctggcccggctcaagcgtcgggtcgtaaacgatcttggtggtgaacggaagatccacggtctcagagacctcaggggccggatccggggtgctcggcttcttggtgccgatgcggatgaccgcgttcaccggagccttggtcacttgggtggtggtgaccggctcgccggacggggagccgtcgacaagcttgtgcgtcgtggtaactacctcttcaccgagctcgccctgggtaatgacctgcttgccctcctcgagggtgtcgtcgtagatcacactggtcttgaactcaatcgggcgggtcagctgggtcgagatctcgtcatcgttggcgcgcgggccgtactcgacgatgcggttgaccggctcgactcgctggttcgtgttctcaaccgtggcagattcgccgttggtcttgaactcaacgtagtaggtcgcctcgccgtccttgccttcctggacgaccttggtctctcccggagcgaggtccgggttctcgcggaactcagtcgtgaacggaatcggctccgtccaggtgacattctcaccagcctcaggctgcttggtgccgaccttgatgatgcgcggctgcggcgcggtggtgatggtttcatcccgcttggtgtcagtcacctggctattaacgatggtttgggtcaccgtgacgatcttctcgcccggcacgccctcggctgcaaccttgtattcaccagcagggattgccgggtcgtactcgatgacagtctcaaacggcaccgaaaccttctcttccaccacgcgggtatcgcccgtcttcgtgccgacgcggatgacagcgttaaccggctccttggcgcgctcagtgttgacgaccgggtcgccggaaggcttgccgtcaacaagcttctgcgtcgacgtcacaacgtcggtgccgtactcaccctgcgtatcgacgacctgctcacctgcagcgagagtgtcatcgaagacaatctcggtgtcgaacggaaccggcttctcagtcgtggtcaccagctcttgggcctccaagcgcgggccatactcgacgattttctcgacaggctcagtgcgccgcttggtctcctccaccgccgcttcaccgttcgtgccggtgaacgtggcggtgtaggtggcctcgccatcgacgccttcctgcacaaccttgatctcacccggggcgagatcaccgttcgcacggaggaccgtcgggtacgggatcggctcagtccaagtcacgtcctcagaagcggtcgcctgcttggtgcccaccttgatcacgcgcggcttcgcttcatcgatggtctcttcagtgaccgtcggctcaccgtcagcgacaccgttggtcgacggctgggtgacagtgaccttcttcttgcccggggtcccctcctcggcaacctcggaggtaccggccggaaggttcggatcgtactcaatcttcaccggcggctcgatcggtgcctcgaaagagctcaccacgtcgccagatttcttcgtgccgacgcggatgacggcgttcgtcggctccttggtgcgttcggtggtaacggtcgggtcgccggacggcttgccgtccacaatctgctgcgtcgacgtcacaacgtcggtgccgagctcgccctgctggtcaacgacctgatcaccctctgcgagggtgtcatcgaagacaatctcggtctcgaacggaaccggcttttctaccttggtcaccacggaggtgtcctcgggcgccggaccgtactcgatgatctccttgaccggggccttggtctgcttctcctcaggggccaccgttgcctgatcgcccgtagcggagaagtccgccgtgtaggtcttctcacccggcacgcccttctgaacgaccctgatttcacccggcttcagctccgggttcggacgggtctcaacctcaaacggaaccggcgcagtccaggaaaccttctcagaagcctcggacggcttcgtaccgaccttcatcacctgatccaccggatccttcgtgatctcctcagtgatctgcggatcacccggcttggagttgacgatgtcgcgcttaatcgtcaccgtcttctcacccggaacaccctcggtcacaatctcagacgcgccagccggcatgtccggatcgagcacgaccttcacaccgaacggaacctcagacgtcacagtctcggaggtctcaccagtggtcttcgtgcccacgcggatgacagcgttaaccggctccttggcgcgttcggtggtgacggtcgggtcaccggagggcttgccgtcgacaagcttctgcgtcgacgtcacaacatcggtgccgagctcgccctgctgatcgacgacctgctcgccctctgcgagagtgtcgtcaaagatgatctccgtctcgaacggcaccggcttctccaccttggtcaccacagaggtgtctttaggcgccgggccgtactcgatgatctcgttgaccggatccttggtctgcttctcctcaggggtcaccgttgcctcggtgcccttggcagcgaagtccgcggtgtaggtcttctcacccggtacaccctgctgggcaaccttgatctcgcccggcttcagctccgggttcggacgggtctcaacctcaaacggaacctgcgcagtccaggtgaccttcttggaggcatcggacggcttggtgccgacggtgataacctcatccaccggctgcttcgtgatctcctcggtgatctgcggatcgcccggcttggagttgacgatgtcgcgcttgatcgtcaccgtcttctcacccggaacacccggcgtggtcaccttggactcgccggcaggcatgttcgggtcgtacttgacaacgacgttgtacggcgcctcagccttgtaagtctcggtgttctcaccagtggtcttggtgccgacgcggatgaccgcatcctgcggttcagtggtgcgctcggtggaaatggccggctcgccgaccggcttaccgtccttgatctcctgcgtcgaggtgatcgtatccacaccattgacgccctgcttctcgacgacctgctcacccgctggcagcgtgtcgtctgcgacaaacctggtgttgaacggcaccgggttcgtcgtggtggaggtcagcgtctggtcagcgatggtcgggccgtactcaatgagcgcgtccaccggatccttggtctgctcttccttcggggtcaccgttgcgtcgctgcccttggaagagaagtcagcggtgaacgtcttctcacccaggacgccctcggtaacaaccttgacctcacccggcttcagcgcagggttcgggcgtacctcggtgtcgaacgggaccggcgccgtccaggtcacctgctcagtagcctcatccggcttggtgccgaccgcgatgatctgctcggtcggaggagtcaggacctcttctgtggaggtcgcctcgcccttcggctggctgttctcaaccggctgcgtgaccgtgaccttcatcgtgcccggcacaccctcctgagtcaccttggactcgcccggcgccagggtcgggtcgtagacaatgcgggtcgggaacggaatctcggcctcaaccgagttcacggtctcaccggtagtcttcgtgcccacacgaatcttcgcgttaaccggctccttggtgcgctccgtggtcacggtcgggtcgccggaaggcttgccgtcaacaagcttctgcgtcgacgtcacaacgtcggtgccgtactcaccctgcgtatcgacgacctgatcaccagcagcgagagtgtcatcgaagacaatctcggtgtcgaacggaaccggcttctcggtctctgtcaccagctcttgggcctccaagcgcgggccatactcgacgattttctcgacaggctcagtgcgccgcttggtctcctccaccgccgcttcaccgttcgtgccggtgaacgaggcggtgtaggtggcctcgccatcgacgccttcctgcacaaccttgatctcacccggggcgagatcaccgttcacacggaggaccgtcgggtacgggatcggctcagtccaagtcacgtcctcagaagcggtcgcctgcttagtgcccaccttgatcacctgagtgaccggctcggtagtgaccttctcctcgccgcgctcggtctcagtgaccttgctgttgacgatcgtctgggtaatcgtggtggtcttctcgccgaccttgccttcggttacgacctggtactcgccggccgggatttccgggtcgtactcaatcttcgtgtcgaacgggatcggctgcttttccgtcagctcgtgggtgccgttagtcatggtgccgacgcggatcacggcgttggtgggagccttcgtctgctcagtgcttatcgacggctcaccgaccggctggccatctttaatctcctgcgtggaggtgatggtctccacgccgttctcaccctgctggtcgaccttctgctcaccagcggcaagcgtgtcgtcgaggatgaactcggtctcgaactcgataggacgcgtcgtctcagacgtcagcgtctgatcatcgatcgtcggaccgtactcaatgatctggtccttcggagccctggtcacctcttccgtcggcgtcacggtggagtcagcacccacagaagagaagtcagcagtgaacgtcttctcgccgtactcgccctcctggacggtcttgacatcgcccggcttcagattcgggttcgcgcgcacaaccgtcttgaacggaacatccaccgtccacgtagccgtgttggttgcctcgtccggcttcgtaccgacagtcacaatctgctcagtcggctccgtcaccgtctcctcggccacagtcgcttctccgttcggcgcggagttgaccaccggctgggtgattgtgaccttcttcgtgcccggcttaccctcctgggtcaccttggagtcgcccggagccaggttcgggtcgtagaccacacgaaccgggaacggaatcggagcttcgtaggtgttgacggtctggccctcggtcttcgtgcccagacggacaaccgcgtcgaccggctccttcgtgcgctgcgtggtgatcgtcggctcacccaccggcttgccgtccttgatctcctgcgtcgcagtcacggtatcaacaccattgacgccctgcttatcgacgacctgctcacccgccggcaagttcggatccgccacaaacgttgtgttgaaaggcaccgggttcgtcgtcgtcgacgtcagcgtctgatccgcaatcgtcggaccatactcaacaatcttgtcggtcggctcagtgcgatccttcgactcggtcaccgtggcctggccattggtgccctcaaacgtcgcggtgtacttcgcttcgccgttgacaccctcctggacggtcttgacctcacccggcttcaaatccgggttcggccgcacgaccgtcgagaacggaatcggctcagtccactccaccttgtcggtagcggtggcctgcttcgtgccgacggtgatcacctcagtgaccggctgcgtggtgacattctcctcacgcttagtctcagtgacctggctgttgacgatggtctgcgtaaccttgacggtcttctcgccagccttacccggcgtcacgaccttatacgtgccagccggcacgttcgggtcgtactcgaccttcgtctcgtacggcaccggctcggtgtgctcaaccgtgttggcaccctcagtcttcgtgccgacacgcacgacagcgtcgaccggctccttcgtgcgctgcgtggtgatcgtcggctcaccaaccggcttgccgtccttgatctcctgcgtcgaggtgatcgtgtccacaccgttctcgccctgtttgtcgacgacctgctcacccgccggcaagttcggatccgccacgaacgtggtgttgaacggcaccgggttcgtcgtcgtcgacgtcagcgtctgatccgcaatcgtcggaccgtactcgatgatccgatcggtcggctcagtgcgatccttcgactcggtcaccgtggcctggccattggtgccctcaaacgtcgcggtgtacttcgcttcgccgttgacaccctcctgcacggtcttgacctcgcccggcttcaaatccgggttcggccgcacgaccgtcgagaacggaatcggctcagtccactccaccttgtcggtagcggtggcctgcttcgtgccgacggtgatcacctcagtgaccggctgcgtggtgacattctcctcacgcttagtctcagtgacctggctgttgacgatggtctgcgacaccgtaacggtcttctcgccagccttacccggcgtcacgacctcatacgtgccagccggcacgttcgggtcgtactcaaccttcgtctcaaacggcaccggctcggtgtgctcaaccgtgttcgcacccttagtcttcgtgcccacacggatgatctgcttaaccggctcttccgtgcgtgtggtctcgacaacagggtcgccggacggcttgccgtcgacaagcttctgcgtcgaggtcacagtgtcctcgccaagcttgcccgcctgcttcacctcctgcttgccggaatccagggagtcatcgaagacgatctccgtctcgaacggcaccggcttcgtcaccgtggtgaccaagttctggtcatctaggcgcgggccgtactcgatgatctccttgaccggagccttggtctgctcctccttgggtgtcaccgttgcgtcggaacccttcgcggcgaagtccgccgtgtaggtcttctcacccggcacgcccttctgaacgaccctgatttcgcccggcttcagctcggagttggggcgggtctcaacctcgaacggaaccggggcggtccaggtcaccttcgccgaggcctcggacggcttggtgccgaccttgattacctggtccaccggctgctcggtgattttctcctcaacagtggccttgccatccggctgggagttggtgaccttctgggtcacggtgatcgtcttcttgcccggcttaccttcggtaaccgtttcggaggtgccagcaggcatgttcgggtcgaattcgaccttcacgccaaatggaaccgtagtttcgaccgtcttggtggtttcaccctcggtcttcgtgcccacgcggatgacggcatcctgcttgggcttcgtggtctcggtagtcaccaccgggtcgccggagggcctgccgtcgacaagcttctgcgtagaggtcacggtttcttcaccgacaacgccctgcctatcgacgacctgcgtacctgcctcgagagtgttgtcgtagacgatggtggtctcgaacgggatcttgcgggtcgtctcggtgaccagctcctggttgtcgagtcgcggcccgtactcgatgatctcctcgaccggctgcttggtgtcctcggactcgacgaccgaagcctggtcaccagtagcggtgaacttcgcggtgtaagtgcgctcaccgtttacaccctgctgaacgaccttcgtctcacccggagcaagggccggattcgggcgggtggtggtgctgtacggaatcggtgcagtccacgtcacgtccttggacgcagtggccggcttagtgccgacgtgtacgacctcgttggtcggggcggccgtctgctcccacgtgccgtcgcgcttctgcttctcttcacctgccacacccttggtgacagtcttgtactcgccggcaggaatcgtgtcgtcgtagacatattcaactccgaacggcaccgggcgcgtcggaacgtcgacaacgttcacgacggccttaactgtgtccttcgagccatcttcgtaggtcaccgtgacgggaatctcgaccgtgctgcccggctcagcatccaccggtgcggtcgcagtgatcttgccatcgttgtcaacgttgactgtccaaccctggggaacatcgcccaactcgtaggggttgttcgttgcgacgttgacgtcctccggcttatccagggtgactggcagcgttgccgtatcacccgggtacaccgtctcctctgggtagctcggttccgcctcccagctgttggtcagctgcaccacggtggtcacagggacctcggggcgctcgccgttaggcgtttccacggtgacagtgattgttttcttgtcgcccggcttagagcctgccggcggcgtggaagtaacgacaccggtattcggatcgatcgtgtacttccagccgtcttcggttgtcatctcggtgatcggcgagccgtcagggttcgtgccaaaggagaacgtcgatccctccggggcatcctcaacctggtgatctacagcttggttcgggccggtggactcaacggagtagaccggtgcgatatcgcccttgagcacgacgacggtgcccttgactttctgggggtcttcatcgtcgtagtgagcaagaaccgggatgtcgaggatgtagccttcaggcgcagtcttgggaatcgtcgtggtgatcgcacccgtgttctcgtcgatcttcaccgtccacgtaccgctgtcgtcagtgtgggtgtactccgtcgtgccgtcctcgaaggtgtagcgcttcggggcttcatcggtcgtgttgccgctcaggccaacctccgggaccgaaggctgcaaagtgaccttggcgttcggcttgttcgtcaccgtgtcgtaatcggggatcttgatatcgacgattgcctggaactggggctcgatctcgtcggtggtttcgtccgggtaggtggccttcaccgtcggggtgatgatggtgcccggcgcgacagtgtcatccgctttcgcggtgaccttgccggtcgcatcgaccgtcacggtccaaccttcaggcacggtggactcgtcgacctcgaacttagccgggtgaaccggcttgtggcccttcataatggacttggtgcggatctgcgcggtgaggtcgtcgccaatgatgcccttggtcagactcgggcgaacaaggtcagtgacctgggtgttgtttgggtcaacaaccacgagcagctcgagctcatcggtcgagccgttcgagtactcgacggtgaccaccggacgggcgaaggtgcccggcttcgggttctccggagcggtgacggtgacgttgtagtccccgtccatctcgacgttccagccctcgtagacgtacttctcgtcgagggaaaccttggcttcgaagccgccgtcgcccttatccttcatcaggtccttgatcaggtccgggacctgcttgaactcgaccttctgcggctcggttgcgagcgggcccgtcgcgctatcgacgccagagatgatcgaagcgtccgtcttgtcgtacttcgggtcgtggtactcggtgtcgtccagggagaacgccttggagtcgatgacgttcgccttgctatagcgcgtcagcgagttcgagctgtcgaaggccatttcttcgccgaattcgttgctgtgcttagcagcactttgaagttgttcaacggtacgcggcttcgccagaacggagaagttcacgttcttgtcggtcgccagatcggtcccccggtactcgggccaggtgaagaagatgtcgccggtcgtttcgtcgacgcgcaggagctgctcaccgccggaggcttcttggtctgtggtgccaatgaacttaccgttgccgtcgtacgcttccacgaccatgcgggacatcgagtcgtccgtaccgccgttctgcaaggcaggaacattgatcgtaccgaccttggtttcctcaccagggacgatcacatgcttctcggatacctcggttgtcccccacgacaccgtgatcgggttacattcgatgttctcgctcggccacgggtttacggtagcgccaaaagtagcgctggagccctcggtggctttcggggcattaggatcgtactgcttgtagttgctttgccaggcgtaacgcacagggtcatcggcagaggccgaagcgaactgcttgactttctcgtcggtaagctcagcgtagagattcaagtttcgcagatctcggccactagcagtaatgtcgataatttcgtcggccttgtgggtgaccttgctatcaacaaaggtctggccggcctccatggaagacacctggccggtattcaaaacgttcttaaggttccccgaattggaaaagtaccaatcggcgaatgtgcggtccttcgagttatcaaaggagacactcagaccccacagggttttatcggggctttgctcactcggctccagggtgttccagcggaaacctgcctggtttccgctcggctcaccgctttcaacaacacacgacccggccggcaggtcggacgcctgctgggcgtcctcctccaccgcgccggacttgtcgcggatgccgccggtgaagccctccgacgccgcggcagacgatgccagcgggcccgggccgacgacgctcaggccaccgagcgcgagtgcaatcgcagatgttgccgcaatgccgcgcgaggttgaattacggaaacgccgagatgatccggccatttatgctcctctttgaagtgaagtgtcaccacgtcccaacagagaggtgacagatagcatcacattctaaagatcggagaaactactgtctacctaagcatttgcttaacgacgcccccgtgccccagccaggcccaccaccgcaagcagggcggacagcagcaccgccgagacgataccgctgtagtcaccgccgttacccgcagcggacaccgctgtcgacgcccagtgcatcggcgctgcttgcgacaacgccacccacaccgagtcgacctgcgcggtggtcgcggtgcgccacacccagccgacgagtccggtctgcaccagcgcgagcacgccagctgagccaagaccaaccccagcgccgaatgctcgacttaacacggaagccaggccggcgctggcgagcgtgcccagcagcaggcctgcaaacgcaaccccgtattcctgagcgccaaacccggctccgatcaccccggccaagatggtgcccgcggcggcaatcactacggaaccggcgcccaggatccaccattgcccgcgggacgcgaaccacgccgccgccgagagcgcggtgccgccgagtacggccatcgccgcgagtagcatcgccgccaccggtggaagggccggaccggctggctcagcaccgtcagcccccggcgcaaccgccggcaccggaagcgccgcgcgaacggcgccaaccttatcggcgttcatgctcgccatttggttgatcctttccacgccggcgaccaactcttcaatcccgccagtggcctgcccggtctgtgcctgaagttcacgcaggcccgcagccagctctgccgagccacgagtggctgtataaataccgtcgtggaaaccgtatccgggtacggccagctggttggctaggtcgcgggagccgtcgcgaagctggttcatctttgccaccgcgtccggcggcagctgcgcggttagcgcctgctcgcgcaggtcttgcagcgactcgcgcgcctgcaccgcctccgggtctttcgcgtctttgagttcctccagggagcggtcgatcgcgccgaccacctggccgcgcaccgcctcaaaccctacgatctggcccacaatctccccgatggagtccgccagctgcgtcgcgcccgcgcccaactggccggtgccggcctggagctggaccatgccgtcggcaagttcttgggatccggactgggcggccgtgagggcgtcgataagctgctgagcttgcccctgcgcctcgccgatgcccgcggcgagctgacccgcgccctgcttgagcaccgtcgcctgcaggccggcttcaccggcggcacggcgcgcgtcgccaagattgtccgggccgacttgcggggcacccgaaacctcagaatcgcgtcccgcattcgcccacgtgtcggccggactcatgggtaaaaataccccaactaccagcgccaaaagcgcacacaccaaccgccacgcgttgcccgattgcatggcacttttcttagcacccgcacgggccttgtggcgggaggcgcaccgccggaaatgctcaccgttagaaccgtatcgtcacccttgatactgtcgtaagggttcttgccaaaaccatgcattgaaattgggttcaccatgacacttccccttgccatcgggctcgtagcggcaacggtggtgctctccccgttgctggtgcgcgttatggacaggaaggccgggtacccggtcgcggtgctgctgttcgctgcagcggccgtgctgggctccaagctcacctccgtgatggagggcgatgccctggaatggtccaggcagtgggcgaacgatgtgctgggctcgggcacctcggtggcgttcgcgctgcgcgctgacggcctcggcatcttcttcgcgctgctcgccctcgtcatcggcggggttgtcatgtgctactccgccgcgtacctaccggaaaaagagggcaacaccagcttctacaccatcatgacggcgttcaccctctcggtgttgctgctcgtgttggcgaacgacgtggtgctgctcttcatcgcatgggagctcgtctccatcgcgtcgtttatgctgatcgcccgctccggctcctccggcgaggcaggctcgtaccgcaccctgatcctcacgttcttcggcggtctcacgctgctcgccgcgctcgcgcttgcggcggtcaacgccggcacgacgtcgctcgagggcattttgcaaagcgacgtgtggcgtcacaaccccaccgtgaccaccaccgtggccgtgctcgtggccctgtccgccttcaccaaggccgcgcagttcccgttccacttctggctgccggaggcaatggccgccgccaccccggtatccgccttcctgcacgccgctgccgtggtcaaggcgggtgtctacgtgctgcttcgcttctcctccatcttcgccgacgtgaccgcgtggaacgttctgctcaccgccaccggcttgtttaccgcgctgatgagcgcggtgttcgcgatcacgaagacggacctgaagcatctcaccgcgtactcaaccgtgagccacctgggttggattgtcgccgcgatcggcatcggcaccccgctggcactcgccgcagcactcacccacacgctcgcccacgcgctgtttaagtcctcactgtttatgctgatcggtgttgtcgaccacgaggccggctcgcgcgacatgcgccgtctgggcaagctgtatgacaagatgccgtttacgttcgtctccacggtggtggctgcggcgtcgatggccgctatcccgccgctgttcggcttcatctccaaagagtcgatcctgagcgccttcgaggactcggcgtacggcacgctgttgctcatcgtgggcggcatcgccgcgttcctcaccttcgtctactccgcgaagatcgtcttcggcgcgtttgtagacggcccgaaggacatgaccggcgtccacgaagcaccggttgcgctctggttgccggcagctctcccgggcctgatgtcggcggtggtgccctttgggctcatgcttatcgacgcccccctctcctccgcagtccgctccatcacgggggaggactaccactctcacctggcgctcttccacggtgtgaacgcccccttcatcgtctccatggcggtgcttgttgccggcgttttgttcgtcatcttcgcgcgccacaccgtcttcgagcgcgcggagaacaaggagttgctgccgttcaacggcaacgaggtgctaggcggcatcggtcgcggctcgacccgcttcggccgccagctcggcgccgtcgccgacggcttcaacccgtcgcgccacctgttcccggtgctgctgctcgtggtgttgctcggcttctccacgctgctgtttaccgacggcgtcgacggcgtcccgctcgcgcctcgcgccgatggcatcgatgtgtggtgggacctgatcccgttcgccatcatcgcggtgtccgtggtgggcctcatcaccacccgctcgcgccttgcgtccacggtacttgttggcacgacaggcgtgggcatgagcttgcagatgttgatgctgggcgcgcccgacgtcgcgctcacccagatcctggtggagtcgctcaccgtcgtcgtgatgatggtggtgctgcgctaccagccgcgcatcttcccggagaccccgcgccggcgcaaggtgcttgctggaatcttcgccgtgttgaccggcttcgtggccttcctcggcgtctacaccctgctgggccgccacgagcgctctgacctggcgatgtggtacctcaccgagggcggcaaggtgaccggcgccgacaacatcgtcgcggtgatcatcgtcgagttccgtggcttcgatacgcttggtgagctttcggtgctcggcatggccgccgtagtcatcgccgcggtgacccagtcgatgccgcgccacatgttcgaggccggcacccgcccgcgcccgttcggccagtcccagttcaactcgctgccgctgcgcaaggccgcggccatggtcgcgcccgtattgctggtgttgtcgatcatcatcttcttccgcggccacaacgctccgggcggcggcttcgtcgcagcgctggtgatggccaccgcgttcgcgctgaactacctctcgcgcggcgcggacgcctacgtggtgggccagctcaccccgatcaagctcgccgcatggggcatcatcatcgcgatctcctccggcttcctggggctgatcgagggcggattcatgtacgccatccacggcgagatcgccggccagcacctgaccacgtcgctcatcttcgacttcggtatttacctcgcggtgctcggcatggtcacgcaggcgatcaacgcgctcggcgggtacctgcgcccgggcaccgagatccgcaacctggactacacgcgcgacgagccggacaacccgctgccaaacgtgccggaaccggagcacccggagaacgccgtgaagtcccacccggagccgatcaacccggccgacgacccgcaacccgtatccacgaaggagcagtaagagacatggttatggcacttactatcgcggtgctggtcgccggggccgtctacctcgtgctgcagcgcggcatggttcgcattatcttcggcatgtcgctcatgggccacgccgcgaacctcaccctgctggccgcaggcgtcggcgcgtggcgcggcgaggcgttcccctctcgcacccccatggaggatctctccgaccctctgccccaagcgttcgtgctgaccgcgatcgtgatcgcgatggcgaccaccacgatcctgcttatgctcgcatctttgggcagggacgacgacacgttcgacaaccccaccggcaccgacgccgcctacgacaagatgcggctgagcccaagcgcgctcagcaccgcaggccgccgagcccgcctgaacccgcgcaagcttgaggagattcgcaatatggaggtgaaccgatgacagcagacgccctgttgccagtgttcgtggcgctgccgttgatcgtgtccgcgatcaccgcactgagctcgtccaagcagcttaacgacgccctgtccatcatcatccccgccatcaacctcgccggcggcatctggctctacacctacaccgccgagcacggcacgatctcgcacgtgatcggcctctaccaaggcggcgtgggcatctcgtacgcgggcgaccagttctccgcggtcatgctggtgaccaccatgatcgtggcgctggccgcgaactggttcgccatcgccatcggcgagacgcaatcgcgctactacacgccgctgaccctcgttctgatcaccggtgtcaccggcgtcctgctcacggccgacctgttcaacttcttcgtcatgatcgaggtcatgctgctgccgtcgtacggcctgatcgccatgaccggtacccgccaccgactgctgtctgcccgcacgttcgcgctggtgaacctgtcagcctccacgctgctcgtggtgggcgtcggctacctctacggcgtgaccggcgcggtgaacatcgccgcgctccagggcgcggccgccggcaacggcccagtcaccgtcgcgaccgggctggtgatgatcgccgtggccgccaaggccggcgtcttcccggtccacacctggctgccgcgcacctacccgtccacctccgccgcggtgatgggcctgttctccggcctgcacaccaaggtggcggtttacatgatcttccgtctctgggtcatgctcttcgacatggacccgcgctggaacacgctgatcatcgtcatcatggtgatctccatgatcatcggcggtttcgcgggtctcgccgaggacaccatgcgccgtgtgatcgcctaccagatggtcaacggcatgccgttcatcttggtcacgctggcgctgacgaccggcggcaaccttgattccggcgcggcgcgctatgcgctggccgccggcttgctttacaccctgcaccacatgatcaccgtcgccgcgctcgtgctcaacaccggtgcgatcgaggagacctacggcaccggcacgatgtcgaagctctccggtatcgcgcgccgtgacccgtggacctcggcagtgttcgtcgccggcgcgttctccatcgtcggcttcccgccgttctccggcatcttcggcaaggtcacaatcatgatggccgccgccagggctggcgactggcgctcctgggtggtcatcaccgccatcatcatcgcgtccttcggtgcgctgctgtccatgatgcgcctgtggaagaaggtcttctggggccggccaatgcagcattacccggaagcgttgaatgtgcggtggaggtttttggtgccgtcgttaagcctgatgctcctgtcggtcctcatgttcgtcttcgccggccaaatgtggggcatctccaccgcggcggttgacagcctgcttgacgtcgacgcgtacaccaccgccgtactcggcaccgatgccgtgggcgtgcccgacgtttcagcaatccagggaggcaagtaaatgtcacgcatcggccactggatcggctacacgttctggatcatcaaggagatcctggtcgccggcttcaccgccaccgccgccgggttcaaacgcgaccccggcatcgagccgatcgtgatcttctacccgctgcgcgtcaccagcgactgggacatcttctggttcaccacctccatcaccgtcaccccgggcaccttgtccatgggcctgcgccaccgcaccgccccagacgaggcggagaccctcattgtccaagcagcgttcggctcggacccggtcgaggtcatcgagggcctgatcgacatggaggagcacgttaacccgcaggtgaaagcaatgcttatcgacgccacctccgtcccctgggagccctacatcgaccacggcgacaccacgccaaccaccgacctcccgcccgccgaaaggatggagtgagatgtttgaaccaatcgtcctgacctgcatggtcatcatcgccgtgtgcctgttggtggtgctgggcaagctcatcttgagctccgacgagctcacccgcgccgtgctgtcagacttcgtgttctatgccatggtcgccatcttcttggtgtggaccctgtttacggagaccatgatcggctacgacatcgccgtgctcgcggcaattgtgtgcggcgtggtgcccaccatctccatggcccgcatcatctcgagaggacgccgctaatgactatcgccgaaatcgtcgtcgccacgctggtgatcgtggccaccgtgttcgtggtgggctgcacgctgctgcagctgcgcgcccccgacgcgctcacgcgcgcgaacctcttgggcccgctggtgtgcctggcgtttcccatcctgctggtggccaagctagtgcgcacgttctccaccacaggcttcgatctcggtgacctcatcatggcgctgctcgccatcgccggcgtgtggatcgtcggctcggtgggcacgtttgtcatgggacgcgtgctctacggtgtgacggtgtcggacaagcgctcctcgtaggcgcctcgtgagcaggcctgatgacgactacgtcaccgacctcgccttaaaagcggggcggggcgaccgcgccgcccttaacgacttcatcgcgctcacccaagacgacgtgtggcgcttgctcgcgcacctcgcggggcgcgagtacgccgacgacctgacacaggagacgtacctgcgggttttgaagtcgctgccgcggttcgccggccgctcatcggctcgcacgtggcttttgtcgctcgcgcggcgcacgtgggtggattcggtgcgccacgacatggcgcggccccgcaaatccgccgccgagtacgaagacgttgccgccgaacagccgagccacgacaacgcgtcgacctggtccgaggtgatggacgcgcgtgcgctccttgacagcctggcgcccgagcgccgcgaagccttggtactgacccaggtgctcggctacacctacgaggaggcagcgaaaatcgcaggcgtgcgagtcggcaccatccgctcgcgcgtgtctcgggcgcgcgcggacctgatcgcgggtggataagatagaagagctcatttactcgtttacacccctttggagcgagctcacatgctcaaaaccgcgttatttatctcgttcgcgttcatcggcaccgtcgtcggcgccggcttcgcctccggccaagaggcgcttctgtacttctccgccttcggcaccgacggcatctggggagcggtgctctcgtccgcgctgatgctgatctccggcgtgaccatcctccagctcggctctttcttccaggcgaaggagcacatggaggtgcttggcaacatctcctccaaggtcatgtcctggatcctcgatatcgccacgattgtcacgctgttctcgatcggcttcgtcatgttcgccggtgccggcgcgaacctgaaccagcagttcggtttgccgccgtggatcggcgcggtgctgatgctcgcgctgaccatcggcttcggcttgctggacgtagacaaggtcaccggcgccatcggctcgctgaccccgttcctgctggtgctggtcatcatcggctgctcgtggacgcttattaacgcccacccggactggtccaccatcgacgctcaggcggccctggtcgagaccaccctgcccaactggtggatcgctgcgctgaactacaccggcctgaacgtgatgtgcgtcgtctcgatggcgctggtcatcggtggcaaccagttggacacccgcgccgccggcctcggcggcctgctcggcggcatgggctacttggtcatgctgatgctgctggcgatcgcccttttggtgaaggtcgacaccgtcgcgggcagcgacatgccgctgctgacgctgatcaccgacctgaacccgacactcggcctcgtgatgtcgatcgtcatcttcggcatgattttcgccacctcgctcggcatgttctacgcgctgggcaagcgcctttcccgcggccgcgaagacaagttccgcattatcttcatctccacctgtctgatcggtttcgtgctgtccttcgtgggcttccagaagctggtctccgtggtctacccgatcctgggctacctcggcatcctcctgatcgccgtgatggtcgccgcctggctgcgcggcgcgccgaagctgaagaaggaaggtgaccgccgccgccgcgcgatggagctcacccgcctgaagctggacccgcgcgagcgcttcaccaagaacgaccagcgcgagctggagcacgtcacgtcgatgtccgtcatcgacgacgaggagctggcagaggccctcgaagaggaggtcgccacagagcttgcggaggacgaggaagtcgacttcgatatcgaggaccgcgagctcgacccggtcgtgtacgtctcctacaccgagccggtgagccaggcggagtacgagcgccaccccgatgagccgtggaacgacaccacggttgacgagatcatcgccgaggatcaggaagagatcgccgagcgcgaagccgaggaagctgaggccgccgcggaaggcgacgcggagaacgagggcgcggcaggttccacccggttgtaggcgccccccgccacgaaaacccggccacatcggccgggttttcttttggcttgctgctgcctcttagaccagcagctcggcgatctgcaccgtgttcagcgcggcgcccttacgcaggttgtcaccggagacgacgaagatgagaccgcgaccgccgtcgaccgcctggtcttggcggatgcgcccaaccagcgactcgtcgccgccggtggcctcgagcggggtcggcacgtcgacgaccttcacgcccgccgcgccctcaagcaccttggcagcctcttccggcgtgattgggttgtcgaactccgcgtgcaccaccatcgtatggccggtgaacaccggcacgcgcacacaggtgccggacaccttcagatccggcaggcccaggatcttgcgcgactcgttgcggagcttctgctcctcgtcggtctcgttggtgccgtcgtcgacaaggttgcctgccagcggcagcgcgttgaacgcgatcggggcgacataggggcgaaggtctgccggctgcagcagcgagccgtcgcgcgccaaatcgttgagctgcgggccgatctcgcccacctgcgtagcgagcgcgttcacgccggccaggccggaaccagacacggcctggtaggaggcgacgcgcagggtgttgagcccggcaacgtcgtgcagcgccttgaccaccggcatgatcgccatggtggtgcagttcgggttcgcgataatgcccttcttcagctcgcgcgcctcatccgggttcacctcggaaacgatcagcggcacgtcgttgtccttgcgccacgccgaggagttgtccacgaccttcacacccgccgcggcgaacaccggcgcccactcgcgcgaggtcgacccgccggcagaaaacagcgcgatgtcgatgtcgcgcacagagtcctcggtaaccttggcaaggtcctcgatctcaacggtctggccgcggaaggccaccttctcgcccgcggagcgcgccgaggcgaagaagcggacgttgtcgcaggggaaatcgcgctcgtccaagatgtcgcgcatcacgcggccgacctggccggtggcgccaacgattgcaacggttgtcatgatggaaaactccttctagcggccggtgccggcgtagacgatagccggctcgtcgccgcccagctcgaacttggtgtgcagggcgcgcgccgcttccgcgaggtcgtccttgcgcaccacggcggtgatgcggatctcggaggtggtgatcatgtcgatgttgatgtcggcgtcgcgcagcgcctcggtgaagtcggcggtgacccccgggtgcgacttcatgcccgcgcccacgagcgagaccttgcccacctggtcgttgtaggtgatgtcgtcccagccctcggtgtccttcatctcgttcaggaacgccatggtgcgctcgccgtcagccaccggcagcgtgaaggtgatgtcggtcttgttgtcctcgatcgaggagatgttctgcagcaccatgtcgatgttgacctcggcctgcgccagcgcgcggaacaccttcgccgcctcccccggcttgtcctggatacccaggatcgtgatcttcgcctccgagtcgtcggttgcgacaccggtcaacactgcttcttccacgggaatatcctccaatgctccggcgacgagggtgccggggtcgttgctgtaagacgagcgcacccgcatgggcacgttccaggcgcgggcgtactcgacgctgcgcagcaccagaatcttcgagccggacgcggccagttccagcatctcctcgaagcagagctggtccagcttgcgcgcgtcgggcacgatgcgcgggtcggcggtgtacacgccgtccacgtccgagtagatctcgcacacgtcggctttcagcgccgccgcgagtgccaccgcggtggtgtcggatccgccgcggccgagcgtggtcacgtccttggtgtcgcggttgacgccttggaagccggcgacgatggcgatcttgccctggtcgatggcgtcttgcacgcgccccggcgtgacctcaataatgcgcgcgttgccgtggcgctcggtggtgatcacgccggcctgcgagccggtgaacgactgcacgtcggcgccgagcgacgccaccgccatcgcgaccagcgagttggagatgcgctcgccggcggtgagcagcatgtccatctcgcgcgcgggcggggcggggttgacctgcgccgcgaggtctagcagttcgtcggtggtgtcgcccatcgcggagcacacgaccaccacgtcgttgccggcgcgctttgtggccacgacccgttctgcgactgcgcggatccgttccgcgctctcgagcgaggaaccgccgtacttctgcacgaccaaggccatggtctgcaccctttccgtatcttgctgtcagtgccaaccagaataaccgctcgggcgacacgcgttgcagctgcccgttattatcattcgctgtgcagagcaacatcacggcggcaaccttcgcgatcatttccgccgtgttgatcgcggtcggcaccgtgtggcgccaccgtattttgcgtgctggccaggcccgctcggaggccaacgacgcgccgcttgcttccctttccaacattcgctggtggctttcgatcgctatcgcgctgctcgcctacgccttccaagccgcggcgctcgcctacggctccctgctcatcgtccagccgattctggtgctgtcgctcatgctcacgctgatcctctccgccgttgccgaaagacgccggatgtcgcgtcacgagtgcatctgggcggcgctgctcacagcctcggttgcggtggtggtgctgatcgggcgcccgcagcccggcacgcgcgaggtacccgggtgggagtgggttgcggtgatcgcgcttggtctggctctcacggcgggagcttttgcatttgcttatcgacgctccccgcaaacccaagccctcaccttcggcgccacctgcggcgcgatctacggctacctcgcagtttttgccaaggtggcggtcgacgtgctcgcccgcgagggcgtgtgggcgatgctgcggagctggcagctgtgggccgtggtcgcgaccgcggttgtgggtctggtggtgcagcagtacgcattcggcgcgggggatctggccgcgtcgttgcccgccagcaaggtcgccgaaccgatcgtggcccttgcgctcggctacgtcttgttggatgaggagtttgctgtgggggcgtggggaatggggttgatg

SEQ ID NO: 18 - DNA, 33657 bp, Corynebacterium cassirii
  source 1..33657: mol_type = genomic DNA
cgcgggggccgggggagggcccaaacgccgcagggcgacaaaggtgcaggctgtgacgagcgcggttgagcgcgacggcaatttgcacgagctgcttggtgaggcgccgctggtgttgccgaccgtgattgggcacaacgtccgttagacgtatcgccggagtaatacaataggcccatgctgcgcgtgactgatctgcgggaaacgacccccaccacctcacagctgcgccggttgctgccccgcggcggtaccgacgtggcgtctgttttgcccactgtcgctccgattgtggaggcggtgcgcgaccgcggcgccgaaaaggccttggagtacggcgaacagtttgaccgcatccgcccggaatcggtcgtcgtgcccgaagcggtgattgacgccgccgaggcaggtcttgagcccgaggtcaaagaggcgctggaggtggcgattgcgcggatccgcaaagtccacgcagagcagaaacccaaggagcacacgaccacgcttgcggatggggcgacggtgaccgagacatacatccccgtcgagcgcgtcggtctgtacgtgccgggtggaaaggcggtgtacccctccagcgtgctgatgaacgtcatccccgcgcaggaggcaggggcatcaaccatggtggtgtgcaccccgccgcaggttgagttcggcgggtggccgcacccggtgacgctggctgcgtgccggctgctcggcatcaccgaggtgtgggcggtgggcggcgcgcaggcgatcgcgctgatggcatatggcgacgacgaagctggcctcgagccggtggacatggtcaccggccccggcaacatcttcgtggcggcagcgaaacgcctggtgaacggcgtcgtcggcatcgacgctgaggctggtccgagcgagatcgcggtcatcgccgacgaaacggcggacgccgagtatgtcgcgctcgacctcatctcgcaggcggagcacgacgagcaggccgccagcgtgctgattacggattcgcaatcgctggctgaagaggtgcagcgggtcgtcgacaagcgaagtgccctcacgctcaacgcggagcgcgccgcgtccgcgctcggcggcgcgcagtccggcatcgtgctggtgcgcgacgaggaacaggcggtggcggtcgcgaacgcgtatgcggcggagcacttggaaatccacacccgcaacccgcgcgagacggcaaagcgcatcaccaacgccggtgcgatcttcgtcggaccgtattcgccagtgccgctgggggattacgccgccgggtccaaccacgtcctgccaacctccggcaccgcgcgattcaacccgggactgagcacgcacacgttcttaaaacccgtgagcctgatcgagtacgaccagcaagcactgacagagatcggcaaccacatcatcgcgctcgcggacaaggagcagctgccggcccacggagagtcgatcgcggctcggatgggggacaaataaatggctgcctctactacctcggacatcactctggacaacctgccgctgcgcgaggagctgcgcgggaaatcggcctacggtgcgccgcagctcgatgtcgcggtggcgctgaacacgaacgagaacccgtacccgccgtcgcaggcgcttatcgacgatctcgttgcggaagtcgcacgagtagcggcgtcgctgaaccgctacccggagcgcgacgcggtcgagctgcgcgacgcgctcgcggcgtacgtgactaagcagaccggcgttgcggtgacgcgcggcaacgtgtgggccgccaacggctccaacgaggtgctccagcagctgctgcaggcgttcggcgggcccggtcgcacggcgctgggtttcgtgccctcgtactcgatgcaccccatcctgagcgcgggtacgcagaccgagttcatcggcgtaaaccgcggggaggactaccgcatcgacatggatgcggcgcttcgcgcaatcgccgagcacgccccagacgtggtctttatcaccaccccgaacaaccccaccggcgacgtcacgtcactgcccgacatcgagcggatcatccaggccgcgccgggcatcgtcatcgtcgacgaggcgtacgccgaattctccccgtcgccttccgcttgcgagctcattgagcgctacccggcgaaactcgtggtgtcgcggacaatgagcaaggccttcgacttcgccggcggccgcctgggctacttcgtcgcggccgaggcgttcatcgaagcggtgatgttagtgcgcctgccgtaccacctctccgtgctttctcaggcggcggcgcttgtggcgctgcgccatgcggacgagacgctgggcacggtggaaaagctctcgcgcgagcgcgaccgcgtgcagcgggaactcacgcagctgggctatgacgtggtgccgagcgaatcgaacttcatcttcttcgggcacttcgacgatgcgcaccaggcgtggcagcagtttttggaccggggcgtgctgatccgcgacgtcggcgtgcccggccggctgcgcgtcactatcgggctggacgaggaaaacgacgcctttttggcggcggcgaaggagatcatcaatggctgacacggctgacacaaccacttcggcgcgcatcgggcgcgcgacccggaccaccagcgagtccgacatcaccgtggaaatcaacctcgacggcaccggcaaggtggatgtggacaccggcctgccgtttttcgaccacatgctcaccgcgttcggcacccacggcgcgttcgacctcaccgtgaaagccaaaggcgacacccacatcgacgcgcaccacacggtcgaggacaccgcgattaccctgggctgggcgctcgcagaggcagtgggggacaaggccggcatcacccgcttcggctcgatgctgctccccatggacgaaaccctggtcgagtccgtggtggacatctccggccggccgtacttcgtcatgaacggcgagccggagcacatgcagtggcagatcatcggcggccactacgccaccgtgatcaaccagcacttcttcgaaacgctggcgtacaacgcgcgcatcaccctccacgtcaacgtccgctacgggcgcgacccgcaccacatcaccgaagccgagtacaaggccgtcgctcgcgcactgcgacaggcggtctcgcgcgacggcaagctgaaaggcgtcccctccacaaagggtgctttgtaagcagttcctgtgtcgaacccgtgtgattcgggtacggtgccagcgtggattcccccgcgccggtggagccgtgtctgaattgagaagggagtgcaggtttggccctgaacggagcgttcgcgcgcgcacgcagaccgttgaccccggaagaggtcgatagcttcacctcggtatggcgggcgaggggcatcgtgccggtgctcatcgccgtcgcctcggcgttcggcgcgtggtcgttccttctgcccgtggtgcctaccgcggtgatcgacgctggggggccggagacgctggcgggcctcagcaccggcattttcatgctcgccacagtgatcacccaggtcttcactccgtggctgctccgaactgttggctaccgcgcggtgatggtggcgtccgctttgctgctcggcggcggggcgttcggctacatgctcggaatggaaccaggcgcgctgctcaccgtcagcgcggtgcgcggcgtcggcttcggggcgctgtccgtggccgaggccgcgatcatcgcggaactggtgccgctccgcttgctcggcagcgcgacgggcgcgctgggcctggtcgtcggcgcctcgcagatggtggctttgccgctcggcctagcgctagtggacgtggtgggctacaacggcgtattcgctgccggcgcgaccgtggggttgatctcgctgctcgcgtcgctgctgatcccgtcgattccgcccgccgcggaggacgaggcggtgcccagcgcggtgcgcgtgcccacttggcacctggtgctggtgccggcgctcgcgcttatgttcgtcaccaccgcctacggcgccatcaccaactttttgcccgcctccatgcgcgacctcgatccggtgcgcggcgcagcgctcggcggtcttatgctcggcgtgctcaacctagccgcgatgctctcgcgctacttcgccggccgggtgatggaccgaaagggctacccgggaacggtgcttatcccgttccagatctccgcggctgtcggcgtgttcatgatggcggtcatcctcttcctccaactgcccgtgtggaccatggtcatcgcggtgatcttctacggcgccggattcggcgcggtgcagaacgaggcgctgaccaccatgttctaccgcctgccgcgctccaagtcttcgcaggcgtcggcgatctggaacatcgccttcgacggcggcacgggcatcggatccaccgtctacgggatggtgctgaccaccatggcgttcgcgccgatgtacggcattgccagcgcggtgatcgtgctggggctcgccgtgacgctgctggaccggcaactgggccgccaccgcgtggttgaggtgaacaatttggcggtgcgtctcaaagctgtccaagccccgcggcgctaccggtaggcgctacactttccgtccatgactcacaccgccaacaccacgccgactgtggcgctgctcgactacggcgccggcaacctgcgctctgcccaccgcgcgctggaacacgtgggtgcggacgtcgcggtgacgaaagacccgcacacagccgtcgaggcggacggacttgtggtcccaggcgtcggagccttcgcggcgtgcatgcgcggcctcaacgaggttgccgcgccgcgcatcgttggccagcggctcgccggcgggcggcctgtgctgggcatctgcgtgggcatgcaggtgatgttcgagcgcggcgtggagcacggggttgatgcggctgggctgggggagtggccggggagcgtcgataagcttgatgcccccgtgctgccccacatgggctggaacaccgtggaggtgcccgagggaagcgccatgttcgcggggctcgactctgacacccggttctactttgttcactcctacgcggcgcgcgagttcccgctggcggaagacgagtttattgcctacccgaaggtcgcgtgggccgcgcacgggccgagccggttcgtcgcggcggtggagaacggcccgctgtgggcgacccagttccaccctgaaaagtccggcgatgctgggctccagctgctggcgaactgggtgggcaccctgcgttaggattggccgcatgacgtttactctcttgcccgctgtcgatgtggtcaacggtcaggcggtgcgcctgcaccagggggaggccggcacggaaacggtctacggcactccgctcgaggcggcgctgaagtggcaggaggagggtgcgcagtggctgcacttcgtcgacttggacgcggcgttcggcaacggctccaaccacgagctgatggcgcaagtgacccgggaactttccatcaacgtggaactgaccggcggtatccgcgatgacgaatcgctcgagcgggcgctcgccaccggtgcgaagcgggtcaacatcggcacggccgcgctgaggaatccggagtggaccgaaagcgcgatcgcgcgctacggcgagcagattgcgatcgacatcgctgtgcgcgaggaggacggccagtggcgcaccaagggcgacggctgggtgagcgacggcggggacctgtgggaggtgctcgagcgcttcgacgcggccggatgtgcccgcttcgtggtcaccgacgtaagcaaggacggcacgctgaccggcccgaacatcgacctgttgcgtgatgtggccgcggcgacggacgccaaaattacagcatccgggggcatttccacgcttgacgacgtcgccttggtctcctcctacctcgacgaaggcatcgactccgtcatcatcggcaaggccctgtatgagaagcgcttcagcctcgctgacgcgctcgcgcgggtcgcgctgtgaccgaagcagcagatcgcgcggacctcgcggattgccaccgtctcgccgcggctgccgtcacggaggcgcgcggcgtgtttctcgaccacgtgggcgccgcgccggcgctgatgaagggcaagggcgacttcgccacagaagcggatctggccatcgaggcgcttttgcgcgagcggctcggcggggccaccggcattcctgtctacggggaagagggcggcggcgacttcaacgccgaagcctgctgggtggtcgacccgattgacggcacgtcgaactactcctcgggcaacccgaactgcgccattttggtctcgttgatccgcggtggccaaccggtgatggcgttcactgaaatgccgctgttgaacctgagtgtgagcgctgttgagggccagccggtggtgtgcaacggcaccgcgttaccgccgctgggaagcggcggcgcgggcacccacgcggccgcgcaggtcggggtcggttccgtcggctccgacgaccgggtgcgttttcccgcctcgacccgccttgcgctcattggcgagctcgcgaaaaccgagctgcgcccgcgcatttccggttccgtcggggtggacttggccttcgtcgccctcggcatctaccgggctgcggtgagcttttccccgcacgtctgggacaacgccgcaggcgtgctgatcgcgcgcagtgccggcgccgccgccaccgacatggacggccggccgtggtccccgggcagcgccggggcaatcgtggggacccccgcggcgcacgaaacggcgctgcgtacgatgttgcacgttgccaaccagtagcagcacgacacagtaaaggaagttagccatggcagttgcgatccgagtgatcccgtgcctcgacgtcgatagcgggcgggtggtcaagggcgtcaacttcgaaaacttggtggacgccggcgacccggtcgagttggcgaagcgctacggcgaggaaggcgcggatgagctgaccttcctcgacgtcaccgcctccaaggaaggccgcggcacgatgctggacgtggtgcgccgcaccgccgagcaggtgttcatcccgctgaccgtgggcggcggggtccgcagcgccgacgacgtgcgcgagctgttgcgcgccggcgctgacaaggtgagcgtcaataccgccgccatcgcccggccggagcttctccgcgagcttgccggcgagttcggctcccagtgcatcgtgctctccgtcgacgcgcgccgcgtgccggaaggcggtcaaacccagccatccggcttcgaggtgacgacccacggtggcacccgctccgccggcatcgacgctatcgagtgggcgaaaaccggcgccgaccttggcgtgggcgagatcctgctgaactccatggacggcgacggcaccaagtccggcttcgatgtggagctgattcagcgcgtgcgcgaggcggtctcgatcccggtgatcgcctccggtggggcgggcgcagccgagcactttccgccggccgtggaggcgggtgcggacgctgtgctcgccgcgtccatcttccacttcggtgaagtctcgatcagcgaagtcaaagacgagctgcgctgcgcagggctggaggtgcgctagatgtccgttgcaacgtacgaactggacccggccatcgccgcgcgcctgaaacgcaacgaccagggcctcgtgcccgccgtggtacaggaccacgagaccaaagacgtgctgatgatggcgtggatggacgaccacgcgctcgcccacacactcgccacccgccgcggcacctactactcccgctcccgaggcgagtactgggtgaagggggagacctccggcaacgtgcaggaggtgaagtcggtggcgctggattgcgacggcgacacgatccttgtcaccgttgcgcaaaccggcggcgcgtgccacaccggtgacacaacctgcttcgacgcggatcggctgctgtaatggcaccgcacaagctcggggccctgctcatcggcaccggcgcggcgctgctcggcgcgttttcccgcggcatgtgggtcactgcgacgtacaccgacgagcttgccggcggcggggttgcccacattcgcggcgccgagtggtccaccgagaccactgcagttgcgctgctgctgttcgttgccgcgataggggcatttgctttacgacgcaccggtcgccgcctcaccgccatcatcgcagcactcgcgtctctcggcgctgccgtctcccctgcccagctgcttatccgaggcgccgacccggaccgcgtccacgccctgttgaccgcgggactggacaccgctcagaccgccagcactacgcaaggcccggtggtttcggagtgggcggaaacgaccgctgcggacgtcgccacgctcttcccgctactgagcctcgccggctgccttatcgcctttgccggcgccgtattggttgccgcgcgcccaggtgaagatgcgccgaagcagaacaagtacgagaaagaagcggtgcgccgcgagcgactcgccgacgatctggagaccaaccccgactccggccgcgtgatgtgggatgcgctcgacgctgacatcgacccgacggacaccacgcccacgcgaccctgattatcggcgggcggggttttccagctaccttaaagacatgcttgccccgagcgcggtgaacgagatcgtcaccggagtgttgcgtgacgtggcgaagcgcgaagccgtcctaccgtttcaggaagtgaaagcgcgctcccgcgacatggcacccacccgcgacgcccgttccgcgttgttgcggccgggttgcagcgtcatcgccgagatcaagctcgattcccctgtcttcggtccgaccggcgtgaagcggcggaacatcgcggatgtcgcgcgcgccatcgaagaaggcggggcgcacctcatcggctgccagaccgagcggctgcgtttcggcggctcgctcgaggatatggcgcacgctcgcgccgccgtcaacctgccgatggtgtgccgtgacgtgatcgtggatccctaccagatccacgaggcgcgttgctacggcgccgacgtcttaccgctgcaggtgggcattttggaagaagcccggctcgcagcgcttctcgacagggccgagtccctcggcatggtcgtcatggccgaagtgcgctccccccaggaggcggacctggcgctcaaagtcggcgccagcgtgatcgctgtgaactcgtggaccttcgacaccaacgatttgcgccccggcacttttgcggagattgtgccggggctgccgtctgaagtgatcaaaatcagcctcggcggcgtgaccacggtgcgcgacctcctcgacgcagcggcgatcggcgcggacgccgtgctcgcggccgaggcgatcatgagcggcgatgacatctgcgccgccacccgggcgctcgccgcggccggccagcacccggcgtgcccgcgccggtagtgcatactattgcacgtgcacactcagattctcgccaacatcccgtccccgccccagggcgtgtggcacctcggtccgatcccaatccgcgcgtacgccctgtgcattatgacgggtatcatcgccgcgacctacgtcggcatccgccgctaccaggcacgcggcggcaacccggacacggtgtgggacgcgctgatcgtctgcgtgccggcaggcatcatcggcggccggctgtaccacgtgatcacagaccacgataagtacttcggcgagggcaagaacccgtggcaggcgttcaacatcaccgccggcggcctcggcatctggggtgcggtcgcgctcggcgcgttggcgctgttcgccctgatgaagcacaagggcctgccgttcttaccgctcgcggactcgctggcgccgggcgtcgtcctcgcccaaggcatcgggcggctgggcaactggtttaaccaggagctctacggcgcgccgacggacgtgccctgggcgctcgacttgtactaccgcgtggacgagttcggccgctacgctccgctgaacggccgctccacgggcgaggtcatcgcgagcgtccacccgacgttcctctacgagctgatctggaacgtgctcgtgttcttcctgctgatctgggcagataggcgcttcacgctcggccacggacgcgtgatgtggctctacgtcgccggttacaccttcggccgcttctttatcgagctcatgcgcaccgacgaagccaccttgatcctggggctgcgcgtcaacacgtgggtctccgcgattttgttcatcgttggcgtggtgatgttcctccgctcgccgaagggacgggagacgccggatgaggttgacccggcctacgaggcgccgccagccggcgagcgaaccagcgcaaaatgagtatcgttagcgctgtggaaagacgaacgaagatcgtatgcacgctcggtcccgccgtggccaacaaggacgcgatcctggggctggtgcgagacggtatggacgttgcccgcctgaacttctcgcacggggattacccggaccacgagcagaattaccgctgggtccgcgaggccactgatgagaccggccacgccgtcggcatcttggccgacctgcagggccccaaaatccgcctcggccgcttcggcggcgacggcaaaacctactgggaaaccggcgagacggttcgcatcaccgtcgacgacgtcgaaggcacccacgaccgcgtgtccaccacctacaaaaacctggcgcaggacgcgcagccgggggaccggctgcttgtggatgatggcaaggtcggcctcgtctgcgtcgaggtcgatggcaacgacgtggtgtgcaaggtcaccgagggcggcccggtttcgaacaacaagggtgtgtccctgccggggatgaacatctccgtgccggcgctgagcgagaaggacaaagaggacctgcgcttcgcgctgcgcatgggcgtggacatgatcgcgctctccttcgtgcgctcgccggcggacgtcgacctggtgcacgagatcatggacgaggtcggccgtcgcgtgcccgtgattgcgaagctggagaagcccgaagccgttgacgcgctcgagtcgatcatcctcgccttcgacgccgtgatggtcgcccgcggcgacctcggtgtggagatcccgctggagcaggtgccgctggtgcagaagcgcgtgatccagattgcgcgcgagaatgcgaaaccggtggtcgttgcaacgcaaatgctcgactcgatgatcgagaactctcgcccgacccgcgccgaggcctctgacgttgccaacgccgtgctcgacggcgcggacgcggtgatgctctccggcgagacgtcggtgggcgtggacccgcacaacgtggtgcgaaccatgagccgcatcgttcgctccgcagagaccatgggcaaagtgccgcctttgaaccatatcccgcgcaccaagcgcggcgtggtttcgtactcggcgaacgacatcgccagccggctcaacgcgaaggcgatcgtcacgttcaccacgtccggcgacacggcccgccgcgtggcgcggctgcaccccgagttgccgctgcttgtgtttaccccggtgcagcaggtgcgctcccagctcgcggtgacgtggggtgtggagaccttcctctgcccggacgtccacaacaccgacgacatgctgcgcaccgttgacgagtacctgctcgcgctggaccagtaccaagagggcgacacgatggttgtggtggcgggcatcccgccgggagtttccggcaccacaaacaccatccacgtgcaccagctgggcgaggacacccgcaacccgcggtagccgtacgctggggtgcatgcccgaaacgaacgactgcatcgagattcgcgacgcgcacctgcacaacctgaagaatgtcgacgtggacattccccgtggccggttggtcgcggtgacgggggtgtccgggtccggcaaatcctctctcgccttcggcaccatccacggcgaggggcagcgccgctacttggagtcggtggcgccgtttgcccgccgcctcatcggctcggcggtggatccgcaggtcagccaagtcgagggacttccgccgaccgtggcgttgcagcagtccaccaccggcggcggtgcgcgctctaccgttggcacggtctcggcgatgtcgaacaccatccgcctgctctactcccgcgccggcgacaacccggaggggctttactccgactcgttttccccgaatacgcccgaggggatgtgtcccgcctgccagggcaccggcgtggtgcacgagcccacggaacaatccatggtgccggatcccacactgtcgattgaggagggcgcgatcgcggcgtggccgggcgcgtgggccggcaagaacttccacgacattttgaagacgctgggatacgacctcgattcgccgtggcaggacctgtctgaggaagaccgccaatggatcctgttcaccgacgagcgcccggttgtcaccgtcaagccgacccgcggcgccgaccagatccagcgcaactatgagggcacgtggcgctctgttgcgagttacctgactaagacgctggcagagacccagtccgacaccctgcgcaagcgcgtgttgggctacatggagtcgcgcgtgtgcgaagtctgcggcggccgccgcctcaacccggaggcgctgaacgtcacctacgctggcatgcctatcgacgagctcgggtcgcttcccctcgaccgcgtgcacgaggtgctgtcggcgcagacgccggcggagaactccgcggaggcgctgttgctcaagcaggtgctgcctgcgctgcagtccgctctcgatctagggctgaagcacttgagcctcgaccgccccgcggcgactttgtcggccggcgagctgcagcgcatacgcctcgctgcgcagcttcgctcagggcttttcggcgtggcgtacgtgctcgacgagccctcggctggcctgcaccccgcggagcgcggtgcggtactcgacatttgccgcaacttcatcgaggccggtaactccgtgctgctggtcgagcacgacatggaacttgtcgccgaggctgactggctggtggacgtgggcccgctggccggcgagcgcggaggcgaggtggtctactccgggccggtggcggattacgacgccgacactcccacagccagcgccctgaaacgcagggggctgacgcttaacgacgcaccccgcaaaccctccggcaccctcaccctacgaggtgtcaacgcccgctctatcgaggacgcggacgtctctttcgggctcgggcagttcaccgcggtggcgggtgtgtccggctccggcaagtccacgctggtcagcacggtgcttgccggggcattgcgggcgacgacatcgtcaaccgccgcgttcgagggcgaagacgaggagcagcacgaggacaacggttggtcttacgccgagctcgagggtgcggatgcggtgagccgggttgttcaaatcacccagaagccgatcgggcgcacaccgcgctccacaatcgcgacgtacacgggtctgttcgacggcgtgcgcaagctcttcgccgaaaccgacgaggcgaagcgccgcaagtggagcgtgtcgcgcttttcctacaacgtgaagcagggtcagtgcccgacgtgcggcggcgccggcaagattgaggtcgagctggtgttcctgcctgggtcctacaccacctgtcctgactgcggcggcgcgcgctacaacgacgaaaccctcgaggtcacgtgggagggcctcaacattgcggaggtgctcgacctcaccgtggacgaggcgcgcggcgtgttcgccgaggagcccagaatcctccgcgcggtagaaacgctgcaggcggtgggtctgggctacctgcggttgggccaaggtgcaccggaactatctggcggcgaggcgcagcgcatcaagctggccacggagctgcagcgcgcacgcacttctaggcgcggccacaccgtgtacctgctcgacgagccgacaaccggtcttcacccggcggacgtcgacctgctcgcgcgcgaactcaacagccttgtggacgccggccagaccgtcatcgtcgtcgagcacgacgcacgcgtgatcgcgcaggccgaccgcgtggtcgagatgggcccgggcgccggcgccgacggcggcgaaattgtcgccgagggctcaccggcggaaatcgccaagcgcggcaccccgactggcggggtgctcgctacgcgcagcgcgtaaccctgccggttacgcgggttacaccgggtgcaccggcgttggctcgatcttccacacctcgttggcgtagtcgcggatcgtgcggtcggaggagaagcggccggattcgcagatgttgatccagcacatgcgctcccagcgctgcgggtcgttgtagtagtcgcgcgccatgcggtcgcgggtttcgcggtaggaggcgtagtcgcccagcacgtagtagacgtctgggtcgtcgtacccgaagccgtcgagaagcgactgcttgatgtcgtggaaagcaccggagccctggtcgtcgagggtgccgtcggtaagcgcatcgagcacccgcatcaggcccggggtgtcttgcgcgacctggcgggggacataggtgcgcttaagctccggcaggtcctcctcgaacgcgccgaagatgtacgcgttctcctcgccgacagagtcgacgatctccacgttcgcgccgtccatggtgccgagtgtgagcgcgccgttcatcatgaacttcatattcgaggtgcccgaggcttccttgccggcggtggagatctgctcggagacgtcggaggccgggatgatgtgctcggcgggggagacgttgtagttctccacgaacacgacgtggatgtacttcgacacctcggggtcgttgttgaccagctcgccgatggtgttgatgagtttgatgatgcccttggccatggtgtagcccggggccgccttcgcgccgaagatgaaagtgcgcttcgggatgtcgcgctcgccgtcctccttgatgcggaagtacaggtccaggatgtagagcgcgttcatgagctggcgcttgtactcgtgcaggcgcttgatctgggtgtcgtagatcgagtccgggtcgatctcaacgccctggcgctctcggatccagtcggcgaagtcgcgcttgttcgcggccttgacctcgcgcagctcccgcatcacatcggcgtcgtccgcatagtgccgcagctgttggagcttggacaggtcggtgacccattcgtcggaaccagccaggcggtcgagcagctcgctcaggcgagggttgcacatgcgcagccagcggcgcggggtcacaccgttggtcttgttgttgaatttctccggcgccatggcgtgccagtactcgagcgtgtcgcgcttgagaatgtcggtgtggatcgcagccacgccgttgatggagtacgacgcgtagcaggcgatccacgccatgtgcacgcggccgtcgtggaccggggagtagcggtgcgcctcctccgggccaatgccgcgggcctccatgtcgatgcggtagcggcggtcgatctcctgcacgatctcccaaatgcgccagaacagctgcttgaagatggactcttcccaggtctccagcgcctcctgcagcacggtgtggttggtgtaggcgaaggttttggtggtgacctcccaggcgtcttcccaggtcatcccgtggtcgtcgagaagcaggcgcatcagctccgggatcgccagcaccgggtgggtgtcgttgagctggatggagttgtacttgtggaagtcccgcaggtcctcgccgtggtgctcgatgtagttgtccaccagctcctgtagcgatgcggagacgaagaagtactgctggcgcacgcgcagcagcttgccggcgtaggaagagtcgttggggtagagcacgcgggtgatgtcgtgcaccgcctcgcgctccaaaatcgcgtcggcgaaacgctgggaagaaaacgcgtcgtagtcgaactcgtccatcggcgaggcgtcccacaggcggagcgtgcccacgttgtcggtgccgtagccggtgatcggcatgtcgtacggcacggcgcgcaccgacatgtcgtcgaacttcacaaaccgctgctgcgtgccgcggcggacgatgaaggggtagaaggactctttccaggcgtccgggtgctccttctggaagccgtcgacgaactcctggcggaacaggccgaaacggtacaacaggccgtagccggtcagcgggtagtcctgggtgacagcggagtcgaggaagcaggctgcgaggcggcccaaaccgccgttgcccaaggcggcgtcgtgctcggcttcgagcacgtcggacagttcgtggcccatctcgcgggcgagttcctcggcctcgtcgaccaggccgaggttggtgaggttgtttaacagggcgcggccctgcaggaattccgcggagaagtaggcggcttggcggttcgcggcgtaggtggtgcgggtggtgtcccagttgtcggcgatcttctccatcaccgcggcggacaggcccgtccagaactttttgttcgtcgcccgctccggagaggacccggagaagctcttcacgtggccggcgaggctatcccgcagctcgggggtgtttgcgtgggtatccaatgattaacctttctcaccgtttcgcttgacagtcctgcccaagcctaccggcgcacgcggcgttgcctcttacgaggcaaggacactgagcgcggccaccaatcccgcctcggtggcggagcggattgtcggcgcgtaatcgggcaggaagttcggcatgtgattcaccggcgcctcgccgcgttcccacgcgtcggcgggcgtgcacccgatcaaccagaagaagtacggcacgccgaacgcggcggggatggcggggaaatcctccgagacggttttcgggtcggaggtgacggattgggaggaaaagtgggcgtcgaaaagcgtcctgatgccctgataggtcgcttcgtcgttggtgagcagctcgccgtgcgcgaagaactcaatcgtcggttccgcgtccacgccagacgcggcgacctccgcgcgcaccacgcgctcaatggaggcgtaaaccttcgccttgactgcgtcggagtagaagcggcagttcagcaccagctcagcggagccggggatgatgttgttggtggttcccgcgtgcatggaggcgacggtgactacggcgaagtcggccgggtccacctcgcgtccgacgatcgcctgcaggcgggtgatgatcatcgcggcggtgaacgtcgggtcaaccgaggcgtgcggcatggagccgtgggcactgatgcccgggatggtcacgcggatggagtcgcacgcggcgaactgcgggccgggtttgctcatcacgtcgcctgcgcggccgggcatcacgtgctgggcgaagcagacgtcggggcgggggatgcgcaccgttagcccgtccttgaccatcgcggcggcgccctcgcccgtttcctcgcccggctggaacagggcgataaacgtgcccgaccagtggcggcgcgaacggtcgaggacgtcgcacatgctcaacagcgcggtggtgtggatgtcgtggccgcaggcgtgcatcgcgccgttggtggaggcgaagtccgcgtcggtgtcttcgaccaccggcaacccgtcgaaatcggcgcggtgcagcacgactgggccgtcgccgttggtgaacacagcgcaaataccggtgcgcccgacgggggtgatgatctggcagtcgaagcgcgccagctccgacaccaggcgctggtgggtctcggtttcgcgcatggacagctctgggtgctggtgcatccactcgtagaccccgcgctgccactcggcgtccaccgggtaggcgttgatgatgttggtgattgtgcccgcgttatccgtcatgagttctctcctacctggtgttggattgctgcagcatggggttgtagcgcaagatattccgcgccgacccgcactcggccgcaataaggatgccgccggcgatacggcgctcatcgcgcagccggtacaagttggtcaccagccggtccctgatgtcgaagggggaaagcgtgttgacgtagatcttcgtgccgccctcgaagcccgcgacagtggagatgcgccacttcacgttcacgcgccacggcatcggcacgtccaagtccacgggccggtagtgccactcctcgttgcaagctacgtcagcgccggtggctgcgtggagcgcgtgcaaaaggtcggaaaacgcgcgcacttcctccggcgcctgccgccacggctcgcacacggcagacttcgaatacaccgtggcggtggggtagcggtgcccgatctccgccaccagcaccgcgtgctcgttctccgcgatgaccaggttgtggttcagcgcgtagttgacaccccactcgttgtagaggttcacgttgcggcgcagtttctctatttcgatctccgcctgcacgccgcgctcgtcgatcgccacaagttgcttgtgcaggtggtcgaagcttgcgcccgcgggctggagccagttctggaacaccaccacgtacggcgagtacgggttcgcctccagcaggtcgcgcagcgcgtcgatggtgaacacggtgaacgcgtggtgctcgtcaggggtgagcgtgccggagccggcgagctgggagtcgtccgccgcgccgtcgacaaagtggcgcctagcgatgatcacgtcgtggccgccgccgaaatacgccggaacgatcgagagcagctcctcctcgctgtggtcctcgcccatgcccgaggcctttaaccgggtgcgcgcaatgcccagcacgtgctcgcgcccggccggatcagccaggtagcggtccatgtgctcgcgccgggccggcggcatttcgtagccgtaattttgcgcccagtagtcgtaggagacgatctcgaacaggttcggcacccggcggaactcggcgcgggtggcgtcaagctcgccgggaagcaggtcgcgcacgattgcccagccgctttcggtcctcaccatccgggatttttccggcggggtggctagaagccggtcttcgcagaagttgcagctatccgtctgcgcgccgggcccgagggcctccggctccttcgcgcggtgggtcagcggccggttgccgcggccgggcacggtccacacttgcgtcccggagaacggactgacctgcttgatcgtgccgtccgccatggtggacagggcgtttctggctgcgttgaccgggaagggcatgcttctcagactaccgcgctagcctgtacacccatgccagcgattattttcgacgtcctcgttcctcccgcccacgccccgcagatcggggccgcgttccagcgcgcgctggacattctggtcgcccgggggaagctcactgctggtcaggtgcgcgaggagggcattgtgcttatcgacgcccccatatcctcccaactcgcctccacctacgaagccgaccgcggcactgaccccgccgacgacggcgccgaggttcaccgctaccgcattggggcagagggcgctgccagctacaaccagctcgcgatggggctctcacgcatcctcacgccgaaggcggacctgcccgccgaccccgccgcgctcgagcagcaggaccgcttcgaggtgccggcgatctacccctggacggtcgaggtgctgaggtagcgaaccgccgcctcgcggccggtttggcgcagctgatcggggctctgcgaaagcggcaccgtggtgacggtcgcgccggggttgagtgccgacgcgagttcggccaccgcgtcgacgccggcgcctgaggtgatgacaagggaggcatctgcaagcgccgcggccagcccgctggcctcagccaccgcctgggcgccgggcacgatccgcacgtgggaggcgtcgccgtgcagcagcgtcgaaagccaggtgatgccgattggcaccccgcccgcggctgcgatgccgggggaggcggggtcgatgccggcgacctcgcaaagcttcgaaagccccctgtcgatgacctcgaggtcaccctccggcacgtgcccgccggtcgggttgtcagcgccggtgagcagcacccactcgacggcgccggcgggaatgttcaccttcgcggtgtcgaggtccgcgatctgctcgagcttcccgccgccctgcggcagctggtagccgcgcgcgtcgagcgggttcgcgccgagggcgaccaagatgccggcgccgccgtcggctgtggcgcagccgccgagagcgagcacgatagtttctgcgccgcgggtctgcgcgtcggcgatcagcacgccggtgccgtaagtgtcgccggtgagtagcacaggtttgtcggtctgcgctggggtgccggaagctgcggcgacgtcgatgaacgcggtcttgctcgccgcgtcgaacgtgtacgtcgcctccgtcaggcgccccgcagcgtccgtggtgggcagggtgatccgctcgccctcgaacagctcggaggtccctgcgccgccgtccgcgagtggtgcgatcgtgacctcagcgtcgcggatcacttcgcgcacaccctcgcccagccattgcgccgcaccgcccgtattcgcggcagcgctcgctggctgcagcgcgatcacaaccttcggcgaacgcggctgggtagttccggaatccatggggtgctcccttacgtttcaggtcgtgctttccgcacgttgtcagtagggcacgagtttactgtgggcattccgtcagattcctccgcccggcgggcatcggttgtaaaatcccctcccgtactacttttcgcccagataactccggaaggatgttccatgacttctatcgaccaagaagttgccggttactacgacagattgctgaagcgcaacgctggcgaaccggagttccaccagtctgttgccgaggtgctcgactcgctcaagatcgtcctgcagaaggacccccactacgccgactacggcctgatcgagcggctgtgcgagccggagcgccagattatattccgcgtcccgtggatggacgacaacaaccaaatccgcgttaaccgcggcttccgcgtgcagttcaactcggcgctcggcccgtacaagggcggcctgcgcttccacccgagcgtgaacctcggcgtgatcaagttcttgggcttcgagcagattttcaagaactcgctgactggcctgcccatcggcggcggtaagggcggctccgacttcgacccgaagggtaagtccgacgctgaggtcatgcgcttttgccagtccttcatgacggagctgtggcgccacatcggcgagtaccgcgacgtgccggccggcgacatcggcgtcggcggccgcgagatcggctacctcttcggtcagtaccgccgcttggccaaccagcacgagtcgggcgtgctcaccgggaagggcttggagtggggcggttcgctcgcccgcaaggaagccaccggctacggcgcggtgtacttcacctccgagatgatgaaggccaacggcgagtccatcgacggcgcaaacgtcattgtgtccggttcgggcaacgtggcgatctacgctatcgagaaggcacaggagctcggcgccaccgtcgtcggtttctccgactcctcaggctgggtgtccaccccgaacggcgtcgacgtggagcttttgcgcgacgtcaaagagaaccgtcgcgagcgagtgtccacctacgtcgaggaggcacagggcgcgactctgcacaccgacggctctgtgtgggatctgcaggccgacgtggcgctgccgtgcgcgacccagaacgagctcaacgctgagcacgcccgcgccctggtaaaaaacggcgtgaagtacgtggcggagggcgcgaacatgccgtccactgccgacgccatcgaggtgttccgcgagtcgaagacggcgttcggcccgggtaaggcggccaacgccggcggtgtggccacctccgcgctggagatgcagcagaacgcctcgcgagactcctggtccttcgagtacaccgacgagcgcctgcataagatcatgaccaacatcttcaaggtcacctccgagaccgcggccgagtacgaccgggagaacgactacatcatcggcgcgaacatcgccggcttcaagaaggttgcggacgcgatgctcgctcagggtgtggtgtaacccgaaacccctgtccgggccgtacgcttgggagctatgtaccgcgtatttgaagccctcgatgaacttgtccagaccgtggagcaggcgtacggcgtgcccatgacctcgaactgcatggtgccgcgcaacgacatgctggcgcttctcgacgacctgcgcaatgcgattcccgaagaactcgacgatgcgcaggacgtactggaccagcaggacgagatcctgcgcggcgctcaggagcgcgccgatgtcatggtgcttgacgccgaggacgaggcccgccggcttgtcgacgatgcgcactcccaaaccgagagcatgctctcggacgcgcagtcgcaagcaacgcttctggtctccaacgccgagaacgacgctaacgcgactgtttcgcgcgcacgcgaggaagctgacgtgacggtcggccgcgcccgccaagaggccaaccgcttggtcgaatccggtaaccaggagtaccagcgcagcgtcgacgagggcttggcgcagcaggagcgcctcatctccgagtcggaagtcatgcgccgcgcggatgaggaagcgcaccgcctagtcgagcaggcccacgccgagtcctcgcgcctgcgtgcggagtgcgacgactacgtggacgcgaagctggcggagtttgaggagtcgctctcctcggtgctgcgtaccgtgtcctcggatcgcgccgcacttcgtcgcggcgccggtgcctccggtgtgcagcgcaccgagagcgagcgctacgtgccgcgcgagcgcacccgccgtccccgcaccaaccagcctgcggacggttactccgaggagtactaacctcgggcgtctggctgtattgtcagaggcgctatgtctgacaatcctttcatcattgatgtcgccgacgcgctagacggcgacggcctgccaatcaccgtgacgcagacgggcccgtctccgtcgaggatcggcccagaaatgattgcaatcccagccggcaacgaggttgaggtcgaggcgaccatcgtcccgctcggcaacggcgtgatggtggacgccaccgcccgcgctgagctgctgggcaactgcgtgcgctgccttaaagagctgcggcctgttgaaaccatccgtatccagcaggtgttcgccacctctgacagcttcatttccggcgacgcggaagcggaggaggacaagggttccggcgatgagattatgtacgtcgttgacgacaaggtcgatctcgagcaggcgtttgtcgacgaggcgggcttgacctggccgttcaacccgacctgtcagcccgagtgcgagggcgataccgatgtgccgtaccacgagcgcgtgacaagcgaggacgaggagcgcgttgacccccgctgggccggcctggagaagtttctgtgacgcggtcgcgaaagaagaagatcagcgacgaggacgcgtggctgaaagcctttgatgccgtcgaccacgccccgctgctggagaacctgggtgcgcaggtttctcccgagatgctgaagctcgcgctgacgcaccgctcttttgccaacgagcacaatcacctgccgaacaacgagcgcctcgagttcgttggcgacgcggtgctggggctgtcggtggcaaccaagctgttcgagctctacccatcgcggcctgaatcggagctgtcgcccatgcgcgcgtccatcgtgtcgcgctacgggctggcggacatcgcgcgcgagatcggcctcggcgaccacgtgctgatcggccgcggcgaggagctcaccggcggccgcgaaaaggagtcgatcctcgcagacacgaccgaggcgctcttcggtgcaatctacctcgagcacggtttcgaggcggccagcgacgtcgtgctgcggctgttcgacgagaaactacgaaccgccaccgcctcgacgaagcaccaggactggaagaccgcgctgcaagttcgcctcgccgaactcaagctgccggtcgccgagtacctgtcggaggttgccggcccggagcacgaccagacgtttacggcgcaggtgcttgtggacggcgccgtgcgcggcaccggaaacggcccgaacaagaagcttgccgagcaggaagccgcccaccaggcggtgctgtacctgcgagatcacgcgctcgatgcctgaactgcccgaagttgaggtcgtgcgccgcggccttgactgtcacatcgtggggcgcgcgtttgagcacgtcgaggttctccacccgcgtgcggttcgcggaaacacggtcgacttagaaaaggcgctgcccggcagggtcgtaacggccacaggacggcgcggcaagtacatgtggctcgtgcttgacggggtcgacgcgttgcttgtccacttgcgtatgagcggacagatgctcgttaccgaaccgggcggcgcgaaaagcccgcacttgcgcatccgcgcgagcatgagcgcccgcgggggagagccggccgttgatctcaacttcgtggatcaacgcaccttcgggttctggcagcttgccgagtttgttgacgacgccggcacgctcgtgccgctgcccgcggcgcacgttgcgccagatccgttcgaggaggcgttcagtgtgcgcgataccgcccgcgccatgcggcagaagcgctcgcccttgaaatctgtgttgctgaaccaagaggtggtctcgggtatcggctccatttacgccgacgaggcgatgtggtcgacgcgactgaagccgtggcgcactgcacgcacgatgcgccagcgcgacgccgaagcggtgctcaaagcctcgcaagaggtgatggcacgttcgctggagcagggcgggacgagcttcgacgcgctgtacgtcaacgtcaacgggtcgtccgggtacttctcccggtcacttaacgcctacgggcaggcgggcgtgccgtgcgcgcggtgcggcacccccatcgagcgcatagtcgtcggccaacgctccagctatttctgcccgacttgccagattttataaatcaacggttaagattcccgccatggatgcagccctcaatttcgtagacggcaccctgaacggggtcatttggaaagccgtcccttggttccttgtgggcgcgggtatttacttcggcctgcgcacgttcttcgtccaagttcgcatgctgccggacatgttcaaggctgtcaccgagacgccgaagggcaaagacgctgaggggcgcgacctcgacgaggagtacgggggcatctctgcttttaaggcgttcaccatctccgccgcgtcgcgagtgggcaccggcaacatcgccggcgtggcactggcgatttcgatcggcggcccgggcgcggtcttctggatgtggatgctggcgctgatcggtggcgcgacctcgtttattgagtccacgctcgcacagctgtggaagaccaaggacgccgagggcaactaccacggtggcccggcgtactacatgacccgcggactgggctggcgcccgctggccgtgctgttctcgctcttcctcgcgatcacgtacggcttcatctacaacgcgatccagaccaactccatcgtggaggcggtcagcggctcgctggacaacgactcggtgacggtgaaggcgatcgtcgcagccgttatcgccgtgctcaccggcctcatcatctttggtggtgtgacccgcattgcgaagtggacccaaatcatcgtgccgttcatggcgggcgcctacatcgtgctgggcgtgtgggtgctcatcgtcaacgcgagtgagatccctggcatggtctccatgatcgttgagcacgctctcggcattcgccagatcgccggcgccgccgtcggcgccgcgttcatgcagggcatgcgccgcggcctgttctccaacgaggccggtatgggttccgccccgaatgcggctgcgaccgcgaccgtgtcccacccggtcaagcagggcttggtgcagactcttggcgtgtacttcgacactctcgtagtctgttccatcaccgcgttcgtcgtgctgctcggtccggccgtgaactacggcaccgacgacatccagggcgcagcgctgacccaggcggcgctggctgactccatcggcgcgtgggccgcgcacgcgatcacgttcatcctgttcttcctcgcgttcagctccgtgatcggcaactactaccttgcccaggcaaacctggagtacctcacggattccaagaccgcgatgacggtcttccgcgtcgccgtgatcggcttcgtcatcttcggcgcgttcggctccgttccgctggtgtgggcactcggcgacaccatggcgggtctcctcgcgatcttcaacatcatcgcgatcattccgctgggcggcgttgccatcaagctgctgaagaattacaacgaccagcggcgccagggcatggacccggtgttccaccgcgacatgctgccggagctgaagaacgtggagttctgggacggttcggacccggtcacgaggcgaagtgtggaggaccgcatcactgcccgcaaggctcgccaggagggggagctctaagatggccgaggataagacccgaatgctcgcccacgtgcacggccacgtgcagggagtgggtttccgctggtggacacgctcgcgcgcgctcgagctgtcgcttgctggttacgcaaagaatcttgacgacggccgcgtggaggtcgcagccgagggggataaggagggcgtcgacaagctgaaagccctgctggaagagcaaccctccacggcgaaccgcccggggcgcgtggaccgcgtgcaggtgcagtacaccgacccgaagggtgcagaaggtttcgaggagcgataggtggatccgcagcgtttcaaggacgcgatgagccagctcgctgcggccgtctcgatcgtgaccaccggcggtgaggacgatccgcacggcacgacggtgagtgcgtttatgtcgctctcgcttgagccgccgatggtgctagtttcgctcgaccagcgctcgtcgctgctggctgagcttcatgtggggtcgtcgatcggcatcaacgtgctgtccacgcagcagggcacgctagcgcgccgcttcgcggacaagagcgtcgaccgctttgccggggtggagtgggagatggccgacggcgcgccgaagttgccgtgcaaccacacgtgggttgccggcaccgtttcgcggctgatcgagggcggcgaccacgtgctggtgctcatcgacgtcacaagcgccgaggtgaactccaaccagccgcttttgtactggcagcgcgagtttggcacccacggcacgatcgagccgggcgaggtgcgcgcgcaagcggtggattcgacgcgtccgtagagtttcggcgggggctacgggcgaacgtcgacgtcgaggcgagctccggttgctcgagcgtagcgctgcagggtggacaattgcgggtccgtgtccccgcgctcgagatccgagatcgcggactgcgtggtacccatcgcctcggccacgtccttctgagtaagcccggcagctctcctcgctgctcgcagcgcatcggcgagcgcgagacgcgcttcagcgtccgacgcggcgtctcgaatatcagggtctttcacaagctcgtcaaagtcgagcacgacggaatttgtttcgcggtggcgtgtcataccgctgccctccttatcggttcgggccgataataatgtacgcgcacatcgatggggtgcgagccgcgctgtaacatcaagtgaatgcacctgaaatcgctgaccctgaagggcttcaagtctttcgcgtcggcgaccacgatgaagttcgagcctggtatctgcgcggttgtggggccgaacggctcgggcaagtcgaacgtggtggatgcgctcgcgtgggtgatgggggagcagggcgcgaagaacctgcgaggcgggaagatggaggacgtcatcttcgccggtgcgggcgaccgcaagccgctgggccgcgcggaagtcacactcacgttcgacaactcggacaagcacctgccgatcgagtacaccgaggtggcgatcacacgccgcatgttccgcgacggcgcctccgagtacgagatcaacggcgccaaggcccgcctcatggatatccaggagctgctgtcggattcaggcatcggccgcgagatgcacatcatcgttggccaaggcaagctcgccgagatcttggaatcccgcccggaggagcgccgcgcgtttatcgaagaagccgccggcgtgctgaagcatcggcgtcgtaaagaaaaagcccagcgcaagctgacgggcatgcaggcaaacctcgaccgcctcaccgacctcaccgaagagctgggcaaacagctcaaacccctcgcccgccaagccgaggcagccaagcgcgccgccacggtccagtccaccctgcgcgacgccaggctgcgcatcgcagggcaccaggtggttcagcttcggagcttgcttgccgacgccgccacatcctcctcaaccctcaccctcaaagccgacgaagcctccgcagccgtggaagaggcaaccgcggtccaggaggcgatcgaggccgagcagtccgagatccagccggccgtggaggaggcacagcagcgctggtttggcctctctacgctggctgagcgcgccagcgccaccggccgcatcgctaccgagcgcgccaggggcgcaggcaccgaggtgccctatgccggccaggatcccgacgagctcgaagcccgcgccgccgccgcggagatgcgccacgcggaggcccttgaggctgcggaggaagccgcggagcgcctcgaggaggcacgcgagcaggtcgccgaggcgcaagccgagttcgacgaggcggagcgcgagcacatggccaccattcgggcgatcgcggaccgccgggaaggcgtggtgcgcctcctcgcccaggaggaatcgctgaagcaggcggtgcgcacggccgaggaagaggtcgcccgcctgatggagactcacgaggagtcccgcgcccgctctctcagcgcccgccgcgaggcagaagaggttgcggcgcggttagctgagatcgagtcgcagcgcggcccgctcgacgaggcgttcgtccgcgccaacaccgaatcgcaggcggctgagcagcgcctcgcgcagctgcgcgctcagcagcgcgagcacgagcgcatggtgttcacgctcgagtcgcgcatcgcgacgcttactgagcaagcgccgaagtcgcccgcaaccgaggtgcttgaaacccgcacctccgggtttagcgcgctcgccgagaagatgaccgtcgaacccggcgtggataccgccatggccgcggcgctggggccgcacgctgaggcgctcgtggtcgatttgggcacaggcctgagtgctggtgccgaagtcgccggcgcgctcgccgacacgcagcgcaccgtccttgtcaatggcgtctccgccgccgcgtcctcggcgtggcgccttgagacggacgccgccgtcgactggctgctcgaccacgtctcgcttgccgaggacatcagcgggccggtcacgcgactcctcgccgacgttgcgctcgccgacgacgtcgcccacgccgcccgcatcgtttcggaagacccgcgcctgcgcgccgtgacccgagagggtgtggtggtcggcgacggctggctcgccgccggctccggtcaggcgacggcggtggaggtcgcggcgcaggtcgacgcggcgcgcgaagagctggagatcgccgctgcccagctcgaagaactcgcgggcacgctcgagggcgcgacgcttgctgccgaggaggcccgcgtcgccgaagcttccgcgaaagctgcgctgaaggagcacgacgcactcgccgagtcgtggcgccgcgaccacgcccgcctgatcaagcaagctgattccagcaaggccgagcacgagcgcgcctccaagcgcgtggtggaggcccaggagcgcgaggcacggcgccgcagcgagtgggacgaggcccgtgagcgcgtcgcccgagtcgaggacgcccccggcgagcgggagccgtccaccgccgaccgtgaccgcgcgcaggctaatctctcccaagtcaaggctgtcgagatcgaggcgacgatggctgcgcgcgttgcgcagcaggctgcggatcagactgcgggtaggggagaggtgctgcgtcgacaagctgcgcacgagcgcgaagccaaggcacggcacgacaaagcgcaggcccgcaggcgtgccgaggcgcagttggctcaggcggtggtcgagctgtcgctggagctttcggcgcgtatcgacgccgcgttatcttccgcgaccgcccagcgcgacgaactgaacgtccgagctaacgcgcttcgctctcgccaccaggaagcccgcagcgcgcttaccgcagcccgccagcacgcggcgcgagctagcgaggccgctcacgcagctgacatcgcccgctcgcaggcgcaggtgcgtgtggacgaagcagaggccaaggtggtcgaatccctcggcatcgcggtcagcgacttggtggcgggctacaccccggatgccgagttcgacattgacgccgagcaggcgcgcttgaagcaggccgagaaggacctgcgcgccttgggcaaggtcaacccgctcgcgctcgaggagtacaaggctctggaggagcgttattcgttcctctccacccagctcgcggacgtgatccaggcgcgcgaggacctcacaggcgtgatcaacgacgtggatgcgcagatcctccagctgttcaccgacgcgtggcgcgacgtggagcaggagttccctaacgtcttcgccaccctcttcccgggtggcgaggcccgcctcatcctcaccgaacccgaggacatgctcaccacgggtatcgagatcgaggcccgcccgcccggcaagaaagtcaagcgcctctctcttttgtccggcggcgagaaatcgctcaccgcgctggcgttcctcgtggccatcttccgcgcccgccccagcccgttctacgtgcttgatgaggtggaggcagcgcttgacgacgtcaacctccgccgcctcatcgccctcctcgaagagcttcgcgaggactcccagctcatcgtgatcacccaccagaaaccgacgatggacgtagcgaacgtcctctacggcgtgaccatgcgcggcgacggcgtcacccgtgtcatctcccagcggatgagtcccgctcccaagaagccggcgtagtatcatccaaaagttgtagaaaggatggctatgtctgtttcacgtgtgctcagtacctgcggcgtcctcgctgttgcattgctggctgggggttgcgcaagctccggcgacctcgacggcgtctacaccaaggttgaatccgctgggacggtggaatctggttccatcaccagcaccttgaccatcagcggcgacgactgctcgatccacgacaaggccgagcccggtcacgtcgagcgcgaccaaacctgctccgttgaagggggagatttgatcttcactgaaggggatagccaggctgcggtgccgtttgctcgtactgctgacggcgacgtgcgtatcggtgtgggcgacggggaactctaccgcaagactggcgaggcctagatagcaccgcgtcccccaagtgttgtcagccgatcgcggcggcggctggcactatgggtgtcatgactaacacgacaattctttggatcgttatcgcgatcgtggtgctcgtgctgatcatcgccggcatcatcgttgccggtaatcagcggaaaaagtcgaagaccgtttcgtttgaaaaaccggcagaggtggagcagcccaagcagctgactcgcgaggaaaagtcgggcaactaccaagccaagggcggcttcaacttcgcgcaggccgacgccgcgccgaagcagccggagccggtgcgtcgtcaagcgcctagcgctcccgccgcgccggaggcgctcgacacgtcgaagcctgttctcgacccggatctgcagaagcagatcgacgactcgctgaacgagccggcgccggccgagccggagcagacggccgcggacgcggttgaagaggtacaggccgcggttgagcaggaagagccgaagccgttcccaactgaggagacggttgagcgggtggaggagcccgtcgtcaagcaggagcccacgccggaaccggaaccggtggtcgagccggttgaggagcccgtcgttaagcaggagcccccgcgtgagccggtggttgagccggaggttgtaaagaccgaggagaccgcccgtgaggaagccgaggaggctgcggcggccgcggcggaagctgttgaggccgccgacgaagcggtgaaggaagggtcgccggtatcggacgacgcggttgttgtggacgcgccggagacggcggcagttgcggccgagattgatgagatcgcgccggcggccgggcgaattggcaagctgcgtgggcgactgtctcgttcgcagaacgcgattggtcagggcctgctgggcatcctcaccgccggggacctcgatgaagatgcttgggaggagatcgaggacacgctgatcatggcggacctcggcgctgacttgaccatgaaggttgtggacaacctccgcgagaagatcgctgagcgcggcgtctcctcggaggaggaagcgcgcgcgatgctgcgtgaaactctcatcgaggcaggccgccccgacatggaccgctcgatcaaggcgatgccgaacgacggcaagcccgccgtcatcttggtcgtcggcgtgaacggtaccggcaagacaaccaccaccggcaagctcgcgcgtgtgctggtgtctatggggcacacagtggtcctcggtgccgccgacaccttccgcgcagcggccgccgaccagctggagacctggggccgccgcgtcggcgcctccactgtccgcggtaaggagggcgcggatcccgcctcggtcgcgttcgacgccgtcgcaaccggtgtcgatcagggcgctgatgttgtggtggttgataccgccggccgcctccacacctcgaccggcctgatggatcagctgggcaaggtcaagcgcgtcgtggagaagaagagccacgttgacgaggtgctgctggttctcgacgccaccgtcggccagaacggcattacccaggcgcgcgtgttcaaggacgtcgtcgaaattaccggtgtcgtgctgacgaagctggacggcaccgccaagggtggcatcgtcttccaggtccaagaagagctcggcgtgccggtcaagctcgtaggcctcggtgagggtgccgacgacctcgcgccgttcgaggtggaaagcttcgtcgacgcgttgctggggtagctcgcagtttcgtaagggggggacgcgccgcgggggcggcgcattggggg

SEQ ID NO: 19 - DNA, 20046 bp, Corynebacterium cassirii
  source 1..20046: mol_type = genomic DNA
gggaggtgctgggggaggggacgaaccgtcgagaagcaaactgcgatcccacagcccacgccgaggttgaagcgatccgcatggcggcgcgaaccttaggctcctggcgccttgacggctgcgagctggttgtcacgctggagccctgcaccatgtgcgcgggggcgatcctcggcgcgcgcgtgcgctcggtggtgttcggggcgttcgagcccaagaccggggcgtgcggttcgcttttcgacgccctccgcgacccccaccacctccacaccgtagaagtgcgcggcggcgtgctcgaatcagcgaccgggcagctcatgaccggctttttcactgctctccgtgactgaattgttatggcgggcgcgcgggtagcgcgggtaagctcggaaatgttagtaacaaatcgagcaaaggagaccgttatggcattcgaaggcaaggctgaccagatcaagggcgacctgaagcaggctgctggcgacgtgaccggcaacgagtccctctccaacgagggcaaggccgacaacctggtcggcaacatcaaggagggcctgtccgacgctggcgaggccatcaaggacaaggcaaacgaggttgccgctaaggtcgaggacaagcgcgaggagcacgaggctgagaaggccgcggagaacgctgctgaccgcgcaaccgacatctaaaggcgatcttggcgggcaaatttggccgtgagtaccgccaaccgttacgctagctagcggtagcgtgtccgagcggccgaaggtgctcgcctcgaaagcgagtgtgggttaaaccaccgcgggttcaaatcccgccgctaccgccacaactggcacctcaagcaggtgccagtttttcttttacctgccgccgattcgaaggacggagacttggcgaagctgctgtaccggctcgggcgctggtcgtatgtgaacaagtggaaggtcatcgttgcctggcttttgatcttggccgcctccgccggcgcggcgctgtcgctgatgaagccgttcacatccgagttcaacatctcgggcacgccggcgatcgacgcgctggacacgctcgaggacaacttcccgggcggcggcgacgtggctaccgcgcccaccgtcaacctcgtcttcgcggcgccggaaggccaaacccttgacgcgccgcagtacgacgccggcatccaggcggccgtcgaccacatcgcggcgaacctggagatcgagaacacgctgcgcttcggcaacccgctgcgcatcaacggcccgctgcaggacgagctagttgcgcagatgacggagctcggcctgccggaggagacggcgcgcgccgatgcgcacaatctgcgcttgcttagcgacgaccaccgcatcgccttcaccaccttcgacttccaagcagagtccagcttcgccgtgaccgaggaccagcgcgaagtcgtcttggaggcgctggacatcgcccgtgacgccggcctgcaggcagaggcgggcggcgccggcttcggtgacccgatcgaggtcaacaccacctccgagctcatcggcatcggtgtggcgtttgtggtcttgctcgtcaccttcggctcgctggtcgcgtccaccatgccgatcatcaccgccgtggtcggcgtggccatcggcgcgctggccgttctgaccaccacccactgggtcgaacttaacgacgtcaccccgatcctcgcggtgatgatcgggctcgccgtcggcatcgactacgccctgtttatcctgtcgcgctaccgccaggagcgccgcacgcgccccggccccgacgctgccggcatggccgtcggcaccgccggctcctccgtcgtcttcgccggcacaaccgtgttcgtggcgttgatcgcgctcgttctcgcccgcatcgagttcctgtcctggatgggcatcgccgccgccgcgactgtgctggttgccgtgctcgtggcgctgaccatgctgccggcgctgcttggcgcgtggggcgacaaggcgttcgccggccgcatcccgggagtcgccggccaccggggtccgggcaaccggcccgcgaaggacttagacgcgcgctccacgggccgcacgtgggtgaatttcgtgcgccgcttccccgcgctcgtgatggcggtcgtggtgctcggcctcggggccttgagctacccggtgctcaacctcgagatggcgctgccgtccgacaccaccagcaacaaggacacgacccagcgcaaggccgcggatttgctcgctgagggcttcggccccggcatcaacgccccgctgctcgtgattgttgacgcccacgcggtcaaccccgacgccgaggcgctcgccccctacatggcagcgatccccgattccgcaggcggccgcgcagagaaggcggcgctcgcttccttcctctacaccgtcggccaggtcggctccgtcacgggcatcgagcacgcgcagctggtaggggtcaacgacgacctgaccgccgcccagatcctcgccacccccgacggcggcccggacgagcagcgcacgctgaacgtcgcgcacggcctgcgcgagaacaacacccaggtcgaggacaccaccggcgtcaccatcgggctcactgggctgaccgccgtccagatggacatcaccgaggagcttgccggagccatgccgctctacctcgcgatcgtggtgggacttgccatcatcctcctcatgatcgtcttccgctcaatcatggtgccgctggtggcgggcctcggcttcctgctctcagtcggcgccgcgttcggcgtcactatcttggtttggcaagacggcctctgggacttggtcaacacgcccgccccggtcctttccttcctccccatcttcatgatcggggtgaccttcggcctggccatggattaccaggtctttttggtgacccgcatgcgcgaacacttcctcaaaaccggcgacctcgaagagtcgaccgtcgaaggcttcacccaaggcgcgcgcgtggtcacggcggccgcgatcatcatgatcgccgtcttcatcgcttttattaaccagcccctgccgtttatccagatcttcggcttcgccctcggcgtggcggtgtttttcgacgcgttcttcgtccgcatggcgctggtgccggcgacgatgttccttctgggccgcgcgacgtggtggatgccgaagtggctggataccatcctcccagaggttgacgtggagggcacccaattggaggaagcacgatgaccgaattcgacatcacccgcgagctgtacaacgagcctggcaagcacgcccgcacgggcgtcatccacaccccccacggcgacattcaaacgcccgcgtttatccccgtcgccacgaaggcgacggtgaaaacgctcacgccagagcagattcgacaaactggcgcgcaggccatcttgtccaacgcgtaccacctctacctgcaacccggtcccggcatcgtggacgaggccggcggcgtggccgccttcgagaactggcacggccccacctacaccgactccggtggttttcaggtgatgagcttgggcgtcggcttcaaaaaggtgctcgcgatggacaccgcggggcttaccgacagcgacatccgcgccgccaacaaagaccgcatggcgcgggttgacgacgacggcgtggacttcaagtccgtcatcgacggctccgcccaccgcttcacaccagaggtgtcgatgcagatccagcaccagctcggcgccgacatcatgttcgctttcgacgagttgaccacgctcgtggacacccgcgcgtaccaagagcattccgtcgagcgcacccgccgctgggcgcgccgctgccttattgagcacgaccggctcaccgccgcgcgcccggataagccgctgcagtcgctgtggggcgtcgtccagggcgcccagtacgaggacttgcgccgccgcgccacccaaggcctgctcgacctcgaccgcgaagcccgcggcgagggccgccgcggcttcggcggcttcggcatcggcggcgcgctggagaaagagaacctcggtgcgattgtcggctgggtcaccgacgagctaccggccgacaagccccgccacctgctcggcatctccgagcccgacgacatcttcactgctgtcgaagccggcgccgacacgtttgactgcgtcgctccgacgcgcctcggccgccgcggcggcgtgtacaccctcgacggccgcatgaacctcgccgccgcccgcttcaagcgggactttaaaggcgtcgacgaggaattcggcggctacgtcagcgagaactactcccgcgcctacatccaccacctgctcaaagctaaggagtacctcgcaggaaccctgtgcacgatgcacaacctcgagttcatgatccggctggtggacaacatccgcgcggccatcgacgccggcgactacgaggcctaccgcgacgagttcctcggccgctactacgcgtcctaggccgccgcggcctgctcttccttgcggcgcacccacgcgatcgtcgggtaggtgatcggcagcaggatgacctccatgagcgtcttccacaagaagccgaccaccacgtagttcacgaactcgcccgcggtggcgatgccgatcacgcccgcggcaatcgagcagaacaacagcgtgtcagcgaactcgccgaccactgtcgagccgataaggcgcgcccacagccggtccgtgccgaagcggtccttcatcttctgcagcacccacgcgttcagcagctggcccaccacgtagccggccagcgaggcaagcacgatgcgcggcagcagccccagcaccgcggcgaaggtgtcttgcatgtcgtagaaatcggccgccggcagcgcgatggcgatgtagaacgacgcgatcgcgagcagcgcgatgccgaagccggtgaagacggcgcgcctagcggtgttgaagccgtagacctcggcgatcacgtcgccgataacgtaggagagggggaaaaggaaaaacgcaccgtcggtaagcagcggccccaacgcgacacctttctgtgccgtgatgttggagatgagaaacaccgagcagaacacggcgagcaggtacgggtacggggagcgggaaacgcggggcgacatgcgttttatcatggcacacatggctgattctgcagggcgctacgcaccgagtcccagcggggacctccacttcggcaacctccgcacggcgcttctggcctggtgtttcgcgcgccagagcgggcggcagttctaccttcgcgtggaggacatcgattcggagcgctccagcgcggagtcggcggcgcgccagctcgaggatctcgccgcgatcggcatcgagtgggacgagccggtgatctaccagcacgaacgcttcgacgcctacgccgcagcgctcgcccgcctcgacacctacgagtgctactgcacccgccgcgatatccgcgaggccgcgagcgcgccccacgcccagccaggcatgtacccaggcacgtgcaggaatctcacggaggagcatcgtgctttacgacgctcccacctccaatccgaaggccgcctccccgccatccgcctgcgctcggcagcgggcgagtggagcgtgcgcgatttctaccgcggcgactacacggggcccgtcgacgacgtaatcctgcgccgcggggggcgtgtggaccaggcgcaggcgggcgactgggcgtacaacctggcggtggtggtcgacgacggcgaccagggtgtcgaccaggtagtccgcggcgacgacctgctcgcctcggcgcctgcgcaagcgtacctcgcgcaccttttgggctacgccgagccggagtacgtgcacgtgccgctggtggtcaacgcggaaggcaagcgcttggccaagcgcgacggggcggtgacgctgcgggagatggcggcgtccgatggcgcggacgcggtgaaggaagcgctggcgcggtccatcggcgcggacccgggtgacgtgctcggcacgttcgacgctgctgcgctgtcgcgcgaaccgtgggtgtgggcgccgaaagtctaagccgtgaagccgacgtccttgcgccaggtcagctcgacggccgggcgcacgggggagagcggagcgaggatgttgtccacccgcatccactccgcgacgacctcgtcgggggagatggtgaccacgctgtagccgtgcgtgtccaaggcgacgtggcgcaggctcgggttggcggcgtggaggtagctgcgcgcgacacggaagagtgggtggcccacctgcaccttcaacgagtcggcgacgttcggcgcggtgaccgaggagcacacgacctcgcagccgatggggcggccgtcgaaaagcacgttgtgcgcccactcggagtggatgtcgccggtgaggaagatcgggttcttacccaagcggccgagttcaccgatgaggcggcgtcgctcgaagtcgtagccgtcccactggtcgccgttgagcggcacctcctccacgccgggcagctgcgcgttggaggagaggatattcgacgacagcgccttcgccaccggcctcgtcgccgggttctgcatcaccgcgccgaggcgcatgggggagaacatcaccgagtttcccagggcgttccatttcgcgtgtgagcgcccgatggtgtcgatgagccaggtgtactgctcgccgccgagcatggtgcgcgcgtcgcccggttggcgcgagccgcccttccagaactcgacgtcgcggtaggtgcgcaggtccatgatggtgagttcgaccaagtcgccgaagctgaacgagcggtagatccgaccctgcgccgacaactgcgctgctcgcaccggcatccactcgtagtacgcctgaacggcggcgtcgcggcgcgcgaagaagtcgccctcgtgcgcgtggtggttgccggcgccctcgcgccacgtgttgttggctacctcgtggtcgtcccacaccacgatccacggcatcgacgcgtgcgcgttctgcagcgctgggtcggtgcggtagcggccgtagcgggtgcggtaatcggcgagtgagacgatctcgtgcgcaggggcgtgcaggcgcaccggcccgtagccggagtactcgtactgcgcgtactcgtagatgtagtcgccgaggaagacggtgaggtctatatcgcccgaccacccgcgctccgccagatccgcgtaggcggcgaagaagcccgcttcccagttcgcgcaggacgccaccgcccagcgctgccggtccacgcgccacccgaacccaggcgccgtcttcgtgcgccccaccggcgacaccgcgcccgcgtgcggcccgtcaactacgacgaagcggtagaagtacaccgtccccgcggccaagtcgcgcacgtccaccttcaccgtgtggtcggaatccgggtgtgtcgtcacctcgcccgactgcaccacctgcgtgaactcgatgtcgctggctagctcccaccgcacgtatgtaggagcgccttggccggagccgggccacgccgcgtcgtcgggcgtcacgcgcgtccacagcaccaccgcgtccggcagcgggtcgccggaggcgacgccgtgcacgaacggcaggggagcgagctccatctcggccagcggcgcccgggagggggccggctgggagctctgcgcccacgcctgggtggtcacgcccgccccgacggcgcccactgctgcggagcgtcggaagaaagttcggcgggttacgcgtgtcacgccagcaatagtgcggtaccccgcgcgggccagccagccggggaagcggagtttgctgaggtttcgccccgaatttaacccgcgtttacctcttaggagagggtggtgcgggtggccaacgcggcgtcgatacgcaacagccccgagccgtcaccgccgactagctcgagctggtcgacgatctcgcccacggtggcctcttcctcgatctgctccgtcaagaaccagttcagcagcccgcgggattccagatcgcccgcctcgtccgcgatgcgggtgatgttgcgaatctgctccgagaccttcttctcgtgagcgagcgccgcgcggaaggcgtcgagggggccgttcacctgcggcgcgtcgatgcggatgtcgcgcggctgcacgcgctcaccgcggtcgatcaggtgcttggcaaacttctgcgcgtgctccgtttcctcctgcgcctgggcggcgaaccagttgctcaggccggggaaggacaacgcgtccatctcgttcgccaggaagcggtagacgtacgccgccgcgtactcctcggtcacctgctgggtcattgcttctttgagcttttcatcaaccatgcggcaatgatacggcgaaaccggcacccgataacgagtgccggttcgctaaaaaacttggcggaggatgtgggatttgaacccacgagggtcgtgaaacccgcacgcgttccaggcgtgtgacataggccgctagtcgaatcctccattcagcgacaccaaaagcgtctccgcatactgtagtgcacacccacccgcgcaccaaaaccgcagctggcggcggtgggttgtgtcctagtgaagcgtcccgctacagtgaagggcaggatcccacgcggtgttaccttgtgaactcccccagggcgggaacgcagcaagggtaagcgagctctggcaggtgcgtggggtcccctttctttgcgctgtagaattcgtgcctatgaacttggatgagcacgagattgaaaccctgtcggctgaggtccgcgagaagtacgagactctcaaagcgcgcgggctgaacctcgacctgacgcgcggcaaaccgtcgagcgagcagctcgacctgtcgaacgggctgctggcgctccccggcgccggcgactacaccgacgccgccggcgcagacgtgcgcaactacggcaacctgcagggcatcgaggacatccgcgcgctgtgggctgaggtgctggggatcgacgcggcgaaccttatcgcaggcgattcctcctcgctgaacatcatgttcgacttgatctcgttcgcctacatcttcggcacgaacgactcgccgcgcccctggaaggacgaggagcaggtcaagtggctgtgccccgtcccgggctacgaccgccacttcgccatcacggagcatttcggcttcgagatgatccaggtgccgatgaccccgaccgggcccgacatggacgcggttgaagaactggtgcgcgacccgcaggtcaagggcatgtggacggtgccgatctacggcaacccgaccggtatcacctactcgcgcgagacggttgagcgcctcgccgcgatggacgcggccgccccggacttccgcatcgtgtgggacaacgcgtacgccatccacacactcaccggcacgttcccggagaacccggacgtcatcgagatcgctaagcagaagggcaacccgaaccgcttctggtacatgtcgtcgacgtccaagatcaccctcgcaggctccggcgtggcgttcttcgcctcctcgaaggcgaacctcgactggtatgccgagcacgcctccatccgcggcatcgggccgaacaaggtcaaccagcttgcgcatgtgaggttctttgggggtaaggagggcgtcgataagcacatgctccaacacgctgcctccctggcccccaagttcgaagcggtggcgagcatcctggagcagcgcctcggcggcctcggcatcgccgagtggaccgaacccgagggcggctatttcatctcgctggatgtcaccggcgggtccgcgacgcgcgtgtgggagctggcgaaggacgccggcatcaccctcaccaaagccggttccgcgttcccgcgcggcgtcgacgagcacgaccagaacatccggcttgcgccgtcgctgccgccgctggacgaggtgaaaaccgcgatggacggggtggccacctgcgtgctgctcgcgtgtctcgaggcgatgggcaagtaagtaggcttaagcggcgtggctctgtacaggaaataccgcccagcaacgttcggtgaggtcatcggccaggagcaggtgacccgcccgctttcaaccgccctcgataacgggcgcattgcccacgcgtatctgttctccggcccgcgcggctgcggtaagacgtcctcggcccgcatcttggcgcgctccctgaactgcgcccagggcccgacgtccaccccgtgcggcgtgtgcaactcgtgtgtggcgctggcccctggcgggcccggcaacttagacgtgatggagctcgacgccgcgtcgcacggcggcgtggacgacatgcgcgacctgcgcgagcgcgccatgttcgcgcccgctgagtcgcgctaccgcgtgttcatcatcgacgaggcgcacatggtctcgcgcgagggcaacaacgcgctgctgaagattgtggaggagccgccggagcacctgatcttcatcttcgccaccaccgagccggagaagatgctgccgacgatccgctcccgcacgcacaactacccgttccgcctgctcgcgcccgcggcgatgcgggagcttttagagcacgtcgtcgccgaggagggcgtgacggtggacgagaacgtctacccgctggtgatccgcgccggcggcggctcgccgcgcgacaccctgtcgatcctggaccagttgctcgcgggcgcagggcccgacggtctgacgtacgatctggcgctcccgctgctcggggttacggatctcacgcttatcgacgcagccgtcgacgccctcgccgcccacgatgcgtccgccatgttccgcaccatcgacgcggtcatggagtccggccacgagccgcgccgtttcgcccttgacttgctcgaccggttgcgcgacttgctgctggtgcgcaccgttccggacgcgtttgggcaggcgcttgtcgacgcccccaccgaccgcgccgacgtcctccaacaggaagccgagcagttttctgccgcgcagctggccacccttgcttcggagatcaactcgcgcatctccgatctgcgcggtgcgacgtcgccgcggctgctgctggaggtaatgatggcgcacctgttgacgctgccggccgaccagccgcgcgccgcggccgcgccttcacccgccgcgccgagcgtgccggcggctgcgcctgccgcgccgagcagttcaggcgggcagggcggggctgccgcggcggcggccgctgcggctgccgccgcgacgcgcaacgtgcgcagcacctccactccggcgccccaggaggcacccgcgcccgcgccaaagcctgagcctgagcccgcggaagccggcgaggagctgttcgaccgcgtcaagcgggattggacttcgctccgccagtccgtgggcagccgaaacaaagtcgcggagatcatgctcaccgaggcgcgcccgctcggtttcgaagacggcacgcttgtcatcggccacaacacaggcgcgctcgcggagcgcctcaacgcggagagcaataacgccgacatcgtcgccgtgttctcggagaagctggggacccaagtgccggtgcggtgcgtggtgggcactcagatggttgtggcgaaggtgcggagcactgaacgggagccgaacgacgacgccgaggatccagcccctgccccgaaggactggcgcgccgccgcggcagccgcgagccagcaggccgcggcgaaggcgaagcgggagcgcgatgagatcccgccgccacccgagccggtagaggaggagccgccgtacgacccgtgggagggcgagccgcagccggcgccgtacacccaagaggacgaagagcgcgacatggcggaccaggcgcaaggcgaggcgggctcgcccgaccgccgcgacgcaacggaggtcgccatggagctgctcgccaccgagctgggggcgcggccgctgtagtgcggcgggggtacaatagtcggcggactttattagcgatgaaagaaagggtgtcccacaccatgacccagccgaacatgccagcagatatgcaggaactcatccgccaggccgccgaggtgcaggcggcgctgcagaaggcgcaggaggagctcctcgccgcggaggtcgagggtaccgctggcggcggccttgtcaccattacgatgaccggcggcgccgagatcaccgacctgaagattaagccggaagcggtcgacgctgacgacgttgagacgctgcaggacctgattctggccgcgtaccgcgacgcgcacaacaaggctggccagcttgcgcaggacaagattggcccgctgaccaacatcggcggcgacgcggcgccgcagcagggcggcccgttcggcggccagccggcaggcccgggcgagatcccgttcggcggcatcatctaagcgctgccctaccacccgcgcctggcttcggccgggcgttcttttttagcaaggagtgtccatgttcgagggcccgctgcaggacctgatcgatgaattctcccgcctgcccggcgtcgggccgaagtcggcgcagcgcatcgcgttccacctgctgaaaaccgagccggaggacattgaccggctgcgcgcggcgctggcggcggtgcgcgacggggtgatgttctgccgcatctgcaacaacgtctcgcgcgacgaggtgtgccgcatctgcgccgattcggggcgcgacaaggcgctggtctgcgtggtggaggacgcgaaagacatccaggtcatcgagcgcacgggcgagtacaccggccgctaccacgtgctcggcgggtcgctcgatccgctggccaacatcgggccgaaggatctggctatcgcgccgcttctgcagcgcattggcggggtgcagaaggatcttgacgacgcccccgcccccaccatcagcgaagtcatcctggcaaccgacccagataccgagggcgaagcgaccgcgagctacatcgcccgcctgctgaaggacttccccgacctcacggtgtcgcgcctagcctcgggcatgccgctcggcggcgacttggagttcgtcgacgagctcaccttgtcgcgcgcgctcaccggccgactgcggctctagccttcgaggtcctcggctgcttcgtcgacggcgtcctcgataaggaagtcgaggtcgttcaggaacgcggtgacgctgacctgggaggagtcgatgcctttgatgcgcagcggcccaagggtgatgaagtcgatccacttgtcctcgacgggtgcgagcgagagatcctcaatcgccgtgatgaagttgtcgcggtagtagcccaaaagctggcggtgcgcctcggtgcccaaatcgttccacggcgcgccgacagagatccagtccatgccgacgcagtcgatgtcggtgcgggttgccagccactcgcacagctcggggtcgaggcacgggccttgggcacggtagacctcggggttctcggtgcggtagcgctcgaagccggtgcggatgagcagcaggcggatgccgtcgaactcgtcggcgtagggctcgatgtcttcgactttcaccacggattggggttgggatttggtggggacgtcgataagcaaaatctcatcgccgtcgaagttgaagcgctcggggccgagctcagcgagcgtcgtgccgccctcgacgaagtgggcgggcgcgtccatgtgggtgccgaagtggttgggcaggtgcgagatgaagtcgttgctcgcgccgtcctcgccgagcaccgcattgtgctcggtgacaagttccggcgagccggggtaggaggggccttgcgggtcgatgatgtggctcaagtgcacgtacatgcgccccagcgtagccaaaaacgcgtctagctcagccgctccgcgcgcagccggtcgatgaccgggatatccagcggctccagctcgtccaggcccacgccgagcgcctgcgccaaaagcaggtccgccagctgggggttgcgcgccagcgccgggccgtgcatgtaagtcgcgatcacgctgccctgcaccacgccctcgaccgccccgcccgcgccgttgccgacgccgcgcgtgaccttgcccaatgcagaggcatccgggcccaaggtggtcgcgccgatgtggttttcgaagccggtcagcggctccgtcagcgcggctgtcacgccggctcgggtgggttcggcggcgacttcccctatggcgcgggttggaaggggggcggtggagacgtcgataagcgaaatgccctctgcctccgtgccgtgggcgtggaacgcgcggccgaggatttgcatgccggcgcacacggcgaagatcggcgtgcccgacgcggcagccgcctgcaagccgggggaggcggcgaggcgcgcggcggcgattacctgcgaggagtcttcgccgccgccgatggtgtagaggtcgcagtcggcggggatgtcgtcggtaagcaggatgcgccggacgttcgcgtcgatgccgcgcatccgcgcccgctgccgaagcaccagcgcgttgccgtcgtcgccgtaggtgcccagcacgtccggcagaacgagtccgatggtgagcttacgcacggtaatcctcctgcttggtcagcgcttttcgcaggttgagcagcgcggtgtagttcgccagcacctccacgcgccccggcgggcaggcgcggatcgcctcaaccgggtcgtgcaccagttcgtggtcgatgccggcgtagagcaggcgcacggcgaggtcggttgcgcgctcgccggcggcgacgacgtgggtgtcgccgaagtcctcgaacgcgacgtcccacagccaggagacgtcctcgccgtcgccttgtttggcgttgaccgcaatcaccacgccgtccgcgtcgcggtcgagcatggtcagcgcttcctgccaaccggcggggttcttcgccagcagaaggtgcacgtcgcgctcgccgaggtggacggtggtgtagcgcccggcgacgttgtcgacgtcctccgccgcgcgaatcgccctttccagcggcacgtcgaaggcctcgacggcggcggcgatggcttgggccgcgttgccgcggttcgcccgcccaggcagcttgaggtccagcgggtggtcgcccgagggggtgcttatcgacgccccctccaacccccaagtcggccgcggacggcggaactcgcgaccgtcggcaagcggctcaaccgcgtaccagtcgccgtcgtccgtgcgcaccacgtggccgccggagcgggggttggtcaccgagtcgccgagccagccggcgcccgccgcgacccacaccacgttcgggtggtcgtaggcgatggaggtgatcagcacgtcgtcgcagttggcgatgacagtggcgtccgggtgcgcttcgacggcggcgcgcagcgcgcgctcgatcttgttgatctcgccgacgcggtcgagctggtcgcgcgtaaggttcagcagcacgaaggcctcggggttcaggcgttcagcgacgtgcggcacgtgcagctcgtcgacctcgagcacgatatgcgacgccgcgcgccccgccatcagcgccgagatgatgccagcgtccatgttgtcgccgccgtcgttggtggccacgctgtaggtgctgcgcagcgcgccggcgagcatgcgggtggtggtggacttgccgttggtgccggtgaccagcactgcggggcggccgcccgcgagggtggccataatgttcgggtcgatcgccccagccacaaggccgccgatcatgccgcccgcgccgcggccggtggcgcgggaggcggcggtggctgcgcgcgcggcggcgatcgcggcggtggaccttatgcgggcgaagcgagactgctcactcatgggtgacaggttactccgccgcgtcggcggaacccgcgctcatcttctccacagcggcttcgaattcgctgggggtgaggatggggatgtctttgcggtgggcgtgcatcgccttgccccgcagttcggcgcccttcgcggccgcctcggagacgacgagggaggactggcgcgtgagcttctccgagtagcgcagccccgcgcgcacgccgaggtcgatcaccgtgtcggggtcgacggtgaggtcgtcggtgacgacaagttccatgcctttttccagcccgcgggccgggtcgtagacgcccgcaagcggtgaggcggcggcggtgtcgcgctcgccggccttcgccgcgtcgacgcgcagcgcgctgcgctgcaggccgaagcggtcggcggcaagcgcagccgggtcgtgcgtgaccagatcgccagcctctttcagcgcgaggtacatcgacaccagcgtcagggtgtcgtcgcggcccgtctcgttctgcccgacctcgaccccgatgaggtcggcgacggcgtgcaggcgcgcgtcgacgggtacgtgaccctggcggcgcacagttgccagcacgtcgacgattccctccgggcgcggcacgtgccccacacgctggcggcggcggttgccgcgcccgcggcgggagcggttcgcgcgggctgccgcgttcatcgcgcgcttcgcctcggaaacgatgaagccccaggaagtgggggagtcgaagaggatgatgtggcgggcgtcgataagcctgtcaagctccttcaacgaccgtgagaagcgcggcgcctgggcgaagtcgctgacctcaagcccgtgggtgtggcgcgggccggcgtccatcccggggttgaacacctggtggaactcctcgccgacgcggcctgcgtcatcgaaggtcaccgcgtcgatcgtgagcagccgggcagtggtggggtgaatcccgttcgcccgcgctgtcagcgcgacgtaggggaattcactctgctcggtcattcgtcgaagcgtactacacgccgccggtcttaccctcggtcagcgcgcggttcgcggccgagacgatggccttgagcgaggcgcgcgtggtggagccagcgatgccaacgccccacgcggttgcgccgtcgacgtcggcgtagatgtagcaagccgcgtccgcgtcgtcgcccgcggtgcgggcgcgctgcgagtagtcctgcacctcgaagtcgatgccgaggctctccaacgcgttggcgaacgccgcgatcgggccgttgccggtgccgctgatctcgcgctgatcgcccttccacaccacggaggcgcgaacagcggaatcgtcctcgtcgctggccgcgccggtgatctcgtaatccaccagctccagcggggagtccaggtcgaggtagtgggtggcgaagatatcccacatgttcttggagttgacctcgccgccctcgcggtccgtgatcgcctggaccaccgcggagaactcaggctgcatcgccttcggcatgttgatgccgtggtcggtcttcatgatgtaggccacgccgcccttgccggactgtgagttcacgcggatcaccgcctcgtaggtgcggccgacgtccttcgggtcgatcggcaggtacggcacctcccaggtggtgtcgcgcagctcttcccacgacacgtcggtggaggaggcgtcggggcgcaccttctgcgccagcgcgtcgaggcccttgttgattgcgtcctggtgcgagccggagaacgccgtgaacaccaggtcgccgccgtaggggtggcgctccggcacgcgcagctggttgcagtactccaccgtctggcggatcttggcaatgtcggagaagtcgatctgcgggtccacgccctgcgtcatcatgttcagcgccagcgtgaccaggtcgacgttgccggtgcgctcgccgttgccgaagaggcagccctcgatgcggtcggcgcccgccatgtagcccagctcggcggcggccacgccggtgccgcggtcgttgtgcgggtgcagcgagatgatcacgctgtcgcgcttggccaggttgcggtgcatccactcgatcgagtcggcgtagacgttcggcgtgatcatctccaccgtggacggcaggttcaggatgatcgggttgtccggggttgcgcccatcgtgtcgacgaccgcgtcgcacacctcgagcgcgaagtccagctcggtgccggtgaaggactccggcgagtactcccagcgccagttggtgtccgggtagtcgtcggcgatggagaggatcagctcgccggcgtcggtggccagcttcttaatcgcgtcgcggtccttgcggaacaccacgtcgcgctgcagcttcgaggtggagttgtagaagtggacgatgacgtttttcgcgccagagcacgcctcgaacgtgcggcggatcaggtgctcgcgagcctgcaccagcacctggatggtgacgtcgtccgggatcatgtccttctcaatgatctcgcgcacgaagtcgaagtcagtctgggaggcggacgggaagcccacctcgatctccttgaagcccatctccaccagcaagttgaacatgcggcgcttgcgctccgggctcattgggtcaatcagcgcctggttgccgtcgcgcaggtccacggcgcaccactgcggcgcgcgggtgattttcttgtccggccacgtgcggtccggcagggtgatgtcctgaacctcttcggcgaagggcaggtagcggtcgaccggcatctggctgccgcgctgcttgttccagctgggctggccttcgttgcgcgggccgttgggggtcacgatatcgcggggggcaaaaaagtcgttagtgtgcgtcacggtggggctccttgtatctcggcttggattgtatccacggccggcaagcaaaaactccgcgacggggtgccggccgtgttagtgggcctgattcccgccgcggcgtagaaggagtagcgccttttgcgacatgtgacgcagcctacacaatcctggcgcgccaaggggcgctattcggaaaagttcttacttaccgaacagcgtccgcatcgcgccaaacgggtgataggggttggcaaccgggtacccgcgcggcgacacccacgtgggatcgccgtccaccacctcgatccgcccgcgtcttcgcacccagtcatcgtcgtcgttgacgcggttgtggtagcggcacagcatggtcagattccgcatgttcgtcggcccgccgtgtttccacgcctgaatgtggtggacctggcacaggtcggcggcgcggtggcagcccggcaccgggcacacgggtgtggtggcgcgggccaggtcgcgctgtttctgattggcgaagcgctccacccggtacaggttgaccggcccttcaacagggtggaagatcgcggcctcgaggccaacgccggcgtcggaaaaatactcagacaggaattcggcgccggtgatggtggtgccgtttgtaagcccgaagcgcacctcgttcgcatcgcactcgccggcaacaagcgtcgacagcgccggcgccggcaccaacagaagcgggtgcggcacggcgcgagccacgccgcctgagcgaatcacctgcttgaagttcttgtacatctgcggccccgccggccgcgacgcgtccaacccctgcgagcacctaaatgtcaggtccgcggcttctttctcttctgcgaagatcatgattttgcacatgcccctcactgaaggcccgactgtcatcgtcggctccagctctttcggctccgcgggcaccagcttggccaccatacgcgcgaaggcctggtagtcgcccggccgcgacgccgccaccgcctccagcacgtcgaggcgcttccgtccgcgctcgcgggccggcaccgacgacagcttccgctcgatcagcgccagctggtgcagagacaaccgagaccggcgcaccaaaccgcgcgcccgcgcctgctgctggtgggcgtgggtttccgcaaggtacaccgcgtgcagccccgcccacgagcgcacggtgttcggatccagccccgcgtccagcgccgcctgctcgtcgaaaccggccagcgtgtccagcgcggagccggacatggcctgaagcagcgcggcaaacgtcatggcccacacgttatcggcgcgctgagtaaggcgacaccccgcgcgtgcacactatcgtgggcgcgtgagctgcacggttgcaaggagcatgatgcttatcgacgcccccatcaaccccattc

SEQ ID NO: 20 - DNA, 14944 bp, Corynebacterium cassirii
  source 1..14944: mol_type = genomic DNA
cccctctcccggccacaccctcctcccgtccacccccggcgccctgttagccccaggggttgtggctacgtagccggtgcgggctcagttgcctcagcctttcgggaacgggcctggctcacagcgtgcgacgaggtcgcttcctcgtagccgcaggtgcgcagcacgccgtcgccgatgagcaggccggcggcgacgagcaccagcgagccaccggcgagtgccagcgtttgcgggttgacaatcgccagcgcttggttgatccccgccgccgcctcggcgcgctccttgtcgtaaatgcccagaccttcctgcagcttggcgttcacgttctggatcgcggcgttgatctgcgcatgcacgtgctcgagacccgggatcttcacctgggtgaggatgcccagcgggatgagcaggagcagcggcgcggtcaacccggccagcgccgcgatgcacttgccgtccacctcgcgcggcgcctccggttcgactggtgtaggcgggtcaacaggcgccggcttttcgatcggcgtggcagggaccagcggcactgccgggatgacggtgacctcagtaactgtggtgctttcgacctccagcttgatcgagatgatgttggtgatggtcgtgccatcgccgctcgtccacgcgagtttgatgtccccggacaccggagacccgtcgttgcggatgatggtccaggtgttgtcggggttggggcgggtggagtgggagggggcgtcggtaagcacaatcagctctcccccgctgcctgggacggtgaccgtaatggagccgtccgagttcgggtgcgtgaggcggatcgtcgcggcttccgtgaccttaacgacgtagcgggcgatgagctgaccgtgctcgttgcgcacctcgatctcggcctcaccggtagcacccgggcgcggcgtgataatcagcgtgtcgccctcgcggccgacggtgatgatgtcgccgccgcgcactacggtgtgcgtgccagcgccgatgcgcaggcgatgcgtcgcgttgttggggatggtgacggtgtgcgtcggcaccgcggccggggtgatggtgacgacgtagcgggtgtccgtccggccgcggttgtcgagcgattcaacgatgacctggccctgcgccccgtcgcgcgggacgaaggtgaaagagtcgatgagtttctgctcgtccacgtgctcggcgccggagacgatagtgaggttcgtgcccgtcagctggagcgtgtccaaactcgtgatgttgtgcgtgaccacatcgatcggcaccggggtaatggtcagcgtcgtgcggacgatgacgttgccgcgggcgtccttctcctcgatgaccacgttgccgtccgcaccctgcttcgggtcgaggatgattgcgccctccgcgtcgctgttctcgtcgacgagattgtcacctgagacgagggtgagcgtgttcgactggtcgcggcgcgtaacgcggaactgcgtgcggtcggtgatgtcgattgagaccagcttcgtcttgactacgggaacagtcgactcgactttgaacgtgtagcggaaagttggccggttcttgccatccagaatctcaacgacagcgttaccgtttgccccgtcgatcgcctgcacgttcaactcgccgccgttgcgcgacaccgttacgacgtcgcttcctgagacaaggcggtgggtggcatcggcgggaaggtcaagggtgtaatccccgccgtcataaaggttgaaggtaactacgcggacctgcggggtcgtatccaccacggtgatgctgaaccggtgctcgttacccgtcttgtcggtgatcagaaccgtggctttcccgctgaccccgtgcttcgcggtcaccagcaactgtccgttcttctcctctacggtgacgaggtcgtcgccgctctgtagcctccacgtggtgccggggttgcgcagagtcgggtcgtcgatggtgaactggtcgccggattcgagcgtcgctagggaaaccttggtcgccgggcggatgacgatggagatcgtgtgacgcaccgtgttgccgcgggcgtccttgatctccacggtgaactgcttgccgttggagtctggcttcggagtgatgagtagctggtcgccgtcgacacgcgtatcgacgttcccgccaccagaggtgatgccccaatttccgcctgcggggatagtgaacacaccggtgccgggctcgccgttgaacgtccaggtgttcgaggtggtgtgggtcttcggggtagcgtcacctgcggaaagagtcggcgcggtgttgtccaccgtgatcttgtactcgtggtcgcgcccgttcgcgtctgtaatcacaacgatgacgtcgcccttcgcgcccggcttgggggtgatgaggagaccttgggcgtctttggtcacgctgacgagcgaagccccctgcgttacccggtaggtccactcgcccttcgtggcgacggggagtgttttggacggctcgttgtggttgtagacgaaaatgtactcaaaatcgaagtttgctgacgtggtggttgttgtggtcgttgacgtggtgtgaacgttcggctgggcgatggccgtgacggtgcttgtgcatactgcaccggcaacggcgagagcaatgacttgcttttttaggtttgggcgacgcattcctgtgctcctgtggagaagtgtgagggagttcagcgtttgcttaagacacgctgccgagacgaaagcctaaacacagttgacgttcagcgcgctttaagcattgttgggcaaatcatcaaaacctgggattgtatagctaggagcaggtagctcgcggtcagcgcgagtaacattgcaggaaacatgtatctacaagagtgttttgtctactcaagtgggcgcctatacaccacacctttacgggggtagtggagcgacacgccgaaggtgaggatttttcttacaatgtccacaatcgtgagcggaatgatgcggattgcgcacaagagcgacgcggaaatccgggaactgtatgctgcggcccgcagcgccggagtgaccgtgttcgaccatgcggatatttatggcggggggcatgaatgtgagcgtcgatatgcgcaagctctggcactgagccctgctgagcgtgccgagatcaccctgcagactaagactgggatctcactcgatccggcgatgtacgaccactcgtacgtgcacatcgtgcgcgaagtggaggaatcgctgcgtgcgctgcggacggattacctggacgtgttgctgctgcatcggccggatgcgctggtggaaccggaggaggtggctcgcgcgttcgacgagctggaggcgtccgggaaggtgcgcgcgttcggagtatccaatcacacacccatgcaaattgagctgctgaagacgacggtgcgtcagccgctcaccgtgaaccaggtgcagttctcgctcgcgcatgcggaccttgtggcggagggcataaccgccaacgcggcgggaccggcgttcaccggggtggtggatcacgcgaggttgacggggatgacgctgcaggcgtggtcgccgctgaccggtagccgcggcagcgtcttgaacgcccaggcctacccggagctcaacgccgagctcgagcgcttggccagcgagtatggggtctcgcccacggcgatcgccgtcagttggattacgcgccacccggccggcttccaggtcgtgctggggagcaccaacccatcgcgcttcacggccgccgctgccggtgcggacatctgcttgacccgtgagcactggtaccggctctaccgcgccgctggctatcccctgccctagcggcgtgcgagctttcgggcgcgtacgcgccaccgctccgggaggcgcctttgcggcggcgacgtggcaaacccgcgcatcatcgaataccacccacgggcgaagcgccttcggcgctgtgcgctccccttcagcgctcggccgtccatggacacttcgagccaggaaacgtagcggaccgtctcgtcggggcgaacggcaaaggacagctggatgtcgtcgtggacttgggtatccgccaggtctaggccgtcgcgcacacgctgccaccacgccgcgcgaaacgagcagttggtgccgaaaagtggcgggtgccccaaggccgagccgacgcttcggcggtatgcgcccaagtagacgccactgacccactgcggcatggtgtcaaagacggcgtgcccggcgacagcgaccgtgtcgtcggcggcgcaatgccacagcgcttcgatctgctgaaggtaatcaggcggtacaactgcgccggcatcggttcgcacgatgatgtcggcgccgagttcaactgccctatcgtagccggctgccgcggcccaggtaatcccgacgcggtgctcggtgaccacgtccgcgccgtacgcctttgcaatagcggctgagctgtcggttgaggcgttgtcgacggtgatgagggcgtcggcaagccgtgcctgtgccttgaagctttctaagcagcgaccgagaagctcggcgccgttgcggcatgggatcaccaccgcgatggttgggacgagcaaacggttgggcatcggcggattaatccatctgcagcacggtgcgtaactccgcgaagcgctccgggcgcaccctgtgggtgaccgttcgcccggcgcgggtcttctccagcagcccggcctcgaccagcttcttcaggtggtgggacacggtgggctggctcaggcccgattgttgggtgagcccgctgacgctgatgggctcgcacccgtcctgcgcgatctgcgataacagctgcagccggcccggatcggacaggaccttgaacagcgctgcgtaccgctcggcctcctcgcacgagagcaatccggaacccaacgagcaacactgcgtgctgcgctccggtgacacggggatccccgttgccttgtccacctgcacgccccgcctcctagtattgacaggcatcaatgtatcccttagcgttcatatcgaaaaccatcgatgcgttcaaggtgtgatcgtgccacaacaaacccaaacccagcaacaaccatctggcctctccttcctcgatcggtacttgccggtctggatcatgctcgcgatggccgttggcctagcgctcggtcgcgcactaccgggtctgagcaaggcgcttgagtccatggaagtcggcgggatctcgcttcccatcgcccttgggttgctcatcatgatgtacccgccgctggcgaaagttcgctttgacaagacgaaggagatcgcgaccgataagcggctcatggcggtgtccatcgtgctgaactggctggttggccccgcgttcatgttcaccctcgcctgggtgttcctgccgaacgagccggaacttcgcaccggtttgatcatcgtcgggctcgcgcgctgcatcgcgatggtgctggtgtggtccgacctcgcgtgcgcggacagggaagcaaccgccgtgctggtggcgatcaactccgttttccagctggccatgtttggagtgctcggctggttttaccttgaggcgctgccgagcatgctgggtctgcccacaacgtctgcggacttctccttccgctcaattgctacgtcggtgctggtgttcctcggcatccccctgctggcgggcttggcctcgcgcatcattggggagaagaccaaggggcggacctggtacgaagcgcggttcttgcccgccatctccccgctagcgctgatcggcctgctgtacacaatcgtcctgctattttcgctccagggcgagcagatcacggcgcacccttggaccgtagccaccctcgccctgccgctgctgtgctacttcgtgggcatgttcgcaatcgccctcgtggtggcgaagcttgccggcatgggttacgcgcaggccgcctccgtcgcgttcaccgcagctggcaacaacttcgagttggctatcgcggttgccatcggaacgttcggcgcagcctccgccgaggcgctggccggcacaatcggcccactgattgagatcccggtgctcgttggtctggtgtatgtcatgaggtggatcggtcccaaactctttcccggtgacaaaacgttgcccagcaaccagcgctttgccaccaccccagcctagaaaggtcaatcagccttgcaatcgattccccaggtcctgttcgtgtgcgtccgcaacagcggaaagtcccagatggcggctgccctcgcccgcaagcacgcgcagggacaactcgaggtgttctccgccggaactcagcccggttcctcgctcaaccagttggcggtcgaggtgatcgctgaagcaggagccgacatgtcggctggcaaaccaaaggccatcgaccccgacatcctgcgcacagctgaccgcgtggtggtcattggcgaggaagcgcagttggagatgccggccgacgcggcaggcacgctcgagcgctggcttaccgacgagccgtccaaccgcggcatcgacggcgtcgaacggatgcgcctcgtccgagacgacatcgatgaccgagtgtgcgacctcgtcgctgaactgcagggataggcgcatgcaaaaggccggcccttaacaagagccggcgcacgctttccccgaacgcggtgagcttagatcaacttgccgatgatcttgaaaatggtggacaaaccaccctccttcaggatgcgcggggtgaacaggtccttcacgccggcggcggagtttatgatgccgtcggttacctcaagacccttctttgcgttgtccagacgctggctggtgatgtcgatctgggcgcgatcgcgctcgttgcgctcctgccacgaaagctccggtgcgttctcggtagtcaccgtcgttgcggtggcggtctcagcggcctgcgctggggtgccggcgaggatcattgcgcccgccaagacggatgccgctgctgcgttggtgaacttcttcatggtgtcctccttcaagtggtggtcggttggtgtggttccagacagtaagcccgccaccagctcagctcaaggaaaatcggcggttctgcacagacttggtacgaaggtatcttcgcaggtcaaaaggtgatttaccgctgcacgttgcgtggtctgcgtgaacccgcgagtgacgctctccgaggccatgcaagcctgctggaacccaagggcacgttcgtccatccgccggaacctccgtgccgaaatggcgctccttcttgagattctcactttgcatcagagcgcgaatcaaagtgtgcagaggcaatccagtgacaacgagaacgtccgtcagtggactaccgctcgtcaccacaccgcggggaggacatccacgatttcgcctatggcgagcacctacccgtttatcaacgactgccccaagctctccgtctaccaacagaacaccgtcacccactagagttgcggccaatcccgcactcttccccaacgcgcaaaacccgcagaccttgcgatctgcgggtttcatcttgtggagcataggagaatcgaactcctgacatcctgcttgcaaagcaggtgctctaccaactgagctaatgccccaacgttgagcacctcggggaggtactcggtgggcctagcaggaatcgaacctgcgacctcatcgttatcagcgatgcgctctaaccgactgagctataggccctgaaccgagatagaacattacccagcgacttagattgcaccaaatcgccaggtaagaggcctaaactcggttcgacatcgtgtaggttacaccgccgaccaagtcagcgatcgcgttgtaaatcaccgcaatcaggggggccataacggcggtgaagactacaccgatgagtccgagcagcgcggcgccggagagcacgagggtcatgtcgatcacctggtcaccgccgacaccgccgataagcgagttgacggagtccaccaccccggcgcgctcgaggccgtagtagatgatcgcggccgcgatcatccaggccacgaacccgaccagggagagcagggtggctaccttgaacaccgaaccgacaccaatgtgcttgacggcgactttgcgtgctgccatgggttactcctcgtcctcggactcgtcgtcagccggagcctcagcgtcgccggctccggaagcgtcggtgatgccggactcgatctcgtcgtcgtcctcccaacgctcgccggagacacccaactcagaaccctcgccgccggcgctcgaaccggtgtcgccggagtggctggaggatgcggtggcctcctgggcctcctccatcgtcttctggccggtcgccacggcggtggcttcctcttcgccctcgtcttcgacgttcttgtcgatggcgaggagctcgacaccgtcgttaagatcgaccaaccgcacacccatcgtcgcgcgcgaggacgggcggatctgggatacctcggtgcggatcacgccgccggcggaggtgatggcgaagatctggtcctcttcatctacggcgagtgcgccgacgagcttgccgcgcttcggggtgtacttgaacgtcatcacgcccatgccgccgcggccctgggtgttgtactcctcaatcggtgtgcgcttgccgtagccgccggtagtggccacgagcaggtactcgccgtccttcaccacggccatggacaaaagttggtcgtcgccgcggaagcgcatgcccttcacaccggcggtggcgcggcccatcgggcgcagctggtcgtcgtcggcggtgaagcggatggcctggccctgctcggagacgagcaggaggtcgtcgtcgcagccggcaagtgccgcgccgatcagggcgtcgccctcgttcaggttgatggcgatcagcccggcagagcgcgcggactcgtagtcggacaggtgggacttcttcacgcggccgtcgcgggtcgccagcaccaggtacggcgcgtcctcgtaggactgaatctggatgacctgcgcgatcttctcctccggctggaactccagcaggttggccacgtgctggccgcgcgcggtgcgcccggcctcggggagctcgtaggctttgagacggtacacccgtccaaagttggtgaagaacaaaatccagtcgtgcgtggagcagatgaagaagttcttcaccacgtcgtcctgcttcagctcggcgccgcggacgcccttgccaccgcgcttctggctcttgtaggagtcgaccttggtgcgcttggcgtagccggtggaggtaatggtgaccaccacgttctcacgggcgatcaggtcctcctcggtcacgtcgccggtggcggcgacgatgcgggtgcggcgctcgtcgccgtacttctcggcgatttccgcgagctcctcgcccacgatctggcgctggcgctccggcttggccaggatgtccttgtagtccgcgatctgcagctcgatctctttaaggtcgttgacaatcttctcgcgctccagcgccgccaggcggcgcagctgcattgcgaggatttcgttggcttggatctcgtcgacgtcgagaagcctcatcagcccctggcgcgcatcgtcgacggtttgggagctgcggatcagcgcgatgacctcatccagcatgtcgagggctttgaccaggccgcgcaggatgtgggcgcgtttttctgcttcgtcgaggcggtactgggtgcgccggacgatgacttcgatctggtgcttgacgtagtagcgcagcatctggtcgaggcgcagggtgcgcggcacgccgtcgacgatggagagcatgttggcggagaagttcgtctccagcgcggagtgcttgtacaggttgttcagcaccacgcgcggcaccgcgtcgcgcttgagggtgaccacgatgcgcatacccacgcggtcggaggactcgtcgtcgattgcggcgatgccgaccattttgccgttggcgatctgctcggcgatgccgtggatgaagttgtctgggttgacctggtacggcagctccgtgatcacgatgacctggcgcttgcccacctcttcgatctcggtcacgccgcgcatgcgaatcgatccgcggccggtggtgtaggcgtccttgatgccgctgtcgccgacgatgaggcccgcagtcgggaaatccgggcccttcacgcgctccatcacggcgtccagcgtggtttgctcatcggcctcgtggttgtccaggatccactggatcgcgtccgccagctcgtttaagttatgcggcgggatgttggtggccataccgacggcgatgccgttggagccgttcatcagaaggttcggcacgcgcgacggcagcaccgtcggctcctgggtcttgccgtcgtagttcggcacgaagtcgacggcgttctcgcgaatgtcgcgcaccatctccatcgcgatcggggtgagcttgcactccgtgtaacgcatggctgccgggccatcgttgccgggcgagccgaagttaccctggccgtcaacaagcgggtagcgcatggaccacggctgggccatgcgcacaagcgtgtcgtagatcgcggagtcaccgtgcgggtggtagttacccatcgtgtccgcgaccggcttcgcgctcttaacgtacgagcgctccgggcggtagccgttgtcgtacatcgcgtagatgatgcggcggtgcaccggcttcatgccgtcgcgcacgtcaggcagcgcgcggcccacgatcacgctcatcgcgtaatcgatgtagctggtttgcatctcctcgttgatgtcgatgggatggatgcggtcgaagccgtcgccgctgagggtgtcgtcagccatagctcacctttctgtttcgctctcaaggcagtctatcgccccgctagcggcccggcaccgccgacgctggtatcaaagtggtatggctatgacgctgagactaaccgcagaggaggacaaggcgctcgtgctgctcgcctcggcgtgggggtgctccaagcaggaggcggcgcggcgcgcggtggtgtccgcagcatcgcgcatgctcgaaaccgcagaggtcaaggccttggcgcgcgacatgatcccggagtaccgcgccaccgaagcccgcattcgccaggcccgcgcatgaccccggagcagctgctggccattgctgacgagttctgcccgctgtacaaaacgcagatccgctcgttcgcggcgatcgccgcctgcgccgccattcctgacgcacgcatccacggtgtgcgcgtgtgcggctcggcgcgggagggggctttcttgcttgccgacgccatcaccaccttcaaacccctcacctcccacaacgacgcgttcgccgtgatcgcgcgcgacgtctacttgcgcctacagtgaggtgcatgaagaaaaccaccgcggtcgctgcatcggcgaccctcgcaatcgccatggtcgccgcccccagctccagcgcgcgcgactaccagatggacccgaacgacccgtctattcaaaccccggacaagccagctctgggcagcgcgtacaccggcagcgcgccgctgtcgatcacgcttgccgtcctcgccaccgcggcagcggtgcagctcatcgtcgactccgtgccgcagatccgccaggccgtcgacgacgcggcagccgcagccggcctgcagtgggtgccgggttcctccgagggcaaccgcattttcgacgtcccggcgtggatcgctttcgctcagaacttccagctcccggcactgcccccggcggcgaactaggccgagtagcggccagttgttacgcgtgttactgttgatgccgttgtggttgcagtgacgtaaggtgctgtggtggaagagccataacacctcggcggcttgcgtctgatcaggcgttggccgcttccgcttttcttcggcggtaggatcgggcagcatgactgacttaaaggcactgctctcccccgccaaccgcgaatccgtggtgaaggaactctccgcgcttgtggacaccacggtgtccaaccaatccggcctcaccggcatggcgctgaagtccgccgtcgccgccggcaagaaagctgacgcagacgctatccccaagggcgtgaaccgcttcctgccgcagatcgtcgacgagctgcagccgctgttcaacgcctacgagggcggcaacgccgcgaacttcggcgcgtacctttcccacaacgaggacgacgtcgtggagaagattctcaacgcagccgacgccgccaccggggagatgcccggtgcagtgcagaaggtctactcctcgctgcgcggcaaagccggcaagatcatcggtcccgcgctgccggaattcggcgccatcgtggagaagtacgccaagtagcgcgcccgggcccgcgggccctccccctagacgtccaggaagcggacgtctttcgccttgcgggtgatgaagctgcggcgcgccgccacgtcatcgcccatgaggatggagaacagctcgtcggcgcgctgcgcgtcctcgagctccacccggcgcaggatgcgggtctccgggtcgagggtggtctcccacagctccttggcgttcatctcgcccagacccttgtatcgctggatgccgtcgtccgtgttgatcttgcggcccgcctccaggcccgcggcgagctgctcgtcgcgctcgcggtcggaaaacgcgtagccgggctcgcccttctgccacttcagcttgtacaacggcgggttagccaggtacacgtggccttgctcaatcagctccggcatgaagcggaacagcagcgtgagcagcagcgtcgcaatgtgctggccgtccacgtccgcgtcggccatcagcacgatcttgtggtagcgcagcttcgcaatgtcgaactcgtcgtggatgccggtgcccagcgccgtaatgatcgcctggacctcggcgttcttcagcacgcggtccatgcgcgccttctccacgtttaagatcttgccgcgcagcggaagaattgcctggtgcatggagtcgcggccgcccttcgcggaaccgcccgcggagtcgccctccacgatgaacagttcgcttttcgacgggtccttgctcctgcaatccgccaacttgccaggcagaccgcccaaatcggtcggcgacttgcggcgaaccaagtcgcgagccttgcgagccgcttggcgagcctgcgaagactgcaccgccttgttcacaatcgccttcgcctcggccgggttggcgtcgaaccagtcggacaggttctcgttcaccgcgcgctggacaaagcccttgatctcggtgttgccaagcttggtcttggtctggccctcgaactgcgggtcagcgacacgcacagagatgaccgcggcgaggccctcccggcagtcgtcgccggtgaggttgggatccttgtccttgatcagcttgtgctcgcgcgcgtagcggttcatcaacgtggtcagcgccgcacggaagccctcctcgtgggtgccgccctcgtgcgtgttgatggtgttggcgaaggtgtggaccgactccgcgtaggaggagttccactgcatggcgatctccgcctcgtgctcggtgcccttctgctcgaaaccgatgacggtcgggtggatctccgtcttcgacttgttcaggtactcgacgtagtcgatcaggccgttcgggtagtggtactccaccttcttctcgcgcttgcgcttgacgtcggacgcagcgtcaccagtctcctcgacaaccgcctcagcgtcgtcgtcgaaggaatcgccctcgatcagcgcggcggtgtcgccctcctccgcgatggcttcgagctcgagctcttcgtcggtcacgcgctcgtctttcagcgtgattgtcaagcccttgttcaaaaacgccatctcttgaaggcggcgggcaatggtgtcgtagttgaactcgacggtttcaaaaatctccgggtccggccagaaccggatggtggtgccggtgccgcgggcgttgccgccctccaccagcgggtctggcacagcgttgtcgaagttctgcagccagtgcttgccgtcgcgcttaatatccgcctcgacgcgggtagacagggcgttcactacggagatacccacaccgtgcaggccgccggagaccgcgtaagactccgagtcgaacttgccgccggcgtgcagctgggtcatgacgacttggacggtcggcgcgcccgaggggtgcatttccaccgggatgccgcggccgttgtccacgacttccactccgccgtccgcgagcagcgtcacgtcaacgcggtctgcgtggcctgccatggcctcgtccacagagttgtccacgacctcccacaccaagtggtgcaaaccgcggacaccggtggagccgatgtacatgcctgggcgtttgcggacggcctcgaggccttccaggatggtgatggatgaggcgtcatagtgcggttctttatcagccacggaaacggacactcctctttctctacaaagcgcctatacagcgttttaacctgtctcatcttacacccttagggggtcatgcccggtagcagctaaaccggcgagacggcgtttctcgcgccgatttcgcggtcgcgctatccgtaggtgtcgcgcgggccacggcccttgacgtgcaggggacctttgcgccacgacggcgccttcgggccgtagatgtgcagcctggtcaccacgtcggggccgactttttcgctgatagcgcgcaaaactgtggcctgcatgtacttcatctgcgtggcccacgcggtggtgtcgcactcgatatgcacttcgctgtccttaatcatgcgcacggtggtgtgctgcgcgatcttctccccgaccagggtttcccagttgcccatcacccagccgtaggccatgttctccgaccagtcgcgttttttgatttcggtgcccacaagcgagctgaaggacttcacccgcatggctttcggaagagcgcggccgtccatcccggtggcgcggcctcgggtggggcggggtgtggg

SEQ ID NO: 21 - DNA, 13278 bp, Corynebacterium cassirii
  source 1..13278: mol_type = genomic DNA
gcctgaaggacgccaaggaaatggtcgagggtgctccgaaggccatcctcgagggcgcaaacaaggacgacgcagaggctgccaagaccaagctggaagaggctggcgctaccgtcaccctcaagtaagagctctctgcttaacgacgcccccgtcacccggtccacacacccgggcggcgggggtttcgctttgggtggggtattgtgccaaccatgccgaagtcccgcgttttgtctgtgctgctcgtcggcctcggcgttgccttgttggtggggggttgggttgctccgagcttcattcttgatgacgggcggctgcccctgtccctgaagcagaccacgtggacaatgcacgacccggacggggtgcgcgacggccagccggcgccggtgacaaggcagttgcacatggagatccgcgagccgtcgaacgctggggtggcggcggtgcgggtgggccacaccttgcgcgcgggggaagcggcgaccgacttcgacaacttggttacggcgtcgacgtggtcgttcgagatgaaccggaagaccggccgcgtggaggagccggcggacgtgcagctggtgatggggatgccggcagtgcaggtgccggtggaggggttctggctcaagtttccggcgggggtggtggcggagcaggcgcacgaagtcttcgacccggtgctcagggcgtcggcgccggcacacttcgtcgataagaaagagctcaatgggcgcgagctgtaccgcttccggcaggaaatcccgccgacgaacgtggcgcagcggtacgcggcgcgagccccgcgatgaggggcgccagcgccccaagcagtacttcccggaacagtcccaaccccaataccagcaagcccagtacaagcaagctcagtatcagcagccgcagtacgagcagccgcagtaccagcagccgcactccgagcagccgtattacgagccgagctaccaagagccagagcaacgcagcaacatcggcacgattctgttgggcattctcgccgccgtcagctttgtcgcggcggtgtccctgttctttctgtggcgtggcgcggccgcggaggcagataagccaccggtgacggagacccagaccgtcaccaccacggagacgcagaccacttttcagaccaccacgaagttcccctccatcttcggtgagcgcgataacccgacggcgacgctcccgccggaggagccgatgccggtaccggaggtgccgcgcgagttccgcgaggacgcccgcgacattttggaccagctccgcgacggcgcggaccagttcttccaggagcagcagtgatcgagtcgcttgagatcgcccaggctgtcgccgaagccacggccaggcattgcaccgatgtggtgatgagcccgggcagccgcaactcaccgctggcctacgcgcttatcgcccgggacggcatcacagtgcacatgcgtgttgatgaacgctccgccgccttcaccgccctcggcatcgcccgcgttcaacggcgccatgtggcggtggtgatgacgtctggcaccgccgtggccaacgcctacccggcgctcatcgaggcgcacatgtcgcacacccccctcgccgccatcagcgcggaccgccccgcgcgcctcatcggcaccggcgcgagccaaaccatctggcaagagggcatcttcgcgcgctacgcaaccacgcagcaagtgcattcgcttatcgacgccacgtcgctgcacttcacctccccccaaatacacatcaacgtggccctggataccccgctcgtgccgcaggcattgccgggacgcacaggcgcgccacgccgagtgggccctggggtgttgtcgggttcggctgcgtttgtggaccacggggtggtggacatcgacctcacccgcgacaccttggtgattgcgggcgatgaggcgtgggaggtgcccgggctggagcacgtgcccaccattgcggaaccgaccgcgccgacgccgttccatcaggtgcacccgttggcggcccggtttttcgcccagcgcgaggtggccatttcccacgacgggggcgacttcgctgccaccacaaagcctgcgcaggttgtggtggtgggacaccccacgctgcaccgcgacgtgatggcgttgctggcggacccggacatccatgtgattgggctaagccgcaccgacaccttcacgggccaaccggacgagcgcgcaacacgcgtgaatgtcaccggccagcccacggatacgtggctgaagatctgcgaggccgcaggcgaggtcggcgcggacactgtgcgccaagcgctcgcggacgtcgagttcgggttcaccggcctgcacgtcgccgccgcggtgtgcgacaccttggccgtcggcgacacctttgtggtgggcagctccaaccctgtgctcgacgtcagctttgcgggcatgccgtttgatggggttgacacctatttcgcccgcggcgctgctggcatcgatgggacggtgtcccaagccgtcggcatcgccttggcggtccaagcgttgcgcccggacgagatccgcgccccgcgcaccgtcgcgctcatgggtgatctgacgttcctgcacgatgtcaacggcctgctcatcggccccgacgagccgcgccccggcaacctcaccatcgtggtggccaacgatgacggtggcggcatcttcgaatccctcgagcccggcgccgagaccgtgcgcggcgcattcgagcgcgccttcggcactccccacggcgcgcagttggaggacatcgtcgtaggctacggcgcccgctaccgccgggcggaaacacttgcagagctgcacgaagcgctgttggcgtgcgaggcggaaccggacggcatcaccgtggtggaggcggtgaccacccgcgcgacgcgccgggagcttacgcaaaggctcaaccggtgaggtggcgccgccgcgcgcaccagttcgtgctcgcgctctacgcgtgcgcggtgctgggctgcgtggcaatggtcgtgggcccctggctcaacgacgtccagattgccaacaacaccggccgtggcatgggcaccgtgacggaagcgggacggctgcaaacctccgtcaaatacgttgacgaagacggccagctgatcaccccgcgcggcgggttgctctatccttctggtctcggggcggagcagcatgtgtgggtgacctacgccaactacaatcctgacctggtcaaagtggagggccgtgcctggacgctctccctcatcccggcgctttcggtgctcgcggttgcaagcgccatcgcgatggctggatggttcgcggtgaatcgatgggtgccataaaaattcacgcgacgtttaacttgggttgacatgcagttcgcattggggtgccaatgagggccattatgcgtgtgggaatcgttgctgagtcgtttttgccaaacgtcaacggggtcacaaactcggtgctccgcgtgctggagcatttgaagcgggaggggcacgaagccatggtcgtcgcgcccggcgcccgcgacttccaggacgaaattccggactacctcggttttcccatcgtgcgcgtgccaacggtgatggtgccgctgattgattcgctgccgatcggcgtgcccaccaccaccgtcgcggcggcgcttgcggaattcaacccggacatcatccacttggccagcccgttcgtcctcggcggcgccggtgccttcgcggcgcgccaactgggcgtgccggcggtggggctgtaccagaccgatgtggctgggtttgccacgaagtaccacgccgccatgattgccaacatcgcctgggactggacgcgcacggtgcacaacatgtgcgagatgacgctcgcaccctcctcggtgtacatccgcgagctggaatcccacggcatcaaaaacgtccggcactggggccgcggcgtggacacgcagctgttcaatcccacgaagcgctccgacgtgctgcggcgcgcctgggatccgacgggggagaagaaggtcgtcggattcgtcggccgcctcgccgcggaaaaagtcagtgcaccgactcgccgcgctgcacggggacctgtcgatccagctcgtgattgttggcggtggtccggagcgcgatgcgcttgagtcgctcatgccggacgccgtgtttaccggcgccctgtccggcgaggaactcgcccgcgcctacgcctcgctggacctgttcgtgcacaccggcgagttcgaaacattctgccaggccatccaagaagcgcaggcctccggcgtgcccaccatcggcccgaaggccggcggccccatcgacctcatcgaacacggcgaaaatggcctactgctcgaggtggacaccttcgaagacgagctacccgatgcggccgcctggcttctcgacgccgcccgccacccccaactccaactcaccgcacgcgagtccgtagtcgataaaacctgggcagcactggggggccagctgttgggctactacgaagaggcgctgcgcagctaccagcgcaacgtcatccagctcatgggccgggaagtggcggtgccgcactgggtgccggcgcgcatttcgcagccgcgctcggtactgcggtctcgcaccgcgtaggcgcatgcgcgccgccaagtagagtggcgagcatgtctgtcggcgacctgtccaccagcacccagaactacctcaaaggcatctgggcgctttcggaatggtcagatacgccggtgacaacgtcgtctgtggccaagcacctcggactgcggaaatccaccgtctccgacggggtgcgcaaacttggcgagcagggcctagtggagcacaagccttacggcgccgtcgagctgactgacactggccgcacgtacgcggtggcgatgatccgccgccatcgcttgattgaaacgtttttggtggaggcgttgggttacacctgggaccaggtgcacgacgaggctgaaaacctcgaacactcggtgagtgacttcatggtcgatcgcatcgacgcgtttttggactaccccagccgcgacccccacggcgaccccatcccctcagccagcggccgcgtcgacaccccggcggcggtgccgctgaccgctgtgcaacccgggcacactgcgacgatcgagcgcatcgcggacgacgacccgaagctgctgaagttccttgacagccatgggctcatcgtcggcgcgcagctcgaggtggcggtgggcgcgccttattccggcgcggtggaagtccggctggctggcgcgactgcggcggttcagctcggcgaggccgcgaccgactccgtcttcgtgcgcgtcgacgagtagccgcgcccgcctcgaacgccgtgcgggctgagaagccacaccgcggtgaacaccgcgccctgggcgagcacgatcatgccgccagaggccgtgtccaggtagtaggagcagtacaggcccacaatcgcacacgccgccgacatggtcggggcgatgatcagcatcgtgccgaatttgttggtgagcaggtaggcggtcgcacccgggatgatcagcatcgccaccaccaggatcacgccaacggcctggagtgccaccactgacgtcagcgccagcagtgccagcagggccgcaccgagcaggcgcggattcaacccaatcgcgtgtgcatgggtgggatcgaacgcgtagagggtgaagtcgcgccgcttgagcaccagcacgctcaacacgatcgctcccaggatggccacctgcagcaggtccccacgggacacaccaagcagattgccgaagatgatgtggttcagatccgtgtgcgaaggggttaccgaaatgagcacgagccccagcgcgaacatggtggtgaacacaatgccaatggccgcatcctccttcacccgggacgtatcgcgcaccagcccgatcagtgccaccgcaaggaacccgaacaccaccgcgccgacggcaaacggcacgcccagaatgtaggccagcaccacgccgggcaggacagcgtggcttaccgcatcgcccatcagcgaccagccaaccaacaccagccagcacgacaacagcgcgcagacaatcgacgccaccagcgaggtcgcaagcgcacgcatcatgaactcgtacccaaacggctccgtaagcagcgcaatcatgctgacacccccataccgaagccctgtaccaaattgtccggctctaacaccacttcagtcggggcgtgcatcaacacccggcggttcaacagcactgtctccggcgcgagctggggcaaggcaaccaggtcgtgcgtcaccacaaaaatagtggtgccttctgccgcgaggtcacgcagcagctcagtgatggtggcctcggaatgtttgtccacgccggcgaagggttcgtcgagaagcatgatgctcgcaccctgagcgataccgcgggcgatgaaggcacgcttcttctggccacccgaaagctgaccgatctggcggtctgcgaacgactcaaggtgggtgcgctcaagcgcgcgatccacagccgcaatgtcctccgcacgcgcgtggcgggtaaagcccatgtggccgtagcggcccatcatgaccacatcacgcactgtgaccgggaactgccagtccacgtcctcgctctgcgggacgtagcccagcacctgcgtcttgcgggcgcgcatggggtcgatgccgttgatacgaaccgtgccgcgatccggcttgaccaaccccatgatcgccttgagtagcgtggatttgcccgcgccgttcatcccgatcagcccacagatacggcctggttggacgctcaaagttgcgccgtcgagcgcgacgacgtcgccgtagcgcaccgcaacatcgtcaaccgcgattgcggggatcactgcttgcccccgttcaaaccgtcgatgatcaccttcgtgtcgtggcgaatcagatccaggtaggtcggcaccggaccgttttcctcagaaagcgaatcgacgtagagggtgccgccgtactccgcgccggtggccttcacgacctgcatcatcggcgcgttagagaccgtggattcacagaacacagacgggacgttgttttccttcacaaactcgatcgcgccggcgatctgctgcggggtggcttcctgctcagcgttgaccggccagatgtagcgctcggtcaacttcgcgtcgcgagccagataggagaacgcaccttcgcaggtgaccaaggcgcgctgcttgtcggggacagcggcgagcttggtctccagctcgtcttgcacagcctgcagttcctgcttgtatgtttcgccgttggccttgaaatcatcggcgtgctccgggtcgagttcgctgaacgcgtcgacgatgttgtccacgtacttctgcacgttcaccggactcatccaggcgtgcgggttgggcttgccggcgtaggcgtcctccgcgatgtcgatcgggtcgacaccttcgctgaccacggcgtggggcacgtccaggtcggcgacgaactgggagaaccagttttccaggttcatgccgttgtccaggatcaggtcggcgtcggaggcgcgcgagatgtcgcccggggtgggctcgtagccgtggatttccgcgccgggtttggtgatggactccacccgcaggtggtcgccggcgacgttcgaagcgatgtcctggatcaccgtgaacgtggtgagtaccacgggggtgtctttgccgcctgcggcgtcggcgctgtcctgcgaacagcctgccaggccggcagcaagcgcagccgtggcggcgagcgcgagcaccttggatttcaacatgttggtccttttttctttctgtgttctttctgggcactttccgtgcggttagagaagcggcggcgggccgacgcggtgggacgcggcaatgaatcggtcgagcttttgccgggattcgtcgcgcaggtagacggcgagcagccgcatcatgtcccataccggcgaataataaagttcgtctggcagaactttcaagtgttgtcttgtcgtacgacccccgtttgcggggggcgcacggacgacgagggcgatctggacccaacgggcacggtggtcgtggtaccgccgaagacgctgcagccgataccgccgcagcgcgagttccgcttcttgggcgacccgggtgaggagacgtacctgctgccgcaggcggtgctgggccgccacgtccacggcgagctggatccgcacatctggcacgacccagccgcgatggacgcggtggtgcaggtggtgcgggacgagctgtccgcggccgacccgcgccacgccagcgcgtacgccgacaacgccgagcgctaccgcgcccagctcaagcaggtggcgcaggaggtgcgcgcggagttcgaccaggtcccggagaccaaccgcaacctggtcaccacccaccacggctacgcctttctggagcgcgcgtacgggctgcgcgtggccgggtttgtcaccccgaatccgatcgtggagccgagcccgcgcgatctgatggcgctgtcgcgcacgctggacaacttggccgtgccggcggtgttcgtcgggcacggcaaggaagacgaaacgcccgttttgaacgaaaccgctgccttgcacggggttgaggtgtgcccgatctggggcgacaccttagacccgccgggggaggggcctgcgcagacgtatgtggatctgatgagggccaatggaacgtcgataagtaaatgcttgaaaggacaaccatgagaattcccgctattatcaccgccgcaatgatcgcggccgcacccgtcgctgccgcccaggtgccggacaacgacccggcgttgcagcaggtcgtaagagccgacgagcaggttgccccgcagggagagcgcgccgtcatcgacgccggccacgcggacctgggccccgtcttcgtcgacggcaagctgcagttcctggtgcgcgacgacacgcaggacacgcccgtgtggcgccacctcgaggacgtggtattcgccgtgggtgacggcgcgaagcagaccctgccggagaccgaccagttcgcgttcaccggcgcgaagccgggggccgaggtgtgggtgatcccgcagaccgaggtcgtcggcgtgccgtggctggggtggaactcgcaggcgccgtcgcttgtggaacgctccgcaaacgggatgagcctggagttcggtggacatgagggcccgggccagttctccctgtttgttcagcccggcgggttccacgagcctcagcagctgtggaacgggcaggagcccggcacgcagtcgatgtgggtggagccgaacacgcacacccacgccaactgggtgttcaccgagccgggcgcccacctggtgggtgtgcgcgcgaaggtggaggaccaagacggcaccgtgcacaccgacgagcaggtggtgcgcatcgccgtgggcgtggacccagcggaggcggcggatgcccagttcggtgagtttcgggctgagggcgatgggggtgaagcggcgtcgcaaagcggtggcttcaaccttgtgtggctgatcggcctcggcgtgcttgccctggtcgcgctgcttgctgtggtgtttatgaggggccgtcgatgagaaggattgaggtgcgcgaactggcggtgtcgtatccgggccacgacgtgttccgcggggtggatctcacgctgcgcggtggcgagttcgtcggcctgctcggacccaacggcgcgggcaagaccacgctcatgcgcgcggtgctaggccttatccccgctgacgccgggacggtctccgctggcaggggcccggtgcgcaaggtggtggggtacgtgccgcaggcgcacaacgtggcctgggattttcccatcgacgtctatgccgccacgctgaacgccacgctcggacagcgcccgtggtggcgccgcgccggcgagcgcgagcaccgcgccgcccagcaagccttggagatggtcaacctgaccgacctgtccgatcgccccatccacgacctgtccggcggccagcgccagcgtgtgctcatcgcgcgcgccctggtgcgccgcccgggcatgctgcttctcgacgaaccgtttaccggcctggacatccccaccaccgagcacctgctgcggctgttccgccgcttggtggaccggggtctcggcgtggtcatgtccacccacaacatcgccgaggccattgattcctgcgacaggttggtgctgttcaaccgtggggtcgtcgccgatgccgcgacgcatgagctcaacgatgacgccccgtggactagcaccttctccgtcgacgaggattcgccgtggctgcgcggcgtgcgagctcatttggaggctgcccgtgcctgagatttcgtttgtgcaattcctggccgacatggccaacccccagctagcgtttctgccgcgcgcgctggcggccgcggtgaacgcggcggtgctgtgcgcggtggtgggctgtttcgtggtgctgcggggcatggcctttatcggcgacgcggtggcgcacgccgtctttccgggcatcgcggtggcgtttgcgtggcaggtctccgtgttgctgggtggggcggtggccggcgcgatcgtcgcggtgttgatcgcggtgatgtcgcagcggcgcacgatcaaagaggactctgtgatcggcatcgtgttcaccgccgcgttcgccttcggcctggtggtgatctcccgtgcggagggctacaccgcatccgtcagttcgtttctgttcggctcgctcacgggcgtcagctccaccactctggccgtccacgctgtcgccggcgcgctaatcgtggccgtagtggtggcgcttcgcccgtggctgacggcggtggcactcgaccgggagaccgcccgtgcgatgaacctgccggtcgccgcgctggatctggcgctgtacctgtgcgtgaccttcgcggtggtgttggcagtgcagacggtgggcaacatcctggtggtggcgctgctgatcaccccggccgccgcggcgcgcctgttcacgaacaagctgggcgcgatgatgtgcatcgctgccgcgttcggggtggccggcagcgtggcgggtgtgtggctggcgtggtcctacgactcgcccacgggcgcgaccatcgtcctggccgttaccgccatcttcgcgctgagctggctgttcgctccgcgtcgcggcgcgcttgctggctggcttcagggggtgaggcgatgaagcgattcgttgcagcggcggccgtagcggtgctcgcgctcttggccgcgccgcatgcgcaggccgcggagcataaccccggcgacccgggccacggcgtggaactgggaaagattgaccacccgtgcgccgggcgcaaactgctctaccactctcacaacgacgcgctctacggcacctacaaaaacggcaagctcaccgtgatggcggtggacggccagcaagtcaccgaccaggaaaaggtctgcttccgcctcgctccggacgccgacgccgacggcaacgacgtgtccaccttgaccgtgccggaggacggctccctgaaattcctcggcgagcccgccagcaaggtgtgggccgcgccgcaatccgtggactggaccgacagctggcggcccatctggtctggcctgggggctttcgaccccgcgcacgaggcgggtgagatcccggataacttcgtcgacgacgtcatgcacttcgacctggtggagatggacggccccggcgatgtcaacgtgtttttctcctcacgcgtgggcgatccggagcggctgtttagctccgccgacgaggacatgcgcaccatcacctacgacgtcggcggccacggccatttcacctggacgttttccgaaccgggcatctacaaaatgacctggcagggccgcgccgagctcaaaggcggcggcacggagcgctccgagccggttacccagtactggctcgtcggcgacgaccccaccgtcggcttgcccgagggcaccaccaccgatctgcgcacccccaacaccgcgcaggacaccgctagcccttccccgagcgcgacggcgtcgttgcgcccgaaactctcgactagcacgcgcgccacgcccgcgccgcggcccacgacaccggctgaagcggcgccgacgagcaccgcacccgcggaccggcgcaagctcatcaggtcggggcatatggatatggcgttggtggccgaagggccgtcgataagcgcgaagcttattgacgactccgacccccacaaccaggcccaacgtgaatccggcagcttcatcttcgccgtgccggacgcggcgcgaaaaacgctgccggtcggcgtgagagagagctttccggacgcgcccgaagagatgtggattctgccgcaggcgcagcagaaaaaccttccctggctgggattttccaccactcgggtggccgccgacgcgctggcgcaaggctcgaaggtgaccgtggccatgcgtgccgtagacggtcccgggcgcatctacacctggcacgaggacctgcgcgggctgcgcgtggagctcgattccggcgacccggacaaaacgctgggatacccggtcaacgcccacgatcaccaaggctttgggttcaccgaaccgggtgtatacaccgccacgtttaccttctccggcacgtctgccgatggcgaggacttctcagaggaactggtggccaccttcgcggtgggcgacgaggccgtcaccgccgcgagcgagggccgcctgggcggcgccggcgctgcggccggtgcctacaagggcagcggcaagctcacgctgccgggcgtgttggcgaacggcatccgctcgcttgaaagagagataaagaaagccggcgacacgctcgcgtcgcttgcgcgcaagaaggaccacgagggcgacggcggcagtggcggcagcgacgcgaagtcggggccggtgtcgggctcggcggcaacgccggcagcaacgccggcagcaacgccgaaacaaccccaatcggcccccgccgcgcaacccgcggcgcagccgcagcgcgcaccgagcaacaaccgcgccagtaggtcagcgacccgcgaggacaccaaggccacaaaacccgcggtgacgaccgaggtaaaagcgccgtccgaagcatcttcggcgacggccggtagcacaggtacgtccgagtcctatgccgcccagccgaatcccgcaggcggaggcggcacggggattcactcgtcgcttgacgccgccagcgcgcaaccgggcggcggggccacgggaacgtcgccgacagcgggcgggttttgggc

SEQ ID NO: 22 - DNA, 10358 bp, Corynebacterium cassirii
  source 1..10358: mol_type = genomic DNA
ccttctaccccacccccgcatccaccgcgtccctggcaaccagacttgcgcttccagcctccgtcacccgggcactacgaaccctgaacgccaccgacctgcgcgcgctggaacgcctgagtgacctcggcgcggaactcgaccccgtcgacgcggccagcctcgacaaagccttgctacccggagttgaccggctgcgcgagcgcgcgctggtctacgggcccgatagtgcggtgcggatcgcccccggtacgctttccgcgcttccctctggctggcggatgagcgatgtggcgccagagggggtgcgaggggtcgtcgataagctacctgcccaagagcgcaaggtgctcgagacgcttgctgcggccggtggagtgggcacaaccagggcagccgctgtcgacgcggacccgaacacccccgttgcgcgcctcataggccagggactactcgtgcgcgagaacgcgtcgactgtgcggctgcctcgaccggttcgcgacgtgttgaccggtaacgcaccgcgcgtctaccccgctaccgagccggcactgccggcggtggagcagcgcgcggtggacgaagccgcagctggtcagggcctggatgcggtgcgccaactgcgccagctgctgacctacctgctcgcccaaccggtcgcattgaacaaagacgccacggtcggcgtgcgcgcgcttggcgccatgaccaaggatctcggcttcgacccggcgttcctcatcacagtcggcgaggccgcggggctgatcggccgcggcaacgttgacccggcgtccgacgccgacgcgcttgccgccacgaaggacgcgctgacgtggcttgacgcaacgctcggcgaccagtgggccatcctcatggttggttgggtcgcgtcgccgtggcgcgtggacaccgggcacaagctgctctcgagcgagatgcacgcgccggacctgcgccacgcgcggatgaccatccttcgcgcagccggcgaccgcgagcggttgctgtttcaagcgccgatcgcctcgtcaggcatgcgcgacagcctgatcgccgccgtcgctgccgaggcggaaacggtgggagccctggcactgggtgggttatccacccccgcgcaggcacttctcaatggctcggacgtcgccgccgccgccaaggcgctcgttcccgccgaggtggacgcggtgatcgcacaggccgatatgaccatcctcgcccccggcccactcactgccgacgccgcccggatgatggagcgcttcgccacgctggagtcccccggtttggccagcgtgtggcgggtgacggaggcgtcaatacgcaaagccctcgacagcggcgcgaccagcgatgagctccagcggtggctagaaacccacgtgatcggtgaggtgccgcaaaacctgcgcttcctggttgatgacgtcgcccgcacgcacggctccatccgcgcaggcgccgccatgagttacgtgcgcagcagcgaccccacgctcattgccaccgccgccgaccgcgtcgacctgcgggtgcttgcgcccaccgtcgcggtgtccgacctcccgctgcctcagctgatggcgcagctgcggagcgcggggctgcagcccaccgccgaggacgctcgcggcgccgagctgaacatggtgccggagccctccttggtacccgcgacgccgtcgacattgccgcgagagcgccaggtcgagcccgcccaggtggaacggatcgtgagcgtactgcttaccgacgccgcacgaaacgacgaggcaaccggcacccagaccaccgacgccggcgctgacaccatcgaagtgctgcgcgcggctgcccgcgcacggcgccacgtctccctcggctacgtggacaagaacggccgcggccaggttatgacggtgctgccgctttccgtcggcgggggccaggtggacgtgctcgacgaggcaaccgaccgcgtcgtgcgcatcgccctgccccgcatcacccgggcggtgctggcataggaagacccgccccaagcaggtcgctaggagcgggagcaaagtgacaaggggcgtacagccaactcaaatggtcggctcagtagggaggttaaggtggtctacgcaacccggcaaccgctggcgcacgatcataatcacacacatatactcagtggtttagtaagtcacctatctatccctaaggaagttcccgtgaaaaagacagcaagtgtgttcgcaacgtccctcgccgccgtctcccttgcggcttgcgctggcgccgacatcgacggcgactacaccggcaccgttaccgaagacggcatcaccgcgcagatggatctcactgtcgcagatgatgtttgccagttctccatgaccgcgccaatcgttggcgagatgccgtactcctgcgagatcgacaagagcaacaacgtcatcatcctcgatggcgaggagatcaactacacggtcgacggcgattccatcgtcatggagaccctcgaggacgaagaagacgtcgtcctgaagaaggtctccaagtagcacccggctagcgggtcacctgctccagcacctcaagcacgtggtggtactcctcgccggtggctcgcgtcatgcccagctcgcaggtgcggttacaggacgcgtgcacatcgctgtccaagcgctcaacatcgcgagcctccatcgtggtcgccgcatccgtcagttccgggtggagcatgcctcggtcaccggcgtagccgcagcaaccccagctcgtcggcacgcgcacctcggttgcagccgccgcggccaccttctccaaatcagcttggattcccagatgcgtcgtggagcaggtcgggtgcagcgtgatggattcgaccttgtcaccggccggcagcgcgtccaacatgtgctcggcaacgaaggttacggcgtcgatgacgtcgatgccgatctcggccgcgatgtccatcatcccgtgggtgcagctggcggcatccatcaccaccggcaaccgtcccccgcccgtggcgcgaaggagcgaggtctgtacacgcgcctcaagcgcagcatggccagagcgcatgcccttggacgtccacggagtgccgcagcacagcgagtcaatatcgtcgggaacgatgagcgcaaccccggcgcgttccgcgagtcgcacgaacgcctcggtcgcgccgacgccttcgccttgcgggccgaacatcgagttcacgcacgccggaacgaaaacggcgctgggtttggcgaaccggtcccccaccaccgggcccagcttcgatcgggtgcgtccacccttgcccaactccggctggtactgcggcacggtgtcggcaccggcgagcgcgcgggcgacgtcggtcaccttctgcaccagcttggtgggaaggtagtacgcgccggtgagggctgctgacgcggcggtgttggccggaccccacaccttcgccgcggtggtccaaccggcggtttccacagcgccggcttcttcggcgcgcaggtgtttgatgaatttgccggtgtcaatgccaaccgggcatgcggtgacgcacaaagagtcgacggcgcacgtgtcgatcccctcgtattggtaatcctggtcgatggcgctgacggtgcccaggtcgccgtcggcaagcgcctgagccctggcgcgacgcaccacgatgcgctggcgcggcgtcatggtgagatcgcgggacgggcacacgggttcgcagtagccgcactcgacgcacgggtcgatctcgtcttcaacctgggggttgagcttgaagttcttcatgtgctcgcggtcgtcgtcggtgatgatcacgccagggttcatcacgccgcgcgggtcggcagcacgcttgagctcgaccatgacctggtaaagctcgtcgccgtactggcggcggacgtacggcgccatgacgcggcccgtgccgtgctccgccttcaggttgccgccggcgctgaggacaaggtcgaccatcgcctcgttgaacccgtcgtagcgcttcaagttttcgtcgccctcgaagcggtcggtgatgaggaagtggatgttgccgtccttggcgtggccgaaaatgacggcgtcgtcgtaggcgtactcggtgaacagggtctgcagcccgccgcaggtgtcggccaagtccgcgaccggcacggcgatgtcttccagcagcgcggtggttccggacgggcgggcctcggccacctgggcgtagaggcctttgcggaaggcccacgccttggcggcttcgcgggcgtcggtggagaacgccgcgggggtctgcaggtcaaactcggtaagcagcttcgcgcccacctgctcgtactcgcgcagctgctcggcgtcgttcgcgtggtattcgatcaaaagcgcggcctgcccgtcgagctcgaagccggtgatctgctcgggcacggtgtcgaacgagcggcctaccttgatggagcgcgagtccatcagctccagcgtcgccgcgtgcgagtcgaaaagcgcgggcagggagcgcgtcgccgcgtcgatagttgggtagaccgcgatggtcgtcgtcttaagcttcggcacctcgatggtgcgaagcgtcgcctccgcgataaacgccagcgtgccctcagacgcgaccagcaagtgcatgaagatttccaggggcgggtcgtagtccaagaacgcgttgaggctgtagcccatcgtgtttttcagcgcgaagtgacgctcgatggtggcgacggactcggcgttgccgcgcacgcggcgcttcaggcgctcgatcgttgccgtaagttccggctccgcctgcgcgaactgcacctccgcgtcggcgtcggcggtgttgatcaccgtgcccgacggcaagacaaaggtgagcgattcgatcgtgttgtacgtgttgaacttcgtgccgcacgccataccggaggagttgttggcaatcacgccgcccatcgtcgccgcgccctctgaggccgggtcggggccgatcttgcgcccgtagggggcaaggtacgcgttgacctggcgcaccgtcgatcccggctggacgcgcacccggttgccgccgtcgagaacggtgacgccgcggaagtgcttgcgaacgtcgacaagcaacccgctcccgcctgcctgacccgacagcgacgtgcctccggagcgaagcactaccgtgcggcccgaagccgctgcagcgcgaaacgctgctgccacgtcgttcgcactgcgcgcctcgaccaccgcatccggggtgtacaggaagtgcgacgcgtcgtgggcgtacttgatgcggtcgatcgggcgggtggtaatcgcctcgctcgatccgagttcgcgggtgaggtgctccaccggggaagaaattgtggctgtcatagacccatgctagcccccggccccgctgctaccttcgatcgcaaggaggatgaaaagtgaccacaatcgaaattcgggaccttcgcaagcgcttcggcagtgtccaagccctcgacggcatgagctttagcgtgcgcgacggcgaaatctacggcttcgtcggctctaacggcgcgggcaaatcaaccaccatgcgcatcgcactcggtgtgctggaggcggattcgggcgaggtgctgctggacgggcagctgcttgacgacgacctgcggcgccgcatcggctacatgcccgaggagcgcggcctctacggcaaggaaaagatcctcgaccagctcgttttcttggccaagctgcacggcgttgacggcgcggccgccgttaaacgcggcacagcgctgctggaggaactcggcctcggcgagcgcctgaacgacaaattggacgacttgtcgctgggcaaccagcagcgcgtccaactcgccgcgagcctgatccacgacccggagattttgatcctcgacgagccgttttccggcctcgaccccgttgccgtcgacgtgatgagcacaatgctcacggaccgcgcccgagccggtgtgccggtgatcttctcgtcccaccagctcgacttggtgcagcgcctgtgcgaccgcgtcggcattgtcacccgcggccgcatggtcgccgaaggcaccgtggacgagcttcgcagccagggcccggtgcgctacagggtgggcacgcaaaccgcaggttggttgccggagggcaccacgcttatcgacgccacccccacccacaccaccgtcgaaacccaaagcaccgacgaggaccagaaaatcctccgcgccgcgctgtccgccggcccggtgcacgagttcacccgcgtcgtgcctgacctggccgacctgttcaaggaggtagtgaagtagatggctacgcagaacgcgtactcccccatgcacacgatcacgacgacggccgcgcgcgagatccagatcctgttccgcaaaaagagcgtgatcatcacgctttcgatcatgctgctcgcgatcgttgccctgatcggcttcggcacgtggcagaaggagaaggacgacaccgccgacgccacctcggtcgccgcggtcgggctcgaggaatcgcttctcgacgacgccggttacgacggccgagccgccacaaatagggacgaggcggctcagttggtgcgtgacggcgacgtggaagccgccgtcgtggtcgacggcgggacttggcaggtgatctcggacgggatgccgaagagcagcatcctgagcggcgtcgagaccatggcggaaaactacgcgcgcgcagaggcgctctccgcgctcggactcaccgccgagcagtacgaggcggcgaagccgtctgttgatgtcgtcccagtcgacatcaacgacacggacggcgagcagaccgagaagaatttcgtccgcctcatcaccgcgtttgcggcactcatgatggtcattttcaccgtgatcacgttcgcggcgcaggtgggcagccgcgtgaccgaggagaagtcctcccgagtggttgagctcatcttggccaccgtgcgccccatcgacttcctcgccgggaaactcttgggcacggtgctctacgggttcgtcgccaccgccctgctcttcatcgttgccgcactgggacttcgctggtccgggcttgtggacggcatcgaattcgactggtcgattttcccagtcctcctcgtcgcgtggctgttggccatgctcttcttcggcggcctctacgccgccgccggcgcgatggtgcagcgcaccgaggacttgcaatccacccagatgccgattctgctgctcctcatggccgccgcctatatcccgggcttcggctggatgagcacggacaccacctggatgcaggtgatgagctggatcccgccgttttccatcttcgccgcgcccctgtcatacgccgccggtgacttttccgccgcgcagcttgccggctcgcttgccttggccgcgctcgcaacagcgctggtgatgtgggccgccgcacggatttacaagcgcacgattttgaacaacggacgcgtgagcaagtggtccgaggtgctgcgcaggggctaggtcaaccaagctagcgcgcacgcgcctcagcaataaaccgctcgacgtcgaactcggcgtcgagttcgccttgctgcaccgcaacgccgagcgcgtcgaacttgcgctcccgctcctccaccagccgcagcccctcgcgcagaacttcactcgcggaggcgtaacgcccgtcctggatgagctgggcgatgagcttgtcgtagcggtcgccgagtacaactgaagtgttcttagccataaccggcacgctaccaacatgcaaggagatactggcatggcttacggcgacggccctcttattgtccagtccgacaaaaccgtcctgctcgaggtcgcgcacctcgacgccgccaaggcccgcgcagcgcttgcccccttcgccgagctcgagcgcgccccagagcacatccacacctaccgcatcaccccgctcgctttgtggaacgcccgcgccgccggcttcgacgcagaacaggcagtggacacgctcgagcgctactcgcggttccccgttccgcaggcattgcttatcgacgtcgccgaaaccatggcccgctacggccgattaaagctggtgaagcatcccgcccacggtctcatcctggaggccgacgaccccgccatcctcaccgaggtcttgcgcagcaagaagatcgtcccgctcactggcgcaccaatcgacgaactcaccgcacccgtgcacccgtccgcccgcggccagatcaagcaggagctgatcaagctggggtggccggtggaggacctcgcgggctacgtcgacggtgagcaccaccccatcgagttgaaccacgacggctggcagctgcgcgactaccagcagtacgccgccgagtccttctgggagggcggctccggcgtggtcgtgttgccttgcggcgcgggcaaaaccatcgttggcgcggcctccatggcgcaggcgcagaccaccacgttaatcctggtcaccaacaccgttgccggcaggcagtggcgcgacgagcttctgcgccgcaccacgctgacgccgcaggagatcggcgagtactcaggcgagcgcaaagagatccgcccggtcaccatcgccacctaccaggtggtcacccgcaagacgaagggcgagtacaaggcgctcgagctgtttgactcccgcgactggggcctcattatttatgacgaagtccacctcctgcccgcgccagtcttccgcatggccgccgacctgcagtcgcgccgccgcttggggctcacggccaccctggttcgcgaggacggccgcgaggacgacgtcttctcgcttatcgggccgaagcgctacgacgccccgtggaaagaactcgagatggccggctacatcgccaccgccgagtgcgtcgaggtgcgcacatcgctgaccgaggaagaacgcctgctctacgccaccgccgaaactcgggaacgataccgcctcgccgcgtgcagctcgcgcaagatggacgccctccgccgcatcctcgacacccacgagggcgaacccacgctcatcatcggcgccttcgttgaccagctggaggaaatcgccgaggcgttatccgcgccgctcgtcacaggctccactaccacgaagcagcgtgaggaggcattcgctgctttccgacgaggcgacatctccaccctcgtcgtctccaaagttgccaacttctcgatcgacctgccgggggccgccctcggcatccaggtctccggcaccttcggctcccgtcaagaggaggcacagcgcctcgggcgcctcctgcgacccaaggcggacggagcggaagctaccttctacaccatcgtcgcccgcgacaccctcgacgccgagtacgccgcccgccgccagcgcttcctcgccgagcaaggctacgcctaccgtctggtgagtgccgacgacctttagactggctcccatgagcgagatgaaggtgttcaagttcgacgtcgacgaggcctacgccaagcagcacaacgaaatgctgcgcaacacgaagtaccttgtcatctccggcgtcgcactcttcatcatctccctggccgcagccgccgcagtttggttcctcgtcgacccatcctccccttggcacatcctcggctccatcggcctcgcacttttcggcgtcatgatgctcattgtcgcgctcgcgattccccgcagcgtgggcaaggtgcagcagctttacgacgcccaccccctctcccccgccatcatcaccgaaaaccacggcacggcggtgacccttaccgccctcgtcaacgccaacgtcgaccccgacttgccgccgcgctgggccctcacctccctcgtgaccaagccgatccccggcgcccacgacaccaccggcacaaaaattcccgtcaccgccgtcggcgcccagcagtccgttcatgacaaggcccactggcaggtcatcacacccatgccgatcgcttgggccaccccggaccccgacgttgttacccaagcccggacctccatccctcaccgtcagtggcaaacccttgagcacgccgcgaaggatagtgagcttgtcgaggcctcaaagaagaccctccagctcctctagcccctctcgttccccagcccgctggcccgctcctccgcccctccgccgccgccgtccgtgcgactcgctaatagcgggtatctcggcgacagttgtgtgtttccgcaggtcgcgttgcgcggtcgtgggagttacccgctatcagtggttgtggcctgtagctcccagggtttcagtgtgtcaacgacagggggttttgcacctaccgatgaggctgtttgtcgtcgggagctacagggcgcggcgcgtgcgtcgcccgtgtcactgccgcctatgtgccgggagcgccccgata

SEQ ID NO: 23 - DNA, 5402 bp, Corynebacterium cassirii
  source 1..5402: mol_type = genomic DNA
ttttgttgggtggttttgttttggttgggtttgggcttttcacggctcggtttcttttactgaaatgtttttgtggagagtttgatcctggctcaggatgaacgctggcggcgtgcttaacacatgcaagtcgaacggaaaggccagtgcttgcactggtactcgagtggcgaacgggtgagtaacacgtgggtgatctgccctgcacttcgggataagcttgggaaactgggtctaataccggataggaccacttcgttgttgttgtggtggaaagttttttcggtgtgggatgagctcgcggcctatcagcttgttggtggggtaatggcctaccaaggcgtcgacgggtagccggcctgagagggtgtacggccacattgggactgagatacggcccagactcctacgggaggcagcagtggggaatattgcacaatgggcggaagcctgatgcagcgacgccgcgtgggggatgacggccttcgggttgtaaactcctttcgccaaagacgaattttgacggtatttggagaagaagcaccggctaactacgtgccagcagccgcggtaatacgtagggtgcgagcgttgtccggaattactgggcgtaaagagctcgtaggtggtttgtcgcgtcgtttgtgtaagcccatggcttaactgtgggactgcaggcgatacgggcataacttgagtgctgtaggggagactggaattcctggtgtagcggtgaaatgcgcagatatcaggaggaacaccgatggcgaaggcaggtctctgggcagttactgacgctgaggagcgaaagcatggggagcgaacaggattagataccctggtagtccatgccgtaaacggtgggcgctaggtgtgagtcccttccacggggttcgtgccgtagctaacgcattaagcgccccgcctggggagtacggccgcaaggctaaaactcaaaggaattgacgggggcccgcacaagcggcggagcatgtggattaattcgatgcaacgcgaagaaccttacctgggcttgacatacaccggatcgctgcagagatgtagtttcccttgtggctggtgtacaggtggtgcatggttgtcgtcagctcgtgtcgtgagatgttgggttaagtcccgcaacgagcgcaacccttgtcttatgttgccagcatttggttggggactcatgagagactgccggggttaactcggaggaaggtggggatgacgtcaaatcatcatgccccttatgtccagggcttcacacatgctacaatggtcggtacaacgcgcagcgagcctgtgagggtgagcgaatcgctgaaagccggtcgtagttcggattggggtctgcaactcgaccccatgaagtcggagtcgctagtaatcgcagatcagcaacgctgcggtgaatacgttcccgggccttgtacacaccgcccgtcacgtcatgaaagttggtaacacccgaagccagtggcctgtttggggagctgtcgaaggtgggatcggcgattgggacgaagtcgtaacaaggtagccgtaccggaaggtgcggctggatcacctcctttctaaggagctttttttcaaaaaagtcctcacggttgtggggcgagtgtggttgaggtgccgagtgtgtacctgccatgttgattgtttccgggtggacacatgctgcacgtgcatannnnnnnnnnnnnnnnnnnnnnnnnnnnnnnnnnnnnnnnnnnnnnnnnnnnnnnnnnnnnnnnnnnnnnnnnnnnnnnnnnnnnnnnnnnnnnnnnnngccttgtatgggttgtggttgtggtgtgcgcggttgatcacggtttgcagtaatcacgtgtatcaaacaaaagttttttggtgttggcatgctgttgggtgtctggggcagcacagtggttgtgtgtccttgacttgcattgcttgcatgcgcgtttgtgtgtgtgggtgtgtgggtgtggtgtgtgagaactggagagtggacgcgagcattattttttgcttttttctttgtgtcttagtgtgcgcattgtgcatgccgtgtggtgtgtgtggtgcgttgtgattgtgtgtgtttgttgatcaagggcgtacggtggatgccttggcatgctgggccgatgaaggacgtgtgaggctgcgttatgcctcggggagttgccaacaaagcgttgatccgaggatgtccgaatggggaaaccccgtaccagttgtgtggtgcgacctgcaggtgaatgcatagcctgtatgggggttaacgcggggaagtgaaacatctcagtacccgcaggagaagaaaacaagtgtgattccgtgtgtagtggcgagcgatagcggatgaggctaaaccatgtgtgtgtgatacctgggtaggggttgcgcatgtggggttgtggggcaacagctcggtgggctacctgaccgccgcagcaggttggtgtgtgtaagcggaagcgcctgggatggtgcaccggagtaggtgatgagtcctgtacgtgaatgcgcatgctggtgttgtgttgttgttcccgagtagcagcgggctcgtggaatctgctgtgaatctgccgggaccacccggtaagcctaaatactcagtgtgaccgatagtgaattaagtaccgtgagggaatggtgaaaagtaccccgggaggggagtgaaagagttcctgaaaccgtgcgcttacaatccgtcagagcacctcaacgtgtgtgtgatggcgtgccttttgaagaatgagcctgcgagtcagcggcatgtcgcgaggttaaccaagtgtgttgggtagccgtagcgaaagcgaatccgaaatgggtggtaagtggcatgtcctggacccgaagcggggtgatctacccatggccagtgtgaagcagctgtaagaggttgtggaggcgcgaacccacttaggttgaaaactgaggggatgagttgtgggtaggggtgaaaggccaatcaaactccgtgatagctggttctccccgaaatgcatttaggtgcagcgtcatgtgagcttgccggaggtagagctactggttggttgagcgggactatcatcttagcaatgtcagccaaactccgaatgccggttaaagtgttgcatggcagtgagactgtgggggataagcttcatagtcgagagggaaacagcccagatcgccggttaaggcccctaagggtgtactaagtggaaaaggatgtgggatcgcgaagacagccaggaggttggcttagaagcagccacccttgaaagagtgcgtaatagctcactggtcgagtggttccgcgccgacaatgtagtggggctcaagtacaccgccgaagccgcggcaaaacattatgttttgggtaggggagcgtcgtatatggggtgaagcacgatcgtaagggcgtgtggactgtatgcgagtgagaatgcaggcatgagtaacgagagatacgtgagaatcgtatccgccgaatgatcaagggttcctgggtcaagttcgtcttctcagggtgagtcgggtcctaaggcgaggccgacaggcgtagtcgatggtgaacgggttgatattcccgtacccgtggtatcgcgaccaatgctgaagcaatgatactaaccacccggaactgtgcctgcctgcatctttgatgcgggtgggtgtggtgatgcgtggggcctgatttgtggtaggtaagtgatggggtgacgcagagtggtagccacgccagttattggattctggtgcaagcgtgtagcacggcatcttgtcaaatgcggatgccaatacagtgtgaggcgtgatgcgtagcccttatgtgggtgatggtggtgatcctgtgctgccgagaaaagcctctagcgatgtggtgtcacggcccgtacccgaaaccgacacaggtgatcaggtagagcatactaaggcggtcgggtgaactgtggttaaggaactcggcaaattgcccccgtaacttcgggagaagggggacctcactaggttcagagctaggtggggtcgcagagaagagaggggagcgactgtttatcaaaaacacaggtccgtgcgaagacggttaagttgatgtatacggactgacgcctgcccggtgctggaaggttaagaggacctgttaggtagcaataccgaagcggagaatttaagccccagtaaacggcggtggtaactataaccatcctaaggtagcgaaattccttgtcgggtaagttccgacctgcacgaatggcgtaacgactcccctgctgtctcaaccacagacccggtgaaattgcagtacgagtaaagatgctcgtttcgcgcggcaggacgaaaagaccccgggaccttcactatagcttggtattggtgttcggtgcggtttgtgtaggataggtgggagactgtgaagccgccacgccagtggtggtggagtcgttgttgaaataccactctgaccgtagtggataccttaaccttggcccatgatctgggttggggacagtgcctggtgggtagtttaactggggcggttgcctcccaaaatgtaacggaggcgcccaaaggttccctcagcctggttggcaatcaggtgtttagagtgtaagtgcacaagggagcttgactgcgagacttacacgtcgagcagggacgaaagtcgggactagtgatccggcacctacttgtggatgtggtgtcgctcaacggataaaaggtaccccggggataacaggctgatcttccccaagagtccatatcgacgggatggtttggcacctcgatgtcggctcgtcgcatcctggggctggagtaggtcccaagggttgggctgttcgcccattaaagcggcacgcgagctgggttcagaacgtcgtgagacagttcggtctctatccgccgcgcgcgttgaaacttgaagaaggctgtccctagtacgagaggaccgggacggacgtacctctggtgtgccagttgttccgccaggagcacagctggttagctacgtacgggagggataaccgctgaaagcatctaagcgggaagcctgttttaagatgaggtttcatttgaggttcccagaagactactgggttgataggccagaactggaaggtaggtaactacttcgaggtgactggtactaatacaccaacaacaaacaccaacaggtgacacaaacacaaaaaagcgaactgctgcgcgtccactttccggtatctgacacaccacaccagtggtcaccacaccaacccaatttggtgtgccccaacactgtgtcggtggttgatagcggcggggaaacgcccggacccattccgaacccggaagctaagcccgcccgcgccgatggtactgcacccgggagggtgtgggagagtaggttaccgccgacccaacaacaacaaaacaac

SEQ ID NO: 24 - DNA, 20 bp, synthetic construct
  source 1..20: mol_type = other DNA
gacgaacggatggtcgaagt

SEQ ID NO: 25 - DNA, 20 bp, synthetic construct
  source 1..20: mol_type = other DNA
cgaggcgatcttctacgagg

SEQ ID NO: 26 - DNA, 20 bp, synthetic construct
  source 1..20: mol_type = other DNA
tccactcgtccggggtgtcg